European Patent Application EP 4 722 390 A1, published April 8, 2026. Title: A compléter !!!!!!!!!!. Applicant: Laboratoires M&L. Application EP. The sequence listing filed with the application follows.

SEQUENCE LISTING (12 sequences)

SEQ ID NO: 1 - RNA, 1458 nt, brevundimonas massiliensis
  source 1..1458: mol_type = rRNA
ctgagagtttgatcctggctcagagcgaacgctggcggcaggcctaacacatgcaagtcgaacgaacctttcggggttagtggcggacgggtgagtaacacgtgggaacgtgcctttaggttcggaataactcagggaaacttgtgctaataccgaatgtgcccttcgggggaaagatttatcgcctttagagcggcccgcgtctgattagctagttggttgaggtaatggctcaccaaggcgacgatcagtagctggtctgagaggatgatcagccacattgggactgagacacggcccaaactcctacgggaggcagcagtggggaatcttgcgcaatgggcgaaagcctgacgcagccatgccgcgtgaatgatgaaggtcttaggattgtaaaattctttcaccggggacgataatgacggtacccggagaagaagccccggctaacttcgtgccagcagccgcggtaatacgaagggggctagcgttgctcggaattactgggcgtaaagggagcgtaggcggacatttaagtcaggggtgaaatcccggggctcaacctcggaattgcctttgatactgggtgtcttgagtatgagagaggtgtgtggaactccgagtgtagaggtgaaattcgtagatattcggaagaacaccagtggcgaaggcgacacactggctcattactgacgctgaggctcgaaagcgtggggagcaaacaggattagataccctggtagtccacgccgtaaacgatgattgctagttgtcgggatgcatgcatttcggtgacgcagctaacgcattaagcaatccgcctggggagtacggtcgcaagattaaaactcaaaggaattgacgggggcccgcacaagcggtggagcatgtggtttaattcgaagcaacgcgcagaaccttaccaccttttgacatgcccggaccgccagagagatctggctttcccttcggggactgggacacaggtgctgcatggctgtcgtcagctcgtgtcgtgagatgttgggttaagtcccgcaacgagcgcaaccctcgccattagttgccatcattcagttgggaactctaatgggactgccggtgctaagccggaggaaggtggggatgacgtcaagtcctcatggcccttacagggtgggctacacacgtgctacaatggcgactacagagggttaatccttaaaagtcgtctcagttcggattgtcctctgcaactcgagggcatgaagttggaatcgctagtaatcgcggatcagcatgccgcggtgaatacgttcccgggccttgtacacaccgcccgtcacaccatgggagttggttctacccgaaggcgctgcgctgaccgcaaggaggcaggcgaccacggtagggtcagcgactggggtgaagtcgtaacaaggtagccgtaggggaacctgcggctggatcacctccttt

SEQ ID NO: 2 - DNA, 1079165 bp, brevundimonas massiliensis
  source 1..1079165: mol_type = genomic DNA
ccgccaaggcgcccagggtcaggcacagctgccgctcattccccgccagccccacaaccacttcaccgcgcacactgttgaatcccactggatattgcgccatcttaagctctccttctattcgacttcgttcgacgggagtcctggtgcgcaccaaagtgaagagcttgctcagccccaagggtcgcctcgctccttcgccttactggcgccgtttggctgttctgctcacgctcaacatcgggctcaacgcactggcgcatttccggctcgcgccggaggcgttcctgctcgttgcgtcgtttcccatctgctggatgaccttctgcatcgtcgctcagcggctgcatgacttcggcgcggacgtcacgtcgatcatcctggcgtgggtcggcctcggcttgcttgcgggcattggcttcgtgatagccgccgccttcggtgcgcaccctcttgttctcggccttttgggtctaagcctctcccttgcaccccttggtttcctgatctggaccggtcttcaacgcggaacgcccttccggaatgctcacggtcggggtggcagtgcagcgccgggggctatgcccatgggtcagctcacgccctgaggtcagatcgcgctgaacccgaccgcgcccgcgctggccaggctgatggcgaaggtcgcctcgccctcgtgctcgcccgcatattccagcgccgacaccaggaacggtccctccagcacgccgaagtccggcacgatcagccgccaagtcttcgccgcctgctcgaaaaaggcctcgcggatcagcgcgtccgacgccgcgtcgcgaaagatcccctgccccgacaccgcagccgacttcacccccgccccggccagcagctcgcgccagcgcccggcgctgtccccgtccgtcgcatccaccgtgcgcgcgttcagcgagatcgtccgcgcccggaggcccgcaacggtggtgaacacccccgccgcgccctcgatcttcaacagaatgtccttgccgcgttgcgccgccatttcagtcgccctctccgctcgtttccgtcaccgcccgcacccgcaccaccgcatgggtccggcgccagtcgcccgttcggaacacgtcgctgaacaccacgcccaggctgaccgtgcgcaccccgtccgcctccagcaccgcgtcgttcagcgccgcccgcaccgcgctggcgaccgcccgcgcctcctccgttccaggaaatcgcgacaccgccgtcagcgtcagccgatgctcgatcccgcatccgtccgccgccaccggccggctctcgccgcgcccgatcagcaggcggggaaagccgccgtccgccggcggctggtcccacacgcgtgcaggctcgcccagcaccgcccggacgccggcgtccccgcgcagccgcgcgatcagcgcccgatgcaaggcgccctcatggtcgctcatcgcacccgctccagctccagcgtcgcccggcctggcgccctctcggcgtccacgcccgcgatccgccagtccgccccgccgaaccgcagcacccgaccctccagcaggcgggggtcggcgcgcgtctccgcggtcagcgtctccaccccgcgcggccctccatcagcgtccgcccgctcacgccgcctgcgcgccccgcacttcagccaggccgagccgaccggctcgaacgacacgctgcgcccgccatccggcgtccccgcctcctcggtctcgaacaggcccgccagcacccgcatgcccccgctcacagccgcaccacgcgatagggcgcgatccacgcctccaccggcccgatcgccatgtcgctctccccgcgctcataggcgcgcagcaccagcatcaggatcgccagcctcagcggcgccggcgaggtggacgtcaggctcaggcccacatccccctccacccgcgcccgagcggcctcgatgagggtggcgatcagcccgtcctccgccgcgtgctccacgcgcagaaacagcttcgcctccgtcaggtcgacgggtgcggtcatggtcgtctccgattgtcaggaaatcagcgggccgtccggcccggcccctctcccgcttgcgggagaggtggcccgtcgatcggcaaggccgatccagggtcggtgagggaagtctccgaggagactctccccatcgtcagccgtgtcgcttcgctccgcgaaccgacactccccccgacaagcgggggaagatcactcaggcgctgaacttcatcaccttgacggcgtcgaagttctgcaccccgccgccgacgcgcttggtggtgtagaacagcacatagggcttggccgaatacgggtccctcagcacccgaacccccgcccgatcgacgatcagatagccgcgctggaagtcgccaaacgcgatcgagaggctgttggccgccatgtccggcaccgtctcgatctccgtcactggatagccgagcagcgacgccgtctcgcccagccgcgccgccggctgccagatgtagttgccgtcagcgtccttgaacttgcggatggccgacaccgtgcggcggttcatcacgaaccgaccgttcggccggtactgggccttgggcgcatacaccaggtcgatcagccggtccgccggactgcccgcggcgaaaccgcccgccgcccccgacgccacaaagccgatctgaccccaccccgccgtcgcgtctgcaaccgtcggatagctcagaaagccgcgcggcttgttcaccccgtcgccattgacgaacgcctgcgtctcctgcgccgcaaaggcgtcctccacctcggcggccagccattcgtctaggtccagcagggcgtcgtccagcagcgcctgcgtcgccgccggattggcgtagaggtccgccgccggaaactccagcagcgccagcgtcgccggatccgtctccggccgcgccgccgtctcggccacccagcccgaggcgatcccttgcgtcgacaccggcttcctgaacaggccggacgccacggtcctgacggtggcgatctcgcgcatcggactggccgccatcagccgccgctcgatggcccgctcggtctcgggcggaaccacatagccgccggacgacgcgccccccgacaggcccgccttgacctccagcatctgcgcggccgtccccgtcttcagatagccgtcccacgccgacttctcctccccgtgaaacggggagggggaccgcgaagcggtggaggaatcccccagcatcgggcggcgcgtctccactccgatccgctccagccgcgcctgggcctggctcaccgcctggtcgatgcgcgcgaccttttcctccagcagcccgtccgccgccttccgctcgatcgccgccagccgctggtcgttggcgtccttgaacgcctcgaacgccgccagcatctcgcccatcacaaggcgcgcctccggcgaacccgccggggcctgtttggtctctttcatgatgtctccgggttgaagaaccgcgtgatgcggttaaggtcgggacgtgacgcgcacgagcccgaattttatggatgcgctccagcgctcatggctgctcaagctggtgtggctgctcgtcccattcgtgcccatcaccgccgtggctgccagcaaccattcggcggcaggtaacagcttcaacatcatttccatgctgccgactctgcttgttctaagcggtgcggcggttccatttgccatcgctctcgccgagatgccgacaaggcgggcgcggcgccgggcgctctcaccgctgcagcggatgcagatgtcggatgaagcagacgccatcaaccttgcggacgccttgagagttgctgaaaagccgcctgcgaactcgcttccccgcctccttcaagccgccatttttcgtttcgggaccccgacgcctcgtgcactctccggcttgatcgaaggtctgggcctcgtggttttgatcctggccagcgcgatggccttcatggacgatccgttaggcgatctctcccgctggatcggtcgatccctgccccttacatactggcctacctacgcgatcttgctagctacggccgtgggagtcgccgtgtggcggtggctgcgcgaaatgcatgaccattactccgccgtggccaacgcatccggccgctgtcccttcttggcgccgcagtagtcactcgcatcttcgggagcattctaagaacctcaacacaaccgagcgaacgacgtccgatccgctctgacgaaccgcgcccccggcagcatgggaaaggtcaccagcgacacttcccacagctccactccgctcagcacccgcaatcgcccgtcccgccgagcccttgcggtgcggtagccgatcgacagcccgtccagcgcacccgccctagccagcgcctccgccaggcgggacacggcggaccacggctcgatccggccgcgcacccgcaggccgcgctcgtcctccgccacgtcgtcccagacgccgaccaccgcaccgccgtcatggccgtgcagcatccgcacgccggccgcgccgcttcgggccaggctgtcgcgaaaggcgccgcgctgcaccacgtcgccgttcaggtcggccacgccccaaagcgacgcatagccttcgatcaccagaggcgtgctcatcgccgctccagccgctgttcgatccgctccacggccgcgcgcgtcgccacgccctgttcctccagccgcgccagccgttcggcgaccagccgctgctcgcccatgcgcgcctccagcgccccgatccgcgccgccgccccgccggcccagatcaggcccgccgccgtctgcacgatcagggccgccaccaccgcaggcggaacccgtttccactcgctcatcacgcccccaccctcgccatccgccggcgctcctcttcggtcaggaatgtcgccgcgttcagccgcgcccacagcgcgtcccgctcgggctgcagcgccggaaccgcctccaggtccggctccaccatgcaccctggaaacctctgccccagccatccggtcagcgcccccgccgccttgcgcaccagcgggatcaccgtcccccgccagaaggccgcattggcctcgcgatagttggcgtaggtcgcatcgcccggaatccccaacagctgcggcggaaccccgaacgccagggcgatctcgcgcgccgccgcatgtttcccggcgatgaagtccatctcggacgggctcaggctcatcgacttccagtccatgcccccttccagcagcagcggccgtcccgcgttcgccgcccccgcatggccttccgccagctgcgccttcagcgcctcgaactgttcggccgtcagccgctcgccgtcccgcgcgccatagaccagcgctccgctcggccgcgccgcattgtccagcagcgccttgttccaggcgcccgaggcgttgtgcacgtcgatggcgaaggccgccgcctccagcggcgaaaacccgtaccagtcgtcggtcgggtgaaacagcttcagctgcatcaccggcgaccagccgtcggcgcggcgcacaatccgggcctttcgcccgtccaccgcatactcccacgcctgcggccagccctgcggacccggaaccaccgtcatccggtcgggccggaggctccacagctcctccggaggcccgtccgcgtcgcccgtcgcctccagataggcgttgcccgccacctgcagcgcgccgtacagagcctccatcagctcggctcccgactgttcgggattgggcttggccagcagccgcgccagcggatgcccatcgtcgcgcaccccttccacgaacacctggaacggcgcggacgccgccgcctccgcgatcatccgcacgcagcgataggccaccgcatttcgggcgaacccctccgtcgccagcgagcgatagtcgcgcggtgtccaccgcgcccgccccacgtgcgaaaaggcgatcagcggcccggccgcgcttgccttgctttcgggcgcagacgcttgcgccgcctgaccgaacggccagcggattcccttcatccccatctccctggtttgttaaagcgagaccgtcgccgccatcagcgcgtagccggcgggcttcggatgcagcccgtcgccggtcagcgccccttccgccggcgccttccagcgcccggtcgctccgtcctccagcaccgccgccacatcgaacacgcccgcgaggtgcggcgacggccccgatctcagccaggcgttgatcgcctgccgctctgcctcgttggcgtaagcgctctgcccacccagcgtcgcccatccgtcggacgatgtggtgcgcggcgtcagcgtggtgtggaacacctccagcccccgcgcggccaagcccttccacagggccaagaggctcgcctgcacctgctgggcggtgcgtccgatcaccaggtcgttgatcccgtggttgcacaccgccgtcgtcgcaaagcgtcccgccagcgccattctgcggccgccgcctgtcacgatctgcgccgcctgttccgccggcatggccaggctggaccagccgcagcgcccgccgatcgcccgcacgacaaagcccgtgtcgttggccggattgtccgcctggcccgaggcgatgctgtcgcccagcaccaccaccgcccgctgcgttcccgccgtcagtcccgtcaccgccagcggcccgtagccataggcgaacaccgtcggcaccgtcccgctcgtcgtcaggtcggcccctccgcccgccaggttgccgccctctccgtcgcccggcaccgtggtcacgcccagcggccacttgcccccgctggcgaccgacacatgcgtccgcacccaggcgacggcgcccgccgggatcgagacgcccgcgccctcgtcgctttccgcctgcgcgcccggctcgatcaccgcctcgcgccgcccgccgaagaagaccggcgtcagcgtcccggccggatattcgatcgacgccctgaccgtgatcgcgttcggtcccgccgcctcgcccgccccgctgggcatgcgccagttggcgtagaccagcccgacgtccagcgcgtcctccgcacccacggtgatccgctgccgataggtggcggatgtcgccacgccgtccgacagcccgtttcgcaggatcacgccgcgcccggcgaccagccgccgacgcctcgcctccacctcgtcgcgaaaggccgctccggcgcctctcaaggtcacgaacccgctcatgccgccgcctccaccatcaccgtgcgcccttgatcatcggtcacgatccacccgtcgtgggtcaccgccgcgaatccctccggcgcctcggccgcgccgccgcgcgccgccagcaccccgccgggcgccgtgctcatcgcctccagctcgatcatcagtcgaacagcgccacgatctgcccggcgctcgtccccgtcgccagcacccgacgcacctgcaccggcagataccccgccggatggttggcgaagaccaccgcctccccgtccgccgcatccaccgtcagcacccgcacgttgccgcccgtccccaggtacagggcctttgcatacacaggcaggtcgccggcatcgtccggcgtcaccgcccgcgccctccgcgccggcccgcccgcgctccgcccatggttcagcagcccgtctcgatcagcgatcgccggcatcgtgtgtgtctccgtcttctctgcagttggtccaggccggttggtccaacccgcccgttgtgttaggttcgtttcatgacgatccaggtgaatatcgcccgggccaaggccacactgtccgagctcgtcgccatggccgaagccggtgaggaggtcgtcctcgcccgctccggcaagccggtcgccgtgatccgcgccgcctcgtccggacgaccgcatttccgcatcggcgccctggctcatctcggcccgctcaccgaccaggaagcgacggcgttcctgcagcccgaccccgagcttgagcgtctcgcccgcgccgaggacgaggatcatctctaccgttgagcggcgtcctcctcgacacccacgtcctgatctggagcctgttcgacaggccggaactcacgccatcggctcggcgccgcatcgatcccgatcggccgatctacgtcagcgtcgtcagcatctacgagatcgatttcaagcgcgcccgcgccggcgctcgttctgccgacagcttcctgcgggccatgccccgcgacttgccggcggtcctccccggcctcggcttgacgcttgtgccgctggacgcccgcatggcgcgcgcggcggcgaccctgccgatcgaccacggagatccttgggatcgcatcctcgtcgcccaagccttggcgctggacgtgcctctactgagcgccgacacccgccttcggatcgctgccgacgctcacgccgacactgccggcgtcgtcgtcttctagcctgcacctctcctccccatcgctgcgcgacagggaggacaatccgtcacagcacccgtatcctcggccctgccttgcgtccgttcagcatcagcgccgtgaccgcccagaccagcgcatccgctcggtccgggctcgggccgccgtctgcggcccccagcgccatcagctcttcctccagctgcggaaacggcccgcagtgcaccacccggccctgttcatacagggccgccaccggctcggcccgcgccgccttggagcggctggcgtgcaccatcttcacctcgaccgaacagcccgcctggaccagcacgttgcgcaccatgtccccgccctggttgccctcggcgatcaccgcatcggcctcgaactctcgaaccgcccgcacgacctcgcgcgcccagcccagtgggctcagcccccgaaccgtccggtcggccagcacaaagacccgctcgtccctgcgccccgccaccacgatgccgcaggcgtcgccgcccgccgtggccggcggatcgaccgcaaccactgtccgctccagctccgccggacgcgcgccccgcgcccgcttcagatcctcgaccctgaacagggcgccgtcgctttcgaccagcacgccctccatctcctgcgcctccagccgtgtgccgccgtacagcgccttcagatgctccaggaagccgggcgccaggttccgggcgttcagccccgtggccccgcgatccagcaccagcccggcctccgccatcagccgccgcagggccgccgtcggccggggcgtcgtggtcaccgccagccggggcgcatcccccagccgcagtccgaaccgcaggttcgacagcaccagctccggctgtctccaggcgcagaactcgtcggcccaggccgcatggaactgcggccctctcaggctgtccggatcctcggccgaaaaggcgtaggccgccgatccgttcttccacaccagcctgcgccgccccgcctcccagcgcggccggtcgcccggaacgccgaagctcttcagccccgacgtcccctccaccatcacctcgcgcacgtcgtgcagcgccggccccaccagggcgaaggtccgcggcgtctcccgcgccagaaagtcgatccaccaggaccccgcaaacgtcttgccggacccgcgcccacccagcagcagccacgtccgccagtcgtcacccagaggcgcaatctggtggtacagcagccccgactttctgtgctcgatcgcgagcggctcgccgctcagccgcttcagctcgcttctgttcaagcatcccttcgagctgatcatagcgctcggcggtctctcgacgcagccgctcgtctcgttcgggatcgtcgtgtccaccggtcatctcgtcctcgtcttcgcgtggagaggctgtgcaggcgcggcgacgcaggtcgtcgacgaacttggccgtgcgcgcgatcacgcccacggtccgcatccgcttctccacctcggccgtgttggcgggcttgtcttcggcgaccagcacctcgacgctctcgtccaccaccgccttcagcacgccgaacagcccgcccagccacccggcgccgtcgtccgccgcccccgccctgtccccttttcccgccatgcccagaacataccggaccagcgtccccaggcgcgcagatcgccgcgagaaaagcccaagtcattgacgatgttcatcttccaccagcgtcattgcgctggcggccacgcgatggtcagcagccgcgctccacggcccattcgggcgcctcgaagtccagcgcgtcctcgggctcggccagcgacagctccgagatcgtctggtccttcaccgacacccccgccgtgtgcaccgtgttccggtcgcccgacaccaggtggtgccagcccgccagatcccggccctcgtggatgcggcgataggcgcaggacctgggcatccactccagcgcctcgatgttgccaggcgtcagcttgatgcagtccggcacatgcgccttgcggttcgcatagtccgagcaggcgcagaccttgggatcgaacagcttgcagtgcacccgcgtcgggatcacctcgccggtgtcctcgtcctcgaaccggatcacgcagcacagcccgcacccgtcgcacaggctctcccactcggcgggagacatctcgtccagggtcttggtccgccagaagggctgcatgttccgcctcttagcgcccgatacgggcgaagtcgcggcgcatcccgtattaccgcatcgtaatcttcacatgcgcggttcgcctgctacggtcgcctcagcccaatccgccgccggaagcccgatccatgaagcgtctcgccctgctgtccgcctcgatcctttcgctgaccctcgccagccccgccctggcccaggtcgcgtccccgccgtcgctggacgccctgacgcccgcgccgcttcagttcacccaccgcacgctagccaacggcctcaacgtctacgccatgcccgatcccacagccggcacggtgacggtccaggtctggtacgacgtgggcgccaagaacgaccccgccggccgctctggcttcgcccacctgttcgagcacatcctgtcgcgcaagacgatcaacatgccgctgggcaccatgaacgccctgaccgaggacgtgggcggaacccgcaacgcctccaccggtgccgacttcaccaactactacgagaccgtcccgccccagtatctggagaccatgctctggacccacgccgagcgcatggcccgcccggtggtggacgaggccgtgttcaaggccgagcgcgacatcgtcaaggaagagctgcgccagcgcgtgctggccccgccctacggccgcctgcagcgtttcgtgatcggcgacaacagctacgacacccacatctatcgccgccccaccatcggctccatcgaggacctggacagcgccacggtggaggacgcccgcgccttccatgaggcctactaccgcccctccaccgcgaccctgatcgtgtcgggcaacttcgacccggcccagctggaccgctgggtggaccagtatttcgcccccatcaccgccccgaccgaccgtccggtgccgcagatgacgcgtccgcccgaggtgcgccgcaccgagccgcgctcggtcgtggcctacgcccccaacgtgccgctgccggcggtcgccgccgtttggcagggcgtccccgcgaacagcccggacgctgcggccctcgacgtgctggccggcgtcctgtccagcggcgaatcctcgcgcctgtaccagtcgctggtctatcagcagcaggtcgccgccagcgccagcctctacagcggcgcgcaggaagaaggcggctccatcgtcgcccaggtcatcgtcgccgacggcaagacgccggaccaggccgaggccgcgctgaacgccgaactggcgcgcatccgcgacacggccgtcaccgaggccgaactggccgaggccaagaccgaaatcctcgcctccgccctgcgcagccgcgagaccgcctcgggccgcgcctttctgctggggcaggctctagtcagccggaacgacccccgtgcggccgacaccgacctcgccgccgtccgcgccgtcaccacagccgacgtccagcgcgtcgcccgccggtatctgggcgatcagggccgcgtctccatccgctacctggacgaaagccagcgcccggccggtcaggccgacgcctgggccaatcccgcgcccctgcccgagttcatcaccgtgccgccggcgctgaacgcgcccaacgaactggcgccggaaggccggcgtcaggcggcgccggcgccgtccgccccggtccaggcccgcccgccggtgatcgccgaacgcacactgcccaacggcctgcgggtggtcgtcgccaagtccaccgacctgccgatcatgaacgcccagctggtgacgcgcggcggctcggccgccgacccggccgagcgctcgggcctgtcggccatgaccgtggccttggccggccagggcgcggggggacgctcctcgaccgagatcgcccgcacgctggaggccctgggcgccagcaccggctcgggcgccggccgcgacagcacctcgcttgtgctctccgcccccgtcgcctcggccgatgcggcgggtgcggggtttcgcgacatcgtcaccaccccgaccttcgcccccgaagagctcgagcgcctgcgcaaacagtccatcgacggcctgcgggtcgagctgcgacagcccggcccgctcgcctcggccgccctgcgccgcgtggcctttggcgacggcggctacggcgcgcccgcgcgcggcaccccagcctcgctggcggccgtcacccgcgaggaaatcgccgcgctgcacgccgcacgctggcgccccgacaatgccgccctgatcatcaccggcggcatgagcccggaggaaggcttcgcctacgccgagcgcctgctgggcggctgggccaagcccggctcgcccctgcccgtcctctcgccggccgcttcagccgccgccaaggcgacgccgcgcgtggtggtcgtggacctgccgggctcgggacaggccgccgtcgccgccgccgtgccggcgccgctgcgcaccagcgacgactggtatcgcctggccgtcgccaatgcggtcatgggcggcggctccaacggccgcctgttccaggaggtgcgggccaagcgcggcctgtcctacggcgcctactccagcctgggctcgggcgcctcggccgacctcgtcaccgcctccacccagaccaagaacgaaagcgccgccgaggtcgtggacctgatcctggccgagttcgaccgcctgggcgccgaggccgtggcggccgacgcctccacccgccgttcgacctatctgaacggcggcttcgcccgtcagatcgagaccacggcgggtctcggcggcttcctgtcggacgcggtcgaatatggcctgccggtcgacgacgtcgccacctatccgcagaagatcgcggccgtgacgcccgagactctgcaggccgccgcccgccagtacgtctcctccgaccgcgcctatgtggtggtggccggcgattccaaggtgttcatcgacgccctgcgcaccaagcacccggacctggtcgtcgtcccggccgccgacctggatctgtcacgcgcggacctgggcgcggactgaggctccgcctggcggcgacgggtcacaggcccgtcgtcgccatccgagcccgggcgcgctcggcccgcacgccgcgccggcgcagataggtcgtgatcccgagggccagcccgaccgccacgcccaggaacatcgcccccagcgcgccgaacaccgtgcccaccaggccgcccatgaagtcgtggcccaccgcgatgaccgtctgcggccccgcggcgccggcatagtctgcggcgacgacgtaggagcctgcggtcgctacatcgaactcctggatcgactggccgctgcgtcccccaaagctgtagttggcgctggcgccgggcgccctaagcgccagcggccgcccctgcgggtcggcgacccgaacctgaaggcccgacacctcggcgaccgaaaaggccttgccctcggcgacgcttgtcagctccaggaacacggtctggcgccccggctccagcatcagggtccgcgatcccggaaccacgatctgctccaggccatcgtccagcttggtgatctgcgtcgccaggatcgccaccatcgttgcgaccccggcgagaatcgccgccacccccagcccgtatccccagcgcccgggcgcccgcttgtccgccgtcatcaccgtctcccccagccgcaaccatgttgggcgattacatcgcgccggacgccgcctcgtcaaacgcgcccgatggcccccggccggcgcagtcgctatatgcccgcccatggcagcccgtccccccctcgtcgccctcaaggacgtccgtcttcaggacgggccccgcccgctgttcgacggcgtcgatctggcggtcgagccgcgctccagagccgccctggtcggccgcaacggcgcgggcaagtccaccctgatgaaggtggtcatgggcctgatcgagcccgacagcggcgatcgctcggtccagtccgcggtccgcttcgcctatgtgccgcaggagccggcgattacgggcgccacgctgctggattacgccgcctctggcgaggcggaatcctggaccgccgaggcctggctgaccaccttcggcctcgaccccgccaagtccacgcagggcctgtccggcggcgagacccgcagagcggcgctggccaaggccttcgccgaagagcccgacctgctcctgctggacgagcccaccaaccacctcgacatcctggctatcgagctgctcgagaacgagctcctccaggcccggttcgccgtgctggtggtcagccacgaccgcgccttcctgaaccgcgtcaccgacacggttcactggctggagggccgccgcgtccgaaccctgaacaagggcttcgtcgaattcgacgactggtccgccaaggtcatggaggaggaggccgagtccctgcgccgcctgaccaagaagatcgaggccgagacctacaccttctaccgctccatcaccgcccagcgcacgcgcaacgagggccgcgcccgcgccctccaggccatgcgcgccgaccgcgccgagcgggtcaaggatctgccgcgcgagctgaacctcggcgtcgattccggcgccctgtccggcaagctggtggccgacatcaagggggtgtccaagagcttctcccctcccccactgggggagggggaccaggcgcagcctggtggagggggccaaccccgcaccctgttcaagaatctcaccacccgcatcatccgcggcgaccggctaggcatcgtcggcccgaacggcgcgggcaagaccaccctggtcaaggtgctcctgggcgaactcgcgccagacgagggctccgtccgcatgggcgccaacctcgagcctgtctatctggaccagtcgcgcgaggggctgaagtcggacatgaccctgtgggacgcgctgacgcccggcggcggcgactccatcctggtgcgcggccggtccatgcacgtcgcggcctacgccaaggacttcctgttctccgaggcccagctgcgccagccgatctcgaccctgtcgggcggagagcgcaaccgcctgctgctggcccgcgcgctcgccaaacccgccaacctcctggtcctggacgagccgaccaacgacctggacatggacaccctcgacaagctggaggagcttctggagggctacgacggcaccctgatcctggtctcgcacgaccgcgacttcatcgaccggctggccacctccaccctggccctgaatggtcgcggcgccatcgtcgaaacccccggcggctggaccgagttcgtgcgccagaacccgggcttccttcagcccatcgcctcgtcctctccgatccgggaagcagccggcgagagcgccaaggcgccccagccgcccgccgccccgcccaagaagaccgccaagctcacctacaaggacgcccgccggctggaggagctcgaacgcctgatcgaaactctccccgccgaaatcgcccgccatgatgcggcgctggccgacccggacctctacagccgcgaccccaaggccttcgaccgcgccatgaccgccgccgcccaggcccgcgccgacctcgaggccgccgagatggaatggctggagctggaggagaagaagtcggctctggcgggctgatcgtcgtgtacccgtggtggacaaatcccacggctttgctccaagctgcgactgcatgggcgacaggagcggcgggtgcggaccatcgcgatcatcacggcgattacgggaacggcgttcccaagtttcgcacaggtcttgccgccaccacccgtgctgacgcatgggccagcgtcatcatcgcccgccttgattctgcttgacccagtggccgagacgacctgcggggacacgcccattcagcccgcctatcgcgaggacctgccgcctgtatctgcttcggaaggacctgaagggcctcaaacaagcgtcttccggttcgcggtggccgcggacggccgcacgcgtgacatccgcccggatggaaccgggggatcttcctataactatgcgaacgcttcgcgcggcgtaacggtccaggccaatctcgccgcctggcgcttcgacggcggggcgcgaagcgactgccgcctgaccgtcacctaccattccacgcggatcgaggaggcttcgccgtcgctgctgatgcgctactatgcggttactcgcgaccgaggcccgttgcgcgacgccgccgcacgacgcctgtctggaccgagcggcaactgcatgagaccggatcggccccgtcggcgaccccagacaaccagccaccccgacttcgagctcggccagcgcccgccacccggcggctacgcctggaccgtggtgcgctggaacgtcgacgccgccggtcgctacacggatatagagacgctgggctcgtcgggcgacgcggtgttcgacatggaggcccgtcgcgccatgggcgacagccgcctgcatccgggtccgccggccaccggctgcgtctacaacttctaccgtgcgggtccgaaccttccggcgccccccatcccgccaaaagaggagcgggaggatccgctgcagcagtgccccgacgccatcgccgcccggctgtctccggtgcgcgagttgccctatccgccggccttccgggcgcgcgggatcgaaggctgggcgctggtgcgtttcgatatcgcgtcctggggtcagataggcaatgtggcggtgctggaggcccagccggctgccgtcttcggcgaggcggcgcaaagcattgtcagccagcgccgcgccacaccgggcttcgaaggcgccattcgctgtgtccagccggtacactatcgcatgggcgcggacctcagcgaggatccgttcgacgagaccccggaacgctgaccgcctttccaccggcgccgtcgccgcctaaacctgcgcgatgagccatttcgggaatcgtcgccttgcggaccgccgacaggccctgttcggcggcgcggctctggcgctggggggagcgctgggcggcgcgggtctggtcgggtgccggcgggtcgaggcgccggtggacgaacagggtcgggtccggctgcgggtcgccagcgacggtccggccgaggcgcggcacggcgccgtctatgcggccatcgcctccggcgcctacgagaggcgcgggctgaacatccagatcgtggcgggcgactccgtcggcgacgccgcccagcgtctggcgcgcggcacggccgagctgggcatggcctcggacggcgcctcgctcttcgccctggccgccgagggcgctccggtgcgggccgtggccgcctttttccagcgcgatccggccgccctgatggtgcgggacgtcccgggtctcgacggcctgtccgacctgaacgaccggccggtgctgctggcccaggccgcgacctcgcccgcctgggcctggctgaaggcgaacgccggcttcaccgacgcgacgcttcagccgttcgccggcgacctgcagccgtttctcgacgaccccccggccgtgcttggcggcctggtcaccagcgacccctatcggattcagcgccttggcgggttcgagccgcgcacccttctgctggctgaagaaggctatccggcctacggcggcctggttctggcccccaacgccttcgcccgcgacaacgccgaggcgcttcgatcctttatcgccgccacggccgagggctggcgcgactacatgcgcggcgacccatccccggccgacgccctgatccggcgcagcaatcccgacctcagcgagcccgccctgaccgccgcgcgcgaggccctgcgcgacaacggcctggtcgacggcggcgacgccgccctctatggcctgggggccatgaccgccgagcggtggcaggcgttctttgacatggtatcccaggcggggttgacgccgaccggcctgaactggcgcgatgcctttacggacaactacctgcctggtcgcggctgaattttcctccgttagcgcaggattaagcgcgacggtttagtccggcctctcgacccgtctgcgcggagagagaaccgtcgtgcgccacgccccgtcccgacttccggcccttgcgaccgccgccgtgctcgccggcgctctgatcgcgccgtcggcccaggctcagaccgcgcctgcgtcttccggcgaggtcgcggggctccgctatctgtcctggcccggcaaggcggtgcgccagactccggcccgcgtcgtcgccggctcgaccccgtccccccgcgcctccgcgctctccgccccgcagccggtcgagaccgcctcgacgcgacccgaggcctcgccgcgccagggactgacccccgccagcgccttctacacccccggcgcctcgctgggcggccgcttcggcgccgagccggcgcctgcgcctgcgcccatgccggctcccgcccgccaagccgcgtcggagccagagcctgaacctcaagccgcgcccgagccccggatgcgccgcgtggcgccctcgccccttgaggccgcctcgacccacgcctcgccgcccccagcgcctgtcgctcaggtccacagcgccccgcttccccgcgatccagccgtcacggctccgacggccgagacagatccggcgccgaccgaagccgcgagggtcgccgatcccatggctccgcgccgcgatgcgccaatcttccgcctgcagcgtcagaccgcgcccgcgcctgcgctcgccggagcggaggcttcccaggcgacgccgtcgacggtcgagccggccgcatccggcgcccgctactattcggtgcatcgccagcacggccagcgccccgacgccatcgccgcgcccgaaccggcctggctggacgcgatgccggttcagctggccatcgcaccggcggcctcgacgaccgacctcgccgccccgccggccgcgcccgccctgcgccgcgacgcctccggcaagctgcagccggccgcgcccctggtaagcggcgacccgtcatgagcgacaccctgaccccgccgccccctgtccaggccgcgcctgtcgtggacggctcgcgcctgcccgacctgatcgccctggccggcgaagcgtccagcgacaagcgccggctgctgctgcgcgagctgaccgaccacttctttggcgcgcccaaccattcggcgacggaagccgctctttatgacgcggttctgtccgacctctccgccgagatggagaccgccgtgcgcgccgaactggcgcagcggtttgcggagacgccgcaggccccacgcggcctgatccggcgtctggcccgggacgagcttgaggtggccggcccgatcctgcgcgcctcgcccgtgctgaccgaccaggacctgatcgacgtcgttcagtcccagggccaggggcacctgcgcgaagtctccagccggccgcatgtgtcggaggccgtatcggacgccattgtccggaacggcgacgacgagacgctgggaaccctgctgcgcaacgacggcgcccagctgtcgcgcgccgccaccgaaacggcggtggagcgcgccaaggccaatccggccctgcacgcctcgacggtggagcgacgcggcctgcccgccgacctgctgaacgagatgtatttcgtggtcgaggcccggctgcgccagcagatcctcgagcagaacgcccggctagatcccggcctgctggaaagcgccctgaccgccggccgcgtacgcgtcgccgccgaggacggcgccctgccggccgactacgccgaaagcctggcctatgtggaggagctccgggccgccggacagctgacgcccccgacgctggcccgcttcctgcgctccaacggccgcaccgccttcgtcatcgccctggcgcagctggccgatgtcgacttccacaccgccgcccagatcatcgagcggcgcgaactggacgccctggccgtgatctgccgcgccgccgatctggatcgcgccctgttcctgacctatgcggtggtgctgttgaacaccgagcgcgacgccatgacccgcgcgcgcggctacgccgccatgtacagcgacctgacccgcgaggccgcgctgcgcaccctgcgcttctggaagctgcggcgaagcgcgggcgcggcctagcgcctccaccacgctgacgcgcggtccccctcccccagaagggggaggagtttagtgcatccgcttacttcttcgcgcgaccggcgccggccgtggcggcgcgggcgggtttgcggccgccctggcccaggcccatctgcttggccagatccgagcgcgccttggcgtagttcggggcgaccatgggatagtctttggcgagaccccacttggtccggtattcctcggggctcatgtcgtatttggtgcgcaggtggcgcttcaacgacttgaacttgcggccgtcttccaggcagatcaggtaatccggcgcgatcgacttgcggatcggcaccgccggttccttgggctccggctcaggctcgacagcgccggtggtcacttgcgacagggcggcgtggatgttggcgatcagcgacggcagcgtctctgcggacaccgtattgttgccgacgtaagccgaaacgatgtcggcggtcatttcgagcagttcgggcttttcgtccatgcggatcgtctcacctgttgagttgcaaggtgcgactggtgaatatcagccgccaagacttcgccctctaaggacgttcgccggcgaaagcaacgcatcacgcctgtttcagtcgttgtttcccaccggcggcgcaatcctcgcgctatacgaccggcgtggtcagcgtccgaagtcttgcgccagcgccatcatcgccgcgcgctggggcgcggaatattcatccaccgcctcgtcctcgccctgccgtatcgcgcgaagaagcgtgggcgtcagcgccgacgacagcgaccagttccagtatcgcagaacggtctgagcgcgatcgacggcgagcatttcataggtgacctgcacccgctcccagtcgggatgcacctgaccgtcggccgttgcttcgggtcgccgcatggaccgccagaggttcagcagatcggcgcggcccaagccggtcgccttacacaggatggcgagtggctcgccgcccggatcgcccaggatcttggccccggtcagcggcttgatgcccgccagataagcgatctcggacgcggtctcgcgcgtcaggccgttctgcccggcatgggcgaccgcggcttccaggtcgtcgaacgggctcttggcgatggcggcgcggttgcgctggcgccgctcgatgaactgcagggccttgcgcgagacgggatcggcccagccttcgcgcgcggccatggcgaagacgtcctccgacacctcctgcatcacctcgcgcgagacggcgaaccgctgcaggatggtgcgccggtcctccggcccacaccaccagaacatcacataggcgccggacggccgcagttccggccgcttcagcagcgccgtgcatagggacggcgtctgacggctgacgcccaccaccccctccaatcccacctgcgacaggcgggcggtcgtgttgcgcagcacgcactcgatcacggccgtctcgccgaacgagaacagcgtctcggtcaccacctccgacaggccgcgccggccggccatggcgaagcgatgctccggtcccgcatctcgggcgcacgacaccaggtcggcgtcggtcagggacgcgcattgttcgatcaacaaacccgcgatctcgggctcgtcgcgcagcagcatccgcgccacgctgttgggcagttcggccaagggcgccaggcgcgccgcgacccggcggcgctcctgcggcgcggccagccgcagcatctcgaccagcagatcgccggtgaccgagcgctcgaatgcgttgatgcggctggcgggcagcgacaccacgtcggccaggcgcttcaacagggcgtgacgcgccttgaagcgctcggcggtcccgccgccctcctcgcctgtcgccgccacagcatcgctcatggtcgacgacgctaacggacggcggttaacctgcggtatgcgggcctacagcccttcgaacagcgccgtcgacagatagcgttcggcgaaggaggggatgatcaccacgatggtcttgcccgcgttctcgtccagcgcggccaggcggtaggcggcgaccagggccgccccggaggagatgccgaccggcacgccttccgtgcgggcgaccttgcgggccatgtcgaagctgtcctcgttggagacctgctccaccccgtcgatcaccgagcgatcgacgatggagggaacgaagcccgcgccgatgccctggatcttgtgcggtcccggctcgccgcccgacagcacgggcgaggccgtgggctccactgcgatcatccggagcgagggcttgcgggccttcaacgcttggccgacgccggtgatggtgccgccggtgcccacgcccgcgacgacgatgtccaccgccccgtccgtgtcgttccagatctcctcggccgtggtgaccttgtggatggcggggttggcggcgttctcgaactgcgacgggctgacggcgttcggggtcgaggccagcagctcctgcgcgcgggcgatggcgcctttcatgcccttctcggccggcgtcagctccagccgggcgcccagcagcgccagcatcttgcgccgctcgatcgacatgctttcaggcatgcacaggatcaggcggagacccttggcggcggcgacaaaggcgagcgcgatgcccgtgttgccgctggtcggttcgatcagcacggtgtcggcgtcaatgcgcccctgcgcctccagcgcctcgatcatcgccacgccgatgcggtccttgaccgaagccaccgggttgaagaactccagcttggccagcaccgtcgccttggccccgtactccgccgacaggcgcggcaaccgcaccagcggcgtgtcgcctatggtgtcgacgatggagtcatagaccttgccgcgccccgacttgcggtggcgcgaggcgtcgtagtcggccccgggccgggcctggactttggcttgggcggcggcgtcggtcatggctttaagtctccgcgggcgtttcgtatcgccaacagataaggcctcaggccacgacgcaagggccggacggcgatgatttctgtcgccgcccttcagatttccgcgtcagctgcgtgcgaaggcgagcacccgcgcctgcgcctggtgcacgggcgaggacgaggtcgagaggtcgtccgacaggcggaagcgctcgatcagctgcgccaggccttgcgcctcctgtgtcagcgaatggctcgcggcggtggcctcctcgaccatggcggcgttctgctgggtcacctggtccatctggttcacggcggtgttgacctccgccagggcggtggcctgctcctgcgtcgaggcgttgatctcggtcatcagtccggtgatgtcgccgatgcggtcgacgatgccggtcagcgaccggcccgtctcgttgaccagggccacgccgctcttcacctgggcgccgctttcggaaatcagcgccttgatctccttggccgcctcggccgagcgctgagccagggcccgcacctccgacgccacgaccgcgaagccgcgtcccgcctcgcccgctcgcgccgcctcgaccccggcgttcagggccagcaggttggtctggaaggcgatctcgtcgatcacgccgatgatctggttgatctgggtcgaggactgctcgatcgcggtcatggcggcgaccgtgcggcccaccacctcgccgctcgcctcggcgtcccgccgcgcctgctccaccacgccgtgggcgcggtttgcgttcgcggccatcaacttcaccgtcgcggtgacctcatccagcgcggcggcggtctcctccagagtggcggcctggcgctcggtgcgccgcgacagatcgtcggaggcgtggctgatctctccggccccggcgcggatggcgccggccttggtgttgatcacgccgatgtcgccttctagctgacccatggcggcgttgaagtcggccttcagctgagcgtagcggcccggcatgtctgcgttgatgcggtgcgaaaggtcgccgctcgccaaggcgctgagcccccgccccgtctcggcgaccaccagcgtctgcagctcggcggccgccttgtccgcctcggcccgacgctcgcgctcgatggtggcggccgtcacgtccgtggcgaacttgatcaccttgcagggctttccgtccgcatccaggatcgggttgtaggacgcctcgatcaccacccgtcggccgccctcgccatagcgggtgaaggtgtcgacgaagaactcgcccgcgttcagcctgcgccagaactcgccataggccgggctcgacgcctccgccggatcgatgaacatgcggtggtggcgaccctggatgtcctccagccgatagcccatggtcgacaggaagttcggattggccgtgcggatcgtgccgtcgaggtcgaactcgatcacggcctgggagcggtgaaccgcatccagcacgctgcgttgttcccagagttgcgcggcgtgttcggcgttgcggcgctttgacatgaacatgtcggggtcctgattcttctatccggagagtcttatgccgaaccgccttccgggcccgtaagggttggttagcgcgctattatccgcatccgaaaccgcaaaggttcggtcactacggtgttaggcagcgcaaacggcgtcgcttgcgccgagttccagtccgaagaagcccaacgtgcctaaccgctcattcaccaagaccgacgtcgccgacatgcaggtggagccgctgaagctcgccatcgccttctccatcatgctggtgggccgtcgctggaaggcgcgcttcgcccacctggtcaaaccatccggcaacacgactgctcggatgggcgctctctactacctcgccgaggcgcccaagggtctcacccaagccgagctttcagagctgctgaacatcagcccggccaccctgacgcggttgctggacggtatggagagccgcggcatgatcagccgccgggccctgatcggcgaccgccgcgccaagctggtgttcatcgaagatcaagggcgcaaggacttgaccgaactggatcaggtcgcgggcgaattgcgcgaccacctgctcgatgaggtcgaagaacaggacctgcgcacgacgcttgccgtgctccgaaagatcgaaagccgtttgcgtgaggacggctccgccgacaccggcttcactggccgttaaccacgacgccgccaaaggttaacggccctgtcgcggccggagaccttcccccttgcgcaacctgatctccgccgtcgaagcgatcgatccgctggtcgtgaccggcaaggtcgcgggcgtgaacggcctgctgatcgaatcgcgcggcggcctgtctcgcctggccgtgggcgcgcgagccgagatcggacggcgcggcgccgagcccctgccggccgaggtggtgggctttcgcgacgccaaggcgctgctgatgccgttcggcccggtggagggcgtcgcgcccggcgccgacatccgcatcatcgacacggcggcggccgtgcggccgaccaccgcctggctggggcgcatcatcgacgccttcggcaatcctatcgacggcaagggtccgctgccgcaagggccgcgccctacccccttcgcgccgcacccccgccgcccattcgcgcggccgggtgggcgagcggctggacctgggcgtgcgcgccatggacgtcttcaccaccacctgccggggccagcggctgggcatcttcgcgggctctggcgtcggagtcggtgctgttgtcgatgctggccaaggaggcgacgtgcgacgccgtggtcgtcggcctgatcggcgaacgcggccgcgaggtgcgcgagttcgtggaggagaccctgggcgaagagggcctgcgtcgcgccgtggtcgtggtcgccacctccgacgagccggcgctgaagcgcaggcagtccgcctacatgaccatggccatcgccgagttcctgcgcgaccaggacctggaggtgctgtgcctgatggacagcgtcacccgcttcgccatggcccagcgcgagatcggcctggctgcgggcgagccgccgaccaccaagggctacacccccaccgtcttcaccgaactgcccaagctgctggagcgggcggggcccggaccgacccggccggacggcaccacggctgcgcctatcaccgccctgttcaccgtgctggtggacggcggcgaccacgacgagccgatcgcggatgcggtgcgcggcatcctggacggccacatcgtcatggaccggaagatcgccgaacgcgggcgctttcccgccatcgacgtgctgaagtcggtcagccgcaccctgcctggctgccagaccccgcccgagcgcgagctgaacaagcgcgcccgccaggccctgagcgcctacgccaacatggaggagctgatcaagatcggcgcctaccgctcgggcgccgatcccatcgtcgaccgcgccatcgccctgaacccggcgctggaaggattccttggacaggacaaggacgacgccacgcctctttccgaatcctttacccggctcgaggcaatcctgaaccaaggcatgatcagggagtgatgacgtagaatgaccgcttgggcccaatccctgatccgcatctccaactatgaggtcgagacgctgcaaaagcgcctggccgacatcaacgaacgccgcgccgccgccgagatgaagctggccgtcctcgacgccgaggccgagggcgagcgggaacgcgcccgcatcgacgccgacgccggcctgatgctgtcggcctatctgaacggctggaagaaccgcaagaccgccgccgaaggcgcgctgacgaccctggccgccgaagaggaaggcgcgcgcgaggccctgaccggcgccttcgaggagctgaagaagttcgagcacgtcgccgaggcgacccgcctcgaccggctggtggcgctggccaagcgcgaaaccgccgcctttgacgaacaggccctgcgccggcgtgcggtgtagcctcttcagatcttccctctcagggggaagtgtcgcgtcctcgagcgtagcgagagcagcgacgatgggggaagtctcccgaagagaactcccctcatcgaccctggatcgctgcgcgatcgacgggccacttctcccgcaggcgggagaaggtcgatgatcgaccgccgcacaatcctcacggccatccccgcccttgccgcgtgcgaccggctggcggcggctgaatccccgccggtcagcgcgccgccgctgaagtccgtctctcccgccccgttcgggacctgcatccaggccgggcacatcgacgatcccgcttgggtcgaactcgcccgcgccaacgtctcccagctgacgccggagtgggagatgaagatggagtacatcgccgccgacggcctgaacgcgccctatcgcttcgaccgcaccgaccgcatcgtcgacttcgcccgggccaacggcatggccgtgcacggccacacactgatctggtacgcgcagggagaagatctggtggcgggtctgtccgggcctgatttcgaccgggtgttcgacgactatgtcgccgcggtcgccggccgctatcgcggaaagctgcggtcctgggatgtagtcaacgaaccgatcaccgacgacggcgccggcatgcgcaactgccactggagccgcgagtacggcgcggacggctatgtgctgcgcgccttcgaaaaggccaaggcggccgatcccgaagccgtccttttcctgaacgactacaatctcgagaacacgcccaggaaaggcgccgagttcctgcggctggtggagcggctgctcaaggccggctgtccgctggaaggcatcggcacccaagcccacctcgacatcgaggttccgcccggccagatcaccagcttcatgcgcgaggccgcccgcttcggcctgccgatccacgtgtccgaactggacgcttcgctgcggagcggccggcgcatcgacctgcgcccccacaaggagcggctggcgcagcagaccgggcgggtgcgcgaactggccgccgccttcgcggacctgccggagaagcagcgcttcgccttcagcgtctggggcctgcgcgacaccgacagctggctgcgccagggcgacaacgacgacggaaaggacagccccctgcccttcaccgccgccggttcggtcaatccgatggcggcggcgatcgcctcgggctttcaggcctgatcggcgaccttgccgtcgatgaagtggcggccctgccgatcctccacctcaactacccacaggtcggggtcgtagcccacctgtcgcccgacataggcgtccagctcgccttccatctcgcttgagaccggctggatccactggcgctcgccgtccaggccgaaggcctcggtgaacagccgcgcccggcgggtcgaggtgtcgaacgccttgacgatcaccgccccgccgcgcggatcgccgcgccgcaccacggtggcgtaggcgccttcgattccggcccggcggatcagggccgacacccagatgtcggtggacagcagcaaatgggtaaccctgatcggaaaccggaaaccaaggcggcgtgcgccataagccgcttatgagacccgggcctctcgccatcaacgccaaagccgcagccgccgcgaccgcgctggcgctggcgctcgccgccgtgccggcgggggcgtctcccaatggcgcggccgaacgcttctacgagcgcagcttcgttctcgccgccgacgcccggtgccgcctgttcgagccgcgcctgacccatgctctggaggcggcgacctggcaggcgcgcggcgccgccttgcgggcgggcgtcgacgccccgcaactggccgaaagcgccggacgcgcgcgggcgctggcggcccgcacgccctgcgacgccgccgatctgaagaccgtggccggccgcgccgaaaacgccttcgccggctggaagcggctggcgcgcctgaccctgccgggcgcgcggcgggactggagcgccgaccgtttcgcctaccagagcccgacctaccggctggtgcaggactccgtcaccggcgcctctccggtgcgcttcggcctggctgggacgatggacgcggaggacgcgccgctggcggtggtgtcctggttcggccggccgcgtccggtcgccgcgcggctggtgctgcgagacgcaggcgtcgccccccagccctggctgaccggcgacctgcccccgtcggcccaggcccgcacgatctggtcatccggcgccgaggacgccccgacgacgctgctgccccgcgatcgcaaggcgggtcaggcctggcgctttcccgcaggagccgccgaggcgctcgccgcgctggacccgcgcgaacccttcgccctggagttcttgttccgcgacggctcggtcgcccgcgcccgcttcgaggccggcgacttcgccgccggacaggcgttcctggcgatgggggcggtctagaatcttcccccgcttgtcgggggaagtgtcagcgacgtgacgcggagcgtcacggctgacgatgggggaaatgtcgtcttcaagaagattcccctcatcgaccctggatcgctgcgcgatcgacgggccacttctcccgcaagcgggagaagagtctagcgcgccagcggcaaccgcaccgtggccgcagcgccttcgcccagggtgctgtccagggtcaggcggccgccgtggagttcggccagggagcggaccagcgacaggccgagcccggtgccttgcgcacgctgatcagcggcgcccgcctgctcgaatgggcggccgaggcgggcgagggcttcgggcgcgatgccgacgccggggtcggacacgatcagctccaggtcgtcgtccacctggcccagcgagacggtcaccgatccgccggccggcgtgaacttcaccgcattggacagcaggttcagcgtcatctgcttcagcgcgcgtcggtcggccgaggcggtcaggacgtccggcggcagcacggcggacaggcgcacccccttgtcctcggcctggggccggaccagggctacggcggcggacaccggctcgcgcgcatcaaagctctcgatcgccagctggtagcgttcggcctcgatcttggacaggtccagcacgtcgttgatcaggtccagcaggtggccgccggcctgggggatgctgtcggcgtattcgccgtagcggtcgggcaaggggccgaacagccgctggcgcatgatgtcggaaaagccgatcacggcgttcagcggcgtgcgcagctcgtggctcatggtggccagaaagcgcgacttgccgaggttctgggcctcggcttcggcgcgggcggcgtccagccccagttcgcgcgcgaactgcacggtgccgtcgaacagctgggcgatcaggcgcggcggatcgccgtcggccaagcggcgcacgatcagcaccacgcgccggtccagcgcgaggcggggcgtgaacaacgcctcggcctcgccgcccgccgccgcccgcccaagcgccgccagcagcgccggccggtccggcgcgttcacggccgcgatcagccctccgtcgaacagggccggcagcgaaagcgccgagggagccgcgccgtgcgcgtccagcagccgcccctccggcgtcaggatcagcagaaggcccggctgggtctccaggaggccttgcgcccgcgtcgccgcccctcgcgcctggtgggcggcgccggcctgttcgcggcggaccagcagcatggcgacggcggcggcggccaccaccagcaccgccgtcagggccgaggtcgcggacggcaggggcgacgcggcctgcgcgcccaccaccgccatgcccgatcccaccgcgccggccaggatcgcccggccggagccgcgatccagcagcaggcccgcgaccaccggcatgaacagaaagggcgaggccgtctcgccagtccgagccaagaccgcgcaggcggtgatcgaggccagagcccacgccgccagcagccagccgcgcaggccgggcccgtcccgccacgcaaaggccgagcccagcaggccgggcgccgccatcgccgcccccgccatgacgacggcggcggccttgccgtcccccgcaccctgcccggccgccgccagggcgacagccgccgcccagccgagatgccaggcggcgcgcatgggcgacctcgacatgtctcgttctgaacgggcggcgaaaggcgacaagggcgtccaagctgttgaaagtgttcggcctgagcttacggaccggtttgagtcgaagcgagggcgctcccccggcaggagagtcctgcaagggccggaccatgcatcttctggggacgatccggccattcatcatgaacgcgtttgccggaaaggccgcccgcccctatctcgcggccatgacgacatcggtccacagccccgaagacacgcccgaacaggcgctcgaagccctggccgaggacttcgacctgctggaagactgggagagccggatcgaatacgtcatcgacctgggcaagggtctggcgccactgccggacgaggcgcgcaccgaggctcacaaggtgccgggctgcgccgcccaggtgtggctggcgccccgacgcgagggcgagcggctgtggtttgccgccgactccgacagcgccctgtccaagggcaacatcgccctgctgctgcggctgttctccggacgcaccgcgcgcgagattctggacttcgatgctcgtgcggcgttggaccggctggggctgccctcggccctgacccgccagcgcgcgaacgggctgaacagcatggtggggcgcatccgcgaggcggccatgcaggccgaggtcgaggcggcctgaacctttctccgggcggaacattaagggaacccgcacaggagattccctcatgaccgacgccaacgagaaccccaagctgcaggacgatcccggctccaacaccgtcaagaatccggcggactgggtgtccggcgacgacccgatgaccggcgcccaggcgtcttatctgaagaccctgtccgaagaggcgggccagcccgacatgttcgccgccgacctgtccaaggccgaggcctccaagcgcatcgacgcgctgaagggcggcgacagctgatcctccccccaaaggggaggagcatgggctatagtccgtaatgctccgccagcgcctgcaggccctgcttcagcagggtcttgccctggcggcgacgcaggccaagcccggtctcggccaactgcaggctgtcgcccgcgatgcagatgcgcgccaccatgggccgcaggcgcggaccgcaggcgagcagggcggcctcgacccgccggccggcgctgagagccagatcgccaggctccgtccgcaagcctgatccgccgccggatcgcggcagggcgtcccatcgcatcgtcagcgacgggccggccgaggccagttcgccgtcgcggcgcaggcgctcgcccgccgccacctccgctggcgtcagccagggacgacccgaggcgtccttgcggcgcgctagccacaggatcggcgactcgcccagattggcgcggcgagcgaccagggcgccgtctggctgaatcaccatgcgctcgccttcgatcatcccgggacgaccgggcggaagggcggtctcggccgcatccccggcccgccgcgcgacccagccgccgccgtcgcgaaggcgcaggccgggcgccgtggccagggccctgaactcggcctcgtccagggtggtggtgatccgcgcccgccggtcccggccgatccgcaagaggtagcgcccctccatgccgtccagccaggctccaggccgcacgatcaggccgcgcagccgggcggcgcgatgagccacctcttcgtccctgccgctcacgccgcgatctccacccgggcgccggccgtcacggcctggatgcaggcctccagctcggtcagcagggcgtccatggccgggcggtcccgctcgtcctcagcccagcggcaggccgtgctggcggtggcgcggtttaggccaaaggcgtgggcgacatgctccaggctccagccgaacgacacatgcgtcaggtacatcgccagccagcgggcgcggcagttgcgcggatccagccgaccgcgccccttcatcctctcgggcgccgccccggtgcgcgcccccaccagatgcagcgctagacccgccatggcgcggtcggcgtccgacaccggaacccgatactccttgatcacccttcaactccctgcgcgtgtgttcaacgacgccaacctatctcagcggcgatgcatggataggaatgttgtcctatgtcgcgtcagaagcggtcgactcgccagccctgcggcggcgttgcgaggaggcgggtccgagggtgggtcgtcgatccgtgacgggcgagcggaaaaaagttaacgcgcgacctggccgcccctcgacgccgattcgcaaatcagcctacgattcgcctcaatcgggtggcgttaacccttcttaaggttttccgcccttaacttacgaacaaggttacccggtcgtgggccagggtggttaccgtcaagctttgcctggaggggcatgaatgcgcgtcctgctgattgaagacgatcacgcgactgcccagagcatcgaactgatgctcaagtcggaaggcttcaatgtctatacgaccgacctgggcgaggaaggcatcgatctgggcaagatctatgactacgacctcattcttctggacctgaacctgcccgacatgagcgggctcgaggttctgcgccagctgcgcgtcggcaaggtcaacaccccggtgatgatcctgtcgggcagccacgagatcgagaccaaggtcaagacgttcggcggcggcgccgacgactacatgaccaagcccttccacaaggacgagctgatcgcgcgcacccacgccgtggtccgccgctccaagggccactcgcaggcgatcatcaccaccggcgagatcgcggtgaacctggacgccaagacggtcgaggtcgacggccaccgcgtgcacctgaccggcaaggaataccagatgctggagctgctttcgctccgcaagggcacgaccctcaccaaggaaatgttcctgaaccacctgtacggcggcatggacgagcccgagctgaagatcatcgacgtcttcatctgcaagctgcgcaagaagctggccacggccgccggcggcaagcactacatcgaaaccgtctggggtcgcggctatgtgctgcgcgacccgtcggaaggcgcccagagcgtcgccgcctgatcggctccgtataagagtttggaacgcccgccggatcccaccggcgggcgtttttcgttccggaccataacccctccgtcccgaggcttgcgcctcgcgccacctccccagcgcttcgcgacagggaggagaaggcggacgtctctcctccccatccttgatggggaggtggatcgacggcgtgagccggcgagacggaggggtcccctcccgtcccctcctgctctaaacacgcacgatgaccgacctccccgcccccgccgtcatcctcgacaagccgcaactggccgacaacatcggggcggtggcgcgggtgatggcgaacttcggcctccacgacctgcggctggtcagcccgcgtgacggctggccccaggaccgggcctgggccaccgcatccggcgccgactgggtgctggacgccgtcaccgtgtttcccagcgtggccgaggccatcgccgaccttcacaccgtcttcgccaccaccgcccgcccgcgtgagacgcgccagcccgtgcgcacgccgcgtgagagcgcccgcatcctgtatgacgacacggggtccggcctgaagaccggtgtgctgttcggcggcgagcgggcggggctggagaccagcgacatcgcgctctgcgccggcatcaccaccattcccatcgatccgcgccaccattcgctgaacctggcgcaggcggtggcgatcaacgcctatgaatggcgcaccctggtgctggacgcaccgccgccgcgcttccgcgagggcgagccgccggccccgggcgccctgctgctcggcatgtacgaacatctggagactgaactcgacgccggcggcttcttccacccgcccgagaagaagcgctccatgagccagaacctgcgggtcatgctgggccgcgccgcctttacagagcaggaggtcgcgaccttccgcggcgtgatccacgctctgtcaaagggacgcggccgggtgctggccaagctggcggcgcaaaaggaggcggcgcgcgaggccgaggagcggtgaagaccgccctgatctatccgctggcggccctggccgagatcgccggctgcttcgccttctgggcctggctgaggctcgaccgctccccgctatggatcgcgcccggcgtcctcagcctcatcgccttcgcctggctgctgacgcttacgcccagcgacgcggccggccgcgccttcgcagcctacggcggcgtctacatctgcgcctcgctggtgtggattgcggtggtggagaagacggcgccggatcgttgggacctgctcggcggcgcggcgtgcctgatcggcgcgggcgtcatcctttttggcccgagaagttaaggcctcctagcaccggccagccccgaaagcgtcaagtgaaacttgacactttatagccgactcaccattctcgccctgtggagatcgccagcatcaggcacaaggctttgcgccagttcgccgagaccgggaatgcaaagggtctgccgggaaacctgctcggaaggctccgcaacatgttggcctacctcgtcgcgatctccgccgaggaggagttgctggtcccgccgaacttcggcgcacacaagctgacgggagatcgacagggcgagtggtcgctgacggtcacccgcaactggcggctcaccttcatcatcaacgaagccctcgcgatcgaggacatggatctggaggactatcactgatggctatccgtcttcattcctcattcgccgttcatcccggcgtctgggtgcgggaagagatcgtcgcgcccagaggcctcagcgtcacagcgctcgcagaggcgctgaacgtaacgcgtcaggcgaccagcagcctcttgaatggacgcgcaggtctgtccgctcaaatggccattcgtttcgagaaactgtttggtgtcagcgccgacaccctgatccgcatgcaggcggcgcacgaccttgctcaggcccgcgcgggcgagaagtcgataaaggtgcgtccgctggcggccgcctgattgggcgatgaggagactaaacgcgccgcttgcggtcaggtacagcccgtgatcctctccagcagcatcggggaggatggatgatgctggcttggctgttgatggtgtcccttgcggccggagacctgtcgcaggcggcgcaggcggccctgcggccgttgaccgacgcgatccgcgaggcccgctccaagcaggcggctctgcctccggacgccgctccgaaagagcagttggaggcggttcttgcattggaccagcacccgctgattgcgatgcaccatgttgatctgtccggtctgtcgccggaggaccgcacggccgcccgcgccgaggcggacgcccaactgaaggctatcagcgatgagaccgtccgcaccgtcctgtcgcttgtgccggaagacggctggttctcgggcaaggtgtatggcgaagaggccgctcagggcgcctttctggtcgtgcagcatgcggacacggccctgcagaagcggttcctgcccgctatccaggcgatgtctgaacgtggcgagacgccgagatggcagtacgccatgatgcatgaccgggtcgccgtcggcgagggacggccgcagcgttggggcacccagatgcagtgcgtgaacgatcgcatggtcccggcgccgaccgaagacccggatcgcctggaggaacgccgcgcccccatgggcttccgctggccgaactacgaggcctatctggcgaacttcggggcttgctgaacccgccggttctcacgcaagggagggcgacacgtcaggagccatcgccatgaagacccgcgccgccgtcgcattcgaagccaagaagccgctggagatcgtcgaggtcgatctggagggaccgcgcgcgggcgaggtgctggtcgagatcaaggccacgggcatctgccacaccgacgcctatacgctggacggcctggactcggagggtatcttcccgagcatcctggggcacgagggcgcgggcgtggtggtcgaggtggggccgggcgtcacctcggtcgaggtcggcgaccacgtgatcccgctctacacccccgaatgccgccagtgtaagtcgtgcctgagccgcaagaccaacctgtgcaccgccatccgcagcacgcagggcaagggcctgatgcccgatggcacctcgcgcttcagctacaagggtcaggcaatcgcccactacatgggctgctcgaccttttcgaactacacggtgctgcccgaaatcgcggtggcgaagatcaggaaggacgcgcccttcgacaaggcctgctacgtcggctgcggcgtgaccacgggcgtgggcgcggtggtcaacaccgccaaggtcgagccgggctcgaactgcgtcgtcttcggtctgggcggcatcgggctgaacgtcattcaggggctgaagatggtcggcgccgacatgatcgtgggcgtggacatcaacgactccaaggaggagtggggtcgccgcttcggcatgacccacttcgtgaatccgaagaacgtcagtgacgtcgtcgcccatctggtggagctgaccggcggcggcgccgactacacctttgactgcaccggcaacaccaccgtgatgcgccaggcgctggaggcgtgtcaccgcggctggggcgaaagcgtcgtcatcggcgtggccgaggccggcaaggaaatcgccacccgcccgttccagctggtcaccggccgggtctggcgcggctcggcctttggcggcgcgcgcggccggaccgacacgccgcgcatcgtcgactggtacatggacggcaagatcgagatcgaccccatgatcacccataccctgccgctggagcgcatcaacgaggccttcgacctgatgcacgccggcgaaagcatccgctcggtggtggtgttctgaagagccgcagttgacggatgatagcggcacgctatcatccgttcatggctcaagtcctagttcgtgatctcgacgaccagatcgtctctcgcttgaaagtgctggcgaaggcgcagaacatctctctcgagcagaagttcagggacatggccgcgcgcgaggtgcaggaggtcgaggatcgctttgaacgtgtcgcggcgcgcatccgcgaacagacccgaggatcacagctcgacagtacggctctgatccgcgaagaccgcgatcgttgagcgtcgccgttttcgacgccagcgtcgctctcaagtggctcgtcgcggaccatctcctggcggcgcccgccttggccgctcgcggcgagttcgagccggtcgctccgagcttcatccagatcgaagtcgcaaatgcgctttggaaatatgttcgcacgggccaggcggacttggacgacgccatagagggcgtggcccttctcgccaaactcatgaacctctatcccgacgatgatctgctcgcgccggcccagcggttggccgccaggctgacgcattcggtgtacgattgcctgtacttggcgctcgctcaacggctgtcctgtccgctagtcaccgcggaccgccgtctcgctgaacgggccattcacttgggcgtgtccaccacactgatcgcaccggaatgaccatgcagatcaccaagacccacgccgtccatggcggaaccctgcgctatctgaagcacgacagcgcggtcaccggcacgcccatgacgttatcggtgtggacgccgccgggcgaggggccgtttccggtggtgatctggttgtcggggctgacgtgcaccgaggacaacttcaccaccaaggcgggggcgtatgcggcggcggccgagcacggcgtgatcgtggtcgcgccagacacttcgccgcgcggggaagcggtggcggacgatccggcctatgacctcggacagggggccggcttctacctcgatgcgacgcaagagccctgggccgagcatttccgtatggaaagctatgtcacgggcgagctgatcccgctgatcgaccaggcgttcccgaccaccggctcgcgttcgatccttggacattccatgggcgggcacggggcgctgacgctggcgctgcgccatcccgacctgttccgcagcgtctcggcctttgcgccgatcggttcgcccacgcgatgcccgtggggcgaaaaggcgttctccgcctatctgggcgacgaccgcgccgcctgggcggcgcacgacgccgcccggctgatcgagggcggcgcggcgcgcggcgtctatgacgacatcctggtggatcagggcgacgccgaccccttcctgcacgaccagctgaagccggaactgctgcaggccgccgccgacgtcgcgggccaaaaggtcacgatccgcatgcagcccggctacgaccactcctacttcttcatggccagcttcatcggcgagcacctcgcctttcacgcggcccgactgaaagcctgacgccgatggccgacgcccccgactatgacgccatgttcgccgccctgtgcagcgaggtggggttctgcctgcatgacaaggggcaaaagcgggtgatcgaggccttgccgaacggtctggacgcagccgtgcgcgccgtcttcaaggcggaaggggtggacgaacccaatgcgccgggcgacctgaagcgagcggtgcgcgactgcatcaaggcgcacgttcagtcctgaggcgggaacgaaatcggcggccccggcttgggttcggcgacggcgtctcctagatgaggcggacctgcaaagccttgacctgaaggagcatctcccatggccttttccctgccgcccctgccctacgcctatgacgcgctggagccggccatcgacaaggagacgatgaccttccaccacgacaagcaccaccagacctatgtcgacaacctgaacaaggcggtggaggcggactccagcctgcagggcaagtcgatcgaggagctactggccaacgtgtcgtcggcccccaaggcggtgcgcaacaacggcggcggtcactggaaccacagcctgttctgggagctgctggctccggaaggtcagaccggcgagccctcggccgaactggccgccgccatcgacagcgacctgagcggcatggacaagttcaaggaagacttcaacgccgccggcgccggccagttcggctcgggctgggcctggctgatcgtccaggacggcaagctgaagatcacctccacgccgaaccaggacaatccgctgatggacgtggccgagcagaagggcgatgtggtcctgggcgccgacgtctgggagcacgcctactacctgaagtaccagaaccgccgggccgactacctgaaggccttctggtcggtggtgaactggaacaaggtcaacgaactgttcgccgccgccaggcgttaagccggcgatccgacgcccgtcggagcctttcggcgggcgtttcccatctcagcggaggcggctgtgcgcgcattttcgatcctgaccaccagcgcggcggccgccgcccttctggcgctgggcgcctgttcgtctcctgagcagcgcgagaccacccacggcggcaacatggccgacgacggccaggccagcgccggccaggccaagcccgcgcagaagcccgcctattggttcaaaatcggcgacgtcgacgccatcgccctggcggacggcgagaacccggtccccaacgacaacaagatcttcggcgtgggccagacgcccgaggccgtggccaacgtcctgaccgccaacggcgagccgggcgacaccctgcggctggaggtgcatccgctgctggtgcgcgccgacgggcgcacggtgctgttcgacgccgggctgggtcagtcccagggcggcacgctgatgcagtcgctgcaagccgccaacatcgatccggccagcatcaccgacgttctgatctcccatggccacggcgaccacacgggcgggctggtgctggacggcgccctcgccttccccaacgccgccatccgcatgtccgaggcggagtgggcggcggtgcgcgcgaacccggagatggcggagctggtgcgggtgatcacgtccaaggtgcagaccttcaagccggacgatgagatcctgccgttcgtggaggcgcaggacacggcgggtcacacgccgggccacacctcctatctgatcacctcggggcccaaccacctgctctacaccggcgacctgatgcaccacttcctggtctcggtcgaacacccggaatggaacatgggctacgacgccgaccagaacgccgggcgcgagcggcgcgagaaggaagtgtcggcgctcttggcgtcgggcgcgcacatctacacctatcacttccccttccccggcgtcggccgactgcagcagcgcggcggccgcgcgatcttcgtgccggaggcccaatccgttcctcagggcggaaacggcatggcgacgcccacccgcagcatcggcggcgcgcctcagggcggctgacggcggcgcctgcgcgctcagaccgacaggtcgaagcggccgccggcgcgttcgcacatgcgctggcgatggcgattacggaccgtccgtcgttgacgcagcatctcgtgaatgccgtcggcgaggtccagcagttgctcgtcgctcagcggctcgaccagatcgaccagttctcggcgcaatccctcgaaggcgcgctgcgtcaagcctgaagaaacggatgtggcgcccaccggatcaggtcccttgtgcaaacaggcgacatcgattgtcgtgctaaggaaagagcaggaacctcacgttgttccgccaaatgatccttaacgccgccttcagcttgactccgcgccttcgcgccagcataagcgcgccctccccgcatccgccccaggcggaggcgcgaagccactacggacgatgcgtggaccgccgttgagatcgtctcttcattcgggaagagaccgggccgcatcactgaaaagagaacagaatgtccaagcgccacagcgccaagtacaagatcgaccgcgccatgggcgaaagcctgtggggccgcgcaaagtcgccggtcaacaagcgttcgtacggccccggtcagcacggccagcgccgcaagtccaaggtttccgacttcggcctgcaactgaaggccaagcagaagctgaagggctactacgccaacatcaccgaaaagcagttcgccaagacctacgccgaggccgcccgccgcaagggcaacacctcggagatcctgatcggcctgctggaagcccgcctggacgccgtcgtctaccgcgccaagttcgtgccgaccccttgggccgcgcgccagttcgtcaaccacggccacatcctggtcaacggcaagaaggtggacatcgcctcctaccgcgtgaaggccgacgacgtgatctcggtcaaggagaagtcgcgcaacatggctctggtgctggaagcccagcagtcgggcgagcgcgacgtgccggactacctggaactgtccgaccgcagcttctcggtgcgcttcgtgcgcgccccggaactggccgatgtgccctatccggtgaagatggagccgaacctggtcgtcgaatactattcttcgtaagcgaagcgaccacgatgttcagaagggccccggatgcgtccggggcccttcgtttttccaggccctgttcttcggagacgaacaggcgcatcctccgtcatggaggcgagatcgggagggcgttcggtggaacggctgacgactttgaccaagggcgtgacggccgccgcgtgcgtggcggtgctgctgagcgcctgcgccggaacgcgggacgagacgccgacggcctcgaccgccggcatgcccggcgctctggagcccgtgcgcgccgccgccttcacccaggatcaggccgtgttctgggtcacctccaacggctgcaccgaaaaggaagacctgctgccgatcgtcagcctgcagggcggcaaggcggtgatcaccctgcgccgcatcgacgaggacacctgcagaaagcctcaggacgaaggcgtcgagctgaaatggtcgttcgacgaactgggcctgcccgccggatcgccggtggtggtgaataatccgtaccagctgccttcgggcggctgagggcgtccggcgcccctctcctccccatctacgatggggaggtggcgcgaggcgaagcctcgtgacggaggggtgggctccgacacaaggaccccctccgtctcgccggctctcgccgccgagccacctccccattcgctgcgcgaacagggaggagagcctccaccttgactttgggggcttaagcgcccatctgcggcgctgtcgcaccttcgcggcttccggcgtctccagcgcgtgtgggcttttccaaagcctgtctgtagcagccgccggcctttccagttcattcgctgcccggacacgcggggcggcgcccgatccatcttcggccctccccggtcgaactggcggcgctgcttttttcggcttttcagccggccgcgtcgcgcatgcgaaagacgatacgttgagcaccacctttgaatccatgggcctgaacaaggccctgctgaccgccctcgccgccgaaggctacgtcaagccgaccccgatccaggaaaaggccgttcccgacgtcatgctgggcaaggacctcctgggcatcgctcagaccggcaccggcaagacggcggccttcgccctgccgatcctgcaccgcctggccgagaaccgcaccccgcccgtgccgcgcaccacccgcgccctgatcctgagccccacgcgcgaactggcgacccagatcggcgaaagcttcaaggcctatggcaagcacctgggtttccgcaccgcggtaatcttcggcggcgtgaagtacggcgggcaggagcgcgccctgcagcagggcctggacatcctggtggccgcgcccggccgcctgctggaccacatccagcagaagaccttggacctcgcctcgaccgagatcttcgtgctggacgaggccgaccagatgctggacctcggcttcatcaagccgattcgccagattgtgtcgcgcatgccggcgcgtcgccagaacctgttcttctcggccaccatgcccggcgagatcggcaagctggcgggcgaactgctgaaggacccggtcaaggtccaggtgacgccccagtccaccacggttcagcgaatcagccagtcggtcgtccacatcgaacaggggcgcaagcgcgcgctgctgaccgagctgttcagcgatccgggcttcacccgctgcctggtgttcaccaagaccaagcacggcgccgacaaggtcgcggcctatctggaggccggcggcgtcgaggctggggccatccacggcaacaagagccagccgcagcgcgagcgcgcgcttgaggcgttcaagaccggcaagctgcgcgtgctggtcgccaccgacatcgccgcgcgcggcatcgacgtggacaaggtcacccatgtggtgaacttcgaactgcccttcgtgcccgaggcctatgtgcaccgcatcggccgcacggcgcgggcgggcgcggacggcacggccatcagctttgtcgccggcgacgagatgaagctgctcaaggacatcgaaaaggtcccccgccagaagatcccggcgatcgaccgccgcaatgacaaggccttggcggcgctggacgcctccatcatggcctcgggcgtcggcaagaaggcgaccctgccggaacgcgaaggcggcgagcgcggcgacggccggggcggtcgcggccgccgcaatccgcaccgcgacggcgtgcgtcccgagggcggcggccagccgcatcgccagcgcaagggcggccgcgccggcgccgaacgcgcagcccccgtgcgcgagtataatccgatgagcggcgagcgtccgcgcccggcggcggcgcccgcctcggcccctgccgtgtccgccgagccgcgcccggaaggccagatgaagcgccgtccgcgtcgccgcccgtccaacggcggcaaggggtacgcccagcaggggtaagagtcttcccccgcttgtcgggggaagtgtcagctcgtggcgcggagcgacacggctgacgatgggggaagtcgactgtcgaagaagattcccctcaccgaccctggaccgcttcgcggtcaacgggccacctctcccgcaggcgggagagggtcttgaataaaaaaacggcggctcgggaaggagccgccgtttccgtttcagccgtggctgaaagccttagaacgcccagcgcaggccggccgagaagccgacgccgtagccggtcgcctcgccgcgcaggttggaggtgatcagaccgttgccgtagacgtcacggtcgtccgagatctcgctgtcgtcgatgccgatgtaggtcaccgcgccgtcaagcatcatgccgggacggatctccttggtcaggccgcccgaaaccaggaagcggtcgccgtccgggatgcgggcggtgcgctggccgtccggggtcggggtcggatcgaagcccactccgccacggaccgtcagggtggggtcgatcttgtagtcgaaaccgatagcgccggtggtcacgtcgtcgtagttctgttcgatcacgctgtcgcgggtggagtccacgcggatggcgtcgaactcgctccagccgatctggttgacctgggcgttcagggtcagacgatcgttgacgtggtagcgggccgacagggtggcgaaccacggcgtgttgaagcttgcggtgccgccggcgctgaagttcgcggccgccagggcgcccgcgagacccgagacggtgacttcgccgtccagctcatgctcgatctcggagcgataggagacgccgaggtccagggcgccgaagtgcatctgcgcaccggcgttccagccgtagttccagccgtcgcccttcagcgagttgaagccgtcggtggtggagggaatgaagcgcgccgtcaggccgcccgtcggaaccacggtgggcaggttaggcagggccgaggtcagctccgcgtcggcgtattgggcgtcgaagcccacgccgacgtccagccactcggtgacctgcatggccaccacggccgacaggttcaccgacagcagcttggacttgatcgcgtcgtagcgggcgaagtcgtcggcgtcgtattcggtggtgaagttgtaaggcgcctgggcggccaagccgacggtgaagcgatcaccgaccggcagggcgacggcgaagttcggcaccacgccgctttgcaccacttcgtggatgtgctggtcgccgccaacgggggcgcttccgcggaagatcgagccggccgggaacggcgggggcggcgcaggcagggcgtacgtcagggtcgagccggtgttgtcgacgtcggaatcgacgatcaggccatgggcgccgatgtagacttcgcggccgctgcgggcgatcgaggcggcgttccaccacagggaggacgcgcccatgtcggcgccttcgcccgagttggcgcggccgatgccgcgcaccgactgttcctgcagatagaacgagccggccgaagcgggcgcggctatggcggcggccgaagcggcgagcagggcggcggcgctgacgcggccgaggatcctgggggtcatgtttctcttacacctaagataaagcgcgccgggcctcatggaccgggctgtcggggagcgctcgcacagcgttcatggcggtgaagcgttgcttgcggggctggtctcggaccggtttctggcgaaactgtgtcacacaggacgcaggagatcacggctgcgagaggtgacgcagcggcatgttcgtgccggaaaccatccgttccccaggctgatatttgcgccacaccctcgacccctcaccacgggcgacgggcttgagctttcgtgctaggctctccatctcacggccgcatcacgtctgcatccgagtctccatgtacgaagtttccgacctcgaatccgaccgccccgtccgctccagcgagatccgcatctacgggctggacgagttcgagggcatgcgccgcgccggccgcatggtggccgaggcgctggacatgatcgccgagcacgtgaagccgggcgtcaccaccggcgaactggacgacctggtccgcgagtggacgctggcccagggcgccaagcccgcctgcctgggctacaagggctatgagaagaccacctgcatctcgatcaaccacgtcgtctgccacggcatccccggcgaacgggtgctgaaggaaggcgacatcgtcaacatcgaccacacggtgctgctggacggctggttcggcgactccagccggatgtattcggtcggcgccgtcaatgcgcgcgccaagaagctggtcgatgtgacctatgagtcgctgcggctgggcctggagcaggtgaagcccggaaacacctttggcgacgtcggcttcgccatccagaaatacgtcgaagcccagcgcatgagcgtggtgcgcgacttctgcggccacggcatcggccgggtgttccacgacacccccaacgtcctgcattacggacgacgcggcgagggcgcggtgctgaagcccggcatgatcttcaccgtcgagccgatggtgaacctgggcaagccgcaggtgaaggtgctgtcggacggctggaccgcggtcacccgcgacaagtcgctgtcggcccagtgcgagcactcggtcggcgtgaccgaggacggcgtggagatcttcaccctgtcccccgccggcctgttccgcccgaactgaaccggagccgccgctcgggcgcttaggacggtgagacccaccgttacggagcccgacatgaccaaggccgccctgttcgccaccgctctttcgacgctgaccctggccgcctgcggacaacaggagcccgcgcccgcgccgccgcccgcgccgatgaccgaacaggccgccctgcccgccgcctcgcccgagcccgcggctcagcccgccctgcccgccgtggccgcgccatcaacggcagccgccgctcccgcccgccccgcgccggcgtccacgccgacgaccagcgcctctctcgacgcctgcatggagggggcgaacaccaccgtgcagatgcgcgaatgcgcgggcgccgagcacaagcgccaggacgaccggcttaacgccgaataccgcgccgcccaggatcgcctgacgggcgcccagttcaccatcttgcgaaacgaacagcgcgagtggctgcgtcgcggcacgggatgccgccagggcgaaggcaccatcgctccggtcgatttcgccctgtgccaggcgcgcgagaccggcgcccgcgccgactacatcgccagctatcgcggctgatcgcgcagcccttgcgtcaggaggcgcaatcggtcgatcctgcatccggtttcgggctgggggaggatcggatgctggacgatgcgacgcctcctctgaaggcggaggcgaagccgaaggcgccgccgcgtcatggcgggcaccgcgaccggctgcgggagcgggcggccaagggcggcctgggcgccctgcccgactatgaactgctggagctgctgctgttccgcagcgtgccctataaggacaccaagccgctggccaaggacctgctggcgcggttcggcgggctggaggggatcggcgcggccagccacgaggcggtggaggacgtggtcgcccgctcgctcggctatcagcccggcaaggccacgcgggcggtggcgctggacctgcagctgatctttgatgtcacccggcggatcgccaaggagccgacacagaagcgcaccgtcatctcgtcctggtcggcgctgctggcctatgtccgcgtcgcgcttcagcacgagccgagagagcagttccgggtgctgtacctggacaagaagaaccaacttatcctggacgaggtgcagaaccggggcacggtggaccacgcgcccgtctatccgcgcgaggtggtgcgacgtgcgctcgagctgtcgtccagcgccatcatcctggtgcacaatcacccgtccggcgaccccacccccagccgggccgacatcgagatgacgcgccaggtgatccaggccggcctgcacctgaacgtcgaggtgcacgaccacctggtcgtcggccgccacggcgtggccagcttcaagcaactggggctgatgtagccgggcattaagcttttgcggccatgctgggcggcgaacgagccgagtgtttgccatgcccatgtccgccgaagccctgcacgccgatctggccgaggcctttcccgacgccgagatcgccatcgacgacctggccggagacggcgaccactaccgtgcgcgcatcgtctcggcggtcttcgcgggcctgccgcgcgtgcgccagcaccagctggtctatggggcgctgaagggaaagatgggcggggagctgcacgccctggcgctggagacctcggcgccgtcgggcggagagggctgaaccgatgcgctatcgtccgttcggaccgtccggcgcggccgtctcagccatcaccctgagcgtcggcgccgacatgctggcgcgcggacgcgaggcggccatgtcgctgctgttcgccgcgctggagcagggcatcaacagctatcggctggagaccgccgatccggtggtggccgaggtgctgggcgaggccctgtcgcacctcgatcgcaagctggcgctggtgtcgctgacgctgggcgaggtcgatccccggcggcaggtgcgcgacttcacctccgaaggcatcaccgccgccgtggaccgggtgctgcactattccggcctgggctggatcgacgtggcggtgctggacgcgccgggcgagcacgagctgcgctatgccggtctgaacgcgctgaagaccatgaagcggaccgagcggctgcgcctggcgggagtggccggcgacggcgaggccatggacgcctttgtctcgaccggggccttcgacgttctggtgacgccgtgcaacgtgcgttccgactggaaggtgcgggcgcgcatccgcgccgcgcgggaacaggacatgatagtgttcgccaccgacaccttcccgcaggcgctgctgcgtgagccggagagcgaaggcgcgccggtgcggcgcggcctgttcggcctgggcgccaaggccgccgccccgccgcctgcggccaacccctacagctttctgacgcgcacggcccgttggacgccggagaccatctgcctggcgcacgccctgaccgatccggccctgaccagcgtgatcgtccaggcccgggacgcccagcacctggaagccctgtccgagacgcccgagcgcgacctgccgccgggcctggccgcgcagatggagatggcgcgggtcgacgcggcggcgtgacgccgcgcgcccttgaccccggctggggcggcgcctagctgacgcgcaaacgaaagggtcccccatgaccgacgccaccgtccagtcgaccagccagaccaccgaccaggccgccgaccccgtccacgccttcatcgcctccaccttggccgagcacgacgtggtcctgttcatgaagggcacgccggaccagccgcgctgcggcttctcgtccctggccgtgcaaatcctcgatcacgtgggcgcgccgttcgtcggcgtggacgtgctgcaggacgagacgctgcgcgaaggcatcaagagcttcaccgactggccgaccattccccagctctacgtcaagggcgagttcgtgggcggatcggacatcgtgcgcgagatgttccaggccggagagcttcaggcgctgatgacagaaaagggcgtggcgctcggcgaggcctgatccgtggcgcgcccgctgcaccagccgcgcgaggaccgcgaggtctttgtcgtgccgcttgaggtgcggcctgaacacatcgacgccaacggccacgtcaacaacgtggtctatgtcggctggctgcaggacgcgggcacggcgcactggaacgcccgcttctcgcaagacgaccgcacccgctggtcctgggtcgccctgcggcacgagatcgactatctgcgcggcatagagccgggtgcaaagggcgtggtcgcccgcacctgggtcggcgagccgcagggcccgcgcttcaaccgctatgtgcggatagaggacgcccaaggccgcgtctgcgcccagggcgtctccgaatggtgcctggtcgacgccgagaccttgcggccccagcgcatcccgccgttcatgctggcggtgttcgacacggtggcggcggcctctgaagaccaggcggacgatgcggagcaggctgcacggcgttgacgctttccaccggcgacgccaaggtctccgcctgaacagcgaccaggaggcgccgtcctgaagatcaaagccgcaccagcgatccgccagatgtactggtgcgacttctggaccgaccatcgcattcccgagatgggcaagaagcggccggtcgtgatcgtgtcgttcaagaacaccctgcacggcgtatcgctggtggtccccacgtcgaccgacccacaggaaggcgccagcgcgcgatgggcgcacaagctgtcgatccaacctgacgggcaacgccagtcgtgggtcgtgtgcaaccacctctacacggtcagcaacgccaggctggagcctttgcaaggcgcagtcatcccgcggctgtcggagaccgagttcaaccagatactcgccttgatccacgcctggttacccaaggcgcctgaagcagccggctgacttgactccggcgactatcgactccatcttgaagccactcgcggcctcgaaagagtgtccgtttcccgaaagggagtgactggcgaagggcgtccgaaaggacgccctttcgttctttctacttcagtggattgagcacgcgcacgggcgcgcccggctccagccccaggtcggcgtaggtccagcgcagttcgacgccttcggccagaagggcgcggcagttgtcgggcttggttcgcttcagcgtgacctcggcgggttcgccgtccgtcaccgccagttcgaagtccgaggcgctggtgcaaccgttggaatcgacacgcaccacaagcgagccgtcgtggacataggcggtgcggatcgcctcggcgggcgcggcgtcgcggtcgttgacctgcacggtgacgttctcgccgccggtgctgtcatagaccacgcaggcggccagcaagggcgcggcgacggcggcgaccatcaggcccttcagagcgcggccgatcattgagcagccggtgcggtgacgacgcgggtggtcggcttttccgtcgaaatgacgatgcatccgctgagcagcggcgcggcgacggcgatggcgatggcgagacgcagcattggtgttccccatgattgaagcgttgccgtcttgtgacgcgcgtccgtcgcgaaaacacgtgaataatcggaaaggcgggccttgatcagaaccgcaaccgacataggtgctcacgcctcctccctccccggatacgacttcatgagccagctcttctcccccgtcgccatcggtccccttcagctgaagaaccgcgtcgccatcgcgcctatgtgccagtactcggccgtggacggcctgccccagccctggcacgtgcagcacatcggtcggctggcgatctcgggcgcgggcctgacgatcattgaggcgacgggggtggatgcgcagggccgcatcaccctcgaggacacaggcctgtggaacgacgaacaggaagcatctttcaagcgcatcctgaccgacatccgcacctattcggatcagccgatcggggtccagctggcgcacgcgggccgcaaggcctcaacccacgcgccggccaagggcggtgaggcgctgggtcccgatgaaggcgcctgggagacgctggcgccctcggccatcccgttcaaggacggctggcacacgcccaaggccatggacgaggccgacatgcagcgggtggtcgacgcctttgtgcaggcggcggagcgggcggaccgcgcgggcttcgacctggtcgagctgcacgccgcgcacggctatctgctcagcgagttcctgtcgccgctttcaaaccagcggacggaagaatacggcggctcgcccgagaaccgcatgcgcttcccgctgcgggtggcgcaggcgctgcgggacgcctggccgcgcaccaaggcgctgggcgtgcggttgaacggcacggactggatcgagggcggagtcgcgctggaggaggtcaccgcgttcggccgcacgctgcacgagatgggctacgactatctgcacctgtcgtcgggcggaaatgtcgccaaggcgcagattccggcccgcgagcccggctatcagctgcgcttcgccgaggcggtgaagaaagccgcgccggaggcggtggtcatggccgtgggcatgatcttcgacccgcagcaggccgaggacatcgtggcgaacggccaggccgacatcgtggcgatcgcccgcgcggcgctggacgacccgcactggccccaccatgcggcggcggcgctgcacagcgacgaggatttgccggtgcagtatttcggcgcgtccaagggggtttgggccggctaccgcgagaaggcgccggcctgacccgaagctccgggcgaggacctcagtcctcgcccaccatggcgatccacggatcggcgatcccggcctcgacctcggcgaccttgaccgcgggccagccgacggaggccgtggcgctttcggcccaggcggcgacggtccagtcgcgcagttcggccgcgccggcggccaggcgctcggtcacaaaggccgcgccgcgggggtcagtctcgttgaagccgccctgcttctccagccggtagaacgggatcaccgtggccagggtggtcttcagatagcctacggtgcgcgccttgacgtcgaagccgtcggtgcgggccgcgggcatggccgcctcgaccgtgtccagccgcgcgacgcgggcggtgaaggcgccctcgaacacgccgtgggtctggcgcgagttggtgaagccttccgggttcggatagtcgccccagccgttgtagtggatcgaggtgtggtgcggctgggagccgtcgccgacgtagtgggcgagcacgcccaggtcgcgcaggatcagcgcctcgcgccgctcgcgatccacgcggtaccaggccttgcgctccatgttcgtttcgcgcgcctcctgggcgctcagcacgcgccagtaggcgaagtcgcgcaccagctgctgccagccgtccatcatcgcatagggcaggtagccggcgtcatcgacgtccaggccggccttgttcagggcggcgtcgtattcggacttcaggcgcggcagggcgtcgatgctgggcccctgggcggtcatggcgaagccggcgtcgtccaggtcgatgaagtgggcggtgtcgcgctcgcggtcgtgcggctggccggcgcccttccaccgatcgggctcgcgcgccagttcaccgatgtcggcgacggcgcccggcgtgcgcaggaaggcgggcagatcggccggcagggcgcgcatcgccgccaccccgatcagccggtgcccgctcgatccccaggcctccacctggacggccggcagggccaggacgacggcggcgaccgccgcggcgacgatgcgtttcatgggcgaaatccgatgcaaggggaccgcgctgctctagccgatccggtttgcgcgggcgacggaaatccctaagctgaggaaacttctcgcgcttccttccgttcagaggctccactccgcgagaagcggcgacgcttgtctcccccgacgtcgtccgtggatgcttgaccagaaggaaacccgccatgcgcgccaaccgtctcgccgccgttctgtccatcgccgcccttggcgccgccggggccgccgtcgcccaggacgctcccgcccaaaccacgcccgcccaagaggcgcccgtgacggcggccgcacccgcaacgacctctgccggtgacttcaccgacgccgaactgaagtcctacggcgtcgccctgccccgcgttcgcgctgtgtccgaggccctgaacggcggccagccgaacgccgagcagaccgccgagctgcaggccgctgtggccgcgacggggctggagaccgaacgcttcaacgccatcgcccaggccgcggccggcgatcccgtgctgcaggcgcgcatcgccgtgaccgcagcgcccgcctccgccgccggttcggtcggcgccagcgtcacggaagacgaactgagcaagttcgccgccgccaaccagcgcctcggcgccatcgcccagtcgctgaacggcgcccagccgacgccggagcaggccaccgagatgcagaccatcgtggccgagtccggcctggaggtggaacgcttcaacgccatcggccaggcctcggcgcaggacgagtcgctgcgcgcccgcgtggcgctggctcaggcccgctccggcgaataaggcttcaggccacgggctcgtccgcgccgaccggcgcgggcgggccggcttcgtcctcgttcagcacccggccctcgcggcgtggcgtgatgtagggtgcgggttgcggcgtcggcatgttgccgcgcgtcagctgctgacccgccttcaggccccccgtcagttgcaggtccagccgcgcctcgtcgcggcggcgcacgtcggcgatggtctcggcggcctctcggtcttccaggcccagttcgatcagggcgcgttcgccgaacctcagcgccgactcgaacgtctcccgcacctgatagtccacgcccgcctggatcaggcggatcgaatggccccggtcgtaggcgcgcaccaggacctttgtcagcgggaactccgacttcaccagctcgacgatgcggtcggcgatctccggtttgtcgacgcacaccagcacggcctccgccgtctccgcgcccgaggcgcgcagggtgtccagccgcgatccgtcgccgtaatagaccttgaagccgaaggtggcggcggcctggatcatctccacgtcgttttcgatgatggacacgtccacgtcgcgcgccagcagcggctgggccacgacctgggcgaagcggccgaagccgatgatcagcacctggccgcgtaggccgtcggcggcgtccacgtcttcggcgtcgtccgccgtcagcgcgcgctggggcgttaggcgcctcagcagcagggtcgtcagcggcgtcagggccatggacaggatcacgatggccgacatcatggccgccacccgcgcatcgaacaggccggcggcgagcgcggcgccatacagcacgaaggcgaactcgccgccttgcgcaaacagggccgagcggtcgaccgcctcatggtgcgaggccccgaacagccgcgccacgccatagatgccgaccgccttgaccaccatgaaggccaggagcccgcccagcacgatccgccagtcggccgccaccaccgcaaggtccagcgacatgcccacgctcaaaaaaaacaggcccagcaggatggctcggaagggctcgacgtcggcctccagctggtgccggaacgaggattcggacagcagcaccccggccaggaaggcgcccatggccatggacaggccgcccaggctcatcgcccaggccgcgcccaccacgaccagcagggcggcggcggtcatgacctcgcgcccgccgtacttggccagcagccggaacagcggactgaccagccagcgccccgccgccagcaccccggccactgccgcgagcgcaaagacgatcgtgcgccacaagggcggcgcggcctcgtgcgacgcgcccgtcacgctggccagcaccgcgacgatggcgagcagcggcacgatggcgaggtcttcaagcagcaggatggacaccgcgcgctgacccgctcccccggcgagttcgccgcgctcctccagcatctgcatgatcacggcggtggaggagagcacgaaccccatggcggccacgaacgccaccggcgccgccacgcctgcggccatggcggtcagcgtcagcaggccgccgcacgccagcacctgcgccgcgccgaggccgaagatgtcgtgacgcaggccccataaacgccggggccgcatctccaggccgatgatgaacaggaagatgaccacgccgaactctgcgacgtgcagaatggtctccggctcgcggaacaggcccaggccgaagggaccgatggccagacccgccgccagatagcccagcaccgagcccagtccgatcttgcgaaagatcggcacggcgatcacgccggccgccagcagcgccgccgccgcgcccagatccagtcccgtcgcctcggccatgccgccctccccgcatcaagctgagcggtgaaggtggggcgccttggggtggattgcgagcctctgatggaaggatgtgccgacatcgaagacccctccgtctcgccggctatcgccgtcgatccacctccccgccgcctgcgcggcagggaggagagatgcgtgatctctcctccccatcagagatggggaggtggcgcgaggcgccagcctcgtgacggaggggtttgacatggcgcgaagaacgcctccgtctcgccgcctgcgcggcagggaggagagacctatacctcggaccagcggcgcagcaggttgtggtagacgccggtcagttcgatcacggcctggtccttggggcccttgtccgcggccacgcgctgggtggcgacgtccaggcggaacagcatctctcgatcgccgtcgtcgcgcaccaggctttgcagccacataaaggacgagacgcgggcgccgcgcgtcaccggcgtaacgcggtgcaggctcttggacggatagagcacaaggtcgcccgcgggcagcttgatcgactggcggccgtacatctcttcgacgatcagctcgccgccgtcatagttgtcgggctcggacaggaacagggtggcggacaggtcgctgcggatgcggatcgggccgccgcgctgctggcgaatggcgttgtcgacgtgcaggccgaactcgcccccgccctcgtagcggttgaacagcggcggaaagatcgtgtgcggcagggccgcggccacgaacatcggattggcgtggagcgcctggacaatcaggcctgagacctccttggcctcggcgctgtcttcgggaagttgcagattgcgcttggcggtcgcggactggtggccggaggtcatgttgccgtcggtccagggaccggcgtcgagccgttcgcgcaacgcctggacctcggccttggtgaagacctccgggatatgaagcagcatgtccgcgtctccgcttttcagaacagccgaacggccccgccgaatggatgggccgttcgtcttcagcttagggcctcaagccgcgccctagaaccgcaggttcagcgtcaggctggccgagcggcccggcgccggatccgcgtggtgaacgccgttggtgcgcaggatgtagcgctcgtcgccgacgttctgcacgttgagctgaagcgaggcccggtcggtcacgtcataggacgcgaaggcgtccacgcgggtgtattcgggcgcatagatgcggttggccccgccgcccgccccgccctggttgccgccgaagctgtcggacacatagtagacgcctccgcccagcgtcagcctgggcagcagacgataggtggtgaacaggctggcggaatgttccggcgtattggccagcggcaggccttcaaaggcgttggggaccacgaccggcggcgcgcccgtcgtcgtcaccgcgccgcgcaccagttcggagtcctgataggtgtagccgccgaacacctgccacaacggggtgatgttgccggagacgccgagttcgatcccctgaacctcgacctcgcccgcctgttcgtacacgcccacatcgacgaggatggccgcattcctgcgggtcagatggaaggcggcggccgacagcgccagacggtcgccgaagacgttggccttggcgccgatctcgaagctttcgctttcttcagggtccaggatggtgtcggccagatttcccgttccttggccggtggtcgccgtattctggtcgcccgtcgaaaccgtcggcggcgtcgaggaggtggcgtaggagacgtagaggctggaagcctcggtcggcttgaacaccagtccggcttggtagttgacgaagtcccacttccgctcgggcaccggcgtgccggtgatggcgcccgtggtcgcgtcaagggctaggttggtcccctctgtctggtagctgtcccagcgcacgcccaggttcagcaggatgcggtcggtcagcgagatgctgtcgaaggcgtaggcgcccaccgtctcggtcaccgaacggctggcgggcccgcgcacgatggttccgctccaggggtcgtcggggttgggcgcatacagcggggtgcagtcgaaaccggtcagcggcgccgggcacgccgtgccgccggtggtcgtgatcgtgtagctggcgttgcggttcgtctcgcgcgtcagttcaaggcccacgtcgtagctgtgctcgatcccgccggtggagaccttgccgaacacgtcggtgacgttggccagggtgcgggcggggttccagcggttcttcagcccgcgcttcatccaccaggtgtcgccgaccagcaccgcggcgccgccgtcgccggggttggtcaccacatagtcgttcagggtgttggacaggcggctgacgttgcggagggtcagggcgtcgctgaaccggtgggtccagtcgaaggtgaatgtgtccaccttgttgttcaggaagtcgcgggccttcaggccgtagaaggcgctgtagtcgacatccagcaccccggacggatcaggacgcgcggccgtcgcgcccccgcgcttggtgtagagcgggacgccgtagtcgggcatctggttgctgtcgaggtggtagtagctggcgacgatcgtgctgtcggtcccaagacccgccgcgaacgacaacgcagcgccccacttgtcgtagtctacggcgtcgcgacccgcgacctcgcctgaggcgcccatcaggttgaggcgcagcgccgccgtcccgcccagcggcatgttgtggtccaccacgccgcgcagatactcgtccgtgccgaccccggccgagacgttggtgaaggggttcagcttgggcgacttggacgacaggttgatgctgccgccgcccgagccacggccggaatagactgagtccggtcccttgatgacctcgacctgctcgaggttgaagacctcgcgctgctggccgccggtgtcgcggacgccgtccacgaagatgttgttgcccgaggactgcccccggatgaacggccgatcggccagcggctggccgccctcgcccgcgccgaaggtgatgcctggcgaggtgcgaagcagatcctgcagcgaggtggcggccgtctgttcgatgatcgcttgcgggatcacggtgatggagcgcggcgtgtccaccagcggcgcgacatattcaggcgagtgaggcgcaggccggcgcacctggccggtgacgtcgatggtgccgaggttggtcgactgctggaccacgtccgcggtgacgacgacttccggctcctcggccaaggccggggccgcgcacagcatgccggcggcgctggaggcgaacagaagcgcgcgaagagaggcggcgcgggagtcggacattgcggcaggaccttggctgcgagattgcgatgcgctcgcaatatcaccacgacctatggacgcaatagcatctgcgaataaatctcagttgcgcgtggctacagctctgccgttgtgttcaggccgccaccatcttcatggacacggcggtatcggcgagccgatcgggatcgaccggcgtcctcttggcgatcaaggacttgccggccatgaactcgggcggggcgttcaccgcctcgacgcagacgatgcggtcaccgaccagatggaagacggcgaagctggagccgtccgggtcgccgcgctctatccggcggtccgcgttcaggggcaggccggcgatctgcagcttgagatcatactggtcggaccagaaccacgggacctccggcgcgggttgaggccggccggtaatggcggcggcggcctgcttggcctgctcgagcgcattaggcacgctttccagtcgccaggacacgccgcccagagccgggatcggccgccgcgtcatgtcgccgatggcgaagatcgacgggtttccggtcctcgcctccgcgtccaccaccacgccgttgtcgcaggccagcccggcggagaccgccagcgcgtcgcacgcaacggcgccgacgccgaccagcaccgcatcggcttggacggtcccgccatcggccagagtgacgccgttcgccgccacggaccggacctcggcgccggtcaggatctcgacgccctcggcgcggtggcgtgcggtgaagaaatcggacagggtctgcgaggcgacgcgcgccagcacgcgcgcctcccgctcgatcaccacggcctcggcgccaagcgcgcgcgccgacgccgccgcctccagccccacatagccgccgcccacgaccgccaaccgcttgcccgggcccagcaccgccttcagccgctcggcgtctcgcagggtacgcagttccagaagctccggatcatcgccgcctgaaaccggcagctttcgcgcggtggaacccgtcgccaggatcaggatgtcgtaggtctcccggccgccgtcggcgaacgtcacggacttcgacaccgcatcgacagcgacgacggtgaccgaccggcgaaagtcgatgcggtgttcggcgtagaagctttccgggcgcagcagcagggcgtcgaggtcagcctctcccttcagccaggccttggacagcggggggcgctggtaaggcggcgcggcctcctggccggccaggacgatggcgcccgtaaagccgtactgtctcaggaacgcggcggccgaaccgcccgcatggcctgcgccgatgatcacaaccttggtcatgaggcgctaaatagagcggcgtgcggcgggtggcgagtggcgggccgtcttctctcctccccatcgcggatggggaggtggcgcgaggcgacgcctcgtgacggagggggttgtgtcagcgacgcagaacccctccgtctcgtcggcttcgccgccgatccacctccccgttcgctgcgcgaacagggaggagagcgcgctcgccacttccgctgttgaccgtttcatcgttacagcataatggaacacgccatgccgccctcgcccgcccgctcagccctgtacgacgccatcctgtcgctgaagacgcgcgaggaggtggaggcgttcatggccgacctgtgcacgccggccgagctgcgcgcctttggcgagcggtggcaggtggcgcggctgctggacggcggcggcaagtcctatcgtgagatcgccgccgaggcgcacgccagcccgacaaccgtggtgcgggtcgcgcgttacctgaaagacatgccgcatcagggctatcgcctggcgctggatcggctgaaagcctgaaagacctcctcaaatgagcactgttcagggacggcttcgcatcgccgtccagaaatccggccgtctggccgaccgcagcctcgacctgatccgcgacgcgggcctgaagtgggtcaagggacacaacgacctgctgtatcgggtcgagaactatcccatcgacctgctgcgggtgcgcgacgacgacatcccgaccttcgtggcggacggcgtatgcgacttggggatcgtcggcgagaacgtgctggaggagggccgaaacggcgggcgcgacgccgagatcgtcatgccgctggggttcggccgctgcacgctgaagatcgcgacgccgcccgccctgccctatgaagggcccggatcgctggaggggttgcggatcgccacctcctatccggccatcctgcgccggttcctggacagcaacggcgtgcaggccgacatcgtcaccatgcgcggcgccgtcgaggtcgcgccccggctgaagctggcggcggcgatctgcgacctggtgtcgaccggcgcgacgctggaggcgaacgggctgggggccaaggacacggtgctggagagccaggcggtgctgatccgctcgccggtcgcgccagagccggaactgacggaactgctggacagcgtgatcgagcggatgagcggcgtggtgtcctcgcaaggggccaaatacgtcatgctgaacgcgccggtcgcggcgctggaccagatcacggcgctgctgccgggcgcggggtcgcctacggtgatgcagctgtcgggacgcgaggacgcggtcgccgttcacgccgtctgccaggaggcggtgttctgggagacgctggagaagctgaaggccgcgggcgcctcggccatcctggtcctgccgatcgagaagatgatgtgatgcggcgcatcgactggagcagcctggacgccgccgggcgccgcgaggccctggctcgtcccgcccggcgcacggccggggacgtgaccgatgcggtgcgtcgcatcatggacgacgtgaaggcgcgcggcggcgcggcggttgcggactgggcgatgaagctggacggccacgtgccgcgccgcatcgccatcacgcccgaggtggtggcggaggctcgaagcgccctgccgcccgccgacacccgcgccatccgcatggcggccgagaacgtgcgcctgttccaccaggcgacccggccggaggacacgccgtatgtggagaccacgccgggcgtgcggtcccggctggcgtggcggcccatccgggcggcgggcctgtatgttcccggcggctccgcgccgctgttttcctcgctcttgatgctggcgatcccggcggaggtcgcgggggtggaccagcgggttgcggtcaccccgccgtcgaaggacggaggcgtccacccggccatgatcctggcggcggccgagagcgggctggacgccctgtggctgctgggcggggcgcaggccatcgcggcgctgacgttcggggccgagctggacgacgccgtcatcgcgccctgcgacaagctgttcggacccggcaacgcctatgtggccgaggccaagaagcaggcggcggccctgtcgggcgggccggccgtggacatgccggcgggaccgtcggagctgatggtcatcgtcgaccgcgacgccgcccccgagatcgccgccgccgacctgctgagccaggccgagcacgacgccgacgcccaggtgatcctggtctccaccagccgcgccaccatcgactacatcctgacggaggtggaggcgcaggtctcgaccctgccgcgcgatgcgatcgcgcgcgcgtcgctgcgggaagcgcgcgccgtgctggtgcgcgatctggacgccgcctgcgaggtcgccaacctgtacggccccgagcacctggcgatccaggtggacgatccggaggcgctggtcccctcgatccgggcggccggagcgttgttcgtggggcggcacgcggccgagacgctgggcgactacgccgccggccccagccacgtcttgccgaccgacggcggcgcgcgcacgctgggcggggtcacgaccgccagcttcatgacctccatgtccgtccaggtggtggacgagaagggcgcacgggcgctggcccccatcgcggcgcgtctcgcccggctggaggggctggaggcgcatgcgcgggcggcggacatgagggccgagcgatgaagtccgggcagaccctccccgccccctttgcgccgctggtgtccggcggcgaaggcctggagaaatatccgggcgacgcgcaggcgctgcgcgcgcgcatggccgaggtgtatcgcgcagcacccgatcaggtgctgccggtgcgcgggctgacgcacgggctggaactggtctggcggctggccgcgcgcgacggcgggtcggtggaggcgccgaacggagagccgttcgaccggctatccgccatctatccggcgcgcggcgcgaccgtcgccacggtgatccgcgcccttggatcgcccgaagcggtgacggagatcgcgcagcggatcgcgcccgcgttgctgatcgtggacgaaggcctggtcgagttctcggacgcggcctcggccgtcgcgctgatcgaacagctgccgaacctggtggtgctgcgcagcctgtcgctggcctttgggctggcgggcgcgcgggtcggcgcggcgatcggtcagcccgaaaccctggcgaggctggacgaggtgatggagccctacgccctgcccgaaccgctggtgcggctggccctgcaggcgctggatccgtcccgcatgctggagacgcaagcgcggatcgccacagtgcgcggcgaacgcgagcggctagcgcgcgagatcggccggatcatgccggtggagccgggcgtcggccccgccctggtcgcgcgacccgaggatgcgcacaccctgctggccgatctcaaggcctatggcgtcgaagccggactggccggcgaacggctgcgcctgccggtgtcgctgaagcccgaggccaacgaccggctgctggcggcgctgggtctggcggggcaaaatcgccgcgccgcccgcactggccaagccgtgcgcgacaccaaggagacacgcatcgtctgcgccgtcgatctggacgcggccggcccggtgtcgatccacaccggcgtcggcttctacgaccacatgctggagcagatcgcggcgcacggcggcttttcgctcaggctgtcatgcgagggcgacctgcacaccgacccgcaccacaccatcgaggatagcgccatcgccctcggccaggcgctgaagcaggcgctgggcgagcgcaagggcatcgcccgctacggcttcgtcctgccgatggacgaggcggaggccaaggtgtccatcgacctgtccggccgcccctatccggtgttcgaggggacgttcgagacgcccttcatcggcgactaccgcaccgacctgaccgcgcacgtgttccgctcgctggccgaggccatgggggcggcggtgcacatctcggtgacgggccgggacgaccaccacaagaccgaggcctgcttcaagggctttggccgcgcgctgcgccaggcgatccgggtggagggcgacgccgtgccgtccaccaagggggtgctgtgatggtcgatcgatcctccccccgggggagggggaccgcggagcggtggaggggctcgccccagacacccttgcggccgtccgccccctcacccgctgcggtggtcccccccccgttgggggaggagctgatcgcgaggtcacggtgatcgcctacggcgccggcaacgtcgcctccgtgcagttcgcgctggagcggctgggcgcgcgggtgcggctgacggacgaggcgtcggtggtggcgcaggccgagcggctgatcctgccgggggtgggggccgccgcctatgcgatgagccggctgcgcgcgctggggctggtggaggcgatccacgcgtttcagcggccgctgctgggcgtgtgcctgggccagcagttgcttttcgagcgcagcgaggaaggcgcgggcggcgacctgctgggcttcattccgggcgcggtgacgcggctcgatcccggtcccgccctgcccgtgccgcacatgggctggagccggctggagcgggtgcgcgacgatccgctgctggaggggatcggcgccgacgactacgcctatttcgtgcatggctacgtctgtccggacggccctgcgaccctggcgcgcgccgactacgggggaacggtgccggcggtggtgcgtaaggaaaaccgttggggttgccaatttcaccccgagcgctcggcccgcaccggagcgcagatcctcagaaacttcattgaactgcccgagaccgccgcatgctgatctatcccgccatcgatctgaaggacggcgtctgcgtgcggctgatgcagggtcggttcgatgcggtgacccgctatgacgaacagccggcgctgcggctggcgaccttcgcggcggagggcgcggagtggatccacatcgtcgatctggacggtgcggaggccgggcgcgcggtccagcacggcctgatcggcgaactggtcagcgccatcgacgtgtgcgtccagtccggcggcggcgtccgcagcgccgacgacgttgagcgcctgctggaggcgggcgtgcaccgggtggtgatcggctcgctggcggtgacgcagccggattcggtgctgagctggctggatcggttcggaggggaccgcatcaccctggcgctggacgtcaagatcgagaacgacgtgcccgttccggcgctgaggggctggacagagtcctcgggcgtggacctgtggacggcgctggaccgctatccccgaggcgtcgccaagcacctgctggtgacggacgtgagccgcgacggcgccctgacggggccgaacctgcagcttctgtccgaaatccgcctgcgtcgccccgacatggttttgcaggcctcgggcggagtggcctcgctggacgacatcgcggcggtcaaggcgctgggctgcaacggcgcgatcgtcggccgcgccctgtacgaaggccgcttcaccctgcccgaggcgatcgcggcggcgaaacggacgtgaccgcccggcggatcatcccctgcctggacgtcaaggacggccgggtggtcaagggcgtgcgcttcgtcggccacaccgacatgggcgacgcgggcgagctggcggcgcgctatcgcgacgagggggccgacgagctggtcttctacgacatcacggcgagcccggaaggtcgcacgctggactacggctggatccgcgacatcgcccggcttctggacatccccttctgcgtggccggcggcatccgcagcgtcgaacaggcggcgcgctgcctggatcacggggccgacaaggtgtcgatcaactcgcccgcgctggagcggcccgagctgatcgccgaaatggccgagcggctgggctcgcagtgcgtggtggtcggcgtcgacagccgcctggaggacggcgactgggtcgtccacaaatacaccggcgacccggaggcgcggcgcagggcgggcaagcgcacgctggactggctggaccaggcgcaaggcttgggcgcgggcgagatcgtgctgaactgcatcgatcaggacggggtgcgacggggctatgacgtggagcagctggccgccgcccgccgccgcctgaccattccgctgatcgcgtcgggcggcgccggcgcgcccgagcatttccgggacgtgttcgaacaggcggacgtgtcgggcgccctggcggccagcgtcttccacacgggcgcgatcggcataccgaacctgaagcgctacctgacggacgaaggactggagatgcggctgtgatcgacccctcgagcctcgacttcgacaagggcggcggcctgatccccgccgtggtccaggacgccgacaccctgcaggtgctgacgctggcctatatggaccggggggccttgaacgagacgatcgccagccgcgaagcgaccttcttttcacgttcgcgcggcgggcggtggagaaagggcgagacctcgggcgatcggctgcatgtggtcgcgatcacgcccgactgcgacaacgacgccgtggtgctgtccgtcaggccggtcgggaacgcctgccacctgaaccgcatcagctgctttggcgaagcggacgcaccggggctgggccgcatcgcgcggctggaaaagaccatcgcccagcgcgccgcggccgatccggacgaaagctggacggctcgcctgcttcagcaaggccccaagcgcatcgcgcaaaaggtcggcgaagagggcgtggagacggcgctggcgggcgttgccggccccgatgcggaactcgcgagcgaggcggcggatttgatcttccacctgcttgtccttctccatgcccgtaacatggtgtttcaggacgtgctggacgtgttggccgaacgggccgaagcgggcaaaggcgcgggataggccaagcacggccgttgtcccgggatctgggaccatccgggagacgacatggcggcactcatcctgttcggcggcggcggcgacctggcgatgcggatgctgctgccgtcgctgtatttcctcgagcgggacggactgctggccgaggggctgaagatcatcggtgcggcgcgttcggacgagagccgggacgactatgtcgccaagattcgcgaggcggtggagccgcgcgcccggagcgatcaggcctgggatgaagccgcctgggaccggatggaggctcggctcgactatctggcggtggacgcgaccgaccccgaaagcctgaagcctctgaaagccaaggtcggcgacgacgagatcacctcgttcctcgccgtgtcgccgtcgctgtacggccgcatcgtcacggcgatgaagacggccggtctggccgaacgcaacagccggctggtggtggaaaagccggtcgggcgcgacctcaagtcgttccgcgagatcgacgacgccatctcgcacgccttccgagaagagcaggtgttccgcatcgaccactacctgggcaaggagacggtgcagaacctgatcgccctgcggttcggcaacaccatcttcgagccgctgtggaacaacctgacggtggaccacgtccagatcacggtgggcgagaccgtcggggtgggcgatcgctggccctattatgacgagtacggcgcactgcgcgacatgctgcagaaccacctgctgcagctcttgtgcctggtggcgatggagccgcccagcgacctggaccccgactcggtgcgcaacgaaaaggtcaaggtgctgcggtccctgcgccccatcacgcccgaggaagccgagcgcgtcaccgtccgcggccagtatgtggcgggcgagctggagggcaagccggtcaagggctacgacgacgagcgcggcgaggactccgacaccgagacgttcgtcgccgtgcgcgccgacatcgacaactggcgctgggcgggcgtgcccttctacatgcgcaccggcaagcggatgccggaaaagcgcacggagatcgtgatccagttcaagtcggtgccgcactccatcttcgccaggggcgaccggggcgaggtctgcgacaaccggctggtgatcgagctgcagccggaagaggacatctcgctgtcggtcatgaacaagcgtccaggcctggagcgcaacatgcagttgcagccgatcaagatgtcgctgtcgtggggcatggacgacaaggacgcccgcccgccgcgccggcgcatcgcctatgagcggctgctgctggacgcaatgaacggcgacaacaccctgttcgtgcgccgcgacgaggccgaacaggcgtggaagtgggtggacgaggtgtcggaagcctgggagggcgcgggcttcaagccgcacgactatcaacccggaacctggggtccggacgaagccgaaatgctgctggcgcgcacaggccgccgctggaacaccaccgatgcgtgacatgcccgtgattgaaaccttttccacccgcgacagctgggccgaggcctgcgcggcgcggatcatggagacgctggttcaggcggtggaggccgatggcgcggcctttttcgccggatcgggcggatcgacgccctcccccatctatcgccgcatggcgggcgtgggcggcgtcgactggagccgcatcaccacgaccctgatcgacgagcgctatgtgcccgagacctcgccggactcgaacgcccggctgctgaaggagacgctgctgacgggcgaggcggcggccgccacgttcatcccgctgtacagcccgcaagtgacggtggaccgggcggccctgatcgcctcgcacgccctgaacgcagtcggccggccgctggacgcggtgcttttgggcatgggcgaggatggccatatctgctccatgttccctgagaatcccgcactgaagcagctgctcgcccccgacaacccgccgcgcgtgctggccgtgggcaagagccgctcgacctccgctccgccgcaggaccggctcagcatgaacatcccctggctgcggggcgcccggcgcaacatcctggccatcaccggcgaagccaagcggcgggtgttcgaggaaaaggcgctgggcgatcccaccgacacgccgatcgccgccttgctgcattcgggcgccgagcttgaagttctctggacggaggccgcctgaatggccctgcaccccaccatcgacgccgtcacccggcgcatcaccgagcgcagccgcgggacgcgcacggactatctgcggcgcatggacgccgcccgcgacaacggcgtggcgcgggccaggctgtcctgcgccaactgggcccacgccttcgccggccagacggtggcggacaagctgaccgccatgacgggctcgcagcccaacgtcggcatcgtcaccgcctacaacgacatgctgtcggcgcatcagccgtttgagcgctttccccacatcatccgcgaggccgcgcgcgaggtcggcgccaccgcccaggtcgccggcggcacgcccgccatgtgcgacggcgtgacccagggccgccccggcatggagctgtcgctgttcagccgcgacgtgatcgccatgtccacgggcgtcgccctgacccacgacgccttcgattccgccatcatgctgggcgtgtgcgacaagatcgtccccggcctgttcatgggcgcgctggcgttcggccatctgccggtgatctttgcgccggccgggccgatgccgtccggcattcccaacaacgagaaggcccgcatccgcgccctctacgcccagaaccaggtggaccgcgcgaccctgctgcaaagcgaggtcgggtcctatcactcaccgggcacctgcaccttctacggcaccgccaactccaaccagatgatgatggaggtgatcggcctgcacatgccgtccaccgccttcgtccaccccgagacgggcctgcgcgacgcgctcacggcggcggcgggcaagcgcgcggtggatctggcgcgcgcgggcgaaagccgcatggccgacgtggtggacgaaaaggggatcgtcaatgcgatcatcgccctgctcgccaccggcggctcgaccaaccacgccatccacctggtggcgatggcccgggcggccggcatcatcatcgactggaccgacatggacgagctgtcgtcggcgacgccgctcttggcccgcgtctatcccaacggctctgccgacgtgaacgccttccaggcggcaggcggcgtggcgttcgtggtgcgcgagctggcgcagaacgggcatctgcataccgacgtcaccacggtcatgggcaaggggctggagccctactaccaggagccgtcgatggtggacggccagctggtctggcgcgacggcgtgtccgagagcctggacctcgacatcgttcggcccgtctccaacccgttccagaaggacggcggcttgcggctggtcaagggcgacctcggccgcgcggtgatcaaggtctcggcggtcaagcccgagaatcgcatcatcgaggcgcccgccgccgtgttcgagacgcaggaagacgccttgcaggcgttccgcgacggcaagctgaaccgcgacgtggtggtggtgctgcgcttccagggacccaaggccaacggcatgccggaactgcatagcctgtcgcccgccctgtcggtgctgcaggacaagggcttcaaggtcgccttcgtgaccgacggccgcatgtcgggcgccagcggcaagacgccggccgccatccacgtgtcgcccgaggccttggccggcggtccgctggctcatgtgcgcgacggcgacatcatccgccttgacgccgaaagcggcgtcctgaccaccgtcggcgcgggcgagctggcggctcgccccgccgcgcagcggtcgcagagccacgccgacgcctcggcctggggctatggccgcgagctgttcggcgcctcccgccatgtggtgaccacggccgaacggggggcccccgtctgcttcgccttcccccccggcgagccgtcgcctacggatacgcccgccgatcccaacttcgtcgaccggaccgtggacgcctgatccgccgaaccgaccgcaggaaacgaccagatgaacgataagacccttctcgtcggcgacgtcggcggcaccaacgcccgtttcgccgtcgcccgcatggtcgacggccggccggtgctggagcaccacgaaagctttccggccgagcgccacccgacctttctggaaggggtgcgggcctttatcgacggctgcgaggtcaagcccagcggcggcgtgatcgccgtggcggggccggtgacggacggcgccatcgacctgaccaactcgccctggcgggtgtcggaagccgagctcggcacgctgggcctgcagcccgtcaggctgatcaacgacttcgaggccctggcctggggcgcgcccgtggtgcccgaggatcagctggaaagcctgggcggaccggcgaagggcgacgaggacgccgccatcgcggtgctgggccccggcaccggcttcggcgtctcggccctggtgcgcgacgcccacggccagcagatggccatgccgtcggaaggcggccacgcctgcttcgcccccggcgacgcggtcgaggacgagatcctgcgcatcctgcgccgccgctatgatcgggtatcgatcgagcggctgatctgcgggccgggcctgttgaacatgcaccgggcgctggcagagatcgaagggcgcgagacccatatcgacgacccggccgagatcacgcgcgaggcgctggaagaggccaacagcccgtgcggccacacgctggcgcgcttctgcgccatcctgggcgcggtggccggcgacatcgccctgaccaccggggcgcgcggcggcgtctatatcgccggcggcatcgttccgcgcatcctgcccttcatcaaggccagtccgttccgcgagcggttcgagcgcaagggccgcttcgcagactacatggccgccatcccgaccaaggtgatcatgcacaagcacgcggcgctgctgggctccgcgcgcgtggccttcgccgaggcgggctgagccatatagtcacgagcgcgtgaaccgaagcggcgctgtggcgttctggaagctccacaatggaagggagcatcccatgaagaagatcgccatcgccgccgcctcgctgttcgttctcgccggcgtcgccgcctgcggcgaaagcgcgaccgaccgcgccgccgagcaacaggccgacgcggtcgaagcgcagggcgaagcccgcgccgaccagctggaggcgcaagccgccgcgacgccgaacgagcagcaggaaaccgctctcaaccagcaggccgatcgcgtcgaagaacaggccgaccgccgcgccgaccagatcgagcagcaaggcggcaacgccgacggcggcatgaccaccggcaacacgccgtccgcgcactaagctcggccggcttgcagaaagcccccgtcgcgatgcggcgggggctttttcgcgccttctcctcctcatcgcgcagcgatggggaggtggatcggcggcgatcagccgacgagacggaggggttctggacgacggaacccacccctccgtcacgaggcttcgcctcgcgccacctccccatctgcgatggggaggagagatcagcggttgtcagtcgatgcagataccaacgccgaccttgccgtcctcgaccgaggtgtgacagccgaagttgtcgctgtcggcctgacagacgccggcgacggaggcgttgggcgcgggcggggtcgcgccgtcaggcaggcggcagtcgccctggcactggtcgccgtcggtgcagcgctttcctgcgtcggcgtagttcaccacgcactgccagctctgcaggcggcccacctgcttcagggttccgccgcgctgggtgcaggcggaggcttcgacgcttcgcaccgggccatccgtcgtcggggtccgcgtttgcggcgctcaactggccagcagcagggcggcggcaagcaaggtcgggcggatcatggaggctcctaggggggggcgttttcgaagaacagttgagggcgtcaaagcggcggcgctgaggcaacggtcaagctggcgggagcgttcaccgtgcgaaaggatttcccatgacctatgtgacgcgcggcgtattcggcgccgccagtctgttgctgctgctgtcggccatggggctggtggcgttcggggtcgaggacgcctggcagcagatgcgggcgccggacgcctcgggcgccgaggccatcctggatctcttgggctacatcatcgtggccatcgctgtattcgacgtcgccaaatacctcttcgaggacgaggtgcggcgcggcaacgaaaagcgcagcgcggccgaggctcggcgcagcctgaccaaattcctgtccaccatcgtcatcgccttgttcctggaagggctggtggcggtgttcaagaccgcccgcgaggacgtggcccagctgatctatcccaccgccctggtggtcgcctcgaccctggtgctggtggggatgggcgcctatcaacggttctcggccaccgtcgaggagaaggtcggccacaccgacaaggccgaagaggccaaggaggacgcccgccgcgacggcgactagacccgcgtcggcaggaagggcgaaaaggtgatcacggtgaaggtgtcgcgcacatgcggtcgcgtctgcacctgcctggtcacgaaggtgccgatgtcggcgtcacgcggcaggttgaacttggccagcaggtcgtgctggcccgaggtcgaatagacctccgagacattctcgacattgtccacgatgtcggcggcgacgtcgttggcgtagcccagctcgcatttgatgaagacgaagatggcggtcatcatggcggcggctcctgcgctgtcggtcagggccgtgtgttagcggacggcgggatgacgggcgagcctgaactgagcgctgaacagcttgagcagcaatacaacaaccgcgcccgggtccccgatcatccggcggtgatggcgcgctggaaggcggggtcggaagccgcgcgcgcggcgcacccgcccgagcgactggcctatggcgcaggcgagcgggagcggatggactggttcgacgccgggccgggtgcgccggtcgccgtcttcatccacggcggctactggcaggcgctggacgaaagctggttcagcttcgtcgcgccgccgctgctggcgcggggcgtcagcgtggcgatcccgacctatgacctggcgccgcaggtcgggctggaccgcatcgtcgagcagatgcggatggcggttgaagctgtggcggcgcgaacggacgccaagccggtcgtgacgggtcactcggcgggcggacacctgtcggcctgcctgctatcggaagggcgcgcgcgggcggcggtggcgatctcgggcgtgttcgaactggcgccgctgatccccacctccatcaatgctgcgctgcggctggacgcgttcgaggcgcgcagactgtcgcccgcagagtggccggcgccggcgggcgcggtgctggactgcgtcgtgggcggcgacgagagcgccgaattcctgcgccagagccgcgacatggccgaacgctggggacgccacggcgcgcggacgcggttcgaccccctgcccggcctgaaccacttcaccgtgctggacccgctgttcgacgccgacagcgccctggtgcggcgcatcgccgagttggcgcggatatttagataaacatctagcaccaaaaaacgaatacgtctgccgcaaccacctcagatgatcagcttcattatattaagaaaggctatctgacggtgcaaacatcaccgacgcagtcaaatgcagaatctctagctttctcgagatccgatcgattatcttcaggtttacataaactaacggttgcacaagccaataacgcgatgacaccggcaacaatataggatgactttcgatccgctttgtcctgagcatgagaaggggcttccccgactggaacataagctacggcagcttccgaataagtcattttcgaagcggcatcgtagactcctagggcgcatgctcgggcgatcactagacgcttcccgacaccgcgcttctctgcaatcacctcagccaatgctggcgatactgatctgtgcgccttcaggtcagaatctataatcacacgacgagccgtcggatcattttcatttgccattatgatctcttttccgcgggcttgtttcaattcttacgctaccatagcagccacaagttcgccacagtcggagggacgcgcctctcgtgcaccggtgcttgatcaggaaaagctactatgcggccgcctcgccccgccgtcgctcgtcgagccaccacatttcatgattgctgggatggcttgaaagtaaagcaaaatgctatccaggcggccgaactaggcatccccgaccatgtcggggctcggagaggaacacatgctccacgaccgtctcagcgtcctgaacgccctggaaagccaaggcgtcgcgccggtcttctaccatcccgatcccgaggtgtgcctcaacgtcatccgcgcggcggcgcgcggcggcgccaaggtggtggagttcaccaatcgcggcgacttcgcctgcgacctgttcggcgagatcaaccgcgaactgagccgcaccgacccggacatcatcctgggcatcggctcggtggtggatagcggaacggccgcgctctacatcaaccggggagcgcgcttcgtggtcagcccgtgcctggttcctgacgtggccaaggtgtgcaaccgccgcatggtcgcctacttccccggctgcggcagcgtgaccgacatcagcaactcgcacgaactgggctgcgagatcgtgaagctgttccccggcgcctcggtgggcgggccggacttcgtcaaggcggtgaaggggcccctgccctgggtcaagatcatgcccaccggcggcgtcgatccggacgaggcctccatcgccaaatggttcggcgccggcatcgtcgcggccggcatgggctccaagctggtgaccgaccaggcggtgcgcgacggcgactgggccggcatcgaagcccaggtcagaaagaccgtggacgcaatcgccgccttccgcggcaccaagggggcctgatcttcagggcctgatcgtcagggctgcgtcggagccggggaaggcgtctccggctttcgggcgtcgctgcggcgggccaggatgggcgccagcgcacggcgctcggccggcgacaggcgggccatgatggtcaccgcattgctctccagccgcgcgcgtccgcgcatctcggccaagcgagcctgctccatcaacgcctggacttcggcggagttgaacggctcggccgaggcgcgcccgatcgcctcgcggcgcgccgcacgcgcagtgtcgaagtcgggccgcgccgtcagggccgaggcgcgcagttcggcgcggatccgctcgcgcgcttcaaccggcagcggctgcagcagcgcgccgaggcggtcctcgcgcccgggtttcgcctgcgcctccgcctgcttcacagcgcggtcctgggcgatccaggcggtgacgccgcccgccacggcgaacaggttcaccgccaccgacagcgccagggcggtcttcagcgcgcgcgggctcactcgggcgcctcggccagcacttcggcgtcgtccacgctggtgaaggcggcctgggacagcaccgcgtcggcgcgcgcggcctgcgtcgcctgggtggtgacgcccaagcccgccaccacgccggcgcacgccgcggccgcccatccggcgcccagcgtcagccgcagacccacacgccagcgcgtcagccagccgtcgccacgcggcgtcagcccggcttcgatcgccgaggccagcacccggtcgcgcagggccgccgacggcgcaaggtgcggcgacgcgtccagcaggcggttcagatcgcggtcgttcatccccaatctccgttcctagctccgggcgccagatcggccagcgccccacgcagcgcccgccgcccccgcgacaacaggctctccagcgcctcgacgctgatctccatggcggcggcggcgtcgatgttggtcatctcctgatggtggcacagcaccaccgcctcgcgctgacgatccggcagccgccgcagcgcggcgtccacccttgcgcccgtctcggccgccagcagcccgcgatcgggggcaggcccctcgtccggacgatccggcggggtctcggtcgcgatttcgcgccggcgccgcagccggtcgtagcagaggttcagcgccacccggtgcagccaggtgtcgaacttggcctggccgaagctccagcgcggcgcctgcctccaggcgcgcagcatggcgtcctgggccacgtcctcggcctcggccgcatcgccgagcattctgttggccaggttcagcacgcgcggaagcttgcgtgcgaccatggcctggatcgccgccgggtcgccccgtcccacgcggcggaccaaatcctcgtcggggtcggcgctcgcggccaatcacgcctctttcgctgccggccgggaggtccaccctagcgcgtcgcagcgtgcgaaggcgagacgcccgtgcgccgccccttgcttgcgtgactgatgagctttggcccacgcgccgacatccccttccgtggcttgcatcaggttcaacggtccagacggccgcttccgtcgccggaattcagcacggcctcgaaggcggcgcgggcgcgggtgcgcagcgcctgcagatcggccttgagcgtcgggtagtcctcggccccgacggcggcggccaggcgggcgtggaacggctcgggctcgccgtctggatcgacccgaccgtcgaaggcggcggcgaggatttggctgagccgctgctgggtgcgccaggcctcggccaggacgggatcgtcggccagggcgtccagggtcgagggcgtcagcggccgaccctcggccgcggcggtcagctgacggtgctgggcggcgaactcggcgtcgacctggccgccgggcgacagcttcaggtcccagaacccctgcggccgccgctcccggtccatcaggccgcgcatccgcagcacgtcggccgccacgtcgacgccgggccggggcgcgcgcagcacccgttcgatccccgcctccacttcaccggcgaactcgggatcgctggcccacacgacgcgggcgcgcgtcaggaccatgaactcccaggtgtcggcctcgcgccgataatagtcctcgaacgccgacaggcgcaccgcgaccggccccttggagccggtggggcgcaggcgcatgtccacctcatagagcccgccctcggccgtgtgcgccgacagggccgagatcagccgctgggtgaaacgggcgaagaacacctcggccggccagcccctggtctcggaggcggcctccggcggggcggcgtagagggtcatcaggtcgaggtccgagctcgccgtcatctcgcgcgagccggccttgcccagcgccaccaccgcgatgcgcccgccgggcagggcgccgcccagccgctcggtctcgtcccaggcggcgggcgccagggtgcgcatggccgcatcggccagggccgcataggcgaggcccgccgcctccggtcccgcgcggccggtcagggcgtgcatgccgatgcggaaagcctgttcgcggtgcaggcggcgcacggcgttcatgcgtccttcgaagtcgccggcctcctcggcctcccgcatcatctgctcgccgaagccgtcctgctcggccaggtcgcacaggaagcgagcgtccagcaccccgtccagggcggcgggctggcgcgccagggggcgggccagacgcggcgcaaaggccatcacccccaccaccatggcgaacagccgcggctggttcaggaacagggcctgcacctggaccccgtgcgacaggccggagaagaagccggcgaaacgggcgaaggcggcgtccggcgacccggtctgagccaaggcctccaagaggcggggggccaggcgcgtgaacagctcgcgcccccgcgcggtccgggtcgcgaggatgcggccatgatgccagctgcggatggtgttcccgaccgacacgggttcggagaagcccatgcggcgcagggtgtccagcgtctccggatcgttctccacgccggtgaagacaaggctgccgtaggacgaggacagcgtctcctcgccctcgaacagctcgccgtagcggtggttgacgccgaacagcaggccctcgacggcggcgtcgaacaggccgaggtccgcctcgccggacagggcggcgacggcgcggcggcgctcgggatcggccggcaggatgtgggtctgctcgtcgtcctgcatctgcacccgatgctccagcccgcgcagctcggcgtaggcggaggcgagctcttcggcgacgtcggccgagatgtgtccggccccggccagggcgtgcagagcctccaccgtgcggctggagcgcagggctggatcgcgcccgcccaggatcagctgctgggtctgggcgtagaactcgatctcgcggatgccgccgcggcccagcttcaggtttgcgccggccgcctccagcccctcgccggtcttgtggacgtggatctggcgcttgatcgactggatgtcgagcacggcggcgtagtccaggctgcgccgccagatgaagggctgaagcgccttcaggaaccggcgggcggcgcgcaggtcgccgcacaccgcgcgcgccttgatgaaggccgcccgctcccagttctggccgacgctctcatagtaggccagcgccatgggcaccgcgaccaccggcggagtcgaggacgggtcggggcgcaggcgcagatcgacgcggaacacatagccgtcggcgttgcgctccatcagcaggcccgacagcgccttggccgcacggtccacgaatgtctgcggctcctcgccgtccctcagcgccacgcccagcaggcgcggctcgtagaagagcgagatgtcgatgtcggaggagtagttcagctcgtccgcgccgtgcttgcccatggcgatgccgaacaggccgggaaccggaccgcgcgcatcgtcggcgggcgacagcagccggcccttcgcccgctgctcggcgccgacggcgcgaagggcggcgcgcacggcggcgtcggcgaagcgcgacagggcgagggtgacctggtccagatcccagacgccgcccacatcgcacagggcggtcagcaggtgcaggtcggccttgaggaggcgcagcggctggcgcagcgcatccggctcgccctccagcacgtcggtttcggccagcaggcgcccaagctcggcgtcggggtcggcctccaagagcctgcgaaggcgggctggtcgtcgccgcatcagtccggacagatagggcgaggcgccggcgacgggcgccagcgccggccaggcggcctccagcagatcgatccagccgtcgccctgcgccgccgcgcgcagcgtctcgtaaagacgctcggccgcattcgcatccacgacgggaccggcgggacgcaggcggcgggccagagggggcggtgcggacgtcatgccctcttgtagatcaagtcggcgcgggcctcacccctgccctgtggcggccggcagaaccagggcgacccgcaggccggggccgaagccctcgaacacgccggggccctcgtccagctgcacccggccgccgtgcgcctcggccacggccgtgaccagcgaaaggcccaggcccgagcccggctcggtgcggctgttgtccaggcgcacgaagcgctgcaccacccgctcgcggtcggcgtcgggcacgccggggccggtgtcggtgacggagtattcgacctcgcccgaggagcgacgccgcgcccgcagcttcaccgccccgccggccggggtgtatttgatggcgttgtcgatcagattggccagggcctgcgccaggaacgcccggttgccctcgaccagcaggccgcgctcgatctccgagccgaagtccagcgacttgtcctcggccgccggctcatacagctcggccatgtcggcggcgaggtcggcggcgtcgaacaccttgggatccggcgcgccgccggcctggagccgggcgatggccagaacggtgttgaaggtcttcagcagctggtcggcctcgtccagagcgagcgtcagcgcatcgaccccgtcgatcctgccggactccgcgtcgatcagggcgacctccagcttggcacgtatccgcgtcaggggcgagcgcaggtcgtgggcgatggcgtcgccggcgtggcggatcgaggccatggacgcctccagccggtccagcatgccgttcagccccaggcccagttcatccagttcatcgccggagtggcggatgccgacgcgggccttcagatcgccgtcctgcacggcggcgaccacgcggttcagcccgcccatggccgcctcgacccggcggctgatgaacaggccgcccgcaagccccagcaggatcaccatggccatggccgcccacaacgcctgggtcaggcgggacagatagtcctcgatgtcgccgatgtcctcgcccacgaacaggtggcttccgcccgacagcggcatcagcacgccgatggcctgacggcgctggacgcgcccttccggatcggtgtcggtgatgcggaaggtgtcccactgaccttggcccggcgtcaggttctcccccgcctcgaacggcagggtcgagacgttgccggtgatcgtctttcccgccgggtcggtcagcagatacaggtacgggccgccccgcaccgtgcgctccaccagggcgatgttcagcgcatccagcccgcgcgtgcggtggatggcggtcaacacgcccagttcggcctccacgtccgccgtcgcccgcgcctgcgcctgcgacgccgaggcgaaatagacataggccaggatggcgctggccgccgccacgaacagggcgagaaacagcagcgtcagccgaaacggcgtgcggcgaagaagggacggcaggcgcatgatgcgcggtctaggcctccagccggtaccccgcgccgcgcacggtctggagcatggccttggcgaaacccttgtcgatcttggagcgcaggcggctgatgtggacgtcgatgacgttggtctgggggtcgaagtggtactcccacaccttctccagcagcatggtgcgggtcaccgactgaccggcgtggcgcatcaggaactccagcagctggaactcgcgcggctggaggtcgatctcagtcgtcccgcgatgcacggtgcggccgatcaggttcatctcaaggtcgccgaccttgagcaccgtctgcaccccgcccgtctcgcgccggcgggccagggcctcgacgcgggcgatcagttcggcgaaggcgtaaggcttgaccagatagtcgtccgcgccggccttcaggcccgtgacccggtcctccacctcgcccagagccgacaggaacaggaccggcgtctggtcgccgccctttctgaccatctcgaccatgccgacgccgtcgagacgcggcatcatgcgatcgaccacatagacgtcgtagccgcctttctgcgcctccagcaggccaaaggccccgtccaccgcatgggtcacgtcgtggccggcctccgacaggccgcgcaccatggccgtcgccgcctcagcgtcgtcctcgaccaccagaattcgcatgacgccccctctccggaatcaaaatcgccgccgatggtagcgcatcggcggcgatcccgtgagttaaggcttgttcagcttccagatcagtcgtttccgcccagacgcatcacgatggtgcccggcgactgtccggcctgcacgaacagcaagacgctgtcccggcccgcacgacgcgcctcgtcgatcacggcgcgcagatcggcgggcgtggcgaccgcacgctggttggcgcgggtgatcaccatgccggcctgcagcctgacgttggcgaagttgacgctgtcggcgacgttggtgacgaccagaccgttcaccgattcaggcacgttgaagcgttggcgggcgctggcgctcagcggcgacacggacacgccttcgatcacctcgccgccaccggggaccgcagagcctggcgatccggagcccccgtcctgcgaagcctgaagctcggcctgcgaggggcgaacgcccgaccggacattcagcgtctgacgacgaccgtcccggatgatgtccagccggatcgtttcgttgggtcgcgcggagccgacgcggcgcgtggcctccgagctgttcgccaccgcttggccgttcacagccacaaggatatcgcccacccgcgcgccggcttgggcggccgggccgtccggaaccacgctctggacgtaggcgccgtcgaagtcggacggctggccaaaggcttcccactcctcggggcgaagcgtctgtagcgtcaggccgacatagccccgctgaatgctctcgcccctcataagccgcgccgtgatgctcttggccgtctccgccggaatggcgaagccgatgccgaccgaaccgccggtgggcgagtagatggccgagttgacgccgatcacgcggccgtagatgtcgaacgtcggtccgcccgagttgccccggttgatggcggcgtcgatctggatgtagtcgttgtagccggtcggatcgatgtcgcgcgccttggccgagacgatgccggcggtcgccgtgccgcccaggccgaagggattgccgaccgcgatgacccagtcgccgacgcgcggctcggccgtctcctcgaaggagacatatttgaagtcattgccttcgaccttgaccacggccaggtcggtgccctcgtcgcggccgaccaggcgggcgggcagctcgcggccgtccgacagcttgaccttgatctcggtggcgtcggcgacgacgtggttgttggtgacgatgaagccgtcctggctgatgaagaagccggagcctgcgccctgcgccgtctggggctcgtcgccgccgccctggccctgcgggggcacgaactggaacggcaggccggggatggtcagggcgcgcgggcgctcgacgcgtgtggtcacgtcgatctgcaccacggccggggcgacctggtcaaagatgttggcgaagctgttgggcgcgcccggcggcggggcgaaggcgccggcggcgcccgggttgggggtgatgcggttcaccgcctgcggctcggcgtgcgcgcccggccaggtgatgacgcctccggcggtcgcgcccgcggcgatcgtcaggccggcggcggcccccagaatgaactccttgcgcttcagcatcgtcgtccttgcgatccttgtgtccggcgcgacaaggcgccgttttcgcttttgaatatagggcgatgacgacgttcgccaagccgccctaacggagggttgatccgtactagcgcccgtcgtgaggcgaggttgcgtccgcatcgcggcgaaggctttccggtttgagaagttcgtccagccgcgccttctcctgatccgtcaagggctcggtgtcggccgccggccggcggacccgccacagcaagacgccgccggccagcagcgccagcagaaggggcccgaaccacagcagcagcgtgccgatccgaaggggcggtcgaaacagcacatagtcgccgaagcgacgcaccaggccagcgcgcacctgttcgtcgctggcgccgcccgcgatctcctcgcgcaccagccggcgcatgtcggcggcgacggcggccgggctgtcggcgatggcctcgtgctggcacaccacgcagcggatctcggagaacagggcgcgggcgcgggtctcctgcgccgcatcgggcaatggcctgtcgggcgcggacgccggctccgccgccatcaggccgaccgccatcagcggggccagcaggatgcgccgcttcacgccggcctccgacggcgggcgggcgccgcgacccgcaggcggcggtccatcagcgacaacaccccgcccaacgccatgatcgccggccccaggaagatcagccgcgcccaggggttccagtacagccgcacgttccaggcgggacggccgtcggcctccgtccgctcgcccagcaccacatagacgtcgctaaggccgcggaagtcgaggccgacctcggtggtggtctggccgcccgcgggaaagaagcgacgctcggcggtgacggtgcgggcgcggccgtcgtcgccgctcggccgaacggtgaagcggccctgctcggcgaggtagttggggccttcgatcacgcgcacatcgtccagccgggcggaccagccgccagcgaccaccgcctcgcccagagccagcggccgcccggtctcggccttgaagccggtctcgaccacggcgcccagcacgaagacgccaaggcccgcgtgcgccagggtcatgccccaggcgccgagcggcagacccttggcccggcgcagggtctcggaaggcggcgcgcggaacaggcggatgcgttcggcgacctcggccagggcgcccaggatcagccaggagcccagcgcgacgccggcggtcgccaacgccttgcgaggctcccacaccgcccagcccgccaaccccagcaaaagcgacaggccagccgcgacccacagccgctgggccgcgccgcgcaagtcgccgcgcttccacgccagcagcggcccgaacggcaggatcagaaaggccagcgccatcagcggcgtgaaggtggcgttgaaatagggcggaccgaccgagatggtcgcgccggacgccgcctccaggatcagcggatacagcgtgcccaggagcaccgtcgcggcggcggtggtcagcagcaggttgttcagcaccagccccccttcgcggctgatcggcgcgaacaggccgccgcccttcaggcgaggcgcgcgccaggcgaacagggcgaacgccgcccccgccgtcaggcccagaatgcccagcagcatcagccccctttgcggatcgacggcgaaggcgtgaacgctggtcagcacgcccgagcgcaccagaaacgcccccagcatggagaaggtgaaggcgagaagcgccaggaacaccgtccagccggccagcgccccccgccgttcggtcaccaccgccgagtgcagcagggccgcgcccgcaagccacggcataaaggaggcgttctcgaccgggtcccagaaccaccagccgccccagcccagctcgtagtaggcccagaaagaccccagggcgatgccgacggtcagaaaggcccagctagccagggcccacggccgcacccagcgaccccaggccggccagaacggcgtctgggcgcgcccctcgatcagagcggcgacggccagcgagaagcagacggagaagccgacatagccggcgtagagcagcggcggatggaaggcgagcgccgggtcctgcagcagcgggttcagcgacgcgccctgcaccggcgcggggttcagccgctgaaacgggctggaggtgaacacggcgaaggccagaaagagcgcgcccaatcccccctgcaccgcgacggccgacgccttcagcccgaacggcaggccgcgcccgcgcgccagcaccgcgccgaagccggtcagcaccaggcaccacagcaccagcgagccctcatggctgccccaggcggcggcgaccttgtacagcatcggcttgtcggtgtggctgttggccgcgacattcgcgactgaaaagtcagacaccgcgaaggcgtagatcagggcggcgaaagccaccgcgacgctgaaaaaggcggccagagacgcgccctcgcccgccccggccagaaccgggctgcggcgcacgcggcccgcggtcgacagccccgcctgcagaaccgacagcatcagcgacagcgccagggcgaaggccccgagttcgacgatcacaggcgcgacgcccccgccggaggcggcgatccgctctcggggcgccactcgcccgtcgccttcagccggtcggccacttcgcgcggcatataggtctcgtcgtgcttggccagcacctgatcggcgtggaaggtgcggtcgggcgagaacgcgccctgcgcgacgattccctgaccttcgcggaacaggtcgggcaggtcgccgtggaagacgacgcgggtcgtcgccgcattgtcggtgaccacgaatgcgacggagccgtcgttcgcatgctggacgctgccggcctcgacgaggccgcccagacggatgttgcggccggcgggagccttggcctcggtgacttcggagggcgagaagaagaaggtcacgctgtcctgcatggcccacaacgacaggccgaccgccagcgccaggatcggcgcggcggcggcgaccccccacagcctgcggcgcgcctttggcgatttgggaagccagctcacgtcaggcgatgctcgaaactacgggtcggacctgcaagccgtatagcggcgcgaccgccgcgatccaatgcgtcacgatccgccgccgggcagacggcgctccagatcctggcggcggggatcgccgggatccagggcggcgatcagcggtgtccaaagctcgcgcgcgcgatccgcgtcgccgcgccgcagagccgcctcgcccaggaagaagcgggcgcccagctgatcgccgtcgcgcttcagggcctcggcgaaggccgcctccgcatcggcgccgatgcggtcctcgttggcgcgcaccagactttcgcccagccgcgcccaggttgcggcgtcgtccgggcggatcgccagcaggcggcgaaaggccgaagccgcgcccagcggatcgccggcctcgaagcgggcgacgcccagcatggccagggcctggggatcgcccggccggctgtcagccacgcgcgcggcgacggccgccagctgcgccggctccagcgtctcgggtcgggtcgcccactcgtccacgcggcgctcgaagccctgatccggcagtccgggcgagccggtggccagatacaggccaagcgttgcggcgacgcagaccagcaccgcccccagcacgacggggcggtcgccgcgtcccgcgacgggcgggcgcggacccgccgccgtttccgccagaagccgccgccccgcctcggcgcgggcggcggcgtgcgcgtccgcctcaagcaacccgcgcgccttgagccgatccagctcgtccagttcgcgacgcccttcggccacgtcgtcgccagcagcggcgacgcggacgcgggcggcgccgagcaccagacaggcggccagggcggaggcgagcgcggcgaggctccagaacactatcatgccggcaggcttaaagcatcagccgatcgggagcgaggctcctggcgcaaggtcgccgatggccagggcggcttcggatgcggccgcacggcggcgcacggcgcgcgcggcgtccagcgcgcccagctcggtcaggaagcgcgcggccgaaccgaccaggcgcaaggcgccgtccgcgtttgtcgcctcgccgtcgttgatctcgtccagcgcctcgttggcccaggtcgacagatagtccgacagttcgtggccgatccgcgcgcgctcggcctcgtagcccagcacgccgccggccgatcgaagaccttcgatcgacggcagcagttcggcggccagcgccatggcctcgccttcgggcggcgcttccagccagggcgcgaggcgcctcatgcggccgacaatggtccgcttgtgctgcggcagggcggcgtgcacggccgaggcggcggactggagcaggctggaggccgcgcccgacacggcgacgcgcgccagccgcgccgactggccccaggcggtgtccggcttgagtggcagcgccaggtccagctcggccaggacgtcggcgcaccacaggatgtcggcggtgatccgggcgacgttgtcggcgctgaagcggcggctggccccgccgatccgctccacccgcgcctggatcgcctgaagcagccgttcgacgaagacgcccatgtcggactggctgagcacgccctgctggtcggccagcttggaggtgcgggtgacgacacgcagcatccgcccggcctcgggcgcatgggcgaacaggatgtcgaccaggcgccgaccgcccgcctcggagacagcctccgcgtcgcggatcagcaggcgcaggctggccagctgctcggggtcaggccggtcgagccatgcgggcaatgcggaaacgccgacgcgcgccaggtgcgccagatcgaaacagcccgccagttccgccacgcgcggatcgccgggatggccgccgcccggccagacgtctcgaggatcgtcccgcagcagcccggccgcacgggcgcacaaacggtccgccgccgtggagccgtccgcgccgccggtgtcgataaaggcggcgagcacaggctcctcgcgttccacccgacgccacaaggcgcccagcaccgagggaggaaagctcaggctcggcgtttcgtcggctcgaggacgaaacatcggcagcagcggcgcaaaggcgacgcttcggcgcctgcggctggcgccctcatggtccagcatggccgcgagctcgaccgcgccctcgccgggcagagccccgaccgccgccgtcagcccgcccagaaccgcgtccgggcaggcctggaccacgcccagcagcgcagatcgacgagcttgcgaaagggcgggcaacgggaccctccttcaaacgggaaggtccagcttgcggccgcagcggttaacaaccgcttggagcggcgatcaggcctcggcggccggcagctccagcaccgccttcaggccgcccagatcgctgtcggccagggtcagccgcccgccgtaggcgcgggtcaggtcgtccacgatggacaggccgaggcccgagcccggcgcatcctcgtccagccgggcgccgcgcttcatcacctcgtcgcgacggtcggcgggcaggccgggaccgtcgtcctcgatcaccgcgatcatctggcccaggccgttcgggccggccgagacgcgcacgcggcgcctggaccatttggcggcgttctcgatcagattgcccaggatctcctgcaggtcctgacgctcgcccagaaaagcgaggtcgtcgggcgcgcgccagtcgatctcgacgttcttggatgcgaacacccgctccagcatgacggccagttcgtcgacgacttcgcccaccggcgtgctttcgcccaatccgtgtgcggcgcgggcggcggcgcgggcgcggcgcaggtgatggtcgacctggccctgcatcaccgccgtctggcggcgcacgatctcggggagggctccgtcctgcgttccggcttccgccagcatgacagacaggggcgtcttcagcgcatgggccagattgccgacgtgggtgcgctgacgatccaccacctcctgattgtggtcaagaaggcggttgacctgttcggccagcggctggatttcgatgggataggcgcgttcgacgcgcgcggccttgcccttgcggacggcggcgatctcgttcctgagttcatacagcgggcgcaggcccacctgaacctggatgaacaccgccgtcaccaggccgaagcccagcaccagcagggcgatccaggtgatggtggcgaactggcgcgcgtcggcgtcgatgttggagcggtcgatggcggccaggaacaccaccggctgctcacgccccggcaggcgcttcatgctggcggcgacgcgcagcggctcgtcggctggacccagggcgttgtagctgatggtctgaccgaacgcctcctccagccgtcgtggcaggtcccgcggcaccaccagatcggcgtcgtacagcgactgggagcgtgtcagggtgcgcaggcggttctcccctgtcggctcggcgaccacccagtatttgccggaaaagacgcgcagggttcgcgcgtcctggatctgaggcgtcagcaccgcatcctgcggcgtcacggtcgagcgcaccaccagctcgtcaatggaggcgctgagcacattgcccagccggcgcagcgccgactcctggaactgattggtcagcaccaggccggtgatgaccagggctagcacgatccagccggaggccaaccagatcaggcgccgcgtcagcgacctgcccggccgcccgatccatcggccccagccgttcgcccccgccatgcgtgccccttacgccgcctccgcctcgcccgccagcggcgtcagccgatagcccaggccgcgcaccgtttcgatgcggtccgagccgatcttcttgcgcagccggccgacgaacacctcgatggtgttggagtcacggtcgaagtcctggtcgtacaggtgttccaccagttcggtgcggctgatgacccggccctggtgcatcatcatgtagtgcagcagccgatactccagcgaggtcaggcgcagcggctcgccgttgacgctggcgcgcgccgcgcggggatcgaggcgcaggccgccgcacgacagggtcgccgccgcatgcccccgcggagcggcgcagcagggcccgcaggcgcgccagcagctcctccgtatggaagggctttgtcagatagtcgtcggccccggcgtcgaagcccgacaccttgtccgaccaggccgcgcgggcggtcaggatcagcacgggcgtggtctttccctcacgccgccagcgctccagcaccgaaacgccgtcgatcttgggcaggcccaaatccagcaccaccacgtcatagggttcggtgtcgcccaggaaccaggcctcctcgccgtcaggcgcgtgatcgaccgcatagccggcgtcggtcagcgccgtcttcagctggcgcgacaggtcggcgtcgtcttctacgagcaggatgcgcatggctcagcgttctccaaggatgcggccgctgcggccgtccacggtgatgtcggccacccggccgcccggatattcccaccgcaccacgaccacgtcgccgcgcgggctgacgcccagcatgcggccctggcggcccgaagccacgcggcgcaccacgtcgccgagatcgaggcgctggggcgccgcctcaacttgccgttcgcggcggtcgttttcgcggggacgtctcgactgatcgtccacgggcgccgctgcgacggcggtcgacatggagacggcgagaacgagtggaacaaggaaacgaaacatggccgtggagataacgagccccctctgaacagccgctgaacaagacccgcaggtttcgagcgcataggttgaagagatcggcccggaggcgtggcggcgacgatgaacgccaggtgacgcgggccattcagatgcggctcaggcgacatgcgtcaggttcccagccatcgcagccgcttccgactgcgccgcatcgcaaaggaacgatccgatgatcaagaagacgctcatccccgccctggcccttcttgccgcctccgtggcgctgcccgccgcggccgcccaaccccagcacggtcatggccgcccgccggtttatgccgacgccggaggctggaacagcatcaacgcccgccaggcgaatctggaccgtcgcattgatcagggcgtgcgcaacggctcgttgagccgccgcgaggccgcccgcctgcgcagcgagttcggctcgctggttcggctggaggccaactatcgccgcggcgggctgagccgctgggagcgtgacgacctgaaccgccgcttcgaccgcctggccgcccagatccgcaacgagcgtcgggacggggacaatcgtcgcggctgatccctcccttttgcaggacacgggggcgcggctcgcaaggtcgcgccccttgtcgtacatcgaagctgtcggctgcggatgatcgaccttgcgggaaccgggcgacgggacgcgcgtatcagggacccatctgaagagaatatccgcgcgatgatcccccagaccttgtccgctgtccccgccacggacgccgtgagcgatccggacgcatttcaccggcgcatgtcgcgctggaacaatcgccgcctggcgccggccacgcctcacgccggctggcgggacgatgcacgcgaggacgccgagatgatccttctcgagggcgcgtttgtcgagcggatgcgtcaggaggcccaaccctggctgaaggacctgccgaccgacgtggacggcttcgtcgcctggttcgagaacctgcaggggaacggccccggcgaaaacgacccgctgttcccttggctggcggaagaggccagctacgaggagatgcgctggttcctgctgcaggaggtggcgggcgaggccgggttcgaggacctcgtcgcctatgcccaggtcaagatgccgacgcggcccaagctcgaactcgcccgcaactactgggacgagatggggcgcggcaacgagggcggcatgcacggccccatgctgcagaagctggccgacaagctggacctgcaccccaccatcgagggcacggtgtggccgtcgctggcgctgggcaacaccctggtcgccttctccaccacccgccgctacgcctatcatgcgctgggcgccttgggcgcggtcgagctgacggcgccctggcgggcggatcatgtggcccgcggcctgaagcgggtcggcgtgggcgccgagcgcaagtatttcgccctgcacgccaccctggacgtcgaacactcgcgcacctggaacgaggaggtgctgcgtcccctcgccgccgagcgtcccgagtgcatccccagcctggccgaaggcgcggtgatgcggctgatggccggagcgcgctgtttcgaagcctaccgcgcccacctgtgggccgagccgcttcgtcaaagcgcctgaaccatcaggaaacctatcagacgctgcgcgtaaatctcgccgcgtcggcgcgttgaccgaaggggtccgcgcctcaatatcgccgtgtgtcgggcgacctcccccgcccgacacacggagcctttcatgtcgcccacaaccaagcccgagcaacgatcgcgcgcgatgacgccgcgatgtcagcgcgcctgacggtcggcttcggcctcctcttctccgacctttcctcttcaacggcgagccttgcgctgcatcggcgcctgtgcgccggccttttcaggatttctgtaagatgacttcttccactcgacgccgcgctcaggtccggttgcttgcggccgcatcggcgacggccctgctggcggcgagcccggcgcttgcgcaatcggcgtccgccacctctccgcaggacctgacggacgacgcggcgggaacggagaccacggtcgacgacatcgtcgtcaccggcacccgcgcgcccagccgttcgcgtctggacaccctggcccccgtggacgtggtcacggccgagacgctggagacgcgcggcaccaccgagttcgcggcggccctggcccagaccgtgccctcgctgtccttcccccgcccgtcggccaacgacggttcggacacggtgcgtcccgcgaccctgcgcggcctgtccccggaccagacgctggtgctgctgaacgggacgcgccgtcacgcctcggccctggtcaacgtcaacggcgtggtggggcgcggctcggcggccgtcgacttgaacaccattccgacgcccgcgctggaccgggtcgaggtgctgcgcgacggcgcctcggcccagtacggctcagacgccatcgccggcgtggtcaatctgcgcctgaaggaagcgtcgtcgggcggcggcgccagcgtgacctacggtcagtacgtcaccgacgtggagaccgcgcgcggcgcccgtgacgaggaggacggccagagcgtcaccgcctccgcctggcagggtttcgccctcggctcggacggctttctgacgctgtcggcggagtacaccaaccgcgagccgaccaaccgcgccgactatgatccccgtccggccgccaacggggcgatcaccgcgcgcttcggcgatccggaggtcgagcagtggaccgtgttcgccaacgccggcaagccgctgaaccagacgtgggaggcctacggctgggccggctaccagaaccgcgacagcgaaagcgccgcttttccccgcctgtcggacaacgccaacaacgtcccgacggtctatccgaacggctttctgcccatgatcggcgtcgaggccgaggacatctcgggcggcaccggcctgcgcggcgagatcgccggctggttgtcggacttcagcgtcgtctacggccgcaacgccctggatttccgcaccgaaaactcgatcaactcgacctatggcgcgaactcgccgaccagcttcgactccggctcgctgatctatgaccagctggtggtcggcgccgacttcacccgcccgttcgagatcgggctgtccggtccgctgaacttcgcctggggcgccgaataccgccgcgagacctatgaaattcaggccggccagccggagagctacaaccgcggcccggtggccggcgcggccttgcaggccggatcccaggggtttgtcggctttcaaccatccaacgaggtcgacgccgaccgccacaacatcgcgctctacgccgacgtcgagattccgctgacggacaagctgaccgtcgagggcgccgtccgctatgaggattattccgacttcggcgacacccggaccggcaagttttcggcgcggtacgacttcaatccgaacttcgccctgcgcggctcgatctcgacaggcttccgcgcgccggcgctgcagcagtccttctacacctcgaccaatacggtgatccaggacggccagccggtcgagaccggcaccttcccggcgaccagcgcggttgcgacggcgctgggcgcgcgcccgctgaaggccgagacctccaccaactattcgctgggcgcggtggtgcggctgggccgcttcgacctgacggtggacgcctacaagatcgacatcgacgaccagatcgtgctgtccgagctgatcggccggggcttctcgccccaggtcgccagcctgctcgatccgctgggcgtgtcgtctgcacgcttcttcctgaacggcgtgtcgacctccaccgagggcgtcgatgtagtcggtcgctatcgcctgccgaccgagaccttgggcgacttcgacttcaccgtggccgccaactacaacgacatcacggtggaggagacgccgacctcctcctcgaccctgaaccccgttcccccgctgttcggccgcaaccgcgtgctgacgctggaggacggcacgcctgaggtgaaggtctcggcctcggccgactggagccgcgaccgcctgggcgccacgctgcgcgccacccactacggcgacgtgctgcagccgggctccacggcggccagcgattatcgcacgggcgccaagacggttgtggatctggagggccgctatcagctgaccgaccgcgtcggcctggcggtgggcgtcgacaacctgttcgacgaatatcccgactacacgcccgcttcgctgaacaacaacggcgtgctgggcttcccctattactcgccgttcggcttcaacggccgctacgcctacgcgcgcgtcagcctgcgctggtgaggccccgagcgcccgtcgccccagggcggcgggcgttctccgccgaggcggtcagcgcagggatttgctgacccgcacgagcgacgggtcgccatcgatagccgacgcctcaaagcccatttcacgctcgatctgaagggcgctgcgatgggcgtggttctcgatggactcgatgacggcgtagccgcgcgcccgggcgtggccgaccaggtagtcgagcatcgaccaaccgatgccccgccctttcaggtctccccgcagcacgaccgcggcctcggcgcgctcgccttccccatcgccggccaggatcgccgtcgccgccaccgagccgtcgtcgataaaggcgaccaggctttcgttgcgggcgtcgttggcgcggatcatcgccaccaggcgctcgtggccgacatggcgcagggtcgcgagaaaacggaatcgcaggtcttccggcgtaaccgaagcgaagaaggcggcgagggcgggttcgtcctcatcgcgagtgcgcctgacatgcagccgcacgccggcgcgggtgatgatctgttcgctgtcgtgatggttcatggcggtctccttgcaccaggcgacgatggacgcgcccggctggctccgcattgaccctgatcaagccggcagcatcgtgcctgtctccatgaagcgacggtgccaggacagcgcctcgcccggcagggacggggcgtgcaggccgtaggatccgccgtgagcccgcgccgcataatcctggagcagggggcggtagtcggggtgtgcgcaccgctcgatcacctgcctcgcacgctggcgcggcgacaggcctctcaggtcggctagaccctgttcagtcacgatcacctgcacgtcctgcatgatgtggtcgacgtgggaggcctgcggcacgatggcggagatcttgccgcccttggccatcgacggggtcatgaagatcgagacataggcgttgcgcgcgaaatcacccgagccgccgatgccgttctggatgcgcgagcccatcaccagggtggagttcacattgccgtagatgtcggcctcgatcagcccgttcatcgcgatgcagccgaggcggcgcacgatttccggatgattgctcatctcctgcgggcgcaggatcatgcggtcgcggtaggcgctcatgtcggcgttcagccgcgccgccgcctgggggctgagcgaaaaggcggtggccgacgccatgcgcagcttgcccgcgtccagcaggtcgatcatcccgtcctggatcacctcggtataggccgtcatcggctcgaagggcgcgtcgatcaggccggacagcaccgcattggcgatgttgcccacgcccgactggatcggcagcaattccggcggtaggcgaccgcgcgacacctcatgcgccaggaagtcgatgatgtgcccggcgatggcgcgcgccgcgtcgtccggcgccgcgaacggcaggttccggtcgggggcgtcggtctcgaccaccgcgaccaccttgtcgggatcgcaggcgaaaaagggcgtgccgatgcgatcgtccggccgcaccagcgggatgggcacacgctccggcggcaggcgcgtgccgtagtagatgtcgtgcatcccctccagcgccgggttctgccagcggttgacctccaggatcacccgccgggctcggtccagccaggtcttgttgttgccgaccgaggacgaagggatcagcgagccgtcggcgcgcaccccgacgacctcgatgatggcggtgtcgagcgtccccaacacgccctcccaggccatgggagccacctggctgaggtgcatgtcgagatagtcgatctcgcctcggttgatcttctcccgcgcgacgggatccgagctgtagggcaggcgctgggcgacgccgtcgaccgcggccaaggcgccgtccagttccggccccgtcgaggcgccggtccagagattgacgcgaaagggccgtccggcggcgccttcggccgccatgcgccgggccagcgcctgcggcacggccttggggtagcccgagccggtgaagccgctggttgcgaccgtctcgccgggctggatcaggccggcggcggtgtcggcgtccgtgacgcgggcgcgaagcgcggcgcaggcgatgcggtcggtcatgcgggtcctcgaagacgattggcggtgcggggcacccctcgcgcgttcaggcggccctgtcgagcacgatgggctgaagtgcgtcgacggggcgtccaggtggaggatgtcctgttccgcctcgtccatccggacgcagggtcgctgtcagcaacggtcaggttgagaagcctagccgttttgcatgactgactatcgactgcacctcgtccgccacggcgtcaggaccgaagaaggtttggagggagtcgatgacgccgacgctctggcgctcgcgcgcatccatgtgctgtccgacagctccatcacccacgccatgctggttcatcgcgacggccgcagcctaggcgacatccagactgacgtgagttcgcccgctttgcgctgagatagcgcacctgatctcgtcgccttccgcgacacgcggcggagccgttccgtcgtacgctgcggttcccctcgcccggccgcagcgttcctcggcttcagcatgccgacctaggctcaggactcatagccagaagagcacggtagcggcgagggctatggcggacaggaagacgttcgggcatcgatcatagcgggtggcgacgcgccgccagtctttcagacgaccgaacatgatctcgatgcggtttcgccgtttgtagcggcgcttgtcgtagcgaatgggctcagtgcgggttttgcggcctgggatgcagggcgtgatccccttggcctgcaaggcgtccctgaaccagtccgcgtcatagcccctgtcgcccaacagccattgcgccttgggcaggctgtccagcagggctgcagcgccggtgtaatcgctgacctggcccgccgtcacgaacaggctgatcggacgcccattcgcatcggtcacggcatgaagcttggtgttcatgccgcctttcgtgcgaccgatcagtcgcccgaggcccccttttttacccgcaggctcgaagccgtgcggtgcgccttcagataggtcgcgtcgatcatgacggtgcgacgttcggtctgagcgccagacaggccctccatcatccgaacgaacacgccagcttcgctccaccgcttccagcgattgtagagggtcttgtgcgggccataagccgctggcgcgtcacgccagcgaagcccgttgcggttgacgaagatgatcccgctcaacacccggcgatcgtcaaccctgggcctgccgtggctcttgggaaagtgcggccggagccgctccatctgctcgtccgtcagccaatataggtcactcatatccagactcctcgggagcctgaatcagatccagcgcctcacatcaatgggtcctgagcctagtgcaattctcgcaacagcagcagtgaacgccagaagggtagcgcgatagcgaacctcatccgcagccttcatcgccctcgtgcgatcggcaacaccagccaagcgtgagaacagatcatcagctagcgagcaaagcgctgaactcggctgatcgacaggcatcagcaccgccgcgctcgcggctgccttatggcgcacaaccatgatcaggcctcaccgctcctgacaaaccgacaaggtttgccgatcacgcacgcatccagacgcggacgcgcgcccccagcgcccgcttggcgcccagcctccggcacaacacagacccgagcccgccagaccggccgatcgcccacaccaagacgaaagccgtgcaattagagccgtcctgacagttggtcaagcgacaaaaagcagttgccacgcgcttgcttctcgcctgacttcagactagcgtgcgccgcctttagcaaaatgctggaaaatctcacatggatttcttctacgttatcgataccccgtttgcaactactatcaaagacgctttctctgatctttctgaacatctttctcttagtgaatatgtttggattcgcgagaacttggagtatgaccggttcgaagaagggtcgatcaccggagatgggcgggccttggcgacgctgttccggtacatcctgatggctgacaagcagcacgctgacgacctcgccaatcccttcgccactgcggcaaggttgatcaaagacgctggagtgacgaccaatccggacgagcagttccggggcggcaccctctgcaagctcgctccgcaggatgatgaggaggcctaagcagaccggaagagtcccaacgatgagccctgacgacgaccaacccaatggtggcccaccccggcgaacgctgaagcgacgatccagagtaagccagtctgaccttgatcgcgtcttcaaggccagcaagcagcaaggggtcgaggtggagttgatctacgaccattttcgtgtggtcgtcaggcgctcacccgacgagagcgatgaagccaacgagtgggattctgtcctgcccgatcattgatatacaaggccatggcgaagattgatctaccgtacgtgcaaggcttccgggatcggcatggcaggctgaggcactactaccggcggaaggggatgcctcgcactccccttcccggcctgccgggctcccgcgagttcatggctgcttacgaacaagcctgctcccgcgacgcaccagagagacctcatcaggcaagacacggttctcgttcagttcatgccttagtgggtcaatattttcagtcggcagagtttctagcgctgcgaaccacaacccggggagcttatcggcgacagatcgataggttcagggcacagcacggcaccaagagcgtctccgccgtccaaccgcgacacctcgaagcgatctttcacagtatggccagcactccacatgcggccgcaaacctccggaagcggctaaggcgggtattcgctctagctgtgcggctgggctggaggaacgataatccagttcgggacaccgagggccctaggttgaggacagagggtcatgtgccttggagcgatgaggacatcgagaagttcgaagcccgatggcccacaggaagcagggagcggctcgcattcgcgctcctgctctacactggccagcgtcgctcagatgtcgtgacgatgggcatgcagcacgtgtcagacggccggatcagcgtcgtgcagttgaaaacgcagcaccgattgaagatcaagatgcacaccgctctgatcaccgaaattgctgatcgttctgggatgagcctgctcacgacccgcagcggagcgccgttcacgacagagggcttcggcaactggttcagagatgccgtagcagcggccggactatcgaatcgctcacctcacggattgcgcaaggcagcgggccgaaagctcgcagaggcgggatgtaccgctaaagaaattgcggcagtgcttggccacaccaccctcactgaggtggctcgttacacccgagacgcggatcaggtgaagctgggagacagtgctttggtaaggtgggaagaggccgaagcaagaacatccggagtcaaaccggtttgacaaacccgacctaacccgttgtgaccactgctaaattataggtgcatggcgaccccgggaggactccaacctccgacctcggctttaggaaacgatctggggttgttttcaccccgtctcagttggtttcatttcgtaacgattatcacgtagaaacagtatgttcttgcctgacgccctaagtaggtcgtaacctctggtttcatctggtgcgtcccatttgcgtcccaagtgggtgattctgcgtcccagttgcgtcccaagttttctggaggggtaagatcatgccgtgcgtcaatctcaccgatcgttaccttcaaagcgtggtcgcaaaggctggatgtcgcgctgagttttcggacgcctcgaccgcaggcctggccattcgcgtgagcggcaaggcgtcgcgagtgtgggtcatgcgctatcgccgtccggacggtcgcgagacccgtcaccgccttggcgagtatccgacgatgagcttgaaggctgcccgcgtcgaggtcggacgtctgcggggtcttatcgagaggggcggcgatccggtccgcgaacggcaagaggcgaagcagcaggcccgcatggaagcggttgcgacctatggcgtgctgctcgacgcctactggaaagcttgcgaaaccggagagtggcagcccaagcgcaagatcaagcgcgccacgaccctcgcctatgagcgcagactgtcggcccgacacatcgagcccgtgctcagcgcactaccgctcgcatccatcaagcgcgccacgatcaaagcgctgctcagggacatggtcatgaaagggatcggcgcacagacaaatcgggtccaggccgtcatccggcaggtctttaacttcggaatcagcgaagaactggtcgagatcaacccggccatggggtttcccacccttcacgcgccaacaccgcggcgccgggtctggaaggacggggagctgcgccttctttggcgttcgctggcgggggagacctcgctggtcacgcctgcgggcactgaggtttatgtgggaagaggcacgcgaatcgccttgcagctggcgatccttctcctgcagaggcgcaaggagatcgccgggatggacttgtccgaactggacctggaccaggccgtctggctcatccccgccaagcgcatgaaaggcaaccgcgatcaccaggtgcccctgcccccgcggtcggtggccttgatccgggaggccatagccctgacccggctgcccgccgaccggacggtcgggccggtgtttcccaacccgcgcctgcataccgaggccatcagtcctgaggcgctcacgcgcgctatggaccggttgcgggattgcctcggcgtggaggatgcgacagtgcacgatctccgccgaacgggagccaccgcgctcacgagcgaacgcctgcgtgtctcgccctttatccgttccaaggttcttggacatgagacggacacgggcggcggcgcgtcggtctcgagcatccactacgacgccaatgaatacatgaccgagaagcgggcggcactcagcgcctgggagagcctgctgctgcagattgtcagacgcgacgacgatggcgacgccgctccacgtcgcaccggcgtcatacgcggcatgatgttcggccttgagcccgccaatgacgtcggcccgatcgatgcgctggcctccgaccgctgacagccccttccgctaccgagcgggtttgatcgagcccacatcctgcgaagccgccgtcagcggcgagcgttcgaagcgcacgcgttccgagcccgccaggagcgtggccgagaacccggcctgcccccacgcccttgtttgaacgccttcggccgtccaccaggcgtcggcgaacgccgcctttggcaacaaggcccggatccggcgttctatgtcgctgaaggtcagctcgagagtgtcggccttctgtcgtcgcaggaagctcgccagcggatcatatttccccatggggggctgtttagccggaccacgccgcctcgcaaggccgggcctccctgccgccggcgctccctgctccgacgccacgcgcccgccctctcagaacccgaagtcgatctgatcgagcggaaccgcgcgggccttttttctccgctttagagcgggcgcgagaatggcggccgcttcaggcgacacgcgcgcctccggcgtcgcggccacctcgggtgcaggggcgcgacttcgcggcattccgggcagccgcggcgccttgggcggcttgaacggaccctggctgcgcgttcgccgccacgccatcagttcgctttgccaccagccgacccggccaggggagagggcgacaggacgcggaaaggcttcgatgcgctgcagccgccatatcgtcgtgcggctcaggccggtgatctcgtgaacacgcggccaggccagcagctggtcctcgggaccgccgacgtcgagctctgtgggtgttggaggatcagacacgtcgccgcgcccaggctgcggcgggcgccgccgtccggacctccgtgatctggctcaaagcccagtcgcgtagcagcccgcgtgggtagtggggcctgtggcggccgggcaagccatcgccgccggtcgaccagagcctagccagggtcgcaggcttcagcctgatcccaggaccggccaggaaagccgaggcccccttcggcgtcagcaggtcggaggcgccgtcatccgtctgcgtcacgtgaccgtcgtcctgccggatcatggccggacctccgggcgggcgcaggcgcgcgcggagcgcacatcccggcctgcggtcagcgccaggtagcattccacgacggttgcgacataacgccgtgtttcggcgaacggcggcgcgccgccataggcagcgaccctcgcggggccggcgttgtaggccgccagggccagtcgcacgtcgccgaaccgggccagctggcgcgccagatagtcagcgccgccctgcaggttctccaccggatcaaaccggtcggccacgcccaggtcccgcgccgtcgccggcatgagctgggtcagcccggccgccccggcgggactgaccgcatcggcccggtatccgctctccgtcagaaccagggcgaacaggagtttcgggtcgatcccgtgtttcgccgccgcggccagcatggcctcccgatagggcggatcgagcgccggcagccgaaccgccgcctccgtctcgtcaggcatctccgaagccgcggcaggttcggacgcgccgaacagatcgccgccggcggcgccccaatcgaccgcctgggacatgccgggggcggcggcgaacacccacgccagcagagccaaccctgcgcctgttctcaccatgtcacagcctcccgatagactccctgcaactgactgcgctgcaccggcccaaaatatcggctgtcgaagctcgcctcggtgtctcccagcaggaagacttcgccgggcgcgaggtcgcgacaccccgaccagctcggcagagcgacgccccgcctgtccctgaccaggatcggcgcagtcgtccccgccaggacaagcctgtcgcctcgccggcagaccggatctccggcgacggccgccacccgcttcaacagcaggccattggggggcgcgccgagctgacggaggtagatccgcgccccggcgggctgcggcgcggcgaccacaacgccccgctccgccgttttgccgaagcggcgcagataaaggccgcgcgggaggctcggggtctcgttgatgaggacgagcctgggcaggtcgcacacagcggcgaccgagctcgcgcaggcgaccgcggccgccgagagcaggatccagccccgccctgtgaaggtgcgggtcatggctggtacggctccaggatcaggtcgcgggtgatcaggacccgcacccgccctccggcgctgacccgaatggcaggccggacctcaagctcgcgatcgatcagccggccgccgacgcgggcgccctcgatggcggcggcgtccccggcgtcgccaagcaaggaccggccggagtccccgccctcacgggcgatctggccaagcgtggtgatcgcccccgcgaacagggttccggtgatcagcgcgccgatccggcgatccacgcgtccgcgcaccccggtcgcgccctgcgcgtccaccccaggctccgcctcaagcaccaggctcttgccgttgggcaggatgagcctctcccaggccagaaaggcgcgccggtcgccataggcgctgtcgccctcatgcgtgcccagcagccgtgtcccctgggggatgagcaggtgccggccggtgaccgtgtcgtatatgttctgcgtcacggcggccacaaccggcccggggcgcgaggtgtcgacgccggtcagaagaaccgccggcacgatcgcgcctgccttcaactcatagggggagaccggcgctgtcagttcgtgacggttatagacgcctcgcgcgcccgcaggaccgcctggatcgagcgcggacgggggcgcggcgaacgtctccgtcctgtccgccgccaccgctcgggtcggctgcggcgggggcgcgccttcgaagaacaggctcgaacggaccgccagctggtttggtccggcaggcgcgggaccgatgctcgcggccggggccggataggggcgccgggcctgcgggagcggcgtcccgcgctccgctttctcctcgcctggcgccgcctccgcatcccttgtccgcggctccggcaaccggtcgtacgaggcgggctggtcggtcacctgttccgcaggccgcacagcgccgtgcgcctcgctctcccgcgcctcccccgcgcgtgaccgggccgacgcccgcagttccggctggaccacaaaggcccaggccagcgagcccgcgacaaggatgcagccgcccgcgaccacgacctggatcgcggatcgtctcagccgcacgacaggcggacgcggggcgcgaccctccaggtccgtcggccccgatttggcggcgggccggggcgtccccgatcccgctgctccagatgaccggtccggttcctggttctggacctcggtcatcgccgctctcccgcgagacgccggatacgcaccacctgcggccgccgatcccccagtcgcagctccgcccgttcgaacaggcgatcgacgacgaacaggccgtcggactggcggtagttgacgagttgcggctccccatccgccgcgatcaggaaaagcgccggcgcctcgccgacccggagatcgggcgggaaggcgatgaaggtgcgccgtccgtcgtcaaaaaccgccgacggggtccaggcgggtcgccggcccaccggctcgatgcgataccgcgcgttgaggagcgcctctgggacctgcgcagccgccgccggcgctgtcgccgaggctgcctccgccgcagccgggacagtccccgccggttccggcgtccgccaggccaccgccgggttgtacgcttccgccgatccgcttctcagcaggatcatatagatccgccggtcggtggcgagcagcagattggtctccagaccgcgctggagcggcttcagcaccacatgggtctgcagggccccgttctcgcccgaccggacctcgccgagctgccagcgcaccgtgtcgcccgcggccttggagagaagggtctcgcctggctccagggtcagggtggtcacccgcagaggcgcggtccagacctcgaacacccgccccggcgcccaggcgaacacctgcaccccgccttcgaaccggtccgatcgggacgcggtccgcgcctccgcattggccgcggcgattgcgcggcgccccgaccgcagagggtcgtccggcgccacataggggcgggcgtcggccggacgaagcggcgccggcttcgtctcgccggccgcggccgcggtcgccacgccgagacccagggaggcgccagccagggcggcggctgtcatcacgaggcgtcgggtgtccatgacacatccttgatcttgaggcccagggggttcttcatcagctcggcctcggtccggggcggctgcaggtcgatggtgatcagcgctcgccagcgttctgcgcccgccgtctgaccgttgacgaaccggctttcgcgccactgcagatcgaaggtgcggcctgagcggcggaccacgttcagcacctcgacattgatcgcctcgcgcccgacatccgcaaagggatcgtgggcctgggcccagccgttcaggaaggccgccgccctgggtgtgagcaggtcataggcctcgagccagttctgccgcagcacaatgggatcgatgctcttggagcgcacatcccggacccagccggccagcgcatggccgatctgggcgtcattgggctcatagcggccgccgatcgcggtgatcctctgggtctcgccccagtcggacacctcgaccacaaagggtttgaccacggcgcgatccgcctgaacccaccagccggcacccaggaagacggccagccccaggttggcgacggccatgcggcgccagttccgcgcatgggccagggacaggcccatgcggtcgtcccagacctggccggcgcgctggtagggtgtggcgtccggggccgaggtgaggacccgttggggtctgaagaaggggtgcatctcacgtctcctctgttttcaggtttggcgacagcacgccgctggtctcgccggagggcatcaggccgcgaccggagttggccacaaagaaggcctgcagcgcccgcgaccggccggacgcggacgaccccgttcggcgtggatcgccgcctgcggcggcgcggtggaagtcgctccgggcggcggccgtctcggccgcgcgcacggtctgcgaccgggcgttgggcggggacgcgtccgccgggctcccgtcgcccgcggccgggcacatccgcgacagcccgctcccttggttggagccgcccttcgacgggctgaaatccggggccggcccggcagatgcggtgcgggcgcccgctgaacggctcccgcctgaagaccaaccccctgccccgctcccgcctccgctccctgcgggcgacgctgcgggaacaggaggaggcggaggcgaagaccgccccgacccagcgccggcggccgcccgcgcgggtccggcgagccgcgccgcgccgcccagcgccgcccccgcgccgaccactccggcgccggccagcagcccgaccccgccgacagccatgccgccggtcagcgccgccccggcgccgagcgacgggccgccggtgaccagggccgccgcgaggttggggatgaacatggccagcatcgccagcaggatggcggcgacaaggatgctgagcgcctcgtagatgtcgggattggtcgagggctggagttgatcaaagatcgtccgcgcgccggacacgaccacggccagggccaggaccttcagccccgaagacaccacatagccgagcggccgttcggccagaaaggcggtgcggttccagatcccgaagggcaggagcacgaagccgcccagggtgacgatcttgaactcgagcagggcgacgatgatctgcagcgcgagaacggcgaaggccagaaggatgccgatcatggcgaggcccaggatcagggcgtcggtcatgttgcccaccacgtcgagcggattgtcgaccggcgccggggtctcgccgagagccttcacgatctcccagccctggaccaggaccgcccccggattgaggaagtccgcccgggacagggatccgccgcccgccgtcagtcccagttcgatgaagcccgcatagagggtctccgacagccgctgccagtcgttgatcagccaggcgaacagcccgaccagcagcaccttgccgaagcccgccgccagcacctcccggttgggagacagggcccactggatcccggtcagggcgaccaccagggcgatcatcaggccgaacacaccggcgacggacgcctccagagccgcgaacccggccgtgacggtgtcggagaaggtcaccatcagggcattgggcgtctccatcccgacggtcatgatctcagtcccgcgcccgagagaagggatcaaaggccggcgggggcggagcggccgactcccggctccaggcccgccgccgccccgcgttccccgccgcctggtccgccgcgccgcgggcggcctgttcggccatcaatcgggactgggccagcatgatcgtcctgagcccggccaggtcctcggcgagtacagccaggatctgattggtcgactgaacggccgccgtctgcccctgagcggactggctggccgacagggcgccgctgaggcgtccctgccgcgcctgcccaagctgttccagttcagcggcgtagcgcgccagatcggccgcgctgcgccgcgcattctcgcggcgcgcctcgccctggctgatcagctccagaacgccggccgcgctgacatcggccggataaaggctgtcgaactgccgctccaggcccgccaccgtggtggccagaccctgggcactgcgggccaaggccgccatgtcccgcaggctctggctgttctgggccagatggctgtagggcgaggccgcaaggcttttcgcctcattggccaggctttccagctggcgcgcggcggccagggcgttctccaggtggttgcggggatcatagacgatctgctgggccgagacgggcgccgcggcgagcgctgcacccagtgcgagcaccagacccggtcgcgcacaccggcgcctattcggccgtggacggacgcgcgaaggcgtcaaggacggcgtcgacattctgcactcccttggctttgaggaattcgcgcgcgaaggcgcctggacaggtctcccgcggaccggcgtgcgcgagcacggcatcgatcagggcctggtcttcgggcgagccagccccgcacagggccagggccacgccggtcagacgaagatcaaacaaccgccggccctggggctggcgccagtagtaggcgcgcttgggcggggcaaaggcgatcagttcgagctgacgccggctgaggccgaaggcgctgtagagttcggctgacgagggctcgagcgcccgcggattaggcaggaagacctgggtcggacagctctcgaccagggtagcggcgatcggcgaggccgccacatcatcgaggctctgggtggcgaacacgaccgccacccgcttcttgcgcagggtcttcagccattcccggatcttggcggcgaaggccccctcccccaggaacagccaggcctcgtccagcacgagcagggtcgggcggccgtcaaagccgcgctcgagctgatgaaacagggcggacagcaccggcgccgtcaccgagggcgtcgccatcagcgtttccagctcaaaggtgtcgaaccggccgggctccagatcgctgtccgccccgtccagaaggctgccgtgtggacccctcagggtcaggggctccagcgcggcggcgaccgcccgattctgcaccagggcgcagaacaccgtcagggtcctttggtcgcgcggggcggccgccagggcgttcatggccgcccagatctcttcccggatcgtggggacgggttcgaggccggcggagcggaccgcatcggcgatccactcggccgcccaggcccttgcgcccgcgtcgtcgatgtccgccaggggctgaagcgagaccggcccgcccggctccagcgcgcgccagcacccgccggcggccagggtcgcggcgcgggccgaccgccccttgtcgaagaagatcaccctggcgcgcggatagcggaaccactgcagggcgagaaaggccagcagtgcgctcttgcccgagccggtcgggccgatgatcatggcgtggccgacgtcgccgacgtgaagaaccaggcggaacggcgtcgaacccgtcgtgcgcgccgtggcgaggggcggaccgccgagcgccggatcctcaagcgggcccgcccatgcggccgacaccggcaggaggtcggccaggttcagggtcgagaccagagggcggcgcacatcggcatagggttcgcccggcaaggcgcccaaccaggcctccaccgcattgagatcctccacccgggcgatcagcccctgggcgttcagagcgccctcgatcgcacgcgccttggctgcagcccccgcctccgtctcgtcgagcaccgagaccgtcagggtcagatagccaaaggcgcaggcgtcggagccaagggcggccagcgccccgtcgcactcctcggtcttggagaccgaatccgtgtcaagaagcggcgtttcctccttggtgatggcttcgcgcagcaggacgcccacgcccttgcgcttggcgaaccagcgcttgcgcagcttgatgatctccagctcggccgccggcttgtcgagcgcgatccatcgggcggtccagcggtaggcgaacggcaaggcgccgagggcgtccagcaatcccggccgggtggacgacggcaggctgcgcaccgacaccaccttcagccagcggtcgccgagccggggcgccaccccgccggacagcgccgcatcggcaagccaggcgtccaggaacatcggaggatccggcggctcaaccgccaccgaccgggtcgagaccgtgtcgtgcagccaggtcagcagcgcgccgtcgtccagcggctcgatctccggcagggcgtcggcgagcaggtccaggagggttccgacctcgcgccggaactgttgcagggcctgccgccagtcgcaggtccggacctctaagccgtcgaacagccagccttccatgcggcgccggtcgtccgcgggcggcagccaggtcagggccagacggtggtcggtctcaaaagcgggatcggcgtccttgaagcgatgccgacgctcggcgtcgagcagccaggcgacgcccaggtcgaaagcgctctccggataggcggcggcggcgcggcggcgggcctccacgtgcaggcaccagccggcgcccagacgtttcagggcgttgttgacccgggcgcgcaccgccatcagctccgcctcggtcgaggattccagatcgggtcctcggaagcgcaggccggtggtgaaggagccgtccttgttgaggatgatccccggcgcgaccagggcggcccagggcaggtgatcggccagactggcgggccgtcgccggtgttcgtcgagaaaccgcatcgccgcctcacgcgtccagatggccgggaagggcgagatgccggcgcagcacgtcaaagaagcgcgggtcggaccgcgcggcccacaggccgaccgcatgcgcgacggcccaccagaggagcccgagccaccagatccgcagcgccaatccgaggaccagggcgatggtgcccatggcgatggcgtagtcgcgcggcatgccggccatcagcaccggcgccgccagggcctgggcgacaggcagatcccatcccgcgggtggatcgccggcctgcgccatcacgcgacctccagaccgccggcgaagccgaagaagtccagaaagaaggtggaggcggcaaaggcgatgcagaggccgaagatgatgctcaggccccgccgcatggaggagccgttctcgctcatggccacgccggctccgaacaccaccaccgccacgacggcggccgcctggaccaccggtcctgtgatcgactccaccacctgctgcagaggcccctcccagggcatgcccgatccgccggcgaaggccgggcccgccaacaacaaggcacaggggatcactgcgccgccaaggcggcgtgaaagatgtccacgcatcgtctgcttcctgaatgaggggacgtttcagtacgtctcaccccattgcaaacagacttatccacatgctgtcaaattgtttttacgaggaaatacagcgacttgcgtaagggtcttgcgagactttcggcaagtcgttcgtaggcggacgcaacactctgcgggcgcaggcgatttccgcctccgcgactttccacgacttggatggccccgcaggggccgcgggccgctccctctcgcgacaagcttcaggcgcgcgaaggccgcgcccctgtcgatccgcccggcgtccgcctggcgtgggtcccgcatatggggcggggtcctgcggaactcggcaagagatcgacctgccggctctacgggcgccctggtctctcttctgagccctcaccgggtcgtgggtcagcttgagtttccatatcggcgggtgggtgctcacgggctgggaaacaccatggaccaagtcgatcaggtggctgagccccggaccggaccgctgcgccttggtgatatcccttgcgttggacactggcgcctggcgcttaaggctcttgacgctgtggcgaccggaaacgctcagcgtcagttttcgattgaaactcagcccccgccgtcctacgtatactcgtacgaaacggcagtttttgaggtgagaacgccctcctcacgcaccatggccggctcgccggctcgggtaaagtaggccacaaaccgaagagatgcaggagccttgccgttctgaacggcgggctgaaaaatggggatcctgccatgaactgccgaagaggcccctgcggaaagcgggggcctcttcaattgcgcttggggatgatcaatcggccgttctggcgtcggttctcgatcttgccgttgccgatcggatagcacgaagccacgttgtagttgcccttccgatccggttcgatcagcagcgccacgagtaatccgccgcccagcgcgggaattctcgccaccagctcgattccggcgttcttgaagtcatctcccaaaaaatcgggtcgtgcgacgacaccgccgacatggggaagacacttgggaaagtcgtcgggatgacggcgagcggcgtggatctgagctgcagtcgagaagatcacatctccgggaccgaggtcatgacccagtgtccggttgatctcctcaaaaggcagaggaccaaggttgagctccagaggcgcagggtgttttggcttggtcacgacgccgcccgatcttcgtagggtccgcgcttgccgggagcctttcctgcggtgtcaacactagcaacgcggtgggacatttcccactgtcggtttgccctgcctgcggccatcgcacgggaccttgacgcgctgaggcttgcccgcggcattctgggaagacgtagaccagggcgacatcataccggtccaaacggagccggctctttctaaaacgaggggcgcgatttccagaactgacctatcaccgcgacccgccaactccggcgtccgcggagcttcgaacccgagcggtggcggacctaagagactgccggggcgcttctgcaccgaccgacctgtcatgatcggacaaggggcgctcccgaggctgacgaagctgtgagccgtctcgtcgccgccgcgccgacagccacagtccggtcaggcgtaatgtaaggctgcgcttaatcaaagctgggacgcccttgtaatcataggctggcgatcattacgcaccacagagtccgccagaggaggcctgaatggccgtgcgcgcgagcgcatgcgccgaagatgcctgcacctttgaacgccttcccgcctcgatgacctgcccagcgcctttcggactcatcccgtcaccggtgctcaggccagaggcgtgatccggtagccgccgttcccgtcatcttccaccgcaaggatcgcctccacgcgacggcccgcgcccgttctctggatatgcacaatgcgatccacggcttggccgatcatgcgccgcggcaagtggaccgagacttcgccaacaagatcttcaaggcggcgaagcacatcatgggccgagttggcgtgcagggtcgacagcccgccgggatgtccggtgttccagcttttcagcgtctcaagcgcggcggccccatcccgcatctccccgatcacgatccggtccggccgcatgcgcagggcgtcccgcaccaggtcggccacgccgatgcggaccggcaggcgccgcgtcagcaccgccaccacatcccaggcggcgcattgcagctcagcggtgtcctccacgaggaacaccctgtcgccgacaaacgccggctcggccaggaccgcattagccagggtcgtcttgccggatccggtcccgccggaaatcaggatgttgcggcgctcgctcaccgcatctctcaggatgcgggcctgagcttcgctcaacacgccgtcacgaacataatcgtccagcgaccagatcaccggaggccgcttgcggatggaaaaggccggaccggaggcgaccgggggcataagggcctggaaccgctcgccgccgggcagaaccccggagaggcggggatcgtcccgccccacggtctcgccggcgaaatcggccaccaggcgaaccgcccggtcccgtgaagcggctgtcattgtcacgcccgtgtcctcccgcccctccccggcgcgatccaggatcagccggccgtccgggttgaccagcacttcaaggacggttgggtccagaagcgccccgaggatgtcgtcgcccagcgcatggcgcagcgccgcctgtcgacgctcgtgtgacagcgcaggctcgttcatcaagcttctcccgccgtaccgcgggcgtcgttttcacggcgacggcttccggccacgatccgcgcggccgtgtcgtccagaagccgttcgatccgccggtccaccgcagcctgcacggtgggatcctcgtcgatcaccgcgtccggcagcctgaggaaaagggcgcgggcgacctcgacaagaagctcctgaacgatctgcatgtcgcgcgcggttgaacgcatatggtcccgcagagaccgttccagcgtctccagccgatcctcgggatcggcgcggggattgtgctgaagcccgcgcgcgatcgcccggccggcggcctggctgagcgccatccgaccggcccgcgcttcccggttcagtcccgtcacgaccttgggatcgctgagatacacctgcaccctgcagctcgccgccgcctttctggtcattgccgcccccgttccagctgatccagcaccgcttcctgggcggtcatctcgccaagggccctgccgtaggcctccatggccttggccgccgtcttccggtcctgcatggccgccgccacctccttgaacagcggcagcgaggcctgtgcgtcctcgccgcaaccccggcgccccgaccaggggtgcggcggcgcgcccggcgtgtccaagagcaccgcctgattcggggcgaccgcccccgcgcgctcacggaacgggcgctgcttgtcgtactgcagcttgcgggttcgcagcggccggatccctgccgcgaagacgagctgaacaggctccggcagtgaccgcacctcgcccggttccagcagcgggcggtcgatctgcgaccgcgacacgctgccgtgtccatgacccaggccggcgggactggaccggctggtccttgtctcaagcacgcttccggtcagacgcgacaccttttcctgggtgaccgggtcgagcgcggcgaaggcggtatagaccgcgcagttgtccaggatcgtattgtgggggccataggtctcaatgatgtcgttcagcgactgcgccacgaacatgaccttgaccccgaagccgctgagcagccgcagggacttctcgaagaagctgatccggcccagcagcggaaactcgtccatcagcatcagcagcctgcgctgtttttcacggccgtcggccgtgtgcttttcgtggctcgtgaaggcctgggcggcggcatggaagagcagccggaccagcggcttcagggcggccgcgtcggcgggcgccacctgcacatagagggagacgggggtgggcgaagccatcagatcacccagggcgaagtccgaacgggacaggacccgttcgacgtcgtcgcctgcgagccatttgagataggcccgcgccgtgccctggaccgaggtgcggaaccggtcatgcatggccgcatagccccgggccgcggtggcgataaagggatgcagctccggcgccccgcccggtccggcgcgatgcagggtccgcaccatgatttcggcggtctggtcgaggtccgccaggagttcgcgcaccttgagcagggtcttgtcggcgtccggcgccgtgtagagaacgtggaggatgacggcttccaggatttcggaggcggccttgtcccagatggcctcgtcgtcccgcccgccgcccgggtccgagaggatcgccaccagccgctgcacatgggccagctcgccaggacccggacggatttcggcaagcggattccagcaggcggaagcggggtcgcggggatcaagataaagagcgtggctgaagccggcccgccatccggccgtcagccgccacagctcccgcttcggatcgtgcacaagcacgctttcgctccacgacagcagggtcggcacgacgtggccacggcccttgccggagcgggtgccgcccgtgaccagggtcggcctcaggtcgagggtcgccagtatgcgcctgttgtggcgtcccaggatgcagccgccccgggccatcagcccggcggcgcggacctcgcgccatcccgcccacccccgtgttcgccgcagcccatttccgccaaggcctgcgcctgcggccagcccgccgacagcgcccaggacgatgagcagcgccgcctgcgacagggccggtctcgcctcgccgcggtgccgcctggcccagacgaggatcgaccagggcggataaagggcggcgccggtcgaggagcgccaggcgacgccgagaaccggggcatggtcataacgccaggcgaacgcctgggtggcggcctggcatccgaccacgcatcctagaacaaggcccgtcagtcggtggcgcatcccctcagtttcccgcctcggagtccgccgcgtcggcttcggcgttgagcaccagcaccggcgcgagagccatcctgcgctcgtgataggcaagcaccagcgccggcgcctgctccggggtcgcctccatcacggcggcggcctccgcttcaaggtcgtcgaacagtcgcctctccgccgcgctgaaacgcgccagatggccctggacctggtcaaaggcctggagaagggcgacgtcgccaaggctgcggagtcgccagcgccagaagggcacaagtcgatccgccgcggattccggcagcaggcccggcggcggcggtccctcaatcctcatggtcgcttgcagcaggcagaggcggcggaacccgtagcgctgcgcaagcacgccggcttcaaggcgcggcgcaaaaaacccgccggcgccgccccgttccaccagcccttctcccccaagccagcagagcgcctcccgaaccggggtggtggagagacgcagtgcgcgcgcttcgtcgctgatgacgacctgacgacccggcgcgtaccgcccgtcggcgcaggcccggcggatcgcctccagcgcctggccgaacggatcgcgagtgcgggtcacggacatacccccggttgatcggtatcgcggtgaagacggcaaggtttgcgctcgcgcacaagttgcgaactgccataacgtcacagaacggcggcctggccgtcacaaatcgtcgggacccggcgacgctttgggtggaaactctggcgaaagcctgaacagcgcacacctgttcacccccagcgcctagcttgtctcggctcgcattcgtggaaaggcctggtcgtgagacagctcacctttgatcatctgcgcgacgccacgaccctcagccgcgccctgaaggccgtccgcaggttgcggaacatgacaggggcggaggtcgcgtccggcatgaacatcagtgtccggacctatgagcggttcgagtccgggcagacgcgaatgaacctggagtatctccatcgcttcgccgaggtgacggacagcgatttctacgcccttctgtgcgccgccacctttggcaccgccgacttcgccgttcattgcgccgacaaccagctcgccgccgttctcgcatccggcctgcgcaacctgatcgaggcctgcgggccggatctcgcggcgctcagcacccgcgacatcatcgagaccatgcagccgatgttcgaggcgctgtcgcgcagggccgaggacgcccggctgctgcggcagggcgttctgcgccgcggctccgccggtcccgcttcggagtagcaacgccggatataggtcggataccgcttcgtatcgggtgtctccgggcgcttccttccgaagccgcactctgcggcgcttgaaaggagacgatcatgaccaccccgatcctgaaccgcatcagcctgggtcgcgcccgcgacctgacccgcgactcgcttggcggcgcctttacggaaatccaggcgaacgacagccgcgcgcccatcggctgagccccgagacggacggcggcgtgtccgtcgtccgtctccatgccgccctgggagacccacgtcgcgccggcccgtcgggccggcgctttcgcgtgggcgcctgaatcgagcgtgccgaaatatccgccggatatcgtttcctatcctcgagcggggcgcgctcactgggccggccacatccgtggcgatcaacccggagacagaccatgacccgcccgcaactgaaccgcctcgaccttggccgcgctcgcacggagacccgcgacggcactctaggtcagttcgtcgaaatgctcgcctatcccagccgcacgcccgtcggctgaaatccccggcggacgggggccgcgcctccgtccgcccctccgcgaagggaccgaacatgaccgcaagcctctggtgcgccgagagcgtgtcgatgacgcgggtttacgaggacgtcgtcgtccttgatgtcgcccaggaccgctacgaatgtctggtcgacgccgcgagctggctcgatccgcagcctgacggcggcctccgcgtccaggacgagctcctggccgaccagatgatcgaagccgggctcgcatcgctagagccgccgtccgcccgcgaaacccttccgccgcccgaccgggccctggcgcccggcgcgccggcgaaccgcctcgcgatcatccgcgccggtcttgtgctcgccgcggcgacggcgaccttccacaaccgtcgtttcgccgacctgacaaagccgcgtcgagagtcgccgccggccgcagcagtcgccgacgaagacacggttcaggccgtggtcgccgccgccagggccgcggcgccctttatcccctttgaaggcgagtgcctgcaccgcgcctatgtcctgcgccgcctccttgagcaccagggcataggcgcgaactgggtcttcggcgtcagaacctggccgttcgccgcccattgctggctgcagatcggcagcctggttgtcggcgacacgctcgaccgggtgcgtcactacagccccatccggatcgtctgaaatgggcgcctatctcgtggtcatccggacgtccgaggcgccgtccgccatcgcacgctccaagacgctgcgggccagggctgtcgccgccggcatggtcatagacgacctccggcccaacgcctggatcggccgcctgggcccctccctccctcctttgcgaccgatcggcggctggctcctgatcggggacgtcatggaccggcgccgacccgtcctgccgtcctccgcggcggacgacccctgggactacgagcgccgtctgctctgccgggtctggggccggttcgtgggtttgcggttcggcgccgacggtcatctggacgctatcctgcgggatccttcaggcgcgcttgactgcgtcgcctggacccaggacgagctgatcacggtctcctcctcggcccccgactggctgatcgcggagacgcagccccgatggacgatcaatgtcgctcgggtcgccgccgccctgcgcagtccccagctgacccccggcgcactcctccttgacgggccgacggccgtcgagccaggcagtcttcagcccctgccgctggaggcgggccccgtgccgctctgggaggcgacggcgttcgcgcacaagagcctgacctcttgctccgatgtggaaacgtcggcgatgcgcctgaaggatgcgatcgaggaagcggtgtgggggctggcgcgtctgccgggcgccgtggcggccgaggtgtcgggcggcctggattccagcctggtggccgcttcactggtcgccgctcccgacctgaagatcgaaccctggctcaacgcctatggcgtcacgcccgagtcggacgagcgccgctgggtggacgcgctggccgggcaactcggcatcacgccggtccgcgcggcccacgtcaccgcgccgctcacggcggaggggttcgaggcgaccaatcgggggttccgtcccgggctggccgccctcgacgtcgcccacgacctggagtggagccgccggctcgaggcggcgggggccggggccctgatgacgggcaagggcggagactccgtgctgatgcagggcgtcggcggcgatgtcttcaccgatctctggctgcagcgcggcgtgtccgtcctcctgtcgcacgaggcgcgcgcgctcgccctcgccagcgaaaaatccctctggtcgctgaggcgggaggcgcgccgcttcaaagcccatggcgccccgcctcccgagcgggacgacggcctgctgcgagcccccgaggaaacgccggccatgatcagctggcggcgccatgccgccgcctttggccccgccaaggccgggcaactcgccggcgtgcgcgacaacatctcccggcatggtccctccatgctgacccgctcggtggatctgcgccatccgctctgcgcccagcccgtcgtagagacctgcctggccaccccgtcctggatcctcacgctcggcggacgcgatcgcggcctggcgcgccacgccttccgcgatcgccttccggcggcgatccttgaacggcggtccaagggcgacatgagccggctctacgggatggtcatcctcgaaaacctggacttcctgcgcggctggctgatccacggacgcctggccgatcgcggcgtcatcgacccggcggcggccgaccgtctcctcacgcgggagaccctcatctggcggggtcgctatgcggcgatcctgacggcggcggcctttgagggctgggttcgatcctgggagcgtcgcctgccgccgtcctgagctcggaggccgcgggcagtgtctcctcaagccatcggaacacctggccgtactggtcacggatgttggccgggctccagcgggcgtggtgttcaccccaataggtcacgagccgggcccggccgccgagccgcgccagggcgctgaagacccgctcggagttgccgagggcgacgtagtccatatccgccgtcagcagcaggatgggggcctcgatctgatcggccttgagccaggggctttccttcatcagggcctccggattcccccagggcgtggctccaacctcgccctggcccgtctcgacccagccctgctggagccgcaggctcatcccgttctcgggctggatgcgggtcggggcggtcagttcgccccagtgcgcgaacatgtcggtggcggccgaggacaggatataggactggtaccggtccgagcgggtcgcggtcaccagtccgatgtagccgcccatgctatgaccgaagatggcggtccggtctcggggaagctccggatgcgccgcaaaggcggcgtcgacggcccggtctatgctgtcgacaaagaactccgggcttcgggttcccgggcgatcgtaagccatggcggggtggagcaccgcatagccggcgcccgccagcacagccgcccggatgttgtaggtcagcaccagcggcccgaaccattcgccgccgtcgacgtgtccgggatagacatggaccacgaggccccgcaccggtcccttgggaagaaacagggtgctgcgtcccggctctcccagggcgtcggggtgctccagccattccggccggatcagttcgacgtccgctcggtccgcattgacgacatcaagcgccagatcctgctcgccccgtctcagccgcagggtctccaccagctccttccggtccagcacaagcagggcctgggccgatgaggccatgatctgtgttccgcccggctcacctcgcccgcccaggggctgcacgccgtcgtcgccgacaagaaccgcctggccgtcctcggccacggctgcgacgctgcgggcccgcggcgcatccaggacgatgcgcgtggggcgttcggagtccgccgtgaagaccggctgcagtcgcagaccctccggagtcagaaggtgaacgccttccgcatcgaggcgccagtatcccccgtccgcgaacagcctcagggttccgtcgcctggcgtggccgcgatcctcgcgggcggggcggccagcgcagcggtcagggaacgctgccccactccgtccaggcgatgccaatccgggcgcgaggctccgttcgcgcggccatggatcacgggaaccccgttcagccagtcggcgcgcaccccccggaggatgttgtggtcgccgcccagatcgagctcggacggccaacgccggatcccgccgtccagatccatcgactgaagcgacccttcgctccagcgctggtcatcccgccgcccccagaacagcacctcccgggaatcgggcgaccagcgcagcatctgcgccgcgacgtccacccgcgcctcgggtcccgtccgtcgaccatcctccagccggatcagggtcagcctctgacgaaggggctcgtcgaactggaccacaggatcgccgagaggcaggggttcggccccgcccagcaccgccaccgtccggccgtccggagacaccacctgatcggtcaccgcgccttccgccaaggtccggacgatccggccggacgcgacatcgatctccaccagacgctggggcggcggcggcgtctccggagtctggacgcccccggccgtgtccaccacggtgcgcgtgggcgcgcgaccttcggacttgcgccgccaggcttcgctgatgcgctcctgcgcggtgttgtggaacgccagcaggggcggcaggctgccgtcgggccggatgaccgcgatcagccggtccggcgacagccaggagacgggcgcgcccttgggcagatattcgggggtgagccctgtccatcggacggagcggctcgccggggtggccacgccaagctcataggcgccgtcccgcatcctgaacaccgccaggcttgcgccgtcgggcgaccagtctcccctcagcaggcccagcggctcatccggcaggagccgttcagggcggggagcctcggccgccagatcgaccctccagaggtcggtgatggcccagatcgagcgttgcgcgtagtcgaagcgcgggatggtgtcataggcgccgcgcttctcatacaccgcccagcgtccatcggggctgatggaggcgcggccgaagccttccagggcgaccacgtcgtccaccgtcagatcacgggtttgcgccagcgccgccgtcgcaaggcaggcgcaggccgccagggcgcccgaaaggcgcttcagaaatcgaaacatcatgacggcctaccagcgctggatgagttgcagcgcgacgatgcggccaaacggattggcctggccgggatcaaacccatagcccgaggcggcgtcgtggaacggcggatcctcatccagaaggttctggacgctcagggccagccgaagcccctgcgccggtcctgacgtcggcgcccagctcaacgcgccctccagcgtttgccaggaagagatcgccttgccgaggcggtcccgccctccggccgcatggttgaggtgcagggcggccccaaaggcgccccgggtccaggcgccgccggcgcgggctcgaacccgtccgggatagccggtcaggccgaccacgtcacggacggccgatgtcggggtgggctggctctcatagtccaggatccaggaccccgtgccctccagcgtaagatccccgcctgcgaagcggagggggtagcgcgcctccaggtcgaggccgcgcaccctcaccgcgcccgtattgacccaccgcatgtccacgatcgcgccataggtcgccgccggataggtcgcgggataacccggcaggtcggcgtaggattcgacaagggccagatcgtcggggcgggtcgagggggagaccagccggacaaaggccgacagcgccggatcgatcagggcgccggtggggttctcgctgaccggctgggcgatccggtcggtgaagcgcgtgtcgaaatagctgacatccagattgaggcgaccgcccggacgccagttgaagcccgccgtgaaggtctccgccgtctcgggctcgagatccgggttgccgccatagaccagcagggagagagtctggctggcgtcaggccgggcgagaaacaggcccgaggctccggccgcatcatagatctgcggcagggacggcgcccggaaggacgtgccccaggtggttctcaacaggaggtcgtcggagggggcccaggccagaccgaccctgggattggccgtgtctccgaagtcgtcgtagcgctccagccgccccgcgagggacaggtccagtcgccggagcccgggccgcgcgttggcttccccgaccaggggcagccgggcctcggcgaagacggcggcgatctcccgccggcgctccggcgtatcggacacaagcggcgtcaccgtcgagacaaaggtgcgggtgcccgtctcgaaactctccatccgccactgcgctccgaccgccagccgcatctcgccgcccggcagcgtccagagcggcccctccgcgagcaggttgagggagccggcgcggctgtgatcgtgcgcctcggaaaagccgctgccgatgaagtccagcaccgccgcgctgttggctcctcctccgccgaacaggttgagatagccgtcccgcgccgcggagaacggcgtgtcgggattgtccggcagggttcccaacgcttcgttggcgaagcggacattgacccggttgcggctgctgagggcgccgcgctcctcggccagggcggcataggcgtccaggctccaatcggccggcgcctggtagcgggccgcgatcgtcccgccgaggctttccgagcggccggattggcgcccccctcccaggtcattgaggaaggagtagccgatcgtgtgggacgccgcgcccacgggcgacacgaaatagggatttgcggcggtgacggtgaataggcccgcgctggcgccgccggtcagttcgtagtcgcggcggctgtatcggaggtccgccgacaggtccagcgcggcgccgatcgcctgcgacagccgcccgtaggcgctgtagcgctcgatggccggggtcaggtccgcccccgagttcagcgcccgccgattggcggccgcggccgcgaagtctgcgggaccggcggcgacgcccgaggcgccgggacggatggcgaagcgggagacataggcgcccgcggccggatcgaaggcgaggatgtttccgggcgcatcgtagaggctgcggtgatcggtcccgccataaggccgcaggtcgccgtctgcggtataggcgcgatccagcgtgctgagcggccgggtgttctggtattccaccgacagataggctccgccgcccgaccatgtgcggccaaggagatgggaggctgtcaaatcctccccgccgccctgggccgcagagacccgaacccggctctcctggccgtcgaacgcccggcgcaggatcacattgaccacgcccgccaccgcatcggcgccgtacagggccgaggcgccgtccagcagaacatcgacccgctccacggccccggacggcagggccgagacatcggcgaactccgcgcggaagccggaaccggcgagacggcggccattgatcagcaccagggtggaggtgggccccaggccccgcaggttcagtcctgtggcgtagacggagttggacccggagcggtcggaccccgccccctgcaccaacggcgttcccgccccggcgtaattctgcggcaggccgaccaggacttcggcgaccgtggcctgcccccgggcgtccagttcggcgcggccgagggagagcaccggcgacaccggcgggccggggtcccgcagcagactgcccgtgaccacgatctcatccagctcgaccgcagagcccccggccacggcctcctccgcgccgcgccgcagatagatcacgcccggccgtgtttccgtccagacaaggccggtgcccgccagcagccggttcagcgcgtccgacggcgtgaagcgccccttcagccccggagtgtcgcggccccggacaagatcgcccgcaaagaagatctggtgctcggactgggcggcgtaccggttgagcgcgtcgcccaaagggcccgccggtatgtcataggcgcgcgcgctctgcgcgcaggcggcggtggaggcgacaatggcgaaggcgcacgccgccccgccggacaacagactcaaacgactcatctcttcttttctcccctcgacgcgcgacgcgtctcgagaaggagacaaccgagccccggccctaccccggagccgagccggttttattttccgcccgcagatgaagccgtccgtccggcgccctggacggcgtcagtccgaacacggcggacaccacctccacaaaggcgtcgcggtcgccggtcctgaacacgccattgaccggcaccgccgccaggtgcggcgcgtcgagcaccacgcctcgctcgagatatcggttcacctcgctcaccgcttcgcccaggggacgatcgcgaaacacgatgcgtccgtcggtccagcttgtctcgctgacagcgtccaccgcacggacccgcgcgccttgggccgagaccctcgcctcctgccccgccgccaggcgttgtcccgcccggccgccgtccggctgaacctcgaccacgccggaaaccagcaccaccttgaccggacccccggcttcgcgccggacgtcaaacacggttccgatcgccgtcaccgacgcccctcccgcctccaccacaaagggacggctgcgatcgggcgcgaccgtgaacagggcctggccgcgttccagcgacacccgccgccgcccctggtcgaagcggacccggatctccgatccggtatccagccgcaccgtcgatccgtcgtccagctgcaccagttgctgttcgccgacgcgggtcccgtagacgttcgacgcccgccccgtccagacggcgatcccgatcgccgcggccagcgaagccagggctgcgccgccgacgatccaggtgcgcgggcgaggcgccctgcgatcgcccgcgcgtgacagcgccccggcgagcgccgcgttcaggccggccgaggaggcgcggtcgccggccttgcgccacactgtttccacgcggcgataggcgtcgtcgttttccggttcacgccgccaggcgaagaagtcctcgaccatctgggtggtgacccgcggttcgcccagccgggcatgccaggccgccgcttcccgctcggctcggcttgcacgcttggcccggtccgtcatgtcgcgcctcatgtctagcgccggagctgcgccgcgcagtgcgccagtgccttggtcatccgccactcgaccgtcttggggctgacgcccagccgttccgcgatctgcgcatgggtcaagccgccgaacctggagagcacaaagacatcgcgcacgggttctggcaaccctaggatgatctcctcgacgagcaggccgaggtcctggccgcccgagacggcggacccgctcatggcctcgaagcccgagacctcggcgccgtcgcgcttgcgccgcctgccgtgattgtagcccagtcgcgtggcgatggtcagaagaagcgctcgcggatgccgcacctccccgtccgccacataggttcggatcaggcgtccccacgcctcctgcgccaggtcctcggcctcatcgccgaaacggccgcgcagccgcgtgaccagccagtcggcatgccggcgatacaggccgccgatgccgcccgcttccgctcccgcttctcccgtcctgtccgacacggacctgcctccctttgcaaagaggcaggcccggccgatgccgggtgttgagaacgtgattgaaacacgcgcgagcgcctttagccggaggcgaaccccaggcctggacatgcgcgctcgccacgccgcgcaccggaacagtgtatcgggtcagaacagttcaatcgaggttctcacgcctcggcgtccaaacgaacgcacaaggagtctcatccaaaccggcgcgcctgacaagaggccggttgcggctcaatccacctgacgtagagtgcggcgtccgaccggattgccgtcgccgtgtccaagcgcccagcgccaagggcgacggccatgccacagtcatgattctcacgcttccggtcggacgccatactgctgagtggaggaggctcgcaggagacagggttccgagctgcaggccgcggctgatccccccagctctctggcctcgaatgccgtgagggagttcgcagaggcgccgccccccagggccgcgttcttcaaagccgagccctcgcaaggcgacaccagcctggcgactcgactcaacgtccgagtacgcctggtcaacgaagaagccggctcccgctaccgagagcagcgtcgcctgaggacagcgggtgtgaggacgcgacgaccggctgaaggaagggagccctgcatcaactcccagccgcgctcaggcatggcggagaccccttgcccactgcccatgcacccggtcatcgaggaatgatggttccgcttcggtcgacacccgagccgccacctctgttagcggcgggtctttcaacccgccgccgaaggcaccgacggcgggccgcgcgcccgaaggaacgaagacctcggtcatggcaggaaagtcctcaaggataagaacgcagggtcctcaggatcggccaagcccgtcaggtggtgagatatccggaatgatcggaggcggcggcaggcgcacccggctgtggcgagcggtcggcgacgaaggcggggtgctggatctgggtcatgctgcagcctcgagacaccgaagccgctgaagcggctgcaacgctggccggggatatcgcctgtcgagccagagagcatcgtcaccgacaggctcggctcctacgcctgcatgctggaaaggtcggaactcaggcttctgcttcgggatgcaggctgatgccgcgggagatgatcgagcggggctcgttgcggctcaggagatcctgacggcgcagttgcagcgccacccttgattttaccgggttgatccgagagatcggggattaaccacgccgagcgcctggaggatgacgtgtccgaagcagttcgggttttgacagaacgcgaacggcagtgtctgcgccttgttcatgcgcatttcagctccaagcagatcgctcgcgagctcggcatcaagcccggcaccgttgatcgccattgcgagaacgccgctcgcaagttgaaggtcgatacgcggatcgccgcagcgctcgcgctcgccgccgaggaaacgatacagaaccattcccaatgggacccgcccggaatggcggcgcgttggccaagggtgctcgatgttgcggcggagggggcgcaccatgatccagattaaagcccccacccccgccataagctggcgagaactggagaccatcctgcaagggatggcgaccaccgaaaccaagaggcggatgatccggcaccttatggagggcacgcgcaagcaggcggtgttcctctcggcgggtggcgtgatgacggagatcatctacatcgctgcggcgatgctggacgtgaacttcagtccggaaatcgcgaacatgggcggctcggaagcatccttctcgtcttcggcgtcgccgccgcagtcgtctggatcgtaacagccctcgccggcgcgcagcagttcgccttccttctgcagaatctgcggtacggaggctgacccactcgccggcccatcggatacaatgcccatgaaaagagccgaacaggccgcgatgatcgcggcgcgccttcaacgcgccctcaaccgcgcagaagcgggacaggatcagtccattcagcgtttgggtcagttggcccagaccctgacaaggagccgcaaggaagcgggcttggccgccaccgtcggtcagcaggccttcgacgccctggcgcgcgcgatgagcgcccaggtcgcggcgcagaaggcgatggtcgaactccatgaagccctggccgaagtgaaggacagcactcggttccgcagtatccgactggggggtctcgacaagcaggaggagccggtgacccggccaaccggacgcttgagccttgttgagcgcaccggctgaatccagcatgggtgatatggaggctccatgtcacccatctacctcttcacgcttgtgctccttgccgccacggggctgttgaccttctggcgcggcggcgcctgggagcgaaccatggccgtggcgctcgccatagcgtggatcatatccgatctcgcccccttcgactatcgaacgccaccctgggccgccatcggggccgacgccgccgtgttcatgtgggtgctttatgggctgctcagatccggtcgtcgatggatgtctgcggcggcggccttccagttcctggttctggccactcacttcgtcttcgcgacccgcgccgatttggagcagtgggcttatgtttccgcctactacgtctggaccattggcgttatagcctcgctttgtgctggcgctcttcaacgacccagggcgtcttcggaacgggaaaggccgcagaggcgagcatgatcacagagccttctcagtcgcagcacgacccgatcgatcagcaggtcggcgcgcagctgaaagccctcagactagcccgccgcatgacgcaggcggagctcgctggagccctgggcgtgactttccagcaggtgcagaaatacgaacggggcgtcaaccgactcgcggcctcgaccctcgcccgggcggcggcggcgctgggctgtacggtggccgatttctacccgaaggagaaggaaaactcttctccttcggagtcggaagccctcgctgagctcggcgggctctttgtccgcatgcaggcacgacagaaggaagctctactggttatggcgcgagccttgaccgaggtgcgacgctgaaggcggcgggctcgtcggcggcggcagtccggcccgcgcagggatgacgaaccggccagcgctgacgaagtgctgcaggcggggcctggttgcttctacgacgccccgccagtcttgaggtgcggcggccaggggccagaggggcctcccacggggtaggctcgcggctcgacgagaccgacctgcgcaatcgtgtggcggggccgcctctccgggtcagttgacctgagcgtccagcatacgggtcagccgctcggcttcagcggggctgaggaggcggtcgcagaaggcgtcatccaccatgagataggacggcagctcggcgccattggcctggccgccgggatgcatgtcgaacagggcggccgagaggatcgccaagtcgagcgatatagcgcgggtgacgacaacgccgaggaaacgctcagtcggcggtgcggccggctccgagaagtggatccagaaccgtggcggctgcagcgaccggagcgtgcggtcggtactgaggatggtcgcgatctgcaccgccagatcggaacagagcggctggcccttcagcggcgccatcagttcggtgacgcggcggcgcatcggctcttcgacctgagcggagacatccaccccgcccctgtcgaccaggcgctggatgatgccttcgatcgattgcggcacggcctcacccctgctgctggacaatccgacagtagacggcgcgccttacccctttattgctcagcttggaaggcagagtgcggccgcctccacagcgcgattacgccgcaaggcctggacatcggcacggttctgaagccgcgccgccaccttacggtcgacctcgccgctgagcgtcgccccccccccgcgctttgggattggtcggttgttgatcggcggcgatgggcaggacagggttgtgacgtgatggtgtggacgacctccgcctgacgggctgttctgggtgtgtcgtcatcagggacgtcacgtctaggagcggtatcatgcagaccatcgctgtcgtcgggctcgatctggcgaagactgttttccaggttcacggtgtagccacagacggcacggtcgtcgtgagacggcaactgcggcgcggccaggtgctggccttcttccagtcgattggcccgtgcctgatcgggatcgaggcgtgcgcctcagcccaccactgggcgcgtgaactgatggcgatcggccacgatgttcggctcatgccgccggcgtacgtgaaggcctatgtgaagcgcggcaagaccgacgccgccgacgctgaagcgattgccgaggctgtcacccggccgaccatgcggttcgtggctgtgaagtcgaaggcccagcaggcggtgttgatgctgcacaagacccgggatctcctggttcgtcagcgaacgatgctgatcaacgcactgcggggccacctcggggagttcggcatcgtcgcgcctcaaggtccagctggggtgcgggcagcgctgaagagtctgcgtgaagagggtcaggccctgccggatctggcgcatgccgcgcttggcgggctggcagaacagctcgaacaccttggcgcagagatcagccgtatggagcgtcggattctcgattggcatcggcaggatgagacgagccggcgactggcgaccatcccaggcatcgggccgatcactgccagcgccatggcggccagcgcgccagatccgagtctcttccgttccggtcggcagtttgcagcctggctgggactcacgccgcgggccaatagcagtggcggcaaggaacgccagggcggcatcagcaagatgggtgacagctaccttcgacgtctcctggtcgtcggggccacggcggtcctgcgaatggcccggcagcgaggacgcgagggctgggtcggcaatctcctcgaacgcaagaagccgaaggtcgccgccgtggccttggccaataagacggctcgcatcgcctggaccctgatggcgcgacaggaggactacaagcccacagcggcatagagatcgggccggtcttcacccaggaccggcgccgtagacgaaggagtggtgagacgtgatgacgaaccggccgcagccggggatcggtgaaacccagggggtcagagcgcctcgagcgcgttgacgtgattagggagccggtccgcggacttcatcagggccagcagcgcaaacagctgcatcaacaggccgaacacatgactgcactcgaccgagcgccaacgtcgtttccactcttgcgtcttggaggtcgtccacacatgaccccctgaaactcctccaggagtagctagagttcgccctcgaaaggacggacagaatgaagcgatcacggttcacggaagagcatcgggatccttcgcgagcaggaggccggtgttccggtggcggacctgtgcaggaggcacggtctgagttcgccgaccttctacaagtggaaggccaagtatggcggcatggacgtgtcggaggcccggcggctgaaggcgctggaagacgagaacgccaagctgaagcggatgctggcggactcgatgctggacaacgtcgcgctgaaggataaccgacgggcggcgcttccgcatcctgacagtgatcgacaactgcacgcgggaatgcctcggcctcttcgccgacacctcgctgtcaggccggcgggtcgcgcgcgagctgacgccatcatccaccgacgaggccggcctgacaccatcgtcagcgacaacggcacggaatacacgtccaacgccatcctggcctgggctgacgacgccgacgggggctggcatcacatcgcgtcgggcaagcctcagcagaacggcttggctgctacgcgccgcccttcgggtcaacgagagcttcaatggtcggctgagcgacgaactgctggacgagacgctgttccgttcgctgccgcacgcccgagtcgtgctcgaagcttggcggcgcgactacaacgaaacccggccccactcgaagctgggatggctgacgccgaaggcctacgcacaggcgctcaccggacagagcggccggtctgctgcgctggttgaaggctgcgctgaccggcctattgccaatcccaccaaccccagttcagatcagcaaagtactctcgttatggctgaatgagaaacgggggtcacgtcatgagcgaacagcgattcgtttgcaccgaagaggaggttacgggagccgctagctgcggctggcaaatagccgatggtgcgcatggtttcggcgttaaccccctgatcctgcgttgttcaacaagaatcgagcatgccaggtagaggttagttgagtctcaaactgcggctcagacgaacatgtatgttccgggcgatcgtcaacatgatcagattgctcaaggcagctttttcggagccgtggagccgctggttaaccacgcaccggaaagcgctaggctgcttgaggagatcttctgtcgtccatactcccgggcgtcagcagcggccggctcatcgccgaccgctgccgcagcttgaattaggctgtcagcctactggcctacgctgcccagacttcgttcaacactttcgcagccagcgccgccttgtcttgaggaaggaagcgcccgtaatgcgcggccaccgtcgctggcgtgtcctggatggcgtagctggcttgttcgtatgaacccgtctgcttcagcacatgagtcgccaacacgtccctaacgctgtggggaccatgggacatcaagcccgctaccgcgccccggccggtccaaggattgtagatgccgtagcgctggatgatcagccgccaagcctcgtagaagccggactgggtgaacgacgcgtcgcgcgtggtcgtctttgccgtcttgacgaagaacgtgccgggatcggcggcgcccgccagcaaggctgcgcgatcccgcgccaggtagcgctcgatccgttcatagagccccccaaggtcgggtagaacaagacggtaaggccgcctggagaagtaggccgagttcgcgttcttgaaggctgcacacgggatgaacacctcccagcctgcatctcgaacggaccaccgcagctcgccgcgcttgagcgcctccagttcccgctcggtgcgcggtgcttcgtcccgcgcacacaccagcagctggcgcagatttttctggcgaacgccgaggtgcagaccgagccggatcatgagaaacgcccgaacggcttctgcggctgcccgagggtaacgccgctcatccggcatcctggagacgacctcttcggcgatcttgcggtattcgccgactgggctgtcagcctccaggatcggaaggatcggctcgaatgggtcgcgatgcaccctcgccaccctttggatttcgcgcgttctcgccaggccatgccggtgtgcgatctcgcatgcagcgctccagtccaggcgcgccgcctgagcctcgttttccgaaaccacgccttggacggggacgaggcgatcagcgagctgcgggttctgccgcagccaacccgtgcgctccttggtaaaggccgctgcgagcagcagcatttccgcctcccaacccgtgtagaagccgcgacggcgttcccgccattgaacataccagtcccagacggccggaaagacgagcaggccaatcgtgaggtgctccatgggcacaccgagccctttcacctcactgtccggcggcgccgccagcgcgcccatcatcagcgctaggtgctcaccgcgttgcgcggctgtcgcctcgccccagacgcctgatcgctcgaagccaaggtctgtcagcgttgcggacttgaagcggatcagcgccgccatctcttcacgaaggcgaggcgcggcctgcagccaggcaggaccgttcccgtcgaaacggaggccgaagcggtgacgggagacctccgcatggtaccgccggtaggctgtgccgcccgccaggatgtgcgtgcgaacccactgcaagattttccgcctgctgatccaaactccgagaccggaagtcgtccggcaagtgccaggcgagccttcgcgtttctgctcggggaatcgaggccggcatctgacgcgcgatcgcacgccgacgcctcatgcgggccatgaagtagccaggcgcaaggcggtaccgaacttctatagccgaaagcacagcaagggcctgcggcgtctgcggagttttggacccacgccgccaagcgacgatcgtctggtagttgatggccgcaccagccgccgtcacggccttatgcaaacggtatacgctgtctccatgccgggcgatctgagcgtcgagcgcggcatggaaatcgcccggatcgttgatcaggctccagagtggttgtggatgtagaaccaccagatcaggccgacggcctcggcgagcggttggcgagttggaagagggattgaacaaggacgcctcgtggatgcatcgcccctgaggcgacgatacctagacagttcatccagcctgcaaccctggtcccattcccctggaagctgtggaagtttgcgttccgccccaggcgcgtgctccggacggtacaaagcctgcagcgaacgagcctgacggcatgcggtccttcaactccgacgccttggagcgagcatgaacgagccagtcaggccggcggggtatcccctgcaagggagaggctcatgccgccggtccccagaaacgcctttgtggttccgaccagctcatccgccgaacggcgccctcgccctctcagtgcgcactcccagactgtaagaacccgccatccggcagccagaagcgcagcctcgctcgcttcatcgcgcaccctgtttcttcgtattttgtcttcccagaatcccgaacgcgtgccgggcatgactcccagcgcgcagtcgtggccgtgccagaagcaaccgtgaacgaatacggcgacccgtggaccggaaaaaaccaagtcgggggttcctgcgaggcttcggtcgtgcaggcggtaacgcaggccagccgcatgtagcgcgcgacggagctggagctccggctttgtatcgcgggagcggattctcgacatgttgtagctacgctgcgcgacagtgtgacggtccggcgcagtggcccggcgggagggcaatggtcatctcctctcgttactgccgtctcgcgggtgcgaaaaccgacatagctcagcgctccaagctggaacgatcatacaggtcttcgggtgacggaaagtgtgcagttgtgttgactgacgggggccgtcttgggattcttcttttgttcgggagcgattcgatgagcgacgtggtgcgcgtccaggttttgatgagacctgaccaggctgagatattcgatcggttctgcgccgatcgcggtcataagaagtccacgttgatcgcccggctgatccgggagcaccttcagcgcgagggctatgcggctgagactaggatcgcaggagccgggcgttgacggccgacgcgattacgcgcgcgaagatcgagcgtcttcgtcgaggcggcgcaccgcgcgtcctcgaccttttcgctggctgcgggggactgtccctggggttcaaggcagcgggatttgagattgcagccgcggtggagttcgataaggacgccgcagcgtcgcacggtcgcaacttccaccctggcgatccgcggcacgccatcgcccgcgacatcacccgcctgtcccccgaggcgctgtgcgaggacctcgagctgggtgatcccggttcagccttcgacatcattgtcggaggcccgccctgtcaggccttcgctcgcgtcggacggtccaagctgcgtgaagtggccgagcacccggaagcctttcggctggatccgcgcgcgcgcctgtatctgaagtatctcgaatacgtcgagaccttccgccctctagggctcctgatggagaacgttccggacgcgctcaaccacggcggccagaacatcgccgaggagacccgcgaagtcctcgaagagatgggttacgtcgcccgctacaccttgctgaacgccgccttctacggggtgccgcagatgcgcgagcgaatgatcctggtcgcctggcgtcttgagctgaccgatcaggtcaccttccccgatccgacccatttcctgacgcttccggcgggctatgccgggagccgtcaggtcgcgctcaaactgctgaagggcgcaccggcggacaaggcgccgggctatgttccgccgccagaggcttcgaccgatctgccgcccgccgtcacggccaaggacgcgctgtcggacctccccacgatcaccgaacatctggaaggacgtctgtcgaagggcgcgcgccgcttcgacacgctcatcccgtatggaaaagaaatcgcgagaggctatggcgcctttatgcgtcaatggcctgggttcgagaacgacgaaggcgtgcgggaccatgtgatccgctatctgccgcgcgactggaagctgttcgcgcgcctgtcgccaggggaccagtatccgcaggcgcacgctatggcattgcggatgttcgacgaagcgctcgacaccgaggccgtccgaaccggaaagcgtccgtgtcgtgactccctggcctggacggctctcaaagcctccatagtgccgccctacgatccggggaaattccccaacaagtggcgcaagatggagccggatcagccagcgcggacgctgatggctcacctggggaaggacagctacagccacatccactacgacagcgcccaggcccggacgatttcggttcgggaagcggcgcggctgcagtcgttcccggatggcttcgtgttcagcggcacgatgaaccccgccttcaaacaggtcggcaatgcggtcccgccgcttctgtcccgcgccatcgccgccgagatgatggccaccctcactcaggctctggaaaggcgatcgaatgtccttcgcgacgcggcagcagcagtttaaggccgcggtccgggaggggctgcctgacgacgtcagggtcgccgaaaacttcggcttctccaacagcgcccgcgtgatcgaggggggcctgttcgcggccaccgttaacatggagttgccgtccaagctcgcgtttgagggaacgccgaccctttcgggctatgtcttcctgtgcgttttgaccttcccgccccacgacgaggtctatttcgcgatcaccgtccgggatggcggtgcggcgctgaacgccggcctagccaagctgtatgagctccgccgcgctgagctcgcgggcagccagggaggcaagattaacaacaacgtgaaattcttcctgacggacgacggccgcatcgccttcggcaacgagttcaccgatcgcctggattcctcgacgatcgatccggacctcagcgcgccggtggatttcgtcgagttcgccatctggccgccggccgtgtcggcgaggcgcagcctgctggcgcgggagttcgtgggctacctgggccggctggtcggacgagatcgcgttcacgaacgggcggtgtggacggaagaaaccgccgtcggacctctgatgcagcgcatgccggcgaccctggagcccgctgcgcttcgacaggcgatcgccgatctggggggacactaccccgacgccctggtcgaccgcttgcatgccgggttgaaccatctccagcacaagcatttcgtcatcctctcaggcctttcgggcaccggcaaaacccaaatggcgctgcagtacgcgcgggcggtgcacggtctgcagtcgatggacgccgccgaccctctgctgttcatctgtcctgtgcgacccgagtggaccgacccgtccggcctgacgggctacgaggatcggctgacggatcgctatgtcacgcctcccttcctcgaggccgtgctggtcgccacagcgcatccgaactcgccggtgttcgtcatcctcgacgaaatgaacttggcgcgcgtcgagtactatttctcggacgtcctgagcgccatcgagagccggcatgcgctacagctgcattcgagcggcgtgccgatggaaggcagcacgggcggcgaagtgccggccgatctgcgcatcccagacaaccttttcctggtcggcaccatcaacgtcgacgaaaccaccagcaccctgagcgacaaggtgctggaccgcgcggtcgtgatcgacatgtcggaggtcgacctgcaaggcttcttcgccaagctgtcgggcgccagcccggatctggcggacagtgttgatgcgtctgcaccgctgcttgaggccctcagcggcatcctgcagccgcacggcctggggttcggctatcgtcttgcggaggagttcgtgcgctaccacgccttcgccgtcgggcggctgggacgggcgtcggctgaagttctggacgacctgctgctgcagaaggcgatcgcgcgtctgcgaggcacggacgcccagcgcgacatgctgaccgcgttgtcggccgcgcttcaaccctatccccgcgctgctgacttggtggcgcggctgcgccgggatctcgaagaactcggcgccttccagaccgcgcggtgagcgcgcgtctggaaatctggcccggccgagacccgtctcgggcgatccgggtctggccggctgctgacacgccagagtccggcgcggttcaggaggctggcgagcacctgttcgtcctcctcggcgcggcggatgcttattcggccgatctgctaatcgatgacgttccgcttgaggcgctgcgcgctccgaccgcggatcaggcgcggtggcgatggatcccaggcttccacgcaggacaggtcgaggcccgcctcgttcgaccctcggggtcggtgcggttcgagttcgtcaccgatccggccgtgcggaagctgacccgtgaggccttcgaccagatggtccgcgagacccttgaagacaccttcgcgctcttttccctctccgccttccgggcgggcgtggcgctcggcgccggcaggagggcgccgccgatcgctcgcctggagtttctgcgcagccggatggccgacctgaaggcgtcggtgcaatctgtggacgcccgcccacggcgcgtgctgcgcgccgagatcgagagggtgccggctcacagggcggcgcgggcgaccgccccggaggtgctgcgctccttccggacggggcgtcttattcagacggatcgcgctgaccgccttcccgcacggctaaaggggcgccttccagaagtcatccgcagaaacgcgcggcgcgtcagccaggacattcccgcgcaccggcagattaaggcttcgctggcgctctgggcccgctggctagaggcggtcgctcggctgctgaaccgccccggatcggatcccgacgccgcgccgtgggcgcgccgaacgcgctcgatggcccgcgagctgcgagggctcctggcgctggacatgttcgaaggcgtcggcgatgggccgccccgcccggacgcctcaccgatctggcggggtgatccccgctatcggcgcttcgcccggcttcatcgggacatgtcccttggcatcgcagcggtgttcggcgatttcctgcagatgccgctggctcgaacgttcgagctgtacgagctctgggcctacctgagactggcccgcgccgccgtcgaacgctggggggcctcggctgaggatgtggccgagctgttcgagtccggggcaggcgtcacactggccgctgggagcgcgcgactgaacctgccgcaggccggcctggcgctcagctttcaacggcgatttcgggagtactggctggagaaggatggccgcggcagtttcagccgcgaaatgaagcccgacatcgtcgtggagcggccgacgaatgaggcgggcgggctcatcgtccttgatgcgaagtatcgcatcgggtctgatctgaacgacgcgctgtcctccacccacatgtatcgcgacgcgctcgtccgcgaagacgacgacgggcctccgcgccgcgtggtgcaggccgcctacctggtcaccccggctgcgcccgtcccatccgaggactggcgcagcgcgtcgatgcccggacgactgttccacccggagtatcgcggcgccttcagcttcggggccgtgacgcttacgcccggcatgtcgctcgaggccgtcgccgacgccctggatctcatcctggcggatgcaacccaggacgccggcgtcactgcagggtcctcagccagcgcagcagggcggtcccgcccgcgacgctgagatgggcccgcgcccgggacaggccgacataagccagcgccctgttgtctgctaacgagggctctgcggcgatgaccaccgcccgacgctcaagacctttgaaggcagcgatcgtagagaccacggcggcggacgccgtcttcggcagagccgatcgaaccccgtccaccgccgactccgtcactgtgagaatggccagctctcggggatcgaccttttcttggacgagcaggcgccgcgcttcctcgatggctgcgccgatcgcattgctgtcctcgatccactggatctccccgccttcaggtccatccggcgtgaccggaagcccctcgtaaaaccgggaggcggcggcgtggatcgtccgggtgttgcgcagatttcgggtcagcgcgatcggcgccatctggaagcccgccagctccccggacaggtcgccgtatacgccctggttggcgtcaaaataggcgtgcagccggctgagacgaacgtcgcggagagccgcctcaagtgcgatccaccagtgacttctgaagtcctgcgcctcatcgacgacgatggcgtcgaaccgctcggcgggcgccgccagcatcgcatcgtgcagctcctgcggcccctgcgcctcggtgaagggtcggcctgagacgcggcggcacaaagcggagaacgattccaccgccacctccgagcccttcattcgctcacgcagcgcttccgccagaggctccgacacgcaggcaagcagggttctcagtccctgctgcgccgagcgggcggcgtcttcgcacgcgacgatcgtcttgccggcgcccgcagcgccgcccacggccacgcgcggcagcgcctggatggcgtcaaggatgtggaactgctgtggggtcagcgtgtcgatgacttggtcgtcgtcggacaggcacgccgccagcggcgccctcaggctgaagggaaaggccagcaaccgctcaagcgccacaacaccgtcgcgaccgaaatcctcctcatcgccgccggccagccgctgctcgatccactgtgcgatcctgggcaggtcgtcgtggcagcagaatagctcacgaggcttgtcgacccccagattgccgggcggcgccagggcgtcagggaagatcacgccatgccgcatccgataatttcgggccgcaggaaaaccgcgcgacgctttaaggcgacggtccagctcgtatttggccttcttggcctgctcgaccgggttcgagatgcggtggcggaacccatctcggtcacggctcagccagtcctccatcgacggatcgtagctgatcccgccgcctttcacttcgatcgccaagaagccgcggcgcgggtgagcgacgacgaagtcgcactccccgtcccgctctccgcccgtgcgggtcacgccgagccagggccggctgtagaataccgtccagtccggccccagcgcctcgcgcaggcgacgccagacctttacctcagcggcgcgatagcgatcggccaggaccgactgcggcaggaccgccggccacatgcgagggccgctcatgagcgttctccggaaagcagatctgtgaagaagcccagtccgggctgtgaaggcgtcccaaccaggagcgcacggtcgaggaagcggttgaactcctcgcacgacgtctcaggcgcgaggacgcaggcatggcacgcggccagcgtgagcccatcgcccggcgccatcatgtcttcgatgcagagcggatccgaggagcaccaggcctgagaccggacggcggcttcgaccgtgcggccgatgcgttccggatcgccctggcgctgcagcccgcccagcgtgccgtcatcgtcggtggtcgccgtgaagatcagcaggcccgccatcgcccggtcgccggatcgtacgtacaggcgctcacgcagcgccgtcgacgagtagccgcagtcaagcgtaagctgacccatcagggcatgcgccagggtatggatcatcagcagacgcggggtgatgatctgagtccgcggcagatcggggccgtaacgctcgagccattccgcgccccatcgcgcgtcaaccgtcgccgcccgggcctggacctcggcccgcgtctcccaggcgctaagggcctccgcgtcgagttccaggaacacgccctccccgcggacctcgatcgctggcagccagtccagcggccgcgcggagagccgagccgcgagcgacggatcgccagggggatggacccgcgtgaagcccgtcatggcccgcacttcgcgaagccgaacggccttcaccaggcgtgagaaccagggccgaatgttcaccggcacgggtcgcggcctcacctcgaattccttgtcgagactgctcgccgcgacaccgcccaggaactggcgatactcctcaaagcgaaggtcatcggtgtcgatgtcggcctgctgcgcctcgcgacgatccagttcggcggacaaatcctcggccgtcatgctcagctcggccagaaccggcgccagatcgttccgagcaaggatgcgaatgaacggccccctgtcttcgggatgggcgttcatgatgttgtcccagtggacgccgagcgcctcctgcaggcggtccgaccagggcggaatgctcagggcggattcgaccaccgggaagtagaggtttgaggcaccgcgctgcaccgcgcggggcttgcagccgcagctttcgtccccttcagcgatccagggccggcgcccccggcagtcggccatgcgctcccaggtggatttcgagaacacgccgtccatggagcgtcgctcgtggcagctggggcagctcagcttcaggcccgccagacccgcctcttctgaacgcagctcaagaaagccggtacggttgcggcagtccggcttgtgaccgacccagtagtgccagggaaactcgtccagatggccgcgctcgcaggcgaggacgaaacgcaccgggatcgtcggcaccggcgtgcggcccggcgccgtcgcagtgcagggcgcgcagtatcgtccggcccgtcccggcggatcatcccacagggaggccggaccgattctctcgcagcggggacactggagccattcggggaagcggacggccacgagcgcccgattggcgtcgcggtcggagccggggtcgcggaccggcggcagcctgaagcctcgaacgttgagctttttctgcagacgttcctctcggatcgcctgcgggtggaggaggccgccaggggggaagttttcgtcccattcctccagaccgcccgcgaccgcgctgataggcgcatcgccggctcggaaatcaatcagggcgccggggccgaaaccggcggctgcggcgctgcggcgcagatcgccgagatcattacgaggcattttcactccgacggagacgctcggcgagacgatagggggtggacggctccaccccgcgaagagtgttgggcgtcggccaggccgaacccggggtccggccggacgcccggcgcgccgcggcgtcctcggcgctctgaagcagagacgctccgggggcgttgtgacgccagtaatgctgaggcgcgcgccgacgccaccggcggaggcgttccaggagttcgtcgcggacctcggtttcgagcggatcgatcgcctcggcgcgcgcggcgatgcggtcgatgagcctcagcgcttcgtcctccgcgtgctgcgtcagcgccggactgtccagcatgcccggccccagatgccgcacaagcgccaccaggacggcgtggagcgcccgatcgcgtgctcgcgaggcgaacggcgtaacgcttgtcgcctccacgtttcgataaagagcgtcgtgccacgtccggaaggtctcatagtgggagcggtcgcgcggcttggcgttgttgagcacgctgacgacgaggccggcgacggcgccgcggccaacccggctggtggcttggatatactcggccatggtcttcggctggccgttgaccagcatcagcccgagccgggagacatccacgccgacactgagcatgttggtggccaggacgacgtccagcgcgccggcggtaccgatggggcgcccgagacgatcgagcatgtcgacgatctcggcctggctgcgccgagatgtgagttcctcgacggatgccggctggcgcggcggttctccgcgcgcccctgcgaggagcctcagcgtatcgttgacgtcgtcctgcatcagcacaagcgcgccgccgagctcgcgcagggagttgaagtaggcgacgagcgtcgaccatggatcgcgccgcctctcagacagtgcgcccgtcgacgcctgcaacagggaggccgagacggcctgaagggtgaacttcgccgaccgccccgcggtggtcacccccgcataaagtcggccgtccgcatccggatcgacgaccgcgaatccggaatcggcggcatcgagaccgggcggcgggaactggcagatgttccgatcgaacaaggcgcggacctgttccgcggcccggcggatggttgcggtcgacccgatgatcttggggcgggatccgtccgccgagagaatgagatcgagggccgtttcgtacaggcccgcgagcgtacccagcgggccggcgatcagatgcagttcatcctgaaggatcagctggggctgggcgccggagcccacggcaaagagacgcgcggtttcgctgcgacggacgatctgcgcgaacttgtcaactgtcccgatcagcagcgtcgggcgaacctcatacacgtcctcgtcgacggtccagaccggcagccgcgcctccgccagtgcgcagtcccggctgcggcaccagacctcgaccggagccctgtccgcggcttggcgatagtcgagaggctgccgacaggcgggacagtccgtcagctgccggggcgacggtcggccgggatcacgccagctcgcgaaggcgtcctcgcgccggttgggcgtggcgctgtcgccgacccacagaccaatggagaagggctcggagccgagcccggcctcgccggcacgccgaagcgcctcacaagcgcagatcatggccgcggcgcgctggaactgctgcgacgtcagaaggcgcagcgtgtaacgcatcagggcggcgacgcccgcgcccttatcgggtgcggcgcgggacaggcgacgatggaaggcggtcagggcgatcagggccaagtaggcctccgtcttgccgccgccggtggggaaccacagcagatccatcacctcgcggtcgggatggtcgccgtcgagcgtagattcgagggaaagaagcacaaagccgagctggaaggggcgccaccgcaggtccggggcgccgccccactgccgctgcaggagcatcgcccgattggccagccgaaacgacctcagcaccacgggatccctgcggagtcgctggacgcctgcggccatccgagccagcacgtcctcgcaggccctgaggtgacggcgcgcggtggccgccagggtctctggaagccgggcggcctcgtcggtgcgttcctccacccagcggccgtaggccgcgcagaaggcgtcgagggaaaccagggtctcatccgcctccgcttccgccagccaggacgctgacaggcaggacgcgccttcacttctgaagccgctgaagcaggcgtgcccgtccgggctgaccgcggaggttacggtcgatggaatccaggtcgtccgcacccagtctgcggcgtccggatcgtccaccgcagccgcccattcagctgaacaggtgtggcccgacgcgaactcgcgcgccctgcggtacagcagggctcccgacgcgtcgtcctcgtccaccaccgcgcgacggctcgggcgagcgatgaggcggctcccgggagcggcgacgatctccagctcggtctggaacagggtcagcgcctcgagggcgttgcggttcggttcgcgcgtcgccgcgccgttgacgagcgtcacggtggtcaggagcccgcgactgaagcgggcggtgcggatgttcaggcgcaggcccacaacgccgccgtcggaaagatcgaggtcggtaacccccgggctcagcgtggcctcgcgcctcagttcgaccgcacgtctggcccagatgcgcataccgtcgccgccgtcctcaggctcatagacggcgaagcgaatggtcaccccgatggccggcgcctcggtcgccgcaaccgcaaacgacaggccggccgtggacgggcggcgcatcggcgcggtggcgggctgggcctgagcgcctccatcgtcatcggcgtcgccaccggtcggcgccaccgcgagagattcgtcttcttccggcgcaagttcggtgttgcgcggccacaggatgcccgtcagccagacgtcggacggccgggaggtcagcctttcctcgggtcgggacgggccgaccaggtcttctctcagtcgctgaaggacgatctcgcggcaggccgcggaagaagtgtcggtcatgaaggggtccttgatccaccgaaacggccgaaggcgaagccagtcagcaagggcgccagcatcaggccgctggtccgccagggttcgtgcagtcgttcgagcacggggtcgtcaggcgccagcgcaaccgtccggacgccgaggctcctcagccaattaaggcggccaggcggccagcggttcgcctgcttcgcaatcgccctcagattcgatttcaccccatcggacaggacaccgagacggtcgccgtcaacggactccagggagtagcgatagtccaggtccgaacggctagtcgctatgagccccagggccgagctttgggagacccgggcctgcgccgcttcggcctccgccgaggacgcgaaggccacagtcccgacaagcccctcagggcgaatatctccctcccggccgatctcgacctgaacgccgttgttcttcgaacgacgccagacgcgtccctcttccgaaccggcatggcacagtccggcgtttccgactcgcagggtcaggcgaggccgggtcgccccgacgaaggccacgcggatctcttcgtcgtcggattgggatgcaccctcgctcagaggcggcagccagaggctcacatgatcggcctctcgtcccttgctggcgtggatcgtgccgacgatcggcccctccgacccgaactccggggtcgcgacaagcagcggcgggctggaccgtgcaagctggcggcgcagacggtgcaggtcgagactcccgtccgcctgcccgccgagctccatgaggagcgcccaccgcgcctgagattcgccctcctcgacgccggccgcgaccgccagcgccagaaaatccgctgacccgatccgccgatcggtccagttccatagcagctcggcgatccaggggtggatcggggccggcaggcccgacattcgcaggcgatagggccggccgttggcgtaggacgccgccttcagcacctcggcgcggcgccggaacagaatgagcctgtcggctcctgcgctcgccaagccgccgtcctggcccggctcggcgcattcatgcgcgagacgaaagatgtcgtcgcgcacggcgacgccccgatccttcacgccgccgcgggacatcacgcgtctgcgagtcttcagaaatagctcccgcagccggggacagcgcgtccgccgcacctcctccagcgcccggcgcgcgaagtcgttcgggatcaggctcagaagcgagactccgccgcccagaccggcctcatcctcggtgaagccgtagatcgcctgcgccggatccgcaaaaatcgtgacgcccgcgtccggatcgagacggtcgatgatcgccgacacgagctgggcccggacgcccatgatgtcctgagcctcgtcgacgatcaggtgacgcacccgagccagatagtcctgaagatccgggtccgtcctcacgcgctccagtgttgcggcgatgccttgatcaaaactgcccgaaagcgtggcctcggcgtcaaagccggactgcagcgcccaggcataggcgtccagggtggacaccctgacggaggcggcgtcctgggcccccgtgaaccccgcaatgcggtttcggatctcgctcacggccgcgcgcgtaaagctgatcatccagatcttggaccccggcgtcccgccgtcgatcagggcacccacccgcgcgcaggcggcccaggtcttaccggttccaggcggcgcgtccaccagcaggcgacagtccgcttcggcgttgacgattgcggcctgcggatcgcgctcagccgccgcgccgatctccggatcggccggcgggcgcggcgcggcctcaagcggcgggccgtccagatcaatgacgccgtcccggaccggccagcgccgcttccggtagacgatgacggcttcgttctcgcccgtgaacggagcggccgtcacccgatcgatctcccgcccgcccttgcggaccgagatcaccacatcttccacctgacgcgccccacaacccactttcgcaaccagtggtacccaagtattgatgctgtgcaaatacggggcgttgcattttatgtcggctgtggaaattgtcacggaggcggctgcgtctctgaccgcctacgcggagcggctctgcgacgaccgtctccaggcctatctggccgccccgcacgacgcccgtgaacacgccaacgtcgagcagtccgttctcgccggcggctatgcctatcgccagatcgcggaactagtgcagaacgcggccgacgcggtggtcgagggcggcgcatcgtccggccgcatcgttgttcaggtggacagcttgggtctctgggcggccaacacgggcgacccggtggatgaagccggcgttctcgcgctgctcaacgcgaacacctccgggaaacggagcggccagatcggtcgtttcggcctcggcttcaaatcgctcctcaagcttgggggcgacatcgcggtgctcagccgcagcgtctgcctgctgttcgatccgcccgcctgccgggcgcagatccgagagctgctcgatctggacagcgaacagcccgcgccgggcctgcgcctcgccgaggcccttgcgtggaccgaggggctggcgcgcgtcgcgggtgctgaccgcttcaactgggcgaccacgatcgtcttcgcccagctcaagacgccggactcagcagtccgcgtcatgcgcgaaatgcgggatttcccggccgagtttcttctcttcctgccggtggatgtcgagctggtgctcaagggtgaagatttcgagcggcaccttcgacgccgctcggaggatgacggggccgtcgtcatcgaagacctctcggacaccagcaaaacgcctcagcgctggcgcgtgttcagtcggcaggtcgaggtcaccgacccgcttgcggtggaggacgcgacggacgtgcatgcgcgcgaacgaatcccgctgatctgggcggctccggtcgggcgggcgcgggagcaggcaggccggttcttcgccttcttcccgacctcgaccgagactcgcaccctggggatcctcaacgccccctggaaactcaatagcgaccggacggccttgatccgaggcgcctggaacgccgccctgatggaggcggcggccgagttcatggtcgacaacctggagaccctcgccggggacatcgaaccgggcgccgtcctggacgcctacccgcgcgaacttcagacgcaggacgagcccgccgcgcccctggtcaacgcgctctggcggcgacttgaggccgacgcccgcctgccggactgcaacggcgacttccggcctgcgcgcgacctgaagcgggcgccgcttgatctgcccgacctgggcgtcatgtggagtcggctggcggacgaggaggcctgcgccgagcacctgcaccccagctgcacggcgtcggctgggcggatcgcccgcctgggagagctcacgcggcgactggtcggggattccaaggcccctgccacagccgtgctgtcgaagtcggacccggcggactggctcgaagccgccgcctccctcgaacccgacggcgccagctcggcgctggagctcgcggatcgctacgcccaggccgcgaccggttacgactgggaccgcgttcgggaacgactgcgcatcatcctggacgccgacggcgcgctcaggccggcgccggaggtgtcgctctcttccgacgagcagggggtgctgagcaaggtccatcccgacctcctcgccaacgcccccatccgcaaggttctcgaagaccgctttcacctaagggacgcatcggacacggactgggatcggctgctggaggcgcaggccggggtcgcgcgcgacacggacgactggtccagggtctgggagcttctgcggcgcatgccctgggaggcagtgaccgagtcactcgactgggtggatgtcgaggtgaagacactggaaggctgggccgcgccggatcgctgcttccgcctgggcgagctgatccgaccggaagacatcgatgacgcgaccgaagagaaccggccctatctgaggtcctggctcgtcgatgagacattccatcggcacgacgccgccctgctcgcgcagctcggagtcacgagcacgccaaaggcggaatgggagatggtctggcgggtgccgcccgatacggatccggtttcgaaggcctggatagaaggctggtccgaccagtggcgttacacctaccaccgcgatctcgaccatcgaccggccattggatacctcgggcctgcggatctgaggctccccataggatgggagcttctggttctggccggcgcagacgccaaggcacgcgtgtccgcctggctcctcgaggcgtgcctcagcgccccccccggggcgctgaggccggcggtcttccgtcacagcactcaggccaagtgggcggcgaaggactatccgcatccgatctggtctctgatgctcgcacacggctggcttgaagtgtcgggcaccaagatcgacaccaccttccttctgatcgacgtcatcgcggagcgcggcgcccttctgccttcgctgtcagggttcctgtcgggtctcgacgctcttcggaaggcggcggggggctatcagagcagtgttacagacgaaaagctgtggccggcctggctggagatggccgcgcgcgagcgaggggaggcctccggcctcgctccaatctacgaggcggcaggacgggcggggttcgcgccaagtgaagtctgctccagagacggtcccgtgcccttggccgacatcctgatcggacgccacgctcgtgacgtagtccaggccgcagacgccggccgctcgtgtatcagcctctccgccgaggtcggccgcctctgggtaaagagcggcgctcgctggttccatgaaatcactcagctgcagtggatcgccggcgagtccggggcagaggccgtacgtattgttcaagtggagcccgcgattgcggaggtgctcagcgaaagcgccggcggcggcgcggtcctcttcgtcagtcatctgactcagaccatcgccggagaagactgtgcgatcgcctgggcagtcgatagcgatcggctgctcgtggacgagcagcattatcagcgactgggctggaaagaccgcgtcgccctgctgctcgaggggtgcggagccctcagctggctcagcgttcccaacgctctggaagtagtcacctctggcggcgtggccgcgcgtcgccgtcacgtcgcggagggcaccgatctgcccgaccgactgctgcgcgccgtcggcggttcgcgggcgttcctggagctgtttgacgccgaaatctggacagagctggccggggacgatcaccgcgccgctcaagtcgttctgaccctgctcggaccggcggtcttcgcggagcccgtcatacgagcggcccttgtggcgcaggggctcgagccgccggagcgctggggcggagagcaggcctccgcgttcatcgcggagatcggatttcccggggaattcgcggcagccccgggtcggcgccgagaacctgaactgttcgtctcggggccggtgcggccacggcctctgcacgactaccagatagacgtcgtctctgatctcgaccacatgctcgccgctacgcaggacgcgcgtcgacgtcgcgcggtgatcagccttccgactggagccgggaagacgcgggtggcggcccagaccgccgtgacacggacgctcgccccagacagcagcaacaggctggtcgtctggatcgcccagaccgacgagctctgtgaacaggcggtccagtgcttccgcgatctgtgggcgacggacggggtccggggagagagcctgcgcgtggttcggctttggggcggccaatccaatcctcaggccgctgagcctcatgaaccgaccgtcgtggtggcgacgatccagacgctttcgtcgcgcatgaacggcgtgggcgtcgactggctgagccgaccgggcctgatgatcattgatgaatgccatcacgccctgacgccgacctacaccagtctgttccgctggctgaagcctgacggagacggcgaggcggaaccgccggtgctcggcctcagcgccacgcctttccggggccgtagcgaggatgagaccgccgcgctggcccgtcgtttcgacggccggctgatccccgctaatcaagccgggctctttgaaaaactgcagggcaaaggcgttctggcgcgcttccgatacacgcggctggagatgcagacgcccttcctgctgaccgctgaagaggaacggcatctggagacctttcggacgcttccggattcggccctcgaacggctgggcgccagccgcgaacgcaacgacctgattatcgaagcgatggccaagtcgaccgagcgatcggccctggtgttcgcaacctccgtcagccatgcgcgccggcttgccgcgcggctcaacgtgctgggcgtgccgtccgctgcagtgtccggcgagaccgaccgcaactcgcggcgctggttcatccaggccttccagaagggcgacatccgggtgctatgcaaccactcggctctgaccaccggcttcgatgcgccggccaccgatctgatcgtcattgcgcgccctgtcttcagccctgcccttttcatgcagatggtcggacggggcctgcgcggcccgctgaatggcggcaaggcggcgtgccggatcctgactgtccaggacaatctggacctctactccgatcagctcgcgcatcactacttcgaacagtactacgtcacttaggggaagcctttggcggctgcagtcagactgaaatgggaattgatggagttcaccgcggcggacgtcagcggctgggttccgtttcgcaaagcggtgaacttggctgaacgcaaaggcgtgctgtctcagagagcggtctatgtgatccgcatctgcgagccgttcgccttcgactatgatgaggccttctcgccggtggtctacatcggcaagggccagttccagcagcggatcacctcgcacctgaagagctggattcgggagctcgcgaagcgaattccggggctcaagatccgcatctactactgcgagcccagggtgcgcaggttgggcacgatctgcgagggcgtggaagctgacctcatcgatcgcttcgtgatgcactatggtcggcgtccgctgcgcaaccgcaacacccccacgcaccccggcgtgcggacgtacacaccaagcgaactgcacgtccttcaccccggaaaggggcgtcggtatcactgggcgctccgacctctgccgtcctgccacttctaccgctgacacccctctcttcgccaacctctcggcccggttcgtcggccgccccaggatcttgccatggacgtcaatctccgcgtcaccgacgctcctgaagaatccagcttcagcgacctagtgtcgggcgacaatgtgctgtcgatcccgctgtttcagcgcccctaccgctgggcgaataagcacctgcagctgctgctggacgacgtcgaggcggtgcgcgaggaaacagcctcgtccgtcttcctgggcgtcatcgtcacgtacagtcgcggaacggggccgggccggccggtgacctgggaggtcgttgatgggcagcaacgggtcacgaccctctatcttctggttatggcggcggtcgaagtggcgagccgcaagggcgcgaccgaatgggccgccgcggtgaccggcagctatctgctggtccggccgctggcgagcaacccggtgaacaccaagctggtgccctcctatgccgatcgcgcccagttcgcggcgctgtgggcgcggatcgccgatctgcccggcctgaagggcgacaagtcgttcgcgttcaacccgccgatgccgccgcccgccagcggcccggcggaaggagagatggcggagcagtacaaacgccttcgtctgcacctggcgaagctcgcggacacaaacggggtcgaagcgctcgagcgcttcgtcgagatcgtcgtgcgccacctcagcttcgtctcgatctcgctgcgcgatccggccgtggcgcccaagatcttcgagcgcctgaacgctcgcgccgaacccgttacgatcgcggatctggtgcgcaacgaagtgttctcacgctcgggcggcgacgcgattaccgctcagcatgtcttcaacacctactgggagccgtttgcggccagcttcaaggcgaccagcacggacctcgctcgcttcctgtttccctacggcctcatctccagtccggggctgcgcaaggccgacctgttcgccgagctgcgtcgccgctgggcaggctacacgtcaccccaggacatcatcgccgatctggaacgctaccgcggcacctatgtcgccctggaaggcggcaacgccgatccgcatctcacgccggaaatcagccgccagctccaccgcatccacagcgtcggacgtccgtcgtcgacctacgccttcatcctgcgtctcgtggacgcctggaaacagaacgccgtcgaagaggcggtcgtggtcgatatcctcacccgactggagtcgtttctgttcagacgcgcgctgatgggcattgaaccgacgggtctgcacgccgtgttcaaagggctctggaacgaactggtcggagccggcgacgggtcaaagctgacgggcgaggccttccaggccgccgtgtccggcaagcccaccatcatctggccgaacgacgagcagttcgccaacgccatccacaccggcaatctatatggccgcaaggtgcgcaactacgcccttcgggaacatgaggcgtcgctgtccgcggaaaccgcctccgatatcttccaggtcgaacacatcgcgcctcagagcggcacggacgcctggcgtgaaaagatgggcgagccctacgaccggctgatccatacctgggggaacctagtgccgatcagcggcaagatgaacccgacgatcggccagaagccgttcgagatcaaacgcgctgagttcgccaagtcgatgttcgcgaacgcccggcatatcgcggaaacttgcgaagactggtcggctgaaacgcttgaggcccgtaatcaggcgatcgcggactgggcgaagacgcggtggtcgcactgacgcgtatggaggcgctccatctgcacccaatggtcaagctgaaggaatggctgcaggtgtcgacccagccggcgatcgaggaagacctatggcttgagcccgcggacatagaggttatcgccagcgccgttaccgagatggtccgacgagtcagacgcggcgatcctccgatgaagccaggcgtccccttgtcgcttctgggcgcgcgtctgcgagccgcaactccgggcgcgcccgagccgcgagctattcgcgccggcacgcattccagtatcttcggaacatgcacgatcgacctaagcccctttccgatcaatgctagcgatattggccctctacaagcggacctgacggagttcgagaccgcgatgctcggactgctggcccacgaagcgtcccacgtgcggcagcgcgaaggaggcgagcggacatccgcgatgcaccaagcgtccgatagggccagccaacgggcgtggcggacaaaactttacgacgactacatcgcttatctcaagacacctctcgagacggcggcccatgcaacccagctggcggtcgagcttcgacacttgcatggtcctgatttaccatccggatcctttctccgtctctgccgagcgagccccatctggatgcatatgagcaaccatcctgactgcccgccaacttcgcctgcagccggtcgaaaggcatttggtcctgtgtcccggcgtctcctgtggaacgcttggtgggtctatctacggctgacgaaccggcctcctccgtggcgaacgcgcgcatggcgctggttggtcgatcggctgccctgaggaccacaacggccgacgaactacgcggggacgtgcgtcctcctggcccaaaggtgcttgttcatcgtcgggagatgatgttcagcgccgatgccgttgaaaaagggggcctccagcgatggcatgagggcgccgcgctgattcactctggtcgttgaggccggaggtgcagcgatgatgggagagcggcgggtcgatcaatcggctccgttctacgagttctcgctggagcggcatgtgccggcggaccatcttctgcgggcgatcgaccggttcgtggcactggacggcctgcgggcgcatctggctccgttctatagcgccatcggccgcccctcgatcgaccccgagttgctgatccgcatgctgctcatgggctactgcctcggcatccgctcggagcggcgcctatgcgaggaagtccgcctgaacctggcctatcgctggttctgccggctgggcctggacggcgacgtgccggaccactcgaccttctcgaagaaccgtcatgaccgcttccgcgacagcgatctgctgggggaactgttcgagacggtgctgcggcgctgcatggccgagggtctcgtcggcggcgagggcttcgccgtcgacgccagcctgatcaaggccgacgccaaccgccagcggtgcgttccgggcgacgaaggtctgccgcccgaagccgccaatcgcgccatagacgcgtacctagctgcgctggaccacgcggccttcgggggcgcgactccggtgacgcccaagttcatctcgccggctgatccggcctcgcgctggaccggcgccaacaggggcctggccttcttcgcctatgctaccaactacctgatcgacctggaccacgcgatcatcgttgatgtcgagccatccaccgccgtgcgccaggccgaggtgacggcggctcgcaccatcatcgagcgtgcgcgtgagcatcatgacctctggcccgcccggctggcggcggacaccgcctatggctcggccgagatgttggactggctggtccacgaccagggcatcgagccgcacatccccgtcatcgataaatccgagcggatcgacgggaccttctcgcgcgccgacttcgcctatgaccatgccgccgacctttaccgctgtccgggcggcaaggagctgaagcaacatcggcggcccttccgcgcggaccaccccgataccccgccggataacacctatcgctatcgcgccagcaaaatggattgcgacgcctgcgcgctgaagagccgctgctgccccaatgcgccggcacggaaagtgacccgctctatccacgaaggcgcccgggacttcgctcgcgacatcgccaagtccgacgcctacgtcgtctcacgacgcgagcggaagaaggtcgagatgctgttcgccgccctcaaacggatcctgaagctggaccggctgcgcctgagaggtcccaacggcgccagggacgagttcctcctcgccaccgcccagaacctgcgcaaactggccaagctgatcccgccaccggcgccggcgttcgcctgaggcggaagaaaaccgccacgtcctttactggcgacgagctcatcagcccgcccttttcaacgaaatcggccacttgcagaagttgggatcacgccatgcgtcggacgttcagcgagccgctgagtttaacgcgaacactcgcttaccccttgcttcaatggtgctgtcactcccatcatgaggcggcaaaggtgccgtcgctaggcacgactgaggtttagttttcaaaaaccccaccgactcctgtaggacatcgatcgaactcacgtgcttgcagaacgtgatgcgacttgaggggttggggacgggatagaatgagcgctggagcttggacaccgattgaatcttatgccgatgctgcagcccgttcatacttagccgctatcgtcttggaggacattggcgatccatcgacgtcgggtcacctgtatggcgtggcggcagagtgtgcggtgaaggcccatctccagagcgcagggataacaatcgaccggcccctgaaagtccatttccctctcctgacccaagcggtcaaccttcatggccagagccgtactatgatgccgctgctgggcttgctgttggaagggccgcccgaacttcttgaaggttactcgattcattcacgctacgctcaagacggcgatgtcgatgatgtgcgctgcggcgagtggaagaacgacaccaagcagatcatgtccttctgtgggttttcgatatgaccacgcttgcgccgaccattgattcgggccttgacgccttcgtcgagtatcttgacaccacgctaggagagacttcgtcggaagggcgtatcgtccgagatgtattcggtcgattgaccttcatcgccccccctgccttagacgacgcaacggtcgcggcggcaggcgctgacttacctgaggccctgaggccgttcttgacccccaaggcgccgctcctgcccgcttcttcgagcctagcgacgccgcttcttgaggaggccggcgttccgatcgtcgcacctctaggtgcgcgctacattttactggaccggcgtgtggccggcgagggttggcttagcgccccgccacacgaggtgtccgcagtgccgcgcctagccttctacggcctcaaaggcggcgtgggccgctccacggcgctagccgtttgcgccgccgatctcgcactgaccggtgccaacgtcctcgtgctcgacctggatctcgaggctccgggcttggagagcgttctcctgcgtcctgaccgtgtgcccgactacggcgtccttgactggatggcagccgccacggccgggctggacgtcagtcagctggtgccggacatgatcggcggttctccgttcacgtcgggatcaggcttggtggacgtcgtgccggtcgtcggtcgattgactcaggcgcgtccagacacgttcctcagcaagctgtcgcgtgcctacacgcccggggcgccgtccggtgagttcatgggcaaatccttcgcccagaaggtccaggtcctcctagagcaactggaagggcgtcggcgttacgacgtcgtgctgctggacgtgcgcgctggcctgcacgagacctcggccgcctccctgctaggcctaggcgcaaaggttctgctcttcggaaccaactcgcctcacaccttttcgggatattccattctgctgtcgacggtccggcaagccatggaggcctgggagtcggcacccgagcttcgcgaccgcttccagatggtccatgggcgggcgctcaacaacgcgcaggatcgtgcgctttttctgtcgaactgctggcagttgtggctggagcatctttacgacgccgtcgatgatgacgttgatgtcgaagcgtttagcttcgacttggacgatcagaccgcgccgcactaccctctgacagtgtcatcggccgaggcgttcatgaacttcaatccagacgccgatcccgatctcctaacggcgcacggctacgcaagcacctatggcgaactgctgagctttgttcgcggctacgttttcacgaaggcttcctgatgagcgcgcttcccgccacaccgcttcgcatcgcgttgagggagctgaagggcaagaccgctgagatcgcctccgacgctccgggttgggaacgagtgctgacggtccgcgatcatgaaggcgccttggacccctcgcgaccgatcgtgatcggcgatcgcggcactggcaagagcttctggacgggcgcgctgctcgacgccgacaggcgagagcgattgtcggccgtctatccgcggctggcgctcgacaagatcgatgtggaactaggattcggcggtgacgagttctcgagcgctcatccgaccagcagcgaactatccgaccttctaaagcaaggctttagcgccgaagcgatctggcgcgccgtcatgctctcggttttgcccgcgccggtgcgtcctgccgaggtcacgacaggagactggcgtcggagcgtggcctggatcgccgaggatcctgccttgcggcgcgcccagttccaagcggccgacaagtatcttgtcggtcaaggtcggcagcttctggtgatcttcgacgcgctcgacacgctatcgtcagattgggacgaaatctccaagctgatgcgcggcctcctacaggtcggtctcttcctgcggcccgcccgcgggttacggctgaagctcttcttgcggccagacatggtcgacgatccgcaactctgggcggtcggagactcctccaagctacggcatgacgaggtcatgctggcctggacccggcgcgaccttcacgccctgctcatccagtatctggccaaccatgttgaaacccgggctctgatccagcaatacacacgcgacaacttcaggaaggagctgaactacgagtcggaccggttcgaggttccgtccgaactgctgaacgacgagaccgcccagcagaagtttttcgcctcggtggccggcaactatatgggccgcagcgcgaccaaggggcggacctacacctgggtgcccaatcacctcgccaacgccaagggacacgccgcgccgcgaagcttcctcctagcgctgggcgtggcggccgaacgcagcgagggtgatctcgtggcgctggaggtcgaagggatcaaggaaggcgtgcgccaagcctcgcagagccgcatgcgcgaactgggcgaagactatcggtggatcgacgcggtgtttcggccgctgcgcgacatgcaggttccgatcgatcgccgggatgttatgagtcgctggaaggctggcaaggtcattgccgcgatcaccaaggagatgaaggccgacaccaccggccgatatctcccgccgccgaggatcgcctctcaaaccgatgatgcggccacgcatgcggccctgatcgacacgctcgatcatctgggcatcattgaggtgatcggggatgggcgcctgaacatgcctgaccttttccggctcgccgcgggcgtcaagcggatgggcggcgtcaagctccgtccctagccggggatggcagatgctcctcgagaacttcagtccttaggagacgcccttgtaaaaagcccgcgcgctagcgcttctgtgaccttgcgtaccgctcctgtcccttggcgttctggaccttctaatcgccaactcaggcttgtggtcgcggttagccacgccttgatcaaaaggggcaacgcttccttggctttggtggtgaacgcttccaaggagcgcggtacgttctggaagcagcccttccaaacttctgagaagagtcaacctcgactattcggcggtccctaagcccaagggctcaacctgactcaaaggcgaactttggaagctctgctttcgggcagcctctggcggatgcgggcccgcgacaccccgggcgcgattgccatcagatatagaatcggaatggcaatggagcggtgacatctgtcggcccggctgtgagtatctcacccgtcaggtcggcaaaacgcagcgtgaccggcaagccatctgcgaaactggcgttgttgaagttcagcttggtcagcgccattaggtcggtgagcacctggcggatgtccgcctcaccctggacgatgtccaccgtgatggggttcggcacctcccggccgggataggtgttaagccgaggcgtgaagccggtcgtccagagataggcgcgacgatccgaaacgaggatggcggtccccctcaacaccggccgactgccgtagcgaaacagcttcagttcattctggcggcggatgcgaatgccgatcagtttggtctccggcggcacggtcgatcggaaaccttcccattccgccgtctcgaaccaggtcttgccgtgaatgaacagttcggatggcgggcggccgtgaatctcggtgtaggaggcaatcaccatccccatcagttccgcggccttttcgcggctcaggtggaaactgtggtcggtggatgaaaaccagggcccgacggcacccttgaaaaccacgccttcgccggaatccaaaaacatctgggccccgcaacaggcgttgtcgcggcccttggcgttttcgatgtgcttgaagaccagcccgacgtagcagacgccctcgcggacctccgcgacccgccaagggcgaccacccgccttgtagaagctggtcgtcgcgaggttccaagccaccgacgccggatcctgcagcgacctgcgggctccttcctcgaactcggaaggcgtcaaggtcgtttcccgaaccacttgcaggacctggcccgtgtcgagcaggcgagccttcagctgattgtgaaagttgagctcatattcatagagcgcggcggcctccatctcttcgacgaagagcgagccccccgacaggatggatttcgcggctcgacgaccgatcgtccctgacgtcttctcccgctgatcccgaggcacgatggatttcggccgaccgaagcgatgcacttcttcggggatgaccacgaaccagaactgcggtcggccttcctgttcacgcagatacttccgcaaggcatcgccatagacatcgaccgctcggaagattccgtcatgccgatcctcgctgcggatgcggcggctcagaaggtcgccgtcgatcgtgatcttggcgaagggcgtcgcgggccagggcacgccgaacgccgcctgaaatcccggccacattgtcttgttctcttcgcggccgccttccggagccgcgatcgtcgtggctaaggccttcacccaggtttcataccgcctgatcccctcagcagttccgatcacgcccacatccatgcgggcgggattttgattggacgctggcgggccgaacaggaacaggccgtccttaggatgctctgtcttctgattgaagccgaagctgagcagcggttcgtcgatgtgggtcagcgtccattcgctcattcctcgccctccgcatcggcgtcgaaggcaccatcgttgtcatcgtcctcaggttcgtccggatcttcggcgtcgtcctggaactgcagatctccaacgatttgtctctgggctgtcagctgaagcagtcggccggcgagggtaagtctctgatcgccatcgagcgggatgacacagtccgcctgtccgtccgccagccacgcggcgaaggcctcttgcagctggcgccaatgctggttccaccagttcttgcagaagcgcctgcgtatcggcgtggtccgcttcggatctgtgatcgcgacctgtccgtcgtcggagaaagcgacatagggtttgaatctgatgaacgccggcggtccgaggacgacggtgaccttcatcgccagatgccaatagacacggttccgctcgctacggcccactaccttcttgtaggtccgctttccggacgctgccgtatagatcaccttgttgctggccaggagatcggcgggaaaatagaaggccgacccagaacgttgctcaagaggtttgaggccccggttcagcagatgccgctccacatgctgccggagcagagccgtcgcgatattctgggcgtcacctcgcttagggctggtaacgtcggctgagggtcccttcagaaaatgctgcaacggacgttcggcgcggagctcggcgacaaacggcgtcggcagggccgcgttcacctcatcgaggtcggcgaaggtcagaagcagctgatagaagactgaaaagggtatgccgctcgtgcgcaatgactgggcgacgacggcagcgtctgcgttgaccttgaggtagcgcaggttgaccggcagggcgttgatgggagacaggctggtgagcaccggctccggctcggcgttgactaaggctgcggtctttgccgcgtccaggcgccagcgttcgaactcggcggtctggtcgtgctcgaggcgcggcacgttggcggtttcgagcgtgtcgagcagctcaacgagtttgggcccccagcccttactgaaatcgatggcgttgagctgatgcacgaggatcggaaagtcggcgaagccgacgtcgtcgatcctgaccgggatgatgaaggcggggtccgccagcgccttccgcacggcgtcggccaccgacagttcgtttcttaccccttggcgttgaggatcgacgctcgctttggaggcgacgaagatgaccttacaggcatgctcccgaagtgcatcctcgatcgtactccagaagggcgttccaccctttaagccgaacatatcggcccacaccttgtagccgtggcctgtgagcctcgcgccgagccaccggacgaaatcgttatcgtccggagtagcgtggcagatgaagatggtgtcccgagacatgtcgctgccgaatcagttcaacccagtctagtccggttcggaccgcgaaccgccagttgagttcacagcctccgccagacctcgcgcccgtctcctcacctcaatgtccgctctccggcatgcgctcaaggtccgcaactggcgccaaggcgacccaagagtctccgaccccgaacggccggggcagcggtttgattatgccgctcgtatattcctgtcagcaccgcccttccgtggtgcagcgcctgctttttcggctagactcgcctgatgcggtcagacctcgatcatcttccggagcgtcagcagcgcgaacttgaacgcgtgcgcgacatcctgctggccggcttcgaggccgcgaagaacggcgggggcggcggcacctcgacttggcgacgcggcgggatggtcctgaagatcatcctcttcggatcgtacgcccggaccgactgggttgatgagcccgagaacggctacctctcagacttcgacctgctgatcgtcgtcaacaatgagaagctgaccaacatcgccgactactggtggaactcggaggatcagatcctccgtgaccccgccatcggccgcaccgtcaacctcattgtccacgacgtccacgaggtgaacgacgcgcttcggcgaggcgagtacttctggaccgacatcgttcgcgacggcatcgctctctacgagatgccaggacatccattcgcgaccttccagccgatgaccccggcggatgctgtcgcagccgcagagcgccatcaacgtcattgggctaaacagattgatgatctgctcaagggcgctgacttctacgcctcgcaaggcaatcggaagctggctgcgttcagcctacatcaagctgtcgaggcgtcttacgcctgcttcctgctggtccacaccttctatttcccgcgctctcacaacatcaagttcctccgctctctagcggaagacgtgaatacgcgcctgaccgaggcgtggccgcgcgagcagcgcttcgatcgccgccgcttcgaactcctgaaacgcgcctacgtcgaagcccgctacagcgaccagtacgacgcgtcggccgatgatctcgactggctgatggcccgcgcccgcaccctgcgcggcctcgtcgccggcctctgccaggagcacatagccgaactcagatccaaggctgagatcgtctgatccgtggtgtccggttccttactcgatcacgttcgcgcgagactaccgaggcagtgcgaacaggctgaaaccgggcgaactctcctgaaaccgacctgcgcgagctggctactgagccgccttggagactggcttgaccgggagtggataatcgctgcccgatgaactccttagatgggagttctcgcgatgaccggcctttaccttggagatgctgaagacgtcctgcttacccggaaggaggcgtccaccgagttgctgcggatgggcatccgccgttcgccggccaccttggcgaagatcttctgcactcgctcggatggaccaccctgcgtgcatctcggccgcacgccctactacccccgccaccggctgcatgactgggcaagaagccagctgaccgccccgcgttcatcctccagcgaaccgcgccgttccggccactggaagtctcccctcccggccgacgacgcacacgcctgatccgctgcggggcgtgtgcggctcagaggctgcgcccagacgcgcctcgccctgctctgggaatgatctgcgccacgcctcgggcgtccacacccagcgtcgcctgcgcccccaccgacggcagggccgtcccggccgccaagcggacatagtggtctgcgccctgggcatcccgcaccatcacgaagggcgacccgcccagttcgtcgtggaagcccacccgggtcacctgaccggtcaccctcccctcgcggacgacatcggcggtcctgccgcttcccagccggtgctggttgagcgtccggatcacatccttggacatctgcagccgccgcaggcgcgcctccaggtcgtccgccagcttgaattgacgtccctgccgctcagctaggccaagcgcctccagatgcgccagacgtccgcgcgtaagggccgcccaggcgcttcgaccgccgacggcatcctccaccctgccgtcagcatccatcccggccagtaaccgtctatcgaagccggtgaagccgtccctctgggtctcgcgccagatgcgccgctcggcgtcgatccgcgacaggtcgcccagtcgctcctgcgccgcctcctgcgcccgcgcccggaagccataggccacatagttccgggggatcaccaggtcccggccgttcgcccgccgccccggcatcaggatgtgggcgtgcggctggtcggtgtcgtagtggcagaccgccatccacagcaggttcggctcgcccaggtccgcgcagacccggcgcatcacgtcgcgggtgtagtcgcgcagctcggcgatgcggtcgccatgctcgggcgagacgatgaagcggaagtggtggcgatgctcggcccagtctccgatccgctcggccccattcaccgcatcggcctcccggtcgaagaaggtccccgcctccccttcgcggccggcgccgtcgcggccgagatagcggacgtgggccgccagggccttacctcgagccattccattgccggcgtggcgcgagaccagcgccttgacgatcacccgctggcgtacatccaggcggaaggcgctcccggaccgcttggccgccgttctgagcgcgccggccctggcgccgtagttgaagcgcagggtcgaggagagccgcttgaggattgcggtgtggacggaggcgtcccgcttcaggctcgtggccagcctgacctggaccccctcgtcggcaggtgcggacagagcggccatgcggagatcgagatcgctgcggacggacatgacggcgtcttcttgaagacccgaaccgctccccaaccgccctaagtcgtcgcaagtcgccgggccggtcgggagcgcttgctaagggctgagaacaaagacaaaaagcgaagcgacgccgtcttcttttatcttgccctgcctccctgtctctaagcggctgatggctgctggtttctcctgattaccaggcgcacgcttcgcgcttcaacgatcccggcgcttccggttcagcgccgggtcagcagcagccgaagctggctccccgcttcggtcttcacttccgccgtttccgccacgctcagcccccaggctctccctggggctgagctcttcaggactccggcttcgctgtccgacccagcgatcgtcatggctcagggatgacaaaggaaaacccgcccggccgaagccgagcgggttgctcatcccaggtccggttgttcaggccgcccgcgccttgatagacacatgccgcagcccgacctccgcagccttctgtccgaggttgagcgcgggtccgaatgggcgctgttccgtccggccgcgatccagtgaatgcaccagggtgaggcagcagaccggttcgagcgcgatcagttcgtcgttcgcccggaagggagccgctttgccgtgggcctcgaagtccgcgcgcgccaggatcagcttcacccccttctgctgggcccatttgatcgccagcttctccgaacccttcgccccggtcgtcgccagggccatgtccggccattcctgccgggcccagttcagggcgtcgaagattcggccggcgtcatcggcgctgtcggccccgggcgcgccccggaaggcgatcaccggaccgcccggatccgcctccccggctttccgcgcccggatcgcccggatcgcctgtttcgcctcaagctgcgccgctgtcagaagcgtgccccgccggcttccgcgccacgcggtccagacctcgccggtggcgaccgtccaggtgtcggacgccgcgtcccggatccgttcgcaagccagggtcgccgcgtcgccggcgcgggccctggctatcgcctgctgcagctctacatccgccgcctccgacccgtcgaagtcgcgatccaggctgcgcatcgtgtcacgagcgcggtccgcgtcccgctcgatcctcccggccgccgaatgaaaggcgccgatcagagcctcgcccaggatcgtctggtagtcctccagcgccgtgtcggagatcacatcgaccagttccgtcatgagcgcgcgcccgagctgcaccagggcctcctcgctcggatgcgggcgcggatcgcccagggatgcggacaggtcatcgaaagcagagtcggacttctcggcgcaggcggaggcggtgttgaaggggatcatctgatcattccttgaataaagaaacgccgtgcgccccatgcgcaacgaccccggttttggccacgtcggggtccccggacgtcaccggagcgggtcgccctcgcggcccgcacaggggaacggcgcagccgttgacgtccggggtgacgtgacaagatcggagggcgttgtgtgggggcaggtcgtcgtcgcctcttgcgacgacgacacccctcggcgccgtcgcgccgatgcggaggcggatgcggcgactgtcctccccgtcggcgtcggcgcgccgacgacgccccatcgatcctggcggcgccttgggtgcggatggggaaagacgctatcggagtttggaaatccccgcccaagaagaagcccgcggcgccgagccgctcggagcctctccgggccactccgagccgcaatgatgacgtgtcccatcgggtccgtggtcgcgtcagacgccgcgagggcggttgttcgccgccggccgttggatctggccgagcgcccctcttgggaccgccgctcgagcggctctgcgacaggtccgccgctgccttcatcgtagctagcgccgtccgagcctgcggctgatcgggttgcccgccgaatgcgaaacggcggcctcatggaggccgccgtcacaggtcgaggcttatggatcatgtcggggggcgtttattcgagctgcgccaaccgctccagatgccgcaccgtctccggcgcaggcgtataggctctggccgcatgcggttcacagaaggcgccgcgcgcgatcggccgcccgcagaggctgaagtcagaggccttgggatcgcccaagggccagcggcattggcgccggccaaccgacagcacgctcgcgagcccttgctccggcgccggcttcgccggctcggaaggcaggggcggcgccgccggagccgccggcgccgacggcgctcgccgcttctttgacggcgcctgcgcgccatgcggccggacatttcgctgaaccggcgcgcggccggtcgacaggcccaggcgatgcagcttgccgagcacggcgctgcgggtgatcccgttcgccagttcgcgcgcgatctgttcagcgctccagccgtccagccagagtgtcttgagacgacccacacggtcttgggtccaggcggaggcggtcatggggggctcccgatgcaacaagcccgatcggctcgcccgtccgttcccttccttcgtccttttcagcacgcgaacggcccgacgctcgcgcaccgggccgcacctcgccgcacctcgccgcggagggagggggtcagaagggaatgtcgtcgttcagatcggcgccgccgtcaggctcgcgcactgtgctggcggaagccccgcgccggccctgatccgaggggtcccggcggttcttcaggcggatctcggagacgaccagacgaaggtcgtagtgttcgacgccgtccctgcccgtccaggtgtcgttctcgacatggccctggatcaccacccggctgcccttccttgcgaagggctcgatatacttctcggccgtggcctcattgaagcagatgcagttgaagccggtggttcgttcgccgggcgtgccgtcggcgcgccggaaccgggtggtctccagtacgcggaagctggcgcgcttccggccggtcccctgcgccgacaggatggaggggtcggccgcgagatagccttccagagcgaaggtttgcatgttcggtgtccttgaagatgtgaagatcaggatgtcaggcggcggcgcggtccgacgccgtgtcggcgtcccggtccccggcccaatccagaacggtcagccgctcgatcaccagctccttggccgtgcgttcggtcccgtccctggccgcataggccgtgtcgatgaagccgccgatcaccagcgcctcgcagccctgggccagaccccgaccgatgaccttttcgttcagccccctggaccagctgacgcagttgacgccgacgacccggtccttgcccgcatcgtcgacgcctcggttctccagcagccggaacaccgccttggcgaagtccgggctgatctgggggtcggccgcaaggcggcccgtgaacaccatggtctgcatatccagtctcctgttgatccgaagccgtacgaggagccgatctcctccatcccgcttcgccccgaaccctccctgcccttctcctcctcccgcgttcgggccctccagcgctggccggcgagccgatgcccgcgcttcgggcgaacacccgctgacccccagctctcgccgcatccccgcgccggcgagccgccggtcgtccggcttcgccctgaagggcttgagcctcgcgaacgagccggaggcgcatgccggcgaccctgccaaaagcgcccgctctctctggagccccccccgatggacgacgcctgggtcagccggatccaggtgcttccgacaccggcgtgtgggcggctgtgttcaggcggccgccgcgtccagcatcgtcaccaccggatggcggcgcagcacggcttccaccacctccggccgatccacgggcacgaacacacggggcgtgaaggcgatgatctccacaaagcagccgagcgcgacaagcgcgtcgcggtccgttcgcccgcccacgacctcgatccgccagcgatccatcacgcgcgcccgcttcagccacaggccgccttcaagggagagctggacgccgcgctccagcaggctcgccgccgttcgtgcgccgtcggtccacgcctcgccggccggggtcaggcccagacccgccttcaggcctccggcctggaccgggtccagcacccggcctagccagcgccgcccatccggcgcgcgaaccctgcggaccgagcagccccgcgccggcagccgtccccagatgggcagcagcaacccggtggcgagcgtcagttcgcgggttcgccagggatccagcgccgcgacctcgctgtcccagatccgtcgccagtcggctatggcgaccgccttccaggccgactcctcgaacacggtctccggcagggtctggcggctgtccgggcggaccagccggaccgcggcgaccagccgatcctggtcggtggcggtggtcagccccagctcagcgatcgcggcccgccccgacttctcattcagaaccagccggtgggcgacgccggccgcccaggccaacgcggcctccgagatcaggatgtcgcgccggaccctgagcgagaaggtcaccaaggccgtctcggcgccggtggagacgtcggtccggatcgtctcctgatccagaacctcaagcgcttcggcgtctatgtcttccagcccgcggtccagctcgcccgaagcggcggcgcgctccagaatcccggagaggatggcgtcgaacgcgctgaacagggcgttctggtcgtcgatgcgcagcgccagcagccggttcaggaaggtgtggatcggcggcagggcgtcggacggcttcaacccgccgtcggcgtcgagcagcctgagcccagtcttctcggcgaaggcctccagcgtcatggacgccagctccccgaaggccagcgcgccatagaaaaccaaaagggcgcgccgcgcccaggggctttccagattgtcctcggcccggaaaaggccggcccccgccgtgcggcgctcgccgcgcgtcagagcgccgagtgaatccagccgccgcgcgatcgtcgaggtgaagcgcttttcgccctggatgtcggtgatgaccgggcggaacagcggcgccgaggcctggtgcgtccggtgactgcggccaagaccctggatcgcggcgtccgcccgccagcccggctcgaccagatagtggacgcggcgctggcggttcgcggccgagagatcggcatggtagctgcgccccgtgccgcccgcgtcgggaaagaccagcacccgcttttcgccgcgcatgaaggcgtcggtctcggcgcggaccgcagcggcgccgcgccgctccacgcaccgccgcccctcccgcaccacgacccggcgcgcccgaccggtgatctcggccacactgtccgtccccaaggcctccagcagcgcatccagcacgccgggcacggcgggcaggcaggccatcttgaccagcagggcctcacggcgggcgagcgcctcctgactgacggcggggcgcccattgtccatcaccgggaccatggcgacggcgccgtccccgtcctcgacggcctccatcaggtgaaccgggaacgcctcccgaagatagtcgaggacatattccctcggcgtcaagtcgatcgagagattgttccattcctccggcgggaccgaggcgagccgccgctccatcaccgcctcattggtcgagacgatctggaccacggacgagcgcccacaggcgaggtcctcccggatggcggcgatcaggctgggcgccttcagccccgccagcagatggccaaagaagcgcaacttggcgccttcaaaggccgaatgaaccacagaggccgcaagcgggctcctgggcgcgcccgcttcgtcgctcaggccggtcgccttcagcgcctcggcgagattggcgtggatcagctgaaaggcgtcggcccactggtcccagatggcggcgtcgtctgcgctgagaggatgaaggaggggcgcgtactccacgccttcgaacgataggctgcgcgccatataaaggccgagcgccttgagctcgcgcgccaccagctccatggccgcgaccccgccgcgatccatggcgtccaggaagtccgcgcgcgacatgaagggcgcctccggcccgccccacaggccgagccgggcggcataggccagattttccgccgtggtggcgcccgtcgccgagacatacagcacccgggcgtccggcagccggttctgcagggcgaggccggccatgccctgctgagaggccttcccgggtccccgcgcgccctttccgcctccggcggcgttggccatggcgtgcgcctcgtcaaaggcgatcaccccgtcgaagtcggagccgagccagccgacgatctggtcgagccgggactggcggccgccacgcgccggctgtcgcagggtcgcataggtggtgaacagcacgccgcgatcgaggcggatggcgtcgccctgtttccagctcgccagcggcaggatgtcgtgggcgtcgccgccgagggctgaccagtcgcggcgcgcatcctcgagcagggcgtcgttgcgcgatatccagagcgcccgaagccggccctgggccatgttgtcggcgatcacggcggcgatctgacggccctttccgcatccggtgccgtcgccgagaaagaagccgcggcgcagctgaacggcgtcctcgccggcgtcgggggcgaggatgagctggtgggccgcctcatccgcgcgccaccatcccggaagacgcccgccgtgggcctcgccggcatagatcaccgtctccaactgggcatcggacagtcggccctccgcccggatcgaaggcggcagcatgggccggtagttcggcgccggcggcggcaccgaggccatgggaccggactcgaccagaggcgacggatgggggcggggttcgggaaggatgatccgcgccagcgcatgcgcctggtagaggccgacgtcgcggccttctccgctccacgccctggtctcataggtcacaggcgcggcgcttgagaggaaggccagccgccccgatggaagagcgaggtttcgatcctgcgggccgataagggcgccgggcgtgaggtgaaggcgctggcggggcctggcgctggagcgcgccggccagccgccgatcagacggcaggcgtcggcgagatcgccggcctcaagcaccgccgcgggctcggcggcggcgccccggtccacgaccagcaggccggtggcgaccgatgtgccgtgcttggcgaaggcgcccggcggaaaggcgaggcggccgatgatcctgccgtatccccgaaggcggcccagaacggcctcatccgtcagagcggccaccggcgtgatggccgccaggcggccgccgtcggccagcgccttgaggctcgccgccagatggtcggcgaggtccgaaaacggcggattgctgacgaccacctcatagccgccggcgccggcgtcgaggtcgtggatgtgccgggcgtcatggcgagacaccggcgtcgaggggaacaggccttgcagcagcccggcccgccccgaggccttctcattgagcgccagcacgccgccgcaggcctcggcgacggcggccaggaggccggttccggccgagggttccaggacgcggtcgccgggccgaacctgggcggccaggaccaccagcgccgccagctgcggcggggtcgagaactggtcaaacgccacctgttcctcgcttcggcgggtctgggtgaggcctagcgccgacacgttctccagcagggcgcagatttcagaaggcgcgtcctccaagcgcgcgacctgggccgaaagccgccggacctgcaggaccgtcgccgcctcgatcgcatcataggcgtcgcgccagagccaggctccctcggcgtcggagccgccaaaggccgtggtcatgaccctggccgccagcttgcgatcgagcgtgcgggcgcgggccagatgcgcagccagggcgcgggcggcggcgagcacatcggccgccctgtccgaagacgcggcgccggagaacaggggaaggctgtgggtcggggacatcggcgaggttccggtcgcctggagcggagggcgcatccctcccgatcctccaggctcgccttgccccgaccttcctctcctctcctctcctggcctcgcttctcttggcctcacctcgcgtcgcggcgccttggttcgccccggcgcagacacgacggcgtcgccctgacggatgccggggcgacgccggagatgccatggcgctaagcggcggcccgcccgatgaccgcctcgccttccggcgtgaccgtgaacgcgcccgttccatcatcgcgctccgtccgggcggcgggagccgtgacgccgtcgccggcgtgcggatccccgtcgtcctcgtcgccgattcgggccgccccctccccgacttggccgctcccgtccgagcggtcatcggccgggccgtcctcgtccgggttgttcccggcggggccgccggcgtcggggctgaccgttcccggcgaagggccccacgacagaaccggcggcgcccaaccgcgggcggcggcctgttccgccacccagtccaccagcgcggtcttcttcagcgtcttcgcacggtcgtcctccgcgcccatggcctccagcatggccagcagcagcgccttggagtgcggctgcaggaacggcgcgtccggcgtccagtgcaggctgatatcggcgccgcacaacccggcgatctcggccgcctcggcccgggcgctgcggcggatttgcacagtcttctcctcccgcaggtccaggctgatggcggtcatctcggcgagcaggctcatcttctcaccatgcgacaggccctcgatccatccgatcaccgtatcgcccgaggcctgccaggctgacctgcggccgtcgaggcgctggcgcacctcgccgtccagcgcctcgatgatccgtccgcctgctgggttgaagcctgccgcgacgatggaaagagcggagtccgagcgggcaacctgcgtgcgtcgaaccaggacgttgaacaggcgcgcgatcagggcgaccagggcggcggacggatcgtccgccagggcccggatcaagccccgcgttgccgcgtccgtgcgcactgcgtgcagcgcgtgattgagcccttccgtttcgggctcgggcgtccgcgcctcgggcggcgcataggcctgagccccgtcgccgctcgatgattcctcggcctcgacgacgacgacgtcggtcgtgatgctctgcgacagcctggctgcgtagcaacggacatcgacgcccgtgccgggcgccggccacagcaccagcgtcgtcacctggcgttcgccccagcccgcctggtccatggcgatgcgggcgtggatcatgtccacgatcgccagatcgacgaggtcgggcccgtcgccgcgctccagcgccgaccggaccctctccgccgtgtcgttgaaccgctcgcgctgctcgcggtagcgcgccatcgcttccgacgacagctggccgccgtagacataacccagcgcttccagctcgtcggggaggtccggctccggccccgcggtgacatgcaccgccatcccctcggcctcgaacacggccgcgacgccccggacccgctcggtccagagccgggtcagcacctcgggatcgagcaggaccggcgccagctcgccaaacagatcggtctcggtgcgccctccggcggcgccgtaggcttcggcgtccaccaggatgcaacggcgatcgcgggaggtcacccgtccgtcgtcaagccgctcgaggatgcgccagtcctgaaagccgcacccgtcccgcgccgcttccgccagcgcctcgcgctccgcccgatctggaagccggacgaggagtttggcctgtttcagggtcaggcggccggccttcatggcggccagcgcggcctgcggcaggtcggccagggccgccagccgcttcacctcgatctcggcatagccgagcgccttggcgatcgcgcccacggtcagcttcgacttcagcatccgaccgaccgccgcgatgatgtcggcgacgtgaacgggcgcggcggtgttcgtcagcaggaccgccgcggcctggcgctcaggctcggtctcgacaaagacctggaccgggtgatcctcgctgatctcgccgccttccagcagcagggtcagggcgaggcggcgacggcggccgtcgagcgccatccagggctgttccctgcgacggcgtccgggccggacggtcaggggctgcagctggcctgcggcgcgcagggtggcggcgagtagggggatgtcgtcgtccggcggctcgtcgaagcgcaggttctcacgggcgacgccgatgtcgcggaggcggaccgttcggatgtcgcgctcgatgacgcgggccggagaggggacgaaaacaggatcggtcatgaaaggtagtctcccgccggtcgacagggctcatccccgacgctccggcgcccctcagcccccttgctttcccctttgcagcgccgcctcgacctcgacctcgttccagtcgccgaacggcgccgccggccagaccacgaccccgtcgactcccatcctcagcagccgccgatgcaggcggtctgcggcgtcttggcccacctcgccgcggtcggcggcgatcaggacctgtcggacgccgggcggcggcgtccaggccgcgagattgtgcgcggccatcagcgcccacccgggcagccggaaccgctgcatcgccgacagggtggtgaccactccctcccccaccagcatcgcctcggcggcccgggcgagccgcaccgccgcgccgggcgggaccaggccgaccgtcttgcgcctgagcgcaagcccgctcgccagccggccgctggcgtcgagataggtcagctcgatcgccgtgagctggtcggcggagtcgctgacgcgcgccatcaaggcggggcaagcccgccccgcgcgcctgtagaccgagacgggcgcggttggatggtgaagcagattgagcgcctgtgcgccggcctccacggcacggcggcgaagatgccgcgccgagggcgtggcgtcatgaagcgtcacgccgccgcgccagagttcggccgccgtctccaggcgaacccgccgatcgggccggggcgcggacggcccggccgagccccggcccgtcagccgcccggcgtcgtcgatgaagccgcgcctgcgcagatcgtcgcgtaccgcgcgccaatccgcgccgccgaagccgtggatgatcacccggccctctgccagcatcagcgagacggaacgatcggcggcgctgtgtccgggggccggcacattggcgcgacagcctccggcgtaaagttcgccgcccagagcggccacgagagggtgcaaggtcatggcggcctcacatcagtcccagggttcgaaagctggcgacgccctcgcgtcccaccaccaggtggtcgtgaacctgcagtccgaacaccgtggccgcgtcgacgatctggcgggtcaagacgatgtcggcctgggagggcgtcggatcgccggatggatggttgtgcaccaggatcagagccgaggccgaaatctcaagcgcgcgacgtataacctcgcgcgggtagacaggggcatgatcgactgtcccgtcggcgaccagctcgtcgcgcatcaggatgttgcgccggtcgagatacagggcgcggaactgctcccgaggcagatgcgcgatggcggctcgggcataggccgagagcgccgaccatgacgacagcacgggacgcatgcaggctgcgtcgcgggtgatccggacgctgagctcgcgcaggagcttcagctcgagaatggcggccggatccagcggaccggcccgagccagttccgctgcgtccgccgcgacaatgtccgccaggctgccaaaacgctccatcagcgcctcgaccatagccgcctgccccgcggtggcacagcggcgttccagcagaaggcgcagcacggctcgatcgtcgagacgcgtcagggtggagggatcggtctcgaggtcagagcgatcgcgagggggcgaagagcgcgcgaccgcacgggtcagggtcaaggtcgtggtcatggcggtgtcctggtgtcagctccccatcggagcgccaccggccgcccttcccttcttctttcgctggatgtgcgttcctggacgccgggctgagcgagcagagcctgtcggctggggaggccacgtcctcaggctgtctgaacggccgcgacttccttgcttgtcgccgcgatacatgccgggaatggtttcgcgcctcgctggcgccggcgtccgacccgggcgtcaggccttacacaccatcgatggcgaagagggcatgggcttagtgacactgcgtccggaaggcccagccgcgccgctgcggccagccggttcagggctgtgtcggcgcgtaagcccgcgctgccccgttctccgccactcagcctcatctgcaagccagaactcagggccgccggtgagcctttgcagcgacttggggttgcattgtcttgccaacggccatcagccggcgctcataggcccgctcgcggctcgccggcggcgatgtcgatccaggctgccgaagccagccgctcaaaacagcgccatgatccagcccgccaagccaaccagcccggccaggctccagacccgcagcgcgcgctcgctcttgagacggcggctgcgaccggcgaatacggttgacacggcgccctcctgaacagcccccggccacggcatagcgcgcccaccatggttagcgagagcttaacgcggcgccgcgctgcacttcatccggactctgtagcgccggaacagccagcggccctcacgcccagcttcgaatcatctccaggcaaacgcctgcgctgcctctctgaagaggatttggagcgagcctcctccgatcgggtacctcaagctggaagcctctatgcgcaccgtcctcccacgacccctcatcgttgggtcaggggacgggtcgcgtccattcctgggttcaactgctggagcggcttgccgtgtcgtcaacggcatcttgcggcggcagcccagggcctctgctgagttcaggccctaccctcggccgcgcgcgccatctgtgcctgttcgagcagttgacgacccagcgcctcggccgcgtccagcgtcatgaccagctgtttcgcggacaggtccatctcgccgctcagttgctcctgcacctcggcgtactcaaggcgcagcgccaaggcctcgccctctgcgacggcgatctcgacgccgcggagaacaaccagcgtcagttcgccgttgtcgcgtctttcccagtccatcaggcgtgctccggcatcagcgggtgaacgaacgcaccaggttcaggatcgcgccccgctggtcttctgtcagcgtggaccaacgggccagcagcgtgcgggcgcccgggagatcggtggcgaaggtctcgcccatcagctccgacgcggtcgcgtccaggaccacagcgatccgcgcgagcgacgcggctgagatgcggttggcgccgcgctcatacttctggatctgctgaaaagtgacgccgatggcggcgcccaactgcgtctgcgtcagaccctgcgccgcgcggcgcacgttgacggcggcccccagccgggcatcgaagtcaccagtcatcgggggaccgtcaccgatgccagttaccgggtcaagccgagcgacatgcgaccggggtcgagcgggcgtgtggtcgcgtcaggcttgtatcatgtcaggcagcggataagcttctctcggctgttcagggggaagccatggatcaagccacaacagcctacatggccaacgcggctggtcagcttgcctccatcagcgcttttctgggcggcttcgctgcgacaatcctcgcgaccctgatcctgagcgatccgcgctcaaggatgggcggtctcgtcatcggggcgtccgcggcggcggcggtcagcttcgtggtgtgcgcgcttgccgcaaccacgctcggcgccggcctcaacccgaacgtcccgtccggcttcttcgcggaggcttatctcctgcgagcgcaagtggtcatgacgctggccttcatgagcggcatctgcgccttgctgctcgccatcggcgccagcggctggctccggtcgcgccgcatggggtggacaacaagcgccttcgccctgctgggctttgcggccgcagtcttcctgacggttcaggtcggcgcctaggtccgggcaagcgcctccgctgaagtcagaagggcgccgtccggcaaccgccgttgcagcgccttcgcctcatgccagggcgcggacatccacgcctcacactcttccggctgcgtcaggatgaccggcatggccttgggatggacggcgccgacctccgcgttcggttcggtcgtcaggaaggagaacagatcgcacgtttccacgcctgtcttgatcttgcgcacgccggtccacgctggcgccgtgatgccggcgaagaaggccagcggctcggcgcccggcaggctgaaccagatcggccgggacttgccggcggcgtcacggcccggctcgctgaaggcggtgaagggcacgagacagcggctgcccggtcccaggtgcggcttccagtgactgctgatcgtgttgcggacattggtcacgccgctgtccggctccatgctgaggagggcctggaaatcgacctcccggcccctggcgcgcagcttgtccgcacgctttgaagccgcatccatcagcaccttgcgcgacgtcggcatgccccagcgcgccagaacgacttcgcgcacgccgtcagcgccggtgcggacgataggcgcggcgtagtcggggtagatgtcgccaggctgcaggttgccgacgtccgagcgcatggcgcgcgccagatccatgatggcctgtgggccgctgcgctggcggtagaggttgcacactcggcgacgctggcacagggaatcgggtttgtggagtcgccgaagcggacgtgctgaacgtcggctggggtaaccagcggaatgcaacccctccagcccgagagcaccagtagcggagcagatgttcttcgcctgtgatcgacagatcaatcctgttgacaacgattagacgattagctaatagtcatatcatgagttcggtcttcaaagccctttcggatcccacgcgtcgccgcgtcctgcagatgctgcgtgcaggcccgctgagcgccggtgcgatcagcgatcagttcgacgtgtccaagccgaccatgtcggcgcacttcgcggttctgaaagaggctgaccttgttcacacggaaaaatccggcaaggccgtgatctatcatctgaagctctcggtgctggaagacgcgctgctgggcttcgtcaactctttcgagccgagcgtcgggactccggccgccaaggacacagcgaaatgaacaaggacctgatcaagagcttggtggtggccggagggctgatcgccgtggcgctcgccgccacctcagcccgatcgatggggctcctcgacggcgatgccgtaacccgcgtggtcatgggagccaccgggctgatgctcgtctggtatggcaacagaatgcccaagaccttcgtgccggcggcgaaggcgcgccaggtccagcgcgtcggaggctggtccatggttctgagcggcttgatctacgccgcgctctgggctttcgcaccgcttgacctcgccttcacggccggttgcgcgacggtggttgctggcgtggtcgtgaccgtcggctactgcctgtcgcttcgacgcaaggcggtcgcctgaagcgccgagcaggtccgacaactcgtcgccagccggtgaccgcaggacttcccgcctgatcgcgactgcgatcgactgacctacctttccccttcctcgatcccacgcgcggagcggtccgcgtgatcaatccctcatgcccggagaccatccatgaaccgaccaaccttcctccgccgagccgttatcggcgcgacgctcgcattgagcgttctcctgtcgagcgaggcggtcgcccatacgccgtcatcgccccgcccggcgctgtgggtgctgagtgacgcggactcgaccctctaccttttcggcacgatccacttcatgcgaccggacacggattggcggaccgacgaagtggcggcggcgctggcggcgtcccagtcgcttgtgctggaggttgccgatcccgaagaacaggcggcggtcgttccactgatccagcaatacggcagatcgtccgagagacccctttccaccctgctgagccctgatgagtttcggcgcttggacgccgcggcaagaactctcggcgcgtcggggactcagatggacaccctgcgcccctggctcgccggcgtgatgctgtcggccgccattccggcgcggggcgggttcgatgcggcttccggcgtggacgtccttctccgcgccgacgccaagcgtgcggggttgccactcaaggggctggagacgcccgaggatcagatccgtatgctctcgggcttccctgaagacggccagctcgcattcctgcgcaacactctcgacacgttcgcccaggcgcccaccgaactggcgcaactggcggacgcctggggccggggcgatgtcgacaggatcgccgacgttacgctcgacccgatgaagatgcgcagtccggcggtctaccaaaccgtgatcgtcgagaggaaccgtcgctgggcaagtcagatcgcccagatgcttgaaggctcaggcacgacctttgtcgcggtgggcgcgctgcatctcgccggagacgacagcgttcagcacttcctacgccaggacggcttcgagacggttcgcattcagtgagatcggaatgagggccgtaagcacggccctcgtcagtcgttgcgttccgatgatgtcacctctcagcgccccgtctgcacggtgtcacaaagaggagttcgcgatcggtagaaagcggacatcagtccgtgccgctggccctcacagccgatcgctgctggcgtctcgctgaacaaaggcgggatcgtcgcatttgaaccgcatggctcctccaaccgatccttccgtcctcgtcgttgacgatgacgcaatcatccgcctcgacgcttgcgccatcctcaatgatgcaggatttcgctgctatgaggccgcgagcggcgatgaagcgatcgcgatgcttcatcagctcggccaggccctcactctgctcttcaccgatgttgagatgcccggatctacggacggtttcgccctagctcgcttcaccgccgaacaatggcctgagatcgagatcgtggtcgccagcggcaggaggcgacccgatcccggcgacatgccggagaaagccaccttcgtgggcaagcccttcgacgagcatgtcgtgcacagccatctcgcccagacgcttccccaagggaagaagcctgaacctctgaggcagcttctctgaccacccaagcttcacagatcgccgtgtagagccgtggagcattctgagaacgtcgagaccccgggagggcaaccgaggtcagcacgacctgttccaatcaaacccatgcggatcgaacgcggcccggatcctttgcggctggcgggttgccggccaggtagatgaagcgacatcgaagatggagatatccgcacagggggagactccatgcggatatcgaagcgatgcgctaggctctcgaggctgccgcagaaagaccggaatgtgaatcgggctcctcatgacgtgatggtgtggacgacctccgcctgacgggctgttctgggtgtgtcgtcatcagggacgtcatgtgtggacgacctccaagacgcaagagtggaaacgacgttggcgctcggtcgagtgcagtcatgtgttcggcctgttgatgcagctgtttgcgctgctggccctgatgaagtccgcggaccggctccctaatcacgtcaacgcgctcgaggcgctctgaccccctgggtttcaccgatccccggctgcggccggttcgtcatcacgtctcaccactccttcgtctacggcgccggtcctgggtgaagaccggcccgatctctatgccgctgtgggcttgtagtcctcctgtcgcgccatcagggtccaggcgatgcgagccgtcttattggccaaggccacggcggcgaccttcggcttcttgcgttcgaggagattgccgacccagccctcgcgtcctcgctgccgggccattcgcaggaccgccgtggccccgacgaccaggagacgtcgaaggtagctgtcacccatcttgctgatgccgccctggcgttccttgccgccactgctattggcccgcggcgtgagtcccagccaggctgcaaactgccgaccggaacggaagagactcggatctggcgcgctggccgccatggcgctggcagtgatcggcccgatgcctgggatggtcgccagtcgccggctcgtctcatcctgccgatgccaatcgagaatccgacgctccatacggctgatctctgcgccaaggtgttcgagctgttctgccagcccgccaagcgcggcatgcgccagatccggcagggcctgaccctcttcacgcagactcttcagcgctgcccgcaccccagctggaccttgaggcgcgacgatgccgaactccccgaggtggccccgcagtgcgttgatcagcatcgttcgctgacgaaccaggagatcccgggtcttgtgcagcatcaacaccgcctgctgggccttcgacttcacagccacgaaccgcatggtcggccgggtgacagcctcggcaatcgcttcagcgtcggcggcgtcggtcttgccgcgcttcacataggccttcacgtacgccggcggcatgagccgaacatcgtggccgatcgccatcagttcacgcgcccagtggtgggctgaggcgcacgcctcgatcccgatcaggcacggcccaatcgactggaagaaggccagcacctggccgcgccgcagttgccgtctcacgacgaccgtgccgtctgtggctacaccgtgaacctggaaaacagtcttcgccagatcgagcccgacgacagcgatggtctgcatgataccgctcctagacgtgacgtccctgatgacgacacacccagaacagcccgtcaggcggaggtcgtccacaccatcacgtcaccgtcttcagagactaaaaagcagggaaccgccagtctcacaggttcgcacggcacccgcaaaacggcgctgaagctggggatttcgacccctcaataagggcggcgtcgctgtttcgtaacgggcagttggcggagatgatcccccgccggcgttctcaatctcaagcgccaagcccaacaacacgctcacaggacggcacggtcaaacgatgcgaagtgaccccgctcggacggtcatccttcggaaaaggagaggcggtaggcgtggcgctggcctccgccccacgaccaagccagcgctggccttcataaagtccggtgcgggcgacgctctgagccggattgcaggccgcgatccggcaatctccgccgcaggctggcgtcacacaaggggagcgccgccttgcggcaagcctctgccgctgccggtgtttaaggatggtggcggtgctgtcagtctaacgctaacttgtctccactggaggccgacgtaccggctgattggggacgacttccgtgaagccgctatctttcaagcgccaccgctttcccgcggaagtcatccgccacgccgtttggctttacttccgcttcagcctgagtttcagggatgttgaagagctgctcgcggggcgcgggatagacgtgagctacgagaccatccgctgctgaacgatcaaatttggcccgcagatcgcccggcgactgaagcggcttcgcccctccccttccccacgctggcacctcgacgaggtcgtctgttcgatcggcggcaagcgcatgttcctctggcgcgcggtcgatgatgagggcgaggtcctggagcttgtcgtccagcgcaggcgagacacggaggcggctctggtgctgttgaagcgattgttgcgaaatcagcctgttgagccagaacgcatcgtcaccgacggtcttcgttcgtatccagctgctcttgaggcgttgggcctgcgccatctgcattccaccggccggctttgggaaaacaatcgggcggagaactcccacctgccgatccgacggcgagagcgacagcagcagttgttcaagtcccaggcttcagcccagcgtttcctcaccacccacgccgcgatctacaacaccttctacacccaacgtcacctcgtcagccggcccacgcttcgacgcttccgcgccggagccgaccaggcatggatggcggctacagcctaagatttcgccgcgtggggcaagttgccggcttggagcacttagcctgacagcgctgttccaagttgtcagttccaaatgacttgatgacgcaagcgattcatatattttggaattaagtcccaataattgggtcgtcatgaatcatagggaaacggtcggtttgtttcgcaaggcaccacttcgcggattgatggcatgtgcgagcatcaacttcctcatggcctcggcgttcgccaatgctgaagttccacatttggagcggttggatcggtccgtcgtcagcacacaggcccacgacggcggaacgttgcttcaatggcggctgctggtgacggacgcttcagatactcgcttcgaagtgttcaggaatgacgccaagatagccaggatagccgctgctgacgcgacggactggcatgacgtaaacggcgacccgctggcgcgttatgcggtgcgccgcgtgggcgacgaaagccttactgacgcgctggacctgcgtgagggctatctcacaatcccgctggatcgcccagatggcggcgtgatgcccgacggggtggcctatgaatacgaggccaacgacgggacggtcggagatctggacggcgatggccgatacgaaatcatactgaaatggcagccgacgaacgccaaggacaacgccttcgccggcttcaccggcccgacgctgatagacgcctacacgctggacgggcggcggctgtggcgcatcgacctggggcgcaacatccgttcgggtgcccactacacccagataatcgtgcaggacttcgacggcgatggacgggctgaggttgtgctgaagaccgcagacggcacgatcgacggcaccggtcggatgatcggcgacgtcgaagccgactggcgcgaggatgacggcgaaatccccagccgcgaccgcaccggcgccgagcagaagccggacggaaccctggcggcgggtctgaccggccgcatcctgtccgggccggagttcatcaccgtattcgacggccgcaccggcgcggccctggccaccgccccctatgtcccctcgcgcggtcgatccggagacgaagcgacgccggaagagatggcggccctctggggcgacggctatggcaatcgatccgagcgttaccttggcggcacggcctatctggatggtcgtctccccagcatcgtcatggcgcgcggctattatggacgcaccgttgtcgcggcctgggactggcgcgacgggcggctgagccagcgctgggtgttcgacagcgacgccgcgcccgaaggttacgccggtcagggcaatcatcagttcagcgtagcggacgtggacggcgacggacggcaggagatcgtctatggcgccatggcgctggacgacgacggaacgccgctgtggaccacgcggctgggccacggcgacgccatgcatgtcggcgatctggacccgacgcggccggggctggaaaagttcggcgtccatgagaacgtcggcggcaacggcggcgtcggctcggccatggtggacgcccgcaccggagaaatcctgtggcgcacgcccggccagcacgacgtcgggcgcggcgtagccctggacatcgacccccgctatccgggcaccgaggcctgggcgtcgaacggcggcgacctgtattcggcggacggacgggtcatcggccacacccggccgcaacagatgaatttcggcgtctggtgggacggcgacgccctgcgcgaactgctggacggaacgcgcatcttcaaatgggactggcagaaccagcggtccgtccccctgctgagcgccgagggcgcggcgtcgaacaacggcaccaaggccaatccggttctggtcgccgacatcctgggtgactggcgcgaggaggtcgtgtggcgaacgccggacagttcggcgctgcgcatctatgtgaccccgcatccgaccgccatccgccgcgtcaccctgatgcacgacgcgcagtatcgatcgcaggtgtcgggtcagaactcggcctataaccagccctcgcaccccggtttcgccttcgacgccgtcccgccggcggagcgcgggcgatgagggcgaaccgacgcggggttctgttgggcgccgccggtctggcggggtgcgcgagcctgccccgatccggcgcacggcgtctttacgccgacgacttccgccacggccttggtcagtggctggttgaactggagcagggacagggaacggtgcgggccgccgacggggcgatgatcttcgacgtgcccaagggggcgaccgcctggttccggcccgaactgacctcgccggtcgaaatccgcttcacggccgaagccgtgtcgggcggcggcgcccatgaccgggtcagcgatctgaactgcttctggatggccgacgatccgcgcagtcccggcgcccttctggcgcggccccggtcgggggcctttgccgactacgacaccctgcggacctactatgtcgggctgggcggcaattcgaacacctcttcgcgctttcgccgctatgtcgggaacggagaaaggccgctgctgccccagcatgatctgtcggcgccggacgacctgatcgcagccaaccggccctatcgcatccgcctgatcgccgacgggtcgcgcatcgaatactggcgcgacgaccggcgcatgttcgccctgaacgaccccgccccttatcgtcgcggctggttcggcctgcgcaccacctggaatcacatgaccgtccgggacttttcggtctggaccgtcgcctagtttgaggaagccgatgaagaagcatgccctgatcctggcgctggccctggcggccgtgacgcagacagccctggcgccctgcgcccaggccgagacccactgggcgcgaagctggaacgcctcgcccgtggccgccgcgcccgaccgtcgcccgccgacgctgaaggacgtcaccgtgcgtcaggtggtccgcgtcagcgcgggcggcgaccgcttccgcctgcgcctgtccaacgaatacggccccgtcgtcgcccggatcgaacgggtgcggatcgtgcagttggccgacgacggaaagcccgtgcccggcacggcgcgcgacctgaccttcgacggatcgacgggcgccgtcctggcgccagaagcgcccctgctcagcgatccggtcgatctggccctgcccgcgcttagccgcctgtcgatcagcctttatctgccggacgaggtggccgatcccaccatccacctgctgggcctgtcgtccggctggatcgcccccggcgaccagacggcggcggccgaactgacgaacccggtgcttgtgacccagcgcatcctgatctcgggcatagacgtgcagcgggccgagccggggcgggtcatcgtcaccctgggcgattccatcaccgacggcgccaacggcacgcgcgacgccgaccggcgctggcccgatctgctggcggcccgcctgcaagcggccggtctgacctcggtggcggtggccaacgccgggatttccggcaaccgcatcctgaagcccaagcccggtctgggcgtcgccgccctggcccggttcgaccgcgacgtgctggccgtgcccggcgcgaccgacgtgatcgtgctggagggggtcaacgacttcggcatggcctggcgcgaccacgatccgcagccgccgaccccggccgacctgatcgccggctatcgccagatcatcgcccgcgcccatgcgggcgggctgaaggtcaggctggcgaccatgctgccctacaaggacgccaactactggtccgaacagggcgaggcgacgcgccaggccctgaacgcctggattcgcaccagcggagaggcggacggcgtcatcgacttcgacgccgtgatgcgcgacccggccgagccgctgaaactggccgccgcctatgacagcggcgaccatctgcacccgaacgacgccggtttccgcgcgatggccgacgccattgacctgacgccctatcggtgaggcgtgaacggcggcctgacgcggatcaggccgccagcatgtcgcgcgtcatgcccgcgacggacttggccccggtcagggtcatggcgacgcgcatttccttttcgatcaggtccagcaggttctcgacccccgcttgcccgtccgccgccagcgcatagacgaaggcccggcccagcaggaccgcatcggcgccgagcgagatcgcccgcaccacgtccagaccgttgcgaaccccggaatcgaccagaatcttcagatcgccctgaaccgcatcggcgatggccggcagggcccgagccgaggacagcacgccgtccagctgacgcccgccgtggttcgacaccacgatcccgtcggcgccgaagctgacggcgtcgcgggcgtcctgcgggtcaagcacgcccttgatgatcatcggcccgtcccagaagtcgcggatccattgcagatccttccacgagatcgacggatcgaagttgttcgccagccagccgatatagtcggccaggcccgccggcttgcccagataggccgagacattgcccagatcgtgcggcgtgccgcgcaggcccacgtcgaaggcccacatcggatgggtcatggcctggatcatgcggcgcaggggcgcgttcggcccgctcatgcccgaatgggcgtcgcggtagcgggcgccgggggtcggcatgtcgacggtgaagaccagggtcttgacccccgccgccttcgcccgctccagcgcattcttcatgaagccccggtcgcgcaggacatagagctggaaccacatgggccggtcgatggcgggcgcgacttcctcgatcgggcagaccgagacggtggacagggtgaagggcacgccgcgcgaggccgcagccctggccgcctgaacctcgccccggcgcgcgtacatgcccgtcagaccgaccggcgccagcacgaccggcaggcgcagcgtctcgtcgaacagccgggtttccaggctgaggctggtcatgtcctgcagcacgcgctggcgcagggcgatggcctgccagtcctcgacgttgcgcctcagcgtctgctcggcgtatgcgccgccgtcgatatagtggaacaggaagggcggcagcctgcgccgcgcggcctcgcgatagtcgctgggggacgagatgatcatggccgcgccttactggaagttggcgaaggccccgccgtcgaccagcagggccgcgccggacatgtaggacgccatgtccgaggccaggaaggccacgaccgaggcgatgtcctggggccggcccagccgacccaacggaatgcggccttccatatactcgcgcttggccggatcggcgaggtcgtccttgttgatgtcagtggcgatggtgccgggcaggaccgagttgcagcggatgccgtgacgccccagggccacggcgcaggactgcatcaggctgtgcacccccgccttggtgggggtgtagtgggtctgcatctcgccgccgaccagggccgagatcgaactgatcgccacgatggcgccgccgtcgccctgtttgaccatctgattggccgccgcctgcaccatgaaataggcgccgtgcagattgacctccatcgtccggcgcagggtctcgaccggcatgtcgaggaaggtgtggaaggggcagatgccggcgttggagacgaagacgtcgacccggcccagcgcctgaacggcggcggcgacgaaggcagcggcgctgtcgggctgggccacgtcgccgtcgacggcgatggcccggcggccgagcgcctcgatctcggtgaccacttcggcggcggccgcatcgtcgcgataggtgttgagggccacgtcggcgccctgacgcgcggcctcgatggccgtcgcccgtccgatgccccgcgatgcgcccgtgaccaggacgaccttgttctcaagcagcatggggactcccgcgatggttcggcttcagggtttgggcgaccagcccagatcggcgctgatggcgtcggcggcttcggtcacggtcttggtcagttccgtcatccgggcgtcggacatatactgggcggcggaagacacgctgagggcggcgacgatctggccgttgaccgaacgaatcggggcggcgacgcagcgaatctgatcctcgttctcttccagatcgaaagcgtagcccttctgggcatagccatgcatccgctcaagccagaccgcgcgggccgacgagtcgaaggcggcacccggctcggcgtagaagtcgatccactccggctcggtcttgtccagaatcagcgccttgcccaggcctgtcgatgcgatcgggtgccgctcgcccagacgcgagccgatgttgattcggcgacgaccggcgaccttgtccagatagagcgcgtgacggccgtccagcacgcccagatgcaccgtatcgtccgtctgggccgacagttgttccaaccagggccgggccacgcgcggcagatgcatctgctggctggcggcgtggcccaattccagcagtttgggaccgagggagtagccctcgcgcgggcggaacgacagcaagcgacgctcgaccagcgcagaggcaagacggtgcgtcgtgctgcgcgtcagctccagcttttcggacagttccgccaaaggcagagagccttcgatgagggcgtcgatgacgtccagaccacgcagcagggtctggctgccggacgccttggcccccgcctcttcttccctatcgacctgcatggtcttgattgacgccgatcgtcccatttcgtaatcctcattctcagaatgtagcaaaacgcgcaagtcgtctggggccacacaggggacattgacgtgacgcacggaggaaagccagtgaaatcccgcattatgggagcggatcactatttttcggtgattgcgcgatgagccgcctgcctcgcatcaaacatgttcgcgccttcgtcgtgaagaacgacggaaccgggggcggcgccgactaccacgatcagggcgacggccactggatcgacgaccacatcgccacgccgatggcgaagtatcccgaataccgccagagccgccgcagcttcggcatcaacgtcctgggcaccctggtcgtcgagatcgaggccgagaacggcgtggtcgggtttgcggtcacgaccggcggcgagccggcggcctatatcgtcgagaagcatctggcccgcttcctggaaggccgcgatccgtccgaggtcgagaagatctgggaccagatgtatttctccacccagtattacggccgcaagggtctggtggtgaacgccatctccggcgtcgatctggcgctgtgggacctgctgggccgcctgcgtcaggagccggtcttcgccatgctgggcggggcggtgcgcgacgaactgaccttctacgccaccggcgctcggcccgataaagccaaggaactgggcttcatcggcggcaagatgccgctccaccacggccccgccgagggcgaggaagggcttcgcaagaatctggccgagctggaggccatgcgcaacgcctgcggcgacgacttctggctgatgttcgactgctggatggcgctggacctcaactacgccacgcggctggcgcacgaggcacacaagctgggtctgaagtggatcgaggaggccctcagccccgacgactactggggctatcaggcgctgaagaagaacgcgcccaaggggatgctggtcacgaccggcgagcacgaggccacccgctggggcttccgcatgctgctggaaatggaatgctgcgacatcatccagccggacgtcggctggtgcggcggcgtcaccgaactgcagaagatttcggccctggccgacgccaagggcgtgctgatgatcccgcacggctcgtcggtctattcctaccacttcgtggtgacgcgccataacagcccgttcgcggagttcctgatgatggcccccggcgccgacgaggtcgtgcccatgttccatccgcagttgatcggcgagccggttcccgtgaacggccgcctgaaggttcccgacacccccggtttcggcgtcgagctgaaccgcgacatcgccctgcatcgcccctacgcgcgttaagacgaaagcccttcctccaccatgaaactgctgcgttacggccccaagggccaggaaaagccgggcacgctggacgccgaagggcgtatccgcgacctgtcgggcgtcatcgccgacatcaccccggatcaactgcatggccccgcgctcgacgccctgaaagccatcgacccgaccacgcttcctctggtcgagggcgaaccgcgctatggcgtgccggtgaacggcagccgcaagttcatcgccatcggcctgaacttcgcggatcacgcggcggaatccaacctgccgatcccggaagagccggtcgtcttcaccaaggccatcacctgcctgaacgggccgaacgacgacgtggtgatcccccgcggttcggaaaagactgactgggaggtcgaactgggcatcgtcatcggcaagcccgcctcctacgtcgccaaggatcaggccctggatcatgtcgccggctatgtgctgatcaacgacgtgtccgaacgcgccttccagaccgaacgcggcggcacctgggacaagggcaagggctgcgacaccttcgggcccgtcggcccctggctggtcacggccgacgaggtgggcgaagtgcagaacctggacatgtggctggacctgaacggcaagcgcatgcagaccggcaacaccaagaccatgatcttcggcgtggccgagatcgtctcctatctgtcggagttcatgacgctggagcccggcgatctgatcaccaccggcaccccgcccggcgtcggcctgggccagaaaccgccgctgtatctgaaacctggcgacacggtccgccttggcatcgaaaagctgggcgaacaaggccagaccttcgtggagtggacccgatgaacgcctatcgggatcgtttcgcgggccgcgccgccgtgatcaccggcggcgcctcgggcctgggcaaggcggcggcggcgcgcatcgtcgccgaggggggcaaggtggccctgtgggatctgaacgccgacgcgctgaaggccgccgccgaagagatcggggccagccatgtggtcgccctggacgtcgccgacgccgatgcggtgtccgccgccgccgaacagacgcacgggcttctgggcggtatcgacatcctgatcgcctcggccggcatcaccggggccaccgtgccggtgcaggacttcccgctggacagctggcgccgggtcatcgacatcaatctgaacggcgtcttctactgctgccgcgccatcacccccttcatgctgaaggcgggctatggccgcatcgtcaacgtcgcctcggtcgcgggcaaggaaggcaatcccaacgcctcagcctattccgcctccaaggccggggtcatcggcttcaccaagtcgctgggcaaggaactggccggcaagggcgtcatcgccaacagcctgacccccgccaccttcgaaagccccatcctggagcagctgccccagagccaggtcgactatatgcgctccaaaatccccatgggccgcctcggcgaggtcgacgaaagcgccgccatggtctgtttcatggcctccgaggaatgcagcttcacaaccgcctccaccttcgacacctccggcggaagaacgacatactagacggggacacgacatgggcggctggattttcggatgtcggcgcgcccgtgtcgcgaccggagcggcggcggtcattctggcgctcggcggcctgctgtcgccggtcgcgcgggcccagaccgccgacgccccatccagtctggcccaggacgatctgctccagacccgaacctacgggttgaggccgggcgaggacgacgcatccctgaccctgttcgcgccgcagaacgggcgacgcagcggcgcggcggtcatcatcgcgcccggcggcggctatgtgaacctcgcgggcaatctggaggggcggcaggtcgccgactggttcgccgcgcgcgggatcagcgccttcgtgctgaaataccgtcacggcgcgggccgtcccctgccccagccgatcgaggacggagagcgcgcggttcggttcgtccgcgccaacgcccgcgccttcggcctggacgccgaccggatcggcctgatgggcttttccgccggcggccatctggcggccatgacggccagcctgtcggacgacggcgacgccgccgcccccgatgcggtcgagcgggtctcaagccgtcccgatttcctgatcctggcctatccctggcttgaggcgaccgatctgaacgccgagggcggctccgaatactgccgcttcgcccgcatggcccgttgggattgcgcccctcgggactatatcgcctatacgcccctgccgggcgtcgtggccaaggccccgccgaccttcatctatcacaccaccgacgacgccttggtcccggttcggggttcggtcgatctgtattcggccttggcgacggcgggcaaggacgtggagatgcacctgttcgcccacgggtcgcacggctcgggcctgggcggcgccgaccccgccctgaccctgtggccgcaggcgctggacgcctggctgcgggcgcgcggttatttcagcaaggaggcgcagcccgcgtcatgacgtccggtcttcgcatcatcgacagccacgtccacctgtgggacctgtcgcgcgcccgctatggctggcttcaggacgatcccctgccgaacaatccggcgggggacatgacgcccatcgcacaccaggactatctgctggacgactatctggccgacacggcgggctggcgcgtggacaagatcgtccatgtcgaggccggacagcccaggggccggcaactggccgagaccgactggctgcaagccctcgcggaccagcgcggctatcctcacggcatcgtcgccggagccgatctgctggaccccgatctggacgccctgctggaggcccacgccgcgcggccgaacgtgcggggcgttcgccagatcgtctgctggcatgaagacccgctgaagacctataccgaccgcgacctgctgctggacccgcaatgggtcgcggggttcgccagactggcccggcatgggctgtcgttcgatctgcagctctatccatcgcagatggcgacggcggccgcgatcgccacgcgccatcccgacatcccgctgatcgtcaatcacgccggcctgccgaccgatcgcggcgccatcggcatggagcgctggcgcgccgggctgcgcctgctggcggcccagccgcaggtgtcgatcaagatttccggcctgggcatcaccgaccgcgcctggacgccggattcgatccgtcccatcgtcctggagtgcatcgacgccttcgggaccgagcgggccatgttcgcctcggactttcccgtggaaagcgtccacggaaccttcgacgccttctgttccgccttcgacgccatcacggccgacttctcggccgaggagcgggatcggttgttcgccggcgccgccgagacgatctaccgcctctgacgccggcgcgcagcggcgatcacggcctgtagcccagacgcgccgccgcctcttccagactgtcgccgatcagggccagattctcgatggcggccaggctccattgcgccgcgtcgttggtcgacacctgcgggtcctcgtggattggacgcagcacctcggtcccgccgaccgtgtcgccacgtgcgttcaacagggcgcgcagcttggccggatcgttgcccaggaactcgctccaggcgcgctgggccagggccgcgtcccgctcctcgtgcgcagcgtaggcggtcaggcgcgaatgggcctcggtcagcgaccgccccggcgggacctggcccaggaggcccgaaatctcctgcggcgaggcgttgtagtagcggcagtactccagccacgcgcggcggtaggacggcacgtccagcaggtccagcagctcggcgttcatctccgccacgccgaagacggcgttcagatgcgacacggcgacatagtcgccctggccctgatagcggccggtggccaggtcgaacggcgcctccccggcgaaccagcggcgcttcaacccgccgatggtggtcatgccgttgacgatccggtcgcgccagcgccggtcgcccgtccgctcccattccgtcagccaggcggcgatgaaggcgccccacgacgtgccgaagccggacaccacctgcccctcgggcacggcgcgacccggcgcgggcggcagcttgcgcgaaatgtcgacgttcagaagcgcatggtccgaggtgttcagttcgcgcatcaggtcgccgacccgctcgtctgccgtcaggaagtaatagatacggcgataggcgacgttcgagacgcgcggctgcttggacgaatccgaccagtgctgcactccgtggcgcgtgccgaagcccttgaaccggcccaggtgatagacgtccacctcgcccgtgtggcgcgtcatggcctcagccatcttgaacagatcggcccgccccgtccgcagatagctggtccacagccacaggtccgtcgaaagctcggagttgtcccaagcgtatccgcccacgtcgtagcgccacatatgacgatccggatcgtaggtgtgcatcacgtcgccataagaccagaagccgtaccagcgccgctgatcgacctcttgaacataatgatccagaagatgggtcaaacggccttccaacgcggcgcggatcggcgtcgacgtatcgggcaaggaccaatcgccgaacacgcccgccacatgcagccgctccggctcgaccgtcagacgcgccggatccgcgacctgttgcgccattgcggagaagacgtcgtgcgacggggtcgcgcccagcgcccacagggtcagctcggacgtgcgggcgatgccgtgcgcgtcgtcccagccagcctcatagtcctcataggtgatgtccagaccgaccagctcctcggccgtcgtgtccatgccgttggcgctgcgataggggcgcaggtccatggccggcgcatcgggcgaccacatccaggcggtcagctgggccgtgtccgtatgggcgttgcggatgtccagcgcgaccggcgcccgctgccagaagtccttcaggcccagggcgaccccgcccgagacgccgccgacataggccaggccccggctgcgtttgccggcattggaatcgatccaggcgtgcccctcgctggtccgcttgcgcagggtgaaaccgtcgggcgacagctggttgaaggcgaagtcgccccattccggcacccattgcaggccatcgttcttaaggatgtcgggcaggtcggcgaaggccaccgcccggccctcgatctgggcctggcgcacggcggcggtcggattggcgcgggtgcgcaggcccgtcagggtgcggaccgcctcgccccacacgccctcgccctcaccggcgaaacggatgtggcggttatagctggcgtccgtcatcggcgtgtcggcgacgacgcccaggccgcgaatgaagtccgtcttcggatcgccatcgaagatgaagctgtgaacgatccgcacggcgtcggacccggcgtagaaatacagccgcaccgacaccggcagccactcgcgcgtcccatcggtgtggacgccgtccagcttgatcaccgcgcgcacggggccggactgctccaccaccgcctgacggatgcgaacgccgtagcgcgaggacttcaccgccccgcccgcctccagttccggcttgtcctgcgacagggcgaccagcgacagctcgcccacgacaggacggccgccgcgcgtggcgccggaaaccaaggcgtcgcccgacttcggcacgcgccattctagatcgccgaccgtaacgacgatctgctggcccttatcggcgaccctcaccggcttggcgggtgcaagcgaggcgccgggtgccagcgtcaggccgtccagcgccgcatcgccggtcaccgcatgggcagaccatttcagagacccgtcgggccaataggcgatcggccaggactgggcgggcgttgcgcgacccgatccgtcgaggatgctgaacgcctgattgggacgcagggcgccacgcggccagggcacgccaaaggtcgtcccctccagccgtgcgggcttgcgcccgtccagccagcgcagcggggtcgcaggcgcgctgcgacgtggcgcagccaaggcagcgccggacacagcctgagcggctgcgagagaggcggcgcccatgagcaggtgacgccgagaaggttggaacgccatggtcaactcccgccgccccagcggcgattaggctctgaaagacaaacggccgccgcccgctggggcgacggccgtgatcgtcgtcacgatcagtatttgtaagtcgcgcccaggaagaagcgacggcccgaatagccccgattgatcagacggatgtcgccggcgtaggtcgactcgtcctcctcggtcaggttcttgccttccgcaaagagcgtcagccccttcagaccgggcttccacgaaatcttgccgtccagatagccggtcggttccttgatgaccgggttgcccgactggtcggccgccgtgaccagatactgagacctgtagttataggccagacgcgcgttgatcggcccccgctcgtaccacagggtcgcgttgtagctgtcgctggacaggccggggtaagacagttctgaaccatccagttggctgtagacgcccacgtccgacgcttcctgataggtgtagttcagatcgaccccgaagcccgacaacagccccggcaggaaggtgaaggcggtcttggccgtcagctcgacgcccgaaatcttggcgccttcgccgttgatgaagctgttgtagtagtacaggaccccgtcaccgaagacgtcccgttgccccaggctggtgcgcgacggcaggtagaaggtctggatgtccttgtagaagaagcccgccgaaagctgggtgtcgcggttcggatagaactcgaacgacaggtcgtactgcgacgcctcatagggcttcagatcggggttgcccgccgagcagctgtccggaccatcgtccgccgtcccatcgttggcgtagttgatggtgcaggtcatgcttgggatcagatagttgtacagcggccgcgccatcagcttggcgtaaccgacgcgcatgctcagcttgttgtcgatcaaccaggcgttgacgttgaagctgggcagccacttcgtatagtcccgcgtctgctcgaccagggtgttggacaccacggccgtggtcgcgacaccgttgaccaggcgcgtctcgctgcgggtgaacttcccggccgtctgggtctgggtgtggacccggcgcagtcctagattcccgacaaggtccaggccgaagatcgacagggcccaatccagacggacatattgggcgtccgtctgctccttcacccggtaggggatttggtcgtaggtttttccgtcattgccgacgccggaatacagattgtccagattgaagtgggtggtgtccaggttttgggcgatggcgttaaagttgggatacagccagttcgcaggcaaaccaccgccagcgtaatggaaatcggacggcagcggcgtcatcgccgaggcgaagaccgagttcgagaaggcccgcgaccaagtctcggtcgtgttccaatagctggtctgatacgggtttccgtacagcggcgcggtctggtcgatcgtcgccgcgttattcacccgcgccgtcgagttgatcgaattggcgtagatgacgttgttatcgacttccgacgccagattggccccagggctgacgatgaagccgccgtagtcgtaaccctgagtttcggcgttggagtagcgaccgccgaacttgatgttggtcaggaaggtggtgcggggatcaaaatcaacgtccagcttgtactgatcttcgcggttcgatgactgcgagggccggtactgaatttgatactggctgacggcggcggcgtcggcgggcgaagcgccctgagcgaaggtgaagatcggcgccgaggtgcccggctccaggctgacgaccagacccggcgtgttgaagctgaccgaaacgttgttcgtctggctcagcgtctcgctcttggcgttggcgcccaagaaatccaccttgaagcggtcgttataccacttcagtccataggtgatgtagtcggagttggtttcgtactggaagtcacgcgacgagatgctgaaggacgtgtcgccgcctcgtccggaggtgccgaggcagctgcccaccctgtactggatgacgttgtggttcgcatccacgaccacgcccggcacactttccgccgtggtcgtcgtcacccgcgggcagccggcggcgtagttcaggcgatcaaggctggtgaaatccgtgccgtagttgatgtcgttcagttgctgcgtccgcttgttcgtctgataggtgacgaaaccacgcagattgtcggcgaacttgtactccgccgtgaattcacccgaagtgcgctcatcttcccgcgtccagacgcggtagcgggggatgcgcggattatagtcgtaccattggctttgacaggcggtgcgcgcctgggccgtggtcagcgtgtttgcgtccggcgtggttattgtggcgcaggccgcttcgctgccgatggacgcgatgtagtcgttcaccgcgcggctgtaggactggttataatagttgaccgtcttctccggcgaattgtcgaaatcggccagacgcgcccaggagtggtcgtcgtagaagtcgccgcgtgtcaggacgctgtcataggtgacattggccatcaggcccaggcgaccgtccagcaactgcgtagcgccaaagaagctggcgcggggcttccagtccggcaaggtgtccagtttttgacccgacacggtcatcgagaaggtggggttacggaaatccaggggcttgcgggtctgcaccgacaccgtgccgcccaccgcgccttcggtcatgtcggcggtgaagcccttgaatacgtcgatcgacttgacgatttcggctggcagttcgcggaagtcgttggagcgcccgccgccgccgtagacgttcagattgcccgccgtggacaggacgctgacgccgttgatctcgacgcggttcaggtccggctcgacgccgcggatcgaaacggcgttgccttcgccgaagtcgcgcgacagttgaaccccggtgacgcggcccagggcttcgcccacgttcttgtcgggaaactgaccgatgtcgtcagcgacgatggaatccgaaacggtgctggccgaacgcttgcggttcatggccgactgcaggctggagcgagtgccaaccaccacgacctcgtcgacggtggagaccggagcggtcgaagcctggctctgagccgtgtcctgcgcggtcgctgcgcccgcggcgcccagcatcagggcggcggcgccggcggtgtacatgaagcggcgagccaaacgcccgttcgattgtgtcgtcactgaaaatcctcctccggcctggggccttattgttttgatcgacgccttcgcggccgctccccggcggttcattctctgaaggcggtgtcgcgggccatgatcgcccgccgtgtcctctcaggtcgtcgccgcagaccggcggccctgcggaccccgctcctcccggcgcgccttgcgcgcttccctcctgcaagcggtccttttgcggactcgaattcttgttgcgagaacagctatagcacctgcagcgatttatgccaaatatgaatttgtcgtctcatattttgagaaattaggcctggagcgtaaaaaaacgccgtcaggacagcctgttgcggccccacagtttttcgaagggccagccggtcaggctctcgaccaccgatttggcttcaggcgtggagggttcggtcgctcccgcgcgcaagcggtcgatctcgctcatcagaatcttgtggctgggttgatccagacggaaagaccaggacaggatcgcgcccgcccccatgaccaggatcggccctgcgaccagcagcccagccaccgtcgcgactgcgcccggcgtctgaaccacggcgacgcccgccgccccggccttgggcgagacatagccccccgcctctatgatccagcccgtcaggatgatggcgccggactgcgcgaccttgcgcaccagcgtcatgacgccggcaaaaatgccttcgcgccgctgccccgtgaccgcttcatcgacatccggcagatagttgtagaccgaccacggcacgaagttcagcgtgccccgacccagccccgccagaacaatcggtcccagcagccagaaggcggcgcccaggttgaacccgcccgagaccggattgatcagggcgaacagatcctgaccgccgatgctgggccgcacgaaatagaaggccagcagcagaaccaaggcgctggcgaagaagcctgccgcgatccggtaggcgatcaccggaccgatgcggatgaccagattgatcgcgaccatcaccgagatcagttgggccacatacatgaccgtcatcatctgcgagatcatcaccgtcgcgcccagcatcaccgtggccacgaagatcgggaaggcggtgttgaagatgtcctgcgagatatagccgcccagatagatcgacagatgctggcggaaggcgcggatgcgcagtgtcgaaaacaggtcgcggaacatgttgaccgggatcagagccgcccgtcgcaggttcagcggctcggccttcatcgccttctcgccgtcggtgaacggccgctcccaggtgaagatcaccaccaggatcaccacggcgctgaacaaaagaccgaagatggccgccatgatcaggaaggtctgggccgaatccttgccgccgaagttgttgatgatcagggtcggcagataggaggccaggatggccgagctttgcgccaccagcatccgcgccccggcgaacttggccttctccttgtaatccttggtcatctcggccgcgagcgtctcccacggaatgagaaacatcgtgtagagcagttcgaagaagatgaaggtcgtcagataatagacgaaggtctggccgctgatgaagatcagggcgaagctgggcagcaggggaatggtgatcagcaggaagatcttcctgcgccccacggttcgcccgatccaggtgtggcgcagattgtccgacacatagccgatcagcggacaggtgatggcctccagcaggcgcggcagacccagaatcaggcccgcctcaaccggcgtcaggtcgcagaaggtcgtgaagaagtagaacagccagccggtgatgacggcctgcgcccccgcccccagcatgtcgccggagccccagccccagtagttgtaccagcgcgggctgcggggggacttttgcgtggacgtcatctcgacttctcctgaccgcgccgcgtcagatgtactgacgcaggaattcacccaggcacaggatcgccaaggactggccgtaaggcatggaggtcaggggaatgtccttgtagccctgcagatcgtcgaagaccggggtgccgaacgacacctgctgcagttcgccgtcgtccgaaatgttggccaggacgcccttgaccgccttcagcgccatcggggcgtattcggcgctgatgtagcgtttacggaccgccttcaggattccgtaggcgaagccggcggtggccgacgcctccagatagctgtcgtggtccgggataagggtgcgccacaggccgctctcgtcctgatgctgggccagggccttcacctgggcctccagcgtctcgatcaggaaccgacgcaggctgtcctcgggcggcaggtccagcagctcgatgaactccgggatggcgatcgtgacccagcagttgccgcgcgcccacagcgcatcggcgaaattgtgccgccccaggaaggtccaaccgtggaaccacaggccggtcttgcggtcgaacagatatttgatgtggatgaggaactgcttcttggcctcctcgacatagtgcgggcggtccagcaccaggccgatcttggccagcggcaggacgctcatcatcaatgtgtcgtcccagagctcctgcgggttctcgtcgttgaagacgatgtgctggaaaccgtcctcttcggtgcggggcaggccgtccatcagccattccgcccaggtgtccagatacggaatgaaggtctggtcgcccgtctgttcgtacagataggccaggatcaggaagggcgagaccgtgttgatgttcttggtcggcgtcccggcggcgaagcggtcgcggaaccagttgagcatgatgtccagcgcggccggatcgttggtctgctcatacagtttgtaaatgccatagaggccgatgccgtgggtccattcccagtcgttccagcccttggtgtcgatcacccggccgtcttccaggcgcagcaggaactcgccggtgtcgtccttgatgttcaccagattgtccatcaggcgcgcgatggcgtcgcggacgtcggcgtaaggcaggtcgtggatcaggttcggcatcgcggattcccaaggcgccggggcgccgtcattcacatcagggcggagatgatcaggcagggatttccacgggcgcgacggcgacaagccgtcacgcgcgcccttggccttcccgacagtttccaccctattctcgaaaacgacgcctagcaacgccgtcccatttcttatatgccactctcattatgtgagcataaatgccccgtcaagaacggggccgagactctgtaaagccttcggggcggccgttcggagaggacgggcgtcgcgaccaacctgttcgaggccaaagaccatgtccgaccccatgtacgacaagatttatcaggcgacccacccggacatgatggacggcgcgacgaaccagcagttgcgcgaccgctatctggtcggcggcctgttcacgccggacaaggtcagcctgaactattcgcacaatgagcggatggtgctgggcggggccatgccggtcgccggcgccctgagcctgcccacccattccgagccgccgtccctggcgggcaagccattcctgcacgcgcgcgaactgggcgtggtcaacatcggcggcgccggttcgatcaccgtggacggcgaaacggtcgagctggccttccgcgacggcctgtatgtgccgatgggatcgagcgacgtcaccttcgcctcgaaggacgcggccgaaccggcccgcttctatctgatcgccatgccggcccacgcccgctacgacctgaccaagatctcgatcgaagaggccgtgccgctggagatggggtcgctggagacatcgaacgagcgcaccatctatcagtacatcgtcccggccaaggtgaagtcctgccagctgctgctgggcgtgacggtgctgaagcccggttcggtgtggaacaccatgccgccgcacctgcacgaccgccgctcggaagcctatctctacttcggcctgggcgagaacgaccgcgtcttccacttcatgggcgagccggacaacgcgcgccacatcgtcatggccgacggcgaggcggtgatcagcccgccgtggtcgatccacatgggttcgggcacctccaactacaccttcatctggggcatgggcggcgagaacctggactataccgacatgtgcaagctcgacatctgccagctgcgctgatcgggacaggggagagatacaccatgagcaatccgtttgatctgaccggcaaggtggcgctggtcacgggcggcaatgtgggtctgggtcagggcatcgccctggccctggccgaggcgggcgccgacatcgtttcggtggccctgtccgattccgacgacacggtcgcccaggtgaaggccatgggccgccgcgcccacgccgtcagcgccgacctgacctccatcgagccggtcgagcgcgtgctggccgaggcgctggaggcgatgggccgggtggacatcctggtcaacaacgccggcctgatccgccgcgccgacgccgtggacttcaccgaggccgactgggacctggtgatgaacatcaatctgaagacggtcttcttcatgagccaggcggtcgcccgcctgttcatcaaacagggcgacggcggcaagatcatcaacatcgcctccatgctgtccttccagggcggcatccgcgtgccctcctacaccgcgtccaagtcgggcgtcgccggcctgaccaagctgatggccaatgaatgggcgccgcacggcatcaccgccaacgccatcgcccccggctatttcgccacggccaacacccaggccctgcgcgatgacccggtgcgttcggctgagatcctgggccgcatccccgccggtcgctggggccagccctcggacctgggcggcgccgccgtcttcctggccagccgggcctccgactatgtccagggcgccatcctgccggtcgacggcggctggcaggcgcgctgacggcgggttagcgttccgatatgaccagcatcgcttcgggttctccggccgtcgatcacggcgccatcctctcctttggcgagatgttgctgcggctgtcgccaacccagaacgagttgcttttgcagtcccccgccctgatcgtgcgtccgggcggggccgaggcgaatgtcgccgtgtccctggcccgtttcggcgcgccgacgcgtatggcgacggtgctgcccgacaacgccctgggccatgccgctcgcgacgaagtgagaaagcacggcgtcgacaccacccccatcgtcttcacccccggacggatggggctgtatttcctgacgcccggcgcggtgcgccgtccgtctgaagtcctctatgaccgcgccggatcggccttcgtggagcatgtgaacacggccttcgactgggaccggctgctggacggcgtcgagtggctgcacgcctcgggcgtaaccccggcgaccggccccaatggctccgccgccgccgtagccctgatcgaggccgccgtccgcaagggggtgaaggtcagctatgacggcaacttccgcggcaagctgtgggagcaatgggatggcgatccgcccgcgaccctgggtcggatgctggcgggggcgaccatcgcctttgctgacgaccgcgacttcgctctcgtgctgaaaacccgattcgacagcgccgatccggccgagcgccgtcgtcaggccgcccaggccgccttcgccgccttccctcgcctgcaacgcatcgcctgcacccagcgcgttcaggaaagcgtcgccgaccaggctctgtcggccgtcatgctgacgcggaaaggcgacgacatcatcgagaccggcgccgaggccatccacatgacgggcgtggtggatcgcgtcggcggcggcgacgccttcgcctcgggcgtcctcttcggcctgtggagcggctggacggatcagcaggcgctggatttcggattggcggcggccgggctgaagcactcggtccccggcgacttcaacctgttttccgccgccgaggttcacgccgcactgggtgatggcgggttcgatatccggcgataggcgccgtcccctcacgaagagacacctcgatgctgacggcgattctgatggcggcgacgatatcgacttggcgtttcgacctggagcctcgcccgaccgcgccggaccggatcgcagtccagcccagccagacctatcagcccggcggctacggcttcgagccgcaggcgacgccggagggctttgtcttctcggcggcggttcctgaaggtctctatcgcgtgaccatccgctttggcggggccgaggccgggcgcacgacggtcaaggccgaggcccgccggttgatgttgcgcgacgtcgtcaccgcgcccggcgcctatcagatccgcagcttcctggtccatgtgcgcggccccgccctgcccccgccgcccgccaatgcgcctggcggaacggccgtggtccttacgccgcaggagctggcctcgcgcacctgggacgaccggctgacgctggagtttctggatcgcccgcaggtggcgtccatcgacatcgagccggtcgacgcgccggtggtctatctggcgggcgattccaccgtcaccgaccagccgtcggaaccggcggccagctgggggcagatgctgcccgccctgctgacgcccgacatcgccgtggccaactacgcccagtctggcgagacgctgaagtccttcatcagcgaacttcgcctggccaagatcctgacgacgctgaaggctggcgactggctgctgatccagttcggccacaacgaccagaaggcccagtggccccagacctacgccgatcccgaagccacctatccggcctatctgagggtcttcatcgccgaggcgaatcggcggggcgctcatcccgtcctcttgacgtctcccgagcgccgcaacttccgtgacggacgcatccaggacaccctgggcgcatacgccgaggcggcgcgccgggtcgcgcgcgaagaggacgtgccgctgatcgatctgaacgacgcctcgcgccgaatctacgaggcgctgggtccggatctggcggcgacattgttcaacgatggcggcgcggatcgcacgcaccacgacaacgccggcgcctggctgctggcccgcgccgtggccgcccagatcgcagaaaaggcgcccggtctggcggaccacatcgcgccggacttccgcaccttcacccctgacgccccgccgatggccgagatcgacatcgcgccgagcctgagcgccagccgcgaacgtccgcgcggcgattgatcgcgccaaacccggtttgacgcgcctgccgggacggactaccaaataatgaaataaaataccgaataatcggaaccggaggaaacatgggcacgcttcacgccttccgcatgcagctcaagccgggcgccgtcgccgaatacaaggcgcggcacgacgccatctggcccgaactggccgaattgctgaccgccagcggcgtcagcgactattcgatcttcctggacgaagagaccctgtcgctgttcgcggttctgcgccgcgcggacgaccacacgctggacgacctgcccaaccatcccctgatgcgcaaatggtggacctatatggcgccgctgatggaggtcgagccgggcgacaagccgcgcgaatggcccctgcaactgatgttccatcaagcctgatgcgcgcgcttctcctcgcggccgccgtcgccgccgccccgctggttcaggcctcgaccgccgtcgcccaaacggcccaggccaccgccgacttcaccgcccccgcccagaccttcggccgggtctcttacgacgcccgctccctgatgatcgacggcaagcgtctggtcatctggtccagcgaaatgcaccccttccgcctgcccagccccgagctgtggcgcgacgtgctgcagaagatgaaggccagcgggttcaacaccgtcgccttctatttcgactggggctaccacagccccaaacagggggtttacgacttcaccggcatccgcgacctggatcggttgctgaagatgtcggaggaagagggcctctatgtcatcgtccggcccggcccctacgccaacgccgaactgacgcgcggcggcttccccggctggctggtcaatcagcgcgcgccgtcgcggacggattcgccggactatctggccgccgccgacgaatggctgacccatgtcaacgccatcattgcccgccaccagatcaacggcgacggccggggcaaccagggctcggtcatcctctatcagatcgagaacgaactggcggtaacgacgcccgcgcaccgccgctacatggatcatctgtacgccaaggcgcgcgcggacggcatcaatgtgccgatcttccataacgaccagggccgcaacggctattgggcgcccgagaactcgccggtcgaaaaggtggtccacgggccggtcgatctgtacgccttcgacggttatccgggcggcacctgcaccgtcggcggccagaccacgcgcggcgcggcggcgcccgactggggcttctatggtcccggcggggccaagggcggcgcctcggcctcgccttcgacgcccggcttcatggccgagatcggcggcggctggttcgactattggggctccaacggcggttacgagtgcaacgcccgccagcgcggcgagcggttccagcgcgtcttctatggcgtgaacctggccaacggcatttcgcttcagagcatctatgtcggtttcggcggcaccagctggggctggctggcggcgccggtggtcttcaccacctacgactatggcgcggccatctccgaagcgcgggacctgcggcccaaggccgaggagatgaagcaactggccggcctgcttgagtcggtccccgatctggccggcatgatccccgccgggcctgtcgagatttcctcgccgaacatccaagtctatcataaccgcagcccggaaacggacgcccgcttcctgctggtcacgcacaagccgtcgaacggacagaccaacgacgacttcaccgtcaccgccgacctgcccgacggccgctatgtcgtgccgatgacgctgaacggcttcgacgccaaatggcttgtcgccggggtcaatctggcgggacagcggctggtctattcgacgtccgaggtgcaggcggtcctgccgtcggcgcgccagccggtcgtcctgatgtacggccgcaaggacgagccgggccagacggttctgcgcttcgcctcggccccgacggtgacggtgctggaggggcaggtccgctccgcctttgatccggcgaccggcgacctgaagctggactacgttcatcagggtctggcccgcgtgaagatcagcggcggcggtcgtcccgaccttctgctgctgatcggcgaagagaaggaggccgcgcgcttctggcgtcagggcgaggcgctggtgcgcggcccggccctggtgcgccatgcccgcatcgaacgcggccaactgcttctgaccggcgacaccaaggccgaaacgccgctggagctgtggtcgtcggcgcctttacggtcggtgcgctggaacggcgcgacggtggccacgcgcgccacgacgtcgggcgggttggaggcgcgcgccgccctgcccggtccggccgatttcgccctgccggcgcttacgaactggcgctcggcccccggatcgccggaagccaagcccgacttcgacgacaacggctggcaggccatcgacaaccgcgcctacgccagcaacaccctgcgccccgacggccagccgaacatgctgatggacgcctacggcttccacgaaggcgacgtctggtatcgcggccggttcgagggcgggccgaacgccgaaacgatcgaactgttctatggcgcgggcggcgccgggatgttgcagctgttcctggacggcgaactggtcggtcaggacgaactgccgaccggcatgccgcgcccgatcaccacgggcctggcgcgcttcaccctgcccgccgccgcgcggacgccgggaccgcacgtcctgtcggtcatggtgcgcaacaacggccataactggaatctggacgccaacgacttccacaaggaagcccgcggcctggtctcggtctcggtcggcccgcgcgccggccccggcttctcggtccccatcgcctggaagattcaggggcgtcagggcggcgagaacttcaccgacgccgtgcgcggcgtcgccaacaacggcggcctgttcggcgagcgaaacggctggcacctgccccagttcgacgacacgcgctggagcgccgccacggtcggtgaggccctgcagccgggcgtgacctggtatcgcaccggcttcgacctgaatgtgccccagggccaggacgcctccatcggcctggcgttcggcgacatcgacacgccgcgctcggacaaggcttaccgcgttctgatcttcgtcaatggctggcacatgggccagttcatcgccaacgtcggaccgcagcgggtcttcaccctgcccgagggcatactgaacgcacggggccacaacaccctcgctctggccgtctcgaccgacggggcgcccggcaatgtgctggaagatgtccgcctgatcacccagcgcaatgtgcgcggcggtgtccagaccaccacggaaggatcgcgccgatgaccacgcctcgcctgccccgtcgcaccctgtttgcgcttggcgcaggcgccttggtcgcccccgccgtcgcccgcgcccagactccggcgccgccgcctacgccgttcgaggtccgccccctctggcccggcgctgcgccgggcggcgaggcggtgacggttcaggaacaggtcgtcctgcgcaatccgaacggagaccccaacgacacggccttcgtccatgtgcgcgatccgtggatcatgctgcgtcgccccgcacagcccaatggcgcggcgatcctgatgatccccggcgggggctatcagcgcgtcgcggtcagcaaggcgggcggccccatcgacgcgcgtctggccgagatgggctacaccgtcttcatcatggactaccgcctgcccggcgacggctgggccgccggtcccgccgtcgcccttcaggacgcccagcgcgccatccgcatcgtccgctcgcgcgcggccgaactgggcttcgatcccaaccgcgtcgccgtcgccggcttctcggccggcggccatgtggccggaatgttggcgacgcggttcgctcaggacgcctatgcgcccatcgacgccatcgaccgcctgtcggcccggcccgacttcgccggactgatgttccctgtcgtcaccctgaccccgccctacgcccacggcccgtcggcccgcgcgctggtgggaagcgacccgaccgaggccgcccgcgacgcctggtccatcgaacgccatttgcccgccgacatgccgccgaccttcatcgccgccgctgcggatgaccgcgtcgttccggtcgagaacagtctgatgctgtggcaggccctacgcgctcagaaccgccccagcgaactccacgtcttcgagcaaggcgggcatgggttggcccagacggatgcttcgggtgcgcccgcctggatgggcttgttcgacgccttcctgaaacgggaccgttcgccaaggtcgtagccagaagtctaaatcaagcgacgtcgatcagagaatccgcgtcacggtaaacacaagggggaatgaaatgacggatggggtgtctgaaacggtcgagggagccacgccgctggcgaaggactcccgcctggttatcctggcgtcatccgtcggcacggtcatcgagtggtacgatttctatctgtacggctccttggcggccatcatcacggcccagttcttctcaggggtgaatgagacgacgggcttcatcttcgcgctgatggccttcgccgcaggctttgccgtgagaccgttcggggccatcgtcttcggtcggcttggcgacctgtggggacgcaagaacaccttcctggtcacgatgctgctgatggggctgtcgaccttcgtcgtcggtctgttgcccagctatgccgccatcggcatcgccgcgccgatcattctggttctcatgcgcctgatccagggcctggctctgggcggagagtatggcggcgcggcgacctatgtcgccgaacacgcgccgcccggcaaacgcggcttctacacctccttcatccagatcacggcaacggccggcctgatgatctcgctggtcgtcattctgggcgtgcgcaccgccgtgggcgaggcggccttcctggactggggctggcgtattcccttcctggtctcgatcctgatgctgggcgtttcactgatcatccgcctcaagctttcggaaagccccgccttcaaacagatgaaggccgaggggcgcggatccaaaacgccgcttaaggacagcttcggccgctggccgaatctcaagctggtgctgatcgccctgttcggcctagccgccggccaggccgtggtctggtacacgggccagttctacgccctgttcttcctggagcgcgtgctcaaggtcgacagcgcccaggcctatctgctgacggcggcggcccttctgctgggcacgcccttcttcgtcttctggggctggctgtcggacaaggtggggcgcaagccgatcatcctgaccggctgtctgctggccgccctgacctatttcccgctgtttcatgcattgacgggcgctgtgaacccgcagttggccgccgcctccgcccagtcgccggtcacggttcacgccgaccctgcggactgttccctgcagttggacctgatcggcaaggcgaccttcacccagtcctgcgacgtggccaaatcctatctggcgcgcgcgggcgtcagctacgacaccgtcgccgctccggccgggtcagtggcggagatccgcatcggttccgtcgtcgtgcccagcttccggggcgagacgatgaccccgcccgacttcaccgtcgccaagaaggcttgggacgccggcgcggccaagcagctgaaggccgccggttatcccgccaaggccgatccggccaaggtcaacctgccgctcaccatcggcatactcttcatcttggtgctgtatgtgaccatggtctatggccccatcgctgcggccctggtcgagatgttcccgaccgagatccgctacacctcgatgtccctgccctatcacctgggcaacggctggttcggcggcttcctgccgccggtggccttcgccatcgtggccgcgacaggcaatatctactacggcctctggtatccggtggcgatcgcggtgctgacggccgtgctcggcttcgtcttcgtcaaggacggccgaaagacggacatcaacgcccgcgccgactgacggtccctgatgtccaggcggcgggcttgccgccgcctggttcctgtcagagccggatcaggttctggggcaggccgggcgtttcgacccgcacgcggaacaggccgcccaaggtcggctggacctcgcgcttgtcggcgttgcccagccaggcggtggtcagatagaggtcgcgcaggtccgcccccccgaaggccgccttggtgacggtctggacgggggccgtgatcttgccgatgcgttcgccttggggcgaaaagcgcgccaccccccagccgttgaacaggccgacgtgcagaacgccgtcggcgtccatgctaggcccgtccgcatagccgtcctccgtcacggcgaagacgcgccggttcgagatcgcgccttcgtcgtgatcaaacgccaggatggtcttcttcagcgtgtcgtggtgatagagggttcggccgtcggggctcaggcacggcccgttggtgacgccgtagccgtcgtcgtgtcgcgtcagctcgccccggaaccagcgatagagagcgcccgtctcccgttgctcgctgtcgtccattgatccgaaccacagggccccgtcgggcgcgacatagccgtcgttaagccggttctgcggccggtcttcctccaccggttgaaaccgggagaagtcgccccgatcaggatcgaagcgatgcaggcggccgcgaaccccgcaaatcagagaaccatcttcggccggcagggcgaacccggtctggtccggcgtatcccacgaacgcgtcccgcctgtcgcagggtcgtatcggtgcagcttgcgccccttgatgtccacgaaccagacgacgccgcgcgccgcatcccagacaggcccttcgcccagttcggcctggacgtcccagaccagttcgacgttgctcatgagttcctctggcgttgcgctcagtgactgtcgcgcggcaggccaaaccgatcgacgagacgatgatacttcacggcgggttcaagcacggcgccggtttccagctggccgaccacggcgcgctgcatttcctgccacggagtctgggaggcgggataggcatagcccccggcggcctcgaaggcccggcgacgatcggccagttcctgatcggaaatcaggatgtcggcgcggccggtgttcaggtcgatgcggacccggtcgccggtcttcagcagggcgatgtttccgcctgccgccgcttcgggcgaggcgttcaggatcgagggggagccggaggtgcccgactgacgtccgtcgccgatgcaggccagggcgctgacgcctttcttgatcagataggcgggcggccgcatgttcacgacctcggccgcgcccggatagccgatggggccggcgccgcgcatgaacagcagggtccgctcggtgatgcccaggctctcgtcgtcgatgcggtggtgatagtcctcgggtccgtcgaagacgacggcggggccttcgaaggcgttcaggtcgtcggggttcgacagatagcgttggcggaactcttccgagatcacgctcagcttcatgatggccgatttgaacagattgccggtgaagacgacgaaaccggcgtcggtcttcatcggagcgtcgaaggtcttgatgacgtcgggcaggacgatctcggcgttcctgcagttgtcgccgatggacttgccggtgacggtcagggcgccttcgcggatcagcccctgtttcatcagttcggagacgacggcgggcacgccgcccgcgtggaaatagtcctcgcccagatactcgcccgccggctgcaggttgaccagcagggggacgtgcagcccctcggtctgccagtcctgcaacggcacgtcgacgtgggcgtggcgggccagggccgtcaggtggatcggggcgttggtcgagccgccgatggcggagttgacgacgatggcgttgtggaaggcgtccttcgtcaggatgtcggacggcttcagatcctcgcgcaccatgtccacgatccgcaagcccgtctcataggcgacctgggcgcgctcgcgatagggcgccggaatggccgccgagccgggcagcgacatgcccagcgcctcggccagcgaattcatcgtcgtcgccgtgcccatggtgttgcaatagccgaccgacggcgccgaggaggccaccagttcgatgaagccgtcgtagtcgatctctccggccgccatcatctgacgcgccttccagatgatggcgcccgaacccgtgcgctcgcccttgtgccagccgttcagcatcggcccgaccgacagggcgatggcggggatgtccaccgtggcggcggccatcaggcaggcgggcgtggtcttgtcgcagccgatggtcaggacgacgccgtccagcggataaccgtaaaggctctcgaccagacccagataggccaggttgcgatccagaccggcggtcggccgcttgccggtttcctggatcgggtgaatggggaactccatcggaacgccgcctgcttcacggataccgtcccgcacccgctccgccaaaatcaggcgatgacggttgcaaggcgacagatccgacccggtctgggcgatgccgatgatcggcttgtcggactgcaattcccgccgtgtcagaccgtaattcaaatagcgctccagatagagcgccgtcatgtcgggattttccgggttgtcgaaccaggcgcggctgcgcagcggcttcttgggctttgagttgtcggtcattcaggtccagccgccatcgacgacatagtgttgattggtgatcgcccccgactcatccgagcacatgaagacgaccacgcgggcgatgtcgtcgggcacgagccggcgcttcagacactggttggcgtagatctctttctcggtttcgggcgtgacccaaagctcaagctgccgctcggtcatgatccatcccggcgctacggcgttcacgcgcacgccgaagggaccgaagtcccgcgccagcgaccgggtcaacccgatcacggccgacttgcaggcggtataggccggcatgccgccctggccgatgatccaggaggtcgagcccagattgacgatcgcacccttgcccgcggcctgcatgtccggcagcaccgcctgggcggcgaagaactgatgtttcaggttcaccgccatgcggccgtcccaatatgcctccgtcacgtccagcgtggcgtggcgttcatcgtgggcggcgttattgaccagaacgtcgatgggcccgaacgccccgcgtacctccgccaccgccgtcttaagggcaggaatatcggtcaggtcacaggcgacgaaacgtgcgccctggcccagttcggcctccaacacacgcccccgctccacgtcgatgtccaggaagccgacacgcgcgccctgagcgtgaaaggcgcgcgtaatcgcctcgccgatgccgcctgcgccgcctgtgacgatgacggtcttgtccttcagatcgggatagatggcggccatcaggggtgcgcgcctccacgcggctactttcacaaatgaaagccaatatcgtcagcaaaaatgacgcctaacgtcatcgctgtcaacgcggcgaggctcacgcttgggaggcggcgcccatctgatcggaaatgaaggcggcggcctgaactagccgcatcgccgcctcgcctagggcgcaggaggcgggctgctgttcgatgaagggcgtgatcaaggtggcgatcaccccgtccgccccctggatcggcgcgaccagatcggtgacgcccttcacgaaatcgctgggacgcgcgacgtgatcgtttttggtcagggctcgcgcctgcttggcgaaggccgccacgggctcggcgccgaactgggcgaccagcagatcgtgcagatgattgcgcgtttgcggattggcccgcgcgtagaacattaggcccgaggtggcgtgcagcatgtttcgccggtatccgacccgaaccgaatagcccaggtcgcccgggctctcgatccgggcgatgacgacgatctggtcgccgctcgggacgaccaggtggcaggattgacgagtggcggcggccaggtcacgcatcggcggcagggcgacctccaccagagaacgcgccggcgtttgggccatgcccagggcgaacagccggttggtcaggcgataggccccagcgtcctgttcgatatagccgcgaaactccagcacctggaccatccggaacagttcgctgaccgaccggccaagcgccgccgacatttgggacaagctcatggcctcggcctgcgccgacagcagttccagcacatccagccccttctccaaggccggcgcacggtatttccgatccgcggagggcgacggatcggtcatggcggattctggtctttgcggcgctgacattcccagacgataccgtgagtgaaaacccaaagcatatataaaaagcgcattgccgcgcccgccgctgtcccttaggctttttgaagcggtcgcgtcgccggccgggttggggagtaacgcaccatgaagctcgcaggcatcgatctggcgattctggcgatctacgccatcttcatcttcggcctggcccagtgggtctcgcgcagcaaggcgggacatcagaagacctcgaccgactatttcatggcgtccaggagtctgccttggtgggccatcggcgcctcgctgatcgccgccaacatctcggccgaacagatcatcggcatgagcggatcgggctatgtgatcggcctcggcatcgcctcctacgaatggatggcggcgctgaccctgctgatcgtgggcaagttcttcctgccgatcttcctgcgcaacgagatcgtgaccatgccgcagttcctgcagcagcggtacgggccgacgatccgcaacgtaatggccgtgttctggctgctgctctacgtcttcgtgaacgtgacctcgatcctgtggctaggcgccatcgcggtgcacaccgtcacgggcttcaaccaggattacgccatcgtcgccatcggcgtcttcgccctggcctaccagctgtggggcggtctgaaggccgtggccctgaccgacatcgtccaggtggccctgctggtctgcggcggtctgatcatcggcttcatcgccctgtcgaccatcggcggtgcgggcggcgcgatcgccggcttccacaccctgctgaccgagttcccggacaagttcgacatgatcctgtccaaggacaatccccactatcaggaactgccgggcatcgccgttctgctgggcgggctgtgggtcatgaacatcagctactggggcttcaaccagtacatcatccagcgggccctggccgccaagtcgctgccggaagcgcaaaagggcatcgccttcgccgcctatctgaagctgctgatgccggtgatcgtggtgctgccgggcatggccgccctgatcctggcccccaatctgtcggcgccggaccaagcctatccgacgatgatgaacctgctgccggtgggtctgaagggcctggtcttcgccgccctgatcgccgccatcatcgcttcgctggcctcgaaggtgaactcgatctcgaccatcttcaccctggacctctacgccaagatcaagaaggacgtgcccgagcaccagttggtcacggtcggccgcatcgccgccgtcgccgccgtgatcatcggcatcctgaccgcccgcccgctgctgggcggcttcgatcaggcgttccagttcatccaggagttcaccggcttcttcacccccggcatcgtggtcatcttcatgctgggcctgttctggaaacgcgcgtcggaagccggcgccctgaccgccgccatcggctcggtcgtgctgtcggccatcttctggtggctgcaggaaaccggtcagttcatcttccccttcatgaaccgggtcggcgtggtcttcgtcatctcgctgatcgcggcggtgatcgtgtccctgccggtcccggccaagcccgacgccatgaagatcaagctggaccagattagctacaagacctcgccgggcttcaacctggcggcggtcggcgtgatcgccttcctgatcctggtctatacgatctggtggtgaggtgagttcagcgaccggactgatcggggtcgattggggcaccagcaatctgcgcgtcatgcggatcgccgagggcggcgtggtgctggacagccgcaccgacccgcgcggcgccggcggcctggcgccgagccggttccgcgacgtgctgaacgaggtcgcgggcgactggctggacgacggcctgcccgccctgatcagcggcatggccggggcgcggggccggtggcgcgagatggcctatctgccgtgcccggccggcgtcgcggacctggcgagcgccgtggccagccccgatgacgcgccccacgtctccatcgtgcccggcgtcgccgtggtcgacgacggccgtcttcaggacgtgatccgcggcgaggagacccaggtctttggcctggacgcgccggacgacgcggtggtcgtcggtcccggcacccacagcaaatggatccgcacggctggcggacagatcacccatttccgcaccttcatgaccggcgaactgttcgccgccatccgcaagggcaccatcctgggcgccgacatgggcgagccgggcgtggacgacgacgccttcgccgctggggtggagcgggccttgcatgatcccgccgtgaccgccgccctgttctcggtgcgggtcgagggcctggccgggcgcctttcgccggcgtcctcggccgactatctgtcgggcctgctgatcggggccgaggtcgcggcccaggtcgatgcgaaccatcgtcccatcatcctgatcggcgccgaggctttgagccgccgctatgccgccgccctggcgcagggcggtttccaagacgtccgcatcgcggacggcgccgccgccacggccagaggcctgtggcgcattcatgaggccctctcccgatgatccctgtcgccatcgaaagcctggaccccctgccgctgatcgccatcctgcgcggcctggagccggacgaggcggtcgcggtcggcgaggccatcgtcgccgccggttttcgctgcctggaagtgccgctgaactcgcccgagccgctggagagcatccggcgtctgcggcaggcgctggacggccgcgccctggtcggcgccggcacggtgctgagcgtcgcggcggcgcgagaggtcgcggacgccggcggccagttgatcatctcgccaaatgcgaacgtcgaggtgatccgtgaggccaagaccctgggcctgttgtccctccccggcttcttcaccccgtccgaagccttcgccgctttggacgccggcgccgacgccctgaaactcttccccgccgagatcgccggccccaagggtctgaaagccgtccgcgccgtcctgcccgccgaaacccgcatctaccctgtcggcggtgtcgaacccgacagcatagccgattggcgcactgcgggcgcgtcgggcttcggcatcggatcagcggtgttcaagccgggccagcccccccagaccatcggagcccaggccgcccgcttcgtcgccagatggaccagaccctaaggcctagctatcgctatgtgttagagcgggacgacgtctccgttcaagcgaaccgagagctgctgtcagtccaacgctaacttgtctccactgggcgcacacctctcctgcccgccagccttcaggcggcgagcgccttccactcggccagtgcggccgagcgtcgagctttgaagtgatctcggctgatgaggtggcgatccagattgaagtggttgtggaaggcggcgtgaacggcactgaatttctgcagggtcttcatctggcggaaccgctgcatcgcccgttctcgtcgtcggaacggaaggtgggagttctcgacgcggttgttgagccagcgccccgtctcctgtttcccggcgccaccgatctgcttcagagcggcgctgtaggaccgcaatccatcggtgacgatcgccttggccggtccgtgccgccgcatcgctttcttcaggaatttcagcgccgcggccttgtcccgcgtcctggtgacgaaggattccaggaccccgccctcatgatcgacggcgcgccagaggtagtgacgctcgccgttgatccggacgaacacctcatccagatgccagcgccagtgggtgaaggatcgcatggcctggacccgcttcctccggatttcgccggcgaacatcggcacgaaccggttccaccacagccgcacggtttcgtggcagatgtcgatgccgcgctcggctaagaggtcctcgacctggcgcagtgacaacggaaaccgcacatacatcatgacgacggtccggatcacctcaggcgagctgtcgaaccatcgaaacgggttgtcggatttggccatcaggtcaggctatccgacccgatcaggggagcaacccgtttgggctgacaagaccgcacctggtgatccgacgacgggagcgaaaacagcagaggttcaaatcccaaggatcagcccagaggttcctctccacacacggaccaatctacaacgcctttaacctccagccccacctgatctcgcgacctagccttcgcattctgcgaggccacgccgaggccgcttgggcggccgcgacccaagcggcctgaaccgggtcagggaaagggcgtactgcggacgtcgcgacttaagttgtcagttccaataaattggcggtggcggtgctgtcagtccaacgctaacttgtctccactgaacgcactcctcccctgctcgtcgctcttcacccggcgagcgcctgccactcggcgatggcaaccgagcgtcgggctttgaagtcgtctctgctgatgaggtgacgatcctggttaaagtggttgtagaaggcggcgtggaccgcgctgaatttctgcagtgtcttcatctggcggaagcgctgcatggcccgctctcttcgtcggaactgcagatgtgagttctcgacgcgattgttgagccagcggcacgtttcctgttttccggccccgccgatatccttcaaagcacctctgtgggatcgcagtccatcggtgacgatcgctttggccggaccgtgccggcgcatagcttttttgaggaatttcagcgctgcagccttgtcgcgcgtcttggtgacgaaggattctaggatctcaccttcatggtcgacggcgcgccagagatagtggccttccccgttgatgcggacgaacacctcgtcgagatgccaccgccaatggatgaattggcgcattgcctgaacccgtttcctgcggatctcgccggcgaacatgggaccaaatcggttccaccaaagccggaccgtctcatggcaaatatcgatgccgcgctcggccagaaggtcttcgacctgacggagcgaaagcgggaagcggacgtacatcatcacgaccgttcggatcagctcaggcgagctgtcgaaccatcgaaacgggttgtcggacttggccataaggcacgctaaccgacccgatcagaggtgcaacccgtttgggctgacaagacctctggacgaaatggtctgttggatcggcggccgacggatgtatctgtggcgcgccgtcgatgacgaaggcgaggtgctcgatctcgtcgttcagcgacgacgggatacggaggcggcgctgaagctgctaggtcgcttgcttcgaaaccagccgatcaatccggaaaggatcatgaccgacggattggcgtcatacggcgcggcgctgcgagagcttggcctggctcagatccaccgaccgggccggctgcgggagaacaaccgggtcgagaactcccacctgccgatccgacgacgagaacggcaacaaaagggcttcaaatcccaggcctccgcccagcgattcctcaccactcacgccgcgatctacaataccttctacgtccagagacatctaatcagccgccctacccttcgtcgcttccgcgccgaggcggatgccgcgtgggcggcggctgtcgcctagatcggatccggttgggcgtattttatccgcaggcggctaagctgacagcacctgcgcgatagtgctggttgtggcctaacgaaggccgaggttaaccggatcaaggccggtgcagccaagcctgcagccgagccttgggtctctacaagtagcacaggtgtctggtagtcgccggcgccttttggccgcagcagttgatgtcgcttaatcgacggcgcgctaatgtctgcaatgggtcggaccacgacatcgacaccagcgctgaaagtggatcgacctcaaagcccaaaagcggtcgcgccaatatgccgatacggatggaaggcggacataaagatgaaacacggtccggagagcagcatttcctcagcgtgtccggcctgaggactgacggctctatcagcccgtcacttttgcatgatttttttcaaaagtgagtctcactgaacgggcgatattgcccattctaacttgttcaacgatccaagcatcgatgtccttgccatcttcccgctgaagctcaactcccgcgtttagcattcgggtcaggtacaccgcgctgccgtagttgacgctggagatccattgacgcatttcaagaacctgctcggcaggaatggtgggacacgcttcaggctgtaccttcatatgatgttcgagatggtccatcagaagtgcaaaggcttctgtcagattgtcgctcatgcagtcgcactctttagctagtttcgacgagatcgtgtccttctcactcttctctgacaagaaacataatctcccagcgctgtcgaagaaacttcgatagttcagctgtcctaactcgaggctggtctagaacgtccgcaatgggtcgatttcgttgaaaaaggcgggctcgggcaattggcataatgggacgtcgctgattcactctggttgttgagacgggaggttcagcgatgatgggcgagcggcggtgacgtgatggtgtggacgacctccgcctgacgggctgttctgggtgtgtcgtcatcagggacgtcatgtgtggacgacctccaagacgcaagagtggaaacgacgttggcgctcggtcgagtgcagtcatgtgttcggcctgttgatgcagctgtttgcgctgctggccctgatgaagtccgcggaccggctccctaatcacgtcaacgcgctcgaggcgctctgaccccctgggtttcaccgatccccggctgcggccggttcgtcatcacgtctcaccactccttcgtctacggcgccggtcctgggtgaagaccggcccgatctctatgccgctgtgggcttgtagtcctcctgtcgcgccatcagggtccaggcgatgcgagccgtcttattggccaaggccacggcggcgaccttcggcttcttgcgttcgaggagattgccgacccagccctcgcgtcctcgctgccgggccattcgcaggaccgccgtggccccgacgaccaggagacgtcgaaggtagctgtcacccatcttgctgatgccgccctggcgttccttgccgccactgctattggcccgcggcgtgagtcccagccaggctgcaaactgccgaccggaacggaagagactcggatctggcgcgctggccgccatggcgctggcagtgatcggcccgatgcctgggatggtcgccagtcgccggctcgtctcatcctgccgatgccaatcgagaatccgacgctccatacggctgatctctgcgccaaggtgttcgagctgttctgccagcccgccaagcgcggcatgcgccagatccggcagggcctgaccctcttcacgcagactcttcagcgctgcccgcaccccagctggaccttgaggcgcgacgatgccgaactccccgaggtggccccgcagtgcgttgatcagcatcgttcgctgacgaaccaggagatcccgggtcttgtgcagcatcaacaccgcctgctgggccttcgacttcacagccacgaaccgcatggtcggccgggtgacagcctcggcaatcgcttcagcgtcggcggcgtcggtcttgccgcgcttcacataggccttcacgtacgccggcggcatgagccgaacatcgtggccgatcgccatcagttcacgcgcccagtggtgggctgaggcgcacgcctcgatcccgatcaggcacggcccaatcgactggaagaaggccagcacctggccgcgccgcagttgccgtctcacgacgaccgtgccgtctgtggctacaccgtgaacctggaaaacagtcttcgccagatcgagcccgacgacagcgatggtctgcatgataccgctcctagacgtgacgtccctgatgacgacacacccagaacagcccgtcaggcggaggtcgtccacaccatcacgtcaccatcagaccccacacagcccatgctgccagcgcgcccatcacggccacggcgacgcctgcgaagacagcggccacgccaaatacacgcttcaggaacacagccactttccaccccttcgctctacgtgagccatcacagggcatccggcggatgtctgcaatccaccccctccagccatcggcagcgtccgcttttcggccttgaggcgcatgccctgctctgcccccttgccgatgttgtccggcccgtttcagatgatccaaatgtccagtcgagaatgaccaaactgaccattcaccacaatagctgcacagctgaacaaccttggagcgttcgtatgcagcgtcaatataggtgggcttctaccataacccaaacgacagccgccttgtcgtacctaagaagatcccggcccttgggtggactgtcaacatagccaagccggaggcgaagttggctgtagcgctcatcgttctggtagctgttgtcggggttgcggcgctgtttttgatctgaccttcaaacaggcaggcgacagcagttccacttgccaagcccacgacagatatcttcgtctatagcgagccgagcgtccgctcccacccttgcacgagatcatcctcccgccgagcatctggttgtttctacaccgacacgacggccagccgacgctgtctccgcctcgcccagacggagactcatgcccatgagctgcggctggcggatcgatcaacaccagtggctcgcgacgctccagaagacgatccgcaccggatcgggcttgccgcataagctaaacagcggctctagacggccttgccgacggtgtccgccacgaccgctccccgcgcgccaaggggttgcggagcgccaatggtggtgtcgcgcgccgtctgatgttcgatttctgagttgagctcggcgcccagcaggaagaccatgctggacagccaggtccaggtcatgaagccgatcgcagcgccgagcgcgccgtaggattcgtcgtagttgccgaagttcgcgacgtagaaggtgaagcctcccgacatcgccacccaggcgatggctgagagaccactgccccaggtaatccagcgccagcggacccgatcgcggctcgggccgaagcggtagagaagggtcatgcctatgaccacgcccaagaacagccccagccagtagatgactgtatagacgccgccggccagggcgccgaagcgcgcgctcacgccggctccgaacgcgcccagtccaatcgccgtgatcgcgaaagtgatcagacccagggtgaaggccagcgggacgagcgtcttcttcagcaatcctcgtttctcctcctcctcataggcgatgttcaatccggtgatgatggccttcatcgcgccgtttgcgctccacagcgcagtcccgaggccgagaataaaggcgaaggacaggccgccctcccccgctgcggcgaccttcagcatctggtcgccgatcaggctgatggcgccggcgggcagcaccccagacatctcttgaacatggctttgcgcctcggcgacatcggcgaacaggccgtagagagcgacaaacgcggtgaccccgggaaagagggcgagcagtgtgtagaaggtgcagcccgccgcgatcagcgggatctggtcgtcaccgaactccttccacgtccgtacaagaatgtccttccagccccgcgccgggatctcgctgggacgctctgcgtcacggccgcgaccgggctgattggcctcatggaggttggcgggcgacgcttcgcccttcgccagagcggcgctttgttcgtccggctgacgaaaccgattacgccgaacccttggcgcaacgcctctgacgagttcagccgtcgcggcgcccgcgagaaaactggcgccgagttcgaggatcttgcgcatccgcccccctgttggtgtccgaacggaatgagacgggacgcggtccgttccgccgaccgcccgaaactgattgcccgctccaccccgttcaaccgcccggatcggcgggccagagcgctcatccagccgttgcagatcggctggatgagtgtcggttcctccgagcggcggtgtccagccgcatcgctacagctggacaccgcttcagaagtttcctgggctaagcgggagcatgctcgccgctcagcctgaaccgattacaggcgatcggtcgtagagcgtccgtcctcgtcgatgtcgacctcggtatgacgcaccgtgtcgttgatctcctcggtgcgctcgccgctcgtcttggacacgacgacctcttcgactacccgcgcctccttggctaccacggcctcttcgctgctcgcggtcacgtcgacgacccgctcgcggaaggcgtcgccgtccactgcggaaagcggctggtcgaccgcgcggcgctcgacgttgatgcgttcctggcgcaaacgaacctgctcgtgcaccggaacctcggagacgtaggaccggacgcgaacgccgccacgatcgacttcgcgcttgccaacgaccagttgctcttcgacgatggggatcacgtcttcgctgacgttgttcgcgcccgccgtcgcggcgccgcccgctacgcctagcccgccctgagccggatagtcccagccctcggcgcgccaggactgtgtacggtcgtccaggtcgatggagttcgcctcctccagcgctcgcactgcgtcgtcggccttgtcctcgtccacgtcggccgtcaccaggaagccgccgcggcgcaccccctcttcataggcgtgacgatcctcgtcaggcagaaaggcgttcttgatcgaggaccagaggccacggtcttcatgattggagtaggcgccgctcgtggtgtgcgacgactggtcgtggatcttcacatgatcggcgtccaggccggcctgatgaagacgctccacgccggcttcggcgtccgagcggctgtcgaaaagggctgtgatcgtgcgtgtcatggtagtctcctgaggttggaagtgatcagcgttgggtgacgacgagttcggtccggcggttctcggcctggcccgtcgccgtggcgtttgtgccgacggggtcctgctctccgcccgagacagcctcgatgcggccggcctcgacgccctgggcgacaagagcggccttcaccgcatcggcgcgcgcctggccgagcgtgacattggcggcggtggagccacgcgcatcggcatagccggcgatgcgcacccgtgttgcgggatactgcttcagtgtagccgcgatggaggcgatttcggctgcatcagcagaccggatctcgctctgcgaggtctcgaagttcagttgctcgaacgtgaagctctgcggagcgggcgcagcgcccgccaggtaaggccccaagccggatgttccggcaagaggcgccgatgcgcctgcattcggcgtagccgccacgacctgcccgccggggggtgcgaccgtcgcatccgttgcagccgcaggtgcagctgcaacaggggcttcctcatcacgtccgcagcggctcaacgcaaagagcagcgccaggagccccagcgccagcaggatccagggcaaccagttccgcttctttgtctcgatatggacgtggctcggcggcgcgccgcccgtcctcttctctggctcggccatcagtcttccttttggtgttgatgagatggatcttgctcgacaacggcgcgggttgagcgaagactgaccggcacttcgatctgctcggtggttgtggtgtgacggatcaccacttcttcgatcacgaacagcgcgcgcttcaggaccagccgctcttccacaagggaaatcacggtggcaccgtcctcgccgcgaggcggcggggcggacggaacttcgcgttccacggctcttcgttcgacactgaggccgctgcgctccaggctttcggacagcacctcgtcacgaatatcggtcaccgtgcgaacccgcacgtgtccgctcgggaccagccgtttgctgatccgcgcctcttcctcgacgatcggcactcgatcttctggtgcggagatcgaagacatcagaccgcgtcgactctgaagcagagaccgacctcggcacggctcatcaccaggccactaaatggctgttgagacagcgcaggcattgtgggcacgctcccgattatgttctgcacatcgcaacattcaggggcaataacgactgcacaggcctgctgttccgtaaattttggcgcgatctacataacgccgaaatagaacatttgctgtagcagtacatatactcaagctatcggcattcagcgcttaccgtgaagctcgggaaaccggtgtttgatccctccgctgcaaagccagcggtcacgctgcatcaagcaagagctggaggagcgcgcactgcgagcagtctccgacgaagcggtctgggcggctttggggcggaccagaccgcgcggtttgcttgaagccgcttcgaggcgttctggcgggcttttagcggctgagcggtgacagcgcgtagtctgcaagcagcgctgcgacgtcgtcgtaaaccgccacggcgccagccgcttcaagcgcgtcgtccgagaacccgccggaccgcaggccgatcgcggcgatgccgcactttcgggcggcttcgatgtcgtagggcgtgtccccaacgacgatcgcatcgggagctccgaagggggcgagcttcttcagcgcggtttcaaagatgtcgggcgcgggcttggtatgcttcacgtcgtcggcgctggtggtcgcggcgaccagatcacgcacctccagcaggtcgagatagtgctccaattcggcctctgacgccgaggaggccagcaccaccttctgacctgcctcatgggcgcgcatcaggagatcgcgcgcgccggggaatggcctcacctcgtcgaggtaccggctcttgaagatcctgccgtgcgcttctccgaaggccttctgatctgcgccgctggcctccggcagcaaggcgggaaccagcatgtcggcccctttgccgatctggtcatggatggtctgccggtcgaaggttgcgccagcgtcgcggaacacctcctcccacgcgaggacatgctgttcattgctgtcgacaagcgtgccgtcgatgtcgaaaaggatcgccttgcaggccatgcgtcatccacgtgatcgagctggagcgccgcacaggggagtttgcgctgcgccttcttgtctcgacagcgaccgtggcctgataacgttccgcctctgcccgaacgtcggcgagcgctgatgcgaaaagcttcagcgaagcgcgtcagcttcacgcaggtcctgcactcggcggaaccatcatgacgacgctctgttgctcttgtcgctgcaagaggaaccgccgcatgcttgctatggactatcgcggaccccgtcgtattcgcgtcagcgaaaagcccatgccccagatccgccacccgcgtgacgcggtcgtgcgggtcacccggtcgtgcgtctgcgggtccgatcttcacctgtaccacggcatggtgccggacacgcgcgtgggcatgaccttcggtcacgagttctgcggcgtggtggaggaggtcggtcccgaggtcggcaatctcaagaagggcgaccacgtgctggtcccgttcaacatcgcctgtggccagtgccacttctgcaagcagggactgttcggcaactgccacgagtcgaatgctcaggccacggcggtcggaggcatcttcggctattcgcacacggccggcgggtacgacggcggacaggccgagtatgtgcgtgttccttacgcagatttcggtccaacgctgatccccgattggatggatcccgacgatgcggttctgctgaccgacgttgtgccgaccggctaccaggcagccgagatgggcggcattcagaagggcgacaccgtggtcgtcttcggcgccggtccggtaggacttctggcggcgcgttgcagttggctgttcggcgcagggcgcgtgatcgtcatcgatcatcacgagtatcgcctcgacttcgcgcggacctattgcccggcggaggtctacgacttccgcgagatcggcgatccggtcgtgttcctgaagaaggcgaccgggggccttggcgctgacgtttgcatcgacgcggtgggcgccgacgcttcggggaacgcctggcacacgctcttcggcaagaagttgaagctggaagccggcaacgccgtgcctcttcattgggcgatcaactcggtcaaaaagggcggcgtggtgtccgtggtgggcgtctatggcccgaccggcaatatggtcccgataggcaatatcgtgaacaaaggtatcacgcttcgcgccaaccaggcctcggtcaagcgcttgctccctcggctgatcgatcatgttcaggcgggacggctggatccaaaggcgatcatcactcaccgcgtgccgctggaggaggtcgccgaggcctaccacctgttctcatcgaagtccgatggctgcatcaagccgcttctcattcccaacgccggctgatcggagagcttcaaagatgacgcaaagcacccgagccgaagccgccgccgaaacagcgcaagcgctgatcgaccctttcaccgtttcggggtggggcgtggacgccgatccagagaacgatcccacctggcccatgcgcgaccgttcaaaagacgacggccccgggatgaactgggatcgccctgctcttcaggcggctgaggtggagatcctgcagtccgtggagcatgttcgccggccggcaagcgtgggcgagtcgaccccgccgcacggtgtcagcggaaggatccggcggcaggcgttcgccttcagcgagagccagtggggtcactggttgttgctgatgctcgccgaccgcatcgacagcgtcgagggcgtcgtcgacgatctcaagcgcggcaggttcccaaacctacttgtcgagacgggactggtgaaacgggcgcggtcgcgcgaagccgccaccgtcaccgctatcgtggtcgcaggagcagccctgggcctgctcctgctggcccgcaagcgacggtagccgtcagctcggatcgatcctggcgacagcgccctctaccgccccgacgatttgaagggctggctcagaaaacgggactcggccaagccgaagcgccagggcgtctccacgcccttgtgtatcccgatccttgagccctgcagcacctctggcggaacgacgggcgcttgaagctcgaacggagccgcggccagattggcagtgtttagctgtccgtctatcgccgatttcgttgaaaaaggcgtccgttggcaattggcatgaaggcggcgcgctgattcactctggtcgttgagacgggaggtgcagcgatgatgggtgagcggcgggttgatcagtcggcgctgttctacgagttctcgctggagcggcatgtgccggcggatcatcttctgcgggcgatcgaccggttcgtggaactggacggcctgcgggcgcatctggcgccgttctacagcgccatcggtcgcccctcgatcgatctgatcctccctcggtttggtggacacccatgctagcttttcggagctggagaggagtgtctgatgagtgttcaacgccggaactttccggattctttcaagcgcgaggccgttgaccgcgtcgccaacggcggcctgagcgtcggggcggtggcccgcgagcttgggctgcacgagacggtgcttcgtcgatggatgacgcagttcggggtgcaggcgacgggggcgtcgcggcgccccacaacgcaggcgtcgtccccgtcgccgtcggatctggcggcggaggtggcccggttgcggcgagagaacggtcagctgcggatggagcgggacatcctaaaaaaagccgcgctcatcttcggagcggcctcccgatgaagttcgggttcgtcgatgagcatcgtcaggtctggccggttcgcgtgatgtgcgcggtcctgggcttgtcggccagcggttactacgcctggcgcggtcgccccgagagccagcggtctgtcgccaatcgcgagctgaccgaggatatccggctgatccatgcggagagcagcggctgttacggctcgccgcgcgttcacgccaccctgcggcggcatgggcgtcgggtcggtcgatcccgcgtggagcggctgatgcgccgcgccggcctgcggggcttggcggccttgccgcgtcgcgcccggacgacgaacagccgccacggttatcccatcgcgcccaacaggctggcccggaacttcgaggcggcggcgcccaaccaggtctggctcgccgacctcacctacatcccgaccggcgaaggctggctctatctcgccgccatcctcgacctgcacacccgcaagatcgtgggctggtccatgcgccagaccctgcacaccgagatcgccctcgacgccctcaacatggccgtcgaacgtcagcgccccgcgcccggcctgatccatcattcggaccggggcatccaatacgcagccgaagcctatcgatcagccctggcccgatccggcatcaccccgtcgatgagccgaaagggcgactgctgggacaatgccccgatggagagcttcttccacaccctcaagaccgaacgcgttcatcaccgcgtctacgccacccgagaccaggcgcggcgagacctgttcggatacatcgagggcttctacaatccccatcgcctgcactcagcactgggctatatcagccccgctgaggccgagcgcaaagcggcttaaccccgtccacttttacgggggaagatcaagttggttcttcaggcgatgggagagttcgtcgttgagcagacgttgctgacgttgcgcctccgccaggcgcgctgcttcggccaacagcgccgcttcctttgcctcccgctcaagatcgatgaggttgcgtcggtcggcggtcgcatggaggttcttgatgatccgccgcagggtataggcgatcccgatcagcatgagcatgaccaggctgtagaggatcgtcgccgcccatcggtcagcatcgacgctcccctgctccatctcataggagacaagcgtagcggccacggacaggaaagcgccaaacagcccaggcgccgcgcccagcatcagggtcacacccagcacggctggaatgtagaacaggaacggcaggaagagcgcaccgagcgcagcccgcgcgacagcgacgaccaagatgatcaacgccgtcaacagcagtcggcgaggcataggtagccggagcttcaacgaccagacgagagcctgctcgagagccgtggacgtaatggtgaacggcatagctctgcggagatgaatggcgcccttccacgggccaggcgtaggtatcagatcgctaaggctaagcccataacagccctccaactgttcctggttgacagctggcgggtcctcaacctcaccctcgccaatcacgccgccagggcatccgcccacgcactctccctcttccaggcagtgtctggccgccgccgccgggacgggcctgcgagcaagttgagaacgtagagactgaggctgacggcgcttttcagccacctgcaagaaaaagccgccgctgattgtcagcggcggctccggcaagggccttcagtgcgcgtggttcgactgcgcttgcgaacttggccttgcatgtgcctgcatctgactgatctcgtgctgctgcgtctgcacgatgtgctgggccagctggcgcagctctgggtcgtttccgctttccagataggtgttggccatgtccacggcggcctggtggtgcgggatcatcagggcggtgaagtcgtgatcaagatcgcccgtcacctgcacggcgttggtggcgtcgtgcatgtgctgcatctgcgccatcatggccgcagccgctccggcccccggcgcgcgggtggcgcccgcttcgccgtggtagtgcgtctggccgcgccagaaggcgcccggggctgctcccgtttcaggatgcctggacgactccgcccgcagcagggtcgcgacatgctcgttgctgctttcgtagatgaggtggtgcaagccggcgtaggagcccattgtcaccgcgagcgcaatggcgaggccggccggcacgaacagcgcacgacggcgacgcggagcgatctccagcgcctggtcgcaaagcggatcggcgatcaccaccagcagagccgcaaggatggtcgcatgaccaatcagatcgacgcggccgaacggataaacggcggcgaacataagggcgaacagggccaccgccgagagacgccggatcagcggcgaccacagcagaccgaagcccagggtgaactcggccacgccggccatggtcgtataggggccgaacggcatgccgaaggccaggaacggcttttcctccagcagcggcaggaaccactgcgggtacatgaacttctccatgctcgaccaggtcagcgccagggcgatgccccagcgcagcacggcgaagcggcggtcatgccacttgccgtcgggcaggcccgacagcagcagatagcccgcgatgccgaggcccaaggccagatagtcgaacaggtggaacaggtcgtagctgccgatcgtcagcacccacagcagcacgatcatcgccgccgcgatcgggcgcgtgcggcgcgcgacgatcagcatggcgatcacaagctgcatccacgggacccaagccgcatcggtcttgagctcgggtgtcagaaaggtgccgcccatggcgaacagggccaggaagaaggcgcacagcacgcccaccagaaagccgtcggcgttcttgctgatcagggacgtggccttgtcgagcccgcccatgacgacctgccccggccgcttggcctcgaagaacgaggtgaccaggaagaagcccagcaccagtgcgatcccgacccagaagaagggcaggctcagcgtggtctggatcgatacaggcttggccgagacctcataggcctcgaaccatttgacgtgcgcataggcgatggagggaacgcccagggtcaccagggtaagggcgttgcgggtgatcttggagcccagtcggggcggcgggaaggtcgccggcgcgcgggcgagtgaagttgggaacatcggttcagccttgtcatgccgccgatcacagaggcgccggcggtcaccctgtccctaggccgtgaggggaaccgccggtattcggatgatcgccctagccgtcgccccctaaggggtttcccggaggtcgcgccggcgtcagcccagcgaggccagcgtggtcatgcgcaccaggtcggacaggctcttggcatgcatcttcatcatggcgttggcacggtagacctccaccgtgcgggcgctgatgtcgaggtcaaaggcgatccccttgttggcgtgcccggccaccaggccgtccagcacctcgcgctcgcgcggcgatagggtggcgagccgttcaaggattgtggcgcgctccagcgcccgttcgtctcgtccggcctggcgcgcgagcgccgaacgaatcgcatcgaggatggcgtcatcgctgaaaggcttttcgatgaagtcggagacgccggccttcatggcctggatcgccatcggcacgtcggcgtgtccggtgatgacgataaccggcgccgggcagccgcgcctcgccagctcggcgacaagttcaatgccgttcatgccgggcatcctcacgtcggtgacgatgcaggcgtgatccagcgcggggctggccgccagaaaggcgtcggcggaggggtggccgcgcaccttcaggccagcgcagtcgatcagaaactccagcgaatggcgcgccgcctcgtcatcgtcgatcacgtgaatggtcggctcagtcgccattaaaaagttcctccttgccgatgcgctgtagcgtaaagcggaagacagcgcccccgccatccttaggctcgacccagatacggccgccgtgcgcctccacgatcgtcctgcagatcgacaggccgacgcccatgcccgtccgctttgtggtgacaaagggctggaacagctggtcggcgacctcagggctgacgcccggccctgtgtcggacacgctgatgagagccgtctcgcgactggtcggcatggtcgcgatgacaagctctcggcggtccggctcggcctcggtcatggcgtccaccgcgttcctgacgaggttcagcaccacctgctgcacctgaaccttgtcgaccaacacgaggtccacgtcggggtgcagctcgaactggacgcggatcccatgctcgcgcgcgccgaccagggccagtgcgctcgcctcctcgatcagcttgggcaggctctcgatccggcgctcggtctcgcccctggacacgaagtcacgcaggcggcggatgatctcgcccgcgcgcagggcctctgcagccgcacgatccacggcctccgagatccgctccagcggcgcctcctctcgcgccagcagcatgcggctgcccttcaggtagttggcgatggccgacaggggctggttcagttcgtgcgccagggcagaggccatctcgcccaaggctgtcaggcgcgagacatggaccagctccgactgcagctcctgtagccgggtctcggttctctgacgctcggtcaggtcgcggatgaagccggtaaaataccgccggccgtcgatccgcatctctccgacggccagctccatcgggaaggtggagccgtcgcggcgttcgcccaccaccacccgtccggtgccgatgatgcggcgctcacctgtgttgtaataccgctggagataggcgtcgtgcgcctcccggtacgggtttggcatcaggaggttgacgttgcgcccggcggcttccgcctggctccagccgaacaggcgttcggcggcggggctgaagtcctggatcagggcggcctcgtcgatcaccaccatggcgtccggcaccgtgtccaggatcgagcgcaggtggatctcgcgccgcgccaggtcggcgttgaccgcctcggcctcgcgccgggcgcgctggaaccactcgccgccgacggagatcgaaacgccaaccaggaagaaggcgcccgccgcgatccagttgcccgcgccgattggcccccaggcaaggtcgcacagcacgccggccgccgcccccagggcgcttgcagccacgcccgcccgcaggccggacagggccgcggccgccaccacagccggcacgaagaagataaaggtcgctcgctgatgcagcgcctcgctgaagcccagccgtatggcgacgccggccatcacgatcaggagcgccagcccgacggccttgaacggcgacagccgaggcagcaggacccgcgcgggtccagccggcttttcggacaaatgcataggcgcaaagcctcctttggccgcagggcggtgtcgcctccggatctatacctaggggatgcgccgtggggagatcatccgaatgtcggctgtcgtggcgtcaccctaggttatgcgtcaaccctgtcaggcgccggcgatgttccgccggccgcatcgcccggagacggagatggaacccgcccgccgcatcatccttattgaaccggacatggcggtccgcaaggcgctgatgttctccctggggctggaaggcttcgaggtcgagacggttgatccgtcgcaggcgcttgatcgactggatgaggaggatgacgatgcctgcctcgtcatcgaccactacccctacaacgccgacgcgctgcagctgctgacgcgcctcaccggcggctcgagacgcccggctgtggttctggccactcacccggccaaagtgctgcgggagagggtgtcggcggccggcgccgtgctggtcgaaaagccgctgctaggcgacgtgctcaccgaggctcttcgcgccatcttcgaccagcctcgggcggcctgacatgcctcacgtttccttgaccgagcaggatctgcgcacggtcgtgcacgccttctacgaccgcgtccgccgcgatccgacgctcggtcccgtctttgaagacgccgtcgatgactggcctgcccacctcgacaggctgacggctttttggtcctcggtgatgctttccagcggccgctacaagggcgaccccgtgggcgtgcatctgcgtcatctggaccggatcaggcccgagcagttcgacctctggttggcgctttgggaccggaccaccgacgatctgttgccggcgccggccgccctcgcgctgcaacttcgggccgcccgcatcgccgacagcttgaagctcgccctcttcttccgcctcgcgccccatcccaacaaggccgcctgagatgaccgtccagccctatcgctcgtcacccgttttcgaccaggacaccccgcccgccgccctgaggtccaggcacaacgcgaaggccggcgtctgagggcgcatccgcgtgctggagggccgcttgaagctgacttcgctcgatcccgcgttcaaagccgtgctggaccccgacacgcccggccgcctgtcgccggaacagccgcactccgtcgagccgctcgggccgatgcggatgcgcatcgacttctatcaccagtcgccgaacgactgacccctctccccttctcgaacttaggaccccgccatgtcgcgcaggctcagcgaacgcaccatctctctcgtcaaggcgacagtgcccgcgctggaggcgcacggcttcgacatcacgcgcgagatgtacagccgcatgttccgaaacccggacatccgcgacctgttcaaccaatcccaccatggcgatggtggctcgcagccccgtgcgctggctgcggccattctcgcctatgcaagcaacatcgagaacctcggggccttggcgcccgcagttgagcggatcgcccagaagcacgtcggcttgcagatcctgcctgaacactacccctctgtcgccgaggcgctgctcggcgccatcaaggccgtccttggcgacgccgcgaatgacgagattctcgccgcctggggcgaggcctactggttcctcgccgacatcctgatcgcccgcgaggatcgcctctaccatgagcaggccgaggccgagggcggctggaacggctggcgcacctttgttgtcgaggaaaagcggcccgagagctgcctgatcacgtcctttgtcctgcgccccgtcgacggccgacccgtgcttcggcacaaggctggccagtatctgactttctggatcgagatccctggccacccgccactcaagagaaactattcgatctcagacgcgtccaatggcgaaacctttcgcatttcggtgaagcgcgagccaatgggcctcgtctctggatggttgcacgaagaggtcgtcccgggcgcggtgctgaaggttggggcccccgccggcgagttcttcctgcaggcccaatctggacgaccggtggtcctgatgtccggcggcgtcgggctcacaccgatgatggccatgctggagacgatcgtggcgcagcacccggatcttaccgtccactaccttcatggaacccaggacggcgccacccacgcgttgggcgctcatgtaaaggcgctagcggcgcagcactcgaatgtccgcgccaccaccttctagcagaccccgcgcccacaggacgaaatcggacgcgattacgaccgcgccggcttaatcgacgaggcttggctccgttccgagacgccgctcggcgaggcggactactatctatgcggccctcgcccgttcctgcggacctttgtctcaacgctgacgctggccggcgtcccttccgaccgcatccactacgagttcttcggccccgccgatgaactgctcgcagcctgaccgagacgacaaatcgtgtcagatcgagacaacaaacgcatcgacaggcaccaacgggatctcctgcgacgttccgggttatgaggaggcgatcagcgaaagcggttgctgacatgtacaagcgacgtgtcgccgtcgatgaccgacgcctcgaatcacatcttgcgcgcgatttgaagggccttgccactggcgtggttctcgatggaatcgatgaccgcgtagccgcgcgcccgggcgcggccgaccaggtgatcgagcagtgaccagccaaagccctggcccttaaggatcctcctcagcacgatcggggacctcagttcgctcggcttctccatcgcccgccagggtcgtcgtcgtcgccggagccgtgcacgacaaaggcgaacaggctctcgttgcagacaccgtctgcgcggatcagcgccacgaaacagtcgtggttgacctcgcgcagggtctgtagaaagcggcatcacaggccttccggtgtcaccgaagcgaagaaggtgccgggagcgccgcgatggaagccggagaagagtccccctcgccatctccgagccgccgaaagctggttccattgtcagcaatggttcaggtttggaggcttagcggttatccatggctgactaccgattgcacctcatccgcgacggcgccagaaccgaagagcgcctaggtggcgtggacgacgccgacgccttggcgctggcgcgcatctatgtgctggccgacagatccattacgcacgcgatgctgcgccatcacgacggacgcagcctcggcgacatcaagctcgactcgggaacgcctcccctgtcgggaggatcggagatctgactacagcgtccttggcgaaagtcgttgaagcggagaccgccagcagggcggggttcgttgggtagatcagtctttgaacgttccacttgtgcagagcttcggtgctcccgacgaaacagggactgggcgtcctgagggggttattctcgcgcttgctcgctgtgacctccgcgtcgctgagcgtcgcctggttcgtttggcgtttcggcaggatgggccaggacggcggcgtaagtgatcgtagaggccgaggccgtgcttagcagtcaaaggcaggttggaaggcgcatggatcctccgccgactggatagacgcgctgaagcgctgctaatctcagggccgttcatgtacccacttgaggcgcgcccgccctcggcgagggccgtccaattgcgtctccaccagacaccactgttacgctggcttggttcgcaccagctcggcacgaagtggcaggttgaacgaggctccatcacccccagagcagttgatcctgcacccgcttgaacgccttggaaacctatcgaaaaggtgtcggctgcgtcccagatgcgtcccaaatccaggggtccacgtgagtcagccgactaagtcattgattttatggcgaccccgggaggactccaacctccgacctcggctttaggaaagccttgctctatgcagctgagctacggggccacgcggcgtccacgtagcggttcgggggcgttcggggaagaggcgccgcagaaaagcgctttccggccccgccttgtggttaaggcggcggcttaacctacaccatatggcggtgaacagggacggaaccgcgcgatgtggccgattcggtcctgattcgtttccctgtcgttccgccgcggcgggcgcggcgttaactctctgcaatgtgcgcggacacagcgcggaggccggcgagcaactgggcgctggcttcgctgacgcggcagccctcggccaggatcagcgtcagggcgcgggcgtgcaccgcaacggccggccaggaccaggcgccgcgctcggtcatgcggtccgagatgtcgcacaggctataggccgcctcgtagaagggaccggtgtcgatgaagcccgcgatatccagaagcgccgtgccgagggcgtagacctgcggctccgtaccgggcgcgcccgcggcgcagagggcgtccagccgctgcacggtggcggccagggtgcgcagcgcctgatcccgctgggcggccagggccgtgttcgccatgcgctcggcctcgcccacggtgcggccgccgtcggccgaggccatctggcgagacaggctggagcgcacgcgcaccatcttgggcgggcgggccgcgctcacagggccacccgcgtgggtctcatcagcatgtcgatgtccgactggtccatgttggcctccaccgcctcgccgagttcaccgctgagatccccggcgcggcggccgtccatgccggcggggggaccggcgttgcgcacgcggcggtccgggccgcagtaggtgtcgcagtccacgaactcgcgttcgtcacggcccagccacaggatgcgctgaagcaacacggcgggcgtcagcggcttggcgaccacgaagctggcgccgcagtcccggctcttgtgcacgcgcgactgggccgcgtggccggtcagcatgaccacgggggtgtagcgcatcggctcgggcgtctcgcgccgcagccaggtgatgaagtcatagccgtccatgtccggcaggacgcaatccaccaagatcaggtcgacgggccggcggcgcaggatctgcgcgccctcggaggccgagccgcacttgatctgctccttgaccccgaagccgtggaagatcgaactcagcatgtccagcgcctgctggttgtcgtcgatcagcagcacgctggagtggctgaggttgatgcggtcggagggtgcgggccgggacatggccgttctcggtcaaaaaagttgcaggtcgccggaagcggctgaatcgggcgcggcgtcatcggcctgacggcgaacggcggggcgcagacgctgggccatgtcggacaacgggatggccgccacggccagctccggcggctcgcctgcggcgacggcgcgggcgaggccggacagggcctgaagacgctgggtgatctcgtccagtcgctgggcgtccgacatcacctccagccgctcggccggcggcacgcggcggacaaggtcgccgagcagatgagagatggcgtccacgcccgcgcggaggtcctccagttcgtcggcgacggcgtccagcagggcgggatcggcggccggcatcagaacagctccagcgcgccggtgtcggcgggcggcggcggaggcggcgcgggccggggcgcggcggcgtccgacaccgtgtgctgcagggcccggcccgacaccggccagtagtgcagacgccgaccgccctcgccacgcaggctgccgccgaccaccgaaatgccctcgtcgcgcaggaaacgctctgcgaagtcggcgttggcgcggcctacgtcgcgtagggagtcgaacatgcgcccgccgccgaacagcttggcctccagccggtcgcgtcggccgccgcgcttcagcacgtcgttgatcaacagctccatggcgtaggcgccgtagcggcggcccgcgtcggtgcccgctccttcgccttccggcaaaaggaagtggttcatgccgccgatccccgcccccggatcgcgcaggcacatggccacgcacgagcccagaatggtgctgagcatcacatgcgggtcgtcggtgacgtagtgctcgccctgaccgacgtggacgcggcgctccagcggatcggcggcggcgatcatgtcagaggcccgaacacggcttccagcttgtccttcagctgctgcacggtgaacggcttgaccaggtagttgttgacgccgaactgcaccgcgcgctgcaccagctcgcggtcggcgcggccggtcagcatgatgaaggcggtcttggatgtcggcggatgggcgcggatggcccgcagcaggcccagaccgtcgaggttcggcatgttgaagtccgagatcaccaggtgggccggcttggtcacgatctcgcgcaggcccgcctcgccgtcggcggcctcgcggatgtcgcgcatgccgatctgctgaaggctggtgcggaccagcgaacgcatggtcatctggtcgtcgacgaccagaacgctgatggcggaggcggcgggcatctacgcggtccttgaggcggggctctgcgcggaggcggcgcaggcgtcgagaatggcgggggtcagacggtgcagaggcagctggcgctccaccgcgccgatctcctgcgcggcgcggggcatgccgtagaccacggaggtggcctcgtcctggcccagggtgcgggcgccggcctggcgcatcgccaggaggccctgcgcgccgtccttgcccatgccggtcaggatcacgcccgtcatcggccgcttcagcacggcgaccgagcggaacaggacatccaccgaagggcggtgaccgttgacgggatcggtgggcgacaggcggcagcgcggctgggagccgccggagacctccaggtgcgcctctccgcccggcgcgatgtagatatggccgggtatgacgggcgcgccgtcctcggcttcggtcaccctgggggcgcagaccttgtcgaggcgtgcggcgaagctcttggtgaaggtggccggcatgtgctgggtgatgaccgtggcggggcagttggcgggaaagccgctcagcaccgtcagcagcgcctccaccccgccggtcgaggcgcccatggccaggacgccgcgcggatccggctgatagccgatgggcgccgtcgccgttgcatgctcgccgcgcggacccacgcgcgagcgggccgcagccttgaccttggccgccagctcgccgaacgcctcgggcgtggcggaggcgggcttcgccaccgcgtccaccgccccgatctccagcgccgccagggtcacgtccgtgccggccgccgtcagagtcgagaccatgaccaccggcatgggccgcagccgcatgatcttctccaggaactccagcccgttcatgttgggcatctcgacgtccagggtgatgacgtcggggttcagggccttgatggcggcgcgggcctcgatcggatcggcggcggttccgaccacctcgatctcggggtcgcgattcaggacggccgagatcaggccgcgcatggtcaggctgtcgtcgacgacgacgacgcggacgggcgcgctcacagcgaacccgccgtcttgtaggtcgtcaggccgcaggtctgcagctgcgccgaggccggaccggacacccgctcggaatggccgatgtagagggtcgcgcccggcgtcatcagcggggtgaagcggctccacacccgctcctgcgtggcgtcgtcgaaatagatcacgacgttgcggcagaagatcacgtcgaacttgccgcgcatcggccagtcgccgatcaggttcagttcgcggaacgacaccaggcggcgcagctgatcgcccgcgctccaggcgccgcgctcgtcggctcggtcgaaatacttgcgccagagtgtggcgggggccggctccagcaggtcttcggaatagacgccggcatggccctgggcgaccatgttgggatcgatgtcggtggccaggatgcggacgtccaggtccgccgcctcgggcaggaccgacagcaccgtcagcgccatggaatagggttcctgcccgttggagcaggcggccgaccacaggcgcacgcgtcctccggcctttgcgcgccgggcgagcgccggcatgacccggtcgcgcaggtcgtcgaaatgatgcggctcgcgatagaagcgggtgacgttggtggtcagggccgccgtcatggcctggcgctcgtccaccccgtccgcgccgtcgaccagggcgcagtattcgcgaaagctgcgtaagcccagcacgcgcagccgcttggccaggcgcgaatagaccagcgcggccttgccctcgctcagcgcgatgcccgagtgggcgtgcagcatggaggcgatatggcggaagtcctcggcggtgaagacgaactcgccttcgaccagaggcgcgcgcccggcggccgaggtcatgcggcttcggcctcgcgctcgggcaggatgcggtccagctcgatcaggctgatcatgcggccgtccaccgcgaagatgcctttcacaaaggtcttgacctgatccgacgcgatgtcgggcgtcgcctgcacgtcgccctcgttcatctggatgatgtcggacacagcgtcgaccagaaggcccacggtgcggccgccgatatgggccaccatgatgacgtggcgggcggtcggctcggacgtctccagaccaaagcgggcgcccaggtcgatgatcggcagcacggtgccgcgcaggttgatcacgcccttcatgtagccgggcgagcggggcagcggcgtggccggcgtccagccccggatttcgcgcaccgacatgatgtcgacgcagaactcctggcggccgatgcggaaggcgatcagttcacgttgggaagcggcggattcggtcatgggatcagctcgcgagcttgaggtcttggcggggcgaaccccggcggcgctgggcggccacaagggcgtcgatgtcgaggatcagggcgacgcggccgtcgcccaggatggtggcggcggcgacgccgtccaccggctggtagtttgtctccaggctcttgatgaccacctggcgctggccctggatggcgtccaccagcagcgcggcgggctggccggattcggtctccacgatcatggcgatgccccccgagggcgccatcggctgctcgcggaagcccatggccatggccacgtccaccagcggcacgaaccgctcgcggaagcggatcaccggatcgaccccgccgacgtagtggatgtcctgctcgcgcggggtcaggctttcgacaatggccgacaagggcgcgatcagcgtctgttcggccgcgcccagcaccattccatccagcaccgccagcgtcagcggcaggctgagggtgaaggtcgagcccttgccaggattagaggcgatcgagatgcgcccgcctagcgcctggatcgagcgcttgaccacgtccatgccgacgccgcggcccgagatgtccgacaccaccgccgcggtcgaaaagccgggcaggaagatcaggttgtcgatctcttcgtccgacagagaggcgtcttcggggatcagacccttgtccatggcgatcctgcgcacgcgctcgcggttgatgccctttccgtcgtcggcgatctcgatgacgatgcggcccgagcggtgcagggcggcgagccgcacggttccttcggccggcttgccggcggcgacgcgctcctccgggctctccagcccgtggtcgatggcgttgcgcagcatgtgggtgatgggttcggccaggcgttcgaccacggtcttgtcgacctcggtgtcctcgccggcggtgaccaggcgcacctgcttgccggtcatgtccgcgacctcgcgcaccaggcgcggcatgcgctggaacaccgacttcaccggctgggcgcggatggccatgacgctgtcctggatctcgcgcgtcaacagctcgaggtcctccatgcccagcgcgatgttggacgagcgggcgaggccgctctcggccacgcgctgggccagcatggcctgctggatcaccagctcgccgaccacgttgatcagccggtccacccggtccaggtcaacgcggatggtgacgggcgcggcggcctgaggcgccgacgccagaggcgccgaggtctgcgtagccggcgtctgactagtcggcgtctgcgtagtcggcgtctggggcgctatgggctgtggcgtgatctgcaccggagctacgggcgcgaccgggaccacaggagccatcgggggggacgcgacaggcgtgggcgcgacgggggccggcggttcggcctgcgcctgcacccgcgccaggagtgccgcgatgtcgaggtccggcgcggaggcttgagccaggacagcggcgtcgccgccgtcgtcctcggggaccgacgtgacggcggcttcggccgcgccgccgagcggagagatgatgaggtcgcagtccgattccacgaagtcgaacacgtcgcgcacctcggcctcgctcaccgccgcgtcgagttcgatggtccaggtcagataggcatcttcaggggcgagcacgtccagcaccggcagatcggtttcgtccagcgacacggccgcgggacctagccggccgagttcgcgaagcaggatggccgtctcgttggcgctggcgtacatgcggccgtggggcttgaagacgatgcgccagccggttcgctccgtcagagacgacacgtccagcgaaggcagatcgccgacaggtgcgggatcaaaggcgccgagatcgaacgccattggcgtgaagccgaagtcgtcctcctcctcttcgaccaccaccggggcggcgccgccgtgggtcaggatttccagctcgacgaccaaggccgccgagcgcgcgggatcgaccggcggcttcaggccctgggcggcctgcacgtggtcggccagcacgtctgaggcgcgcagcagggtcttgaccgtcaccgcatcgcacggcttgcgacccgcccgcagctcgtccagcagcgtctcgaagacatgggcgaaacggaccaggtcctccagaccgaaagcccccgccccgcccttgaccgaatgcacagcgcggaagacggcgttgatcgtctcgttgtcggtctgacccgactcaagcaccagcagcttgctctccaggtccgcgagcagttcgtcgcattcctggaagaaggtcgccttgatggcttcgaaagcgtccatggcgggagggtccggccttcctgttcgaacttaagcggcgacgcggcggacggcttccaccagcttgacgggatcaaagggcttgacgatccagccggtggccccggcggcgcgggcgcgctgcttcttctcggcgtcgctttcggtggtcagcaccagaaccggcgtcgtgcggtgatccgggttcgcgcgcatgccttcgatgaagccgaagccgtccatgcgcggcatgttgatgtcggtgatgacgacatcggcgcccctggccgccagcgtctccagcccgtccacgccgtccaccgcctggatcacggtgtagccggccccttccagcgccagcagcagcatgtcgcgcatggtgcgggaatcatcgacggtcaaaactgtctttgtcacgcgagggctccctcgatctgtgaaagggcggaggcgccgaacgcctcccactgagccgcgaaggcgtcggaggcggcccggacggcgaacggctgaccatccgccgcccaggtcttgcgggccgacaacaggacctggaggcacagaccgccgagccggtccacgcccgaggcgtccagcgccagagcctcgccgcgccggctcagaagctccgccttcagcggttcggccgcgcgcaggtccagcaccggagcgagggtcagggccgccgtcatcagaactcctcccatccgtcctcgaccgcctgggacgcgatctgggattgcggcttcagagcggtgacgccgcgattgatggtcttcatcgcgcgcgccatgtggccttccggcttggacgcggccgggcgggccggcgcgcgcgacggcgcgtaggcggcggtctgcgtctggccgattcggaagcgggcgacggaggcctgcagcgcgtcggcttcctgcgccagcgagtggctggcggcggtggactgctcaaccatggcggcgttctgctgggtcacctggtccatctggttgacggcggtgttgacctgctgaagacccgtcgcctgctcgctggcggaggcggcgatctcggacaccaggccgtcgatctcggccacgcgatccacgatgcgttgcagcgactggccggtctggcccaccagcttgacgccctgatcgacctgaccggtcgaggccgagatcagggtcttgatctccttggcggcctcggccgagcgctgagccagagcccgcacctcggaggccacgaccgcgaagccacgacccgcatcgccggcgcgcgcggcctcgacgcctgcgttcagggccaggaggttggtctggaaggcgatctcgtcgatcaccccgatgatctggctgatctgggccgaggaggactcgatcgcggtcatggcggcgacggcgtcgcgcaccacattgccgctggtctccgcatcgccgcgtgcggcctgcacgacgtccgaggcctgcttggcgccggaggccgtcttgttcaccgtggcggtgatctggtccagggcggcggcggtttcctccaggctggcggcctgctgttcggtgcggcgcgacaggtcgtccgaagcctggctgatttcgccggcgccggagcggatgcccgccacgttctggaccaccaccgcgaccgcctgctgcaactgggcgacggccgagttgaagtcggccttgagctgttcggcgcgcggcgcgacctccaccgtcatccggtgcgtcaggtcgccttcggccatggccgacaggccggcggccagggcgcccagggcgacgcggtcctcctcggcgatccgggccttctcagcttcgttggcggcgcgttcctgctcggacagcgagcgctgggacagggcctcggcttcaatgcgcttcttctcgatcgccgcatcgcggaaggccaccacggcctggcccatctggccgaactcgtccttgcgttgcgcgcaggtcacctcgatggaggtgtcgccgcccatcagtttgcgcatgtagccgatcgtctcgaagatcgggcgcacaatggcgcgggtgagcgcccaaccggccagcagggcgatcaggcaggccgtcgccaggccgacggccagaccgatcagcgccatttgggattgatcgtcctgcgccttgcggatggcggcgaggtcgacttcggtcttgctcttgatggtctcgaccgcctcttcgatcggcgcgatgtacttgtcggcgacgccgtccggcgccaccagaccgcgcgcctcttcccggcgagccggatcgcgggacagggtcacggccagagtgcggacgttctggtaccagtcgtcagccgccttctccgccctgtcggcgtctgcggcgcgcgagtcgccagtgtccctgcggacttcttccagcgccttcttgaactcggcgcgatgcccgtccagccgctcaaggtagtaggagtcgttcgacagcagaaagccgcgcagcgcgttctcctgcttggccagtcgaaattccgccgtcgcaatggcccggttggccgcgttggctatttggcgttggtccccgaccttgttcagcgcaaagagattatagccgaccgaaacgcccatgacggcgatggcgcccagcaccacggcgaaggcgatgaacagtttccgcccgacgggcaggttggccaggatattcacgagcaagcttccccttacgctgccttctgcaggcgctacagtttgacgttgaacttcagggcggggtgatccgacggacatcgcgccggcgcaccggcccgcgacgctccggcaggtcccccgtccccgcctctgaagttctcagaaccagatgccgttaaggcttcatattcttcatgaagacggtgatacgttaaaatacctagcaaaccgttgttgcgacccggcgaggcgccgcgccttgccctccggcgcgagggagaacagactggctcgccggcgtcagtcggctgaaagagcacgcgcttgtccttgtcgccgaccctctcgagcgatcgacgcctctccgcccgctccgatccagcggggcgcgcgtccgctcagtccgtcttcatcgtcgacgccgacgccggcgcgcgcatcgaactgatcggtctcttgcgggcccatggaatgcgggtgcgagggttcgccacggccgcggatttcctgcagaacacgccggacgatgcgacggcctgcgtgctgatggaggccgtgctgcccgacctggacggcgtggacctgatcaatcgcgtgatcgacaggcatgacgacgcatggcccgtgacggtcgtgagcggccaggtcacggttgagaagtccgtcgccctgatgaaggcgggcgccgtcgacctgatcgaacggccgttcagcgtcggtcggatactgcaggcggtgaacgactgcctccgctcgctggcggcgcgcgacgccggccggacccgcaagcgcgtggccgaacagcgactggcggcgctgaccccgcgagagcgccaggtgttcgacgggctcatccacggccggtccagcaaggagatcgcccagagcctcgaaatcagtccccgcacggttgaagtctttcgcgcccgcgtgatggacaagatgcaggcgccgcacctgcccagcctggtgcgagccgccgtgctgctggacctgccgcgccccgacgaggatgaagaggcttgaggaacctctccggcgtcgccaccttgagatcatgagcgatcgctcgacaggcatggccccgtcccgcgtcaccgcggtcctggggcccaccaacaccggcaagacccacctggcggtcgagcggatgctgggtcacgcctcgggcatgatcggcctgccgctgcgccttctggcccgcgagatctatgagcggatcgtgaagcagaggggcgccgccgccgtcgccctgatcaccggcgaggagaagatcgttccggcccggccgcactacttcgtctgcacggtcgaggccatgccgatggagcgctcggtcgagttcctggcggtcgacgagatccagctggtcgccgacccggagcgcggccacgtcttcacccagcggctgctgcatgcgcgcgggcggatggagaccatgtttctgggcgcggggaccaccgagccgctgatccgtcgcctggtcccggaggtggaggtggtcacgcgcgaccgcctgtcgaccctgtcctacgccggctccaagaagctgacgcgcctgccgccgcgctcggccatcgtcgccttctcgacagatcgggtctacgccatcgccgagctgatccgccgtcagagagggggcgcggcggtggtcatgggatcgctcagcccgcgaacccgcaacgcccaggtggcgctgtatcaatctggcgaggtggacttcctggtggcgacggacgccatcgggatgggcctgaacatggacgtggaccatgtggcgttcgcaggcctgcgcaagttcgacgggcggcgcacccgctggctgcacgcccatgagatcggccagatcgccgggcgcgccggccggcacctgaggaacggcaccttcggcgtcaccgccgaggcggaggagctggacgacgacctggtggaacaggtggtcgagcatcgcttcgatcctgtcgaggcggccgagtggcgcaacccccggctggatttcgacaccctgcccgacctcttgcggtcgctggtggtgacgccgcagcgttcgggacttcagctgacggccgaagcgctggacgaaaccctgctgcgccgcctgatcaaggacgaggcggtggcgcgcgtgggccgctcgcgcggcgccatcatgcgtctatgggaggcgtgccagttgcccgacttccagaagaccacgctggacgagcacgcgcgcctggccaaggacgtgttccaggccctgaccggcaagcgcgggcggctgacggaggactggatcgcgccgcgtttcaacgacgtggatcgcgacgacggccagatcgaccagttgtcggcgcggctgtcgggggtgcgcaccctgtcctacattgccaaccgccccgactggctgcacgacgccgcgcattggcgcgagaagacgcgcgcgcttgaggaccgcttgtccgacgtcctgcacgagcggctgaccgcgcgcttcgtggaccggcgcaccaccgcgctgatgcgggcgctgaacgtgcgcgaggacacgctggcgggcgtggccgacgacggcgaagtcacggtcgaaggccaggtggtgggccagcttcagggcgtgcgcttctcggccgaaaagggcgcatcggcgctggaggaccgcgccctgcgtcaggcggcgatccgcgcggtggggcctgaggtcgcgcggaggctgggccggctggcggccgagccggacgaggccttctccgtcgcgcccgacggcgacgtcctgtggcgcggcgtgctgacggccaaggttctggcgggaccgaacggcgccgacgccttctcgccccaggtgcggctgttgggcgacctgggccccgcgccggcgcgcgaaagggcgaagcgccgcatcgaagcttggctggcggccgaggccggacgcgcgctgcgtgatctgcgtcgtctgcgtcaggcgggggaggcgggaacgcggaagggcctgccccgcggcgtcgcctttcgcctgatcgaggcgggcggcctgattgaccggcgtgaggtggagcgcgatctggcggcgctgagccaaatcgagcggcgcacgctgaaggccttcgccatccgcgtcggcgcccattccgtctggctgccgggtctgatgaagccccgcgcgcgacatttcgcccaagcctttatcggcgcgccgctgatccccgcgacgcccgggctgctgcctgtcccttccgaagcgccctccccgcgtgctttgtcggcgcatggcctgcggctcgccggacagtggatggcccctgtcgaggcgctggagcggatggccgaactgcgcaccgccggcaagggccgcctgtccgacgaggcgctggctgaactcggctggaccggcgaccaggccaaggctgtcatcgccgcgttgaagaccgagcgcgcccgcatgccggacaagcccggccaggcgcctcgccccgtcaaggattcgcccttcgcggcgctggcgatcctgaacgcgccgccgccccccccgccgccggccaagcgtcgccgcccgcggcgcaagcccgcgccccccccaccccggcctccggaggaacatgagcctgagccacgaacccggccgcctggccgaccgcgacgacgcctgccgcatcgacgtctggctgtggcgcgcacggttctgcaagacgcgcgggatcgccgccgccctggtcgagcgcggcgcggtgcgtctgacccaccacggtcgcgaggtgcgcctggacaagcccagccgctgcgtccaccccggcgacgccctgacttttgtccagaacggccgcgtcacctcgctgcaggtcgaggccctgggggaacggcgcgggcccgcagaagaggcccgcgcgctctattcgctgcttactgcttgaggacgaactcgccctcgaggtgcagttcgacctcgtcggagacggctggcagggcgtagttgatgccgaactcggagcgcttgatggtggcttcgccgtcgaagccggccttgtaggcgccgcccatggcggggccggcctggtggaactcgacttccatggtcactggcttggtgacgccgcgcagggtcaggtcgccgacgacggtggcctcggtcggatcgtcgttgtcgatcgtgatcgagcgcgaaacaaaggtcgcggtcggatgattggccgtgtcgaagaagtccggcgtctgcaggtgcgccttcagctgatcgtcgttgggcgccacgtccgtcagcgggatggtcgcggtcaggcgcgaggccgaagggttggccgggtccagcaccagctcggcctttacgttcacgaactgaccgacgtaggtggaaaagcccatgtgcttcaccgaccaggtgatcttgccgtggctggattccagctcgtaggtcccggcgcggacctcggccgggacttgcgtcagctggccttgcgccaccacggcgccgccggcgatcaggctgagggcaagcgcgcttgcggcaacgcggcggaacaggggagaggtcatgaggcgtccttccgaggagagggccgcccgtcgcggccaatctgcaatacgcttagttacgaatgccctttgcagccgtcaaggcggcgcttggctggatagcgctccggttgacagcgggttgcgagggctccatgtcgcaggccttcccctcacccgccgaagtccgccgccgcccaatgacctacatcgtcaccgacgcctgcgtgaaatgtaagttcatggactgcgtcgaggtgtgtccggtggactgcttctacgagggcgagaacttcctggtcatcgcgccggacgagtgcatcgactgtggcgtgtgcgagccggaatgcccgatcgacgcaatcgtccccgatactgaggacgagccggacggcaagtggctgcagatcaacgccgaatacgccaaggtttggccgaacatcaccgtcaagggcacgccgcccgccgaccgggaacagtacgagcgcgaaacgggcaagttcgagaaatacttcagccccaagcccggcaagggttcctgattctcgcgcgttcgggggtcgagcgtcgccacagcctcgcgcttcgtctgtggacgttttgaaaatccgttattttgtggtaggttctgtttcattggagcggacgttcggccttttgccgcgacgcccgcgtttgcgacagaatcccgccctatgaagacgggatcggccagaggtttggtgatccgtttccgcttttgacgctcgcatcttggatcagccgacgacttcccccagtcgccggctgaaatcatgcgtgcgcccgacgcgccttcgcttcgcccggccctgaccgggaaaggacgattatgacgagcaagactggtctggagttcaaggttggcgacgcggtcgtctatccggcgcacggcgtcggcaaggtccatgcgatcgagacccaggaagtcgccggcatgtcgctggaagtctatgtcgtgacctttgaccacgaaaagatgaccctgcgcgtgccgaccaagaaggcgaagaccgcgggcctgcgctcgctggccggcgacgacgttgtgacgaaggccctgacgacgctgaagggccgcgcccgcatcaagcgcaccatgtggtcgcgccgcgcccaggaatacgaagccaagatcaactcgggcgacctgatctccatcgccgaggtggtccgcgacctgtaccgcgccgacacccagcccgagcagtcctactccgaacgccagctgtacgaatcggccttggaccggatggcccgcgaagtcgccgccgccaacaagatcgacaaggatgcggcagtcgaactgctctccaagtcgctgagcgccaagaagccgatcccgaccgccgaagcggcctgatctgacctcatcgccgaagacaacaaaggcccgggagcgatcccgggccttttgctttgtatgatcgacaaggccgaggcgctgatctacgcctgaacgcctctccttctcagccccaagatccgcccatgccttccggccttatcgccctgctcgacgacgtggcgggaatcgccaagctggcggcggcgtcgatcgacgacgtcggggcggctgccggccgggcgtcgaccaaggcggccggggtggtgatcgacgatgcggcggtgacgccgcgctacgtgaccggcctgtcccccagccgcgagcttccgatcatcggcaagatcgcagtgggctcggtccgcaacaagctgctgctgatcctgcccgtcgccctgctgctgaccagtttcgcaccctgggccatcacgccgatcctgatgtgcggcggcgcctatctctgtttcgaaggcgccgaaaagctgatggagatgttcggcgtaggcgggcacgaaaaggcggctcccgtggccggcgacgccgccgctctggaggccgccaccgtctcgggcgccgtgcgcacggacctgatcctgtcggccgagatcatgacgatcgccctggccgacgtgtccgacgcgccgttgctgatgcaggcgggcgtgctgatcgtggtgggcctggccatgaccgtggcggtctatggcgtggtcggcctgatcgtgaagatggacgacatcggcctgcacctggccgagcgcccgtcccgcgtcgcgcgagctttagggcgcggcctggtcaaggccatgccggtggtgatgagcgccctgtcgacgatcggcacagtggccatgctgtgggtcggcggcggcatcctgctgcacggctcgcacaccctgggcctggcctggccggcagagccggtcgagcacctggcccatgcggtggccgcagctctgggcccgctcggcgccgtcgccggctggctgaccacggcggtgatctcgggcgtcatcggcgtggtcgtcggcggcctcatcgcccttgtgctgcatcaggcgatgcggctgaagcccggcgccgcccactaggggcggtccggacaagcctgcgacggctcagaagtattccgcgttcgccgggcactgggcgctgatgcgacgcgcggtgatggtggcgggaatatagggcgtgccgcgcagcagctgggcgccgccgcggaagcggaagctggtctgctcataggtcccgttcaggcgcacgttcacgtgccgccccttgggatcggtgcaggagccctcgaaccgcgccgcgccgtcgccgaccacgcgcgtcggataggtgcagcgccagcggcgcgtcgacagcccgccgaagaagcggttgatctcgctgggccgcacgcatttgcgctcgctgtcgccctggcccagcgcgctgaaggtgtattcccaatagccgggcaggacctcgctctgggcggcggtctgagccacgggggcggcggccggagcggccagcatgacgccgccggcgatcagcggggcggccagcgccaggaagcgtggcatgcggcgggcgggtttggtgttcaatgaggcggtcatgatggtctgatatagggtgcgtcttgaatggccgctgaacaagcctgttcccgcgacgcggcttgacgcgcaagcgccccttcctttatacgccccctctctcgcgcgggacgtcctcccgcgcgtccttgtttcatgcgttcgccggtcacggctgatcgccgcaccttaaggatcctgacgatgtcccgtcgttgcgaactcaccggcatcggcccgatggtcggccacagcgtgagccactcgaacatcaagaccaagcgccgcttcctgccgtcgctgaagacggtcaaggtcacttcggacgccttgggccagaccttcagcctgcgcatctcgaacgccgcgctgcgcaccctggacttcaagggcggactggacgccttcatcgtcaaggctcgcgacgagcagctgtcgatcgccgcccagcgtatcaagcgccaggtccgcgccaagctggccgaacaagccgccgcctgatcggcgaggctgacacgatctggaagaggccggcggagacgccggcctttttctttgcgcggttttcaagcttggcctaaccgtctgctccggctgttcatcccgggggctgcaagatgactgtttccgccgtgcgcgcactgatgctggctggctcgatgctggcgctcgccgcctgcgccaccccgcccgagccctcgcccgttccacccccgccggcgcgagaatcgacccccttcaccctggccaccgaccagccgcggccgaccgagcaggtcgccatgcagttcgacaaggcggacctggcgatccgcgtgatcccgcaggatcaggccatcgacgccgtggccgtgctggacttcaccgccaccgcgccgctcgaccggctgatcgtagagttggacaccctcctgaccatctcctcggttcaggtggacggacaggatgtgccgaccggacgctggtcgaacccggaaggccggctgacggtggaactgccgcagaccctacccgccggccgctccaccagccttcgcatcgcctacgccggcaagccgcgtgtggcgcctcgcgcgccttggaacggcggcttcgtctggtcgaccgcgccctcgggcgagccgtggatcgcgacggcggtgcagggcgagggctgcgacctgttctggccgtgcatcgaccatccgcacggcgagcccgcgcgcgtggacctgcacatcaccgtgccgtcgaacctggccgcgccgtcgaacggccgcttcctgggcaaggtggatcacggcgacggctggtcgacctggaactggtcggcccggcggccgaacacctatgcggtggcgttgaacatcgggccctacgagcgggtcgccagcgaatatcagagccggttcggcaacaccctgccgctcgaatattggcacctgaagagcgacgatccgcagcaggtacaggccctgttcgccgaattaccgctgatgctggacttctttgagtcgaccgtcggcccctaccctttcggcgatgagaaggtgggcgtggtcgagacgccgcacctgggcatggagcaccagaccatcaacgcctacggcaacggctacaagctggacgggcgcggctacgactggctgatgcagcacgagttcgcccacgagtggttcggcaaccaactgaccaacgagaacgccgacgacatgtggctgcacgagggtctgggcagctatatgcagccgctctacgcccgctggctgaacggcgagcgctacatgcagcgcgaactggccgaccagcgcgaggggctgatcaacaagttccccgtcgtgtcaggcagcccgaagaccgaggacgaggtctattttggcggaacaggtcccggcaacgacatctattccaagggctcgctgatcgcgcactctctgcgcatgctgatcggcgacgcggcgttcaaggaggcggtgacgcggctggtctatggccgcccggatcctcagccgggcaacttcgagccgctgtatcgctcgacgccggacttcctgcggatcgtcaatgaggtgaccggccgggattacgaatggttcttccgtggctacctctaccaggcggccttgccggttctggaccagacccgcgagggcgaccggctggttctggcctggaccacgggtgacggagcgaccttccccatgccggtcgaaatcgagatcgacggacgcctgcagacgcttcccatgacggacgggcggggttcggtgaccgttccgcccggagcgcatgtgacagtcgatccgcagaacaaggcgctgcgccagctcgacttcgtcgacgactatcaggcctggcgcgaggccgagcgccagaagcgcaccgcggcgcggccggcgagctagagcgtctcgcctgtctcgccggaaaaaagtgacaggcgaaatcaaactgttaaggtggcggcatgatcgccactccggccctgcgggcccttcgctccgcaacggggccagcccacgaagccctggagacgcaagcccgcatagaagcgcgcctggcggatcgcgccacgcgcgggtcgctggtggccgacttccaccgctttcatgccgggcttgaagccacggcccacccgatggtcatgaacctgcgcgacgattatccggtgcgctcgcgcgccgagggtatttgtcgggacctgagggatctggggatcgcaccgccgtcggtccgtccgatgcccccgccggcctcggtgggcgaggcgctggggcgggtctatgtggcggagggctccatgttgggcgggcgcatcatccgtcgccgactggcggctcaaggggtcgatctgaccggcctggcatttcttgatccctggggcgacgacaccggggcgcgctggcgcggcttcgtcgccgccatggagagcgcctgtgtcgaaggcgtcgccgatgtggacgcggtggtgcgtggcgggatagatggtttcgcgttcgcccaacgtgcgctcgccgaccgatgtggaacggagacgcccgttgactgacgccgaggtgcaactcgcgcccctcctgaacgactgcgatcgagagccgatccatattccgcaggccatccagccgcacggcttcctgctggcgctggaccgccgagacctgctcgtcgccgaaggcgccggcgacatcgaagggctgacgggcgttcgcgcctggacgggacagccgatcgatctggtgctgggcgaggcgcttgggcgcaggctgcgcgagatgatccggagcggggaaaccggctttgtggaccgctggcgcgggatcaaccggatcgactacgacgtggtcatgcaccatgcggccgaccgcaccgtggtggaggtggagcagtcgtcgcaggccgcccgcctcggcatcgaactggtcggacgtctggatacggccggcgcggcgctggaacgcgccgcctcggtgcaggcggtgtgcgaagtcgcggccgaggcgttccgcaagctgaccggcttcgaccgcgtcatgatctatcgcttcctcgacgacgacgccggccatgtggtggccgaagcgcgtgaggagacctcgtcctcgtttctgaaccaccactttccggccaccgatatccctcgccaggcgcgcgcactttacgtccgcaatccggtccgcgttattccggacgccgtctatacgccccagccgctgcgcggcggcgaggaccggccgccgctggacatgagcgactgcgccctgcgcagcgtctcgcccatccacctgcagtacctgaagaacatgggcgtgcgggcctccgcctctgtgtccatcgtcatcgacgacgcgctttggggcctgatcgcctgccacaacgagcggcccaagctgctgccctatgaactgcgcgtggcctccacgacgctggcgcgcaatctggcgcgtcagatcaaggctcgcaccgaagccgagctttaccgggaacgcgtacgcctgcgccggctggaggatgatctgctggccgccctgcccgccgaccggccgctggccgacggattggcggagcggtcgcaggggcttctgagccttgtcgccgccgatggcttggccattatccaggacggccggactcaggcttttgggcgctgccctcccgccgaggcgatcgaccgactgagcggctgggtgtcgcaacagccaggcctgcggccgatggccagcaacaacctttcggccattctgcccgaggcgtcggcctggaccgcgcacgccagcggcctattggcggttcgcgtcaccggcgagcgccccttgtcgctgatgtggtttcgttccgagattccggaaaccattcgctgggcgggcgacccccatacggcggtcaagtcgaacgcgcgcggcgttctgaccccccgcgcttctttcgaggactacaccgagacggtgcgcggccgtgctcgccgctgggatgcggcggcggtggaatcggccgcccgcctgcgcgacgcccttctggatttcagcgcggtcagtcagttgcgacgcatgaaccagacgcttcaggccagcctgaccgaacgcgacctgcgcctcgagcagcagcaatatctgatccgcgaggtcaaccaccgggtccagaacagcctgaccctggtctccagcttcctgggtctgcaggcgcgcgagcagaccgacggcgtcgcggccgccgccctgcaggaggcgcgtcagcgcgtgcgcgcggtctcggccgtgcactcgcggctgtatcgcgacgcccagtcggtctcgatcgacctggcccgctacatcgaagaccttgtcgacgacctgggcgcatccacgggcggggaatggcgcgacgccatcgacacgcacttggcgccgatcggcgtggagtcgggtcgttcggtcaccatcggcctgatcctgaccgagctgatcatcaacgcccagaaatacgcctatgacggcgccgtcgggccgatctgcatccagttgtccgagcccgaggccggagtgctccgcctctcagtccgggacgagggccgtggcggccaccaatccggtgcggggttcggatcgctgatgatccgcagcctcgtcggccagctcgggggcacgctggactaccatgaccgttcgccggggctggaggcggtcctgcgcgcccgcatcgatcccctggtctgacgtcggcgccttaagcggctgttcagcacgaccgcacacctggtcttgaactgtccgcggcatggtcggcccatgctgaccccgcgccgccttgtgcacatcgcccggctgatctttctgatcggcgtcgtcgtcctcgccgttctggtgctgggccccttccagggtctggaggagcggatcggcctgagcgacaagtccgcccatgtgatcgccttctacctgctgggcgtctccgccctggccgtcgcgccgaagtggcggcggacggacctgatgctggccctcctgggcggcggggtgctgatcgaggtgctgcagggcttcaccggccgatcgatgtcgctgggcgacctgggcgccgacgccctgggcctggccgccgccgccgcgcccggctttatcgaacagttgcgccgcctggcgcgccgccaccccgacctgtccttcgccgaaatcgccgcccgagcccgtcgccgcccccgccgcgccgaggcgccggccgcgccctacggctccagctcgatgtcccagtagaggtagtcgagccagctttggtgcaggaagtgcggcgggaagcgtcggcccgcttcctggagctgccaggcgctggggcgaagcggggtgcggcggatcggcatggcggcctgctgcggcgtgcgcccgccctttctgagattgcacggcccgcaggcggcgacgatgttctcccaagtcgtgcgcccgccgtgcgagcgcggcaccacgtggtcgaacgtcagctcggcgttctcgccgcagtactggcaggcgaagccgtcccgcagaaagacgttgaagcgggtgaaggcgggctttcggtcctgatccacataggtcttcagcgcgatcacgctgggcagcaccatctccatggacggcgagcgcaccaccttgtcataggtcgagaccacgtcgacgcggtcctgatagacggccttgaccgcctcctcccacggccacagcgacagcggataataggacagcggccggaagtcggcgttcagcaccagggcgggccagccggaggggggacgggagagaacctgcatcaggccctcccgtggtatgcggggggtggtgaggcgacaggactgaagacgcgtctccttccttgtctgaccctctcagcctagacccgattcgccgacgccgccacgacgaagacgcgaccgccgcgtgacgatctcacccccgcgcgcgatcgggaaagcccggcaggctccagccccattgaagcgcgccagcccgcaggccgaagccgcacagcgccgcgacgatggccgccggccacatgggcgtctccagcatgcgcaggcccacgaacagggtggccgccaggatcgccgccgaaatggtgatctcgcgccgcagcaggatcgacggctgtccggccagaaggtcgcgcaccaccccgccgaagcacgccgtcagagcgcccatgacgatgcagatcaggggcgccacgcccgccgcctccgccttggccgcgcccatgacgccataggctcccaaacccagcgcatcgagccacagcagcgcgcggaaccgccagtctctgcggcccaggagccagatcgccagggcgcccagcaggcacacgccgatgtagcgccagtcctgcacccagaacaccggcacgcccagcagcaggtcgcgcatggtgccgccgcccacgcccgtgacggcggcgaagaaggccagggtcaccaggtcgtgcttctcccgcgccgcggccagggcgccggtggcggcgaagacggccacgcccgcgaaatcgagggcgcccagcaccgcctgcggatcgcgcaacggttcggccagcgccggatcgaccagcggcgtcatggcgcgaccggctccagcacgatctcgccgcgcttcacgcccgtgtaccaggcccacagcagatgggtcgccacggcgcggtagggccgccagatctcggcgcgggcgtaggcctgcttctggtcgggccgcacctcggcgccgtccacccagcggatcgcctcctgcagcgctacgtcgccgccgggaaacacgtccagccggccctcgcacatcatcagataggcctcggcggtccacagtcccacgcctttaagcgccgtcagggcggcgatggcggcctcgtcgtccagcgtcgccatgtgctccaggtcgatctcgccggccagctgcgcccgcgcgatgccctggccgtaggtggccttctgccgcgacaggcccatgccgcgcagctgctccaggtcgtgccgcagcagggcctgggggctgatttcgcccatgccgtcgcgcagccgcgcccagacggcggcggccgaggcgacggagacctgctgttccacgatcatgcggaacagtccttcgaagccgccggctctcagccgccattcgagaggcggcgtggcccggtccgcgcgcgccaacgccggatcggccgcggccagggccgcgcgcgcacgggcgatgtcttcgggcgtgggcgcaagcggcatccggcggtctcgacggttgatgtcggatcgaccatgtcccggatcgcgcccgcgccgcaaccgcgcagccgcatcgacgtccgatatgcgctagtcccaacagacgacttgaaccgaacgcgacgcggcgatataggcacgcctcttccgcacgggccggacccgatgcgagcccagcggctgggtagctcagatggttagagcggtggattcataacccacaggtcggcggttcgatcccgcccccagccaccacctttttccttcgatagggtgctgcgcttacgctcgacagcgagcgcgccgcgtggtcctttctgcccatgttgatgacaggtctgctcctcgctgtcgcgctccaggcgggtgcggccgaccccctgcaggcggcctacgccaacaccctggtctcgacctatccggacgggcgaacggcgcggctttggttgaatgcggaccgcacctatacaggccaggggcggcgcggcgggcgcagttcgggagtgtgggaggtgcgcggatcggacctgtgcctgcgccagcggcggcctctgccctccccgatgcgctactgcacgcccatcgtgtccggaggcgtcggggcgcgctggcgagccaaggcggtcacgggcgagcccatcacggtggaagtggtcgccggccgatgaccgacgccgcttcttcgaaaggacgtccatgaccgacagcgaacttgaacggttcaaggccgcgcgcaccaccgccatctataggctggacctgatcgcgcggggcgcccggctgagctatgaggacggcacgcccatcgacatgggctcggagaaggcgcggctggaggctgtcgtggccgacatggaccggcgcatcgcccggcttgaaggctccatccactgatggcgcggatcgtcgggtcggagccgatccacgccggctggtcgcggctgcacaaggcgaccattcagaccgatgacggcgcccgcatcgtacgcgaggtcgaggaccacgggaacggagccgccgtcctgccctatgatcccgagcgcggcgtcgctttgctggcgcggcaactgcgaaccggcccgttgttcgcgggagcggccgatcccctgctgctcgaggcgcccgccggcctgatcgatccgggcgagacgtcggccgactgtgcacgccgcgaggcgctggaggaggtcggcgtgcggctggacgctgtggacgccgtggcgagcgccttttcctgccccggcgtctcgaccgagcggttgtttctgttcctgggagcctatcaggcctccgaccgggtcgaggccggcggcggcctggcgggtgaacatgaggccatcgaggtggtcgaggtggcgctgtcggacctggcccgcatggcggaggcgggagaggtggaggatctgaagacgctgcacctcattttgtgcctgcgcctgcgacgacccgacctgttcggctgacgcgccggcacgcaaccggcgccgtgcagcggcgtttggcccggcaagatcaaccttgaccggaacgatatcatgatcacgcgttcaaagaccctgctcgccgccgccgtgctggcgctgggcgccgccgcctgcaccgaagccgagcaggagcagaccgaagccaacgccgaagccgccgccgaccgcaccggcgacgccgccgccgaggcgggcgccaatctgaaggaagaggcccagcaagtcggctcggccatcgccgccggtgctcgcgaagccggtcaggagatcgatgaagcgaccgaccgcatggccgtcgaagccgacgagcagaaggctgagaccgaggctgacacgcgcggcaactgatccgggacttcaggccggctcggccaagagggcgtcgatcagcgccctcgcctcagggccggcccagtccgcctcgcccacctgccaggcgcggatgcggccctggcggtccagcaggatcgtctgcggcatccgcccggccccggcgaactcgaacggcagctggaagcggatgtcgttgtagagcggcagcggcctctggtcctgaaggaaccggccggccgcctgcacggcctcaggcgtcgcatcgacgttgatcggcagcaccgtgaggtcacgcccttggtaggcgcgcgcaagcgccgccagcgtcggcatctcggtcttgcacggcgcgcaccacatcgcccacagattgaccaccacgacctgaccccggaaatcggcgaagcggacgtcccggccatcggcgtccttgaagacgtagtcgggtgcgggctgaaggtcggccggcgtctccagctggcccaacgatcccttagcatagcgagccagttcgcttttggccgccggcgtggcggcttcgaaagcttcaggggcttggacggatgcgtcccgattggcgtatagccaagccgcgccgccgcccgcgctgaccagcacgacggccgccagcacgcccatcgtcgttttcgagcccgccatgaccgatcgccccactgatgccgccgggacccacgccacggccaagcctgcggggcaggatatgtggggcggccgcttctcttccaagcccgccgacatcatgcaggcgatcaatgtgtcgatcggcgtcgacaggcgcctgtgggcgcaggacctggcgggctcgcgcgcccactgccgcatgctggccagccaagggatcatcgaaaaggcggacgccgacgccattctggacggactcgacgccatcgagaacgagatcacgggcgggaccttccccttccgcgaccagttcgaagacatccacatgaacgtggaggcccgcctgtccgagctgatcggcgagccctcggggcggctgcacacggcgcgcagccgcaacgaccaggttgcggtggacttccgcctgtgggtccgcgaggcctgcgaccgcacggttgaacagctgaagacgctgcagggcgcgttgctcgaccgggccgagcagcacgccggcgacctgatgcccggcttcacccaccttcagaccgcccagccggtgacgctgggtcaccacctgatggcctatgtggagatgttcggccgcgacgcgggccgcttcgccgacgcgcgggcgcggatgaacgagagcccgctgggcgccgccgccctggccggatcgcccttccccatcgaccgccacatgacggcccaggcgctgggcttcgaccggccgatggcgaactcgctggatgcggtgtccgaccgcgacttcgcgctggaaggcctggccgccgcttcgatcacggctgggcacctgtcgcgtctggcggaggagatcgtggtgtggatgacgccgatgttcggctttgtctctctgcccgatgatctgaccaccggatcgtcgatcatgccgcagaagcgcaatccggacgcggccgagctggtgcgggccaagacgggccgcatcaccggctcgctgatcgccctgtccatggtgatgaagggcctgccgctggcctattccaaggacatgcaggaggacaagccgccggtgttcgaggcgttcgacgccctggatctggcggtgggcgccatgacggccatggtgcgcgccttgcagcccgacacccggaagatggccgccgccgccggcgcgggcttctccaccgccacggatttggccgactggctggtgcgcgaactgggcctgccgttccgccgggcgcaccacgtcacgggcgcggcggtgaagcgcgcagaggggttgggcgtcggtctggccgacctgccgctgaaagaattgcaggcgctcgaacctggcgtcaccgaagcggtttacaccgtgctgactcccgaagcctcctgcgccagccgccagagcttcggaggaaccgcgccggaacaggtccgtgcgcgcatcaacgactggagacgacgcctgtgaagacaaccctgatcgtcgcgggcgcgctcgccctcctgacctccgcctgcggccgcatggccgatctggaggcgcccgtgccgaacggcggcgccatccggggcgccagcgcccccggtccggtcgagccggcgaccgtcaacgcgccctcctccatccaaccgatcgacggcggtccctccaaccccatcggcggcaccgccgcccagcgcgatccgcgataggccttgcaccatttcgacctgaagaacggcgcgctgcacgccgaggacgtttcgcttgaggtgatcgcggacgaggtcggcacgccggcctatgtctattcgtccgcgacgctgaagcggcactacggactgctgcgcgccgccgccgacgcgcaccgcgaggcgctgggcgaggcgctgatcgcctttgcggtcaaggccaactccaacctgtcggtgctggcgaccctggccaggctgggctccggcgccgacacggtgtcggagggcgagatccggcgcgccctggcggcgggcgtgccggccgagcggatcatcttctccggcgtcggcaagaccgacatggagatggccttcgccacgggcgtgggcgttcgccagatcaatgtggagagcggcgccgaattggatcggctgatcgccgtcgcccaggccatggacgcgcgccccgccgtggccatccgcgtcaatcccaacgtcggcgccggcggccacgccaagatcaccaccggcggcaagggcgacaagttcggcgttccggccgacgaggccatgcgtctctacgcccgcgcctcggtctcgccgcatgtgacgccggtgggcctggcctgccacatcggcagccagatcgtcgatctggccccgctggaggcggcgttccaggtgctgcgccagatgacgctggacctgcgggcgcagggtcatgcggtgacgcggctggatctgggcgggggtctgggcgtgacctattcgggcggatcgacgccgccgtcgccggccgactacgtcgccatggccgcgggcgtgcttcaggggctagaggtggaggccgcgttcgagccgggccgcctgctcgccgccaacgccggcgtgctgctcagccgggtgatccaggtcaacgaacgctcggacggccggcggttcctggtgctggacgcggccatgaacgacctgatgcggccggcgctctatgacgcctttcacgacatcaaggccgtcgagcctctgggcggcgaggatcaggcctatgacgtggtgggtcccgtctgcgagacgggcgacacttttgcgcgagaccggcgcctgccgccgctggaggcggacgacctggtggtcttcaccggagcgggggcctatggcgccgtcatggccagcgaatacaacagccgcccgctgatccccgaggtgctggtggacggcgaacgctgggccgtgatccgtcctcgcccgacctacgaggacatgctggaccgcgagccgttcgcccactggctatagccttctctcctccccaccgtagatggggaggtggcgcgaggcgaagcctcgtgacggaggggtttgcatccgcgttacaaacccttccgtctcgccggctcgcgccgccgatccacctcccattcgcttatgcggccagggaggagaggtgcgtcgcgatgctcctagtccctgggcgcgggcgcatagacgacgcggcagtcgccctcgatggtggtgaagcggccgttggcggcgtcgacgaacgacagacgcccgccctcgtcatactcgaccttgccggtcgagcggccggcgaagttctgcgttccataggtccagcaggtgatgtcggcgggacgatcgccccacttcacgtcgcgctgggccttgcggctgtcggtgcagccggacaccaggactgcgagggcgaggcaggtcaggaccgggatgcgcatgggcggagcttgcggcaagcggcgccgtttcgcaagccgcctcagtccagcgcgcagatgtccggcaggccgcgcagatgtccggcgtggtccaggccatagcccaccaggaagcggttcggcgcttcccagcccacgaagtccggctcaggcgcgcgcggttccggccagggctttcgggcgaagacgcaggtcagcacctcggccgcaccggcctcgcgcgcgatgcgcacggcctcggccaaggacaggccggtgtcgaacacgtcgtccaggatcaacacgcgtcgcccggcgatcggccgctggaacggcgcatagacgtcgatccggccccggctcgtctgctcgtcgccgtaggaggccagccacagggcgtcgaaacggacgtgccgcccaacccgcgccagcgcgcgcgtcaggtcggcggcgaaccacaggccgccggtcagcagcacggcggccacagtctcgtcgtcgatcacgggggcgatccgcgcggccaggtcggccacgacgcgggcgacctccgcctcgggcagcagaacggtcggcgtgggagcgggctcggccatgacgggaggcctagcgcctagtgatggcccttgtccaccgaggccgcggcgggcgcgtgatcgtccacggggtgagcgtccaccggcgcctgcgccgacgcgctgtgatccgcggccagggctggccgcaagccgccctctgaggcggaggcgtgcgccgccggcgccggaggcttgtccgccgcctcgccgtggtcggacgaagacggcttgtggtcgccggcgggcgcggcgtgaccggccccgtgcgtggccgcggctggaacgaagttcacgttgatgtcggccgcatggccgccgggatcggggatcagggcggcgaagccctgcaccttgccgggcagcacgggcgccgcgtcgatccgcaccaccttgtgcccgatctccgcgccatgcgcgtccagcagggcgacgcggacgggcggcgcgacgatctcgccgtcgcgcacgttcctgagggcgccggacaccagcaccatgccgggatggcccggagcctccttggcgctcatcgcctcgaagtccagaccgacagggttcaccggcgagccgaccatggcgtaggcggcggcggcgcggggaaaggcctccaccacctccacgcggaacagccaggccgaagcgacgaggcccacaaacacgctggccatgccggcccaggcgatcccctgcgccgccgcgcgccgcaggcggcgctgctgttcggcgcgggcgcgaaacgccttgggcagttcgggcgccggggtctcggccaggctgacctccggatccggctcgatcacgacgggctcgggcgcgacggtcagttccagcggttcgtcgttggaggctttccacacctcgccgcacgacttgcagcggaccttgcggccgttcggaccgaccaggtcgtcggcgatgaaatagctggtggcgcaggcggggcaggtcagtatcatgttcgctgactgcgaggcgtctcgccccctcctgttcggggctgctcgccccgtgccgaacccagatcgatgccgtcttcgcccgccacccccgaaccctcagccgcgcccgagaccgtccgcctgcagggcgtgggcttcggctatgcgacgtccggtgcggttctgcgggacgttaacctcattctgccgcgcggctctttccattttcttaccgggccgtcgggcgccgggaagtcgtcgctgctgaagctgctgaccctggccgcgcggccgaacgccggaacgattcatctgttcggacaggatgtgacgcggatcgcgcgccgcgacgcgcccgcccttcgtcgacgcatgggcgtggtgtttcaggacttccgcctgctggatcacctgtcggcctttgacaacgccgccctgccgctgcgtctggccggcgagacgcgcgaccagcacgccggcgacgtggaggagatgctgcgctgggtgggactgggcgcgcgcatgcaggcccgaccgcccgagctgtccggcggcgaaaagcagcggctggccatcgcccgcgcggtgatcggtcagcccggcctgatcctggcggatgagccgaccggcagcgtggacgccgccatgggcgagcggctgctgcggctgttccaatcgctgaaccggctgggcgccaccgtgctgatcgccagccacgatcagggtctggccgaacgctcgggcgcgggcctcttgaggctggaggccggtcgcctgacgggccaggggacgacggagccgatcgccgcatgatcccccgcccggcgttcctgaagcttgaaggcggacccgcgcccctgctgccgcgcgcctcggcgggcgagccgtggctgatgacggtgatcgcggtgctgtgcttcctggcctgtctcgccgccgtgggcgcatccgccgccgaccgcgcggctcgcggctgggccggccagctgggcgccgaggccacggtgcaggtgcgcccacgcgtcggcgagacgggcgccgccgccgccgcccgcgccgccgagaccctggggggcgtcgacggcgtggaggaggcgcaggccctggatcgccgcgcggccgaagacctgctgcggccgtggctgggcgaggcggttctgcccgacctgccgctgccgttcctggtcaccgtgcggctgtcgccggatgcgcccgcatcggcggtgaccctcagccgggctctggcgcaggcggggctcgacgcgtcggtcgacgaccacagcctgtggcgcggcgaggtcgagcgctcggccggcgccatcggcgccctggcgggactggcgtttctggccacggcctttgcggcggcggcggccatcgcctacgccacgcgcgcggggctcgccgccaaccgcgcggtgatcgagacgctgagcctgaacggcgcgggcgacggactgatcgccagcctgttccagaagcggttcgccgtgctcgccgccacggccggggcgatcggcgcgcttgtcgccgccgtgcctgtggtcctgctgcggttcatcggcggatcggatgggatcagcgccgccctgccgctggcctggagcgacctcttgctgctctcgccatgcccgcttctcgccgctacggtggcgcttgcagcggcgcggatcgccgcaatgcggacgctggcggatggcagggagggcgtatgagatttctgacgattatagtcgtcgccgccctgatctggctggccggcctgttcgccttcgcccagcacgtccgcgacctgacgccggcgtccgatccggcgcgcgccgacggcatcgtcgccctgaccggtccctcggccgagcgggtcaacgccgccatccgcctgctggaatacgacaagggcgaccgggtgctgatctcgggcgtcaaccgcgaggtgcgccggcgcgagctgcgcgaactggtgcccggctcgtcacgcctgttcaactgctgcgtcgatctgggcttcgaggccacggacaccgaaagcaacgcccaggagatcgccgcctgggcgcgctcgcgcggctatgacagcctgatcgtggtgacgtccgactatcacatgccgcgctcgctggccgagatcgagggcgccctgtcgaatgtggagctgacgcccttcgccgtctccaccccttcgctggacaccgaggactggtggcgcacggaacccacggcccgacgcatgacgctggagtactgcaaatacctggccgccgtggtgcgcgagttctggcgcgacctgaccggcgacgaagacgccccagccgctgaaaaggccgccgcctaagtgatcaccctgcgatccctgttgttcgtcgtctggctgtacctgtccatggcggtgttcgccgttggcatgtcgccggcgctgctgctgccgcaccgctacgccatgtgggtgatcaagtcctggtcgcggttcgtgctgttcggcctgcgctggatcgcaggggtgcgggtcgaggtgcgcgggctggagcaccggccgaccggcgcggccctgatcgcctccaagcaccaggggatgctggatgtcatcgcgcccttcgcctttctggacgacaactgcttcatcatgaaaaaggagctgatgcccctgcccttctttggctggttcgcctggaagacgcggatgatcgcggtggaccgctcggcccactccaaagctctcaaggacatggtgcgccaggcccgcgcccgtttcgcggaagggcggcaaatcctgatctttcccgagggcacgcgcgccgaggtggaggccgagcccgactacaagcccggcatcgcggccctgtaccgcgacctggacgcaccctgtcatccggtcgcaaccaacgccggcgtgcattggccggcccacggctttcggcgctatccaggcacggtggtctatgagttcctgccgcccatcccggccggcttgaagcgggccgagttcatgcaagcgttgcagaacagcatcgagtcggcctcgacgaagctgctggtgcagccaaacggccgtctcatgcattccggcgacggatcaaccgcctgaaagcccacgtccgcatgtcgctgcgtcttctctctctcgccgtcgtctccttgtccgccatcgccggatcggcgctcggacaggcccagccctaccctcggctggaggagcccagggaatggcgcgtggacgtcggcggcggggtgacgcacggcttctccgccaccggcaacaccggcaaggacgtgaactggaccgcctggggatcggccaactggcgcgagatcgtctacgccaacggcctggacggtctgggatggaacgccgtctattccgacgatttccgcgccggcgttcaactgcgcccgcggttttcggccggtgacatcgagggttccgatctggatcgccccggcctcggggcggacggaacgctgtacgcctacaagcgcattcccggcgatttcgtggtgggcggccggatcggccatgacgtgacgggcgacgatgccggcctgagctacttcgcctccatcggccaccaggacgtgacgcgcgtcggcctgctgcgtacctcggcctatgtcagcggcggcgatgatgagcgggtccggcgctactacggcgtgaccccggccgaggcgcccggcagcggcttttcggcctatgagccctcgggcggcctgaccggagcgggggtcgccctgttcctggccgtgcccgtcggagagcggttcggcgtgggcggcttcgtcaactacgagcgtcgtctcggcgacgtaaaggacagcccgctggtggacggcgccgatgtctggcgcgccggcgtgatcggcgtggtccgcttcagcagcccgaactagaccagcgagccccacgacagggcgtggacgcggtcccgccccagggcggcggccatgggcgggctggcgaacaggccggcgatggcgggatcgcgcacgttcaagccgccggtgaaggcgccgaacgccggcagcacgatgcggcggccgtccgtgatgaagcagggccggcgcacgccccggctgtaggcgacgaccttggcggccgggtgcaggtggccggcgacttcgcccggctggtctcccggctccggctcgtgggtcaggcgaagcgcgcccagcgacagggcgggaacgacgcttcccggcaacagcgacgtcgcgtcgtccgccgcgttcagcgcctcgcgatcgtggttgccctccagccacagccactcgcgcccggcggcgagccgatgcagccgctgcagatcatccgccgccatgcgtccgatcgatcgcgcatcatgaaagctgtcgcccagcagcacgaccattcggggttccagttcggccacctccgcctccagccggtccagcgtggcgcggctgtcgaagggcggcagcagttggccgcgcgcggcgaaggccgagcccttctccaagtgcaggtcggcggcgaccaggcatttgtgagccggaacccacaaggcgcccgaacagcgcagcacgcagggcacgccctcgatccgcacgcgcagggagccacacgccttgcgcgccggctccagcgtcttcagctgggccgcgttcaagccgccatctccggctcggcctcatccagcacttcggcgatcagggcctcggcgctttcgtccaggatcatctcggcggcgcttccgcctacccgctcgcgcccgatctgcaccagcaccggcacgcagaagggtgaggcgcgggtcaacgccgcgtgacgcagcttgccctggatgcgcatcagcaactgtcccagccgcgccacgtccaggagccccgaggccgcatccgcccgcgcggtcttgagcaacagatgatccggctggtgccgccgcagcacgtcgtagatcaggtcggtcgaaaaggtcacctgacgtcccgtcttctccgcccccggctggcgccgctcgatcaggcccgacaccagggcgcagttgcgaaacgtgcgcttcatcatgaagctttcctccagccaggcctccaggtcgtcgcccagcatgtccggctggaacagggcgtcgaggtccagttcgtccatcggcaggatcgaccagatcgccagcgaatagtcggtcaccacgaaccccagcggcccaacgcccagccggtctagccgccgggtcagcagcatgcatagcgtcgtgtgcgccagcctgccctcgaacggataggccaccaggaagtggcggcttccgcgcggaaaggtctcgatcagcatggagtcggcgcgcgggatcagcgaccgttgctcctgcagctccagccattcctgcacgtcgggcggcaggacgcgccaatggtcgcggtcctccaccatggtccgcacccggtcggcgagcgaggtggacagcgggaactgcgatccgccccacgacggaatctttgggtccttgtcctgggcgtgggtgacgagagcgtccatgccggcgatgccctgaaacgcccagacctgtccggcgaagacaaaggtgtcgccgggggtcagcggctcgaaataccactcctccgcttcgccgatcttgcgcccgccgacccatcgcttcgagcccccgccgccccgccgctgggcgaccttgaggttcagcgtgccggcggtgacgatggcgcccacattcatgcggtggcgctgggccaccagctgattgcgcaccttccagcggccttcgcggtcgcgtacgatgcgggcgaaccggtcgtaggttcgaagcgcgtatccgcctgtggcgacgaaatcgaccacctcctccagcgtctcgtaggtcagctcgcgatagggcccgcaggaggccacctcctcgaacagcgcttccatggtgaagggctccgagcaggccagtcccatgacgtgctgcgccagggtgtccagcgtgcccgtatgcaccggctcccagtcaaaggcgttttccgccaccgcctcgcgcgccgcctggcattccagcagctcgaaccggctggcgggcaccagcagggcgcgcgacggttcgtccagccggtggttggcccggccgatgcgctgaaccaggcggcttgatcccttgggcgccgccatctggatgaccagatcgacgtcgccccagtcgatgccgagatccagcgtcgaggtgcagaccaccgcccgcagctccccgcgcgccatcgccgcctcgacctttcgccgctgctccggcgccaacgaaccgtgatgcaggccgatcgccagattgtcgtcattgacggcccagagctgctgaaacacgaactccgactgccagcgcgtgttgacgaagatcagggccagggtcgagcgctggatggcggcgtagacctccgggatcgcatgctggccggtgtgccccgaccacggcacccgcccctcggacaccaacacgtccaccaccgccggcgcgccgggatcgcccttcaccagccgcacggcgtcgcggctctcggcagggtcgcctctctgcggcgccagccagtcgcggatcaggtccggatcgtcgatggtggccgacaggcccacgcggcgcatgccgggcgagaactgctgcagccgcgccagccccaggctcagcaggtcgccgcgcttgccgctccagattgcgtgcacctcgtccagcaccacgcacttcaggtctgcgaaataggcccgcgcaccctcccaggcgcagaacagcgccagctgctcgggcgtagtcagcaggatgtcgggcggaaagtcgcgctggcgctggcgcttggactgtttggtgtccccggtgcggctctcgacatggatgttcagcccgatctcgcggatcggcgtcatcagattgcgctccacatcggtggtcagcgccttcagcggcgagagataaagggtatgcacccccgaccccggcccgctctcgggcttgggcccgcgctcggccaggtcgatcaggctgggcaggaaccccgccaaagtcttgccgccgccggtcggcgcgaccagcaaggcgtgcgatccggcctgcgccgccgcgaccatctccagctgatggcgacgggcggaccatccccgccgcgcgaaccagtcggcgaacagcgggggaagctttgcgggagcggcatcaggcgtcacgcggctcatatagcatgttcccgttccgtttcagccccgcgaacgctatctatcgaaggtgtcagacgaatccgtcatcaccgaagcgcgctcgtggatcgccgacgccgcgtccgccctgccgcctgccttggcgacgccgccaggcgcgggggcggtgtgcgacggagagggcgcgcgcaaggtcgggcgcggtgcggcggaaggagtgttcaccggcgggccggtgctggtggcgcacgcgtcgctgacggcccggcggctgggattgtcgccgccgccgcgctctcccgagatgatggacgtgctggagctctacgcctttgtacgcccggcgcagttctgcgcgccctcgcccaccggtctggcgctggcgttgggcctcgccgagccccggacggccgaagagcaggcggcgtccctgcgcgaggcggcggccgtgctgctgcgtgagctggcgcagcccgcctatcccgagcgggaggcggcctatgtgctggcgcagacgctggagcgcgccggctgggcctggggcgagcgggcgtcggacgccctgcgggccggaggggtgcgtcagcgccagcatcgcggatcgggcctcgatgtctggacgcgcctttccgaatgggaggacgaggcgccccgcggcgaggcgggttcggccccggtcgacagcgaaagcgcgcgcatccggctggacaagctgttgcaggcgcggggcctggacgagacgcgcccaacccagtccgactacgccgccgaggccgccttcgccttttcgccccgcaacgacgaggggcggccgcgcgtcctcctggccgaggccgggactgggaccggcaagaccctgggctatctggcgcccgccagcctgtgggccgagcggaaccagggcgcggcctgggtctcgacctacacccgcgcgctgcaacgccagatcgaccgcgaaagccacgccctgtggcccgacccggcggagcgcaagaccaaggcggtgatccgaaaggggcgcgagaactacctgtgcgtgctgaacctgcaggacatggtgcaggcggcgcagctggggaacggcgacctgatcgggctggcgctgaccgggcgctgggcgctgcacacgcgcgacggcgacatgaccggcggcgactttcccggctggctgcccggcctgttcgccacgcccgccgcgcacgccgcaagcgccggcaatctggtggaccggcggggggagtgcgtccacgccgcctgcccgcactaccgcacctgctttgtcgaaaagaccatccgggccagccgccgcgccgatctggtgatcgccaaccacgcgctggtgatgacccaggccgccttcgacggcgcacgctcggcgcggggactgaagcaggacggcgagaccgcgacgctgaagcggattgtcttcgacgagggccaccatctgttcgacgctgccgacagcgccttttccgcctgcctgtccggtcaggaggcggcggagctgcgccgatggatccgggggccggaaggacgcggccggcggggacgcggtcttgaacagaggctgggcgaccttctgggcggcgacgaggcggcgaacagggcgcttcaggacgccatccgcgccgccacggccctgccgggcgaaggcgtgaccggccggatcgcgccggcctcgggagaggtcaatccgatcggccccatcgaagcctttctggccgcctcgctggatcagctgcgcgcccgcacctctgacagccgaaccccgtccggcggcgagttcggcatggagtgcgcgttgaagcccgtgaccgaccccgtggccgagaccgcgcgtgcggcggccggcgcgctggcggccatcgaggcgccgctgctggcgctcgcgcgacaccttgaggacatcctggacgacgacgcctccgagctggacggctcgcagcggtcgcgactggaaggggcgctgcgggggctggaccggcgcgcccgcatgaccctgcccggctggcgttcgatgctggccgcgctggaggacgggggcgaccagccggacccggacttcgtcgactggctgtcggccgagacggcgttcggccgcatccacgacgtggcgctgcgtcgccactggatcgacccgaccttgccgctggaggccgcggtgatcgcgccctcgcatggggtgctggtgacctcggccaccctgtccgatccgctgcaggaggacccgttcgatctggcgcggctgcgcaccggttcggcccggctgatcgagccgccgcgcaccctgaaagtcgatagtccgttcgactacgccgccaacagccgggtcatcgtggtcaccgacctggtcaaagacgatccgcgccagacggcggcggcgatgcgggagctgtttctggcggcgggcggcgggggcctgggcctgttcaccgccatccgccggctgaaggcggtgtacgagcggcttgggccggatctcgcgcgggccggcgtccccctctacgcccagcacgtcgatccgctggaggtcggcgcgctggtggacatgttccgggtcgaggagaacgcctgcctgctcggcaccgacgcggtgcgcgacggggtggacgtgccgggccggtcgctgcgggtgctggccttcgaccgcgtgccctggccgcgcccggacctgctgcacaaggcgcgccgggaccggctgggcggcaagggctacgacgacgcgctggcccgcgcccgtatcgcccaggccttcggccgcctgatccgccgggccgacgatcgcggcgtcttcgtgatgctggacgccgccgcccccacccgcctgttcgccagcctgccgccgggcgccgagctgcagcgcatggggctggtggatgcgatcgaggtggtcaaatcgttcctggactgaccggctcagctctcgaagacgatctcgatgctttcggacgagcggtccgccgggccgtggaacaccgcctcgatgttgttcccgtcggggtccagcaggaaggcggcgtagtagccgggatgatacggccgcaagcccggcgcgccgttgtccgcgccgcccgccgccaggccggcggcgtacacggcgtcgaccataaccctgtcgcgcgcctgaaaggccaggtgaatgcggccggtgacgcgaccctgcgccccctcgctgtcggcgctggacacgaccagttcatcggcgccgaacatgccaacgtcctcgaaatcgatggagacgccgagcacatccagcaccgcctcgtagaagcgacggctggtggcgaggtcggcggtgacgatctgcacatgatcgatcagccggccgcggaacagcttctgcatctccatgggccgcctccgatccgttgtcggggttgaacgcgtagcggagggctgcgttgcgccaccgcacccgctgttccgctttgagcgatctgctagaggccgttcatgaccgacaaagccacgcccaagcgccatagccgaaaagggctctacgcccccttcatcctgctgctcgtgctgctggcgggctggaccggctggtggttctttctgacacgccagatcgagacccggctggaggcgcaagccgaggcgatgcgcgggcgcggctggacgatcgactacgccgacccgtcgatcagcggctggccgttccgcgcccgcgcggccctgccgcacgcatcgatcacggcgccgtccggacatgcggtcgccgcgcccgagctggtggccgaggccaacgcctatcagccgaccaggtgggtggtggtcgcgccggacggcctgacactcacccgtgcggccaagggcaaggtcaatgtgcgcggcgacgcggtgcgcatgagcgtgcatggcctggaccagcgctggccgaacctggcgctggaactggtcaatccggtcttcaccccgcatccggaggccgagccctttcccatcgcccgcgccggtcgggtcgagctgtattcgcgcccgcacgtcgccggcggcgtgacggcggcggacgacgtggacgtgctttttcggctgatcgatgcgcaaggccgcccggcgggtccggttgagggcttcgcccagcagggccggctgaccctgcagatcgagacggtgctggaggacgccagccgtctgcgcgccagcggaagcgacggcctgttcgccgcctggacccgcgcgggcggccgcttcacgcaggtgcggggcgaaatgtcggcgggccagagccgcgcgaccctgtccagcgacgaactgcgggccgaggccgacggccgcatcgcgggccaggtggcgctgaaggccgagcagcccttgcgcgccatcgcagggctcgcccgttcgggcgagggaaccgtgaaccggctgggggccacaggcgcggccgcagccgccggcgccgccgacgcgacgggtcagggggacgtgcagctgacgctgctgttccgcgacggccgcacctggctgggccccttccccatcgccccggcgcccaagctgttctgatgctggaggaggcgcaggccgacgagaggcgcgcggcgctcgatctcgcgctgctccgcgcgatccgagagcggctggaggccggcttcggcgagcgcccggacggcgacgccatcgccctgcgcggcctgctggccgaggcgacgccggcgcaggccgccgcctttctcgccctgcgcgggcggctggaggcggaggctgcacaggtggtggtcaggggcgccgcagccgcgatcttggccgcggaccgttacggcctgaaggtccgggcggtcgaggacgccgacgccgcattcgccgccctcgcttcggggggtttggcggtgctggacgtcgcggcggcgcgtccctggtgggggcggctgctggcgcggcccgagctgagcgtcgtcgccgccctgcccgacgatcgccgcgcgcaaccccaggcgctggtgatctcggcccgcaaatccggccccacgggcgaggaccgcagcttctgggtcaccgacgccgcctggcccgacagccgcatcgtcgagaccctgtcgcaggccggactggccgccgagccgctggcggcgcgcggcggcttgaagctgttcaccctggcgggctatgtgcaggccgacgacgggcggctgatcgacgcacccggcgccctttccggcgtcatcggcgcggcgcccgtattctgaaccgccaaggacttcttcacatgaccgacgcctccgcagccggccccgtcgccaagcccggcgtcatggacatcgccccctatgtcggcggcaagtcgtcgatcgtcggcgtggccgagccgatcaagctgtcgtccaacgaaaacccgctggggccgggcgacaaggcgcgcgccgcctatgaggccgcagtccgcaacatccacctctatcccgacggcaaggccggcaagctgcgcgacgccgtcgccgatcaccatggggtggaggccgagcgcctgatcttcggcaacggctcggacgaggtcttctcgctgctgaaccagacctatctcagccccggcgacaatatcgtctgcggccagtacgcgttcctagcctatcgcatcagcgccctggcctgcggcgccgaggtcaagctcgcgcgagagcccggctaccgcgtcgagatcgacgccctgctggagcaggtcgatgcgcacaccaagctggtctatgtctccaatccgtccaacccgaccgggacctggaacacggccgacgaaatccggcggctgcacgaagccttgcccgcccacatcatcctggtgatcgacgaggcctatgccgagtacgtcggtgagccggaatgggagaccgccttgccgctggcgcgcgaggcggccaacgtcgtggtcacccgcaccttctccaagatccacggcctggggggtctgcgcatcggcttcggctatgcaccggcggccgtcgccgatgcggtggagcgcatccgcctgcctttcaatgtctccctgccgggcatcgaggcggcgacggcggcggtcaaggacgaggcgcaccagcgcacgtcgcgcgagttggtcgacgcctggaagccgcgcctgactcaggccctgcgcggcttcggcctgaaggtcctgccttcggccggcaacttcatcctggtgctgttccccgatcccgcccgcacggccgcgcaggccaacgaggttctgatgaagaagggtgtcatcgtgcgtgcggtcggcggctacggcatccatgacggcctgcgcatcacgatcggcaccgaggaccaaaaccgcgcggttctcgacgccctcagcgagttcgcggccggctgaccgcccaattccgcaccgccatgcccgccgctcccgccgcctcgtcgcgcgccgttcccctgatcgtgctgttgatcgccgcaagcgtcctgggccttgcgcccatcctcgtgcggctgacggagaccgggccggcggcggcgggattctggcggttcgtcttcgccatcccgctgctggcgctgatcgtcgggcgctcgggcggcgaagggttcgcgcgtccgtccaagtggatgctgctggccggcctgttcttcgccatggacctcagcttctggcactacggcatcgtcatgacctcggtcaccaatgcgacggtgctgtgcaacctgacgccggtggtggtgacggccttcgcctggctggtgctgaaggagcgcccgggcaagctgttcatcgtggccctgatcctggccatggcgggcgccttcgccatggcggcggcggccagcggcgcgcaggggaccaatccggtgttgggcgacgtgctctccctgctcgtatccttctggtactcgggctatttcttggcggtgaagctggccaggcgcgacgccggcgccatgcgcgttacctggtgggcgacgctggtcggcgcgcccatcctgctggttgtgtcgctgatgctgggcgaagacctggttccggccagcgcggccggatggtcggcctgcgtcgccatgggcctgatgcacgtcaccggacagggcggggtcgcctgggcgctgggcaagctgccggcgtccctgacggccgtcaccatcctgatccagccggtggtcgccggggtcctgggctggctggtattcggcgagaccctgacgccgatccaggcgctgggcggcgccctggtgctgggcgcggtagtgctggcgcaggtctcggcgcgaaagaaaacaggcgcgccggccaaagccgacgcgcccgtcaatccataaacccgaaggtcggacttagaggaccttgaggtccaccgccgacgtcttgccgcgctggttttccagctcgtaggacaccttcgcgttctcatcgaggccttgcaggcccgccttctgaacggcggtgacgtgcacgaacacgtccgagccgccgctgtcgggctggatgaagccgtagcccttggtggggttgaaccacttgaccgtaccggtcgccatgtctgcgtctccgtaaacgcgcttttttccaggcgaggttcccgaaggcaaaccccgtcagcccatctggacaagctcgttcaggcgaaggagcgagacgcgggtttggaccccacgctgaaatccggactgcgccgatgttgtcacccggcttttcgggccggtcaacagcaaagcgaatcgcgcggtctcagccgcacaggccgcgcggcgccccgtccagatgcagatggtcggcgtgggcggcgttgtagtccgggtccagagcattggagaacagccgacaggcgccgtcgcgcaccgtgcggagaaagcggctcccctcctccccccgcggccccgagcccgaccagtcgttcagcacgctgacgctgcgcccgtcctccagccggaagcccgagacgtccagggcgttggcgcgcgcatgctcgctgggtcgctcgttcgcgtccgacgagccgtagatgcggcggcatgagtaggtcccgaaattctccacccgcgccggctccgaccccatcacctcgcgggcggcgggacgcagcacctggcgatcccagatgacgtagcgcacggccagcgggcattgcatgaccacgccgccggggctgagcggcgtcacatcgccgccggtgatccgcactgcgccctgcacgatgcagaagccgccgtcgttgcggtccgccgcgcgttcgacccgcacgcccgcctctcgcagcagggtcatgcaggcggcggtggatcgctccacttcctcggtttgggccacgcgcggcagatcgaaggccgacaccttggacgccgtcgccgcgccgatcggacgagacaggtcgagcggcttccacggcaggtcctgcgcgggcgcaaagacgttcagcagggcgaaccccgcgcaccccagcagcgccagctcccaaagcagattccagaagtcggcgacgtcgcgcttcatgcctctccaacacgcggccggaagggccagacggtgaacgcgcgctcagcggctaagctccgcgacttcatgccgcagcgaagccgtcgcttgcgaccctggtcgcacgcgtccactgtcaggagatgagtcagaccgacaaagactacgacgccgaactgatccgtctgcagaccgctctggtggaaagtcaggcctgggcgatccggcagggcttgcggatcgtgattgtgttcgaggggcgcgataccgcaggcaaggacggcgcgatcaagcgcctgacggaatacatgtcgccgcgccagacccgcgtcttcgccctgcccaagcccaccgagcgggaggcgacgcagtggtatttccagcgctacgtcccgcacatgccggcggcgggcgagacctcgatcttcaaccgatcctggtacaaccgcgcgggcgtggagccggtgatgggcttctgcacgcccgagcaacacgaccgcttcctctccgacgcgccccggttcgagcggatgctgacggacgacggcatcgtgctgatcaagctttggctcgacatctccaagggggagcaggctgaacggctggccgcgcgccgggacgatccgctgaaacgcttcaaggtgtcggacctggatgccgaggcgcaggcgcgatgggacgcttattccgccgcacgcgaccggatgctggccgagacccactccgccttcgcgccctggaccgtggtcgccaccgacaagaagaagaaggcgcggctgaacattctccgccatgtgctgcgccgtatgaacgcgccggggattgaggcggccccgcccgatccggacgtcgtcttctcgggtgacgacgccgccggccgcacggcgccgtagaatcgcgcgcgggcgtggtgacgcggagcgcgcggcctcctacttagtcagccatgaccgtgcacgtttccccctctcccctgctcgagacctcgggcgccgatccggcggaggcgctgtcgatcctgcagggcgcgctgaccggcgcggacgatggcgagctgtttctggagcggtcggagagcgaaagcctggtgttcgacgacggccggctgaagtccgccgcctatgacgcatccgaaggcttcggcctgcgcgtggtggcgggcgagaccgccggatacgcccacgccaacgagatttcggccaccgccctgcgccgcgccgccgacagcgcgtctctggccaaggccggccatgccggcgtggtcgccgaggggccgcgcgccaccaaccagaagctgtacggcgaggtcgatcccctcgcctcgcccgccttctccgacaagatcgccctgttggctgagatcgacgccttcgcccgcgcgcgcgacccgcgcgtcgtccaggtgtcggcctccctaattggagagcggcgcgagatcgacatcctgcgcgccgacgcgcgctccgtgcgcgacgtgcgtccgctggtgcgcctgaacgtctccgtcaccgtcgagcagaacggccgccgcgaaagcgcctcggccggcgcgggcgggcgtgcgggcttcgagacctgggtcgcgccggaacgctggcaagcgcaggtggacgaggcgctgcgccaggccctggtcaaccttgaggccgtcgattgcccggccggcgagatggacgtggtgctgggcgcgggctggccgggcgtgctgctgcacgaggcgatcggccacggcttcgagggcgacttccaccgcaagggctcgtcggtgttcaacggcatgatgggcaagcgggtggccgcgccgggcgtgacggtggtggacgacggctccatcgccgggcggcgcggctcgctgtcggtggacgacgagggcacgccgacctcgcgcaccgtgctgatcgaggacgggatcatggtcgggctgatgcacgaccggctcagcgcgcgtcagctgggcgtccagcccaccggcaacggccggcgccagtccttcgcccacatgccgatgccgcgcatgaccaacaccttcatggagggtgggcgcgacaacaaggccgacatgatcgcctcgactaggcgcggtctttacgccgccaacttcggcggcggccaggtggacatcaccaacggcaagttcgtgttccagtgcaccgaggcctatctgatcgaggacggccggatcaccgccccggtgcggggcgccaccctgatcggcgacggcgcccccgcgctgacccacatccggatgatcggggacgacttcgcgttcgatccaggcgtcggcgtctgcggcaaggcgggccagggcgtgccggtgggcatcggccagccgagcctgaagatgggcgggctgaccgtgggcggcacggccgtctgacgcccggcggaaccttcgccgcgaatcccgggttcaagctccaccacaacaggaggagatttccctatggccgatgaacgcgtgaccgaacgaaccgacggcgtgaaccacgagcgcgtggtcgaacgcggcgccggcggctccaaccccgtgatcgtggagcgtcgcggcggcggcatgggcggcgtgatcgccctgatcatcggcttggccgtggtcgcgctgatcgcctacttcctgctcaacatgaaccgccaggaagaagtccgcaccgacgcggtgtcggccgcggccgaaagcgtgggcaacgcggccgaaaacgtcggcgacgccgctcgcgacgctgttccggatcgcccggcgaactgatttttttcgatcgggggtctcagcgccagtccggccctgagacctccagacccttggccttcaggcggtcgagcacgccgtcctcgccgcccacaaggttcagcggcgcgaccgccatggtcactccgtgctcggccagcgccttgtcgatcccctcgatccaggcggcgcgcagttgagggccgatggtggggtcgccccacggccagcagcggcccagcgccttctccagcggcgaatccagcaccgcccgcacgcggaaccgcgtccagtcctcgccgcgctgctgaaccggcccggcgcccgcctccgtcgcctcaatcgccgcctgcatgcaggggaccagccgctcgggcggagccgtcagcaaatcctcgacgagttggtcgccgcgtccgccggtcacggcccgcaccgggatgcgcgcctttctcgcggcgcggcgcaccacgtctccggcgtcgtccgccgtgtcgcgatcgaagtcgagctggtccgtcagcaggtcgcggctggagagcagaaagctcttgcggctgtgatcgacacggtagcgcgcctccagcgcgtccagcctcgcctgccactccggcgacagatagtcggccgaggtccgcccctcgggcaggcgcgtcagggtgcgtgagcgccagatcagccgcaggatatcgccgagagacccttgcaccccggtgcccagcaggatccggtccgcgcgcagcgtcgcggcctccagcgcatcgggccgccaggcgacggaccgcggcacgccgtcgatggcgccgaccagcagcacggtgctgtcgcccgccgtcaccgtccacatgggcgcccccgaacgccgcgcggtgacgacgatcgtctcgacctcggccgcggcctcatccgcaggcgcctgagtcagagacgaggaggtctgggcccgcgcctccgccgccagccccaagatcgccacgccgcacatcgtcaagacaagtcgcgtcttcatgttcacccctcatgaccgaacactcggcaagtataggcgtgatctatccgacattactttcccgcaacacttacaagcctgtaatgctgtcgccgatttaatccacctttcagccttgtaactggagacaaacaggcccgggcggcacacctctcgcaacatgacgagaggccaaacatgacccgcaccatcctgctgacgaccaccgccctgctgctgagcgcaggcgcttcgtcggccgaaaccacgccgcccaggcccgcgccgcaggcggcccaggcccccgttccgaccggccccacgacggtggcgccgctggccgatgcggcccagcagggcgtgctggtcttcacccccgacttcttcgccgatcagcgtccggatacggcgctggacatggtggagcgggttcccggctttcagatcgacgacggctcgggcgcgcgcggcttcgagggcgcggtcggcaacatcctgatcaacaacgcccggcccgcctccaagaacgacaccggctcgtcggtgctgtcgcgcaccctgtcgcgccaggtggagcggatcgagctgatccggggcggcgcgcccggcatcgacatgcagggctattcggtcgtcgtgaacgtcgtcctgaaggccgaaagcagccgccagtcggtgttcagcgccaaccgcgtcttctttgaaggcggccatgacgtgtccggcggctcgtaccagttcaccgcgcgcgagggcgagcgcagttggggcgtgaccctgtcggacggcgtcagcatgagcgactccaacggtcgcggccgcacgatccgccgcgacccctcgggcgtcgtcacccgcgacgagcagacggtgaacgacggctacggcgggggcaactccatccggggcaactacgccggtcccctggcgggcggcaagatcgacctgaccgcccgcatcggcgtcaacgattggcagggctacgacatcagccagagccccactgtgttccgcgaaaaccagagcgcggaagacggtgtgaacggcgagttcggcctgacctacactcgccccctgacgcccacactgaagctggagacccggctgatccacgaattctccgactatgacggcgcctcgacctacactgtgctgaatgatgggttggaccagcccgagcaggtcttcagctatgacggcgagagttcggaatcgatcctgcgggcgctggtgcgtcaggagcgttcgccgcgcatcaccctcgagctgggcggcgaggtcgcctacaacatgctggacaccgaacaggcgttgacggtcggcggcgtggtgatcccgctgcccagcgcctcggtcaaggtcgaggaaacgcgcggcgaggccttcagcaagggcacataccgcgtgcgccccaacttgacgttggaagcgggcctgcggctggaggcctcgaccatcagccagtcgggcgacgccgatcaggaaaagagcttcttcttcgccaagcctcgtctgctggccacctggacgccgatgccgaacaaccagcttcggtttcggttcgagcgcgagctaggccagctggacttctccgacttcgccgcctcggccgacctggaagaggagaacgtcttcggcggcaacgtcgatctggagccggaacagcgctggatcagcgaactgacctatgagcgccgcttctggggcgaaggcgtgctgtcgctcggttatcgccacgacgagatcgtcgacgccatcgacgtgatcccgctggccgacgacctgtccgcgacaggcaacatcggcgacggctcgctggatcagctggcggtcagcctgacgctgccgaccgacaagctcggcgtcccgggcggtcagttcaaggtgagcaacagctggaatcacacggaggtcaccgatccgaccaccggcgagacccgcgccatctccggcgtgcgtcccagccaggccgagttcaacttccagcaggaccttacccgctggaagctgcagtggggcgtcttctacctggcgggcttccgcgaaccgcgcttcgaccccgatcagcgccagctggtgcgcatcagcgactacaagcaggcttggatcgaatacaagccgacggccagcctgaccctgcgcggcgaagtcaccctgtgggatgatttcaccatcgaccgcaccttctacggcgaccgcgaaacgcagacggtcgccttcaccgaacaccgcgagatcgacccgcggactttctatcgcgtcagcctgcgcaagacgttctgacggcgacgtggctggaatgaaaggccccggcggatcgctccgccggggcccttgtcttcttcatggtcgtcggatcagtggacgcccgccatgcccttcttcagcagcggcgagatcaccaaaaggaagacgccgacgccgacgccggtccagccgatggtgccgaagatggagccgtaggtctccagcgccagctgcgggctggtcaccacgcccgcgaccgtgtccgtcgccgtggcctgggcgatgatgccggcgacgatgtgcgccaccgagctggacaggaaccacacgcccatcatcaggcccaccacgcgcgccagcgacagcttggtgatcatcgacaggcccaccggcgacagacacagttcgccgatggtgtggaacacataggtcaggaacaggaaggtcagcggcacgcggaaggcgtcattggccagattgtccgccgcaaaggtcaggaccaggaagcccaggcccacgaacatcaggccgaacgagaacttgaccggtgttgacggctcaagcttgcgcttggccagccagacccacagggccgccatgatcgggccgccgatgatgatcacgcccgggttgaacatctgggtgtagccggcgttgaaccacgacggcatctgggtcgactggtccgcgaacagggtcagcgaagagccggcctgttcgaacagggcccagaacagcaccgagaagaagatcagcacctgggccaccagcatgcggctgcgctcgacgcccttgagcctcaatacggtgtatcccaccacggcggcgaagatgacgcccgcgatccacggcagcagggtctcgatgatctcgtgccgctgcatcagcagccacaccggaatcacgcagatcaggccggcgatccagaagaaggcctcgaccggaacgcccaggatggagcggcccttgagcggcacgggcggcccgccgcggccctccagccagctctggcccagcacgaacgtcagcaggcccagcagcatgccgatgcccgccaggccgaaaccgtaggcccagccgtaggtgaagcccaggtaggagcaggcggccgtggccaggaacgagcccaggttgatgccgacatagaagatggtgaagccgccgtcgcgacgcggatcgttctcttcatagagggcgcccaccacggtggagatgttggccttcagaaagcccacgcccatgatgatcagcgacagcgccaggaacagcaccggctcgcccatcgccgtgtcgcgcgtggtctccagcgaatagccgccggtggcggtgaaggcggggaagccggcctgggccgaagcttgaggagcggcctgcgtcgccggatcgagcgcccccgtcggcggcgtgcccaagcccgtgcccacggcggcggcggccgcatcggcggcgttggcggccgacggctcggcgcccacggtggagacgccttccggcgagatcgcgatctgcacgcgctcgtcgccgttgacggcgaacatgcggcggttctggtcgcggccctcgacctggatgtcgtaggtcgtctcgccgatggtcaggcgctcgcgcccgcccgagccttcaaacgccatggtgaagtgacccatcaccagcagcaccgcgccgatgatcacggccttgcgttgtcccagatatttgtcggcgatcatgccgccgatcaccggcatcaggtaaaccagggcggcataggcggcgtagatgccctgcgcctcggccgggccgaacaggaagtgctgcgtcaggtacagcaccagcagcgcccgcatcccgtagtaggagaaccgctcccacatctcggtgaagaacaggatcaccagcccccgcgggtgacccagaaaggtcttgcgaggcgaaagcgcccccccatccgtcgtcgtcaacggctcactcccaactgccgcgcctcggacgggcgcgcgaaaggcgcataagcagcacgggctgtttgtccgaacaagccttaacctcgtcgagccagcccgcgcgcacctttgcgcaactttcggttgttagtagtggcccgtcatctgcaatcaagggcgtcatgccgttcgcgcgtgccagacagggatggattccaggatgatcgtgcgcacggtccaggcagacgactaccccgggctcaatcggctgcacgcctcggtgggctggccgcaacgctcgccggacggctggcgctggctggccgacaaccccgcgcggcgcgagatcggcgcgcccgagggctgggtgctcgtcgacgccgccgatcggccgtgcgccatgctgggcaacctgatccagcggttcgtgctggacgggcgcaggctatatggcgcaaccggcttttcgatcatcgtgccgccgcagcacaagggcgccagccgtccgttgatccaggcctttctggatcaacccggcgtgttcgcctgctacacgctgaacgcgaacgcccggtcagcgccgctctatgggcgcctgggcatgcggccgtggccggaacagacgcacgcgctgaagctgtcctggaccatcgatcccctcgcctgcctcgcgggccgggtgctgcgtcgggtctatggccgcatctccgccgaggccgcagaggggatgggcgaacgactgatgaaccggcggctgtcgcagcctcaggcgctccggctgccgggtgacgtcgtggaaattcgcgacgtctctccaggctcctcctatggcgagttctggcgcgcgctgtccggccagggcggcctgtttgcggaccgaggcgccgagatgatgcgctggcgcctggccgatccggacctgccgcgccggcccctgctgcttggccggatggagaacgggcggctgaccgggaccgccatggcgatgacatccaagaccagcctcatcgatccgcccagcctggagatcctggatctgcaggcgctggacggctcggacgccgttcccctgctgacgcgcgccctgatccgcaacgcacgcggcacgggcgcggccaaggtccggctgcaggcgctgacgcctgaactcctgacccgcctgggcgcgctgggcggatcggcgcgtcgcgagggcggctggggtcacggccacgccgtgttccgcgacgaagccttggccgccctgtggcggccgacgccgctggacggcgattatctggtgtgcaaccgcccggccccggtcgcgtccgggcgtcgccagaccacgcgccgcagccaggcgggccaggcatccaaggcttgacgcccggtcaggcgcccgggcgctggcgaagttcgtcgcggatctcggccaagagcgactcggtcgccgtcggcgccgagggcgcgggatcaggctgggccgcctgctgccggcgcagggtgttgatccccttgaccagcagaaacaccacccaggccacgatcaggaactggatcaccgtgttcaggaaggcgccgtactgaaccgcgactttctcgacctcggcggtcgcggggttctccggccgcagcacccactccagctcggagaagtcgatgccgccggtgatcaggccgataggcggcatgaccacctgatcgaccaggctcttgacgatgccgttgaaggccgcgccgatgatcacgccgaccgccagatcgaccacgttgcccttgacggcgaactcacggaattcggacagcagtcccatggaggctcactcctgctcgtcgcccgaggcgttcagccgctcgcgcagctccttgccgctcttgaagaagggcacgcatttggcgggcacctcgacggtctcgcccgtgcgcggattacgtcccgcccgcgccgggcgcgcccgcaccgaaaaggcgccgaagccacgcagctcgacccggccgccctcggccagcgaatccgtcatcttgcccagaacgacgttcaccagccgctccacctcgccgtgcgtcaggtgtgtgttctcggccgccagcttttcgatcagctccgacttgatcatcgcgccccgccttttacgcggaccgacgttctcgcgccgaccccttccgcgcgcaccctagccgcagaggtccgggtaaaaaagccccagtgagattcagtcgcgcctgacgcgtctccgacgctccgacaacgcttgtcccacaacaagaaaagggcggccggatcgctccggccgccccttcaagacacagcccgcaggggccgtggttcttacgagttgttgcccgcgttcttcagcgcggcgcccaggatgtcgccgagcgaggcgcccgagtccgaggacccgaactgctcgatggcttcctgttcgtccttcatctccagcgccttgatcgacacggagatgcggcgcgaggccttgtccacggcggtgatcatggcgtccacgcggtcgcccacggcgaagcgctcggggcgctgctcgttgcgatcgcgcgacaggtcggacttgcggacaaaggccgtgaccggcgcgtcgtcttcaccgaacttgacctcgatgccgcccgactcgatcgacgaaacggtgacggtgacctgctggccgcgacgataggtgtcgccctcgccgatcggatcaccgcccagctgcttgatgcccagcgagacgcgttccttctcgacgtcgacgtccagcaccttggccttgacggtttcgcccttccgatagcgctggatggcttcctcgcccgagacgttccagtccaggtccgacaggtgcaccatgccgtcgatgtcgttgtccaggccgatgaacaggccgaactcggtggcgttcttgacttcgccctcgacggtcgagccgatcgggtggttggcgacaaaggcgtcccacggattgtcttgcgcctgcttcaggcccagcgagatgcggcgcttggagctgtcgacgtccagcacgaccacgtccacttcctgcgaagtggagacgatcttgcccggatggacgttcttcttggtccaggacatttccgagacgtgcaccaggccctcgacgccggcttccagctccacaaaggcgccgtagtcggtgatgttggtgatgcggcccgtgtacttggcgccgaccgggtacttggcttccacgccgtcccagggatccgactgcagctgcttcatgcccaggctgatgcgctgggtgtccgggttgatcttgacgatctgcaccttgacggtgtcgccgacgttcaggacctgcgacgggtgcgacacgcgcttccagctcatgtcggtgacgtgcagcaggccgtcgatgccgcccaggtccacgaaggcgccgtagtcggtgatgttcttgaccacgccgtcgcggacttcaccctcttgcagctggccgaccagctcggtgcgctgttcggcgcgggcttcttccagaatggcgcgacgcgacacgacgatgttgccgcgcggacggtccatcttcaggatggcgaagggctgttccttgcccatcagcggaccgacgtcgcgcaccgggcgaatgtcgacctgcgagcccggcaggaaggccgaggcgccgcccagatcgacggtgaagccgcccttgacgcgaccgacgatggcgccgttgaccggctggccttcggcgaacacgccttccaggcgggtccaggcctcctcgcggcgagccttgtcgcggctgatgaccgcttcgcccagggcgttctcgacgcgctccagatagacttcgacgttgtcgccgaccttgggcaggacggcgccttcgccctggccgaactcgcgcatggcgatgcggccttcggtcttcaggcccacgtcgatgatgacgatgtccttttcgatgccgacgacgcggccgtggacgacctggccttcgccgaggtcgcggccctgcagttgttcgtcgagcagcgcggcgaaatcgtcgcgcgagggggagagagtgtcggtcatgtagcggtttaggcttccgatggggttgcggcgcgcggccgtgcggccccgcgcgaggtggacagaaaggataggcaggtcgtcaggatgcgaggacgacaggatcgctcagaacgcccgcggaaagtccgagaaccggtgcgttggatttgccaggttgggtcagagaccgtgccgggcgcgcgccgcctcgacgatacggcgggccgcatcgaaggccgcctctatacccatgtcggtggtgtccagcaaggccgcgtcttgcgcctgcaccatgggggcggcgccccggccggcgtcgcgctcgtctctgcgctgaatatcggccagcatgtcttcaaaggcgatgtcgtcgccacgcgcggtcagctgcttccagcgccgggtcgccctcacctcgggcgtggcggtgacgaacagtttggcgggcgcgcccggtgcgatcaccgtgccgatgtcgcggccgtccagcacggccccgccagcctgcgcggcgaagtcctgctgcagcctcagcagcgcggcgcgcacctccgggtggcccgccacccggctggcggcctcgccggcctcgcctgtcgtcaggcgctcgtcctcggctaggcccgcgggaaccagggaccgcgcggcggccgccgcagcttcctcatcgcccaaggcgtgaccgtcgcccagcaccttcacccccaccgcgcgataaagcagaccggtgtcgaggtgcggtaggccgtaggctcgcgccagccgcgcggcgatggtgcccttgcccgaggcggcagggccgtcgaccgcgatgatcagagacatctggccgtccctttatgcaggccattcaagcccaaggcggcgaccgccacacaggccagagaaagcacgctgaagacgcccacaacgctccagaactgctggggatcagacgtgcgatcggccacgaccgctccgacgggtcgcatggtgaaaaggacctcgcccgttctcagccacgcaagcacaggcaggccgaacacgagcgcgccaaccatccccccgcacaatcgtgccatcggcgacgaaagattgaccgtcgcgtcgatcattcgccgatccgtccgcctagcccgttcatcgttccgacaaagccggggaagctggtggcgatcatgccagggtcgtcgacggagacgggcgcgtccgccgcgaggcccagcaccaggtggctcatggcgatgcggtggtcgtgggcggtacgaacgacggctccgcctctgaccggacctcccgtgacgatgaagccttccggctcctcctccaccgcgacgccgcagctgcccaggccggcgaccatcagggcgatgcgatcgctttccttgacgcgcatctcgccgacgccgcgcatcaccgtctcgccggcggcgaaggcggccgtggcggccaggatcggatattcgtcgatcatggaggcggcgcgcgcctcaggcacgaccacgcccttgaggtttgaatggcgcgcggtgatgtcgccgacctcttcgccgccggcctcacggcggttcgagatcgtcaggtccgcacccatttcgatccaggtgtcgaacaggccggtgcgaaggggattcagcatcacgccctcaaccgtcacctccgactccggcgtgatcagcccggcggccagtggaaaggcggccgaggacgggtcgcccggcacggccacgcctgttcctcgcaggccttgcccgcccttcagcgtcacgcgccagccatcgcccgcgggctctacgcccacctcggcgccgaaggcgcgcagcatgcgctcggtgtggtcgcggctcttttccggctccagcaccgaagtgacgccgtccgcattcagcccggccagcaggatggccgacttgacctgggccgaggccacctgctgctcgtggtcgatagccgtcagggctccgccggtcagggtgaccggcaaccggtcctcgccggccagccagccgaagcgcgcgcccatccggcggagcggcgccgtcacccgcttcatcggccgcttgcgcaggctcgcgtcgccgtcgaaggtcgccgtcaggccgtatcccgccgcagcccccatcaacaggcgaacgccggtgcccgcattaccgcagtcgatgacgtccaccggcgtctcgaagccgcctttccccatcacgcgccagcggccggggcccagacgctccacgccggcgccgaaggcctccacggcgcgggcggtggccaggatgtcgtcgccctccagcaggccctcgatctcggtcacgccctgcgccatgccgcccaggatcagcgcgcggtgcgagatcgacttgtcgcccggcgcacacacccgaccgctcagggcctgggatcgtcgcgcggtgaggtgagaggtcatggcgggcccgcgtgaaagctggtcatcaggggatcggccgggcgggcggcgcgaagatcgcttttgacagcggccccgtggggtggcaagggaccgccccgaattccacctgttgaaagtatcgccgtggccaatcccgaactgggcgccaagcaggtctgccccaactgtcaggcaaagttctacgacctgaaccgccgccccgcccactgccctaaatgctccaccgacttcgatccggaagaggcgctgaagctgcgcagccgtcggagccgtcccggctatcccgccgatgacgaggccgaggatcaggtggtcgacaagaaggccgaaggcgacgacgaggacgaggacgaaacggttcgcgctcccgagatcgacgaggaaggccatgagccgattctgacgcccgacgacgatgaggacacgccgaacgacgcatcggaagaacccggcatgggctcgacagacggcgacgacgacgatgtcctggctgacgacgacgatgactccgtgcccttcatcgaggacgaggacgacgactccttcgacgaagagatcgccaagccgtccaaggacgacgactgatcttttcacctgcgcccgtcgcgcctcccgctggtggaggcgcgacgggacagcagcgggattgttgattccgctgtattttcggcccctggaacccgaccgaaaataaatgtcgaaacaggcttgatcgccgaaaagcttcgacataggttccgccgcctcgccgggggccgttgcaagacgaaccgggcgacaccagaccgaaaggtccggggctatagctcagttggtagagcgcttgaatggcattcaagaggtcagcggttcgactccgcttagctccaccaatcagtctccccctttcaccggccggccggggaagggggagactggccactcttttcagacagttagacggttaacgcggacgccaatcccgccgtggagaggatttccgcgcggtttggccggctgttccccgccccattctccaggcccatgtttccacttccgggtttggccgcaggtgtccgcggagaagggttagcccgaaccgagccgccgccggaggaccggcggcgggatttaagtctccgatcgtgaggaagggtcgggtctagccgaccgcgccgatggccatgaacagcctgcgctgctcgttccaatccatcgggaagggatgggcgatcaaggcgccgagtgacagggcctggggctgacgtcccgcgatgatctgctccaccagatccggcgccatgtaggccaggggcaggatctggccgaggtagcgaacacagagattctcggccttggccagttgggcggtcgatccatgacgaccggtcctgaggtcggccgtccatcgcctggccatggcgacggccctgaccagggcgcgatcgatccgattggcggccgttggggattgtccctcggcctcgatcaagaccgcgttgtgccggtgcttcagccggaccggcaggatccactcgatctcgccatcggcccgctcctctcgttcggcgccctggatcgttcggtcaccaggaatcgctcccttggccgtcaggatacgaacctgagtctcgcccagggtgaccttggccatggcggttctcaaacgctggtcgggctcggcgtccagcctccaggctggatcgagcgccggaaggatcctgttggcgacgaaggcctcgatcaccccggcggagattcgcgtcacgctaccggcctcgtccttccttccattttccagggcgaccgaggagtaaaaccggtaacgctggccagccttccccatggtatgcaccggccgcatcgtatgcccccggtcatccttcaggatgccgcagagaaggccgctggttccccgggcgcgatcctcggcgagcgattggctgcgtcgtgtcaaagccgcgttgacggcctcccaggtctcgggaggcactatcgcctcgtgcgccccctcgaccagcttctccttgtgcctgagcgcgcccttgtagacggggttcatcaggatcagccgcaaggcgccgggactgatcacggccccgccccgaaccttgccggccttggtcgtccggagcttggatcgaacgccctgtcgcctcagttcggcctgtagttccaggaccgagcgcagttcgaggtatcgctcgaacatcatcctgaccgtgggcgcctcatcggcgttcgggatcagcctgtggtccacgccatcgtatcccagcggcggcggccctcccatccacatgcccttggccttggacgccgcgatcttgtctcggatccgctcggccgtgacctcccgctcgaactgggcgaaggacagcagcacgttcagggtcagccgtcccatgctgttggtggtgttaaaggcctgggtcaccgagacgaagctgacgcccctggcgtcgaaggcctccaccatcttggcgaagtccggcagcgaccgggtcaggcggtccaccttgtagaccaccacgatgtcgatctcgcccttggcgatgtcggccatgagttgcttcagccccggtcgctccatgctgccgccggaatagccgccgtcgtcatattccctgggcagggcctgccagccttcgccggcctgggacaggacataggcctcgcaggcctcccgctgggcgtgcaggctgttgaagccctgttccagcccctcctcggtggatttacgggtgtagatggcgcagcggagggctttcatggccgccccgctttcctctgaccgaagaaggccggtccgttccacttggtgccggtgatggcgaaggcgacctgactgagggaagcgaagtccctaccccggtagttgaagccttcctccttcacccagacctcatggcgttcgcctcgccagtccttcacgaagcagctaccgggcttaatcctcggggcctgggacggctggtaggcctcgtcctcggcgaaccgctccgccaacctggccaggcgctgttccatcgtccgggacaggccgccctcgcgggcgacctgttcgcgataggcgatctcccgcgccatcaggtcgcgggatctgagctttggcggagcggtcatgaccttgtcccgccattccgcccgcaggccctccagggtcaccgtgtcttccgccatcaggcggccgtgatgcgatagacggtcaggcccccgaccttctcggtcgcgaccgtcaggcccagcttcttgcgaatctgcccggcgatggcgccgcgcacgctgtgggcctgccagccggtcgccgccatgatctgagccgccgtggcgccttcggggcggcgcagtagggcgaccacctggctgatcttgctgaagcgcgcgggctgtgacgcaccttcgccagccggcttcatattgttctggttcatgatttctctccatccgcacccttgcggtggagcgaccaacgcttgcttccgccgccaagtccaatggaagaaggagaaatctcagccttcggattctgtccgccgaaggagttccagggcgcgggccaatatggccgtctcatccgcgagcgccgccacatctggcagggcagccatcacgtcggaggccgtggccaggtcccccgcctgctccagccgcgtccagatcgccgacaacatcatgtcttccaaatgccggggtcgggggtcatcgtcttcactctcggtcatggcctccacacgggcttccttcgaccaggaagtcgagggcgagacgcgtggaaagtcgggttggcgccgatttcgttgaaaaaggcggctgctgaggtcgccgccagtaacggacgcggcggttctctcccgcctcacgcggtcgctggcgtcagcggcgggatcagtttggccagtttgcgcaggttctgggcggtggcggcgaggaggaactcgtctttggcgccgttgggacctcgcaggcgcagtcggtccagcttcaggatgcgcttgaggtgggcgaacagcatctcgaccttcttccgttcgcgtctagagacgacgtaggcgtcggttctggcgatgtcgcgggcgaagtcccgcgcgccttcgtggatggagcgggtcactttccgcgccggcgctttggggcagcagcggctctttagcgcgcaggcgtcgcaatccattttgctggcgcgatagcgataggtgttatccggcggggtatcggggtggtccgcgcggaagggccgccgatgttgcttcagctccttgccgcccggacagcggtaaaggtcggcggcatggtcataggcgaagtcggcgcgcgagaaggtcccgtcgatccgctcggatttatcgatgaccgggatgtgcggctcgatgccctggtcgtggaccagccagtccaacatctcggccgagccataggcggtgtccgccgccagccgggcgggccacagatcatgatgctcacgcgcacgctcgatcatggtgcgagccgccgtcacctcggcttggcgcacggcggtggatggctcgacatcaacgatgatcgcgtggtccaggtcgatcaggtagttggtggcataggcgaagaaggccaggcccttgttggcgccggtccagcgcgaggccggatcagccggcgagatgaacttgggcgtcaccggagtcgcgccgccgaaggccgcgtcgtccagaacggccaggtactcgtcaatggcgcggctggcggcctcgggcggcaggccttcgtcgcccggcacgcagcgttggcggttggcgtcggccttgatcaggctggcgtcgacggcgaagccctcgccgccgacgagaccctcggccatgcagcgccgcagcaccgtctcgaacagctcccgcagcagatcgctgtcgcggaagcggccatggcggttcttggagaaggtcgagtggtccggcacgtcgccgtccagccccaaccggcagaaccagcgataggcgaggttcagatgcacctcctcgcacagccgccgttccgagcggatgccgaagcagtagcccaccagcagcatccggatcagcagctccggatcgatcgaggggcgaccgatggcgctgtagaacggcgccagatgcgcccgcaggccgtccagttccacaaaccggtcgatcgcccgcagaagatgatccgccggcacatgccgctccagcgagaactcgtagaacagcgccgactgatcaacccgccgctcacccatcatcgctgcacctcccgtctcaacgaccagagtgaatcagcgcgccgccttcatgccaattgccaacggacgcctttttcaacgaaatccgccaaaagcggacatgcggaagccgctgtatagtggacgtctgcggcgtcggcagggcacggcatagacatgggtttgggaagagaatgacgatccaaggcatcacatccgacatgcgacagcaactcaccgctgacgcggagcggctgcgaggcgtcggcttaaccgcactcatcgactattatgcagcggctgacgatgtgacgcgggaggctgccgacgcaaccctcagggaagcctataacgaggccgtgaaggcgcagcgtcggcaagacgcgcttgaggagctacaagcggaacatttagcgaagagcgctgacattgcgcagtggctaagaactctgacagccgccaacacgtaactcgctaggcagctcttccaccgagggatgaaggcacgatggttgggattgtagtcgggccaggccatcaggtccaaatcgtcgggcatggcctgaccgtcacgtccgatttcaaactcgccgacggcgtcacgatctctgctgggacgccgatgcgtcagacttcgttcgggacgacggtgggccagctgagcgaagacgccgcgctgattgtaatggaacggctcgccgatttctcgctggtagtctgcgagcctcaaggcggcgagttacttgcggcaaaggcttggaattcgctgtggacgtttagcttgctgggccttgctatcgctgctccggtgatgccgctctacagctactctcaaagtgcaggcttcgcgatcgccaaccgaaacttggtcttcaagcccttgccccgcgccgtcgcagcgacgccagagaacctgcgatgggctgccgaccactatggagacttcgcgaagctgctttccaataacgcttttacttcggcgcaacggtactacaacaatgcgcaatatcttcccgatgacgacgcccggatcatgctgctttgggcggggatcgaaggcctagtgggggtcgaggcagaaatcactcgccggctcgcgctcaacacagcgatccttctacagggcagtggggacgaaaaagctaggatcttcgcggcggtaaaagctgcctataagcttcggtcaaaagtggtgcacgggggtggtggcgatgccgaaacgctgcgccgagggtacgagttcgccagcgatctactagcgcgacttcttcgccgcgtagtcgaactcggccgggtgcctgacgtagctgaatacgatcgggttgccgtcacaggcgagctcgagttgctcgaacgaggtggcgcttaggtagcgtaaagctagcgacggcccgcaagcgccaggagcggttttatcgccgacctccaaaaggcgacattcagacgggctacaaggtccgctctccgccattcggccttgccgcagctattcggcaaggccgcctaggcgactctcctgtcccggcaagcaaatttgcgcttaagtgaagacggacgaggtgtggggtgatccatgggggcggacacgcttagtacaatcgaagctcggctggaggctcacctgggcaagctcgcgaatgggagccttggccgaaccatcaccatgatcgaggtagtcgatgctgcagccctttggtcagatccgctcctcgaactcccccaactcttgggcggcatcgacttcgaggcgctgatcaaggaataccccatctctgcttgtgccgcggcgagtgagatcgggtaccggttcgagggcgttggaacggtcttctgggggaagtttgaagggttgctgggccggccgatcccggtcgggcagcgccacctcctttcatcagcgttcggcagtcttgctgaccgcttcgccctacagcgacctagtgacagcggattcgcgacgcagttttcaatcatcgcgtggccgatcgcaaacgcgctcatgccctacgaattggctgggcccgtctcccggctgctcgcgcgagggcccgtcgccggcgtggcctcagctaccagcacgcgcaggccggacctctcctcccttcgcgcctgggctcagtcgtgggaaggggcccgactgtcggactggttgcagccggagggaccggcggcgcgtgtgattactgcgctactgggcgacaatgggaagggatcgctgcccgatccgaccttcgagcgtctcaaggctgcgtttgcccaccagtcagaggcctttttcgcgttgagagaggcgagacggcgcaggccgacgaccacgacgccgttgctgccagagagcggggccctggggttgcggcggatcggcgaagagtttgtattttcggtcagttggccaagtctccctccaccgctcgtcgaactgggccggaagcaggcgtcagcgagagcttggcgtccgaagctctggggacagtcgcggacggcctccgacaacatgtttgggtcacttccgattgtgatccggctgacggccctacccggtggaaacgggccagccgcggccgacgcgcgaactgtcttcgaggacgaagcggagatcgcggaggcccttatgggccgcacggtggattgggacgcgcccctcgttttcctgcgagcgggcgacgaggccgatcggattgaattgcctattcgcctcgaccagggccacctctgggtggtggaccaggcgggcaagtttgagagccttgctgccgagggggttgttgccggcgcccccgttcggcgggcggacctttctgatccccatgatcgcgcgctgctggcggaagcaaggtggcttggcggaagcgtatcttcgacaaacacggtagcacgcgctccgcaggacgcgcttacgcttccccggcggcacgtgacagcgcagacgccgttttgcgtgatcaatggcgcaggcctgcggatcgagaagttgagccgccgggacggggccgctcacggccttacggtgagcgctccacgcgagccaatgacggcgacgccgggtgtgttcctgttcgaaagggagagcgcgttcgacgctctgatcgaagagcgcctactggcgaaaatccaaagccccatcccgggtgcccgctggccggtcgagatgcttgcgatgatcgacgatgagatcatcgcctacgccactgatgaactgagtgacgaggggaccgggctggctcaatcgagcctgatcctcaacgcactacaggctgagcacattcggctgagaatccttcaggccgggcgtgcgacgctccgggtgcgcgtcgggcggcacccttgggatacggtgcatttgcgacggcgagacggtgatatcgactggtcggcggaggagcctggagcagggctcggccggcccactcaagaagtggtcgcgcaagcgcagcggcccttccggttcaaccttgctggaccgggcggcggtgccatccttcggaccttccgcttcgacgatgggcgcctcgccgcaccaggaagaatcgaggcgcctgatcagtttggatttggggatctcggcagcaatttctcgggaatcgaagggcgccggcggctacgagaggacggcggcggcctgatcgacctagctcgctcacgtcgcgcttgggccaccgccgaggcaaggagcattgcctctgtcgctgcgcgcgtgcgcgtcgtccgccaatttgaagacccgctcgtttcagccctgtgcggtccagaatggcatgcgctggaagggcgcgctgtgacggattcgccgtcgatgttgctattcgacaatatcctaccgcacgcggtcggagaccaagctggcgcgcttgatccgactgatagggccgattttgccggtcgcttcggcgaggctctggcgcggtcctgcccggattggacagacgaaggtgtcattgatgatgcgtgcgccgaccaagcgctcgtcgaggcgttcgccgagatgctgcggaacgcgcaggcccatggacgaatggttgagtttgacgcggacgatatggacttcggcgcctcggacgaccagtggcgcgaagctgcgatagcggcgctcgaggcgtcggggcgatcgccgttgatggatttgatcgcaccgacgtcgggagcgcgggttcttggccggcgagggttcgcgggtagcgatctcgcagaggcctcagttttcctcgcggattggaccgcggcatgggcccttccgcggagccagattggtcttgatgctgcttgtgaggcgctgcagttctggttgaaccccggagcagcggatcccgacaccggcacctttgcagccatgtccagggatgtgtttttggcgcggacggtacggttcgtttcagcgcgcatggcgcgggcggcgtgatggtggaccaactcgctgcatactggttgagcctccacggccaagcgcggctggcagatgccgaccaagctttactcggcgccttaggggtggccgcgttcagctatccccatcaaatcgacaatgtcagtcaaatggcgacggacacggcgtgtcggttcctcctggccgatgaggtcgggctcggcaaaaccatccaggcccttatggtgctgcgcgctctcgctgctcagcgagacacgggccttcgcgtcgccctcgtgacgccggacgatcttaatcaccaatggaacgaggaattcctgtgccggacgcacatcggcgccggtggcgtggcgatcgagccggatgaggagagtccgcctcttcgcccgaggaagggtcacatcgccgtcgagctgttccgccctgcccgtttggccgccggcgccgttcggttgaatgcaaaattctatgatgccctggttgtcgacgagtaccccaagctcgggcagcagatgcgcgatttggtgggcgccgcgagccgcagtattccccacgtgctgctgttgagcgcgacgccggccttgcacgatgaaggtctgcgtcgtgctatcttggagatcctggagcctgatcttgctcgccgagcggacgcgtcaggcgaggatattttggagttgctggcagcccgcgaagatgaggcgtttgatttcattacgggcaaggccgatgaaccggagggcctaacgacgccagcggggatgggccggagtttctacgccgagacccacggcgcgtttcgccgggtgatccggacgaggcgagccgactatccagacgcgctgccgcagcgtcgttaccgggcgatagtcgtggcgccgactgatggcgacgcggatcgtgtcgatgccgcgaggcgctacctgggggcggcagtcagcgagggcgtcaatgtccgcggcgaggcccttctacagacagccctggcgagcccccaggcgctgattaatcgggtcagcacgctcaagcggccgactgccaaaatggcgaccgcgctgcgctcactggaagctgccgcccgcgatcttggagacgctaaactcgacgccttgatcgaccacttgcgcgcgacatttgcggccgcaccggcggctcgggtggtggtggtcgccgacgacaaccgaagcgtcgatcaccttgcagcagccatcgaaaagctagtcgaggtcaaggtcgccacgaagcggcgggcctacggcggatcggatgtcgaaatggacgtccacgttgcgcagttgcgcgatgaggtcgagccgttcgagtcgggcaaagcgaaggtgttggttgccgcggatgtggcggctgagggtcataatttccagttcgctacagaactggtcttctacgttctcccttgggacccgcgggacgttgatcagtggatcggtaggcttgaccggctgggaggtaagggtcggccaggtaaacgaacgatccggatcactccgattgtcactcgtgattccatcgaagcgcggatcctcgaggtctacgaggccgccgatgtcttttcgggtgggcgggtattcgatgaggatgcgtggacgagcctggcgcaggcgatcgatacggccgcctacggcatctcgggtaactggcctgcattgatctcggcagcgacggcgcagcgccgggacattgagggttggcgcagctactcgcgcttcggtgcgccgaagcgggcggctgaggcgaaagcccgctacgaggcgatggtaagccagcgttatgccttgccaatgtcggacgcagacgatgcaccgagaccaaattggttcatcgagcgtgaggcgggtgcaaaacgtcttctcacgctttccgatgaactgagagtcctgcggcttcagaaacggactgatgagaagaccggtcagccctacaggaccctctggtaccctcatcggcctgagcagggcgacgtcgtcgttcccgagctggaaacggacgggccttggcgtcatgtggccctgctgctgaagcgaaccgacctacattcaccgcccaattccaatgtcggcgaacggcggctgcacttcttcgaccatggcgacccggttcacgacagtgtcatcgagaccttctctcagttggcgtggacgagcacgacgaagaacgagcacgtcgttcgcgtgccggaggatcatccggcgtccgggctcaagggcgagcgggtgctactgctcagcgccatgctcaggccgacgtcaggacgcccatttgacccgtcgatcctggaggatcggccttcggctggcgatacgcaggccgagcgcgacgcgatgcaggcggctgttcgcagggcctacgaggaacacttggccgatgcgcgctggttcactgaccttgcgcaaccggatctgtttctacttggcgcgcggctcggccctacgcccgaggaaatcgatccgagggtgctggttggagccagtggccgcgtgagcataccggaacacatctcgagccgaggcctttcgcacggcgactcggccatggcggccaccgctcggggggtgctggtcgaacgtctgaaagatctcgtgagggcaggcatggagcaccgcgggcggcgcctcgccggagcattgccgttacgacgcttcaagacccgcatggaggcgcaggaggcgctcgcagccgctcaagcagtcgaggcggccggccgcttgcgtggcggcacactcgcctttgaccgggcgcgacggcgggccaacgaccttgcgatccttctcgctgaggtcggggccgagatgcgccaagctcatctggacggcatgcttcaggcgctaatgacgtcgcagtttacgccccgctccatcgtcctgaaggtgcaatgatcgttaggcggtgagttgttccgcgaggtcagcagccgtctgcgagacggcccatttccaagggcctacattgtctccggataggtctaaaagccgctgcaactgaaatggcggaggcgtgaagcattggagttggccgtcgtgccaatcaaataccggatccccggcgagcctggtctgtccgacgacggcccagcgccagcggtcgaggttggtgacgtcgaccgcgcggacaccctgcgcagacgctgaaattacgcagttctgccagctgtaggttttacgtcgggaggcgcagaacgccccctcccccaggaggccagtccatcgtccgtctccggcaacgacttgtgccttgccgaagtagggcccccgttttgataggacgcgaagcgccgcgggctcggcacgatccaggcgctcgccgcttgcggcggcgccggccagccgtgtgaagaggccccctggtccaccggtccgttcatccatgccgccgagggccagaatgtgaagacgccattcaggggggccgagttcgtccgccagaccgaccaggggcgcggaaatggtctcgatggccgtgtcccgagaaaggcgacggaccaagccggttaccggcgtcgcggaacccgcagacatcccgagaacgacgacgcggtctgcatcgagctcaaccagccgttcgggcgtcgccacgtagcccagtccgccatctgattggaaagcggttaggtcgccgagccgcacaaggatgtcgcagccttggtgaatgagcgggccgagatcgccatcctcaccgccgaaagggctgtagctttccttgagcgctcgggtgatgcggcttcgcagcagatagggttcgacggcggcggcggcgcggatgtggccgacgacggtctcgatcgtggggaggcccgcgtcgtcaagttcggcgccgatcgcctccgcccaagccgcacgcgtcatagcgcttccagttcggttccgatggcggagacgccaatgatggcggccttcatctggtcggcgaagcttgagttctgcgtcaccacaagaaggtggccccgagcacgggtgaccgcgacgtagaggtcactttccgtgaagagcccgccgacgccgttgatgccgtaaagaatgacgacatccgcctccaagcccttgaaactgcgcgccgtggtgcagaggatggcttgcgccattcgctggcggagtcggttagcttgacgccggccatctcggtccagcgggccaacacgccattcttccaggcggtcgggccgatcagcgcgacctgatcagggttcagacgatggtctcgcagcagacgctgtaactcgccttggacaaggccaggcatggcgccttgggtttgggcgaagatgaggcgcggaggtcggccgaggggggccatctctgcggcttcggccgtgatcttggccgttgccgcggcaaagccgacgatgcggcgcgtgttcctgcagttggtgtcgagatgaaggatcgcagcgttttcgagaggcggatcgacggggtcccggcgcaagctctgatctcgatctaggaaggcccaggtcgggacgtcgtcgccgagaccggtcaggtacgcgagcgcatcccaccaccccgggctgaaatcttgagcctcatcgaccacgagagcgtcgaaaggcggatcatccggataaagtgctgcggctgcagtcgccatctgatccggtacgacgacatcccagtaatgggtgttgtcgccgactggatcgagcgggagtcccgccttcttcaggatctccgcggcgaggccgtggaaatggcggatcgttaaagatcctttgtcgtactcgtcgttggcgatctgctcgttcagccagcgagccaattcggcgttgaaacatgtgaagagcaccgagcagccatcccgggcgaaccggcgcgctctctgcaggccaagcatcgtcttgccggacccggcgacgccgtggatggccgcgcgagggttcgccgcgaacccgttcagaatctggatctgctgacgcgtcagtcgggccagcacctggcccgccgcgtcgacatcgagcttcagcggctcatagactgcaaactccggggcgagcgcttggcgcaccgcttcgaattcgggacctgtcagcgccgtgtggaagcgcccgaaggcgtcataggcgcggtcgattgcgttctcgatgtccgccaggtcatccatcgtcataatggtgcgggccggcaagtccgctggcggagtatctcggaaaacgcagtgtgggaaagcgacggcggtcgcgaaccggaccttctggtagatggtttcgccgcagatcagttcgatgcgcttgcgcagcgccctggcggcccttctcacctgctgcgccgggtcacgtaggtccttcagccggccgccgcctactagccgagaccattgacgattgcgcagtacgacctcgccgcccttcgcctcgatgaccagcattcccttctcgcgatggaggaggacgaagtcggcctccccttcgcgaaccggagaagtgaggtcgtcccgctcgggcgccagccacgggaacgagtggaaaaccagataatcgtcgccgaggcgcgtctggaaggccctcatcaggagggcttccgagtcgtgcggcatgttctctggcagggtgtttgggatgcagatcgccatcagacaacccgccggatgaacaaggcaaccgcctctagcgcgcccggggcgacgacctcgcttgcgcattcggtcctttcgggcgccgcccgatatcggacccttaccccgtccttgacggtttgggtcgagccaacggtccagcgttggtgggtggcaccgaaggtcgcaccgtcgcttcggcgaagcagatagacctgcttagggtcgacgtcctcggagcccagcggacggaagaggcagtagctgcccttgggaacaggggccgcgccgtcgccgagctttccgccgagcgtgtgtgcgtccaacctcatcacgaagtcgccgggctcgaaagctcccacggccacccgctggatgcctgtcggcgccgctccgtcaatcgcggcgtcaacgctgagcagcggcgggccatccgtcgcaggagacggcgggggagccgacgtcttgatagtgtctaggaccagagctgtcgcaagcgggaggcctcggtcgatcatcaagacatcgacgaccttggccgattgggcctccgaagcgaaagcggcggcgctcggattgcccggaaggtcgggcgcgaacgggtggccgacgacgatggcacgcccttcggggctgatgaggccgctcggctcgagactataatcgccacccgcgtcttggacgtcggtcacgagccgcctcagagccccctctgcccatgcgtctgacacgaccgggtcgactccctcgaagcaagcgcggaggagatcagccccgagccgccgatcaaggaaaccgtgatcgaacctgttcttgtaggaacggaggcactggtagcagctgtcttcgcaggtgcagtcgtcaaggagttcgatggcgctgcagacgagacggcgcggatcggatgcggccgccttgacgaagcccgcgccgcccgcggcctggtcgtagatgtagaggtctagaagcgtgttggccgtccgcacgggtgcgaagcgatagtcgccgtcaatgtcgcccggttccaggtcgcggctggcggcacggatcagagcttcaacggcggatttcgcagcaatgaccgtcgcaggtcggtcagggctgagatcccacgacggcggggcctggagccggaggacggcaatgtcggtcttgaactgatttccccagacgaggctcgtcacggcgccgttgcagagctcgggctccttcggcttcgtcggcctgggccgtgcgtgcccggctgatccgggccccagttgcgcgaggttagcgtctagatccgctggctcggtgcgcccgcacttcgcgcaatgccggaagccctgttgggttgaagactgggtgccccgattggtgacgaccaggtcgaggttttcctgccaggcttcccaaccggcttggttggcgaaagtctcgccgccaattcgctgctcgttgcggaagtgcggcgcatcgagcttagcgcgcgtcggacggctgttgacggtgccgtcgatgcgaggcggggcagcaggcatgccgggtggattggcgaagccgaccggccgcaaccagtgctgtgccggacccatgccgctcggagtgttgcatgccgggcaggtgatgaactcacggggacgcccttgatcgcgaggcttgagggtcgcgaaatcgcagatctggcaatggtagtagagtttgcgctctcgataggcgtcccagcggtcgtcgtcgaagttgctccagacgcccatcgacaggtgcgttttgccatcgacccagacggagcggcccggcgcgtactgggctagggccgcgttgagagattgctggggtgaataggccaactgtggctgataggggtcgggatgttcctcgaacaccgcaaacgtcgccacgtctgtagggaacgcataacgcggcatgagaccgagcgcgaacagttggtcgaggagcttattcgatccggcgcccgacttgtcattgtcgggcgcatcctcctccacgaggtcgtcgtagtcgccgtcgtcatctacctcgtcgggcgcgacgtccggagccggctcgtcggccccttcgacgacttgagcggtcgcaagggcaagtttctcttcaaggagatcaggccattgttcgagaagaccgggggcgtcgagcccggggcatgaggccgtgaacagttggtcgaggtccgcgacgagcgcgtctcgattgtcggcaagccagacgcgaaggccagcgagggaaaaaccggtcgcgtcgccggtcaggaaggcgtgggttgatccgagggactcgaagatgttcgggttgcttgaactgatgacccgggcctgttggaagcggccgaggaggaaagcgaatgcctggcgctccgcaataacgcggttgtcgagattgaggaccggatcgggggcgggcccggcgacgatgggggccgggtcgcggaagaagctctggtcgtggctgtccgcgccgcaaaacatgacgacagtggagaggcctgcaccccgacgcccggcacggccggcgcgctgctggtagttggcgcgaccgggcggcacattgcggagcgcgacggccgtgaggccgccgatatcgatgccgacctccatggtggtcgtgcaactgagaacgtcgatgggatcggatggctggccgttctgggccaccggcacatcctggaatcggagttcgtaggcctcgttgcggctcatggcccgaaccgcgttggtgtcgttcaactgagccgagtgctcctcggcgacgagttggtgcggagcggagcctggcgtgtggtcggccatgcgctccgcggcgtgccggaagaacgccttgcggctgcggaagacctggtcatggccggggtcgatcgcctccgtcctgccattgcacgacgggcaatagtccgcgaggagagcgttttctggcgaaaccagggtgcaggtgccgcagcggcgccaggtcacggcgttgcccgggaggagcgcgactttgcgcgccgagatctggaaggtgctgtcgctgctgccgctaaagacggtgcggaggatcggaacgccggtcttggtgaaaccaggaagccaggcgttgtggccggcggctttcagggcgcgggtgacgcgctcgccgaatttcccactccagcggtcgacttcgacatcgatcggcgtcgcgctcaacctgatcgaatgacggtcgagcgcgcaccacagccagaggcgcaaaacctcctggcggactctgtcgtcgtcgagtccggccagcttagggagagggatcgcctcgacagtcttacggtcgaggcgaccgagcttggggccgacgctggcaagagcgagggcgctgagccccgtgtggcgatcctgcagaattgcgtagagcgactggaagaccgatccgggggtggcttccgaggcgtctttcgagaagccagcgatctcctgggcctcgacgtcgggatcggcaatcagttcagcagcccgccgaccccagccgacatagtcgccccgatcatccacgggacgaatgcgcacctggttcagcgcggctgagagacttaccgcgagcggggcgtcatcaaggctgggctgatgaggcgacttcgccaggccctccatcccgtcgagcaacaacggacgcacgctgtcgcggaaggcgaacgtcttcaggaggccagccagccttgaggccgtttggcgaccgtcggagaacactaaggtctttcggcccttcaacggagcgtcggattccgggcgtggcggctggcttagaacctggacggcaaccagttgttggaagggctcgtcgcccttggtctgcaagtcgctgatctgctggttcgcatcgcagcgcgggcagcgatcgaagacgctctgtcctgtggagtcgcaccagatcgggcgggttcgactgccgtctccatcaaggcggcctgtgtagacgtcgaggtcggccgcagccagcggcgtcgcagccgaggcgccgggatcttccaggcagatatgggcttcacgaacgacaccagcatcgtcgctgtaggccgcgccgtcatccggccaaaggtgttgagcccccgcgggcgaccccacgtaggcgtgtgcgatagcgatgccgcaggagcggcaggaccagagttcgaaaacctgagccttacagtcgcagtgccggcgtggctctgcgtagagggcgccggtcggcccgccccgcaaatgctccggcaaagcggcgcagtttgcatcaacgcacgcccataggcccggaaggcctcggaacatgaggtggacgcgagccggcagtagcgggactttgtcgctcgcagggcgtgcgaggctggtgagttcaaggagggcgtcgatcgcccgaagagagcgggtgttgacgtcgccgaacagcaaggtggcgagttgggacaggctcttcgccgacccggtgatcagcttcgggtccgcttctgcggccgcgcccgaggtgatgttcttaagggccgcgacgaccgggaggtccttgagggccagccaagcggtacgggagagatcatccgtcgcccaatggatttggtcgggcgtggcgcggccgagatcgaggcctttgggtctggcgaagcgcacgacgccgtcagccggtaccaccgaggtgacaaggccgaagtgttgtcgggtctcgacaggtgatccggatggaacctggagttcttccacgagcaggcttccagcgcgatcaaggcccctcacctcaacggcggaggccgggccggagacgcgctggaggatgagcggctcggccgcttcgaacggctgccacgcgagaacgggggcgatgacctcggccctctcggcggagtcggtggacagcaaaccttggagaggaacgctggcgaagacgtccgcagcggcggcgtctcctggggcggcattgggctcgagacgcttgcggccgttaagaacggtgatggtggccgggtcgatcccgatgagttgcgccgcaaattgctgagcggcggcggggaccgagaacgacgcgctggtgcagatgaaggtgacgcgtgacgggtctagtttgagacggtccaggaaccgccgaatgaggaaggcgacctcggtgccgttggcgccgcggtagaggtgggcttcgtcgaggacgaagatgaacttttcctcgggatgcttctcgaaaaacgcgcgcgtctcatcgaacaggcttcgctcgataggtcgtaggagcatgtactcgagcatcgagtaattcgtgacgagaaggtcggggcaagcctcctgcatctcgtgacgggtcagcagttcgccgtcctgtgggcgctcaatggctcgatttggccggccttgcgcatcctcccaacgggcgactttggagccgtaccagccgcgcagaccgtcatatgcgccttcggtgctgtcgggcttggctggccagcgccccttgcgctttaggacatcgactagttccgccttctcggcctcgcccccgcgagcggcgtcttcgaggtcgagatagtagccaagcgacttcagcctaactttgtcgcggtctccatcgcgcctgccggggtatagtgtgcggccggtgtagcgaccgaacttcgctggcctgtcagccgtcgtctcgaaccagctgcggatggattcatcgccgaacagggtgcggagccgccccaattgatcgttgacgagggcgttcatcggatagagcagcatcgcgcggaccgcgcgggtcttgaacacctccggacgagcactggcctcctccgccaggcgcgccaggacgggtaggaggaaggattcggttttgccggagccagtacctgtcgtaacgacgattcctttgccgccggtgtcgttcatcacctgctcaagcgcttgggcctggtgctcgtatggcggatcaaagagcaagcccgtgtcggcgagccccgccagtagagcttgaaccgccttaggcagggacagatcgtcgaactttcggtcgccgatgtaggtcggcgtgctttcgacgtaaggctcctgcgagatccctcccgcgctcgacagcaaggcgcgtcttatggcgacggtcttgggatgcgagagatggtaggtggcttcgatgtagccgaccaactgcttccgcatctcgtcaatttcgcgctgcattccgcccccggtgttttggcgcagcaacgcaaggtgaatcgaagctcgcagatcaagcttcgcgcattccaccgagagtttctagggggccgcgcatcgctaggatgtcggcgggaccaatcgttggtacgggccctccctagcgtgaaaagctcagccgttcagaacggcgagtgcgtcaggacggcccccatgctcaagagaacattcatcggccccaatgcttctagcccctgacgccctccttcggccgacttgcccactaagcgggcggagtcgccgtctctcggcaatcgctaggtcgccagatggcccatcacgaggcgccctgtagcgttcttctagccacggctgtgtttcgccgcggttggcaaatcggctttgcgtttgatgaggttggggatgtcgtcacgcgtccaagaccgataatcgacctcgccgcgctcggcccgcggcacgatccagcgttcgcgggcaagatctgagatctgcgacacgctcagcaactttgaaaagtccggctccgcattgccatccttcagtacctcgtaggcgttctcagcgagcgtcgcgataaagacttcgcgctggatgccgtgcctgagaatgttctgattcacgttcagaccgaccagcgcggcccggattgtgcgcagcctccaattcgggccttcgccaaagacatgtctgtcggcgtagtcgtgacctcgttctcgaaggtatgcccgcatcttttcgaagaggctatcggtgatgtgaaagtgcccgaagcctttcgtgaagccgaggggcttcagatagatcgtgtcgtcgagcctcagccgattgtagacggatgatcggcccattgaagaggtggttgtgaccgcaaggagcttggcgtgctttgccgactttgaaatcaccccgaccgatctcccgtaggcgcgctcgaagtcattcaagacgtccttcgaccgaataagacaggccacagccttgccggctaaaagaaagctgtagggtggaaccgctccgagcacgtaagcgtcgaggatgcccaccagacggttggcgcgatcatgaacatcccagccaatctcgatgtcgcggacgttgagattgaacacgggatcgccgagggcgatgacgcctgccaagcggttgtggccgtcgtcccaaaccaggtagcgcagacgccggccgaaaccaggcgagaccggtacggaccaagtcagtgtagcgatacgaaagagatcggcctcaggtgtgccgctgcgcacgagtatcaggcgaaacttgattttggtcggatcgatctccgcgccgttcgcgaagtgtaccagagcgttgggtaacgcccgtgccaataaaggctgagcggcagtccacttcgcgcgccactggctgcgatgaaggcttctaacaacttcctttcctccgtcgggaagaaccaaatcacccgcgtcatccttcgtaaatcccagcgttcgcaggtgatcgcgaagggcgcgcttcagcgccgcctcagcactgaatggctgcgcaacttgcggtcgctttgaagtcatagcccctcccacggccgcaagggtatcgcgcacaccgccacccgacaaccggacgtaaccgggactacttggctatggcgggagacgacgatcgaggccactcgcgacgctcgccccctccgctgaccattcagtcctccggaagcagacgcggccgtcgaccgaaacgccagacgctgacgcactggatctaggttccagtgctcccccggaagcggacatcccgaacgtccgctatgagccgatttcgttgaaaaaggcgtccgttggcaattggcatgacgtcggcgcgctgattcactctggtcattgaggccgggaggttcagcgatgatgggcgaacggcgggtcgatcagtcggccctattctacgagttctcgctggaccggcatgtgcctgcggaccacatgctgcgcgcgatcgatcggttcgtggaactggacggcctgcgggctcacctggcgccgttctacagcgccatcggccggccttcgatcgatccggagctgctgatccgtatgctgctggtcggttactgctttggcatacgctcggagcggcggctgtgcgaagaggtccatctgaacctggcctaccgctggttctgtcggctgggcctggacggcgccgtgccggaccattcgaccttttcgaagaaccgccacggccgctttcgcgacagcgatctgctgcgggagctgttcgagacggtgctgcgacgctgcatggccgagggtctggtcggcggcgaggggttcgccgtcgatgccagcctgatcaaggccgacgccaatcgccagcgctgcgtgccgggcgacgatggtctgccgcccgaggccgccagccgcgccattgacgaatacctggccgtgctggacgacgcggccttcggcggcgcgaccccggtgacgcccaagttcatctcgccggccgatccggcctcgcgctggactggagccaacaagggcctggccttcttcgcctatgcgaccaactacctgatcgacctggaccacgcgatcatcgtcgatgtcgagccgtccacggcggtgcggcaggccgaggtgacggcggcccgcaccatgatcgagcgggtgcgcgagcatcatgacctctggcccgcccggctggcggcggacaccgcctacggctcggccgagatgctggactggctggtccacgaccagggcatcgagccacacatccctgtgatcgataaatccgagcgggtcgacgggaccttctcacgcgccgacttcgcctatgaccacgccgccgacctttaccgctgtccgggcggcaaggaactgaagcaatatcgacgcgccttccgcgcggaccatcccgacaccccgccggataacacctatcgctatcgcgccagcaaaatggattgcgacgcctgcgcgctgaagagccgctgctgccccaatgcgccggcacggaaggtgacacgctccatccacgaaggcgcccgggacttcgctcgcgacatcgccaagaccgacgcctacgtcgtctcccggcgcgaacggaagaaggtcgagatgctgttcgcccacctcaagcgtatcctgaagctggatcgtctgcgcctgagaggtcccaacggcgccaaggacgagttccttctcgccgccaccgcccagaacctgcgcaaactggccaagctgatcccgccgacgaccccggcggccgcgtgaggcggagagaaccgacgcgtccgttactggcgacgacctcagcagccgcctttttcaacgaaatccgcccgttccagactctacctagcttcctgggacagctgccctgcgtcaaaggcggacgcaccgcaaaggcacgcatcccgcgtccggctggacttcctccgcgaatgacggtcagtggcgggcgtggacaccctttcaccagcccaacgctcggagcgtatgtcacgggttcgatcgcgcgacaccaagccggaactgctggtgcgcaagctggtccatggcctgggctatcgataccggcttcatcgcaaggacctaccaggcaagcccgacctggtgttcggtccgcgccgcaaggtgatcctggtgcacggctgcttctggcatggccacgacgatcccaactgcaagctggcgcgagcgcccaagtcccgtgtggaattctggggaccaaagctcgctcggaaccgggaacgcgaccgcgaggtggaacgacggttgaacgaatcaggctgggaagctctgattctctgggagtgcgaactgggtgaccgtcccggattggagcagtgcgtgagggacttcctcggatgagatcgatcgaactgttcgcgggagcgggaggacttggcctgggcgtggccggggccgggttcgatcacgcggcggtggtcgaatgggaccgctgggcctgcgacaccctgaaggacaacaagccctggcccgtgacccagggtgacgtgcgcctgatgtcctatgacggcctggggaccatcgatctcgtgtccggtggtccgccgtgccagcccttctccctgggtggaaagcacaacgcccacctcgaccatcgcgacatgttccccgaggccattcgcgccgtgagggagctccagcccagggccttcgtgttcgagaacgtgaagggcctgacgcgcgcgaccttccagaattacctcagctacatccggctgcagctcgcgcatcccgaggtcacggcccgccccgacgagccctggatcgaccacctcggccggctcgagcgccacgagaccagcggctccaactcgggcctgcggtataatgtcgttctgcgcctgctcaacgccgccaaccatggcgtgccgcaacggcgcgagcggatcttcctggtcgggttccgttcggacctcggtgtcgaatggcgcttccccgacgagacccattcatccgccgccctggcctggtccctgacccacgaggacgagtacttcgacaggcaccgcattggacgcgccgaacgccgactgctgcgggacgccctgcccaccatcaagggcgagaagccgaccgcacggccgtggctcaccgtccgcgacgccttcctcggcctgccggacccagagctcgacccaaggggagccaagggtatccccgaccacagattcatccccggcgctcgttcctatccaggtcataccggcagcccgctggacgccccggccaagaccttgaaggccggcgtccatggcgtgcccggcggcgagaacatgttgcgccgtcccgacggctcgatccgctacttctcggtgcgcgaggccgcccgcctccagaccttccccgacgacttcctgttccatgggtcgtggacggaaaccatgcgccagctcggcaacgccgtgcccgtgcgtctggccggcattgttgcccgctcggtggcggatcagttacatcgttccgatgagcgccctggtcccctacaatccgctggagaagcggcacctggccgaaagcgtggccaacgccctcctgcgcaggcccattgagccgctcgcgccggcccagcccttcgagggcgccggcatctacgccatctattacaccggcgatttcccggcctacgccaaggtcgccgacaagaatcgcgacgggcgccttcgcgctgccgatctacatcggcaaggccgaccccatggggggacgtcgcggcggggatttcgacgccccgcatgggcgggcgctctggaaccggctggcggatcacgccaagtccgtggcccaggccgataatctgaaatccgaggatttcgcctgccgcttcctggcggtcgacgatgtgtgaatccggatggccgagcggatgctgatcagttggcacttcccggtctggaacctggtggtcgacgggttcggcaatcatgatcccggcggacgacgcgccacccagtaccgctcaccctgggacgtgctgcatccgggacgcacctgggcggtcaagctggcggacagcggtgtgacgccggaggatatctccgccaaggtcgcgggacatctggaggctcgagaacgcgcggagcaagagcaagcggcggcgaacgaggcgtcggcccacgcctaaggaaacgcctcaagcgtatcgactggcggagttcagacgcgaccatctggagccgaaggccatgcgcggtggccctagcgttcccgggggccttcgcgacgcggcgaccgccttgtatgtcgggcatgatcagcgggtcgggggaagaaaatggcgacaggcggcaagctcgagaatctgacccagtcagccgctgtcgagagggcaatggaggaattccgcgtcctgggacgtgacgccttcatcgagaagtacggcttcaaacgttcgcgcgatttctttgtgcatgtccaccgcgatcagatcgacctctacaccggcgacgcgagctgcggccgacagtagcccagatagatcaggttcgctccctcgtggtcgatcaccggacgggttggcgccgcccgtgatcgcgatgaaggattcatacgagggcgccgccgccaacaggcgccagcgcgatccacttttcgaaatgagggcgacaccgctcggctctcgcaacgtccaagcggcgtcaattccaagcaccgccatgaatgtccctatgttgcccgccgttcgctcgcttaggcggtcaaccacttttccacatgatcggcaaacgccacgagcagaccgcgccgtcatcaccaacaatcacgcgtgcgggattggcctgcgatgttcagcgacccacatccttgcacacctgctggagctggcgatactcgcggcccgaaacaccctcgccgctgagctgagcgagcgtcgccgcgcatgacggcttgggcttaggccgagtacaggaatacacgggccacgccacgaacatcaggagaagtatgattccgacgatcgggccgtcgttgttttgctgctgactcatgtttgccgctcctgttttgagaccggaaaaccctaacgcacacttccaaaatgctacgtaaacgctgtcgccgtatatgcgtcatccagtcagctttcggagatggcggcgaaggcggacaaacccttgcggaaggtgttggcggagaatctccgccgctatcgcgccaatcgcgggctgagccaggaaagcctcgccgacgaggccggactgcacagaaccttcgtcggcgccgtggagcgatccgagcgcaacatctcactcgacaacatcgagaagctggctggagcgttgaaggtctcgccctatgaattgctccgaccaaaggcggacccattgatcgtccgcccgacgcccggctgagttggcggcttagcagcctagccgcaggccaaccgcgaacccggccaaaccccgcaggatttcgccgcccatggccccaagtcgacgacgcgcgacagcgtgctcggcttcgccgatagaggccctcagcttggccatgttctcttggaaccgcgcctccaggtaggcgtcctggcgcgcgcgccatgccgcccgcgcagcttcctcggcctttgcgaccagcgccgccttttgctccgctgtaaggggcggaacgcggcgcttgccgaaggcgggcggggtgggtcgaggtgtcggttgaaacggcatgagccgaccaacgcttccttccacggcgaagtccagtcgtcaccaggatcgctggacgaccgtcagatcgggcttcgtcgtgatccaccccaggaactggctggtggcgtcgacttggtcatcatgcttcgcgcgagggaaggagatgagttccttcacatactcatcaagccatggcgcatgatccggcaggtggaccgccccgcgttggaatatcggtgtggacgcccaaagccgggagaccttgttttggaccggcgggacgagctccagatcaacatcgggacaggcctgccggacctgttccgcgaccagttccatcccattgaccttctcaagcaggatgacccggcgagtggtgggatatttgttccatagattcgccatggcggtgacgagatctcccccggagaaacggcccctgacgatgtctccaaggtagtagtccttgccgcgcacgatccaaaccgtacccacggaccagtcattgttgtcgcctgttccgaatgccgtgtcccaactgaacaccacctcatcgtccatcgtggccctgaacggcgcgcggtaccgttgcagccattcgagcttgacgacgttgccgcccggcatgacgggcgattgctgatattgcgcctggaagaaatcctcgcccatgctttcgcggatcgccgccagcgtctccatggactcgaaccgaggatttagcggctcgccaatctcccgcgtccaaggcaccccacgaccggcgtcgagcacctgacgttccgtggcggtggcgggcagattgaggtgtgtccacccgcccgcctccaaaagccggcccgacagatcatcgacgtgcaggcgttgcatgatgacgatgatgcatccggtttccttgcgatccagtcgggacagggcagtgctttcgaaccattcgttgacccgcgtgcgaactgtgtcgtaccgcgcgtcctcgggcttgatcggatcgtcgatgattaaaaagtcgccgccgaagccggtgatgggaccgaagaccgtggttccgaaccgtttgccccggtgcttcatcagggtgaagtcggcgtccgcgttggccctcgggttgatccgcgtggccgggaacacccgcttgtaatcggccgtctccatcagggccttggagccccgggcgaaatcctttgtcagagcctccgagtaggtgatgttgatgattttgcaactgggatcgcgaccgaggagccacgtcggaaagacgatcgaggcgaactctgatttcaggttccgcggcggcagattgatgatcagcctcttggtttcgcccgtggcgcatttggtgagcgccgccgctagggcatgaagatgccagccggatatgagtttctggctgggatgcaactgggaccacgcccagacgaaataacccatcaggtcggctcgaagggccgcgtcatactcggcgcgcgtgaaggccgggacgcccatcaaacgtcctccccacgctctccgcgcgccatcaacatcttactggcgatggcttcgagaagcttggtctcatcggtcgacagcgcgtcgtccgcctcctcggcgaattgttccggcagagtggtcttgatcaggctgacgaacagggcagcgtcttgggtcttgcccgtcaacgcctgcgacatgagccgggtcaggacggcctccttggcggagacctggcgcggcacgcccttgatggagatggtgacaggctggtccaggatttcctgcaacagcgtgcgcatggagcgcgcgcccctgggacgtcccgccggattgccggacttccccttggcgaactgcgaagctcgcggcggtttgccgaagccggccacgtaatcggcctcgtcggcgcgggccttctgctcgtcggtcattggacggcgtttcgcggacctcgccattagaggatcgcccacatgctgtccggacccggttccgaaactggattccccgtttcgctttggcgtcgagaccgaacttccgaaaaggcttcgccggtttccgccagcgtgggctcctcgccggtctccgcgatgaaccggcgcagcgtcacatcgacatacttcgggtcgatctcgatcaggcgggcgatgcggcccgtgcgctcagccgcgatcagggtcgtgccggaaccgccgaacggatcgaggacgatctctccctgatgggtgacgtccagtatcgcatcgacgatcatgggcagcggcttgacggtcgggtggaaggacaatgcttcagcccgaccggcgcccaggctggcgcatcccggatagttccagacgttcgacctgtagcggccattgctccccagcccgaaggtgttgacgttgggagcgtcgccgagcttccagatcgtcaggagttcgtgctgcgaccgatagaaggttcccatcccggcgttgtccttggcccagactacaagctgcttgagctctccgaagacggcctcgccggcggcgatctgatcggcgacatggcgtccgtcgatgaaggcgtaaagtagggcgccgtcgacgccgtgctgcttgcaatggtcgaacacctggcgttggaactcgatgaactccgcccgcgtcatctctcccgacgccatggcgaattcgccgtgctgcaccttgccgagccccgagacgttcccggaaatccggacattgtagggcgggtcggtcaggatcagcctgacccgccctccagccaacagaatgacgtagacagcgccatcacggctgtcgccgcagacgatgcagtgccgcccgcagatccaaacatcacccagttgcgtgaccggagcaccgccatccggctcgggcacttcatcctgcagggcgccgacatcgtcggccagggtgacccgatccacgaagacctggtcaaagccggtgaaatccagcgagaactcgatatcgggatcggccaggagggcgatgaaatcggcgcgaaggacagtctcatcccactgcgcatgttcgccgatccggttcagcgacatctgcaaggcgcgcagttcgttcggcgaataaccgctgacgcggatcacggggatggtgtcgtgaccgagccgtttcgccgcctccaagaccgcgttgccatccaaaacgatgttttcgtcggtgacgaggatcggtctgacaacatcgaagcgttcgatcgctccgatgagactggccagttggcgctgactatgtttgcgctggggacgcgggtccgaggagagcgacgccaaggcgacgtactcaacagccactggtcggttggttcgacgtggactgacttcgccgcccacgcgcgtgataggagcgcattgcttagccacgagcgcctcctggcggcatgtggtcctgcccgatagtcgccagccatgctggtccgttcgtcaccttcggcatcacatctctccacgccgcggagagggcctccacggcttcaaaagtttcagttttgatgtgagagggaccggcggtccctgagcgtgaatgccgaggcgacgcccctgcgatatcgatcctgcacgggcggatagccggttttcaagtcagggcggataactttccgcgggctgcgggccggcacgatcaggccggccccggccgattcgatagcgctcaacctggtggcttcatgcgggttcgcgccatccacaccaccgcgctcgatccgtcccaccgtgcggcgtctcctgcggtccgcgtgcttatcgcgtgcgggtcgcctgtttgtgctgctgaggcccgagggcgaggcgtcgggcaagtaccgcatctatcgcctttatcgcaaaaagggcctgacggtgcgtaggcgccgatcacgccggcgagcgattggcacgcggatgccatcctgatcgagcactgcgcgaatgtgcgctagtcgctggacttcgtgcacgatcagttcgacggcgggcgtagcttcggcatcctcgatgtggtcgacgacgtcacccgcgaaagccggacggcgatcccggccacctcgatctctggtcggcgggtggcgctggagctgaccacttttgatcgcgcgtcgagcgcgccaggcatgatcgtcagcgaaccgcagctcggcgcagccttcacatcgaccgccatcctggcatggccgcaggatcacgccgctgcgtggcaccgcgcccggcaagccgacgcagaacggcttcgtcgaatcctccgacgccggatgcgggatgactgctgaacgaaagcctgttcttcgacctgggccacgcccgccggacactggcggcatgggcggacgactacaacaacagccgtccgcactcatcgatcagctatctcactcctgcggcctatgccgagagcctgaccgcaacaggccgatccgctgcgcgggttgaaagctgcgcggaccggcctgttgctcaccccgcgctgcgacgcgtaattgacgctgggactcaggtcgccgctggatgaaaacttaggggcaggtcacgctaggctcaggactcatagccagaagagcacgacggcggcgagggctatggcggagaggaagaccgtcgggcatcgatcatagcgggtggcgacgcgccgccagtccttcagcctgccgaacatgatctctatgcgattacgccgtttgtagcggcgcttgtcgtagcgaatgggctcagtgcgggttttgcggcctgggatgcagggcgtgatccccttggcctgcaaggcgtccctgaaccagtccgcgtcatagcccctgtcgcccaacagccattgcgccttgggcaggctgtccagcagggctgcagcgccggtgtaatcgctgacctggcccgccgtcacgaacaggctgatcggacgcccattcgcatcggtcacggcatgaagcttggtgttcatgccgcctttcgtgcgaccgatcagtcgcccgaggcccccttttttacccgcaggctcgaagccgtgcggtgcgccttcagataggtcgcgtcgatcatgacggtgcgacgttcggtctgagcgccagacaggccctccatcatccgaacgaacacgccagcttcgctccaccgcttccagcgattgtagagggtcttgtgcgggccataagccgctggcgcgtcacgccagcgaagcccgttgcggttgacgaagatgatcccgctcaacacccggcgatcgtcaaccctgggcctgccgtggctcttgggaaagtgcggccggagccgctccatctgctcgtccgtcagccagtacaggtcactcataatcagactcctcaggagcctgaatcagatcgcgcgcctcacatcaatgggtcctgagcctagaggctctaggagcctaaaacggaacgctttcggaccgtttgcgttgacaacccatgatgaaggcggcgaccaaggatctcgtgctgcagccgcgcccggcccaaggcggtcggcccacccaggacgtcgccgccaagcttgagactcacatcctgagcatcgcccttcagcttttgtgcgcaaatgatctggaaggcgccacgattgacgcggtggcccaggccgcccatgtgtccaagcgcactctctatgcgaggtttccgacgcgacaggccctgtttctggctgtgttgaaccacgctgtggaactccggctggcgccgctgcgtcggccggtgctggatggagactggcgtgccgggctcgcctctctgctctcggaaatgctcgaggcgtcggcggagaccgaactccgggccatcgagcgcctgctgctgtgggcgcgggatcacgatcccgatctggtgcaatccatgttcgaccgttcgagcgcccggcccgtgcgtgtcatcgccacgatcctcggcggggcggcggatcgccatgagcttgaggcgcccgacgtcgagcgcatggccaccattctgtttgaagccgccgtcgtcggcccgcgtcggcggatgttgttcggcgtcgaccccaaagagaccgccgaggaccgtcgccgccatgttgccgcggtggtcgagcttttactgggggccgcctcggctccttcgcctttccaacaggagtgttccgatgccaacctatgatgtcgctgtcgtcggcgcgggccataacgccttggtcagcgcctgctatcttgccaaggcgggcaagaaggtggcggtgctggaacgcaggccggtgatcggcggcgcggcctgcaccgaggaaatgttcggcggctacaaggtcgatataggctcctcgatccatgtgcttttcccgaccacgggcatcatggaggaccttggtctcgccgagcacggtcttgaatatattgagttggacccatggggcttttaccccattcggggcacggacaaggccatcaccttctaccgtagcctggacaagacctgcgacagcattgcggcgatcaatccgcgcgacgccgaaacatatcgcgagttcatgaccacctgggccgacgtccagcggctgatatggccggcgatgtcggcgccgccccagatgggacagacgatcgcctctgtgatcaaggcggccttctcccgacccggggcggtgcgcaccgcgctcaaggccgacgacctcgtgcgccaggttctgatcgattccacccggctgcttgaggaactgttcgagagcgaggaattgaaggccgccctggtctggctgggggcgcagaacggcccacatccggacgcggcctccagcgccaccatcctgggccactacggcatgatccacgaggacggcgcctatcgcgccatcggcggctcgggcatggtctcggtcgccctgggccgcgccttcgaagccatgggagggacgatcctgaccaatgcggaggtggaaaaggtttcgagcctctcctcggccggcggcgcccgcttcgaggtccgcgccggcgaccagaccgtgcaggccaagaccgtcctgtttggatgccacgtccagaccgccttgttgaagctgcttgatcgcgatctggtcgagccgaacctggtgcgccggctcgaggcgctgaaggtgatgaatgggtcgggcttcatggtgcgccaggcggtttcggaattgccggcgtatgcgggccaggcgctcaacacccgtggggtgggcgaatgccatcacggcatgcagttgctgtgtcccaccgtcgacaccctcacgcgatcgatgaacctgggccgtgtcggccgcacgcccgactatccgccggtgatgcagatgagcttcaccgccgtcgatcccaccctggcgcccgagggcaagcacctgctctacagttggtcctcctatcatccctaccatctcgacggtgagaactgggatgacatcgccgagcgcgaagccgacaagatctgggacgtggtctgcgaatacacccccaacatgaagggcaagctgatcgatcgctacatccagtcgccgctggagatcgagcgccggatcggcctcgtccagggcgacgtcacccatctggaaatgagcatggaccagatgttcggtttccgacccctgccagacctggccggttacaagacaacgatcgacggcgtctatctgaccggcgccagcacccatccgggcggcggcgtgtggggcgccagcggacgcagcgcggccaaggtgctgctcaaggatctacgatgaaggtcatcaagacgcgctgacgcaattcaacctgggtccggcggcgcctcgcatcgcacttcagttccgggggtgtagggacagtttcgatccaagagcgggtcataacgtgtcggcgacctgggaagcccctttgtcgggcgctgattcaggctgcggcgccaagtctgccgggtctgttgcggcatcgaagatccccaagtcagcccttccctgcagtctaggcctgggcgcccgccagctgcgtgaccagcgtttgcacccgctcgcggaggtcgtcgacctgacgcggcctcatgcccgtcttccttgaaagttccgcgggaatgcttcgggcgcgatcccgcagggcgcaccccagcggtgtcagtgcgacgaggacgcggcgctcgtcgtcggcgtcgcgccgccgtgtgatgagcccgctccgctccatgcgtttcaaaagcgggctcaaagtcccgatgtcgagatggaggcaggcacgcagttttccgacggacatcggcgcctgcgcccacaataggagcataacgagatactgggcgtaggtgaggcccaggggttcaagaagcggcctgtagagccgctgcatgaggttcgtcgccgcatagagcggaaagcagacctgatggtcgagcctgagcaggtcttccccttcggccggatcggtgtctggtttcaccgcgtcttcacagaaagcgcgacatcgatattgccccgggtcgcgttcgaataggggcagaccttgtgcgcctcctcgacgatcgcttcggccgcctcctgatcgacgccagcgatggtgacatcgagcgctacggtaagggcgaacgccccaccggcattgggctccatgcccacggtcgcggtgacctcgacgccgtcgtctccgatcttcttttcccgattgcgggtgatgtggatcacggcgttgccgaagcaggcggcgtaacctgcggcgaacagttgttccggattggtcgcgtctcccttgccgccaaggctcgggggcagggcgagtggaaggtcgagcaatccgtcctcgctgcgaacagagccggcgcggccgccgacggcgtgtaccttggttgtgtagagagcgctcatcattccacctgacagaaatatatggctagccatatattcgcgcggccatggaatatctagctcgcaccgagaggcgccgctgcggatcaccttgctgaaagctgcgctcggagataggcgctccaggacgcatcgtccggaaactccgacgggggtcgaacatcggttggcaggctgctgacccgcgccagcgcatcggcggggatggtgtcgtcgacgagacccagctgctggaacagcggcagggcatagccgggaatccagcgcctcaaatcataccatggcaccgaggcgaaacgttcgggcgccaggttgatgaaggaggtcatgcagctctcggtcagggtcgaatagaacttggggcgctcgtgaacctgggtcgtgaaccgcaggatgcgctcgaaataaacgcggacgacctcagggctctggcggatcggatagatctggatctcgtccggcggcgtcctggccaaccgctcccagaacaggtcgcgctcggtggccagttccggatagatggggtcgcgccggaagaagcccgccagggggtcgaactcggcgcccctcgcctggcgcgcctccatggagacgacgacgtgacggccgtcggcgaaccggaacgacagcatcacatgctccatcgccttcaggtcgccgaacggctggaggatcagatccatcccctcgagggtcgcgagatcgaaagtcgctgtggtccagcgcggcgtcgacgcgacgccaggatcatgtagggcgtcgcggaaattgtggatggtcgcccggtcgccctcaatcaccgcccaagcctcctgagcatgcaggtcgcgccagtcctgaggcgctggcgacttggtccagtaagccgtcaggacaatggcgagcatggcggccgcgacgccgcgcctcgcgcgccgccatcgcgccggcgcgaaccacagccccaggaccagcacggggaacgcaactgcgcccgcatcgcgaatccagaccggccacgggacccagtagcggatcgccagggcgcagaagaccgccaggaccacgatgagaaggctcgccgcggcgcgcgccgttcgattcaacacttatttcctcgcgtcgtcctggcatcgggtcgacaccgataatctgactggatcagcgcgaacccaaatgatacgtcgagttccaataatcggtagcggcatccaggcgtgcgatcaatgattccctttcgaacggcctgggccggtccaggctccctgccccgagccctggcgctgggccttctgctgtttctcggcctgggggtccaggcgtgcgcaaccgcgccgtccggcgtgctgctgccgatcaccacgccccatccgggcgtgcaggagatcagcatgctggtctattccacgcgcgccccaaccgaggcgccgggcgtggtctattcaggcaagaggggggaacacctgacggccatggtggtcgacgtctcgatccctcctgcccaccagatcggcgccgtcgaatggccgcgtcggcgcgaggccgatcccgcgcgggagttcgccaccctctccatcgatccggtcgtcgacgacgcctcggccgaggcgtggatgaacgcgcaactgaaggaaggccgcctgctgattttcgtgcacggcttcaatgtgccgttcgaccgggccgtctattccctcgcccagctgacgaatgattccggcatccaggccgcgccggtcctgttcacatggccctcgctgggccggatctatgcctatgtctacgatagggaaagcgccaactattcacgcgacgccctggaacagttgctccggctggccgcgcgcaatccgaatgtgaccgaggtcaccgtcatggctcattcgatgggcagctggatcgcggtcgaggcgctgcgccagtacgcgatccgcgagggacgggtcgacccaaagatcgagaatgtgatcctcgccgcgccggacctggacgtggacgtcttcgcccagcaggtcgcggttctgggccctgaccggccccatttcaccttcctggtctcgcgcgacgaccaggccctgcgggtttcgcgcctgcttgccggaggcgtgcaacgcgtcggcgccctcgacccctccgaggagcctatccgcagccagctggagcggaccggcggcgtcaccgtcatcaatctggccgatgtccgcggccgtgaccggctgaaccattcagtcttctcagagagccccgaggtggtccggctgctgggcagcagcctggtgtccggcccgggcttgtcgggaagctccgacctgccgctaggcgccttggttctggacgtcgccgaggcgatcacttccgacatctcccaaaaggctccggtgacgcgtcagccccaggccgcccccgccgaggcggtcgcgccctcggacacgcgcacgatcgcagatgacgcccgggacgtcacaccgccggggccgcgcgtcgaagtggacgaagcggacgccctcagttctccccgaccggtgattgatccacatcaaggtgcatccgtggagcgggattaaaagataaaatccatatcactcagcctgtcccagacagccaagcacacggaccgcttcgatgaacaagaaccagctggccggcgaatggaagatcatttcggggcgcatacagcgcctgtgggccgaaagcctcgatgaccagaccggagcgatcaagggcaactggcgcaaccgggtctacggcaatccgctcgacgggctcggctacaatatcgtggccgacgacgggctgagggcgggcgtgcagcttcggccgcattattgcggtaagtcggctatcgaggggctggacctgcccgacctcggcgccgacatggcggtctatggcttcgtccggattccggggaacatctcggtcggcggacgtgtcatgcgcgacatcagcggccagaccgacggaacgacctactacgcctcggcctcgcaccagggcgtgacgcgcatcggcctgttgcagagcaccttgtatgcgcgaggcggtgacgcccgcagcaacgacgcctatttcggcgtcgacgccgacgcggcaagtgtgaccggtcttacgccctatgcgccgggaagcggcgtccggaacaccggcgtcgccttcctgatgctgacgccgatcggcgaccgctgggccgtggcgactttcgccaacgccgagcgggcaatgagcgacgtcgccgacagccccctgatccaggctcgagacgaacaggagatggctatcgcggggggattctgatcgtgcgccgtttcggcggctggtggttttccggtcgggcgatgacgcccggcctccacgcggcgaatgacgccgcaaatgacggggctgaactcatggatacgcatttcaatccgcttggagattttctgagccgggcctggtggttgctgctgttgcgcggcttggccgccattgccttcggcgtcctgaccttcgtttggcctcaggtgacgttgctgacgctggtgatcctctacggagtttacgccattctggacggcgcgttcgccttgctcggggccatccgtggcggcggcctggcgccgcgctggtggctggccgtcgtgggactcgtgggactggcggcgggcgcggtcgccctggccttgcccgacctgaccgccgtcgcccttgtggtcatcatcggcgcggcggccatcgcgcgcggtatcttcgagatcgtcggcgccatccagctgcgcaagacgatccgcaaggagtggctgctgatcctgtccggcgcgatctctgtgctgttcggtttggccgtcatcgccgcccccggcgccggcgccctggccctggtctggctgatcggcgcctgggccatcgtcgcgggcgtgctcacggtcgctctggcgctcaaactgcggaaaataacgagctgaacgtgtcgttcggaaaacggactgccgcccctctgatcgcagccgccctgaaggccgcggtcgagggtctgctggccgaatgcatcacggcgcaggccgagaataactgccctgaggcttaccgtatccgcgatcgtggtctgcgcccttttaagtgatccatcccctatgttggtctgcggaccggaatggatggagccaaggatggccaggaagcgtcacaagcccgaagagatcatagccaagctgcgccatgtcgaggtgctgacggggcaaggcaagtcgatctcggaggcgttgaagacgatcgcggtgacggagatgacgtacttccgctggcgggcggcgttcggcgggatgaagaccgatcaggtcaaacggatgaaggcgccggagcttgagaacgccagactgcgtcgtgcggtgtcggacctgacgctggacaagctgatcctgtcggatacggcccgagggaacttctgagccctgcccgtctctgggcctgtatcgacaaggtgcgggccgagttgaacgtgtcagagcggcgcgcctggggggtgctccaccaccatagacatatcgtgactttggacaggtgatcgtcggccgccgacgatagctacgatgtttattcagatttggctcgagtcgctttacgctctgcctgaaatgacatgcgtttccctgtatttggaaccgcatttctggcgcaggatcgtgaaaaccttctaagaagcattagtttaacggcttaggcggcagagaggatttggctaagtttgagctattccctgtttaagcggctcgatcagggaatcagccggcacattttggatgtgccggtcacggagagaatgacctcccctccttggcacaccaccagtttccgaggggtcagcggttcgccgctggccccttttgcttttcggagccgcgatgcatggggtcgtcccccccccggcgcggcaacttcagatattcgaccccgcgtctgttcgcgctaaggcttaatccagcaattgcctcgtagggtcacgtccaagaggacgtcatgaccaatccctaccaagccgtcgcccaaacgaggcggcgcgaactcaaggcccgcgtggggctggccggtttcatagccctgacggcgtggatgatggcgccctccggctggccggcgatctggctgttggccgtcgcggtcggacaggtcgtcgactggctggtgttccgtccgctgatggaggagggacgcggacgtccggacgctcggtccctggcggcctgctgcctgtcgtgcgcggtgaacagcacgatctactcctcgatctccatctacctgtggggcgcgggcgagaccggcatggtgttcggcagcgtgctgatcgccggcgcgctgcttcacgtcaccctgcacctgaactcggtgcgattgatcctgctggcgtcggtcacgccgcacgccctctacttcctgggcctgccggtctgtcgggcgatcctgaccaacacgccgcaggactatctgatcgcctcggctgcgtgctctacatgacccatctgctggtcgccgtgcgccagagcgcggccacgaccaaggccctgcaacaggccaatgcgaccgccaccgaggagcgcaaccgcgccgaggtcgccagcgccgccaaatccgacttcctggccgtggtcagccacgaaatccgcacccccatgaatgcggtgatggctgcggcgacgctgctcgaccgcagtcgcctgcggcctgagcaacgcgaacaggtcggcatgctgaaggatgcgggcgaggttctggtgggcctgctgaacgatgtgctggatttctccaagatcgaggccggcaagatgcagatcgagccgaccaccaccgacgtgcgcgacaagctgaagggcctcaagagcctgtgggagcctcgggccgacgccaatggcgtggccatccgcctgatcctgtcgccggacttcccttccggcctttgcatcgacgccctgcggttgcagcagatcctgttcaacctcctgtccaatgcggtgaagttcacccagcagggcgaggtgacggtgcaggccgagtggatggccgaaggctccaccctgcgcatacgggtcagcgacaccggctgcggcattcccgccgatcgtctgcccctcatcttcaacagctttgaacaggtcgacgccggcgtgacccgccgctacggcggcacgggccttggactggccatctccaagcggttggccgaactgatgggcggcgccctgaccgtctacagccaggtcggcgtcgggaccaccttcgagctgacgttgccgagcgaggcggtggccgccgtggacgagacggaggaacaggccgaggcggaagccgacctgtccaacctgtcgatcctggcggtggacgaccatccggtgaaccgaaagatcgtcgccatgctgctggagccgttcggctgcaggctgagcttcgcggaggatggggcggaagccgtggcgctggcgcgcgaggttccgttcgacatcatcctgatggacatgcagatgcctgtgatggacgggatcagcgccacgcgggccatccgcgtggagggggcgaaccgccagacgcccgtgatcgccctgaccgccaacgccttggacgtgcaccgacaggcctggctggcggtcgacgtcgacaacttcctgaccaagccgatcgacccggccgcccttgtgtcgaccttggagcgcgcgagccgcgccgtcgccgcgccgcgcccgcctgccctcgccctggaggcctgaatccgcggtgaggatcgccaccttcaacatcaacggcgtgaacaagcgcctgcccaatctgctgcaatggctggacgcggccgagcccgacgtggtctgcctgcaggagctcaaggccacggacgcccagtttccgcatcaacccatcctcgaagccggatacgaggccgcctggaagggcgagcatcgctggaacggcgtggcgatcctgagccgcgtgggggcgccggtggtcacgcgccgccgtctgccgggcgacgacggcgacgatcaggcccgctatattgaggcggccgtgagcggcgttctgatcggctgcctctacctgccgaacggcaatccccggccgggtcccaagttcgactacaagctggcctggttcgaacggctgatcgcccacgccgaaagcctgcatgacgcgcccgcccccgtggtgctggccggcgactacaatgtcgtgccgaccgaggcggacatctacagcagccgctcgtggaagaccgacgccctgctcagcccgcaggcgcgcgccgcctacgcccgcctgctggaggcgggctggaccgacgcgctgcgcgagcggttcccgaacgatccgccgccctggaccttctgggcctatctgcgagaggcctggagccgcgacgctggcctgcgcatcgaccatctgctgctgaacccgaccgcggccgagcggctgtccgatgcaggcgtcgatcgcgacgtgcgcggccgcgacggcgcgagcgaccacgcccccgtctggatcgaactggacccctgccccccgccgcaacgctcccgatccatgacggcgagcctggaaaccagcctgcatacgcttgacgagacccgcgtcctgcaggcgggcggcgtcaccctgacattgggcgggctggtcaccccagcggtggtcctggtcgccacggcggcggcgagctggctcgtcacacgctttctgcgtcggctgcgcgccagggccgagcgcagcgcgcaggccctgtatgtgctggaacggctggccggctacggcatcatcgtcgtcggcgtcatggccgccctgtccgccgcgggcgtcaatctgtcgtcgcttgcggtgttcgccggtgcgctcggcatcggcgtcgggctgggtctccagggcgtggtcaaggagttcgtctccggcctgtttctgatcttcgaccggatggtgtccgtcggcgactacatcgagatcgaggacatcgacatccggggcgcgatcatggagatcggcccgcgcgccacccgcgtgcgcaccaacgacaacgtcaatgtcctggtgcccaactcgcggcttatcgagcagccggtgaccaactggaccctgaagggcgacacccggcgcatccacatccctttcacagtcgcctatggctcggaccgggggcgtgtgcgcgatgcggttctggcctgcgcccgcgccagttccttcaccctgcccgagaccgacgcccgcaagagccaggtctggctggtggcgttcggcgagcggggactggagttcgaactgctggtctggccgacccgcgaggcggtgaagcgtccggcggccatgcacgcggcctatacgtggctgatcgccgacgccttggacggcgcagggatcgagacgcccttccctcaggccgatctgcgcctgcgcagcgcctttggacttcaaggcgaagaggcgctgcaaaggctggggtacggccaggccgccgagccagcctccccgccgccgccccaaactcagcctgcggccaacaacgacgccgccgacgacgtcatggccggggcgcgcggcgaggcggctctggagcccgagcctgagccctcgcgcgaccgcggcggcggctagccgctcgccttggcgcgcagccggtaggcgtgcagcagcggctcggtgtagccgttcggctggaccgcgccttcgaacaccagcgcccgggcggcctggaacgcgagactggcgtccgaatcgtccgccatggatcgatacagcggatcgcccgcgttctgcgcatccaccttggccgccatccgccgcagcgccgcctccacctgcgctgcggtgcagacgccgtgcagcagccagttggccatgtgctgggcgctgatcctcagggtggcgcgatcctccatcaggcccacgtcgtggatgtccggcaccttggagcagcccacgccctgctggatccagcgcaccacatagccgagcagcccctgggcgttgttgtccagctcggccgtgatctcatcctccgaccagttcacgccctgcgccaacggcggcgtcagcagcgcctccagtcctggcgtcggcctcgccgcgatctcgtctctcagcgcgaacacgtccgtctggtgatagtgcagcgcgtgcagcaccgccgcggtcggcgacggcacccaggcggtgttggcgcccgtcttcggatgcgccgccttctgctccagcatctcggccatgcggtcgggcgccgcccacatgcccttgccgatctgcgcccggcccgacaggccgcagctcaagccgatcgagacgttgcgcgcctcataggcggcgatccagtcgctggccttgatgtccgcctttcgcaccaccggccccgcctgcatggccgtgtggatctcgtccccggtgcggtccaggaaacccgtgttgatgaagacaatccggtcctttaccgcgtggatgcaggcggcgaggttggccgaggtgcgccgctcctcgtccatcacgccgaccttgatcgtatggcgcggcaggtgcagcaggtcctccaccgcatcgaacagccggtcggtgaaggcgcactcctccggcccgtgcatcttgggtttgacgatgtagatcgagcctgtggcgctgttggcgaaggcgccgagacccttgacgtcgtgcaaggcgatcaggctggtgattaccgcatctagaaccccctccggcgccgcggacccgtcggccagccgcaccgccggcgtggtcatcaggtggccgacgttgcgcacgaacagcaggctccgccccttcagcgtcacctcgccgccgtccggcgcggtccagcggcggtccggctccagcgcccgggtgatcgtctcgccccccttgccgaaggtcaccgacaggtcgcccttcatcaggcccagccagttgcggtaggtggcgaccttgtcctcggcgtcgacggccgcgaccgagtcctccaggtcgacgatggtggtcagcgccgcctccagcaccacatcggccagccccgccggatcgccggcgcccactgggtggctccggtcgatcaccagctccagatgcaggccgttgtgcttcagcacgatggacgagggcgaggccggatcgccgctgaagccgacgaactgttccggcgactgcaacgccggcaccagcgccccatccgtgaccgaccacgcggcaacgtcggcgtgcgatccctccgccagcggcgcggcggtgtccaaaaacgcctttgcccgcgcgaccacgcgcgcgccccggacgggatcatagccgccgccggtcggcggatcgcccagagcatccgtgccgtacagggcgtcatacaggctgccccagcgcgcgttggcggcgttcagcaggaagcgggcgttcagcaccggcaccaccagttgcggcccggcccgccttgcaatctcctcgtccacgcccaccgtcgcgatctggaacggcggggggtcgggcgtcagatagccgatctcgcgcaggaagctttcggtcgcctgggcgtcatgcggctgtccgcgccgcgccgcatgccagtcgtcgatcctcgcctgcagatcgtcgcgggtcttcagaagcgtgcggttctctgacgcgaaccgctggaagatcgtcgccgctcccgcccagaaggcgtcggcggacaggtccagtcccggcaggacctcgtcctcgatcagccggatgagcacttcggcgacctgaaggccggcgcggtcctggtagctcgtcatgcagcggtccgatcagcttgtaacactgcgtgatctattcaccgacggagcggacccgcaagggtccgcagggtcagctttctcgacctttttcggtcatcaagccttaaccgcgtccgtgaacgggaccgcaagcggacgacgctagattggcgttccggacaactccgcgtcccgacccgaggcagaaagccgcccatgctgtttcttttgaacgacgtcgtgttcgacctggacgaggcctgcccggtcacgcctggcgatgcgcgccgcttcgagcggctgagcttcgattacgtgctggagctgggctgcgacatgttcgccgaggacccgctgctgcaccgcaacgacccgcagcgcgcgcgtcggctggcctggctgatccacgatcgaggccccgaggtcaacgccgccctgttcgccgcgcccgctgcgaactgccagcccgatctggtcgagccgcgcttctgcgccctgcccgagggcgtgatccgccagttgcacagccaggccgacgccgaccgcctcggcctcgtcgaagccgaccgcgccgtctggaaccgcctggcggcctgacgcggcctagaagatcacgccgaacagcagatggcccgccgtggccaccgccacgatggcgccgaaccccacggcaaggcccacgctggggtgcaggcgcccgtgcgtctcggaggcgggcagacggtcttcgggatggatcacagccatgatctgtcgtccttctctctacgtttcctcgcggcgccgacttctgtggccgggtcgtctcgcgaggggagcatgactccattccagccgattggccacagccgaacgcccgaggctgcttgaagccgctcgcgttttatgcaggctgcggtgcaacttcggggggagacgctgatgattggcaagttctggcggcgcgttctgatttcggcggctgctggcttggcgctgtccgcacaggcggcgcgggcggagtggctgcgggccgagaccgagcacttcatcatctacggcgacagctccgagcgcaggatgcgcgactatgcgcgcaaggttgaacgcttcgactccctgctgcgcgcctattatcccatccggacggagcaccatctgcccaagctggaaatcttcctcgcccaaggtcgcgccgacatgctcagggcatatccgggcatcgaggccagcgtgggcggatactattctccgaactcagggcgcattcatgccgtggtgaaccgcgaaagcggcatgggtgacgccgtgctgtttcacgagtacggacaccatttcatgttccagatggcctctgcggcttacccggcgtggttcgttgagggctttgcggaatactatgcgcactcggaggttgaaggcgacaccgtgcgcattggtttgttcagcccagggcgcatgaactcgcttactcgcggcaacgccatggcgccgctgcgtgacgtgatcggctggcgcatcctgaagtccggccgctatccggggcacgactattatgcgcaatcctgggcgttgacccactacatgctcagcgatcccgaacgtgcgaaatcgcttggccgctacctcgcggctgtgtcccgcggcgccgatccggtggctgcagtcgagccggaactcggccgcacgccggagcggctggctgatgaactgcgccgctatcttctgcgcggcattaccgtgctgacgccgcaggtcgatctgcccgacgccgacgtcaagatcacgcgccttgacgctgcggactcccaactcgtctggctggacctgcggctggatcgctaccgcctcaacgacggcgccgacaatgacgaagaggagcaggccggcgaagatgagtcggcggacgacatcgccgaagcccgggccaagagccaggaacagcgccgacttttgatcgctcaggcgctggagaccgcttcccgtttcccagatagcgaaaaggctgcgctggtagccgcgcgcgcgcacattctggccggttcgccggacaaggcgctggaacggctgacgccctggatcgaaggggatgacgctgcaagctccgcgttgcgtgtgggcgcatacgccgccatggcccaggccagaaactcgaatgaagaccagccggacatgatgcgacgggcgcgcagctatctgtcacgtggccttgaaaaggatcctctggattttcgaacctacatcgcgcttgacgacagccggagaggaacagccggctacccgaccgcaaacgatttggcgacacttgaagtggccgctgcacttgcgccgcagtccttcgacgctcggatgcgcgcagcggatgcctatctggcccaccaacgtccggcggaggctgtcctcatgctgaccccggtcgtcaacagcccgcatggcggatcaagcagcgaacaggcaaaggcgcagttggcaagggctcaggccctggttcaggcgtcggcttcagtcgtgcgaagcgaagccgcgcctgcagccgagccctcttcgccaacgtcctgagcccgtccggcatcgacagacgccgagtgacggtctatccgcccgccccatgtcgaaactgaccctctcggaagaggcggcgcgtcgccgcaccttcgccatcatcgcacaccctgacgccggcaagaccaccctgacagaacacatcctgctggccggcggcgcgatccgggcggcgggggcggttcgggcgcggggtgagaaccggcgcacccagtcggactggatgaagatcgaaaaggagcgcggcatctccgtttcggcctcggtgatgaccttcgagcacgacggcaagatgttcaacctgctggatacgcccgggcacgaggacttctccgaagacacctaccgcaccctgacggccgccgactgcgccatcatggtgctggacgccgccaagggcatcgagccgcagacgctgaagctgttcgaggtctgccgcctgcgcgacatcccgatcatcaccttcatcaacaagctggaccgcgaggcccaggatccgatggccctgctggacgagatcgcctcgcggcttcagctggaccccgcgcccatctggtggcccgctgagagcgggaaccgcctgcgcggcatggtggagatgggcaccggccgcttccagccctacgcccgcaaggcggcgggcgtcgccgaagacacgccccaccccgaggccctgcccctggccgacgccgcccggttcttcgaggagggcgagcacgagacgctgttggaggcgcaggagttggtggaggctggctatccgaccttcgaccgccaggccttcctcgaggggcacatgacgccggtgctgtggggctcggccttgcgccactttggcatcgacgaactgctgaaggcgatcggcgactgggcgccgccgcccaagacgctggccgcccgcaaggaagccccgcccgaaacccgcaacgcccccgccccgtccgaactgagggtcgagcccggctcggccgaggtgtcgggcttcgtgttcaaggtccaggccaacatggaccccaaccaccgcgaccgcatcgccatgttccgcatggcgtcgggcagcttcaagcgcggcatgaagctgaaggtgcagaacaccggcaagcagctgagcgtcaacgcgcccatcatgttcttcgcctcggatcgtgaactggcggaagacgccttcgccggcgacgtgatcggcattcccaaccatggcgtgctgcgggtgggagacagtctgtcggaaaccggcctgatccgcttcgccggcctgccgaacttcgcgcccgagatcctgcagcgcgtgcgggtcaaggatccgctcaaggccaagcacctgaagaaggcgctggagggcctggccgaggaaggcgtgacccagctgttccggcccgaactcggctctgacttcatcgtcggcgcggtgggtcagctgcagttcgaggtcatggccgaccgcctgggcgaggagtacgggctggacgtggtgttcgagccttccccctacgccgaagcgcgctggatcggcggagaacccgccgacgtcgacgacttcaccggcaagtaccgcccccagatggcgcgcgacatcgaccaggcgcccgtgttcctggccaagtcgtcgtgggagacgggctatgtcggcgaacgcttcccgaagatcgccttcacccggacaaaggagcggggctgatcgccgcgccatcttttcaccgcgcgggtcgcgtgatctgatgcatgtggtggcgctcgtcgcctgctggagctccttatgatcgcccttggcgttctgatcctcgccggcctggtcggcgccgaacccgcgcaggagaacgaactcgtctcctatgcggaggcggtgcagtgcgcggggctgacgcaggcggcgtcggagctggaaggcggcgaaagcgtcgagggcaagcggctgtatgacgcggcgctgtactggtcgctggcggcgatgcaggcggcgacggcggcgggcaagtcggcgcaggcggccgagggcgaccagacgcgcgcccggatcgcagccgtgcgtcgcctcagcgccgaaggggcggcgggccgcgcggccctgcgccagtgcctgcaaaggacgccgaacctgggctgaagcgcttcgccttatgctcaagccgaaccggtcgcgcggccgggcgtttgctgctgacgcggacgagtggccgcaacggtctccttccggcacaggcgaggcggtatgttcgagttcggcaaggatctgcgtaagctgttcgcccaggcgcggcaggatgacgatctcggctgggtcgagctgatcggcgccgatctcctgcgcatcgaggcgcggcagcagtcgacgaatgcgggccgcgtctcctgcccccggcccttcccggcctttctgcgcgccgccgccctgtggcgcgagcacgcccggcgcaccggggcggccgacagcctggcgcgcgcccgggacgcggcccgggacgcagcccgacaggcgacaggtccggatcaaacggcgctggccgccatggaggccgcacacgtcgcgatgatccggttcgacctgtgcggcggggtcgaggggttggagcaggcgggccgggacatggccgcgctgccgcccgttcggcgcgcgcaagccgccgccgctgcgctcaccgcccgcatcgaggcccgcttggcgcgcctgtcgggcgacgacggacgcctgcgcgaggcggcggccgggatggacgcggcgcttcatgggcttgccggcaaggaccgaatccagggcgacgacctgcggatggagcgggcgggcctggcgctggagatcggcgtgatgcgccgggacccatccctgctggatcaggcggggcgcgaactggcggagctgatcgacagcgcctcgcccgactaccggccgctgacgcgcgcgcgcgccctggccctgtgcggaaccggcctgtcggtcctggcgacgctggcgggcgatgcggacgcggccggacagggccgggcgatgttcgaggcggccgctgaccagttcaccccggatcacagcccgctggactggatcgccatccaactcgtcaggtccgaggacgaggcggcgcccctgctgaccctgacccagtgcgaaaccctttctcagggacaagggctgatcctgggcgccttggcgcgcgaacgccgcatcgcgcgcgagacggccctggtggcgacgctgggcgacatgacgggtctggacgcgatcgagacgcgcattcgcgcccgcctggtcaaggcggcggcgtcagagcccctggcctgggccgccgatcagatcggcatggcgcatgtcgcactggcgcgaaccgcgatggcacgcgccgccttgacacgctcccccttcgccggaagccgcgtcgaggcgccgcccgaactgggcctgatcctgacggaggcggccgccaccgcgcgcgaagagggcgcgctggtgctggccgagcgcgccgagcgcctgctggctcagccgccgatggcgacaaacgggccgttcacgaacccgggcttgccataggccagcggcttgccgtcctcggccagcacccgaccgcccgccgcctccagcaccgcctgcccggccgccgtgtcccattccgagatggggcccgagcggggataggcgtcgaaccgcccttcggcgatcaggcagaacttcagcgaagagtccgtgccctgccagcgggtgcagccgtgacgcgccgccaggcgctcggcctcggcgtccgacacgctgtggctcagcagcgccaagccttcgcgcggtcgatcgcgcacccggatcggttgccacgcttcgccgaagcggcggcgggaggcgcccttgccctcgcggcagggtccggcgtcgctgcgccaggtcaggccggtcgccggcgccgacaccacgcccgcgaccaccgccccctgatgaaccagggcgatgttgacggtgaacgcctccccgcccttcacgaacccgcgtgtgccgtccagcggatcgatcagccagaaccagtcggccgccgcatcaggcttcccttgcgcctccgactgctcctctgccacggcctggacgccggggtagagcccgtccagcaactgcaggatcagcgcctcagccttctggtccgccaaggtcaccgggctttggtcggccttggtctgaaccgccacgtcgctgcgccagaagggcaggatcacccgccccgcctcttcggcgatgtccgccaacgccagcgtcagagcgcccgaggcgaggttgcgagccaatcgttcgtgcacggcgtccgtcatcggctgtcgatagcatcaagccggcggttccaagaaccctcaaatcggggcagggtcccggccgtccccgactcgacccaaggcctcgcatgaccccgtccaactccgcacccctcgatctccccgtcgacggtcaggaactggccgcctatgtcgcggccaagctgtgtcacgacttcatcagcccggccggggcgatcagctcgggtctggacctgatgaacgatccggcggcgcaggacatgcgcgacgacgcgctgggcctgatcgagcaaagcgccagaaagctggtcgcgctggtccatttcgcccgggtggcgtttggcgccgcgaccaccagcgagcggttcaccggcggggaactgcagggcctggtgtccggcatgaccgagggcggccgcgcggtgctggactggcggatcgacggcggtgacttctccaagccccaggcgcgcgccctgaccaacctcgcctatttgacggccttggccctgccgatgggcggagaggctgtgatcaccagtcggcgcgacggggacacggtggttctcgaaggccgcgcgcaaggcgcccgcgcccggttgaagcccgaggtggtcaccggcctgaacggccagcggctgacggacggcctcgccggtcagtggatccagccctactggctgtggctgacggtgcgggatgcgggcggaacgctggacctggcggtggaagacggcctggtcgccatcacggcgcggatgccggcctgagatcggacgcatcccaacgcctcgttaaccgacggggcgcgataatccgacgcgagtcatgcccgtcggccatccgcgcggcgcgcgttttcggaaaacgatcttggacctcaggacctgcctcatcgtcgacgacagccggatcatccgcaaggtcgcccggcgcatcgtggaaggtctgggcttcgaggtcgacgaggccgccgacggcgccgaggccctggcccactgcgccggaatgatgccggacgccgtgctcctggactggtccatgccggtgatggacgggctgacgtttctgcgccggctgcgcgccatgccgggcggcgagcggcccaaggtgctgttctgcaccatcgagacgcgagccgaacggatcgccgaggccctgtccgccggcgccgacgaatatgtgatgaagccgttcgacggcgagatcctgcagtccaagctggccgaggtcggctttggtcaggcggcgacggccgtggcggctaccgcctcatgagcccggaggacttcgagcggctgcagggtctgatgatctcgcgcgccgggtttcgtctgacgcgcgaccgcatccggctggccgagcatcggctggcgcccgtcgcgcggcgcgagtcctatgaaagcgtcgaagccatgctggcggccctgtgggcgcggccggtcgcctcgctcggctgggcggtgatcgaggcgctgctgaacccggagacctggtttcgtcgcgaccgcgcgccgttttcggtgttcgagcgcgagttgatcccggcgctggggcgggcgcgcgccgaccggccggtccgggtctggtcggccggctgctcgacaggtcaggagacatggtcgctggccatgggcgcgctggccgccgacgcccgcgtcgaggttctgggcaccgacctgtccagccgcgcgatcgaaaaggcgcgcgccggcgtctacaccggcttcgaaatccagcgcgggctgagcgcccacgccatgctgcgctggttcgtgtccagcgaggatcagtggcgcgccgggcccgaactgacgcaggtcgtccgcttcgcccgggccaacctgctcgacgagccggtcgacgacgcccgcttcgacgtcatcttctgccgcaacgtgcttggcgacatggagccgtcgcggcgcgcccgcgtgctggcgggtctcgagcagcggctggtggacgacggctgcctgttcctgggcctggacgagcgggtcgagggcgacaccatcgcttttcggccggcgcagggccgccggggcgtctacgtcaagtcgcccgcctcgctgcgccgcgcagcctgacgacagttccggacgcaccttttcaccaccaaaccagaacatcttgtgaaccggaacaaaccgtgcacatagtccgtctcatgagggagcgggtccatggcgggtctctcccaagcattgatgggaatcatggcaagggagacgaaggtaatggcacaggcggcgttgaaactggtgggcaaggaagacggagacaagcagcgggcgcttgaggcggcgatcgcacagatcgatcgcgccttcggcaagggctcggtgatgaagctgggcaaggcgggccaggtggccgagatcgaaagcgtctcgaccggctcgctggggctggacatggcgctgggcatcggcggcctgccggtcggccgggtgatcgaggtgttcggtcctgaatcgtcgggcaagacgacgctggcgctgcacaccgtggccgaggtgcagaaaaagggcggggtcgccgcattcgtcgacgccgagcacgcgctggacccggtctacgccggcaagctgggcgtcaatctggacgacctgctggtgtcccagcccgacaccggcgaacaggcgctggagatcgtggacaccctggtgcgttcgggcgccgtggacatcgtggtggtcgactcggtcgccgcgctgacgccgcgcgcggaaatcgagggcgagatgggcgacagcctgcccggcctacaggcccgcctgatgagccaggcgctgcgcaagctgaccgcctcgatcaacaagtccaaatgcatcgtgctgttcatcaaccagatccggcacaagatcggtgtgatgtacggctcgcccgagacgacgaccggcggcaatgcgctgaagttctacgcctcggtgcgcctcgatatccgccgcaccggcgcgatcaagaaccgcgacgaggtggtcggcaacaccacccgggtcaaggtggtcaagaacaaggccgccccgccgttccgcgaggtcatcttcgacatcatgtacggcgagggcatctccaagctgggcgagatcatcgacctgggcgtcaaggccgggatcatcgagaagtcgggcagctggttctcctacgactcgacccggatcggacagggccgcgagaacgtgcgcgagttcctgcgcaccaatcccgacatcgccgcctccatcgaaaaggcggtgcgcgcctcgaccaacaagatcgccgacgacatgctgggcgcgcccgagccggacgagggccaggatctggagggctgatcccaaagccctcttcgccgctcttcctccgtccgggtccggcgacccgccacctaccccgtcggggcgggacggagaaagcgaaggccgttcgacccgaccgtcgaacggcctttttctttaccagaggcccggagccttcccggcggcatggccgttgatcgggtcccctcttcaaggagcctccccatggccgacgaaaagacccaggccctgagccagttcagcctgtccgagaccgatgacggctatctgatcgagatcgaaggcgacggcggcggctcgctgaccgtggaggccacgcccgagcagctcgacgccatcatcgacgccctggacgccctgctctccgaggacgacgccgaagccgacgaagtcgaaggctgatcgcctctgacgcccgtcatccctgcggcatgcgcggggatgacgaggcggggcccgccctccctttccgaaaacgcatggcttgatcgcgcggctggccctatatggcctgttcctcccagccgaaacgcgcgcccatgcccagcctgaacgagatccgctccaccttcctcgacttcttcgcggccgacggccacgccaaggtgcactcggccccgctggtgccgcagaacgatccgtcgctcctgttcgtcaacgcgggcatggtgccgttcaaggactatttcaccggcgcctcggccccgccctacaagcgcgcgacctcgtcgcagaaatgcgtgcgcgcgggcggcaagcacaacgacctggacaacgttggctacaccgcccgccaccacaccttttttgagatgctgggaaatttttccttcggcgactatttcaaagagcacgcgatcgagcgcgcctggaccttggtcacaaaggagttcggccttgatcccaagcggctgatggtgaccgtctacatcgacgacgacgaggccttcgacatctggaaaaaggtcgctggcttctcggacgacaagatcgtgcgcatcgccggctccgacaacttctgggccatgggcgacaacggcccctgcggtccctgcaccgagatattctacgaccacggcgaccacatccccggcggccctccgggctcgccggacgaggacggcgaccgcttcgtcgagatctggaacaacgtcttcatgcagttcgagaaggagaacgaccagatcgttcgaaagctcgaaaagccgtccatcgacaccggcatggggctggagcggatcgccgcggtgctgcagggcgtgcactccaactatgaggtggacctgttccgccgcctgatcgccgcctccgaagaggcgacctcgaccacggccgagggtgagcgcaaggccagccaccgcgtcatcgccgaccacctgcgctcctcctccttcttgatcgccgacggggtcacgccctcgaacgaagggcgcggctatgtgctgcgccgcatcatgcgccgcgccatgcgccatgctcacctgctgggcgcgcaggatccgctgatgcaccgcctggtgccggccttggtcggccagatgggcgacgcctatcccgaactcgcccgcgcccaggcctttatcgaggacacgctgaagcaggaggagatccgcttccgcaccaccctgggccgcggcatgggcctcttggaagacgcgtcgcgcgcgctgggcgacggcggcgtgctgtcgggccagaccgccttcaccctctacgacacctacggcttcccgctcgacctgacgcaggacgaggcgcgtcggcgcggcttcaccgtcgatgtggagggcttcgacgtcgccatgaccgaacagcgcgcccgctcgcgcgagcactggaagggttcgggccagagcgccaacgcctccgaatggctgtccgtgcgcgaccggatggggcccaccgtcttcaccggctatgactcggtcgacggttctggcgaggtgctggcgctgatgaaggcgggcgaaccgacggacgcggccgaaaccggcgagatcgtcgaaatcctgctggaccagacccccttctacgctgaaagcggcggccagacgggcgaccacggcacattggaatggccgggcggcgaagccgaggtcatcgacgtcaagaagcacgccggagacctgcacgtcctgtcggccgagatcacggcgggaacgctggaactcggcgcccgcgtggcccagctggtcgatgccgacaagcgccagaccacccgcgccaaccactcggccgcgcacctgctgcacaccgcgttgaagaacgtgctgggtccgcatgtggcgcagaagggccagctggtggacgccgagcgcgcgcgcttcgacttcagccacaacgcccccgtgaccgacgatcagatcgccgccatcgaggccgaggtgaacgccgtgatccgccagaacgtgccggcggagaccaagctgatggcgccgcaggaggccatcgaggccggcgccatcgccctgttcggcgagaagtacggcgacgaggtccgcgtcctgacgctgggccggtcgctgaccagcgacaacgcgccctattcggtggaactgtgcggcggcacccatgtggcgcgcaccggcgacatcgccctattcaaggtggtgtccgaggccggggtcgcggccggcgtgcgccgcatcgagggcctgaccggcgaggcggcccgcctctatctggaaggccaggcccggatcgcgcgcggtctcgcccgcgacttcaaggtccagcccgccgacgtggtcggccgtgtcgagggcctgcagacctcggtcaagacgctggagaagcaggtcgccgagctgaagaagcagctcgccttgggcggcggctccggcgcgtccgcggcgccggaggagatcaatggcgtcaagctgatcgcgcgcgtgctggacggcgtggacggcaagggcctgcgcggcgtggccgaggacttccgcaaacaggtcggctcgggtgtcgtcgccctgatcggcgtgacggacggccgcgcggcggtgacggttgcggcgaccagcgacatggccggccgcgtcaacgccgccgatctggcgcgcgcggccgtgctggcgatgggcggccagggcgcgggcggcaaggccgatttcgcccagggcggcgcacccgatggctccaaggccgaagagggcctggccgccgtccgcgcagccctggctggctaggcgcggcctaggcggcgggttcgggcgtcaggcccccgcccgccagcttccagctgaacgccccccgccgctgcatcagcagcaccagcggatcgtccgggcggctctcgcgcgtcagggtcaccgcaaaggtgttgaggtcgcggtaggcccaggactggcgcacgtcgccgcccgagtccgtctgcggcgtctcaggcgcgcggctctgcggatcgggggcctcgccctcgcgcaccagggcggcgacgccttgcggggtgacgaagctgtccaccgcccccgcgaccagctgcggcgccagcagcatgcccagactgcccagcgcgccgccgcgccgatcgccgccgaactcggccagcagccgcgcgctcagttcgtccttcaggctctggcggaaggcggggaaatcgacgtgccgttcgatgccggcggcatcccccgcgcgcgcggccctcaccaggctctgcgcggtcaggaacggcgctgcgaaaaacgccccggcgaacccgagcacgaccaaaacggccagcgtccacaacagtttgcgtttcatggcatcccctcctcgccgcaacaaagacttcagcgcgcggccggttgcgtcagcgcagggcccacgaccgcctgcggcagcccgatgtggaccagccgccactcgaacggtccacgccgttcaaaggtgaacagggtgcgctcgcccccgtcctgaccgggcaccgacacgcgcgcgcggttgaagctccagaacgccggccagggctggcgtcggaagccgcccttcggcgtctccgcgcccgccgtaaaggcgtccgcgcgacggccgtagcccagcgtcagggcgtgcagggcgcgcggcgacagatagatttcgggatcgactgcggtccgcaccggccgcgtcaccgactgctggaactgccggcgcaccgcggcgaccggatcctggaagaaggacggcggcggcgtcagcggctcgggccgtcccgacagctgcggccgcagcgacgcacgcaccgcatcatagtcgatcaaccggctgagcccctgcacgtcggaggcgtccgaagccgcccggatggcgccgaacgcgaaaaagggcgcggcgacgaaacacacgaccacggcgaccacggcgatcaggatcagcttgctcagcagtcgcttgatcgagggctcgcgtcgctcggccgccttgcgttcggcctcgcgcacccagatcgggcgagtgtcggcggacggcggacgggcatcggtcatgcggcggaacgggccttcatactgcgcccagtgggccacgccccctaacgcgcggtcaagctcgatggatgcgaaaacgcccgccggatcgctccggcgggcgtcattcttgttcgggctatcgtgcttcgcactgcttgagcccgtatgtgggctatcgcgctttgtgctgcttgagcccgaagatcctcgccttacgccgcttgcggcagggctgccttcaggttctcggcgaccttgtcgaggaagccttcggtggtcagccagccctgctgatcgccgaccagaagcgccaggtccttggtcatgaagccggcctcgacggtgtccaccactaccttctccagcgtctcggcgaacacgcccagctcggcgttgccgtccagcttggcgcggtgcttgaagccgcgcgtccaggcgaagatcgaggcgatcgagttggtcgaggtggcctcgcccttctggtgctggcgatagtggcgggtcaccgtgccgtgcgcggcctcggtctccagcaccttgccgtccggcgtcatcagcaccgaggtcatcaggcccagcgagccgaagccctgcgccaccacgtccgactgcacgtcgccgtcgtagttcttgcacgcccagacaaagccgcccgaccacttgatggcggccgccaccatgtcgtcgatcaggcggtgctcataggtcaggccgcgtgcgtcgaactcggccttgaactcggcgtcgaacacttcctggaaaaggtccttgaagcggccgtcgtaggccttgaggatggtgttcttggtcgacagatagaccggatagttgcggttcaggccgtaggcgaagctggcgcgcgcgaactcgcggatcgagtcgtccaggttgtacatgcccatggcgacgccggcggacggcgacttgaacacctcgtgctcgatcacttcgccgtcgtcgccaacgaacttgatcgacagggtgcccgcgcccggcatcaggaagtcggtggccttgtactggtcgccgaaggcgtgacggccgaccacgatgggctgggtccagcccggcaccaggcgcggcacgttggagcagatgatcggctcgcggaagaccacgccgcccaggatgttgcggatggtgccgttgggcgacttccacatcttcttcaggccgaactccttcacccgcgcttcgtccggggtgatggtcgcgcacttgaccccgacgccgtgcttctggattgcgtgggcggcgtcgatcgtcacctgatcttcggtggcgtcgcggttctccatgcccaggtcgtagtagtccagctccaggtccaggaacgggtgcaccagcttgtccttgatcatctgccagatgatgcgggtcatttcgtcgccgtcgatgtcgacgatggggttggcgaccttgatcttggccatgcgtgaatccgcctgtgctggggagaaaagaaggtggtggcggtatagccgccgtgttccgcatcgcaaagagcacggcgcgcaaagccgaggcgggtcgtgccttcgttaaccttgccttgaaatcgccttctgcggtcaagctgaaccgtcgccgttcgatggccgttttcaaaccggaagggtcaaccggaacggagatggcatgacggcaacgacggaacagctgatcgacgagtggatcgggcgctttggcgaaccgccgatcctggccgacgcggaactgatgcgcgccctgctcgctgaacacccggcatcccaggagcagtcctcatgacggaaaagaccttcaagtccggcgacaaggtgaaatgggaccacagccagggcacgaccaccggcaaggtcgtcaagaagctgacctcggagacccacatcaagggccacaaggtcgccgcctccaaggacaatcccgagtacctggtggagagcggcaagaccggcgcccaggccgcgcccaagccttcggagctgcgcaaggcgtgacgaccgtacagcctgaagttcttgtgatcggcgcaggcccggccggtctgaccgcagcgacctatctggcccggttccggcggccggtgctggtggccgacggcggggagccgcgcgccaactggatccccgtcagccacaacacgccgggcttcccagagggcctgaccggccgggacatgctggcccgcatgcgtgcgcaggccgaggaatacggcgcggtcatcgaggccgggcgcgcggaaaacctgcggccggtcgaggacggcttcgaggccgatctgaacgggcgcacggtgcgggtgcgggcggtgctgctcgcctcgggcctggaggaccaccatccggacctgccgggcgtcgacccggccatccggcgcagcctggtgcgcatctgcccgatctgcgacggctatgaggccaccggcaagcgggtggccgtgatcgggaacagcgatctcggcatccgagaggcggcgttcctgcgcacctactccgacgaggtgaccctgttccacatcggtccgcccgaggccctgacctgccgctcggagctggatcggctgggcgtcaccctgctggagggctcggtcgagggtgtttcgctggagggcgaccgcgtgcgcgccatcagctggggcgggaccgagcgggccttcgacttcctctactcggccctgggcaccacgccgaactgcaggctggcgcgcagcctgggcgcccggctggcgaccgacggccggcttgaggtggacctccaccagctgaccagcgtgcccgggctctatgccgccggcgacgtggtgcgcggcctcaaccagatcgcggtcgccaccgccgaggccgccgtggccgccaccgccatccacaatctgctgcgacagcaggacggcatgacggtgcgcgactaggcaggcgcagtcaggcctggctggccgtccagccgtccacaatccgctccagcaccgacagcggcacgccccccgcagccagcgccgtgtcgtggaagccgcgctggtcgaagcgcgcgccgaggcggctcctggctttgtcgcgcaggcgcacccattcgttgtgcccgaccttgtaggcgcaggcctgacccggccagccgcagtaccgctcgacctccgatgtcgccgcgccctcggtgtcgccgtatgcggtcatcatgtagcgaatgccctcttcgcggctccagcccttggcgtggatgccggtgtccacaaccagccgcgccgcccggaacatcaacgactgcagatagccgatctgccccgccggatcgtcttggtaggcgccgagctcgtccgccagctgctcggcgtacagcccccagccctcgccataggccgagaagaagaacaggttcatcagcttgggcgccgaggggctttcctgctgcagggcgatctgcaggtgatggccgggcgaggcctcgtgataggtcagggtcggcagggtccacgacggccagtccgccgtgtccttcaggttgatccagtagatgcccggccgcgatccatccagcgaggggctgttgtagtagcccatcggcgcgccctgctcgatcgccggcggcacccgcttgatctcggcgccggccttgggcaaccggccgaaggcgttgggcagacgagcctgcatggcccccatctgctcgttcagcttgccgatcaactcggccttgcccgcatcggtgttgggatagatgtatttgggatcggctcccatggcggcgatgcgctcggccaccgacccttgcgtcatgccctgggccttcagcagcacatcggcgcgtccggacagctcggccacctgctccagtcccgtgcggtggatctcgtcggcgctcagccgggtggtggtgatgtagcgcaggctgttggcgtaatactgctcgccctgcggcagccgccggaccgaggcctcgtgcgtcgcgccgggctgggctgccttcagaacccccgtctgcgccgccagcgccggatagacccgctccgtcagcagccgctcgacccgcgcgccccagtcgccggtcaggcccttgtcgcgggtgcggctgacgaccgattcgaccatcgaggactcggccgccggcgtgccggtcatgccctcctgctgccggatcgccttggccaggatgaagtcgggcggcacaacgcccagggcgaaatcctcgcgcacccgctcggtttcgaccgtcagcacgtcggccagcgcctcgatgcgcgccacataggcgtcggcgtcccccgccgtttcaatggtgtgctgattggccaggaagtccggcgcggactgataggcgccgccctgctggctgacacgatacggattgggccagccgccctggccgtagggaatggcgtaggtggcgatcgtcgcgtccagattgtcgaccagggtgtcgtagtagatgcggtcccgctcgctcatgccggccgcgtccatgcgggccaactcggcctgttgggccagggtgaaggcgcggcctcgctcctccgtctccggggtggggatggtcagctgcgacttggcggcggcgcgcgcgcccttgtcgaggcccaggctggtcaccgtctcggggctgaggtccagcgcctgctcgaaggtgcgatccatgaaggcccacaagggcgtgggcgcaggctcgccttgtgcgagggcgggcgccccgatggcggccatgccggcgccggcggcggtggtctgcagcagacgacgacgattgatcatggcgagaactcccctgttcagaccggcagtggagctcgcgcggacacgcgccgcaagtaggaattccgggtcgtgaccacgtcagcccgcgtgcagctccttcttcacccgctcggccagggtcttgatgtccagcggtttgggcaggaaggacacgcccacctcgtcctgcagcagatcggagaagtcgctttcggcgtagccggagatgaacatcaccggcgcgtcacccaggtagggccgggccttcttcagcagggacgggccgtccagtcccggcatgatcacgtcggagatcagcatgtcgatctcgccggcgtgctcctcggccaggatcagggcctcctcgccgtcggcggcctctatgacctcatagccgcgctggcgcagaaggcgggcggcgatgccgcgaacggcggcctcatcctcgacgaacaggatgcggccggcgcccgacaggtcgcgcggcgccttgaccttgacctcgatcggctgaacctcggccagctccgcctccccggcggccggcaggaagatgcgaaacgccgcgcccgcgccgtccagattgccgacggtgatgtgcccgcccgcctgctgcacgatgccgtagacggtggccaagcccatgccggtgccctcgttaaccgccttggtggtgaagaagggctcaaagatcttgtcggccagttcgggcggcacgccggggccggtgtccgacacctcgatcagggcgacctcgtctgtcgccacggcggtccagcccatggcgcgcgcctgatcggcggtcaggcggcgggtcttgatggtgaccacggcgtcgcccggctcgaccacgccacgcatggcgtcgcgggcgttgaccgccaggttcatcaccgccgtctccagctgggacttgtcggccagcaccaccggcaggtcgcggccgtaatcggtctccagcctcacgtcctcgcgcaacagccggcgcagcagcaccgcgaattcgcccaccagctcgcccaggtccagccgctcgcgccgaacggtggacttgcgcgaaaaggccaggagcttgcgcaccagatcggccgcgcggatggccgtttgacggatttcgttgagcccctcataggacggatcgccgaccgggtgccgctccagcaggcccgacagctgcagctggatggcggtcagcaggttgttgaaatcgtgggcgaccccgccggccagttggcccaccgcctgcatcttctgcgcttgggacagctgcagctccatcgacttctgcgccgaaacgtcgaacagccagatgcggcgcttgtcgccctcgggcgcgacatagaggtgcagcatccggtcgggaaaggcgcgggcgaccagctcgatcggaccggatgacccggcgaccagcttggcgcgcgcctcgccgacgcccgccggttcgaacaggtggccgaaggcggcgtcgccggccgcggccggcccggtcaggaccttgagcgcggcgttcggctcctccgcccggccgacgaacaggtcctcgccgccgatcaccgccgagccgaacggcgcaccggccgccatggcgcgcgcgtcgccgggcagggcggcctgggcgcgcggctcggacgcgccggtcctcagatcgggcagggccgcgtcgggcgcggcgcgcaccagatagcgcccctcgccggccaggccgatcacgacctccaactcgcgctcgccgatctcgagaatagctcggcccgtctgacgacgtcgcgcctgggcgaaggccatgtacagcgcctgagccgacttgccgcgcggcagggcgacgtcggcgccgttcgcctcggcccaggctgcgttgaaggccaacacctgccccgacgccaagaccagcgccgcgggctcggccatggcgtccagcaggtcgacggccacgtcgctggcgggccgccccgcctccgcccgccggaagccgaaaagccccaccagggcgatcagccccgccgtcaggatcaggatcatgcccggcgccgaccacggattgccccggaacgccggataggccatcgccccgaccgccagcgccagcccggcggccatggcggccagcagcggatcgaacggaagacgacgggcggtgatcatgcggcctcgcgcaagggaatcagtcaacggatcatagaggatcgcgcccgatcccgcttatcggcgtttgcgcgactggaatacgaagccgatcacctgggcggcggcctggaaatgctcgggcggaatggtctggtcgatgtccacggcggcgtagagggcgcgcgccaggggcacgttctcgacgatcggcacgtcgtggtcgcgcgccacctcgcggatgcgcagcgccagcgcatcgacgcccttcgccacgcagacgggcgcgccgtcgccctggtccggctcgtagcgcagggccaccgaatagtgggtcgggttggtgacgatgacagtggcggtcggcacggcctgcatcatccgctggcggctgcgctgcatgcggatctggcgcagcttggccttgatgtgcgggtcgccttcggactgcttgtagtcctccttcagctcctccttggacatccgcatcttcttggcgaaactgatcttctgccacagaaagtcggcgccggcggtgaagccgaacaggacgatggcagaggccatcagcgcgaccgccagatcgcgcgacagcggcaggatggcggccggactcatcgccgccaggttctcgagctcgcgcgtgtgcgacttcagcacggcccagcagacgcagccggtggcgatcagtttcacgaacgtcttcaggaactgcaccaggccgtcggggccgaagatgcgcttgaagccggccagcgggctcaccgccttccagttcggcttcagcttctcggcggtgaagatcaggccggtctgggccaggttgccgccgatcccgccgatggaggccgccagcatcaccgcgcccaggaacggcgccatggcccacagcgcgcgcgccgcgatctggccgcccgcgccgccctccagcgcgccgaccatggtgtgcggcgccgcgatgaacggcagcagctgctcggccatggaggtcgcaaaccagccgccggccgacaggatcaccgccgccgcccccgccagcgccagcgccgagccgatgtcctgggatttggcgacgtcgcccttgcgccgcgcctcgtcgagttttcgcggggtggcttcttctgttttcgactcgggatcggcgccttcagccaccggcccctccccccacgccctgcgcgaagacctcggccagccggcgatagcggtcgatgaagacggtccccagcacgcccaggctcagggcgaacaccgacaggcccagcaggatcgacaagggcgccgaggcgaagaacacctggaactgcggcatgacccgcccgaccagcccggtcgccaggttgaagatcagggcgaaaaccagcaccggcgccgccagctgcaccccgatcagaaagctgtcgccgagcgtccgcaccgccaggctggtgaagtcgctcatcatcaagggattggccggggcgatcagccgataggagccgacgatgccggcgatgaacaggtggtgggtgtttgtggcgaacagcagggtcacgcccaacagcgtcagaaaggtcgcgatggtcgatccgggcgacgcctgcagcggattggcggtctgggcgaagctcagcgtggtctgcagcgagacgatctcgccggcggtggccagcgccgtcatgaacatccgcagcagaaggccgatcatcagccccgtgatcacctcgcgcaggatccagccgatcatggcgctcatctccgcgggcagcggcggcagggacccgctgacgatgggccacagcgccaggctgatcaccagcgccagcgacaggcgcacgcgcggcggcacataggcctcgccgatgccgggaatcagcatcaggatggcgccgacccgcgccaggatcagcccgccggcccagacctgatcggcggtcgcgtagggttccactacatgcccgcaatgcgcgcggcgatctcgcgcatgaagccgcccagcatggcccccatcaggggcaggaacaccagcagcgacacgaagatggcgatgatcttgggcgcatagaccagggtctgttcctggatctgcgtcagcgcctgcaccaggccgatcacaacgcccaccaccaaaccgacgatcagcacgggcgcgcacagctggatggtcagccacagggcgtcgcggcccacatccatcacttccgcgccgttcatgcgtccattctccgggaacaaccgggcagaaaatgccgggcgtctggttaacgccgcgctaaccgcccgcccgcctctcccctttggcgcggcgcgcgtctatatcgccgccatgaccgatgcagccgtgtccgccgaagaagccgaagccgccgtccgcaccctgatccgctgggcgggcgacaacccggaccgcgagggcctgctggagaccccggcccgcgtcgcgcgcagctacaaggagctgttcgccggctacgaggccgatccgcgcgcctatctggaaaagaccttcgaggaggtcggcggctatgacgagctggtggtgctgaaggacatccgctttgtctccttctgcgaacaccacatgctgccggtggtcgggcgggcgcacgtcgcctatctgccgaccgaccgcgtggtcggcatctccaagctggcgcgcgtcgtccagggcttcgccaagcgcctgcagatccaagagaagatgacctccgacatcgccaaggcgatccaggaggtgctgcgtccgcaaggtgtgggcgtggtgatcgaggccgagcacagctgcaagaccatgcgcggcgtcaatgtgccgggcgccagcctgtcgacctcgtgcctgcttggagtcgtgcgcgacgatccccgcacccgcgaggagttcctgcgcctggtgcgctgaagccgcttcgaccggcccggctcttgcgacaggtgagctcgaaggagcgcacgccatgccttgggccgccgtcatgacccgaaacgacacaacccccatcgcgcgcgggggctggctagatgcgctgcgtttcatcgtggcctcgctgatcatcctgcatcacttccaggcttcggcccccgtgccgctggccgaaggcctgcacccggtgttcgagcgcggcggctttctcctgaccaacttctttctgatcgactccggctatgtgctgatgcgggtctatggcggcccggtgctggacggccggatgtcggcgggcgacttcttcctgaagcgggtgctgcggggcgcgccggcccccctgatcatggggctgtcgctgggggcgctggtgcttctgggcacggcgctgggggcgccgccgacccatcccgagtggttcgcctgggatcagctgccggcgcagcttctgctggtgcagtcgttcggcgtgtacggcggcctcggctggaacgcgccgtcctggtccatctcggccctgatcggctgctacctgtgcttcccctggataatccgcggcctgatgcggatgcggccgtggacggcgctggcgacaggcgtcgtcgcctacctcctcgccaatgagatcacctgggcgctgctggactttcccgtctaccagatgccgatgcgctacggcttcattcgcgcgctgccgctgttcttcctgggcatgtgcctggcgtggttcgcgcaaagggtctggatttctccgcgtctggcgggctgggccggcgtgctggcggcgatcgcgctggcgaccgtgcagcatttcgacaagcacgcactggcgtcgctcctgttcatctcggtcatcatcctggcggcgggcgccattccggtgacgcgcccgtccaagctgatcgagaagacggcggtggtgtccttctccatgttcatcaccaatgaggtggtgcgcatcgcctggttcggcggcgcgggcgtggcggccagccgactggcgctgccggtgtcggtgcagtggggcctgtgggggctgggcgtcgtggccgcctttgtgttcgccttcctgtttcaccgctggatcgacgatcccattcagcggctgatccgcagacggctggcggcgcgcggcgggtcgagcgccgccgccgccgtaccccgcccggtggtgtccatcgacggctgacccccgccttcatgtcctctgaattgacgatgcgcggcgcccggccaagaggttaatgaaaccttagcaagccaatggacgtgatgaggcggccttgaacaccgacagtttcgcgctggaggcgatggcgcgtggagcgggcgtaagagtcaggtgccccgcatcggcgtcgagcaagcgcgcctttgacgtcgtgatctcggccatgctgctcgtcatcttcgcgccgctgctgctgcttgcagccctcgctgttgcggccgagggcgagggagtgctgtttcgccagcgccgcaccggcctgaacggccacgtgttcaccatcctgaagttccgcaccatgacggtggccgaggacgggggcgccgtcgcccacgcccgtccaggagacccccgcgtgacgcgcatcggcgcgctcctgcgcgccacgagcctcgatgagctgccgcagctgatcaatgtgctgcgcggcgacatgtccctggtcggcccgcgcccccacgccgtggcccatgaccaccactatgcagcgctgctgccgctgtatcgcgatcgattcgccgtccgccccggcctaacgggcctggcgcaggtgcgcggcctgcgcggcgaaatccgccagctgggctgcatggcgcgccggatcgaggcggacctgcattacgcccgccactggtccttctggaccgaccttctgatcctgtggcgcaccgcgcccgcggtgctgtcgcgcgtcaacgcctgctaggggccgctactcggcgtccggctgcatcgccggcgcggtggcggaaaaggcctccagctccatgcacgccgcctcgatcgcctgaaggcgaggccagcgcacctccacgccgaaccgtcgcgcattcgccagctggggcgcgatcacgatgtcggccagcgtcggccggtctccgaacgcgaagggacccggcgtcccagccagcatccgctcgaccgcatccagcccgtccttgatcacccacgcggcccaggcctgcacctgcgactcgtcctgacccagctcacgcagccgcttcagcaccttgaggttctgaaccggatggatgtcgcaggccacggcctgcgccacggcccgcacccgcgcgcgcatcaccgggtcgacgggcagaagcggcggctccggatgggtctcgtccagatattcgacaatggccatggactgggtcagcgccgttccgtcgtccagcaccagcgtcggcagcaacccttgcgggttcagcgccagatactcggtcgagcgctgctcgccctttcgcaggtgatgaaagacgtctccgccccgcagcccttggagcgccagcgggaggcgcccccgccacgccgcgctggatcgaaaatagccgtgcaggatcatgacgccgcctcctcgcgccgcctctgcatgagggtcggcgcgcgtccgaccgagtagcccgcgcgcgccgccgtgttcaacccggatcagaagccggtctgaacccgcagggtggcggtgttgccgccgtcgtcgcccgcgaatacgccggtccggttctccaccgaccaggcgctccagtgtgcggagacgcgggtgttgttggtgggataccagttgacgcccagcgcccaggcgtcgccttcgccgcccgtcggactgtcgctgtagtcggcctggtcgtagcggcccaccagctcgaccgcgccatagccgtcgccgccgcccaggggcctcagcaccttgggacgctgccacgtgccggagcgggtggacagaggcggcgcctcgccggtgagaaagaagccggccgacacggcgtaggcgtcctggtcgaagtcgcgcgcggctgtctccagcacccgccggccgccctcgaccatcagacagcccgggccgcgcacgccgcccagctccagtccaaagccgcggctgccttcgggcgcggcataggggccgctggccagtcgcaggttgtcgttgaagcgcgaggagaccaccaggttgcgcgatgcaatggtcgtggcgggcgtcaggtcctcggcgaaggcccagccgcccaggtgcaggaagccgtcgtcggtcttgaacgccgacaggtgggtgcggcccatgacggtcagggtgtcgtcagtcgtaccgtcgctgatcgcgtcgccggtcaccgacagcgagccgtgccagacgccgcccgtcagctttgacgtcacgcccacgccataggcgccgcgttccggtcctagggtggagaccatcaggctgcgctccaggaacggggtctggtcctcggcggtgccgccctcgacgccccgatcgttgaggcgctggccgacggagacctccaggtcacggccgcccagcttgcgattataggccacgaatgcgttggccacgctgagggcgttgtcggcgaggtcgccctcgacccagtaggtgaagccgccggcgacacgcccctgcgcgcctaggcgcaggccgcgcagctcggtgcccgccaggttgcggccgtcgaagtcggagccgctggtgctggacaggtcggccgtgacgcgcacgcgcggcttgaaggtgaaggcgccgtccgggctgcgcagttcaggcaggccggtggaccagtcgacggcggccggggtcgcggcggtctgggccggacgcggaggatcgttgggtgcggcgggcgtcgcgggcgcggcggctgcggccgccggcgtctgagcggcgacggcgaggggcgcggaggccgagcgctgctgcgcctccagctgctccagcctcgcggacagggcctgtacctgggcgcgcagggccgagatttcatcggcgctcggcgccgtctgcgccagggccgaggtggcgagcgcggccaggccgacacccgccgcgagagtgcggagatggttcatgtcgataagccttaacgggagggatttaacgaagcgcccaagacgctcgtacgcagaagttcgtagtcgacgtcgttcgcgcggaactgcggcgccgccgccagaggcgaacggcgccgctttccggggaggaaatcagtcggcggtgacccgatccttgtcgcccggaccggcggcggggtccggcagggcgctcagaggcttggccggtccttcgagcgcggccttcagcgcgtcgcggtccagctcgccttcccagcgggcgaccacgatggtggcgaccgcattgccgatgaagttggtcagggcccggcactcgctcatgaaccggtcgatgccgaggatcagcgccatgcccgcgaccggcacggtgggcaccaccgacagcgtggccgcaagggtgatgaagcctgcgcccgtgatcccggccgcacccttggacgacagcatggcgaccagcaacagcagaatttgctgctgcagcgtcaggtcgatgttcagcgcctgggcgatgaacagggcggccatggtcatgtagatgttggtgccgtccaggttgaacgaatagccggtcggcacgaccaggccgaccaccgacttggaggcgcccgcgcgctccatcttgttcagcagcgacggcagcgccgcttccgacgaggaggtgcccagcaccagcagcagttcttccttcagatagcggatcagcttcaggatgttgaagccgttggcccaggcgacgaggcccagcacgcccaccacgaagacggcggcggtgatgtagaaggtggcgacgagggccgccaggttggcgatcgagcctatcccgtatttgccgatggtgaaggcgaaggccccgaacgccccgatgggggcggccttcatcagtatggccaccagcttgaagaaggcgtggctgaccgactccaggaaggtcaacacgggcttgccgacgtcgccgaccatggccagggcgatgccgaacagcaccgagacgaacagcacctgcaggatgttgccctcggagaaggcggacaccaccgtgtcggggatgatgccggtcagaaagccgacaatggtcgtctcgtgcgcctgctccgaatatttctcgaccgcgcccgcatccagcgtcgccggatcgatgttcaggccgtttccgggctggaccacattgccgatgatcatgccgacgatcagggccagggtggagaaggtcaggaagtaggcgaaggccttggcggcgacctggccgacgcggccgatgtccgccatgccggcgatgccggtgacaatggtcaggaagatcaccggcgcgatgatcatcttcaccagcttgatgaaggcgtcgccaagcggcttcagctgttcgcccagccccgccaccgcctcgccgttcggccccacggtgctgggatagaagtggccgatcaggccgcccagcacgatggcggcgatcacctgaaagtagagctgggcgtagaagggcttgcgcttcagcggcgcgccttcggcggctatcggaatcatgtcgacctcccgtcagcgctcttggggcgcggttcggccgccatggtgacgcccggcgcgcgtgcggaaaaccgcgaccgcatgcgccggcgagccgtcgctttttctttagaaacaacgttgatccaaccggagccgagagagtgagtgcgaagttggtgacacccatgcagaaattgtgcgaaaatccgcacatgctgcgcaccgtcgctggagcccgccgcctggtgctgatcgccgcagcgatcgcctttgtcacgcttgtcgtgtgggttggcgggcgcatctctggagccgacgccgaggctgagctgcgtcaacgcgcgcaggctgccctggcgctgaacctcgccctgctggacagcgagttgcagcgtcaccgcgccactccggtcattctcgccacggaggagccgctgcgcaccctgctgcagcgaccggacgacgacgcgcgcgccgtggtcaatgcgcgactggaagccctggcgcgacagactggcgccgacgccatctatgtgacggaccgacgggggacggcgctcgccgccagcaactatcgcggccctgcgagctttgtcggcgccgactacgcctttcggccctatttccagaacgccatgcgccagggctcggccgagttcttcggccagggcagcgtcagtcgcgaacccggtctctacatatcccgacgcatcgacggaccggacgggccgctgggcgtggtggtggcgaaggtccagttccaggcggtggagtccgcctggcgtcgacaggacggcgaggtcgtcgtggccgacgccaacggcgtgatcctcctggcatcaaagccggagcgtcgcttttccacgctgtcgcccctgccggaaccgcttcgccgacagctgatcgagacgcggcagttcggcgagtcgccgttgaggtggaccggcgcttccgtctcgcctccggaccaggtggagatcgacggggcgcgtctgctggtctcgcaagccgcgatcggcgccgccggttggcgattgcaggtgtggacgccgatgcgacccgtagaagcgcgcgaggcggtggggcggtggctgggcctcctaggctccatgctgctgctgctggcgggcgcggccctgcgcgcggtcatgctgcggtcgcgacggcgggccgaggccgaaagcgacgcgcgccgcctgctggaggccaaggtcggtcagcgcacccaggccctgacggaggccaatggtcgactgtcgcgcgaagtcaccgagcggcgcgaggcggagacccggcttcggcgtcttcaggcggatctggtgcaggccaaccgcctggctcagatgggccagaccatggccggcgtcgcccacgagatcaatcagccggtcgcggccatacgcgccaacgccgacaacgccctgatcctgctggaccggcgcgaggaggccgaagcccgcgccaatctggcccgcatccagtcgctgaccggacgcatcggcggcatcatcgaaagcctgcgcggcctggctcgcaagtcgcctgcgaacgcgcgtccggtgctggtgtcagaggcgatcgagggcgccgtcctgctgctggccagccgcgaccgcgtgggtcgtctgacggtcaccggagaggtccagggcacgcgcgtccttgccgaccgggtgcgcctggagcaggtgttgatcaacctcttgcagaacgcctttgaagccgtggagggcgcaccggacgcggcggtgaccctgtcggtcgagacggacggcgatcgcgtgcgcctggccgtcgccgataacgggccgggcgtgccgcaggccatgcgtggggccctgttcacccctttcgcgaccggcaagcccaacggcctgggcctgggcctcgtgatctcgcgcgacatcatggagagcatcggcggcgacctggcgcttgatgacggcggcggcggaacaggcgcccggttcgtcgccgccctcaggcgggccgcgccatgaccacgatcgcaacacgggtgctgctggtcgacgacgacgaagatctgcggcacgcccatctccagacgctgaggctggccgaggcgcccgcgcgcggcttcgccggagccgaagacgccctgcgccacatcgaccgcgccttcgccggcgtggtggtcaccgacgtgcggatgccgggcatggacgggctggccttcgcctcccgcatccgcgagatcgaccccgacctgccggtcattctgatgaccgggcacggcgacatcgacatggcggttcaggcgctgaagaacggcgccttcgacttcctggtcaagccgttcgccgccgaacggctgttgacggcggtcggtcatgcgctgcgccagcgtgatctggtgctggagaaccgccgactgaccgagcttgtcgcgcgcggcgacaacggcctggatcagtccggcctcctgggtcagtcgccggccatggcgcacgtccgcagcatcatcggcgccgtggcgagcggggacgtggacgtgctgatcctgggcgacagcggcgtcggcaaggaggtcgccgcccgcgccctgcaccgccagagccggcgcgcgcgcaagccctttgtggtggtcaactgcgccgccttgtccgaggcggcgctggacggcgagctgttcggccgagcggccccgggctccgccaacggccgccgcgtcggcgggcgcatccgggaggcggcgggcggcacccttctggtggacgagatcgacgccctgcccccgccgctgcaggcgcggctgctgcgcctgatcgaggacggcgagctgacgcaggaaggcggcgacagcgaagcggccgacgtgcgcgtggtcgccaccagccggttcgcactggaggaggcggtggccgccggccgcttccgccccgacctctactaccgcctcagcgccgtgtccgtgcgcctgccgccgctgcacgagcggggcgacgacgtggagctgctgttccgccacttcctggtcgccggcgccgcccgccaacgcatcacgccgccgccggtgacggcgcaggtgctggagcatctggccgagcacgactggcccggcaatgtacgggaactcgcgctctacgccgagcggcggcttctgggtctggacgccgaccacggcccggacatcggcgccgaccgccccctgcccgaacgggtggccgcctttgaagcgcgcgccatctcgacggctctgatccaggcggcgggcgatgcgacccaggcccagacgcgcctgggtctcccccgcaagaccttctacgacaagatcaagcgccacggcctcgacctcagggccttccgcggcaaggatcgggcgaaaacctagaggcggctgtcgaatacgaactgaagtgattcagccttcgaccaaaacacgcaccaaatcagacctctgccttccgggtgacgatcagaagtgattcgatctgccgacgatattgagtcagaaggcggctgcggacgacgattgtgattcagcttcagactctgtctgagcgcgccaggatcagggacttcgatcttcgatcttggaacccactcgttctccgggcgtcgagtgcccgcctagcaaggcggccgctttgcgccaggaccggtctttggcgaacagccgggaatcgggccttcaagcagaggcggcgcgaaggtcagctcacgacccgttgcgggaattgcgcgttcctctggcaggtccaatcgctccaaaggtcggtgcatagagacgtcggcgcgcctgctttttatccggcgtccgcgcgttcgcggacggggcgagttgtggtgtgggaacaatccgctcgcgggtccgttcggcttccggggaatagggccacatcacattgaccacacaacgagatggctccgacgatagccgataccgtctgctgatcgagtccatcaccgactacgcgatctacatgctggacccggcaggtcacgtgacaagctggaaccccggagcggagcgcttcaaggggtattcagccgaggaagtgctcggtgcccatttttcccagttctacacgccggaggatcgggaggccggccgtcccgagcgcgcccttgcggccgctgcccaggcgggccggttcgaggccgagggatggcggctgcggaaggacgggactcgattctgggcccacgtcgtgattgatccgatcaggcgtggcgcggaactcatcggctttgcgaagatcacccgcgacctgactgagcgtcgcgaagccgaactggctttgcggcagagccaggagcagttccggattctggtgggcggcgtcaccgactacgcgatctatatgcttgacccggacggcaaggtgatcagctggaacgcgggagccgaacgtatcaagggctatgcgcccgaagaaatcataggcgaccacttctcccgcttttacctacccgaggaggtggcggcgaacgctccagccaacgccctgggcatggcgcgagaagccggccgctttgaaaaggagggctggcgcgtccgtaaggacggcacccggttttgggcgcacgtcgtgattgatccgatcacgagcgacgacggcgacatcatcgggttcgccaagatcacgcgcgacataaccgagcgcgccaacgcgcaacgcgaactcgaggcggcgcgcgaggcgctctaccagtcgcagaagatggaagccatcggccagctgaccggaggcgtcgcccatgacttcaataacctgctggcagccgtcacgggcagtctggaccttctccgcaaacgccttccctatgatccccgaaccacgcccctgcttgagaacgccatccagggggccgagcggggcgccatcctgacccagcggatgctggctttcgcgcgcaaacaggatctcaagctcgaagccgtggacatcccgcaactcgtcagaggcatgagcgagtttattcggcggtccattggtccgaacattgatgtccggatgcgctttgccgatgtgttgccgaaggtgaagacagatccttaccagctcgaaaccgcgctgctcaatctcgtggtcaacgcccgcgacgcgctcccgactggaggtgaaatcacgatcacggcggaccaggtcaccgtgtcgaaggacagaggacaacgccgggcggggtcttttgtcaggctgcgagtgagcgacgatgggatcgggatgcccgcggagacggccgccaaggccatcgagccctttttcacgacgaagggcgtgggcaagggaaccgggctgggactttccatggtccaggggctggcagggcagtctggcggctggatcgaaatcgatagcgaggtcggcaagggcacgagcatcgacttgtggttgccagtggccagcgcggacgtccccaatgcggaggcaagcaaggccgaggcggtcgaagaacccggagagcggcttctcgtgctcgctgttgatgatgaccctctcgttctgaccaacaccgtcgccatgttggacgagctgggtcacaatgttctggtggcgaactcgggcgatgaggccctggtgattttcgagcgtcatcctgagatcgacctcgttctgaccgacgaagtcatgcccgggctctccggcagccaactggcggaacaggtcagaaagctccggcccacgacaaacgtagcggtggcttcaggctatgctgacctgaatttggcaccggaccctgctcaggccaagcttccgcggatagccaagccgttcaccctggctcagctcgccggcttcatcgatgacctcgctctgcaggagcccggcgagggcgggcagcgcaccgacagacacggaaggtgggtttgatcgaccgccttgtttaccggagccaggtcgagaacgttccgccggaggttacgctggagcgaatctttcggatttcggttcccaagaacgcccgcttgcagatcacaggagcgctggggttctctggacggaattacatccagctcctggagggcccacggcccgccctggacgaccttcttcagacgctccgggccgatccgcgccactcgaatctgcgggtcctgttgcggggatcatcgcaacgccaattgttgcccaactggtccatggcgcgggtcgatctcgcaagggccgcgcccaggttggacgcgctgctggaagccggcggcggtttgggcttagtgactttgatggccacgctcgcccacgaaggcgtgaccgcctaacgcgcttggcatccttgggcgactgtccgcctgacggtcgttcaggtgcacgacccagacctgctgggcgatcggattccagcgtgcagcgttgttgagaccctccgccagccaaggcctccagcggcgtccgcagcatggtggagtccggcgtctccttcggccggtaagcctttggccccgcctgtgcgcacaaccagtcgctgcggtagctgtgagcgtctatcacatgcattcggaacagctgcccgtaatccgaagcggcgatacatggttaaaccgttcggacgaggaactgcgccgcagcacgggcatggtctcccaccaggcctgcatggcggcgcaagcgcagcaggatggcctcgagtgacgcgccgtctttgcaggcgtctcccctgggtaccgcatgtcgccgcgaaacctcgccagaagttcacgcgtggcggcgccggcggcggcgatcacggcctttggcctgggcctgatcgcccgtgacggcctcctgatcctgatcgcctggatcgcgagcgtcctcgccctcgggctgctgggcttctggctgatcgcctaggctccgcgcccgaccgccacgcctgggcgcaccggtcggtggcggcgaggctccggccgacgcccggtccgcagcgtgctgctctattggctgaggcatcctcgtgaccgccgcgccgttgcggagacatccaacctgctcgtccggtcgggaacgctcgtgagaccctggtgttgaacttacaggtgccgactcgcgaatgcgaagcggccgcccggcgctccggtgcaccggcaggagagaggcgttgacgatggaagatttcctgggcggtcaacgtgatcggcggctcgatccggggctggcgttcgcccgggcgcagctccactcatcgcgcgccgaccgtcgcatcgatccgagacgacccgttcaggggcatgggccggccgtcgcgaaggcctagacgcgccaggcgccgccgcgatccgcccgcgccccgaacccgctcaacaaggagaccgccatggctgataaccgccccgtctatctgaaccttgcatcgaagactgaactcgacgccatcgacgaactcggcggccgcgctgaaaccgtgattgctcagcgcccgtacggcgactggtccgatctgcgccgcgcggggctgtcggatgaggagatcggccggctcaagagcgcaggattggagttgggtgcgcccggcgaaggaccgatcggcgaagccggcagcggcggcagcgccgacagcccaagcggcaatctgggccgcgcctgatggcgcgtcccggccgccgccaccgctagccggctcagctcatgctcagtggcgtgcacgccttcatccagcctttcgccgtggtgctcgaactgctcggcgccggcattatcgtcggcagcgtggttctcgccacgctcgcctttctgctgcggggtggacgtgatcgcgcctggcgggaagcttacgccaactaccgcgccaatctcggccgtggtatcctgctcggcctagaacttctcgtcggcgccgacatcatcagcaccatcaccgcgcccctgaccgtggagacggttggccttctcggtttggtcatcctcatccggaccttcctgagcttctccctggagaccgagattgaaggctgctggccctggcgacgggccgaactgctcgacgaccgcaagaccgatcagcgctgatcatcgaaaaggagggtgatatcgccattgcgctcaaggtaggcgcagcgaacccggccgaggtccccctggccgtgggcgcgcagcgccatggccaaatcgccgtcgccgatgccggcccgacgcatggcggcgcgatcgacgtcgccgttcttcaccagtcgaacgcgcgcccctttgaccaggaagctcagccaggaccagcgcgctgccgcgcgagctagcgcggcatgaacggcgaccagcgccagggtggccacgagggtggcgacgaagggcgcgcttcctgtcatcgcccgcccgagattggatccgacgatcacggcgaagatgatgtccagcgggctccatttgccgaatgcccgcgacgccgccacccgggcggccagcaccccgacggcgaaaatcagcagaccgcgcagcgtcatctgccaccagctgatcgccgcatcctcggagccgatcagggcgtgcagcgtctccataggtcagccggcgacgcgcggcagcgccgtcagtgagccgtctgtctcaaggaacacggcctcaagctgatcgaggccccggacgcccgcagcccgggcggcggcctcaatctcgccttctgtgatgcgctggcggcgcatggcgcgtgtcagcagccgcccgtcacggacgagcagcgtgggctcggccttgaccagcgcgttgaccgacttgaaccggaccgatgtcgccgtcaccacaaactgcatcgccaccagaagggcgagcgcggtcaaaccttccagcagggccagggacttgctggtgatgatggaggccagggtcgagccgatggcgatggtgatgatcaggtcgaaggcgttaagcttcgacagggttgatcttcccccgtaaaagtggacggggttaagccgctttgcgctcggcctcagcggggctgatatagcccagtgctgagtgcaggcgatggggattgtagaagccctcgatgtatccgaacaggtctcgccgcgcctggtctcgggtggcgtagacgcggtgatgaacgcgttcggtcttgagggtgtggaagaagctctccatcggggcattgtcccagcagtcgccctttcggctcatcgacggggtgatgccggatcgggccagggctgatcgataggcttcggctgcgtattggatgccccggtccgaatgatggatcaggccgggcgcggggcgctgacgttcgacggtcatgttgagggcgtcgagggcgatctcggtgtgcagggtctggcgcatggaccagcccacgatcttgcgggtgtgcaggtcgaggatggcggcgagatagagccagccttcgccggtcgggatgtaggtgaggtcggcgagccagacctggttgggcgccgccgcctcgaagttccgggccagcctgttgggcgcgatgggataaccgtggcggctgttcgtcgtccgggcgcgacgcggcaaggccgccaagccccgcaggccggcgcggcgcatcagccgctccacgcgggatcgaccgacccgacgcccatgccgccgcagggtggcgtgaacgcgcggcgagccgtaacagccgctgctctccgcatggatcagccggatatcctcggtcagctcgcgattggcgacagaccgctggctctcggggcgaccgcgccaggcgtagtaaccgctggccgacaagcccaggaccgcgcacatcacgcgaaccggccagacctgacgatgctcatcgacgaacccgaacttcatcgggaggccgctccgaagatgagcgcggctttttttaggatgtcccgctccatccgcagctgaccgttctctcgccgcaaccgggccacctccgccgccagatccgacggcgacggggacgacgcctgcgttgtggggcgccgcgacgcccccgtcgcctgcaccccgaactgcgtcatccatcgacgaagcaccgtctcgtgcagcccaagctcgcgggccaccgccccgacgctcaggccgccgttggcgacgcggtcaacggcctcgcgcttgaaagaatccggaaagttccggcgttgaacactcatcagacactcctctccagctccgaaaagctagcatgggtgtccaccaaaccgagggaggatcaaagcggatccagcggatctatcgcgaggagcgactgacggtccgtcgacgcggcggtcggaagcgcgccatcggcacccgaagaccgctggagctgccactggtggcgaaccagcgctggtcgctggacttcgtggccgaccagatgactgacgggcggcgcttcgctcgccattgtcctcggaccaatggcggacacggctcgccctgacggtgatcgacaactgcacgcgtgaatgcctggcgctggtggccgacacctcgctgtcgggcgcgcgggtcgtgcgggagttggacgccgtcatccggcagcggggccggcccgacaccatcgtcagcgacaacgggacggaatacacctcgaacgcggtcctggcctgggccgacagcaccggcgtcggctggcattacatcgcgcccggcaagccccagcagaacggcttcaacgagagcttcaacggacgcctgcgcgacgagctgctgaacgagacgctgttccgatccctgccgcacgcccgcgcagtgctcgaagcttggcggcgcgattacaacgaacggcgtccgcactcgaagctcgggtggctgacgccgcaggcctatgcagaagcgctcaccggacagatcggccggtccgctgcgctggttgggggctgcgctgaccggcctcttgccaaccccgacaaccccagctcagatcaccaaaggactcttgtgtggacgacctccaagacgcaagagtggaaacgacgttggcgctcggtcgagtgcagtcatgtgttcggcctgttgatgcagctgtttgcgctgctggccctgatgaagtccgcggaccggctccctaatcacgtcaacgcgctcgaggcgctctgaccccctgggtttcaccgatccccggctgcggccggttcgtcatcacgtctcaccactccttcgtctacggcgccggtcctgggtgaagaccggcccgatctctatgccgctgtgggcttgtagtcctcctgtcgcgccatcagggtccaggcgatgcgagccgtcttattggccaaggccacggcggcgaccttcggcttcttgcgttcgaggagattgccgacccagccctcgcgtcctcgctgccgggccattcgcaggaccgccgtggccccgacgaccaggagacgtcgaaggtagctgtcacccatcttgctgatgccgccctggcgttccttgccgccactgctattggcccgcggcgtgagtcccagccaggctgcaaactgccgaccggaacggaagagactcggatctggcgcgctggccgccatggcgctggcagtgatcggcccgatgcctgggatggtcgccagtcgccggctcgtctcatcctgccgatgccaatcgagaatccgacgctccatacggctgatctctgcgccaaggtgttcgagctgttctgccagcccgccaagcgcggcatgcgccagatccggcagggcctgaccctcttcacgcagactcttcagcgctgcccgcaccccagctggaccttgaggcgcgacgatgccgaactccccgaggtggccccgcagtgcgttgatcagcatcgttcgctgacgaaccaggagatcccgggtcttgtgcagcatcaacaccgcctgctgggccttcgacttcacagccacgaaccgcatggtcggccgggtgacagcctcggcaatcgcttcagcgtcggcggcgtcggtcttgccgcgcttcacataggccttcacgtacgccggcggcatgagccgaacatcgtggccgatcgccatcagttcacgcgcccagtggtgggctgaggcgcacgcctcgatcccgatcaggcacggcccaatcgactggaagaaggccagcacctggccgcgccgcagttgccgtctcacgacgaccgtgccgtctgtggctacaccgtgaacctggaaaacagtcttcgccagatcgagcccgacgacagcgatggtctgcatgataccgctcctagacgtgacgtccctgatgacgacacacccagaacagcccgtcaggcggaggtcgtccacaccatcacgtcaggagcgctgctgatgcagcgcgactgggtctatcaacacacaggttgtctgcgtcacagtcggcggtttgcgaacacgccgggcggcattgcggtgatcgtccaagacgcggtcgccatccggttgtcgaaggatcaggacgaaccgctaatgctcggcgccggccgcacgctcttctcacagcaggtgaaacgcctgggcgacgccatgcagtgtcacctgttcggctccatctacgacagcgacctgcgactcagcgtagcgctgctggtgcgcctgtccggcaatgccgccctggaagcctccagcgatgcgcagcgagaacggcaggtggatgcctggctggacacgcataccgccattgccctgggtcgtctgccgcccagcataatggcgaaggacgtggatgcgccgctcaacacgctgtggaggctgagggataggacgccgctctaggtattcagtcccggcatccgaattgtatgcctctatgacgtagtagggtcaccttgaccaccgccatcgacgtccaagtcgccgaaagcccctgctggcgggggcggtgaatcattgttgatcgtctttgaatcgattcacttcgtcatcgacagcggcgcggaaagtggagcgggcgatgggaatcgaacccacgacattcagcttgggaagctgacgttctacctctgaactacgcccgcgcgcgacggtgaccatagacggggacgggcaaaagaaaaggcccggcggagagccgggccttgatgcggtgtcgggcgatcagccggcgggacggacgtccacgcctctggcctcaagcatcgactgcacgctgtcggcgcccgccaggtgagccgcacccaccacgatgaaggcggtgcccgatcccttcagcagggtctcgatctgaccggcccagttggcgttgcggcggaccagcagggcgtcataggcggcgggcgcatccgtcttcatctccttcacgacgatgcgatcgagttcatcgacgtcgccgccggaccaggccgtcaccatgccgtcgagcagggtcaccgcctcgtcgaaatcctccagcgtcgcacgcaggaagtcgacctggtcggcttccggcaggccggccaggatgcggacctgctcgtcgatggtctcaaagccgtggatcggcttgccggccgcctcggcgcggctcttcaggatcagctcgacgcccgactgggggtcatagcccgccttggtcagcggcgcgacggacagggtcaggccggccagccacgggcgcatggggtccagctgggcgcccgtcgcgcccagcgtcttggccgccgcgtccagatcggcgaactcctctgcggtcagcaggctggagagcggcgtctggggcgacaggccgtgctgctggatcagcggcacgatggcggcctgatcgtcggggttgctgatctccatccacacgtcggacgaggcctcgaaggcggccttgatgcggggcgtctcccaggcggtggtcggacgcagaacgtgcaccgagccgaacaggtagagggtggagtcctcgtcgcggaccacccacagggcgggaccgtcgccctcgatgggggcggcttgcacggccggtgcgatcggcgcctgggcgaaggcgggcttgggtatggcgaacagagcgctgaagacggccatggagaggatggcggaggcgccggcgcggctgacgttgcgggcggcggaggcgaaaaaggcgtgggtgttcatgtcgcggatcctttggataggcggttcacgggtttgcttgtcggcgagtgatggacgcggaggctctaggccgcttcgtccaggaagatggactggatcggttgttcgaaaacgcgggcgatcttgaaggccagcggcagggaggggtcgtagcggccggtctccagcgcgttcacggtctggcgggagacgccgagctggtcggcgaggaaggcctggctccagtcgcgttcggcacggagcaccttgaggcggttgttcatgagcatctcctcaccgccgcgccaaccaccaccaggcccacgccagcgtgtagcccagcagcatcagccccagcatcatcatggccccggcggccgcataggccgcgggcgtggggtcgcccagggtcggtatgcgaatggttgcggcctgcggcaggcgcgacaggatcacgccgacgccgcccacgcacatcccggcgcagccgccccagtaccaggccgacttgtgcgcctcgcgcgccgcctcgtcgatgctgcgcatccacagggcgccgacccagagcgcgccggccatcaggatgacggtgaccgcgctcatggcgaccagcagcgtcaggtcgacgtccaggccgccgctgacgccggcgacgcttagtacgacgcccgccaccagggcggcgacgatgagcagaaagaacgccccaatgggcttgatcagatttctaagtgaactcggcatgacaaccctccttgccgttatgacaaggatgcttgtctcacacacgcagcaggatgtcaagcgtgcttgccacaaggacaagcacgctgttcattccccgatcaggcgtcttcgccgtccacgtccagcgccagcaagtcggacgccagcgccggccgggcgccgccagtcaggcccgtggtctccacgcccttgagcttgcgggtcaccgcccggtggcgcacgcccacgtcgcggaccttgttcttggcctcgtccagcttcttgtcgacggcgtccagcgccgagccgtagtcctcgaacgccttcttggcctcgcccagcacctgggcgatgtcgccggcgttcttctggatggccagggtctggaagcccatcttcaggctgttcagcgtggcggccagggtggtcggccccgtgaccgtgaccgagaactcggccgacagggcgccggccaggcctggccggcggatgacctcggcgaacagcccctcggtcggcaggtacatgatggcgaagggcgtcgtctcgggcggatggacgtatttgtcgcggatgctcttggcctggatgcgcagcgcccgctccagccccttggcggccgtttcgacggcgaccggatcgccggcgtcctgcgccgtcagcagccggtcgtagtcctcgtgcgggaacttgcagtccagcggcaggatcagccgctttccttcggtcgagccgggcagatagacggcatagtccaccacctcgcggctgtcgtcgcgcacccgcacctgccgcccgaactgctcaggcgtcagcatgtcgtccaatagggcgcccagctggacctcgccccaggagcctcgggccttgatgttggacagggtgcgcttcaggtcgccgacgcccgtcgccagcgtctgcatttcgcccaggccccggtgcaccgtgtccagccgctcggagaccagcttgaagttctcgcccagccgctcggccagcgttccctgcagtttttcgtccacggtgacgcgcatctgctccagcttggcctcgttctccttgcgcagggtctcgaggttgccggagaccacggtgcggaccttctccagctcctcgcccatggccttgcggccttcgacctgctgctggctcagcgtctcgaccagccggtccacggcggccttggtctcgttcaggcgctggcgctggctctcggccagatcgtcgccggacttcttctgcaactccgcaaaggcctgaaggcgggtgtcgaagttcgtcgtcagggcgccgatgcgccggtcaaggctgtcggacaggccgttcagcgcttgggacagctccagccgctgggtcgcggccttggcgtcgaactcgccgcgcagcgcggccatctcgcgggccagcgccacggaggcgcggtcatcctggcccgccgcttcggcgatgcgggtggcgcgctgggcggacagggcggcccacgccgcgcaggcggccgcggccacggacgccagaagaacaaggatcatgaaggggtcgatcggcatggaggctccgacaggggatcaggcgaacgccacgatcgccgccgcctgcgacgaagacggtcgcatcgcgcgacgttcaccgtccgttcctaaagggagtcgcccgcctcgaacagccttcaggccggacgacgcgcacgcagggcctgcacgatggtgccgtcgtccagccagtccagatcgccccccaccggcacgccgcgcgccagcgacgtgacctggacctcgtcgcccgcgatccgctcggcgacatagtgggcggtggtctggccatcgacggtggccggcagggccagcaccacctcgcgcacgcccccgcccctcacccgtccgaccagttcggcgatgcgcagatgctcgggccccacgccgtccagcgccgacagcaggccgcccagcacatggtacttgccgcgaaacgcgcccgagcgctccatggcccacagggcgccggcctcctcgaccacgcagatcaggccgttgtcccgcgccccgtccgcgcagatggcgcacgggtcgcgcgtgtccggcgcgccgcagaccgagcaggacaccacgcgctcggccgtttcggccatggcggcggctaaagggaccagcaactgctcgcgccgcttcagcaacgccagcgccgcacgccgcgccgagcggggccccagccccggcagcttggcgagaagggagatgagccgctcgatctccggcccggcggatgcggccatcagaagagcttgggcatgcccgggatgttcatccccgccatcggccccgccgcctcgcgcatcagggcggagttggcctcgtccagcttgcgccgcgcatcggcgtgtgcggcggtgatcaggtcggccaggatctcgccttcgcccggcttcagcaggctgtcgtcgatcaggaccgaggtgatctcgccggggcccttcagcgcgatggtcaccagtccgccgccggacgtgccctgcgcggtcgtttccgccatcttcgcctgggcgtcctgcagcttttgctgcatcgcctgggcctgctgcatcagttgggtgaggtctttcatgcgccgatagataatgcgggtggcggcgtcgcgacaggggcgcccgacggggcggcctcagtcatcgtcgtcgtcggccgcgtccgggatttccggcgtcaccaccgtcggcgcgactgtgcggatctcgcccagcttggcgccgggaaaggcctcaaggatggccttgacaaaggggtcggcctcaacctcggcgcgctcggccaggcgcgcctttttctgctgctcaatcagggtctcgccgccgccctggccgttggcgaccacgaaccagggacgaccggtccactcgcgcaggcgggcgttcaggcgggtggcgagattggcgggcgcgccttcgaccggctcgaaggtgatgcggccgggctggaactccaccggtcggacgaaccgctcgacatccatctgcaggccgatctcgcgcctttcgccgatcagggcgacgacctgctcgaaggtctgcggattgggcagggcgggctgaaccacggggcgcggcgccagttgcgccgatgcgccgccgccgccgcctccgccgcctctcggcacgccgccggagccgccgccggagcccccacccagaggctcgcccgactgcagccgcttcagcgcttcttccggtcccggcaggtcggcggcgtaggccaggcggacgatggccatctccaccgcatccgacggattgggcgcgcgccgcacctcgtccagcgctttgagcagcatctgccaggtccgcgacagtgtccccgccggaatggccgcgcccagcgccgccagcttctgcgcctgatcgttgggcagccgtgtcgcctgcggccccagcattttggcgaccgacgcggcatggcaatgctccagcaggtcgttggtcacctgcacggggtcggccccgtagccgtagagggtgcgaaagctctccagcgcctcgggggtgcggccggccatgatcgattcgaacagggcgatggtctggctgcggtcggccagacccagcatgtcgcgcacggtcgcggcctgcaccgtctgcccccgctcgccctgcaccagcgcctgatccagcaaagacaagccgtcgcgcaccgacccctcggccgcgcgtgcgataagggccagcgcctcgctctcgatccgcatgccctcgcggtccgccacccgccccagatgctccaccagcacctcaggctcgacgcggcgcaggtcgaaacgctggcagcgcgacaggatggtgaccggcaccttgcgaatctcggtggtggcgaagatgaacttggcgtgcggcggcggctcttccagcgtcttcaacagggcgttgaaggcctggttcgacagcatgtgcacttcgtcgagcacatagaccttgtagcgcgcctcgaccggcgcgtagcggacgctttccaggatgtcgcggatgtcgcccacgcccgtgtgcgaggcggcgtccatctccatcacgtccatgtgctggccggccatgatcgcggcgtcgtgccggccgcctggcgtcagctcaagcgacggcttgctgatgacgtccgtctcgttgttcagcgcgcgggccagcagacgcgcggtggtggtcttgcccaccccccgcacgccggtcagcatgaaggcgtgcgcgatgcggccggtggcgaaggcgttggtcagggtcctgaccatggcctcctgcccgatcaggtcctcgaaggtgcgcggccggtatttgcgggccagcacctgataggcggcgtcggatgccggctcgggcggggcgacaggcgagggcgtaggcgcagcagcaacgacgggcgcaggcgcaggcggagcgccgaacatgtcgtccgtgttctggtcgcgctcgacgacgtcctcgtcccagggagggccgtcgagactcgggtcgatgtcgctcatggccgtgtcttagaccaccgccgccccggacggcagatggaatctcagccgtagagatcgcccagatagacgcggcgcacctcaggatcgtgcaccacctcgtcggccgtgccctcgaacagcaccgagccggccgagatgatcgaggcgcggtcgatgatgtccagcgtttcgcgcacattgtggtcggtgatcagcacgccgatcccctcgcccgccagatagcggatcaccgtgcggatgtcggcgatcgccagaggatcgatgccggcgaagggctcgtccagcagcatgaacgacggccggcccgccagggcgcgagcgatctcgacccgcctgcgttctccgccggacaggccggtggccggcgcgtgacgcagatggtcgatccgcagctcctccagcaggcgcgcggtttcggtttcgatcgccttgtcgcccttgtggtgcagttcgaccaccgcgcggacattctgctccaccgtcatgccgcggaagatcgaggcttcctgcgccagatagcccaggcccatgcgggcgcgctggtacatcggctgggcggtgatgtcctgaccatccaggtggatggtgccgctgtccggcgggatcaggccggtgatcatgtagaagcaggtggtcttgcccgcgccgttcgggcccagcaggcccgccacctcgccgcgctgcaccgtcagggacacgtcgcgcaccacctggcgctggccgaaggcgcgcgcgatgctgcgcaccctcaggcctcgaggcggcggcgcaggcgcgggctcgaccgccggctcagggaccgcgcggtcgtccaggttcagggctgacagttccttgcgggccaagcgcgatccggaccgaacccgaggggctcagttggtcccttcgggatagaagacgccctggacccgacggccggccgcgccgcgcggcgcgccctccatgcgggcggcctcggtgttgacgttgtagaccagccggccgccggtcagcacgttctggccttgggtcaggatcacgtcgcccgtcaccaccacctcgcccgtgtcgggcgtatagaccgcgcgatccccgcgcatggattgctcaggcgtcaccagatagaccgtgccgctcgcctccacccgctgcaggtcgcctccggacgaacgcgtcagcgtcatggcgtcggcgcgaaggcggttgccgccctgcacgacctcggcccgaccgcgcaggctggcgcccgtggtcgtgtactcgccttcatccgccccgaaggcgatcggctggcgagaggcgcccgactgggcgtcgccggtggtcggcagagccaggagcgccagagcggccgtcgccgccatcgccttgattgtcgtcgccatcctcaactctccgagcctgaggggttgatgacgcccctcaccttgttgtcgcccgcgccctggaagacgacgcgttcgccctgatcatggatcgcataggacgaagcgttgatcgttccaagggggccggtcccctgcacgccctttgagcccgtcaccacgccggtgcgggtgtcgactacggcctcgggcgtggtcagcgtaaagcccgagccgccgtccgagatgcgcacgttcgggccgatgatgaccttgcgctgcgcctcgtcataggtgccgccgtcggcggtcatctgagtcaccttgcggccgccgaggttcagccgcagcaccggcccgaccaggcggaaatggccggtgtccggatcgcgaatcgcgccctgcgcccccaccaggaaggcgcggccctgcgcgtcctggccgtggaacatgggattttcgaggcggatctcctggctctggctcgcccgtcgctcgacgccggacatgaccgtgcggaacacggtccaggtcagggccgagcccgccaccaccaggatcagcaccggcagcacgcggcgatagaagcggatgcggcgcgagcgcgcgcgccagcgatcgccctcgcgggcgacccgcgcctcgtccgcctcgatgctgcgccgctccgcctcgctcatgggatcagctgtgggcgaacacatcgatctcgtcccagccggcgagatcgagcgccgaacgggtcggcaggaagtcgaagcatttgcgcgcaagctcggtgcggccctcgcgctccagcatggcgtccagccgcgcctttaccgcatgcaggtgcagcacgtcggaggcggcgtagtccagctgcgcctgggtcagggtctcggcgccccagtccgacgactgctgcgccttggacagatccacgcccgccagctcgcgcaccacgtccttcagcccatgccggtcggtataggtgcgcgccagcttggagccgatcttggtgcaatagaccggccgcgtctcgaccccgagatgcagctggaacatgccgatgtcgaaccggccgaagtgaaagatcttcagcacgcccggatcggccagcagccgcttcaggttcggacaatcgtagtccggccgacgcaggcgcacgacgtgggcgtttccgtcgcccgaggacagctgcaccacgcacagcggatcgcggcggaagcgcaggcccatggtctcggagtcgatcgcgacctccggcccaaggtccaggtcgtcgggcaggtcgccttcgtgcagggtaacggtcatcgcgcgatcatatatgagcgggacggttctggcgaaaccgcgccggaaacaacaacggcgccgcacccgaggatgcgacgccgtctgaaagatggtgcccagaagaggactcgaacctccacggccgttaagccactggcacctgaagccagcgcgtctaccaattccgccatctgggccccgtcggcgtcgccttgcggcgtcgtcatcgggaaggcgcggacctctaaggcaggccgcagggcgggtcaacagggcgacgccgcaaaaagcgtcatctttttcccccgcgccgttaacgctgtgcgcttacccggtcttgagccgcgcggggctattcccgaggcgatgaccaagcccgtcgccctgcccacccgcgagcgccgcaccgcgccccgccggccgttccgcaaggaacgccgcgagggcgaacgcgtccgcatcctgggccagcccatggatctggtccgccccgaggaggtgctgcaccacgtccagaacgccgtcgcggccgggcgcaggacagtggtggcgaaccataatctgcacagcctctatctgctgcagaagcatccggagatcgctcgcttttatgagcgcgccgatctggtcgaggtcgattcgacgccgctgatctggttctcgcgcgcgctgggcctgcacagccggccgtttcaccgctgcacctatctggactggcgcgatcatttctggagcctggccgaccgcctgggctggcgcgtcatggcgatcggcggcgccccgcacgtgggcccggccgcccaggcgaagctgtcgctggcctatccccgcgccgacatccgcaccctgtccggctatttcgacgctcggcccaacgcggccgagaacgcccgggtgctggccgaggtggagcggtttcagccgcacatcctgtttgtcggcatgggcatgccccgacaggagcgctggatcgccgagaacctggatcgcctgcccgattgcgccatcctgtcggtcggcgccgccttcgactacgaagccggcgttcagagcgctgcgccccggtggatgggccgggccgggctggaatggctgtatcgcctcctgcaggatcccaagcgactgttccatcgctactgcgtcgagccgtggagcctcctgccgctgatctgggccgacatccgccaggcgcggctccggcgtcagtccgcccgcggctgagcaaaggcgacgtagtcggcgtagtcgtagtcgatgtcgccatagccgtgccgcgcctgggcgttcatgtcgacctgcgtcagcaccacgcccaccgccgccgcgcccgaatgctccagcatcctgagcgcgctcgccgccacccgatcgggcgtgcgccgccagcgcgccaagaggaccgccgcatccgcccgcgccgccaggaccctggcctcgctggtcgccagcagcggcggcgtgtccaggatcaccaggtcgaaggtctcgcgaagccgcgccgtcaccgcctccatctcggccccgcccagcacgtcgcgcgacgtcgcgccgccccgcgccagcggcaggacccaggcgcccgatccctcgtccagccgaagcgccgcctccagcgtcgccgatccctccagcacctccagcagtcccaggtccggctcgatccgcagcatgcgcgcgaccgcacgcctgcgcagatcgcagtcgaccagcacgacccgtccgccggccagggccgagatgcgcgccaggctcagcgcggtggtggacttgccctcgtcgggcagggccgagcatagggcgaccacctgaaccttgcgccccggcctcgaatgcaggatggccgcgcgcatcgtccgaaacgcctcggcgaaaggcgacaacggccgtttcagcacatagtcggcgggcgccaggccccggtccgccttttccgccaccgagcgcagcagcggcgcctggcccaggctcggcttgcccaaccgctgctccacgtcctccgcatgccgcaggccgcgatccagcatctcggacagccccaccgccgccagagccagcatcagggccgccacgagcccgcccgccagcagcagcggcgtgttcggcgacgagggctcggacggcgtgcgggcgcgcgagacgatgcgggcgtccgactgctcggcgccctcggcggcgctggtctcctgaaagcgggccaggaagctctggtagagggtccgcaccgagtcggcgtgacgctcaagctcgttcaggcggacgcccgcggcgttgtcgaccgccagggtgcggcgcgcctcagccaggctggcgtccaccgcccccgcccgatcctgcgcgacctgcacccgggcctccaggttggagacgatgcggcgaatctccgcctcgatctgttcgtcggcgtccgacagttcgcgtcgcgcccgcaccatgtccggatggcgctcgccgtagcggctggacagctcggccacgcgggcggaggcttcggcccggcgggcgcgcagctgctggaccacctgcgactgcagcgcctcgcccacgtcctcgccgctggacccgcgcgccagctgggtccgtgcggtacgcagccgcgccgcctcctcggccagctggctgcgggccgtggcgcgctgctgattgtaggcggagatttcctgttcggtcagggttgctccctcggcgctgagcaggccgttgtccgcgcggtaacgctccaccgcgccctccgccgcctcgagttcgacgcgcagggccgtcagccgctcggtcagccagctgttggcgtggcgcgtcgcgtcgcctttggtctcccgctgctgcagcaggtactggtctgcgaaggcgttggcgatccgcgcggccttggccggatcgcgcgactcgaacgcgacctgcatgacgtaggtcccgcccatgcgtgcgatgcggagcctttccagcaccgcgtcgatcacctgctccctacgggcctgcggatcgaccaaggtcgcgcgcctgtccgcatcgcccagccatggcggggacgccgaggctgcgaactccggatcgtggatcaggccaacggcgtcgacgacccgttcggccagctggcgcgacctcaggatttcgacctcggtgtcgaccacggccgcttcggcggtcagcccggacagcacggcttccgcatccaccacccgcgccctgcgcgtgtcgatcgtcaggctggcggccgccgtatacagcgtcggctgcatcccgatcgccgccatcgtcgccaccacggccagcaggaacacggcgcccgccagccacaagcggcgacgcacgacgccgatcagccgatgcgggtccacgccctccccgatcgcgccgcgccagcccgccggcgcttccgaccttgcgtccatccttctccccccaagcccaccggtcagaaccgggcgaccagcgcccccgccagtcgagcgacctcgaaccccgttcccgccgcccgccctcgcgacgaccgcgactcacggctggccgtcaggctgacgccgtagcgtcggttgatcagataaacggcttcaactgcggctgtgaaccgccgatcttcccgatccacgtcgttgaaggcctggccgcgccatcccaggcgcgcgctcaggatcaggtttcgcagcagttcatgatccaacgccacgcccacacggcgggtcagcgcgccggccgcgccgacccgctcggcctcctccaccacttggtcgccggtcagggtgacggtggtcagcggcgtcgggaaccactccacacgggcgctggcgaccagaccctcgatgtcgctcacgccgggatggtcgaaggcctgacgcacatgacccgccgcgacctgcgcgcggaccagcgccccgagttcgaaatccaccccgaccagagcctcgacgccggccgagtcgcgcccctctgcgcgccggtagtctcgccggttcgtcgcggcctgcacaaacagggcgagcgcgggcgtcaccgcatagtccgcccgcgcgctgaggcgcgacaccgcccggtcgcggtgatcctgatcgatctcgtcgcccgcttccgtctcgccgtcgtggaagtcgaacgtgcgatgctcggcgcgcagggtggtgcggaaacggccgacgacgcggcgagccgccagatccagctcgcgcgcctcgacccggatgggctcggcgctgacgtccggcgcgtccaccgccccgcgcggttcgacccgccgcgacagccgggcgccgaagtccacatccatatcgcgcgtcaggtccagacggcccgaaacatccagcagaccttcagtgctgtcctcgcggccctccgacgcatggcggcgcgccacgccttcccccgtgacgctcaccgcgtgccgcgaccatgcggaccgcagcgacgcgccggccgagaggcgcatcagggtgtcggcgacgggactgtcgggcgcggcgtacaggttgtcgacgaactcggtcgcggcctccacccggggatgaaggacgaagccgcccaggcgcgcccccacaggctgataggccggctgcggacggtcacgcacggccaacccccgatcgcgcgcgaacaggtccgagcggccgccggactgcgccgccgcggccgtcgcctccattgcgagcagaaccgtcgccacggcgagcagcccgttccttgcccccattccgcccgcccccgccggcctgcagcgtcgcaccttggctggcgcgcgcgacccggattatggtgcactaacggtcggggggctcaagatgaaaacgcaatcgccggctgcatggatgatcgctctgatccttgcggtcggcgcagcagcggcggctccggcgctggccgcgccgccgcaggccgagcgcatcgtttccgcgtaccgtctcggctcgggcgaccgcgtccgcgtcaccgtcttcggcgaagaggcgctgggcgggacgttcgtggtggacggggcgggcgcggcctccctgccgctcatcggcgaggtgcgggcgggcgggctgacggtggccgagttccgggacgccgtcaccgcggccctgcgcgacggctatctgcacgagccccgcgtctcggccgaggtggtgaaccaccgccccttctacatcctgggcgaggtcaaccggccgggcgagtacccctatgcggcgggcctgacggtgatgaacgccgccgccaccgccggcggcttcacctaccgcgccaacacccgccgggtgttcatcaagcgcgcggacgacaccgcagagcaggcgcaccccctgaccggctccacgccggtcgcgccgggcgacacgctgcgcatcggcgaacgctacttctgacgccatggccggcgttcggttaaccgcgattaaagggcttgtcgccaagggtttcccgcgatgtccggggccccgcacagcaagagcctgctgaagacgaccgtggccgccgccgcggccggcgcggtcgcgcttgcgcccctgtccccgtccctggcgcaggaaggccggggcggcggcgcccccctgtcggtcgaaatcggccgcaacgacgccttcacccgcatcgagttcggcggcgtcatcggcgggcgctcgcaggtgcgccgcgagggcgagcgggtcgtggtgcggatgggaaccaccgccgcgccccatgtctcgcgcctccgggtcgatccgcccgaaggcgtgaaggcggccgagacccgcgcggtgcgcggcggcaccgaactggtcatcaccctggcggagggcgcggaggcccgttcgggtgtggccgacggcgcggtgtggctgaacctttatgcgcccggcaaggcgccggagagcgagcagcagcccgccaggccggcggtccaggcggtggtgccggtgcgcgccgtcagctcgccggacgagacggtgctgtcgttcggctggagcgcgcccgtcggggcggccgtgttccggcgcggcgaggcggtgtggatcgtgttcgacgccgccgcgaagatggacttggccggcgccaaggacctgggcccggcccgggacgcgcggtgggccgccggacccgactactccgtgattaggatcgccgcgcccgaaggtctggcggtgacggcccaaggcgaaggcggactatggacggtgaccatcggcggctcgcccgctggcacctcgggcgtcgaggtggggcgctcggatgatggatcggcgacgctggtcgcgcgcgtggccggggccaccaaggcggtgtggctgaccgacccgctggtcggcgaccgcttcgccgccgtcactgcgctcgcgcccggcaagggcctgtccgaggcgcgccggaccgtggacctgtcgctgatcccgaccgcgcaaggtctggccgtcgagacctccaccgacgaccttcaggtcgaggccgccggcgacctggtgaccctgagccgccccgagggtctgatgctgtcgtccccctcggcggtgctggaggcgggcgaccacgcggccgacgcgccaaggaaggccgaccatcccggtctgatcctcaccgaatggtccgaactgggcgaagaggacttcaccgcccgccatcgccggctgcaggacgcggcaagcgccgagaccatggcggccaaggacgatccgcgcgcgcctatagaggcgcgcatggcctacgcccggtttctggtcggatcgggcctgaactacgaggccgtgggcgtgctgaacgccctggtcgcgcagacgccgaacatgctgggcgagccggaggtgcgcggcctgcgcggcgcggcgcgcgccgccgtgggtcgactggaggaggcgcaaagcgacttttccggcgcggcgctggccgccgatccggcgaccaaggtctggctgggctacatcaccgccaaccagggcgactgggccggcgcgcgcgcggcgttcgcggcgggcgcctcggtgatcgacgactttcccaaggcatggcgcgcccgcttcggcgccgcccacgccctggccgccatcgagaccggcgatctggacgccgcgcgacagcttctggcctacagcttcagccagcaggcgcccgccgccgaccagttgaccgcgcgcctggtgcaggcccggctgttcgacctttccggggataaggaccgggcgctggcggtctacaaggcggtggcgcgcgcgccgcttgaagggatcgccacccccgccaagctgggcgtgatcgggctggagctcgacaagggcgccctgcccgccaacgaagccgcgacccagctggagcagctgaagtggcgctggcgcggcgatgcgaccgaactggccgtgatccgcaagctggccgacatctatctgcgccagggccgctaccgcgaggcgctggacgcgctgcgcagcgccggcaagcggatggcgcgcatccctggcgcatccgacatactggcggaccaatccaacgccttccgcgccctgttcctggacggcgcggccgacggactgcagccggtgcaggcgttggcgctgttctacgacttccgcgagctgacgccggtcggcgccgacggcgacgagatggtgcgtcgtctcgcgcgtcgcctgatcgacgtggacctgctggaccaggcggccgagctgctgaagcaccaggtggacgcacggctggagggcgtggccaaggcgcaggtcgcgaccgacctcgccaccatctatctgatggaccgccagccggagaaggcgctgcaggccatctggtcctcgcgcacgaccctgttgcccagcgccatgaacgccgagcgccgtgcgctggaggcgcgcgccctgatggacctgggccgcttcgaccacgcgctggaggtgctggacaaggatcagagcgcgcccgcccgcgaggtccgcgccgacatcctgtggaagcagcagaaatgggcggacgccgcggccctctacgaggcgcgcctcggcgatcggttcagcgaccccacgccgctgaagccggtggaagaaagctggctgatccgcgcgggcgtgggctattcgctgggcggaaaccgcgctgcgctgcaacggctgcacggccagtattcgcccttcatcgccaaggcccgctcggccaacgccatccgcgtggcgctggacgacagcctgtcgggtgtggcgggcgccggcgactttgcgggcctggcgggcggcgcggacacattcgtcggctgggtcggcgcgatgaaggacgacttccgaaaggaaacgggcggggcctgagaaggcgcccgcccgtcgaaaagcacgcacaatccgcaacagcggaccggatcggccttagccgttgacggcgtccttcagcggcttggagacgcggaagcgcacggccttggaggcggcgatcttgatcgtctggccggtggccgggttgcggccttcgcgctcggcgcggtcggcggtgtcaaagacgcccaggttcgagatgcggacgtctccgccttccttcaggctcttgtggatgttctcgacgatcgaggtcagcaccttgccggcgtcgccttgcgacacaccggtgtccttggcgacggcggcgatcagttcggcttgagtggtcatgaggatttatccattgcagtcgcccccacggggcgagacctgccgatcaacacggaaaagcgtcgccttggcaagtccggatcgggcgcaaacccttgcggggcggggctcagccgcctccggccgccctctggaagctctccaccaggctgcccgcgaccagccgccagccgtccaccagcacaaaaaatatcagcttgaacggcagcgacaccaccacgggcggcagcatcatcatgcccatggacatcagcacgctggcgaccaccagatcgatcacaagaaacggaatgaacaggagaaatccgatcgaaaaggcctgcttcaactccgagatcatgaaggccggggtgaccacccgcagcggcagctcctgcacgttggccggggcctccacctggctcaggcgggtgaacagggccaggtccgcccggtccacctgacccagcatgaaggtcttcaccggctctgacgccgcatcgaacgcctggggcagttccatctgctggtccagcaacgggcggatgcccgaatcataggcgtcctgccacgtcggagccatgacgatggccgacaggaacagcgccagcgacaccagaaccgcgttcggcggagactgctgcatgcccagcgcggtccgcagcagcgacagcaccaccacgatccgcacgaagctggtggtcatgatgacaatggacggcgccagcgacagcacggtcatcagcccgaccagctgcaccacacgctgggtcaggccggagccggtgcccaggtctatgttgatcgccgatccgctctgcgccgcctcctgcgccaacgcccccagcggccaagccaggcacaccagcgtcgtgagcagcgacagaagcgccgcacgcttcagctcggcgcccgtgggccgaacgaacagggcgggcttcacttgccgccgccgatctggccgccgccgacctggccgccgccgatctggcgcggctcgatcagctcgcgcccctcgcccagcaggatcagtcgttcctcgtcgtccacccgcaccagaaccagccggcgggcgggatccagcaccagggtctcgaccacctgcaggcgccgctcgccgcgctggacctgcagccgggccagcaactgcggcgcatagcggcgcgccgcccaggccgccaggccgatgatgccgagggtgaaggccaggccgaacacggcgcgggcgagatcaaggaagttcatcggacgtgtcgtggaccgtcgcgcacccgcgcgtcgccccacactgttaaccagcagggttaacgagccgttgagataaccccccgttaaccaggcaggcggcattttctgcctatcgggcgcggccgtcgcgctcatcggaggccgtcatgggcgtcgccgacctgccgctgctgcaacagatcaagggccggctcggctggctggacgagcgtcagcgcgtgatcgcccagaacgtcgccaacgccgacacgcccggttacggcgcccaagacctgaaggcgccgaccgacttcgccgctgcgctgcgcaccggcggagggttgcggatggcgcgcaccaacgccgcccatatcgcgcccgccggcgccagcctgcgctacgatccgaccaaggccccggactcggagaccaccatggacggcaactcggtggtgatggaggagcagatgctgaagatggccgagagccgcatggcctacgacgccgccatcggcttctaccagaagtcgatgagcatgatccgcctggccgccaagaagcccggcgcgtgagctgagaaagccctgaaccatgcccgatcccctcacgccccggaacaacgccatggcggtcgccgccagcgcgctgaaggcccagcagtcgcgcatgcgcgtgatcgccgagaacatcgccaacgcccagtccaccgccgatgcgccggggggccaggcctatcgccgccaggtgccggtgttccaggcgcgcgagatggacggcatgaccggcgtgacgctggctcaagtccggccggaccagagcgagttcaagaaggactatgacccgacccacccggccgccgatgcgcagggctatgtgctgcggcccaacgtcgacaccctggtcgaggccatggacatgcgcgaggcccagcgcgcctacgaggccaatctgaacgtgatcgagacggcgcggaccatggaaagccgcaccctcgatctcatcaagcgctgaccggagggcctgacccatgaaccccttgatggccgcccgcgcctattcctccatccagggcggcgccatgcccagcgcgccgacgcccgccgcatcgggcgccggcttcggcgacatggtccagaacgtcatgcaggacatgacgcagcagacccgcgccgccgagacccagatgacccagtccatctcaggtcagggcaacctgatcgacgtggtcaccgccctgtcttcggccgaggcgtcgctggagacggtgatctcggtgcgcgatcaggtgatcaacgcctacaaggaaatcatggccatgccgatctgatcgcgggtggaccattggtcccggcgacacctctcggctttcggcgcattgaagacggcatgagcgaccatccgcgcctgagctccctgtccaccggcctgcgctgccgctgtccgcgctgcggcgaggggcccttgttcaagggcttcttgtcgctgcgggaccgctgcccggcctgcgacctcgactacggcttcgccgatccggcggacgggccggcctttttcgtcatgtcggcggtgggcgtggtcggcatgatcggcttcatgatcttcgacttcaccgttcagccgccggtgtgggtgcacctgttcaccaccctgccggtcctggtcgccttgtgccttggcgcgcttcgccccttcaaggcctggatggtggccgagcagtatctgcacaaggcggaggaagcccgcttcgaccgcccgaccgacccgtcgtgaacggctatctgttcctggccggcgccatcgtggcggaggtggtcgccaccacggcgctgaaggcgtccgacggcttcacccggctggcgccgtccgtggtgacggccgtgggctacgccgtcgccttttacctgctgtcgcaggtgctgaagaccattccgaccggcgtcgcctacgccatctggtctggcgcggggatcgtcttgatcaccctgatcgcctggctggggttcggacagaaggtggacgctgcggcgatcctcggcatggggctgatcgtggcgggggtgctggtgatcaacgtcttctccaaggcccaggcgcactagggctggacgatcgtcagctccggccatcgcgccctggcccgctcgacgacgcgcggccaatccttggcgagcggccgcagaggattcggccggatcaccctgtcgaagacatcgtccaggccaaacggggcgaccaccatcaggtcgccgccgtcgccaagacgcacccccaccgcaaaggccggggccacgaagcgggccagcgcctcgcccgtgccgtccagcgggccatactcctcaccgaatttggcgggaaaccacaacggcacccgagcctggttgcgcacctcgacccgctcccgcaagggcggctcgaatgcagcggccgtgcgccggatcaccacatcctcggcgtcccacgaggtgtcggggtcgaagtagccgacatcgaaatccttgaccccgtgccccgccggccggcccgtcagggcgttccacaccgactgatagaccgcgccggagaacaccagccagtccggcaggtccagcccacgcacggttgccagcaccatcatcaggtcggggtcggcgcggacgatgacgtccagccgctgttcgagggattcgctcatccgcatccaataggcgtccgcctcgttgatcgggagaggaaaggacgtcccatgtcgatcgccaaggtctacgccaacctgtcctgccgggatctgagcgccagcacgcgctggttcgccgtgcttttcggacgcgatcacgacaccgcgccgatggacggcctgcacgagtgggactgcggctccggcggcctgcagctgtacgaaaagcccgagcacgcgggcgccggcaccctgaccctgatcgtcgatgacattgacggcgaacgcggtcggctggaagaggcggggttggtgacggccgaactcgaggcggccgactacaccaccatcatgcggctgcgcgaccccgacggaaacctggtggtgctggctcagccgaacgaagcggccacctagcctctcaccggccaggcgtggtccagcggaccgtgaccgccgcccaagcccggtgcgcggcggatggcctcgccgacataggcccaggcctgcgccaccgcgacctccagcggacgccccatcgccagccccgccgcgcaggcgctggccagggtgcagccggtgccatgggtgtggcgggtctcgacccgctcgctctctagcacagtctcgccgtcgctggtcagcagcaggtcgatcacggccggacccggcacatggccgcccttcatcaggaccgcccgcgccccgagcttcaagagcgcctcgcccgcccgcctttgtccgtccagatcggcgatcgtcagacccgtcagggcctcggcctcgggggcgttaggcgtcagcagcgccgcgcgcggaatcatcagggctgccaccgcctgcaccgcctcgtccggcagcagcggatggccgcccttggccaccatgaccggatcgaccacggccggcgccctggcctcgtccagcaaggcggcgacggtctccaccacctcgaccgagcccagcatgccggtcttgaccgcatcggtcccgatgtcctccagcaccgcgcgcgcctgggcggcgatcagatccagcggcagcggatgcaccccgtgcacgcccagggtgttctgcacggtgatggcggtgatggcggtggcggcgaacccgcccatcatcgtcaccgccttgatgtcggcctggacgcccgcgcccccgccggagtcggaacccgcgaggatcagcacccgtccccttccgttcgcgctatcgccgtccgcgcgacggccggcggcttgagcggcgctcatcagtgcgaaaacagcttcaggccgacgatgcccgagacgatcagcaggatgcagacaaggcgcaccgccgtcgccggctcgccatagaccaggatgcccacggtggccgcgcccaccgccccgatgccggtccagatggcgtaggcggtgccgatcggcagccgctgcgtcgccacccacagcaggaccatgctgcccgccagcgccaccagcacgcccagcgacgtcagcggccggctgggcccgacgttcttcaggccggacgcccacagcacttccagcagaccggcgacgaccagcgtcagccacggattgatcgacatgagccaggacatggcgcccagatgcgccgtccggctcaccggggcaaggccgcctcaaccgccgcctgcaccttcagcgcctgaactgtctcgcgcacatcgtggacgcgcaccatgcgggcgccgcgccgcgccgcctccagcgccagcgccagggagccgcccagccggtcgtccgcctccaccgccgtctcgtcgacggcccggatcgtgcgcttgcggctggcggcgtagagcaccggaaagccggcccccgccagcacctccagccgtgcggtcagctcgaggttgtgctgcacggtcttgccgaagccgacgccgggatcgagccagatccgctctcgacccacgccggctgcgatggcggcctgcgcccgtgcgaccagatgatcgcgcacctccgacaccacgtcgccatagcgggggtcgtcctgcatggtgcgcggctcccccttcatgtgcatcagcacgacctcgcagccgagatcggccgcgactcccatgctgtccggcgcatggccgagcgcggacacgtcgttccacatcccggcccccgcccgaacagccgcacgcgccaccctcggcttcatggtgtcgatgctgatgcgaccgtcccagcgcccgcggatgcgctcgatcaccggcgcggtgcggtcgatctcctcggcctcgcccaccggatcggcgcccggccgggtgctttcgcccccgatgtcgagcacgtccgcgccctgctcggccaggcgcagcgcatggtccgccgccgcctcggccgacgcccagcgcccgccatcggaaaagctgtcgggcgtgacgttgacgatgcccatgaccagcggtcggctcatgtcggctcccgatccccacgagaaagggcgcgcccgataaggacgcgccctctgtcttccagcttcaccggcggctcagtgcaccgtcggcacgctggtggtggcgggcttggcgaccggcacggcgatctcggttccgtccgagaccggggtcaccggcacggcgaccgaaggacccgcgttggggaagttgttttcgtcgcggttcggcgcgacgcccttctccaagaggtccttgatctcctcgcccgacatggtctcgtactcgagcagcgcctgcgacagcttttcgtgatcgccggccttttcggtcaggatgcggcgcgcctcgtcccagccctggccgacgatgcgcttgacctcggcgtcgatgatgcgggcggtctcttccgagacgttctggctgcgcgccactgagtggcccaggaacacctcttcctggttctcgccgtaggccacggtgcccagcttgtcggagaagccccagcgcgtgaccatggcgcgcgccagcttggtcgcctgctcgatgtcggagctggcgcccgaagtgatgttctccaggccgaagatcagctcctccgccacccgtccgccggccatgatggcgatgcggtcgatcatctgctgatacttcatggaatagcggtcgccttccggcagctgcatcaccatgcccagcgcccgtccgcgcgggacaatggtcgccttgtgcacggggtcggccatcttgacgttcatggcgacaatggcgtggccggcctcgtgataggcggtcaggcgcttttcttcctcgttcatcgccatggagcgacgttcggaacccatcagcaccttgtccttggcgtcctcgaagtcgcggtgcgtgaccatgcgccggtccttgcgcgccgccatcagggccgcttcgttgaccaggttggccaggtccgcgccggagaagccgggcgtgccgcgcgccacggtcttgacgttgacgtcggcggccagaggcacgtccttcatgtggacgcgcaggatgcgctcgcggcccgagacgtcggggttgggcaccacgacctgacggtcgaaccggccgggacgcagcagcgccgggtccagcacgtccggacggttggtggcggcgatcaggatgatgttctcggacgcctcgaacccgtccatctcgaccagcagctggttcagcgtctgctcgcgctcgtcgttgccgccgcccagacctgcgccgcgatggcggccgaccgcgtcgatctcgtcgatgaagatgatgcagggcgcgttcttcttggcctgttcgaacatgtcgcgcacgcggctggcgccgacgccgacgaacatctcgacgaagtccgagcccgagatcgagaagaagggcacgcccgcctcgcccgcgacggcgcgggccagcagcgtcttgccggtgccgggagggccgaccagcagggcgcccttggggatcttgccgcccaaccgctggaacttgccggggtccttcaggaactcgaccacctcggtcagctcttccttggcctcgtccacgccggcgacgtcgtcaaaggtcttgcggcccttgtgctcggtcagcagcttggccttggacttgccgaagcccatggccccgcgcgcaccgccctgcatctggcgcatgaagaagatccacaccgccaccagcagcacgatgggcaggatgccgatcagcaggctggcccaccacgactggcgcgtggtcttggcgtcgacgttgacgcccgactgcagcatctgctcgaccagctgctcgttcgggaacggggtggtggcggtgaagcggccgttgttgcgatagacgccggtcacctgatcgccgcggatggtggcctcgcggatgtcgccggcctgggtgcgctgcaccagctgggaataggtgatggtctcgggccggccggcggcgccggggccgcccaccgcgccgttcatggcgccgccctgcgacaccgccgcataggccgccagcagccccaggatgatgacgctggtgatcgccagattacgcaggttcattgaagtcctcggtcgtccggcgcgcgccgtctgcgccgccggtcatgtgttctgcgccaagacatagggggttccaagacccttcgccatctgcgggcgaacgcagatcatcctcatgcgtcgtttcgcccgacaaggaacccagggcgagccgcatccgctgcgccgtcagaccgcggaccgcgacgctctcggcggcgagcacgggcgcgccctcctctcgcatcagcaccggccatgcggcgcgcgctgccgaggaaagacgggataggcgcgcgcgatcggcgggcgacagccgccccatccgtccttgcgccgctccgaccgaccagccgggttcctgcgcctgcagctcgaaccgcccgtcccagaccgcaggcgtcccgggcgtgagcgtcaacgccggcgccgcgcgccgcctcagttcgcccgcttcgcgcacgatcagcacgtccggcccgctcgcctccagccgcgccccggcgagcgtcgcggtgaaatcctcgcccgccttcacccgctccagcagcgcctgcagccggtcgcccttgggctgcgcctcgcctccgccggcacagaccagcgccgccgccagggcctggcggccgacgcctcgcccgcaacgaaacccttcgccctcgaccgcgtggggagggtctccggcaggcgggcggagaggcgtctcggctcgatccagcggatcgccgcccaaggcccggcgcgcacgggcgcgggcgtggcgaggatcgtcgttggcgggatcatcgatccagggctgatctcgcgcagccagccagcgccgcagcggctcgcgccgcgcctcgagcagcgggcgcagcagcatcagcccgcgcccctgcggccacacgggcgacggcgaccactcccgcatccgccccagcgtcgagcctcgcgcgcgcatccactcggactcgtccacgtcgtcggcggtgtggccgaacaggacgacacgggcgtccgcccgccgggccgcatcggcgatcaggcggtggcgcgccaggcgcgcggcggccgcgaggcctgcatccggcttggcgccctcccaggccaacggcagccactccgcgccgcagagtcgggcctgttcgcccgcaaaggcggtccagtcgcggctggaggcctgaagaccgtgatccacggtgagaaccagcagccgccgcccgcgcgtcctggcccagccggcggccatgtgcagcagcgccagcgagtcgccgccgccggacagggcgacgcacaccggcgcgttgatgttcgggctcagccgcgcgtccagccgggcgcgaaccctcgtctcgaggtccggctcgatcaggccgcgcacgccgcgcgggtgcggctctggacggcgcgggtcttcagggcggccggcgcgtcgggatagcggcgcgtgaactccgacagggcggcgcagccttgcgtcttgcggtcggtggccagcagcgcgtccgccagcttcagcgtcgcctcgggcgcccaggcggtcttcggccagtccttcagcgccgctgcgtagtaggacaccgcattcgcgcggtcgttggcctgcacgctgaggtcgcccagatgcagattcgcctcgcgcgcctcggccgcctcgggccaggtcacgatcagcgtctccagcgcccgcacggcgcgcggccggtcgctccccaacagccgcaccgccgccgccaggtcgcccgaagccgcacccgtaggagagttggagacgatgggagcgttcagttcggcttcagtctccaacttccccacccgctcctcggcctgggccaggcgggtccgcagggtctcgttggcccgctgcgtctcgtccagctggaaggtcaggcgctcgccgtcggcgttgacccgccgaaaggtctgctcgaggtcctgcagccgctggtccatggccgcgacgcgcccctgcagcgccaccacctcggggtccggctgcaccagcacgggctcgccggcggcgttgcgctgggtcagcgcccgctccagccgacgcacgttgcggtccaactggtccaggcggcgcacgtcccactggatcgccggcaagggggcggtctgggcgaccaccgcgccgccgatcaggcagacgccgacggcgctcagggcgaggacgcgaggagagacggaaagcttcatcatggctggattgctcccaccgatttgcggcgcgggcaaggcttgggatgcgccgtcagtgccccaggcccagatagacgatcgccgccacgaacaggcccaccacgatgctgctgaagtgcagcaacaaaagcgtgcgccaactcgccgaccaccacgacagcccataggcgcccttcagctgggcgaacatgtgcacggggatcgccgccatcgccagaaaggcaacgggcacggccaggcccgggatcattcccaccagcaccagcgccatcagcagcatggccatgaacgtcagcgagtacaaaacgaacaccccgtggtcgtacagggtgaagccgcgcttccacaggaacagcaaggccacgaacggaatggacagcggaaccagcagaaaggcgaacttgtagatcgtctgctgcagcttgtagagcgccaggtcggggttctgcagcttcttgaccaccaaggcgcccaggcccttgccctggatcctgttctcggccgccatgtccttgatctgggcctgccagctgccggacttcagaccgtccgcccggccgtctcggcctcctgcagctcgtggcgctgctcggcgatccgctcggccatcggctgctcccccgcctcgcggtgcggggcgaaggtcagggcgaagaacatgacgaaaattgtgaacaggaacatcgccagcggcgagacatagcgcgtgcgcttgccccgcacccactcgcgcgtcagccgcccgggattgaaggccagaagcggcagggtgcgccagacgcgggcgtcaaaatgcatcacgccgtgcagcaactcctcgccgagatgaagtagagtgcggtgcgtatgcgccggctgaccgcattccgggcagaacttgctggacacctgcgccccgcagtcggcgcagcgatggccggcctcgcccgcgtggcccgtgggtcgctcgatcgcgccggccaccaagcccgccgacatcatgccgcccgccgcatccacatccatgacgatccccccgaacctcggaagcgatctagccgtccctgaccgtctgcgacaagccgccgcaacgaaaagaggcgccggccgcagccgacgcctcctcgaaccgatgctgttctaaggcctcagcgctgggcgcccgagacgatggccgtgtgggcgttgcggttgcgggcgaaggcgtcttcggtggatccttcggcgatcggccgctccttgccgtagctgatggtgtcgatccgaccggccgggatgccgcgattgatcagataggtgcggaccgcctcggcgcgacgcgcggccagggccaggttgtactcgcgggtgccgcgttcgtcggcgttgccttcgatgcgcaccgcgacgcccggatagcgctgcagccactgggcctgggcgtccagacgcggaaaggcctcgggacgcacctcatagctgtcgaggtcgaaatagacgcggtcgccgacgttgacgacgaagtcctgctccgaccccggcgcgctggcgatgcttccgccggtcaccggcccggtcggggcggtcggataggcggggttggtcgcggggccggacggcacggcgcccgcgtcgggcgtcgtcccctgcgcgggcgggcgacggttgcaggcggccatggcggcgacggccacgccgatcagggccaggcggcccaggcgggacttggaagcggcggacatcatgacggggtcgtctcctgttggtttctcatgaggacaacggcctcaagctttggcgttgcagtctgcgttggcgcggcgcgttgcaccataggctaacgcaggagtgattgatcaggcgggacaggcgtcggcgccgcccagccccgcgctggcgctttcgtccagcagcggcgaccaggccgggtcagagccccgtccgttgtagccggcctgggccaccacgcggccggacaggtccacggtccacaggcgggtgtcgcctcccggcgtctggcgcgcgaacatgacgtagcgaccgttcggcgcccagctggggccttcctcgaaataggacgacgacaggatgcgctcgccgccgccggacgggtccatcacgccggtcgagaaccgtccgccgccctgtttggtgaaggcgatcaggtcgccgcgcgggctccaggccggcgcggtgtagatgccgccgccccggctgatcggccgctggctcgatccgtccgagcgcatcacatacagccgcgccgatccgccccggtccgaggtaaagacgatctgcgagccgtccgggctgaacgacggcgaggtgtcgatgccgggatcggtggtcaggcgcgacagctggcggctgcgcaggtccatcacatagacgtcggtgttgccgcgccggatgatcgagaaggccaccttggatccgtcgttggagaagcgcggcgccagcacctggccgtcgaactcgcccagcgactcgcgccgacccgtcgtcaggttcagcaggtagatgcggctgtagtccttgcccagcgccacataggtgatctcgtcaggctgcgaggtcgagaagcgcggcgacatgatcacctcgtcgccctgcgtcagataaacggggttgtagccgtcctggtccacgatcgcgaggcggctcatgcggttcagctgcgtgccgctttcggacacgaacaccactcgcgtgtcgaagaagccggcctcgcccgtcatccgctgatagatcaggtcggaaatcttgtgcgcgatgcggcgccattgctcgggcgtggcggtgaactgatagctgacgatctggcactggcgatacggatcgtagaggcggaaacccacgtcgttgcggccgtccgggcgcggcgtcaccgcgccatacagcaccgcctgcgccccgatctgcgtccactgcgggaagttgggggcgttggcgagcgtcaggcccgtctcgatgaagctggaggggttcagcggctcaaagaagccggagcgcttcaggttgccgctgacgacgcccgagatgtcagagccgttctggccgctgaaagggacaacggcgatctgcagcgggcgcagcacgccctggtcgatctcgacctccaccggctggcccgattgctggggcgccgccgtctgcgggttctgcgccatcagcggcgaggccatcgccatggccgcgaccgaggccagaagaaggttcagacgcattgggggctccgtgggtcgtgcaggatcgcgcccttatcgccgggcgacggcgcaaccgccagcttcatggcgaatggggcgactttcgggcctggcggttcgcgttttcgtcaggcgcgtccgccttttgcggatgctcgcgaagcgccgcttcgcgccgccagggccagcgtccctcgatctcggtctcaagcgagaagctgagaaaggtccggatcagcaccacgccggccagcagcccgacgctctccaccgtcagcggcgaggtgacggtggcgatgatgtcggcgccgaccagcagctccagccccagcaggatgccccgccccaggttggcgcggtagccgtcataggccctcgcccaacccccgcccttaaacccgttgaccaggtaaagcgcggtggccagccccaccgccagcagcagcacgccgaccccgaacagctccagcgccgtcgccgcctgccgcgccaggtcgatgaggggcccgtggcgatcttcggacaaggcggtcgaggcgttcatgcctcctcgaaccgccaaggtcgcttacctgttccggcaggcgcgctcggtgttgaaggtcgggcgatagacgccgccgggaaagccctgcggcacctcaaacggcgcggtctggcgcagcgcccgcagcgcaccgtccgccgccgcgcgatagaccgagctggactgggcgttgatcagcgacggcccgcgcgtgatccgtccgtccgccgacagggtcagctcgacctggatgcgcagctggtcggctcccgggatgtcgcagggcagaatccagttcggatagacctggttgaagatggccgtgatctgcgggcccgtcgcctggctggcctggcccgcgccctgctgccccgccgcaggacgaccgcggctggcgccggggttcgggcgaccggcgagagcgtctaggtcgaggctgggttcggtgcgctgcggcgcagggcgggccggagccggattgggccgcgcgggcgcaggcgtgggtcgcggcggcgtcggctgcgccttctgcggcggcgagggcgtcggacgaggcggcgtcggacgagggtcggcgccggccggggcgtcggggcgggcggcgggacgtggcgtcagctggggcgtcggctggggcgtcgggcgggcggctggggtgcaggtgtcggcggcgtgggctctggcgtcggcggaaccggatcgggctgctgcaccggcgcggtggcggcgttgtcgggcgacggctccggctgcggattgtcggcggccgccgccgcgacctccgtctccgacacgatcgagaccgggaccgaactgaccagaggcttgggatcctccgggctccgctcaggccatgacagaaaggcgagcgccgccacgcccaggtgcagggcgacggatccgagaacggccgggctcggacgacgcaaggggctcaggcctccggcgccgtgtcggtgatcaggttcatcttggtgaagccggtggcggacagccgcgccatgacccgcgccaccgcttgatagggcgctcggccgtccgcgcgcacgaacaccggccgctcgcccgcctgctcggccccgccggcctcctgcagcagacgcggggccaactcctcgaagggagtctcgctttcgccgatgaacaccgcgccctgctggtcgatggagacgctgagcggctcgttgtttgtctccaccgcgctggcgtccgtctgcggcagctcgaccggcacgcccacggtcaacagcggcgccgagatcatgaagatgatcagcagcaccagcatcacgtccaccaggggcgtgacgttgatctcggtcaggggaccttttcgcccccgccggccacgacggccgccgccgccgcccgatcccccgcccatggccatggctcagaccgtccggttcaggctgatgccgtcggaaggcggcggaggcggaggcgccgcgcccggcgagcccagccggcgcgccaccgccgcctgcaggtcgtcggcgaagctttccagccgcccggtgaacttgcccgcgtcgatggagaacttgttgtaggcgatataggcgggaatggccgccgccaggccgatggcggtggcgaacagcgcctcggcgatggccggggccacggtggtcaggttggtgttgccggccgccgcgatccgcccgaaggcgttcatgatgccccacaccgtgccgaacaggccgatgaagggcgaggcggtggcgacgatcgacaggacgcccaggcccttttcgatccgctggccctcgcgcgcgatcaggctgtccatggcccggtcgatgcgggtcagcagcaatccgccctgttcgccgttcagcgcgcccttctgccgggcctcgcgccagtcggacagggcgatcaccagcatgcgcggcagggcgtgcgacgggttcggcccggcctggttggccacctcctccagcgatcggccggacgacaccgccgtctcgaaatcgtccgcctgcttgttcagcgcggtgaagcggaaagccttgtcgatgatgatggtccaggaccagaccgaggccgccgccaggccgatcatcacgctcttgaccacccagtcggcggtcaggaacagctcaacgggattcatcatcgaggcgtcgacggcggcggtcatgcaggggcgctccgagggacggtgaacaggcgtccttaccagcggcaggacgtgttctttgtgtggcgaagcccgcctctagcggtccgcctcgccgccgtcacctcacagaggagtcatcctcgaatcttcacgctcgccggctcagggtctatgcaggcggccatgacgtccgcccccctccccgatgccggccagaactgggtggaccgccacgcgccggaagggctgaagccgtggctgaagctcggccgcttcgaccggccgatcggcatatggctgctcttgctgcccggctggcaggggatcgctctggccctggctcagtacggcaagacgccgggcgcctatgagatttggctgttcgcgggcttcggcgtcggcgcctgcctgatgcgggcggcgggctgcgccttcaacgacatcgtggaccgcgacttcgacgcgcgcgtggcccgcaccgcccagcggccgattccttccggccgcatctcggtcaagcaggcctggggcttcgtggtcggatgcagcctcgtcagcctgctgatcctgctgaccttgccgacggtcgccattctgctgggcgtcggatcactcgggctggtcgcggcctatccgttcatgaagcggatcacctggtggccgcaggcttggctgggcctgaccttcaactggggcgcgctgatgggcttcgcctccgccctgccgcttgcggccgcgcccctgctgccgcccgagatcgccggcgagttccgccctttcctgtggcaaggcgcgccggcgcgcgaccacgccgtgggtctcgcctggcaggcctatctgcccgccgtgctgctttatctcggcggcgtgttctggaccctcggctacgacaccatctatgcgctgcaggacatcgaggacgacgccatggtgggggtgaagtcctcggcccgacgtttaggggcgggcgtgcgacggggcgtcgccgtcttctatgccctggccgccctgctggccgcatgcgcgctcgcctcggctgggctgggcgtgctggcctggaccggccttctgctctacgccggacacctcggattgcaggtcgtgcgcctgcgggtcgatgatccggcgcaggccctgcgcctgttcaagtccaaccgcgaggcgggcctgctgctgctgttcgctatcgccgccggctcgctcggcgtcgtttcctgatcccgcaaacggagacttaccgatgacgccgtcccgcctcctgctgatcggatgtgcgctggccgccttcgccggatgccagcgccgcgaggaccccgcgccccagccgcccgccgcgcctgcggccgctccggcgcccgctctgtcgactgagccgctgagcttcagcgaacagacaccctacgccagcgtccggctgaccctcccggaagcgatccgcacccagcccgaactgcacacggccctttacgcctccacggtgcgcgagctgcgccagttcatggagggcgcccaagccgaccgcaccgaggcgggctcggacagcagcctgccgccctatgagaagaccatcactgtcgagccgggcgccgatgcgggcacgctgttcagcctgaagcgcaccgactacgactattcgggcggggcgcacggcaacaccctgttcgctggcgtgctgtgggacaaggcggccaagcgccagatcgccgccgccgatctgttccgccccggcgtcgatgcggcggctctggaccgcgccctgtgcgatgcggtcaatgcggcgaagcaggcgcgctcgccggggacggagcggctgacgctcggccggggcgacacctggaactgcccgcgcgccctgcagacgcccatggcgctggagccggcggcgggtcagccgggcaaggcgggcggcctcgtcttcctgatcggcccctatgcggtgggaccctatgcggagggcgcctatcagatcgtcctgccgctgagcgccttccaggggctgctcaatcccccctacgccggcgacttctccggcgccccggttcgcacgggcgacgtaacgcccaggcagggttgaacgcggacctcagtgcccttcggccgcctgcatcagctcgatcagcaccccgcccatgtcgcgggggtgaaggaacaccaccggcgtgccgtgagcgccgatgcgcggctcgcccgtgcccagcagggtcacgcccttggccttcatctcggcgatggcggcgtccatgtcgtccacctcgaaacagacgtggtgctgaccgccgcgcgggttcttggccagaaagccgacgatcgggcttgtgtcgtcatacggctcgatcagctcgatctgggcgttcggcagatcgacgaaacagaccttcaccccctgcgccggcaggtcgaagggctcgccgacgcgggtcgcgcccagaacgtcgcggtatagcgggatcgcctccgcgatcgacggcgtggcgacgcccacgtggttcagcttgccgatcatgcgggcgctctcgacgggacgggctgggcgtagccgagccgctggttcagcttctcgaggaggtcgatggccgtgtccgcgatggccgagccgggcggatagaccgccgccgcccccatctccagcagcggctgcacgtccgagggcgggatcacgcccccaacaacgatggtgatatcgggccgccccagcttctccagttcagccttcagttccggcaccagcgtcaggtgcccagccgccagggatgaggcgcccaccgcatggacgcccttctccaccgcgtcgcgcgcggcctcggccggggtctggaacaggctgccggcggtgacgtcgaagccgagatcgccatagccggtcgccacgaccttctggccccggtcatgcccgtcctggcccaatttggcgatcaggatgcgcggcggcccgccgtcgttctcgacaaaagtcgccaccatgtcgcgggcgcgggcgaaccgcggatcgcgtccggcctcgcgcgcataaacgcccgacaccgtcctgaccgaggcgacgtgccggccgaacgccgcctccagcgcatcggatatctcgcccaccgtcgccttggcgcgcgcggcctgcacggccagttccaagaggttcgccttgccgtgggcgccgcgcgtcagggcgccgagcgcaccttgcgtctccgcctcatcccgctctgcccgcaggcgcttcagcttgtcgatctggcgggcgcggacctcggcgttgtcgaccttcagcatcggaatgtcgtcgggcgtgtctgagagatagcggttgacgcccaccaccgtctgctggcccgtgtcgatgcgcgcctgggtgcgggcggcggattcctcgatccgcatcttgggcacgcccgcctcgatggccttggccatgccgcccagcgcctcgacctcggccatgtgggcgcgcgcccgctccgccagctcgtgcgtcagccgctcgacatagaagctgccgccccagggatcgatcacgcgagtcaggcccgtctccccctgcagcagaatctgggtgttgcgcgcgatccgcgccgagaagtccgtcggcagggccagcgcctcgtccagcgcattggtgtgcaggctctgggtctgtccgcccgccgcggccatggcctcgaccatggtgcgactgacgttgttgaacacgtcctgcgccgccagcgaccagccagacgtctggcaatgcgcccgcagcgacagggagcgcgggtccttgggcccgaacgccttctgcaccgcctcggcccacagcaggcggcccgcccgcatcttggccacttcggtgaagtagttcatgccgatggcccagaagaagctgaaccggggcgcgaaccggtccacgtccatgccggccgccacgcccgcgcggatgtactccagcccgtccgacagggtgtaggccagctcgatgtccgccgacgcccccgcctcctgcatgtggtagccggagatggagatggagttgaacttcggcgtctcctgcgccgtccaggcgaagatgtccgcgatgatccgcatcgaaggctcgggcggatagatgtaggtgttgcggaccatgaactccttgaggatgtcgttctggatggtcccggtcagcgccgcgtgcggcacgccctgctcctcggccgccgcgacataaagggccaggatcggcagcaccgcgccgttcatggtcatggacaccgacatctgatccagcggaatgccgtcgaacagggtccgcatgtcgtagatgctgtcgattgcgacgcccgccatgccgacgtcgccggtcacgcgcgggtggtcggaatcgtagccccggtgcgtcgccagatcgaaggcgatcgacagccccttttgcccggccgcgaggttgcggcggtagaaggcgttgggttcctcggcggtggagaagccggcgtactgccggatggtccacgggttgcccgcgtacatggtcggataggggccgcgcatgaagggcgcgaaaccgggaaggccgtgccgggcgtccagctccgccgtcgcttcgggaccgtaggcgggccgcaccgtcaggccttcgggcgtcagccaaggctcgcgcgcgggcccttgtcccgtcggtgacaggtcgagcgggatcgaggagaagttcggaaaggtcatcgtgcgctcgcctcgtgcggctcggcgaagcggatgggcgtcaggggctcgcagacgcgatcgacggaagaggcggccgggcgcggcgcttcggtcggtgcgggacgcggatcgggatcgacgaacttggtcaccccgacgatctgggccgcgccatcggcgtaggccttctcccgcacggcgcgggcgcgggcgatgcggggctggatcaccccgccgctgagggcgtcgatcaccccgccttccgcctcgatcatctggaactcggcccagccggcctcggccagttcgcgcgtgcggctgtccaggaaccaggagccggcggcgggatcgtccacgcgaccgaggctggcttcctccatcagcaccagctgggtgttgcgcgcctgtcgccgggcaaaggcgtccggtcgcccggaagccgtggtgaagccgtccagcaccaccacgtccgctccgccgacgcctccggcgaagcccgccgccgtcagccgcaaaaggttcggccagggatcgcgcgccgccagcatccgccgcgacgaccgcgcctcgatcagggcgggcgtctcgcatcccagcgcccgcgtcaggctgcgccagatcaggcgcatggcgcgaaccttggccaggctgtcgaaatactcctgatcgaccgacaggccgatcaccgtgcccgcaagcgcccgctcccgcgtcatacccgcgtccaccgccgcccgcgcataggccacggccgatgaggcggcgaaggccagctcctgcgcgatcgatccgcccgcctcgtgcgcgacccggcccgaggccagaaagaagctcgcttcgggataggcgcccgcgtgccgctgggcggtgttggcggccagcataaggtgctcgtccaccggccgcggcgaaccgccggccgcggcgaaggcgccgatcggatcgagatggaaccggagcttcgcgcgcggcgcgcccttggctgcgaccgccagggcattggccgcatccggcccgtcgatccccgcatccagcgcgacgggcgccagttccagcgccacgccgtccagcgcgcgccgcagcggctcggagtcgctcagcaccacgcccgccagcagcaccgacgccgcgccgccttccagttcggccagcaccgccgcattcaccgccgccggatcatcgccctcaacgggcgcgcgcaggtcccaggcccggccgtccgcgtcggacgggcgcggcgcggacaggggctgcacgccgctcgccgccgcatacaggggccgcaccgccaggccgtcggcgtcgagatgaaccaggctttcgatcgcccggtcctttagcgccttttgcgcggcctcccgccattccagcggcgtggggacggggaaggtcacgatcaggccagctcgaccgccatggccacggcctcgccgccgccgatgcacagggacgccacgcccttggagccgcctcgcgcctgcagcgccgagatcagggttgccagcacccgcgcgccggacgcgccgatggggtggcccagcgcacaggcgccgccgttcacattcaccttggcgtggtcgatgttcatttcgcgcatggcgatcatgggcaccaccgcaaaggcctcgttgatctcccacaggtcgacgtcctccaccgaccagccggcctttttcagcgtcttctgcatcgccggcaccggcgcggtggtgaaatgaccgggcgcatgcgcgtgcgcggcgtggctgaccacgcgcgctaggatcggcaagcccagcgcctcggccacgctctgacgcgtcatcaccacggcggccgcgccgtccgagatcgaggacgcgttggcggcggtgatggtcccgtccttggagaaggcgggcttcagcgtcgggatcttggccggatcagccttggtcggctgttcgtcggcggtgaccgtctccacgcccttgcgggtcttgacctcgaccgggacgatctcggaggcgaagccctcgccggtcgcggcggcgcgcgcgcggttcaggctctcgaccgcatagtcatccatggcctggcgggtgaactggtactcggccgccgtctcctcggcgaaggcgcccatcagcttgcccgtgtcataggcgtcttccagcccgtccaggtacatgctgtcggagatgacgtcgtgcccgatccgggcgccgccgcggtgcttggccatgacgtagggcgcgccggtcatggactccatgccgccggccacgatcacgtcggcggtctccgccttcagcgcgtcatgggccatcatcacggcctgaaggcccgagccgcacatcttgttgacggtggtcgcctccacatgctggcccaggcctgcgccgatcgcagcctggcgcgccggcgcctggcccagaccggcggacaggacgcagcccatgtagatctgctcgaccttgtctgcggatacgcccgcgcgctcgaccgccgccttgaccgcgacggcgcccagttcggtggccttgacgccggacagcgcgccctggaagccgcccatcggcgtgcgcgcgacggagcagatgacgacgggatcggacatgatgtttccctgaactttcttgttgttctgcagcttactggaattcgacaagcacgtcgtcggcggccacggggtcgccggccttggcgccgacggccttcaccacgccgtcgcgttcggccttcaagatattctgcattttcatggcttcaatgatcgccacggtttctccggtcttgaccgcctggccgacgctgaccgggacagagaccaccagtcccggcattggcgactggatcagcttggaggtgtcggcggcctgcttctccggcaggcgagcgaagaactcggccgcgcgcggcgtcatgacccgaacacgcgccctggccgcccggtggcggatatcgaagccgtcggcgacccgcttcacctcggcggtgaagggctcgccatccagttcggcgcggaactgcgccaggcccggccgccagtcgatctcggtcagccgtgcatgaccgccgccggtgaaggccagcagcagcgcctcgtcctcgtcgtagctcaggctgacgccatgcggcgccttgtccaccagcacgatccagtcggtgcggtcagacggatcgccggcctgttcgctgatgatctcgtgcatggccatgccggcggcgaccaggatgcgcgcctgccgctcggacggcgtcaggccgtggaagccgtcggggaactcgtccttgatgtagctggtcgatagctggccggaccggaaccgatcctggtccatcaccgccgacaggaaggggatgttgtgccccaggcccgacaggtgcgtgtcctccagcgcccgcgccatgccgtccaccgccgcatcgcgcgtcggtccccaggcgcacagcttggcgatcatggggtcgtagaacatgctgatctcgtcgccctcgcgcacgcccgagtcgttgcggacgacatagccgtcctgctcgccctcctccggctgctcgtagcggaccagccggccgatggagggcagaaagccgcggtacggatcctcggcgtagatgcggctctcgatcgcccagccgtcgattttcagctcgtcctgcttgaacgccagcgcctcgccccaggccgagcggatcatctgctccaccagatcgacgccggtgatcagctccgtcaccggatgctcgacctgcagccgggtgttcatctccaggaagaaaaagctcttgtcctgaccggccacgaactcgaccgtgccggcggaatcgtagttcacggcacgggacagggcgacggcctgcgcccccatggcggcgcgggtctgttcgtccagcaagggggacggcgcctcctcgatgaccttctggttgcgccgctggatcgagcattcgcgctcgaacaggtggacgacgttgccgtgcttgtcgcccagcacctgaatctcgatgtggcgcgggtcgacgatgaacttctccaggaagacccggtcgtcgccgaaggcggccatggcctcggcctttacggcggcgaaaccttcggccatgtcgtcgtcgccgtgcgccacgcggatgcccttgccgccgccgccggccgaggccttgatcatcaccggatagccgatctcgcgcgcgatcgagacggcctcctccggcgtctcgatcaggcccatgtggccgggaacggtggagacgcccgcctccgccgcgaaccgcttggaggtgatcttgtcgcccatggcctcgatggcctgggggttcggcccgatgaaggcgatgccctcgtcccgcagccgacgcgcgaagcccgcgttctcgctcagaaaaccgaagcccggatgcacggcctgcgcccccgtctggcgcaccgcctcgacgatcttgtccgccagcagataggactgcgccgccggcgccggcccgatcagcaccgcctcgtcggccatctcgacggcgagcgagcccgcatccgcctccgaatagacctgcactgtctggatgcccatgcgccggcaggtcttgatgatccgaaccgcgatctcgccccggttggcgatgaggattttggagaacatggctattcttcctttgccgtcatcctaggccttgtgcctaggatccagaatcccggtgtttccggtgcgctctggccgacgatcgtgagtctggatcctcgccacaggggcgaggatgacggtgaaggggggcgacaatggtcgcgcgcgacagcttgatcggctgctacatcatgaccaatcggatgcatggcgcggtatacatcggcgtcagcagccagttgatcacacgggtcgcccagcatcgcgaaggcgtcctgccgggccatacccgcaagtacggcctgaagcgcctcgtctggtacgagttccacgacaccatcgtcggcgcgatccagcgcgagaagtcgctgaaacgatggcctcgtgactggaaggcgaacctcatcgagcgcgacaatccgcactgggacgacctgtttccgggtctcgccacgaacggcgtcgaggtcgcacccgttccaggcgcttaccgcgactggacgcctccagagggttgacgccgcccttcctttttccgtcaccctaggccttgtgcctagggtccagagactcggtcgagagcggcgtgcaccggcgagcaccgggagtctggatcctcgccacaagggcgaggatgacgagagagggcgatgcacggtcatcacagcgggatgttgtcgtgcttcttccaggggttctcctgggacttgttcttcagcgtccgcagcgccttgatcagccgccgccgcgtgccgtgcggcatgatcacgtcgtcgatgtagcccaggcccgccgcgacgaacggattggcgaagcggtccttgtattcggcctcgcgggcggccagggcgtcgggatcgccggcctccttgcggaagatgatctccaccgcgcccttggcgcccatcaccgcgatctcggccgagggccaggcgtagttgacgtcgccgcgcaggtgtttcgagctcatcacgtcataggcgccgccataggccttgcgcgtgatcaccgtcagcttgggcaccgtcgcctcggcgtaggcgaacaacagcttggccccgtgcttgatcaggccgccgtattcctggcgcgtgccgggcatgaagccgggcacgtccaccagcgtcaccagcggaatgtggaaggcgtcgcagaagcgcacgaaacgcgcgcccttgcggctggaatcgatgtccagcacgcccgccagcacctgcggctggttggcgacgatccccaccggctggccgtccagccggccgaagcctgtgacgatgttcttggcgaaatccgcgccgatctcgaagaagtcggcctcgtccaccgtcttccggatcagctccttcatgtcatagggctggttcggattggcggggaccagggtgtccaggctgggctcgtcccgatcgggctcgtcatagctgtcgcgcaccggcggcttttcgcggttcgacagcggcaggaagccgatcaggcggcgcacctcggccagggcctccaggtcgttctcgaacgcgccgtccgccacgcccgacttgcccgcatggacgcgggcgccgcccaggtcctcgtggctgaccacctcgttggtgacggtcttcaccacgtcggggccggtcacgtacatgtagctcgtgtccttcaccatgaagatgaagtcggtgatggccggcgaatagacgtcgccgcccgcgcacggccccatgatcacgctgatctgcggaatgacgcccgaggccagggtgttctgcagaaagatgtcggcgtatcccgccaggctctccaccccctcctggatgcgcgcgccgccggcgtcgaacaggccgatgatcggcgcgccgttggtcagggccatcttctggatcttgacgatcttggccgcgtgcgcgcccgacagcgagccgccgaagacggtgaagtcctgggagaagacatagaccagccgcccgccgatggtcccgcgccccgtcaccacgccgtcgccggggatgcgctgcttctccatgccgaagtcgtgggagcggtgctccacgaacatgtcggtctcctcgaacgagccttcgtccagcagaacctcgatccgctcgcgcgccgtcagcttgcccttcttgtgctggttggcgatgcgggcctcgccgccgccctgccgggccaccgcgcgccggcgctccagttcgtcgatgatcgactgactcatagacatcctcgccctgatgcgggccgtcgccgcctgtatcgacggtcgcgccccgcgtgcgccgggcgctgaacacggcgcccgcaccgaacctctgcgccggctgttcgatcctgtgaaggggccttggcgatgtcaaaccgtggcaaggacttgccgcgcggagcgaataaggcgcgcatggcggcaacagccgccccgccgaaccgtttgcaggcccatgccgcccgtcgccgatccgtccgccagcgcctcgccccagtccgcctccacgccccccgccatgccgacctcgccctgggccctgccgatcttccgggcggtgtggctggccagcatggcgtccaacttcggcggactgatccagtcggtcggcgcctcttggatgatgacctctcttgacgcctcgccccagatgatcgccctggtccaggcctcgaccaccctgccgatcatgctgctgtcgctgtgggcgggggcggtggcggacaatctggaccggcgctgggtcatgctgtcggcgcaagggttcatgctgacggtgtcgatcgtgttggccgcctgcgcctggggcggggtgctgacgccgtggctgctgctgggattcacctttctgatcggctgcggcacagccatcaacaatccggcctggcaggcttcggtcggcgacatggtcccgcgcagcgtcctgcccaccgccgtcgcgctgaacagcatgggcttcaacatcgcccgcagcctgggtccggccatcggcggggtgatcgtcggcgcctttggcgcggcggcggcgtttctgaccaacgccttcagctacctcgctctgatcgtggtgctggcccgctggcggcccgcgcgtccgccgcgcctcctgccgcgcgagaagctgggcatggcgatggaggcggggcttcgctacgtcgccctgtcgcccggcatccgccgcgtgctgttccgcgcggccgtgttcggtctggccgccagcgccgtgccggccctgatgccgctggtggcgcgcgacctggtgggcggcggaccgttcgtctacggcctgttgctgggggccttcggggtcggggcggtcggcggcgccctgtcctcgacccgcctgcgccagcgtctgtcggccgagtggatcgtgcgggtcgcctcactcggcctcgggctcggcgcggccggcgcggcgctcagcccggccttgctcctgaccctgccgtgcctggcgctggccggcgccggctgggtgctggcgctgtcgaccttcaacgtcacagttcagatctcggccccgcgctgggtcgtcgcccgggcgttggcgctctaccagatggcggcgttcggcggcatggcggcgggcagctggatcttcggcggactggcgggggatcatggcgtggcgaccgccctgctcgccgccgccgcggtgcagctgggcggagcattgctgggcgtgctcctgcccgtgccacgcatgcggatgctggatctcgatccgctgggccgcttccaggagcccgagaccgccgtccccgtcgagccgcgcaccggcccggtggtggtcaccatcgagtaccgcatcgcacccgagcgggtggtcgaattccttcatgtgatgacggagcgtcgccgcatccgccgccgcgacggagccaagcactggaccctgctgcgcgatctgggcgagcccgacctttggatcgagcgctatcacgtggcgacctggctggactacgtccgccacaaccagcgccgcaccaaggccgacgtggacaacagcgacgccattttggccctgcattccggccccgagcgcccgcgcgtccaccggatgatcgagcgccagaccagcacccttccttggtcccgccacgtcgatcccggcgaactgcccgacgccctgaccgacccgacccgctccacataaggaaaacggcggccccccgtcaggagagccgccgcttgtcggtcagtcttgcagccgcgtcttagcggtacagggcccgctcgcgctcgatctgctcgctggagtagggatccgcgttcgggtcgaaggccgaccagccggtctggcgataggccgcgccgcgcgtggtggcgtcaaagccgcgacggccgttcagaatgccttccagccgcgcgcggtcatgctcgtcggccttgatgctgaccagggtgccgccgcgacgcacgccctccgcgtagacgttggcttcttcgtcgctgtgaccggcttccttcagggcgcccagcaggccgcccgtcgcgccgccgaccgcggcgcccgccgccgcgccgaccgccgtggaggccagccagccggccgcgaccaccggacccaggcccggaatggccagcatgcccagccccgccagcaggccgccggccgcgccgatcacgccgccggtagtcgcgcccttgccggcgccgtcggccacgtcgttctcgccgtcgccgttgcggtcgcccagcgggccgcctgccgtgcggtcagggtgcgaatgcccggcgtgccagttgtcggtgttgttggagacgatgctgatgcggtcgtgatcgacgcctgcggcctcgaggtccgagacggcgtcgagcgcttgcgagtggctgtcgaacagccgtgtgatggtcgccatggggcggctcctttgatgtgttgtgcgggaaaagaggcgggcgtgcgctactgcgcgctcaccacgcccttgtagtcgacagagacggtggtctgggcgccgtcgcggctggcggtggccgaccagacgccctggtcgttctggctgagctcgccgacgtcggtgtagccctgcttttcgatggcttcgcgcgcctggccttcggtgaaggagttggcgccgggcgtcagggcgccctgctgggacgtgtcggcggtgtcgacggccggattgcgcggcgtttccgacgaagaaacggccgggccttccaccggtccggtttccggcgcggcgtcgttgtcgccgcaagccgccagcagcgcggcggtggccgcgagggcgagaacgggtttgatcattggctttcccttccagaggttgcccgaaaggaagggacccgcccctctatggttcccccgaaaggcgagatgacgcgggtccattcgccttccgccggcgtcgcggctataggaaccccgcccgcaaccagcccctttccgcgcccatgcctcccctagatcgacggctgtccatcgcccccatgatggactggactgaccggcactgccgcgcctttcaccgcgcgctgaccggccgcgccctgctctataccgagatggtgacggcgcctgcggtgatccacggcgatcgcgagcgcctcctgggcttcgacgccgtcgagcatccggtggcgctgcagttgggcgggtcggacccggcgcagttggccgaggcggcgcggatcggcgcggcgttcggctatgaagagatcaatctgaatgtcggctgcccgtccgatcgggtccagtccggccgtttcggcgcctgcctgatgaaggagcccgagctggtcgccgactgcatggccgccatcatcgaggccgtggacgtccccgccaccgtcaaatgccgcatcggcgtggacgaccaggacccggcgcagagcctgttcgccacagtggacgcctcggccagggcgggggtttcgaccttcattgttcatgcgcgcaaggcctggctgaagggcctgtcgcccaaggagaaccgcgacgtgccgccgctggactacgccctggtgcgccggctgaagcgcgagcggccgcatctgtcgatctcgatcaacggcgggatcgcctcgctggacgaggccgaggcgcacctggacgacgccgacggcgtgcggctggacggcgtcatgctgggccgcgcggcctatcacgagcccgccatccttggagaggccgaccgtcgcctgttcggagaggacggcggggacatcgacgcctttgcggccctggagcgctaccgctcctacatgggcgcgcgcctcgccgaaggggtcgggctcgcctccatgacgcggcacatgctgggcctgatgcacggccgaccgggcgcgcgcgcctttcgccgcatcctgacggtggaggcgatccggccgggcgccgggctggaggtggtggaccgcgccgccgaggccatgcgcgaggcggaaagccgccgggatcaggccgcctgagcgtgcacgcaagcttggctgcaagcctccggtaagggctggatggtaaacgggtgtccggacgccctttcttcccctccggagcccccatgatccgcctcgcccgcgcggccgccgtggccgccattctcgtcgccgcgcctgccgcggccctcgctcaggttcccggccccatcgccgtcggcgcccaggtcggcacgcctggcctcggcgccaacatccagttcgcgctcaacgacgtggtcgtgctgcgcggcggctatgatgtgctgcagtgggatcgcgacgacagctatcaggacgtcgactacaacgccgagatcgacttcaagtcgccgggcgcctttgtcgacctgcacccgttccgcaacagcttcttcgtgtcgggcggcgcctatttcggcgatcgcggcgtggagctggacgccacgccgacgcgcgacgtgcgcatcggcggcgtgaccttcactccggcccaggtcgggcggctggacggccgcatcgacctcgaggacaccgctcccttcgccggcatcggcttcgacaacacctttacgcgcggcggtcggctgggcttccgcttcaccgccggcgcggtgttcggcgatgcgccggtcgtgaacctgcaagccagcggcgggaccttctccgacaatccgatcttccaggagcgcctgcgccaggaagaggccgagatctaggaagaggccgacgactacaaggtgttgccggtcgtgcagctgggcctgaactaccgcttctgagaccgacgggcggggacaggatccggccggcccgctagaaggcgggcatgaccgccctgcccctgtcagaactgatcgccttggtcgcggccctggccgccgccgggctggtcgggggattgatcgccggcctgttcggcgtcgggggcgggaccgttctggtgcccgccctcttctatgccttcgaggccctgggcgtgggcggcgaaggcaatctgcacaccgccatcggcacctcgctcctgaccatcgtcgcgacctcctggcgctcgctggccgcacaccgctctcatgccgcggtggacgaggcggtgctgaagggctggacgccctgggtggcgctgggcggactggtcggcgcggccctggcggggatcaccagcatgggtgggctggcgatcgtctatggcgtgtgcctgacgctggtggcggcgcagatggggctcttgcccgagcgcatgacgctgcggcgcgacctgccgaccggctggggccggcgcatcatcggtggtctgatcggcatgctgtcggccttgatgggggtgggcggcggcagcttcggcggcatgactatgaccctgtgcggccggccgatccaccaggcggtggccaccgcgtccggcttcggcgtggcgatcggcgcggcggcggcgctcgggttcgtggtgttcggctgggaggcgagcgggcgcccgcccttttccctcggctatgtgaactttccggcggggctgatcctcggctcgatcacagtgctgacggcgcccttcggcgcgcggctggcgcaccgtatgagccggactctgctcaggaaaaccttcgcggtctatctgctggccactgcggcgtcggtgttgatcaaggcgctctagcccggggatgaccccaaagggcgcacggctttgccacattctcgcctcatcccctaccgacaaggcatgcgtcggctgcgttgggggccggggtctccgcgagacaagtcgatgatcggcacggccgctgcgttcgccatgctctgggcaatggtgtttcccgtcactgatgcgtctgcatccgacggtcccatcccgtacgaagccgcagtcgctgcggactcgaacaagagcaaaacacccgatgcgagcatcggttccgacgaacaagcggccggcgaagatcacgctctggacgcgcagcaagccgaactgatggacggcgatccggattggcgcccgtcggcgcgcctttatcatgcaggcggcggcggcgcgacggggcgggattcgctaggttgccagccaatcgccatgcgcaccgtggccgtcgatcccagggtcattccccgccggacccgcctgttcatccgcgaaacggtcggcatgcgcctggccgacggcacgcgtcacgacggctactggtacgcctccgacaccggcggcgcgatcaagggccagaaggtggacctgttcaccggccatggccgcggctccatggcccaggctcagcgcctcaacatgcgcaccctaacggtcgccgacgccggccgcttcgacggctgccccccggcctgggaaagcgcctccaactaagacttaaggtattcttcccgtcatcctcgcccttgtggcgaggatccatagactcgagcgtctgtcggcgagctgggttgcgaagttacctcggcgtcctggcgcaactggccaggatcgggagtctggatcctcgccacaaggacgaggatgacggttatgggtcaggcgccggcgctggctgctctacggtccgacaagccgcgccagctttagaagcgccgcttgccgctgatcgtctcgaagaacaggcggaagtcgcccatcaggctccacatcggatactggaaggtcgccggccggttcttctcaaaggcgaaatgcccgacccaggcgaagccgtaacccagcaccggcatggccagcagccaccacggattcatcgtcacgacggccagcagaaaggccgcgatcaccagccccgtgccgaccacatggatgcgccggcatgtccggttggaatgctggtggatgtagaaggggtagaaggcctcaaacgaagcgtagcggccttcgggcgtgtgcgacgggctcatggacgcgatgctgcgcccgcatgaggatgcttacaagcccgcccgccgtcagctcggccgcttgcctttgaacccgctcttcttgaagccgccttccttgaagcccggcttgggcttgaacggcttcttggcgcctgcatgggcgaagggcttgtcgccggcggggcgcggcgcgccctcggccttgggctgatacggcttcttcttgaaggccggccgagcctcgccgccctcgccttccgcccgcttgaacggcggcttcttggcgaacgggcgggcgccctcgccgtcctcgcgccgggcgcgcttgaacgagccgggggtgggggcctccgagggcgtgatcttgacctcctcgttggaggcggcgaccgcgtcgcggaacgccttttcatgcgatttggcgatctcgaagcgggtctcttccgggaaggtgcggatggccccgatctgcggcttggcgatgccgccggcgcggcagatcagcgggatcagccacttgggatcggcgttcctgttgcggccgatgtccatgcggaaccagaccacctcgtccggctgcagccgctcgcccggccagggcgtgggcgccagatcatcgccgccttcgccgcgcacccgctcgcgtcgctgcggctggcggtccgcgcccggatcggacagctcctccggcgccggcaggtcggcgcggcgcaagcggaccagggcggcggcgatctcttccggcgtgcgctcggcgatcaggcgcttggctaggatcatgtcctcgtccgtcacctcggcctcgaagaactcgggcgcgaccagccggtcctcatcggccttgcggatctggtcgaacgtcggcgcgccctgccacacggcctcgacgccggcttcggccagcagccgctcggccttgcgacgacgcgagtgcggcaccatcagcaccgagacgcccttcttgcccgcccgccccgtccggcccgaccggtgcagcagcgccgcccggttcaccggcagttccgcatggatcaccaggcccaggtccggcaggtccagcccgcgcgcggccacatcggtcgccacgcacacgcgcgcccggccgtcccgcagcgcctgcagcgcatcggtccgctcgcgctggcccatctcgcccgacaggctgaccgaggcgaagccccgctccagcagcgacgcctgaaggtgacgcaccgaatcccgcgtcgagcagaacaccatggcccggcccgcctcgaaccagcgcagggtgttgaccgtggcgtgctcgatctcgttgggcgcgatccgcagggcgcggtattcgatgtcgccgtgcggccggctcttgtccgtcgcgtcgatccgcaccgcgtcgcgctggtagcgcttggccagggtcgcgatctcgcgcgcgatggtggccgagaacagcagcgtccgacgctcgggcggggactgctccaggatgaactccaggtcctcccggaagcccatgtccagcatctcgtcggcttcgtcgagcaccagcaccttcagcgccgacaggtcgaggttctcgcgctcgatgtggtccttcaggcggccgggcgtgcccaccacgatgtggacgccgaagttcagggcgcgggcctccttgcgcgcatccatgccgccgacgcaggtggtgatcttggcccccgcctcggcatacagccagctcagctcctgggcgacctgcagcgccagttcgcgcgtcggcgcgatggccagcgccagaggcgcatcagccggcccgaaggtctcggcctccccaagcaggctgccggccgccgctagtccgaacgccaccgtcttgccagaccccgtctgggccgagaccagcaggtcctgctcgccatggccctccagcacggcggcctgcaccggcgtcggctcggcatagcccttgttggcgagcgcgcggtcgagcgcggggtggacggcgggaaagggcatcgggaacctggataaacgaacaaggcggccgcttgaaacgaccgcgcccggcgcaaggacaagcctcgggccgggcgggaagatgcgcctctatacacggatcaaggcgcgcgtgcggccgatttcgccgttcaccctgttccttcagccgccgttgagggcgtgcgaccaggatggcgcacgaaggagaccgtcttcatgcaggccctgtcgatcgccgccgccggcatgtccagcgcactgaaccgcttcgagacaggcgcgcgccgcaccgcgtccggaacgctggacactgtggcgcaggacgtcgtcgaacaggttcaggccgagacggccttcagcgccaacgtcgccgtcgcccgcacggccgatcagatgctgggcgccctgctcgacatcaaggtctgaagcggccccattgctgatctggccgaagcgacccaacgagcgtaaaagaacaacgatccgccaggaagcggacacacagcggagggacgaccatgacctacatcagcggcttcgtgacgccggtgaagcccgagaacaaggacgcctatatcgagtccgcgcgcatggcctggcccctgttccaggagttcggggccctatcgatgaacgagggctggggcgacaacacgcccgacggcaaggtcaccgacttccgccgcgcggtccaggccgaggccggcgagatcgtggtcttctcatgggtggtctggccggacaaggccacggccgacgcggccgaaggcaagatgatgagcgatccccgcatggagcagctgcccatgcccttcgacggcaagcgcatgatctacggcggcttccaaacgatcttcgaggcctaggagagaaccttctcccgcttgcgggagaagtggcccgtcgatcaggcgcagcctgatccagggtcgatgaggggagtcttcccaagccgaagacttcccccatcgtcagccgtgtcgcttcgctccacgtcgctgacacttcccccttagggggaagatcgcccgcgcctaccccgcgatctggccgaagtcggcgacgcggcccatgacgtcgcgcacctggcccagcagcttcagccggttctcgcgctcggcgggcacctcagagttgaccatgactccgtcgaagaaggcgtccaccggcgcccgcagacgcgccagcgccgtcatggcggcggcgaagtcctcgccgtccagcgcgatgtccaccgccgtccgcgccgccccgaccgcaaaggccagggtggtctccgcctccggctggccgggcaggcccgtctgcaccatgccggtcggcagctcgcccttcttggcctcggcccgcaggatgttggtcgcccgcttgtagcccgccagcaagttcgccccatcgtccgtcgccagaaacgccgacagcgcctccacccgccgcacgatccgcaccagatcatcgtcgcccagcgcgaatacggcgtcgacaagatcgtgccgttggccttggtcgcggaggaggaccttcaggcggtcggcgaagaaggcgaggacttcatcctggaactgccgtgttcgctcgttgatccagcctcttgcttcctggcgactacgttcctgatccgattgggagatgtactggcggagctctccggttaccggcatgaacgcataggaatggcgcgaaagcgttctcagcaccgcgcccagcgcaagccccgcctcttcactctcctcggcatccacagcaccagaaactacccgcgagaccattgaactccattcggtcaactcgctgtgaccaatgaagacaactcgcatcaccccttcgttgactagatcaaagaccgagatcatctcgtcatcgatctctggaagccggtctcgctcgaattctagttgcgtgcttggatcataaaactcgcgttcacgtgaaagctctcgaacgatccagtcgctcaagagcgtgcgcaaagatccgcgcgcaccactctccagaaccagtcggatcacccccagcgccgcccgccggagcgcataagggtccttcgatcccgtgggcttctcgtcgatggcgaagaagccgaccagggtgtccagcttgtcggccagggcgacggccaccgtcagcggcgcggtcggcaccgtatcgttcggtccctgcggcttgtagtggtcgcgcacggcgtcggcgatggcgtcccgaacttgcggcgtccagccccctccaccgctgcgcggttcccctcccccggagggggaggaataaagaacgcccggctctcccccctctggggggagtggccgcgaagcggacgaggggggctgatccagcaggcggacatagtagccccccatgatcccctgcagttccgggaactcgcccaccatgcccgaggccaggtccgccttggccagacgcgccgccgtctcggcctgatccgcgtccgcgccgaccagcggcgcgatctcgcgcgccagcgccgcgatccgctccatccgttccgccagggtgcccagcttggcgtggaaggtcacgccctcaagcttcttggaccacgcgtcgaagccgaccttctggtcttcctcccagaagaagcgggcgtcgttcaaccgcgcggacaggacgcggctgttgccagccgccagagccttgccgccgtcggacgcctcgacattggccaccaccacgaagttcggcgccagcccctccttcgacagatcgcgcacggcgaaatacttctggtgcaccttcatcgacaggcgcaccacctcgggcggcagcgacaggaactgcgggtccatgtcgcccaggatcggcgtcggccattcggccagccccgccacctcgtccagcaggccgtcgtcgtcgaccaggctcaggccccgcgcggcgcagaccgccttggcctgttcgaggatgcgcagcttcctgtccgccgcgtccagcagcacgtattcggcctcaagcttcctgcggtagctggcgaagtcgctggccgcgaacggcgcccccgatcccaggaagcggtgcccttcggtgagcgcatcggagcggacgccgtcgatctcgaacggaaccaccgccccgtcgaagacgcacaggatgcgcttgatcggccgcacccagcgcagcgttcccgtgccccagcgcatcgacttgggccaggggaaggcgcgcaccaccgcatcgaccatctcggccacgacctcgggcgtattgcggccctgctggctcacttgcgcgaaccagacgccgtcgcgttcgaccagttgatcggcgctcaggccggtctttcgcaggaagccgtccagcgcctgctgaggcgccgaggtcttcggccccttcagctcctcgttgcggtccggcgtcgccgccggcaagccgtcgatcaccagcgtcaggcggcgcggcccggcataggtggtcagcgcctcccacgtcaggcccgccgcgcgcagccgctcggacgccatccgctccaggtcgcgcgccgcgccttgctgcatgcgcgcggggatctcttccgaaaagatttcaagcaggagttcgggcatcaggcgctcgcgcgttcggattcgatctgggccagcgcgcaggctttgcacaggtcgcggatgcggccgatgtagctttgccgctcggccacggcgatggcgccgcgcgcgtccatcaggttgaagagatgcgaggccttcagcacctggtcataggccggcagcaccagcgcctgaccctgcggcccggtcatggcgagcaggcgcctgctctcggcctccatgtcctcgaaccggcgtttcagcccgtcgacgtcgtaaccgtggaagttggcctccgactgctggcgctcgttctccaggaacacctcgccgtaggtggtgccctccttggtgaacttcaggtcgtagacgttgtccacgccctggacgtacatcgccagacgctccagcccgtaggtcagctcgcccgagaccacgtccacctcgatgccgccgacgccctggaaataggtgaactgcgtcacctccatcccgtcgcaccacacctcccagcccaggccccaggccccgaccgtcgggttctcccagtcgtcctcgacgaagcggatgtcgtgcagcttgggatcgatcccgatcgcctccagcgacccgagatacagcgcctgcagatcgtccgggttcggcttcaggatgacttgatactggtagtaatgctgcagccggttggggttttcgccatagcggccgtcgccggggcggcggctgggctggacgtaggcggccttccacggcttgcggcccagtgcgcgcagcaccgtcgccggatgtagggtgccggccccaacctcgatgtcatacggctgcaggatggcgcagccctggtcgccccaatagcggtgaagcgtcaggatcaggtcctgaaacgcgagcggttcggcgggagcggtcaaggcgggtccgggagggtgcgaaaaagacggcggaccatagggcccgccgcctttgtcatcaacacgcctgcggccgagggccgggctcaggcgcccggggtggtcgtgggcgcgtcgtccgccgcatcggcgggagcgtcggcgtcgtcagtgtcatcaccgtcatcaacagggtcggcatcgacctggccgtccgtcgggttggagaccggcggcgaggcggtggtggtcacgtcgtccgtcggctgtccgttcggcgccgtatagggcggcgtctcgctgcccggctggcccggagcggccggcggcggggtcacctccggatcggtcggcgagggctgagcgtcatcgtcggcgtcgtccgtcggatcggtcggctgcgtccactggttcggctgggcgggcgcaggcggcggggtgatgtctggctggtccagcggcgtggtcgactgggtgttgggcgtggtctgctcgccggccggcgggctggcgggcgcggtcgggtcctgcgccagggcggcgggggcgatcagcagggcggctgcggttgtggcggcgaagatctgcttgcgggtcattggacggcatcctttcggtttacggaagaccgcgtccgaggagaggcgcggcccgttccaccttggggaactgcgggattcaaggcgtcatcatcgacgcggttccgcgatcgtgaaacgatttgaaacattcgtgaggatcgtggcggagcggtgttcgacctgccgcaagctgcaccgaaaaggcgtgtttccgcccggtttggcgtagtttcaggggttcagccgccccgccgccgtccaccagtccggatgatgaaggcgcagcacgtccgcggccttcgacgcgtctgcatcggtgtcgaacaggccgaacaccgtggcgccggagccggacatccgcgtcagccgcacccccggcgcctcggccatggcggacagcgcctcgccgatgcccggcgtcagcgcgagcgccggcgcctccaggtcgttgcgctggtccgccaaccagtcgatcaccgcgctccggctccagccggccggcggggccggacgatcggcctgcgccgtcgaccccgcatcataggcgcggtagaccgcccccgtcggcgagggcaggcgcggattgagcagcaccaccggcagagacggcaggcgcggctcgtccgtcagcacctcgccccgtccgccggcccaggccgtgcgcgccctcaggcacatcggcccgtcggcgccgaccaccccggcgatccgctccagcccggcctcgtcgatttcaagcgccagcacttgcgccgccaggcgcagggccgcgcccgcgtccgacgacccgcctcccagcccggcggcgatcggcagccgcttgtccagcacgatacgcaacgacggctctccgacacccgccgcctcggccagcgcccgcaccgcccgcaggaccaggttgtcgtctcccgccaacccttgggcgaaaggccctacgacctccagcgtcagccggtcggcgggctcgaccgtcaccctgtcaccgatgtcggcgaaggcgaccaggctctccagcggatgatagccggcgtcgtcgaccggccccacgtgcaggaacaggttgatcttggccggcgccagggcgtgcaggtgcatctggtggacggccgctaccgcgacacgcccgtagaggccgcgccgccgtccggcagcccccgctccagcttggtctcgacgccggcgcggcgctcggcgtcgggctcgagcgtcagcacgcgctcccactgccattcggcctcgcgctggcgaccgacgcgccaataggcgtcgcccaggtgatccacgatctcggcgttggccggctccttggccaccgcctgctccagcgtggcgaccgcctcgtcgaaccggccctggcggaagtgggcccagcccagcgagtcctggatgttgccgttgcggggctcggcggcgtgggcgcgggcgatcagggcggccccctcctcgacgcgcagtcccctgtccacccacagatagccgagatagttgagcatgttggcgtcgttcggcgccgcctgaagcgcggcccacagctcggcctccgcttccggaatgcggcccagcgactcataggcggcgccccggatgaaacgcacctgcgccccctgatcggccgtgttcagaaccggaccgttcaggatcgccagcgcctcgtcgtagcgctcggcctgcgccagctgcccggccagcaccagggcgatgcgagggtccgacggcgcggcggcggcggcgcgacgcagctcctgcagggcgtcctcgggtcggccgtcctcgtccagcgaaatggccagttgggtgcgggcgttggcgaacaggaccggatcctctgttccgacctgcgaccaggcccggcgcgcctgatcgtccagcccggcgcgagtcagcacctgcgccagccgcgtctcaccttgcgagttgcgatcaaggtccagcgccagccgcagatacacggcggcgaactcgtgcccgccctcggccgaggcttgcgccgccgccgccgacatcgcctcggccgcgccttctctcagggtgggcatggcgggcgcgcgccccctcgcctcgacccgctccagcgcgcgggccagcgccaggtccagttcgttggccttggccgccgcctcatacagggcgcgcgcctcatcgcgccggccgcgccgctccaggaactcgccgtaggggcggcggaacaccgggccggtgatggcgccctcggtcagggacttcagctcggcttccgcctcgtcatagcgccgccgatgctccagcagcagggcgcggttctggcgcacgaatgcggtggtcgccggatcggcgccttgcggcggcggaaccagggcccgctcccagtcgccggccgccgccgcgatccagggcgagatcaaaagggccgcgcgggcgtgcggcgcgccgatcggctcggccgccaggctggcgttggcggcgcgcgcatcgcccgtcgcaaaggtctgaaccacctgcaccagccgcccgccctggaccatcgccggcgagccttcgcccggagccagcgcggccgccacgccaaggtcgccggtcagcagggccgcggtgaaggcctgttcgcgcacccggggctgttcgggcgtcagcgcctgggcttcggccagatagcgcgcgcccagctcgccctcgccgcccaccaccgccgccttgcccgccagataaaggccgtaggcgctgcggtcggaggcgtcggtcgggaccggcgcccactcggcgggaatggcgggctcggacggctcggcctccgcatcctcatccgatgcgtcaggcgcgacgggggctgcgcccggcgtgttgtcgggcgtaggctcctcgcccgaggcgggattggcggcgggcggcgtctcgacaggcggagcggacgcgggctgctgcgccgcggcgccggtcgcggccagcgacagcagaacggcggaacacaacaggcgggcgcgaagggtcgacatggccgaaacccttcacgttttgcccggccgccgcaagggccgccgcaccgccggcctcacatgttcggatagttggggcctccgccgccctccggcgtggtccagacgatgttctgcgacggatccttgatgtcgcaggttttgcagtgcacgcagttctgggcgttgatgacgaagcgcggatcggccttgttggcctcgtcctcgtagaccacctcgtacacgccggccgggcaatacagacgcgccggctcgccgtacttgggcaggttcacccggatcgggatcgagggatcgatcagcttcaggtgcgccggctgctcctcggcgtggttggtgttggagatgaagacgctggacagcttatcgaagctcagaaccccgtccggcttgggatagacgatgggcttgtgcctggacgcctcttcggtcgaggccgcgtcggacttgccgtgcttccaggtgcccatcggcgaccagccgccggtcaggtggttgatccacatgtcggccatgctgacggcgccgcccagcatggtgccgaacctggacaggatcggcttggcgttccgcacgatcttcagctctcgcgcgacccagctgttttcataggccgtctgatattcctccagccggtcgccctcgcgcccggccgccacggcgtcataggcggcgtcggcggccatcatgccggacttcatggcgttgtggctgcccttgatcctcggcacgttgacgaagccggccgagcagccgatcagcaccccgcccgggaagctcagcttcggcaccgactgatacccgcccgacgcgatcgcccgcgcgccataggagacgcgggttccgccctccagatgctcggccaccgccggatggtgcttgaagcgctggaactcgtcgaacggcgacagaaacgggttcttgtagttcaggtgcaccacaaagccgatcgccacatagcggtcgccgaagtgatacatgaacgacccgccgcccgtcttgtcgtccagcggccatccggtggtgtgctgcaccaggccgggccggtgcttctcggccggcacctgccacagctccttcaggccgatgccatacttctgcggctctgccgtgtcgcacaggttgtggcgggccatgatggtcttggccagcgagccgcgcgcgccctcggcgatgaagacgtatttgccgtgcagctcgatccccggctggaactcgccggtcggctggccgtgcttgtcgatgccgaacacgccggcgaccacgcccttcaccctgcctgacggttcgtcataaacgacgtggctggcggccatgccgggatagacttcgacgcccagcgcctccgcctgctcgcccagccagcgcgacaggttggccagggacgcgatgtagcagccgtggttgtgcatgaacggcggcatggcgaaggccggcagggtcgtctgcccctgcggccccagcaccaggaacttgtcctctgtcaccggcgtctccagcggggcgccgcgctccttccaatccgggaacagctcgttcagcgccttggggtcgatcaccgcgccggacaggatgtgcccgcccagctcggccgacttctccagcaccgccacggtgatctcgcgcccgtccttttccgcgcgctgcttcagccggatggcggccgacaggccggccggtccgccgccgacgaccaccacgtcatattccatgacctcgcgctcgacgccggccagcgcctccagcgggggcagattgtcgatgatcgcttcctggcgcgcgttcgccgcgccgccttcgatcgtgtcctcggccatgcctgtccttcttttccccgtcgcgggaatggtttcaccgcttatcggaaggtgacgcggcggcggtcaaggcttatccctgccctcgtccatgaacgcgcaaccccaagaaacggccgccgtcgaaagcctgctcgccttctggcgcgatgcgggggtggacgcctgctacctcgatgcgccggtggaccacacccatgtcgagctgccggcgcccgccaaggcggtgcagaaggcgaccgcctcggtggctccgccgccgtgccgcgacaatgcggcgcaagaggcccgcgcgctcgccgcctccgccgccacgcttcaggacctcgccgccgccatcgccgcctttgacggctgcacgctgcggggcctcggcgccacccagtcagtgttcgcgcgggggaaccccgacgctcccgttcttgtgatcggcgaagcgccgggcgccgaggaggatgttcagggccggccgttcgtaggcaaggccgggcagctgctggaccggatgctggcggcggcgggtctgacggataaggtcttcatcaccaacaccgtcttctggcgcccgcccggcaaccgcacgcccagcccgcaggaacaggccgcctgcgccccgttcgtcgagcggacctttgcgctgctgaagccccaggccgtgctgctgctgggcgcggccgccgcccgttcggtgctgcagaccgaggacggcatcatgaagatgcgcggccagtggcgcgaatggcggctgaacgaaggcgccgtcgcggcccccgccatgccgacgctgcaccccgccttcctgctgcgccagcctcaggccaagcgtcaggtctgggccgatcttctgacgctcgctgttcgcctggaaggcgaaagccatctttccgccggaattgaaggtaaacgctgattacggcatgtttcgccgctgacgaccgatcgccatacgaacgcgccgcctgatcgagacaggcaggcgcgacgccaacgagggggccgctatgctcaacttccgccgcgcgcttgtcgcgtcgacgttcgcctttgccctgtccgccgccggcgcggccatggcggaaggggtcccttacgaaggttcaggcgctggctccggccttgtggaaggaatgtccggatcgggcgtcggttccatgcgcccgacggcgttgagctcggcggaccgcatcagctacaccaccgcctttgacgccctgcggcgcggcgacctggaagccgcccgcgcctcggccagccaggcgcaggatcgcgtactgatgggtcaggtcgagttcgagcgcctgtttcaccgcgaccattccgcgacctacgacgaactggtcgcctggctgagcgagtacgccgacctgccgtgcgccagccgcgtctataacctcgccctgaagcgccagcccgacggcgccgccgagccgccgcgcccggccggcttcggccgcacctggaacagcctggtcgccgccgtgtccggcgacagcggcgtcgatcccgacaagatcgcccgcgtcgcctacaacaacgacgacctctcgggcgcggtgcaggccggccagtcgatcggcgactggtggaccgtgggtctggcctcctggcggctgaacgacttccaggcgtccttcagcgctttcgagcgcgtggcgctggacccgaccgaggacccctgggttcgcgccggcgccgccgtctggaccgcgcgcgccgccgcaaagaccggccgccaagaccgcatcgccgaatacctgcgcctcgccgcgcgctggcccgccactttctatggtcagattgccctgcgccagttgggcgaggagccggtcgtcgagaaccagggtccgcgcgcctacaacgccgtgatgcagcaggcgtcgttccagcaaccggagccgctgggtgtcgaacccgccgccctctcgacctttcttcagggcgacgcgcgcgcccgccggaccctggccttctacgaggtcggccgacgcgacgacgcgcgcagtgaactgcgccagggcctgcgcaccgccgccggcgacaccgcccagaagatgtggggcgcgctcgcccgcatgatgtcgcccggcggatcgggcggcgacgccggccgcatcgatgcggtgcactatcccactccggatctgcagccggagggcggcttcaccatcgaccgcgccctggtctacgccctggcgcgcaaggaaacaggcttcgacgcaggcgcgcgttccggcgccggcgcctacggcatcatgcaggtgatgccgaccaccgccgccgagatgaccggagaccggggcttcgtgtcacagccctcgcgtctgctcgacccggccgtgaacatgaagctgggccaggcctatatccagcgcatgctgcagctgaacgccttccagggcgatgtcctgcgggccgtcgcgtcctacaacgcaggccccggtccgatgctggcggcgctgcgcaagctcggcggcgacgccgatccgctcctgctgatcgagaccatcgacgtgccccaggcgcgcgactacgtcgaaaaggtcatggcgtcctactggatctatcagcgactgctgggcggaccgctgaagacgctggacgcggtcgcctcgggcgcctcgctgatcccggccgcgctggaccatgtgcagcccgcgccgcagacgctgactatcgccctgatccgtacggcggccgttcagtaggcccgtctagaacagcgcgctgagcagcaggctccagaaacacaggctgacgccaagccccaggccatagcccgcgatggggttcagcagccggcccgcgggcgcgtccgcgctcttcaccgcctgaacctgcattgcgccctccgcgtcgccgtcgatgaagatcgaataacgccgtgcggttaagcccgcgtcggcgacaatggttaagcttggatcgctgccagcgcctcggcctcccactgcaggaagtccggctgagccagcagcgtctccacataggcctgcgctacgccgtcgtcgccgtgcgcggccaggtcgatgccgaagtggcggatgcgcgccgcggccggcgtgaagaaggcgtccgggatcgaccacccgccgaacagatagggtccgcccgcgccgaagcgctcgcgcatctcgccccacagggccaccaaccggcgcacgtccttctccagccccgcgtcctgcggcgcgggcgatcggctgtcgcccaccatcgggtgatccggccccatgccgcagacggtgcgcaggctggagaaaccgccatgcatctcgcacgccgccgaccgggccagccagcgcgcatgcgcatcgcgcggccacagcggcgcatcggggtggcgctcggccgcccagacgcagatcgccatggagtcccagatggtgacgccgtccaccttcagcgccggcacgaagccggagggcgaatgctcggcgatccgctcggccgtgtccggctcgttcagccggaccacgatctcctcgaactcggccccgcagcgtttcagcaccagccacggcctcagcgaccaggtggaataggccttgttcccgatcaccaactgcacggcgcgcctccttttgatgcaggggttcgtgccctgcatcggctttccgggcaagctcgccttgactccaccccggcctcgaccgacacgacgcgtccatgatcacgcgctattcccgccccgacgccgtcgccatctggtcgcaggagaccaagtacaagatctggttcgagatcgaggcgcacgccgcgacccgaatggccgaggtgggcgtgatcccgcgcgaggccgccgacgccatctgggccaagggcggggatgcgacgttcgacgccgaccgcatcgacgagatcgagcgcaccaccaagcacgacgtcatcgcctttctgacccacgtcgccgagatcgtgggcgacgaagcgcgctttctgcaccagggcatgacgtcctcggacgtgctggacacctgttttgcggtgcagctggcgcgctccaccgacctgctgctggggggcgtcgatcgggttctggcggcgcttgaggcgcgcgccaaggagcacaaatacacgcccaccgtcggccgcagccacggcatccacgccgagccggtgacctttggcctgaagctggctggctaccacgccgagtttcagcgcgcgcgccgtcgcctcctcaccgcacgcgaggagatcgccacctgcgccatctcgggcgccgtcggcaccttcgccaacgtcgatccgcaggtcgaagcctatgtggccgagaagatgggcctggaggtcgagccggtctcgacccaggtgatcccgcgcgaccgccacgccgcctacttcgccgccctgggcgtcgtcgcctcctccatcgagcggctggccaccgagatccgccacctccagcgcaccgaggtgctggaggccgaggaattcttcgacaagggtcagaagggctcgtcggccatgccgcacaagcgcaatccgatcctgaccgagaacctgaccggtctggcgcgcctggtgcgctcgtccgtagtcccggccatggagaacgtcgccctgtggcacgagcgggacatcagccattcgtcggtcgagcgcggcatcgggccggacgccaccatccacctggacttcgccctgcaccgcctggcgggcgtcatcgagcggctgaacgtctatcccgacaacatgcagaagaacctcgaccggctgggcggcctggtcttctcccagcgggtgatgctggccctgacgcaggccggcgtgtcgcgcgaggacgcctatgcggccgtgcaggagaacgccatgaaggtctggcgcggcgagggcgcctttatcgacttcctcaaggccgatccccgcgtcaccctgcccgccgaccagctcgaggccctgttcgacctcagctaccacaccaagaacatcgacgtgatcttcgaccgggtgttcggggacgcgtgatctaaacggtattgaaaaccgcaccggatttcgtaccttgaacggatgcaacgcatcgaagcccaagtcgccgtcagcgtctccgatctgaagagaagtccgagcgccgtgatggagaacgccggcggcgagaccgtcgcggtgctgaaccacaatcggatcatggcctatatggtgccggcggctgcatacgaggcgatgctggagcgtctggacgatctggcgctggtcgagacgatccgggcgcgcgccgacgaaacgccgctgcgcgtctcgctcgatgagctttgaactccgctttctgccctccgcgctgaaggagtgggaaaagctcggcgtgtcggtctgcgatcagttcaagaagaagctgatagagcgtctggagcacccgcgcgcgcccaaggacgcgctccacggcctgagcgatcactacaagatcaagctaaggagcgcaggctacaggctcgtataccgggtggaggatcaggctgtcaccgtgacggtcgtcgccgtcggaaagcgggagcgtggccgcgtctactccgacgccaaacggcgcggatgaaggcgaacttcccgccggtcgtcgatgcgggcacgcgcttgctgatcctgggcagcctgccgggcgatgcgtcgcttaaggccgcgcaatactacgcccatccgcgcaacggcttctggcctctgatcggcggggtggtgggcgaagatctggtcgcactgccttatgaccagcggctcacgcggctgctcgcgcacggcgtcggcctgtggggtgtgatcgcctcggcggaacgggcgggcagtctggatgcggcgatccgctcgcccgaggccgccgatctgcgcggtctggtcgccgccctgccgcatctgcgcgcgatcgccttcaacggcggcctggccgctcgtatgggccggcgtgttctggcgcccgtgaccgacgtcgccctgatcgacctgccgtcctccagccccgcccatgtccggccgctcgccgacaaggccgccgcctgggccgtgctgaaatcggcgctgtcctaggctcgcaagaaaattcgcctgctgcgattttttggggaaaccaaagtcaggcgcccgtgttctcaaggggcgcgagacgcaaacacgccgggtgagacatccccccaacgtccccggctaaaaagaaagggccgcactttcccccgggtgcggccctttcgactttctgaaatggactgtaagccctactcgccggcgcggatctgctcgcgcgcgatggacatcagctcgtccatctttgaccggatctcgccttccgacaccgtcaggcccgagcccttgaagtcgccggccaccttgcggaacacgtcttcctcacccggctgttcgaagtcggcgcgcaccacggcgctggcgtactgatcggcgctttccggcgacaggcccatcttctcggccgcccaaagccccagcgacttgttgcggcgggcgacggccttgaattcctgttcctgatcgagggcgtacttggcctcatagcccttttcccgatcgtcaaaggtcgtcatctaggtccgcgaagctccacaatccggttcaaaaccggaacaagcgccgtctatagcccgccctcgcccgaacgcacccggacttacgtcgggtgaagcccttgtgtcacaggcaagcccggacccggcgcccgcgtccctgtcatttgtgctggcgcgcggcttcggctaaggaaccgccgcaggtccaacgcccgcccgaccggttcttcagacgcgtcttcccttgcggctttcgcagcctcgggcggcgcgatttttgtttccggcgggcgacaatccccaaggcccgtccgggacagactgatgaacaccaagcgcaagaagctctacgagggcaaggccaagatcctgtacgaggggcccgagcccggcaccctgatccagtacttcaaggacgacgccaccgccttcaatgcgcaaaagaaggcgacgctcgagggcaagggcgtcatcaacaaccagatcagcgaattcgtcatgtcgcgcctgaacggcatcggcgtgaccaaccacttcatcaagcggttgaacctgcgcgagcagctgatccgcgaagtcgagatcatcccgctggaggtcgtgtgccgcaacatcgtcgccggctccatgagccagcgcctgggcatcgaggagggcacgcccctgccccgctccatcatcgagttctactacaagaaggacgagctaaacgatccgatggtgacggaggagcacatcaccgccttcaactgggcctccacccaggagctggacgatatcctggccatgaccgtgcgggtcaacgactatctgtcaggcatgttcggcgcggtcggcatcaccctggtggacttcaagatcgagttcggccgcatctgggagaacgacttcgcccgcgtgatcctggccgacgagatcagcccggattcctgccgcctgtgggacgcgaccaccggcgagaagctggacaaggaccgcttccgccgcgacctcggcaacgtcatcgaaagctacaccgaggtcgcgcgccgcctgggcatcatgaagggcatgccgacggtcatccaggggggactgcactgatggacggcgtgcgggagtccggatcaacattcgacgtttcctccacctctcccgctcgcttccgccgcttcggggcggccggcccgatctatgaggtcgaggcggtggaccacgaccaggcgcgcatccgcgtcgtcgagagcggggaagctctggattatccgcttacggcgctgctgagcgacccccaggcctgatgttcgccattgccttcgatctcgtggtcgcggacgcccaggtcgtccatcctaagggcgtgacccaggcctatggcgacatcggaactaccctggcgcgttacggcttccggcgcatacagggcagcgtctatgtcgtcgaagatgaagacctggccaatctgctgcaggccatgaacgccctcaaggccttggtctggtttccgcagtgcgtccgtgacatacgcgccttccggatcgagcaatggtccgacttcacatcgttcatgaagggcaacctatgaagatcaaggttcacgtcttcctcaagcccggcgtgctcgacgtgcagggcaaggcggtcgagggggccctgcacggcctgggctggaccggcgtcgccaacgcccgcgtcggcaagctgatcgagttcgacctggacggcgtcgaggatccgcaggccgaagccaggaagatgtgcgagcagctgctcgccaacaccgtgatcgagagctaccgcatcgaggcggcgtgatgagcttcaccctttcctccaacgacatctccgacggcggcgtgctgccggacgcgcaggtcaaggccaagggcgatgtgtcgccgcatctggcgtggtccggcgcgcctgacgggaccaaatcctacgccgtcacctgctatgatcccgatgcgccgaccggttcgggcttctggcactggaccgtggccaacatcccggcggacgtgagcgaactcgcgaccggggcgggctcggccggcgggcatctgccgatggcggcggtgcaggggcgcaccgactatggcaaggcgggatttggcggcgcggcgccgcctccggggcacggaccgcaccgctacatcttcacggtcttcgcggtggacgcggagcggctggaggtcaccgccgacgattccggcgcggtgttcggcttcaacctgcacttccacaccctggcgaaggcctcgatcaccgcgacctatgaagacgtcggcgagggctgagcccgcatatggtgcaaagacaaagggccggcggagcgatccgccggcccttttcttgttcaggcgatcgccctgacgatcagcgcatcagcgactggcgcaccaggccgaacgaccattgctgggcgtcataggcgtcgcgcaccacgtcggccatcgagaagaactcgtgcaccgcgccttcgtagttgcggcgctggacctggacgccggcgttgcgcagcgccgtctccagcgtcgcgccgtcgtcacgcagcggatcgatgtcggcgttgacaatgatcaccggcggcaggccgcgcaggttggcgccgatcagattgtagcgcgggtcctgctggaaggccggcgacggcagggcgtattggccgaaccagcccagcgtcgcggtgcgcagcggcaggctggcggtgttcatctgcttggacggcagctgcgggtcgccgttggcgatcgggtaaaccgacaggatgctcttgggctgggtccagcccatgtcgcgcgccgagatggcgacgttcacagccaggttgccgccggccgactctccagccaccgcgatgttgttggggttcccgccccacgacgcggcgttctgcagcacccactgataggcggcgttggcgtcctcatgcgcggccgggaccttgttttcgggccccttgcggtactcgaccgacaccacgatggcgttcaggttgcgggccatggagcgcggcgtcgcgtcatagacgttgatgtcggcgatcacccagccgccgccatgatagtagaccacgaccggcaggttcgagcccgtggcgttcgcgggcttgtagacgcgcaccggctgggtcgttccaccggtcggataggtcaggtcgcgcgtggtcaccgtcgcgtccggcgcggtgggcatgttgcgcatctgcttgaccttcatcaccgcgtctgcgggcgaaggctgggtgcgggcctgctggaccgtcagggtctcgatcggcttggcgcccaaggcggcgtgagcgtccagaacggcctgcatgtcggcgtcgggacggccgctcatgcccatgggggcggcgggtgacggcatgggcgcggcgggcgtcgccatctgcgaggaggcctcgcccatcatcggcatcgaggagcaggcggccagggtcgcacccagggcgacggaggcggccagagccagcggtttgatctgcatggtgtttgtcccggtagaggttcgggcggaagaaccaccagcgatcattgttgttccgaaagaggtcacatttcgtgatcgagcgaccggcggcgcgccatcttgcagctggatgaacagcgtttaggtacgctcctctccacaactctccagcctgaggtgcagcttggctgtcagcccgcttccaccgtctgcccaggcgccgtccgcttcgccgccccgctcggccaaggccgtgctgttcgccctggccatgggcggcttcgccatcggcaccactgagttcgccgccatgggggtactgcccgagttcgcgcgcggcctcggcatagacgagccgaccgccgggcacgtcatcagcgcctatgcgctcggcgtcgtggtcggcgcgccggtgctggcggtgctgggcgcgcgcatgtcgcggcgggtgctgctgatcgtgctgatggcgatgttcgccgtcggcaacggcttgtcggcgctggcgccgacctatgagtggatgctcctgttccgctttctggccggcgtgccgcacggcgcctatttcggcgtcgcctcgctggtggccgccggcgtggccgcgcccggcaagcgcagccaggcggtgtcgcgtgtgctgctcggcctgacgatcgccacggtggtgggcgtgcctttcgccggcttcatcagcctgatgttcggctggcgctggaccttcgccattgtttcggtgctggcgatcctgaccatggccctggttcacgcgcttgccccgcgtgatccgccgcagccgggcgccagtcctttgcgcgaactcggcgcgctcgccaatcgacaggtctggctgacgctgggcgtcggtgcgatcggcttcggcggcatgttcgccgtttacgcctatgtggcctccaccctgacggcggtgacaggcgtgggcgccgaggtggtgccctgggcgctgggcgtgtttggcctcggcatggtggccggcaacatcgcgggcggcgtcctggctgatcgcttcggcatgcgcgccgccgccatgctgctggtatggagcgccggctggatggcgctctatcctctggcgactccggctctgtggtcgatcctgatcgtggtgttcatgatcggcgcgggcggcggtctcggcaccgtgctgcagatgcggctgatggacgtggcgggcgaggcccagactttagcggcggccctcaaccattccgccttcaacaccgccaacgccttggggccgttcctggccggagcggccatcgccgccggatggggcctgccgtccacgggcgcggtcggctgcgccctgacgctgggcgggctggccgtctgggggatcgcctggtgggacggacgccgcgcgcccctggtcgctgacaaggcggcgcaacagtgctagagggccgcccatgagcgccgccgtcatcgtcttccccggatccaactgcgaccgcgactgcaaggtcgccgtcgaacgctccaccggcgagcacgtcgagatggtctggcacgccgaaaccgaactgccccgaggcctcgatctgatcgtgatcccgggcggcttttcgtatggcgactatctgcgctgtggcgccatggcggcccagtcgccggtgatgcagacggtcaagaaggcggcggacgacggcgtggccgtggtgggcgtctgcaacggcttccagatcctgtgcgaggccggcatgctgccgggcgcgcttctgcgcaacaagggcctcaagtatgtctgcaagcccatcagcctgacggtcgccaacggccaaacccgcttcacctccggctatcagggccagcgcgaggtggtgatgacccaaggcaacggcgacggaaactacttcgccgatcccgagaccctcgcccgcatcgagggcgaaggccaggtcgtgttccgctatgtcgacaatccgaacggctcggtgaacgacatcgcggggcttcagaacgcgcgcggcaacgtgctcggcatgatgccccaccccgaccgcgcctttgaagccgaactcggctccgccgacggcgccgtcctgttccagagcgtgatggcggcggcctagggaagccgccctgatggtcacccgccgccgatgcggggggtttcttcgtcttcgtccgacagcccctgcacgccgacgctctggttcagggcatcctcgtcgccggcgttgacggagacgccgttgtccatggcctcgtcctcatcggcggtgcggtcgccgccggggtcgcgctgggcgttcagttcgcgctcgcccatgcccaggccctgctcgcggccgcgggtggcgtcgacctcattgggctgaaagccgtcggggttcaggccggtctggttgatgtcgccctgcgggctggtgacgtcggtcatggccgaagctcctttgtgactgtgatgaagggtcaaccggcgggaatgggcgcgggttccggctgaaccttcacgaggctcgggcgtaatgcagacccgcgttttacgcccgagtgttcccggagagccccatgtcgtccgtcgtccgccccagcccacagcagatgacgcgccgcgtggtggtgctggccgccgccgccttcgccatcgtggcgccggtgatccagatggcgaccggcttcggcctcgaccagggcgagttcgcggcccagggcgaccagaccctgcgcgtcgccggctacgccttctcgatctggggcctgatctatatcggcatcctggcctacgccgtgcgccaggtgctgccgcagacgggcgaaagcgacatgatccgtcgcttcgccatcccctccatcgtcgccttcgtcggcatcggcgcttggatcgtcgccgcggcggccgacgcgcggatcgccaccctggtgctgatcttcgccagcctgatcgcgctcctggttccgctggtggtgcatggcggcctgatccgcgcgctgggcaagggcgaccgggatcgctggttggtcgcctggcccctggggctgcttgccggctggctgacggtcgccgcgccgctgaacctcatcaccgtgctgacggcggagaacgccttgccgctggccctggcgcccaccggctgggcgatgctggcgatcgtcgtcgtggtcgccctgaccctcttcgtcaccgcccgcacacgccttctggcctatccgctgccggtcgcctggggtctactgggcgcctttgtggccgagcagacgcgcaatccgctgttgggcttctttgcgctcggcgccgcgctgctggtgctggtggtgtcgctggtgctggtgttccagctgcggccgggcgtcgagcgcccggccgcctgaagccggtcgtcagggcctggactgctccggatcgtccaactcgggctcgtcctgcacattgcggccttccgcgcccacgtcaaaggcgcccggatcgtcgaagccgatgctgccgacgccggtcgcctcgcccgctaaacgctgccggcggctctgcatcgcctgatcggccgccgaggcgtccatggcggccgtcacctccggatcgttggagcggctcatctgctgcccatccgccggggttgggtcggtcttggcgggagtgtcggccatcacacgccctccccgtccacgccgtcttcgtcgtcggcttcgttctgcgcttcctcggccatgccggaggcgccgacatcgtcggcggcaatgtcgggggcgttgtcgtcgtccggcgtggcggccgggtcgatgggctgatcggtcatggggctctccttggagtgggatcagaagaaccgcccgcgccgccccgatgttccgctctcctgctgacagtcgggcgcccacccgctagaagcgcgggccatgagcgcttcgcaaaagaccatggccgaactggccgccgaatacggcctggccccgaacgaatatcaggtcgtcctcgaccgtctggggcgcgagccgaaccaggtcgagctcggcgtcttctcggtgatgtggtccgagcactgctcgtataagtcgtccaagatccacctgggcaagtttcccaccaccggcgagcgcgtcatctgcggcccgggcgagaacgccggcgtgatcgacatcgacgacggcaacgcctgcatcttcaagatggagagccataaccacccctcctacatcgagccctatcagggcgcggcgaccggggttggcggcatcatgcgcgacgtttttaccatgggcgcgcggccggtggccctgctgaacgcgctacgtttcggcgatccgtcgcatgaaaagacccggcgtctggtgtccggcgtggtgtcgggcatcggcggctacggcaactgcgtgggcgtgccgaccgtgggcggcgagaccaacttccaccgcggctacaacggcaacatcctggtcaacgccatgtgcgtgggtctcgccaaggccgacagcctgttctactcggccgcgccggcgcccggcctgtcggtggtctacttcggctccaagaccggccgtgacggcatccacggcgcgaccatgtcctcggccgagttcgacgacgaatcggaatcgaaacgccccaccgtccaggtcggcgaccccttcgccgagaagctgctgatcgaggcgacgctggagctgatggcctcgggcgccgtcgccgccatccaggatatgggcgcggcgggcctgacctcctcctcggtcgaaatggccggaaagggcggcgtcgggatcgagctgaacatggacgccgtgccccagcgcgaagagggcatgaccgcctatgagatgatgctctcggaaagccaggagcggatgctggcggtcctgaagcccggccgcgaggaagacggctatcgcatcttccagaagtggggcctggacgccgccgtcatcggcgtgaccaccgacaccggccgtctggtgctgaagcatcacggcgagaccgtctgcgacgtgcccctggcgcccctgttcgacgacgcgccgctgtacgatcgcccctgggtccagccggagcttcagccacgcctggatcacgcgggcattcccgcgcccgagaactgggccgatgcggtgatgaaggtcgtggcctgcccggacatggcctccaagcgctggatctgggagcagtacgaccgccacgtcatggccgacaccctgcaggattcggcgaccggcgccgacgctggcgtggtgcgggtccacggcacggacaagggtctggcgatgacctccgacgtcaccccgcgttacgtccagaacgacccctatgagggcggcaagcaggcggtggccgaggcctggcgcaacctgacggcggtgggcgcccgccccatcgccatcaccgacaacctgaacttcggcaatccgcagcgccccgagatcatgggccagatcgtgcgcgcgatcgacggcatggccgaagcctgccgggcgctggacttcccggtcgtgagcggcaacgtctcgctctacaacgagaccaacggtgtcgccattccgccgactccgacggtcggtgcggtgggcctcctgcccaactatgacgtgaccaccggcttctccaccatggccgatggcgacgtgctggtcctgatcggccacacggagggcgagctcggggcctcgctgtatctacgcgaagtgctgggccgcgaggatggcgcgccgccgccggtcgatctccagctggagcggaagaccggcgactttgtgcgcggcctgatcgaggcgggcgagctgacggtggtgcacgacctgtccgacggcgggctgatcggcgcggccgcggaactggcgttggcgtcggacgtcggcgtgaccctggacgccaccagcccgacgcacgcccacatcctgctgttcggagaggaccagggccgctacctcgtcgccctgccagacccctcgcccctgatcaccaaggcgcaggaatcgggcctgcacgcctctgtggtcggccgcgcgggcggcaaggacttcgcctccggttccgaagccggcgacctgttccgcatcccgctggagcacctgcgcgaatggcacgagggctggctgccgaactggatcgagggctgaggcgcggtgccgacggtgttccgccaccgcaggtttcgctttcacttcttttccaacgaaggcactccgcgagagcctgtccacatccatgttgagagcagcgacggaaaggccaaattctggttttggcctgaggttcgcgtggcgtcggaaaacgggtatgatcgcaagacgctggccgagctgacgtggatcatccgcaaggagcgcgaccggatcgagcggagatggaatgagcacttcaacggctaagaaggtctggttcgacgactacaccatgtgggtcgatcttgatgacggccgcacgctgggcattcccctggcgtggtttcctcgcctgctcgacgccaccccttcgcagcgcgaggaggtccgcatcggttatgggggcgagggcctccactgggaagagatcgacgaggacatctcggtcgcgggcctgatcgccggacgcggggacatgacgcgtaggcccgccaccgcagcctgagaaagggctgttctgcaacgccggcgtcatgaagcgtcgctagagcaggtcgatcccgccgccggagcctgcccgatgacccgcctcgacctgtcccgccgcagcctcctgaccgccttcggcggcggccttgcgctgagcgcgtccggtcccagcctggcccagcctgcgttcgacgtgaaccccttccgcctgggcgtggccgcgggcgatccgctgccgaacggttttgtcatctggacgcggctggcgcctgagccgctggccttcggatcaggcatgccgcgcgcgcccatggcggtgtcgtgggaggtcgcgtccgatcgcggcttcaacagcgtggttcgttcgggcgaagtcgtcgcacggcccgaactcggccactccgtccacgtcgaggtggcggggctggagcccggccgcccctacttctaccgcttccgtgcgggcgaggagcgaagcggcgttggcgtagccaagaccgcgccggtgatcggatcgcccctggcgcgcgtgcgctttggcgtggccggctgccaggcctatgagagcggcttctacatcgcccatcgcaagctggcggccgaggacctcgacttcgtcttcctgtacggcgactacatctacgaagggcgcggcaatccgatctaccaaggcggatcgggcccgcaggacaacacccgcgtccatctgggcggcgaggtctacagcctggacgactaccgccgccgctacgcccagtacaccatggatgcggacctgcaggcctcgcgcgcctcggccgcctggttctgcaccttcgacgaccacgaggtggacaacaactgggttacagatctcgatcaggacgggaccgatcccgacctgttcctgctgcgtcgcgcggccgccatgcaggccttctacgagttcatgccgatgcggaaggccgccttcccgcgcggctcggccatgcagctttaccgccgcgcacagtacggcgacctgcttgacgtcaacttcctggatacgcgccagtatcgcaccgatcagccctgcaacgaccgcttcaacaccacctgcgccggcgtgaacgcggccgaggcacaggtgctggggcaggcgcaggaggcgtggctgctgaacaatctggatggctccaccgcccgatggaaggcgctggcccagcagatcatggtcatggatctgaaccgcaacacctcgggcggcgagggggtcaacaccgacagctgggccggataccgcacgccccgcaaccgcctgctgcgccacgtgcgcgaccagcggatcgacaatgtcgtggtcctgacgggcgacgagcaccagaacttcgccggcgaactgcacctgaacggccgcgagccggagggccggccgatcgcgaccgagttcgtctccacctccatcacctcgggcggcgacggctcggaccagcgcgccgacgcccagaggttcctggccgccaatccccagctgaagttcatcaacagtcagcgcggctatgtcgtctgcgacgtgacgcccgaagcctggcggaccgagttcaaggtgctggacaaggtgtcggaccgcgacggcgtgctgtccacccgcaagacgctcgccgtggcgtcgggcgacccgcgcctggtcgaagcctaggcgacttccggcacgctctgcttcagccggccgcccacgcggatcggctcgacgcgcttggccaggccggtgcggtcgtccgtctccacaaaaaccccgcacacggtcgccggccccgacgccggctgatagcgcccgcccgacagccgagtggtgaagcggcgcagcggctcctctttttcattgccgatgacggagtcgtagtcgcagcagccgccggcgtctgtctggtaagccgtgccgcccggcagcacctgtgcgtccgccgtcggcacatgggtgtgggtgccgaccaccaggctggcgcgaccgtcgcagaagtggcccatggccatcttctcgctggtcacctcggcgtgcatgtccacgatgatggcatcggccgccatgcccaacgggcaggccgccagctccttctccacggcgctgaacgggtcgtccatcggatccatgtgcacgcggcccagcacgttcatcaccagaacggtgcgcccgctctgcgtttcgaacagattggcccccgcgcccggcgcgtccatcaggcgcggatagttcaacggccggatcaggcgcggctcgcgcacgatgtaggtcagggcctcgcgctggtcccagctgtggttccccagcgtcaggcagcccgcccccgccatgaacagctcgcgcgcggtgttctcggttatgccgaagccaccggcggcgttctcggcgttcaccaccacgaaatcgagccgcaggtcgcgcttcagccccggcagatgatcgctgatcccgtcacgcccggacttgccgatcacgtcgccaaagaaggccagtctcatgtcagatacggtcccgccggacccgccggccaatcttcacagcgcaggccttcaacccgagcaaattcacgcaggttgccagtcaccacgatcagcgagcggctccgggcatgcccggcgatcaacaggtcgttgctcccgatcatcgttccacgcctttgcaacgacgccttgatgtcagccgcgtgatccgcggcggcgctgtcgaaatcaagcaccgccatacgggacagcagcgcctccaccgcagcgcgctgaacatccggacgcatcgacatcatggcgccgtgcatcaactcatgccggaccacggccgacgtataaagccggctcgcatccgcgttcagcttctcggccagttgcggcggacgattgcgaagcagcctgacgcagatgtcggagtcgaggaggtacacctagtcgagcaacacgacttcatcatcaacaaggtcttcggcgatgcggatgtcgatgccgggccccttgagaaaatcgtcccacaccgcgtccgcaggcacgagcagcagcccgtttccttccctgatgacgcgcaactccttcacgtcatcgggaaaagcgaccgcctttggcaggcgcaccgcctgggaacggttcgacttgaacacggtggccttgatcggagcgttcatgcggtgatcgtagctcacgcacggcatatgtcaaagacatatcccttagcagatcgcccgccagccctcttctgtcagcaccccattgagccgcatgtcgtgcggctccagcgccaaccggtccaccgcctgaccagcgtagccgaacccgatccgcgtcgtgtccggccgctccgcaaaggtgcggtcgtagtagccgccgccctgacccagccgcccgccgaaggcgtcgaacgccaaaagcggcgtgacgatcaggtccggccggacctccgccgccagcggcaggggggcgggacatccggcttggtccatctccagcggctcgcccggcgaccaggcgcggaaaatcatgggggcgtcgcgcgcgatcaccgccggcaggcacagccggcgcccttgcgccagcagggcgcggccgagcggctcgggatccagttccgatccaacggcgcgataaagcgcgaccgtctcgccgtgcggcagctcccccgcgtgatcggcggcgcgcacggcggccgtcgaatcggcctcggccagccgcttcctcagggctcgcatcgccgcgcgcatctggtgcttttcgctcatgcggcctcctagaccatcccgatgcggaaatcccgcacggccgcgcttcgcttaagggaacggatcgggcacaagcctccgatgcctgccgattcgagcctcctttcgcccctgacccaaccgggtctggccgaggcccgcgccctgctgtcgcgcgtctggggccacggcgactttcgcggtctgcagggcgaggtggtgtccgaggtgctggccgggcgcgacgtgctggccgtcctgccgaccggcgggggaaaaagcgtctgctaccagattccggccatcctgcgccgaggccttggattggtggtctcgccgctgatcgccctgatgaccgaccaagtcgaggcgctgaagcaggcgggcgtggccgccgcgcggctggactccggcgtatcgctggacgagcggtcggcgatctggcggcaggcgcgggcgggcgagttggacctgctttacgtctcgccggaagggctggcgtccggcgccatgctggaccggctgggggaactgccgctgtcgctgatcgccatcgacgaggcgcactgcgtctcgcaatggggccacgacttccgcccagactatcgcaccttgggtaggctggccgagctgtttccgggcgtgccgcgcatcgccgtcaccgccaccgccgacgcccgcacgcgcgaggacatcgtgcgctcgctgcggctggagggcgccgaggtcttcgtcgccagcttcgcccgcccgaacctgcagctgtcggccgagcgcaaggaaaatgcgtcccgcgcccgcaccgacgcccgcgtgatcgaactggtgcgggaacggcgcggccgctcgggcgtggtctactgcggcagccgtgacggctgcgaccgggtggcccaggcgctgagggacgccggaaccaacgccatcgcctatcacgccggcatggacacggccgagcgcgaccgccgcctggcccgcttcctggccgaggaaggcgcggtcatggtcgccacaatcgccttcggcatgggggtggacaaggccgacgtgcgcttcgtcatccacgccgatccgccgggctcgctggaggcctattggcaggagatcggccgtggaggccgcgacggcgagccggccgagggcatcaccctgtacggcccggccgacatcgcctggtcgctgcgtcggctcgacacgcgccccatgccggaagaggtcaaggcggttcaggtccgaaaggcgcgccagctgttcgccatgctggacggaagcgtctgccgcccccaggcggtgcgtcgctatttcggggagacggacgcggccccttgcggcgtctgcgacatctgcggcgacccgccgtccctgtatgacgcgaccgtcccggcgcaaaaggcgctggccgccgtgcatcggcttggagagcgcttcggccgcacccgcatcatcgaccacctgctgggcaagaccagggacgtgcagccgtgggaaagcggcctctcgacctggggcgtcggcaaggacacctccccgcccggctggcgcgacgtgatcgaccacctgctgttcgaggggctgctggtcgaggacccgaacgacggcaagccgctgatccgcctcggcgagcccgaggccgtgcgcgccgtctatcgcggagagcgccggatcgaggtgcgcaaacccacggcccgtttctcgggcgcatccgccccgcgcgagcgcacccgcgacggccgcaacgccgcgctggagacgctggacacggatgtccgcgcccggttcgaacgcttgcgcgcctggcggcgcgagcgcgcgtccgaacagggcgtgccgccctacgtcatctttcaggacaagacgcttctggagatcgccgtcgccgaacccggcgacctccagcgcctgggccgcatccccggcgtcggtcagaccaagctggaccgctacggcgcgggcgtgctggaggcgttaggtggcgcggacgccacgcagggtcgtccgagcgatgtcgttgaccgcgcgcgcgacctgcggcgcgacatgaccttgccggaagttcaactatggcaggcgctgaagggccggcaactcgacgggctcaagttccgccgccagcatccggccgcgccctatgtgcttgatttctactgcgcggaggcaaagctggctgtggagatcgacggccaaacgcattctgatggacaagccgccaaggacgcgcaacgcgacgccttcctcttcaagcaaggcgtccgcaccatccgcgttcccgcgaccgccgtgctgaacgatctgccaagcatcctcgaccacatcacccgcgaggcgcgccgctaagaccttctcccgcttgcgggagaagtggcccgtcgatcggcgaagccgatccagggtcgatgaggggagtctttcctgagccggaaactccccccatcgtcaggcgcgtcgcttcgctccacgacctgacacttcccccgacaagcgggggaagatcttacgccgcgcaggcttcgaagccgcggcggaggtcggcttcgtcgaggtcgcggccgatgaagacggcgcggctccagcggcgttcgttgacgccccaggcccgctgcaggtcgccttccaggatcatgtgcacggcctggaacaccaggcggcggtcctcgccctgaacgtcgatgatgcccttggcgcgcaggatgttctgcccctgcgagcccagcagcaggtccagccactgggtgaacttcgccccgtcgatggggcgatccagcgacagcgctatccccttgatgtcgtcctggtgcgcatggccgcgggcgccgtggtgatggccgtggtcatggtgatcgtgcccgtggtcgtggtcatggccgcaatgctcgtcgtggatgtggccttcggcgccatgcggcgggttcacgaagtccggcttcacctccaggatgcgatccagatcaaaggcgtgaacgcccagcacgctgtccagcggcacgttggaccgctcggcccgggtgatcggcgccagcgggttcagcgcccgcagtcgcgcctcgaccgcgtccagcgccgcctcgtccaccagatcgaccttgttcaggatgatgcggtcggcgaaggccacctgctcgcgggcctccttggagtcgtccagccgcgccatgacgtgcttggcgtcgaccagggcggtgacgctgtccagctgggtcttggccttgacgtcctcgtcgacgaaaaaggtctgggccaccgggccgggatcggccaggcctgtggtttcgacgatgatggcgtcgaacgccggcttgcccggccgctggcgcttcatcaggccggagaccacgcggatcaggtcgccgcgcaccgtgcagcagacgcagccgttgttcatctcgaacacgtcctcgtcggcgccgaccaccaggtcgttgtctatgccgatttcgccgaactcgttgacgatcacggcgtagcgcttgccgtgatcctcggtcaggatgcggttcagcagcgtcgtcttgcccgcgccgagatagccggtcaggacggtgacggggatcttggcttgggcgggcgtgctggaggtggtgtcggtcatgcgccgctagatggcggctccggcccggcttggaaaggggcctctagcagccgggacagtccgccagcggcgcggcctcgagctgcagcgtcgtgtgacggatgccgaatcgatcccgcatcagcctttgcgcctcgaccagcagggcgtcggcgtcggcccggtcgtggacgatatgcgccgtcagcgccgtctcggtcgtggacaggccccagacatgcaggtcgtgcagggccgaaacccccggcagcgccaccagcgcgccctcgatctcgcgcaccgccacgccgcccggagcgccgtccatggccaggttcaccgagtccttcagcagcccccacgtgccgaccaggatcaccgccacgatgacgacggagaccagcggatcgacgaccgaccagccggtcagcaggatcaccccgcccgcgatcaccacgccgatcgacacggcggcgtccgccatcatgtgaagataggcgccgcgcgcgttcaggtcgtgctggtccttcatgaacaacagcgccgtgcccaggttgatgacgaagccgaccgccgccacccccatgaccagcccggacgccacgggcgcgggctcggccagccgtcggaccgcctcgaaggcgatggcgccgcaggcgaagatcagcaaaagcgcattgcccagcgccgccagcaccgtggccttgccgaaaccataggtccgccggcctcccgctgccccatgcgcgcccttgcgcgccagccaggccgcgccgccggccatggccaggcccagcacgtccgacagattgtgacccgcatcggccatcagggcggtcgagccgctgacgatccccgccccgaactcacaggcgacaaaggcgagattgacgatcagcccgacgccatagcgccagtcgcccgtgtccaccggcccgtgcgcgtggccgtgatgtccatgcgcgtgcccgtgtccatgcccgtgatgatgatggccatcgccgccgtgatgatggtcgtgcgcatggtcgtggtggacgtggtcgtgggccatgcccggaccctagtgctggtgaagcgcgacgagaagcccgagcccgatcagcgccaggcccagcaccgcgccctcgtagcgcgcccagcgctccagcctaaggatcgaggcgcctgcgcccgccagcgccgtgaacaccaccatgcccagaacggtccccatggcgaacaccgccgtcagcgccgccagaacgcccagcccctccgtcgccgacgacagatagatgggcagcagcacctcgcccggcgacaaggccatcagggcgatcaggccgagaaaggcggtgcggtcagccaccctgggttcgggcgcttccagcgcgggaccgctggcggtcgcagttcgcttcagcatggcgcgcgacaggtaaaaggccccaaacaggaacagcagcaccgccgagaggtgcggcagcagaccctcgacccactggtccagcgcaagacccgccgcgacgatcagcgacccgatcacggctgtcgatccgatgtgcgccaggcccgccagcaccacggcgcccagcgtgcggctggtccgccagctctgcgcccgcccgaccaagacgaacggcagccagtgggtcggaagcgccgcgtgcagaaaggccgccgcgaaaccgccccccagcagggacagcagaacaggttgttgaagatcggccggcgacatgcgcgccctatagcgtgttactttgtaacggtcgagcccctttgatcgtccggcgccttcagccggcgtgcctttcgcgttgactcaacgcccacgatccgtatatgtcgccgcctcttcgcccgcgggtcctaccggcgggcgcattcttttttgcgtttgcgctgaggcttaacatgtacgcggtgatcaagaccggcggcaagcagtaccgggtccaaccgggcgacaccatcgtcgtggagaagctcgagggcgacgccggcgccgaactgacgctgggcagcgtgctgatgctgggcggcgacaacggcgtgaccctgggcgccccgctgatcgagggcgccacggtcgccgccaccctgatcgaaacccgcaagggtgagaagatcaaggtcttcaagaagatccgccgtcagggctatcgccgcaccaacggccaccgccagcaggagtcggtgcttcgcatcaccggcatcgacggcgccggtgaaagcgccaagtgggacggtcaggtcgaactgctgaccaaggccgagatcaacgcccgcgctcgcggcctggctgcgcgcggcgacgtcgccgcctcgtccgacctgggctcgaccgagacggtcgtgaccgacgtcgacggcgccaacgtcgaagccacggtggtcgaaagctccgctccggccaagaaggctccggcccgcaagaaggccgccgccaagacgacggaagcctcgggcgacgaagcctaagcgaattcgatgggcgccggatcggcgtctggtgtgttagattgatcggcgtcgcgcttccccgctgaagcgccgccagggaacggagcagcaagatggctcacaagaaatccggtggttcgtcgcgcaacggtcgcgactccgagtcgaagcgcctcggcgtgaagaagttcggcggcgagcgcgtgctggccggcaacatcctcgtgcgtcagcgcggcaccaccttccacccgggcgtgaacgtcggcctgggccgcgaccacaccttgttcgccctgaccccgggcgcggtgcagttcaccacgaaacgtggcggccgttgttacgtgtcgattctcgcggccaatgacgacgccgcccaggcgatcgccgccgagtaacgccagccgattgatcccggatcgcgttgctcctcgtcgaagcagccgatccggaccaagggaaatattccgcggggagtctggatcaccaggctccccgttcgcgtttccccgcctcgaagtccgcccgagccctgaacaaggaggcggacacgacagcgaggcaacacccatgtgcgtcatcgagacctctcccgtggtggagacgcggcgtctgacgctgcgcgcgcccgccccgcaggacgccggccgcatcgccgccctggccaacgacatcgacatcgcccgcatgaccaagcggatgccgcacccgtttcgggtaaaggacgccgaggacttcgtgctgcaggtcgcggcgcaggacccccgccgcgccaacaccttcgtcatcgagcatgaggaccatggcccggtcggcgtgatcggcgtcttcgagggggacgaccgtgtgccggagaccggctactggatcgggcgcgagttctggggccgcggcttcgccaccgaggcgctggagggcgccctgacgtgggccggcaagcggtggaagcggcgcgccctggtcgccggccatttctcggacaatccggcctcggggcgcgtgctggagaaggcgggatttctctacaccggcgagacgcggaccgccttcagccgcgcgcggggcgagaacgccgacacccgcatgatggtctggctggcctgatccgaccgcccggcggatcaggcggtcagggcggggcccagcacggcggcggcggcgatcagcccgaccgcggccgtggccgccgcgccggcgacaaaggccagggccgtgcgggtgcgccgtcgccgcatgccgccggcgcggacctgccggatgatcacgaacggcgtccggtcgaaagcctccgacccgatgatgttgtgctgggacaagagacgctccccgactgaccccgatcggacgatctgtcacagggctcggggccaaaggatggcgaccggcggtttatgtccgccggcctcgttcaacctagagcactacgtcgagcgcgccgttccgcacgtccaggcggtgcatcagaaccacgggctcgccgccctccgcccgcaccggggcgatcacgaaccaggatccgctggggaggccggtgaagctgaagcggccgttctcgcaccgggtggagcgcacaaaggcgcggtagtcggcgttgggatcgggcacgtcgcgggcgcgcaccacggcggcgggcacggcggcgcgttcggtcgagccgtacagggtgcggaaccgctggcgcgtatagggggtgtccggcgtcagtccgaccgagccgacgcaggcgaagacctggccggcgtcgcgatagtccacccggccgttgatcgccccctgcccggccgccgccgaccaggtgaagtcttggggctggaacaccgccggggcgagcgtgcgcgggggcgcatagccggtcgtgggcgcacacgcggccagcgccgccgccgacaggccgacgagcgcaaaggaacggatcaaacggggcgccatcacgggtttccttccagccgacttttcgttgtgctggcagtctcgcatgatcgcgggcgcgcgaccaccaccgggcgccgcctctggaccccggcccgacaaaggtcgaaagagcagcgcacaaatcgccgcgtcgagcgatgccgacaatagattcgccggggagttcatgaccgtcaccttcgccgacatccaggccgctcagagccgtatccgcggccaggtggaccgcacgccggtgcgccgttcgcgccgcctgtcgcagctgaccggcgccgaggtctggctgaagttcgacaatctgcatttcaccggctccttcaaggagcgcggcgccctgaaccgcctgctgctgctgaacgaggacgagcggcgacgcggggtggtggcggccagcgccggcaaccacgcccaggccctggcctatcacggcgggcgcctcggcgtgccggtgaccatcgtcatgcccgagggcacccccttcgccaagatcaacggcacccgctcgcacggcgcgaccgtggtgatccacggcctggacttctcgggcgccaccgaagaggccaagcggctggaggctgaaaggggctttgtcttcgtctccgccttcgacgacgagggcatcgtggccggccagggcgtctgcgggctggagttcatggaggacgcgcccgacctcgacgccctgttgattccgatcggcggcggcggcctgatcgccggcagcgccatcgccgccaaggccatgaagccggacatcaaggtcttcggcgtcgaggccgcgcgctatccgtccttcaccgcgcgcagagcgggccagccgccgaaatgcaccggccagaccatcgccgagggcatcgccatcaaggccgtgggcgaaatccccttcggcctgtccgaccggctcatcgacgacgtcttcgtctgcgaggaggcggacttcgagcgcggcgtctcccttttggtcacccacgagaagacggtggtcgagggcgcgggcgccggcggcctggccgccatgctcgccaacccggatcgcttcgccggcatacccgtcggcctggtcctgaccggcggcaacatcgacgcgcggatgctggcggtggtgctgaaccgcgagatggtgcgcgagcggcgcatgatcgtctatcgcatcctgggcgacgaccggccgggcatgctgtcggccatggcggcggtgatcgggggcctgggcggcaacatcatcgacgtggtccacaaccgcctggcgctggacgtgccggctaagggcgccgagttcgacatcatggtcgaaacgcgcgatagcgcccacgccgacgagatcggggcggcgctgaaggatcgtggatatgaactccgcatgggttaaggccgcgctggccgcctctctcctgctggccgcctgcgggccggccgccgcccccgccgatcccaacgccggcaaggccgaggccgccgccttcatggccgagaacgccaaggccgagggcgtccagaccctgccctcgggtctgcagtacaaggtgatccagtcgggtccgcccggcggcgagagcccggaccgcaacgacctggtcaaggtcgattacgaaggcacgctgaccgacggctcggtgttcgactcctccttcgcgcgcgggacgccagcggtgttcacgcccgagacggtggtgcccggctggaccgaagccttgcagaagatgaaggtcggcgacgaatggctgctctacctcccccccgagctgggttacggcgaggcgggcggcggcggcaagatcccgcccaacgccgttctggtgttccgcctcaagctgctcgacatcgcccgcgcccccggcggcggctcgggcgtcgggcaggcgatgggctagaactctcctccccaacggcgatggggaggtggcgcggcgcacagcgccgtgacggaggggtctcaggccgcgctcgccgtttcggacccctccacccccggctgcgccggcggtccccctccccatcgctgcgcgacagggaggagagccgtcagccgagccagcgcccattccgccgcatcgcgcaccaccggatcgggatcgtccaggagacgccgaacaggctcgatcagcgccgcatcgcccgagttgccggcggcgtacagcacgttgcggatgaagcggtctcgcccgatccgctttaccgggctcttgacgaacagggcgcggaacgccgcgtcgtcgagccgcagcaggtcgtcgaggcgcggcgccacaaaggcctcacgcggcttcagccgcatctcgcgggcttcctgcgcgaacttgttccacgggcagacccccaggcagtcgtcgcagccgtagatgcgcgcgccggtcgctgtacgaaactcctccggccacgtgcccgcgaactcgatggtcaggtaggacaggcaccgccgggcatccagctggaacggctcgggaaatgcattggtgggacaggcgtccagacaggcggtgcagcgcccgcaatgctcgacctccgcctcgtccggctcaagctccgccgccgtcaggatcacgcccaggaacagccagttgccgtgggtgcggctcagcagattggtgtgcttgccctgccagcccaggcccgcgcgctgggccagcggcttttccatcagcggcgcggtgtcgacgaacaccttgatgtcggccccgttccgcgccgcgatctggcccgccagctgcttcagccgccccttgatcacctcatgatagtcgtcgccgcgcgcatagaccgagatgtagccggcagatcggtcggccagcgccggcagcgggtcctcttgcggcccatagttcatgcccagcacgatggcggtcttcgcctcggcccacatggaggtgggatggtcgcgccggtccagcgtggtctccatccacgccatctcgccgtgccgcccctcgcccacgaatgcccgcagccgctcgcccgccggccaggcgtccgcggccgaggcgaagcggcagacgtcgaagcccagctccgtcgcccgctggcggatgaatgtcttgaggcgctcgctcacagggatggattagcacatctctttcctccttgccgcgcaagcggcggggaggtggatcgacggcgacagccggcgagacggaggggttctgaaagcggacccccctccgtcacgaggcttgcgcctcgcgccacctccccatctgcgatggggaggagaaggttttcagaaatccaggtccgcgtagcaggcggcggcggccacgccgttgaaccgatcgcccagcagcgggcggaagcacggccgcgacttcagcttcatgtaccaggtcttcagcgacggccacgaaccccaggcgacctcgccgaaatagtcgtggatcgacagatgcgccgccgcgatcaggtccgcctgcgacagccgccgcccggccagccagtcccgcgtctgcagcaggtcgtccagcacgcccagatggtggcgcagcgacacccgcccttcccgcaacgcctgggcgtcgggcgagcccagcttcagcagcggcttctccacccgctcgtgcagcagcacggcgtccacctcgtcggtgaagcgacgctcgaaccagccgaccaggcggcgcgcctcggcccgctcggcggcgtcggccggcagcagcagggcgcccttcaccccgtcctcgacccagcccatgatcgcgttcagttcgcacagcaccagcggccggccccgctcggcggtctccagcaccggcggcatgccggacgggttcagcgcctgggtgggggcgtccggctcccacggccgcaccgcgacgtccgtccactcgatcctggcctcgcccagcgccagccgcgccgcgcgggacgccggatggaagggaaaatggtagaggacgcaggccatcgagaacccataggccggctcgcgttaagcgcgcgtttaccgcgtgactacgaccagggaccgcgcgacttgggcggcgcgtccgccgccgggtctcccgtcggctgggtagcggcaggagccggaaccgacgcgggttcggaaagagcgcccgcgtgcggctcggcccgtcccttgggatcggcgtggatcaggaggtcggcggccggatagagcgccagcacccgccgttcggcctcgacgacgatggcgtgggcctcttcaagcgtcaggctgggttccaggtccacgtgcatctggatcagcatgaccggccccgacatgcgggtgcgcagtccgtgcacgcccagcacgcgcggatcgtccagcacggcctgggtgatcgcccgccggtcgccttcgggcgccgcgcgatccagcaggtggtcggccgccgccttcagcatgccggtcgccccccagaacagccacacggccaccacgatgcccgccgccgcatccagccccggcgcgttcagaaaggcgccggacgccaccccgatcagcacaacgatgttggcggcgatgtcggcggcgtagtgggcgcggtcgccggccaccgccagagaccccgtcttcctcagcgcccgcgtctgcatccacaccagccagccagtgacggcgatggacaggccgacgactcccagcgcccagccgccggcggtcaccgggcgcggatcaaacacgcgctgcacccccgcccaggcgatgaaaacggccgaggcgaacaccagccccgcctgcaccagcgcggccagcgcctcgcccttgccgtggccatagcgatggtcctcgtccggcggcgcggcggccccgcgcacggcgaaaaaggtcgccagcgacgcgaccaggtccagactcgagtccgccagcgtcgccaggatcgacaccgaccccgatgcgcctagggcaaaggccttcagcgcgatcagcaccagggctacggccacggacaggcgcgtgatgcggcgggtcgccagatgggcgtcggtcggggcggatgggctcatcgccgccttgtcgcgcaaacgcgcggccttgccaacgcccgcctccatgaggctaagggagcgcacaagggaccgacgcggcgtcggccacagggatcatcgcatggcggactggttggcggcgcttattctcgggctggtggaggggctgactgagttcattcccgtgtcctcgaccggccacatgctgctgctggggcacttcctgggctttgagagcaccggcaagacctttgagatcgtgatccagctgggcgcgctcctggccatcatcagcatctatttccgcaagctgtggacgctggcgacgcgctggccgttcgatgcggaggcgcggcgctttctgatcgggcttcttgtcgcctttctgccggcggcggtcatcggcgttttcgcctatgacttcatcaagaccgtgctgttcgaaacgccgctggtgatctgcatcgccctgatcgtgggcggggtgatcctgctgctgctggaccggatgcccaagcggccgcgctggatcgacgccgacgcctatccggtgcgcctgtacttcctgatcggcctgttccagtgcctggccatgatcccgggcgtgtcccgctcgggcgccaccatcgccggcggcctgctgctggggaccgacaagcgttcggcggccgagttcagcttctttctggccctgccgaccatgggggcggcggtcgcctatgacctgttcaagaaccgcgacgtgctggacttctcggacttggggctgatcgccgtcggcttcgtcgccgccttcctgaccgcgcttgcggtggtgcggtttctgctggaattcgtcagccggcgcggctttgcgcccttcgcctggtggcggatcgtggcgggcgtcctcgggatcgtcggcctggcgatgacgggcgggctttaggcggtctcgccggccccgcccgcatagatcggggcttcggcgaactggccgccgcggcggaaccgccacaggtaggacggcgcgatggcctccagccccgtgggctcgatccccagcgcagccagcccctcggcgcccgaggcgaccacattgtcccgctgcagcatcagcacctgatcgccggtgatcggcggctcgacacccagaaggcccagcggcttcatcagcgtcgccagcatcttggccgcgccgaacggcaggccgatcagcggcttgctgcggttggtttcgcgcagaaccagcttcatcaggtcctcgaacgcatagacggcggggccgcccagttcgaacgtccggccgcccgcctcttgcagcgacacggcgcgcgcgaccgcctccgccacgtcgccgacatagaccggctggaaccgcgtcttgcccccgccgatcagcggcaggcccggcccataggcggccatgtgcgcaaaccggttcaggaagctgtcgcccgagccgaacacgatggagggacgcagcaccaccgcgtcgggatagatggcgcgcaccgccgcctcggcctcggccttggaccggccgtagccggaggcgctgtccgcatccgcgccgatggccgagacctgaacgacccgctcgacgccggccgcgcgtgcggcctcggcgatccggcggctgccctcgacgtgcacggcctggaacgagcgcttgccgccctcggccagcacgcccaccaagttaactactgcgtccgcgccgcgcacggcccgcgccacgtcctcgtcgcggccgatgtcgcagtgcatgaactggatctggcccacatcgcccagcggctggacctcgatggccagcgtcgggttgcgaaccgcgatccgcacccgccagccgcgcttcgccagcgtccgcaccgcctgcgacccgataaagcccgagcctccgaacagggtgaccagaccaggggtgaactcagccattggagggctccgaagacacaggcgcggcggcgtgcaagccgtcttgtcgcgcgggatagacgatgcggccgcagcgagcaacgcaggcgacgcttgggtcgagcccggccgacgcccatatgtcggccatgcccctgttcaccatcggatacgaaggcgcgacgcaaggagacgtcatctgccgcctcaaggccgcgggcgtgcagaccctggtcgacgtgcgcgccgtcgccgcatcgcgccgcgccggcttctccaagaccatcctgggaaacagcctgcgcgccgaggggatcgactatctgcatctgcgggccttgggcacgcccaaggcggggcgcgaggcggcccgcaagggtcgggtgtcggagatgcgcgccatcttcgacgaccatctggccgagcccgaggccattctggcctatcagcagctcaaggcgctggcgggcgagcgccgcgtggccctgctgtgcttcgaggccgatcatgcgggctgccaccgcgccgtcctggccgagcgcctgcaggccgacgacgacatcgaggtggtgaccctctgacgcgcctcccgttgcaagccgcggctttttgccgcttagcttttcagcgaacgcaggggggcccgccatgaccgacaccacgtccacgccgaaacggcgcgtggagctgaccctgcgggctctggcgctgggttgcctgctggcggtgatcttcaccgccgccaacacctatctgggactgctggtcggcctgaccttcgcctcggccattccagccgccgtcatctccatggcgatcctgcgggcgttccgctcctccaccatctgggagaacatgaccgtccagaccgtggcctcggtcggcggggccatgagctcgatcatctttgtcctgcctggcctggtgatgatcggctggtggttggacttccccttctggcagtcggtgctgatctgcgccctgggcggggtgctgggcgtgaccttctccattcccctgcgccgcgcgctcgtcacgggcggcggcctgccctaccccgaaggcgtcgccgccgccgaggtgctcaaggttggctcgcgcggatccgaacagaccgaaagcgcggtgcgcgagaacaaggccggtctttgggtcgtggtcgcgggcgcggtggcctcggtcgcttacgccctgctgaccgccgcccgcctgttcgcggccgaggcggcgcagttcgtgcgcctgcctgcggccctgggcggcggggcgacgggcatgggcttcgggctgcagttcgcgcttctgggcgcggggcatctgatcggcctgacggttggcctgtcgcaactgttcggcctagtcctcgcctgggggatcgccgtgccggtgctgaccagcccggacacgatcgcctggctccaggcgcacgacattccctccatcgccgccaccctgcccgccggcgtctcggccgaggagttagcctccaccgtctggagccgcgaggtgcgcttcatgggcgcgggcgtgatcggggtcgccgccatctggaccctgatcaagctggccgggccgctggtcgcgggcctcgcctcagcgctggccgccaacgcccggcgcaaccacggcgaggcgctggagctgaccgagcaggacctgccgatcaagctggtgggcgccctgtcgctggtttcccttgtcggcatcgccggcctgctggcctggttcgccgggagcgcgccggcgctggcgggctccaccgccatgctggtgatcggcggcctggtctatgtggtcctgatcggtttcgccgtggcggcgatctgcggctacatggccggcctgatcggctcgtccaacagcccggtgtcgggcgtcggcatcctggcggtggtgatcgcctccttgctgatgctgggcgtgatggcggtgtccggcgtgccggccgatccgtcgatcatcgccttcgccctgatcgtcaccggcgtcgtcttcgccgtcgcggtgatcgccaatgacaacctccaggacctgaagaccggccagttagttcaggccacgccgtggcgccagcagacggccctgatcgtcggcgtcggcgccggcgccctggtgatcccgctgatcctgaacctcctgaaccaggccttcggcttcgaaggcggcccgcccgcgatcgcggaaggcgcgcagaccctggccgcgcctcaggccaccctgatctcggccctggcgcgcggcgtcatcggcggcgatctgcgctgggacctgatcggcctgggcgcggtgatcggcgtcgtcatcatcgtgctggacgcggtgctggagaaggccacgaacaagcggatcaagctgccgccgctggccgtgggcatcggcttctacctgccggcggcggtcaccaccatgctggtgatcggcgcggtgtgcggctggctgtacgagcgcgccgtggcgtccaagtcctacgccccggtcgcccgccgcatgggcgtgctgctggcgtccggcctgatcgtcggcgaaagcctgttcggcgtcctgaacgccggcgtcatcgtggccagccgcgacgcggaatgggcggcgctcccgctcggcgaaacctggcccgccatgctcgccggcgtcctggttttcgccgcgctcgcggcggcgctgtacgcatggacgaagagccgagcggcgaaggtctgagaggtcttcccccgcttgtcgggggaagtgtcagctcgtggcgcgaagcgacacggctgacgatgggggaagtctcccgaagaagactcccctcatcaaccctggatcgcttcgcgatcgacgggccacttctcccgcaagcgggagaaggtctggtcgttaggcggccttctcgaacagcttctgccagcggcgcggttcgcggttcttccaggcttcgcggtgataggcgtccgagccgatcagcggcaccaccgtggtcgcttcggcgaagaccatctgctcgtgcgtggtctgcaccttaccccaggaggcggcttccttcagcgtggaggacgagcaggcgccgtcgcgcacgtcggcgaccgtgatctggaccgcatagcggtgcatctcggcttcgacgcccaggatttcggcgcacaccaccgtgtcctgcgcgaagttcttgggaacgccgccgccgaccatgaacaggccggtgacgcccgccgcgatcttgatatcggtcagttcgcggaaatcggcgatggcgtccagcatcatgtagggctgaccggcggcggcgcgctccttctggtgcttgaccaggccgaagccggccgaggagtcgacgaacgccgggcagaagatcggcacgcccatctcataggcggtctggatcagcgagccttccttcttggcgttcccctccgacagccacttgcccatctcccagatgaactcgcgcgaggagtagccgcgcggctccagccggttggcgatctccaggatggtgtggtcgcaggcctggagctcttcctcgtcgatgtaggtgtcgtagatgcggtcgatgtagttgtcgcgcaggacgttgtcgtcgacctggcccgccgcctggtagtgcttgaagcccagggcctcgaagaaatccatgtcgacgatcgaggcgccggtggcgaccaccgcgtcgatcatgccgaacttcaccatgtcgcggtacacatgcatgcagccgccggcggaggtcgagccggccaggatcagccacggcgagcagtccttgtcctccagcgccatgttgaagatgtcggccgcacgcgcggtgtcgcgcgacgagaagctcatcttgcgcatgctgtcgatgatcgggcgggcgtcgaacgaggtgatgtcgacgtgctcgaccacgttctgcagcagctcggccttggcgttggtctgaacgggagcgttcatttcggaggtttccctgtgatttgagcgcccgtcgagatcgcaggcatgccgggacggagcgaccgacaggcccgattgttccccctcaacccgtcaccctcggacttgatccgagggccggaaggtctgtcgcatggccctaagcgagacgtgcggacggtccgatcctcgggtcgagcccgaggatgacaagctgaagaagggtctacttccgacgctgtttgcgctgcccggccttgcccttgggacgcgacagacgcaccaccttcctggccgcctcctccgccgtggtgcgcacggtggggatggagcgcggcgccaggccatagagcgacgccatcggcgcatcctcgaccacggcgacatcatgctcgccatagccgttgaagccggtggtcatggcgacgccataggcgcccagcatgccgatctcgatgaagtcgccttcgcgcacgtcggccggcagccagaaggggcccggcatgtggtcgatcgagtcgcaggtcggaccgtagaactggaacgccttcagatcggtcgagctttccccgtcccgcaccagcttggtcgggaagggccagcgcgagtgggtcgcgtcgaacagcgagccgtaggagccgtcgttcagataaagggcgtcgcccttgcgcaggtccacgcgcgccagcaccgacgacgattccgccaccagcgcccgacccggctcgcaccacagctcggtggtctccgacacgggcatctcgttgaagccgcgatggatcgcctcagcgtattcgttcaggtccggcgggaccatgcccggatagaccgacggaaagccgccgccgacatcgacgatgtccacgatcacgccggcgcggctgatggaccggccgacctgcgccatcgccgcctgataggcggtggggcgcatgcactggctgccgacgtggaaggacacgcccatcaggccgtccaccaccgcctggcgggtggccagcagcagggccggcgcctggtccggcgacacgccgaacttgcccgacagcgtataggccgcgccgtccgcagacaccgccatgcgcacgatcaggttcaggtcgttcgcgccgcccgtggcgtcgaggatcttgtccagctcctccacgcaatccaacgagaaggtgcggacgccgtgatcgaaataggcgcgggtgatggccgaacggctcttcaccgggtgcatgaaagcaagccgggcatcggtggacaccgagcgcaccagctcgatctcggcgagggacgccacgtcgaagccgcgcacgcccgcttccaccagagtctccacgacccagcgcgaggggttcgccttcacagcgtagaagacgtcggcctttagattatcctggaaccagcgcgccgctacggaaaccgaacgcggccgcacgagtgcgacaggacgttcaggaggccgctcgcggaccaggtccaggggaagctggtacgtgcgcaattcacgtaaccccctgttagttgttaacccagaccggcgttagcagcgcgtaacggttagacctacggggtccgccggaaggcgcgatatggggtgatcgccctgtcatgtaaagaggcaatttcgtggccccacgtgcatcctttcatgcggcaaccgccacgctggtcggccgtttggcggcgatgaggtcgaacccatgaaccgatggctgtttctgtggcgccgcctgtcgcgcgagctgtggtggagagccagcctctacgccgccttctcggtcgtggccgcgctggccgcctcgctgctgcagccctttgtgccggagaagatggccgagcgtctgggcggcgagtcggtggagcaggtgctcgccatcctgtcctccagcatgctggcggtggcgaccttctcgctgggggccatggtcaccgcctacaccagcgtctccagctcggcgacgccgcgggcggctgcgctgatcacagccgacgaaagcacgcaaaggtcgctggccaccttcgtgggtgcctttctctacggggttgtggggatcaccgcgatcaacgccggctactacgggccgcagggccgcgcggtgctgttcgtgctcagcctgctggtggtcggtctggtggcgttccggctgctggcctgggtcagccgcctgaccagtctggcgcgcctgggcagcacggtggagcgagtcgagagcgagacctgccgggcgctgaagatcgacgccgagacgccctgcctcggcgggacggaggggcggctggacaccggcgtcgccatcaacgcagcccaaaccggctatgtccagaacatcgacgtcgaccgccttcagacgctggccgaacggctggacgggcggatagagatcaccgcgcggccgggcgccttcgttatgcggggcgaaccgctggcgcggatcgcggcgacgacggtgaccgacaaggatgcgggcgcggtcgatcacgccttcagcatcgtcgccgcgcgctccttcgaccaagacccgcgttacggcctgatcgtgctgggcgaggtgtcggccaaggctctgtcggcggcgatcaacgacgtcggcaccgccgtccaggtgatcggcacgggggtgcgcctgctggagcagtgggccgatgcggcggccggcgcccagcgcgagccgcgccgtccccggctgctgacctatgcgctcgagcccgacgaactgctggacgacatttacgggccgacgctgcgtcacggcgcgggcgacctgacggtggcgctcagattgcgcaaggcgctgcgcagcctcgccgccggcgcaccggccctttcccgcgccgcgacggccatggaggcgcgcctgatggcggcggccgagcgcaccatggaggatcccgacgatctggagcggctgcgggcgggctgagcctgcgtggtcgggacggatagccgaaggacgcgctgtcccggcccgcgcctctggacgtaaaccggccggtcgtgcgattaagggttgccttggcgcacgtctcgcgtcatgcggcgcccctttcgccacagcctcccagcgagttcatgagttcatcagccgccgcagccgccccgggcctggtcctggcgcgcgacgtgtcgaagaccttcggttcgcgcaaggcgctcgacggcgtctccgtccaggtcgccgcgggcgagatggtcgccctgatcggcccttcgggctcgggcaagtccaccctgctgcgctcgatcacgggccttcagaccatcgacgccggcccgggcgtgatccaggtgttcggcgaaaccgtgcaaaaggacggccgcaccacctcggccacccggcgcgcgcgcggtcgcttgggcatgatctttcagcagttcaacctggtgggccggctcagcctgttctccaacgtcatgctgggggcgctgggtcgcatcccggcctggcagggcctgttcggcctgtggcctcgcgcggacaaggacaaggccatggcggccctgcaccgcgtcggcgtctccgactacgcaggccagcgcgccaacaccctgtcgggcggtcagcagcagcgcggcgccatcgcccgcgctatcgtgcagggcgcccaggccatcctggccgacgagcctgtcgcctcgctggaccccgtgtccgcccgcaaggtgatggagctgctggtcgagctgaacaagcgcgacggcatgggggtgatcgtcaccctccaccaggtcgactacgccatccgctactgcgaccgcgtgatcgcgctgcagggcggcaagatcgtctatgacggcccctccatggggctggaccaacaacgcctgatcgaaatctacggtcccgagttcgaggacgcgttctgggagaccaaggcatgagcctgtcccgtcgttttgtcgccgccgtgggcggtctggcgctgctcggcctgtcggcttgcggcggcggcgaagaaaaggccgcgggcggcgcgccgtccgaggtggtcttctccatcctgtcggccgaggggcaggcgtcttcgggcccgctgtggcagccgctgctggacgacatgtccaggtcgatcggcgtgccggtgaagcccttcttcggctccaactacaacgtcctggtcgaggccatgcgcttcaaccagacccaggtcgcctggttctcggccaagccggcgctcgaagccgtggaccgcgcccagggcgaggtcatcgcccgcaccgtcgatccggagggccgcgacagctacacctcgaccctggtggtcaagaagggctcgggcatcacgctggacaaggtgctggcctgcggcaagcagtacgacttcggcatcggcgacgcccagtccacctcgggcacgcttgcgcccatgaccttcctgttcaatccgcgcggcatcgtgcccagccagtgcttccgtaccgtgcgggccgccaaccaccaggccaacgccttcgccgtggccaccggcgtcgtggacgtcgccacctccaactcggtcaacaccgtcttcctgcgccgcgagaacccgcaggtcgccgaccagatcgaggacatctggacctcgccgccgatcccggaatccggcatcctgctgcgcgaagatctggatccggcgctgaaggagaagatccgcgcctttttcctgtcctatggtcagggccagggggccgaggccgatcgccagcgccaggtgctggccggcctgaactattcgatgttccgcgccgccgacgacagctatctcgaccccgtgcgcgagatggtcgccgaccagaagctgagcgaagcccgcgccaagaacgaccaggccggcgtcgccgccgccgagcgcgagctgtcgaccctgcgcgccaagcgtgaggttcagccttgaacacggcgaccgacatggccgcgcgcggcggcctgaacgcgggcgtggcggcgtccgccgtgccgcagccgcccaggaagtccgcctccgcctgggcgctggacgtcctgctgtggggcggcatcgccctggtgctgatcatcagcttcggcccggtggacatgcgccgcctgccgctgctgttctccaactcccagaacatccagctgtacggccgcgacctgctgaacccggacttcaccaacgtccgccagttggtcggccagatgtggctgacggtgcagatcgccctgtggggcaccttcatcgccgtcttcatcggcgtgcctctgggcctggccgccgcgcgcaacatcgcgccgaactgggtggtctggccggtgcgccgggtgatggacctgctgcgctcgatccccgatttggtgatcggcaccctgttcatcgtggccgtcggcctgggcccgttggcgggcgttctcgccatcgccctgaacaccggcggcgtgctggccaagttgttctccgaagccgtcgagtccatcgacaaggggccggtcgagggcgttcgcgccaccggcgccaccccgctgcacgagatcgtctggggcgtgatcccgcaggtcgcgcccttgtggacctcgttcgccctctaccgcttcgagtccaacagccgcgcggccaccgtgctgggcctgatcggcgccggcggcatcggtcagctgctgttcgaaagcatccaggcgtttgattatcgccaggtgtcggccatcgccatcgtcatcgtggtcgccgtgaccctgatcgacatgctgtcgcaggccatgcgcaagcgcctgctctgacggtcccaactcgcgaaaaccagggccgtcggcgttccgcgccggcggcctttttcgtagccctcgtctccttgaaagcgtcatcggccggctagacggactgtcacattcctatgctctaagcgtcgcaaacctcatcgaaggatgcgccgccatgacccgcctgctcaagatcgccgccgcctcggccgccgtgctcgccctcgccgcctgcggcgacggtgaaggcggaacgggctctcagacggcgcgcgccggcatctgggcggccggttcctcgactgtcttccccttcgcgacccgcgtggccgagaacttcgcccgcacctcgggcggcgcagctccgcgcgtcgagagcctgggcaccggcggcggcatccaggccttctgccagggcgtcggcccgtccacgccggacatcgccaacgcttcgcgtcagatgaaggcgtccgagttcgacctgtgccagcagaacggcgtcaccgacatcgtcgagatcaagatcggcttcgacggcatcgtcatcgccaccgcccgcagcggcaacagcttcaacttcgaactgaacgacctctacgaaggattggccaaggaagtgccgggcgcgaatggccagttcgtcgccaaccccaacaccacctggaaccaggtcaacggcgccctgcccaaccaacgcatccaggtctatggcccgccgcccacctccggcacgcgcgacgccttcctcgagctgggcatgaccccgggcgccaagctggttcccgccgctgccgctgttgaagccgctgacgccgatcgcttcgaggccctggcccacaccctgcgcgaggacggcgtgtggatcgactcgggcgagaacgacaacgccattgtccagaccctgacccgcacgccgggatcgctgggcgtgttcggcttctccttcctggagcagaacctcgacacggtgaaggccgagaccatcgacggcgtggcccccaccgccgacaccatcgccgacggctcctatccgctggcgcgcagcctctacatctacgtcaagaagcagcacatcggcgtgacgcccggcctgcagcagttcgtgcaggagttcatgtccgacggctccgccggtcggggcggctatctgcaggatcgcggcctggtgccgctgcccgccgctgagctgacggccgagcgcggcaaggtgcaggccatgaccgcgatgacgcgcccgcaataagcggagccgtagccggaacctacgctgttccgtcccgtttcccctcgcctctttcgtcggcgacgccggcttggctatatgaggcgggacagctgtcaggatcacgaatgaccaccacacccgcgcgtccggcgcgcctgcgtaaagccgtgctgccggtcgccggcctcggcacccgcgtccttccgggcaccaagacgacgcccaaggaactgctcaacgtcgtcgaccgccccatcctgtcctacatcgtcgaagaagcgcgcgaggccgggatcgagcatatcgtcttcgtcaccggccgcgccaaacaggccatcgaggactacttcgaccaccagatcgagctggaggcccagctgctggccaagggcaagaccgagattctggaggtcatgaacgccgagctggccagcgccggcgagatgagcttcacccgccagatgcagcccaagggcctgggtcacgccgtctggtgcgcgcgagacatcatcggccgcgaacccttcgccgtgatcctgccggacgtcatcgtggacggaaaacccggcgcgctgaagcagctggccgacagctacgccgagctgggcggcaacatcatcggcgtcgaggccgtcgacatcgaacaggcccacaagtacggcatcgtcgaccctgccgagcgcgacggccgccgcttcaccatgaagggcatggtcgaaaagcccgcggcgggaaccgcgccgtccaacctgtccatcgccggccgctacatcctgcagcccgagatcttcgacgtcctggccgaccaggaagcgggcgccggcggcgagattcagctgaccgacgccatggcccgcctgatgacgcagcagctgttcaccgccatcgagtacgaaggcgtgacccacgactgcggcgacaagatcggcctgctcaaggccaacgtcgccttggcgctcaagcgccccgacctcggcgacgccgcccgcgcggccatttccggactgctgtagaagcagcggatcttccccctaagggggaagtgtcaggtcgtggagcgcagcgacacgcctgacgatgggggaagtctccggctttgagggacactcccctcaccgaccctggaccgcttcgcggtcgacgggccacctctcccgcaagcgggagagggttctccctcgcacccttggttgagcctcagcccccgccctgctaaccctcctcgcaaatcaagaggagacacccatggccgcttccgaaggctggaccatgccgaccggcgaactgatgaagggcaagaagggcctgatcatgggggtggccaacgccaactccatcgcctggggcatcgcctcgcagctggccgcccagggcgccgagctggccttcacctatctcggcgaagggcttgagcgccgcgtgcgcccgctggccgagagcgtgggcgccaagctgctgatccaggccgacgtcaccgacgacgcctccatggacgccgccttcgccgaactggagcgtgagttcgggaccatcgacttcgtggtccactcggtcgccttcgccaacaaggacgagctcaagggctcgtttgtggagaacaccagccgcgacagcttcctgctcgccatgaacatctcggccttcagcttcgtggacacagccaagcgcgcgtccaagctgatgccgaacggcggctcgctggtcaccatgacctatctggggtccgagcgcgccatcccgaactacaacaccatgggcgtggccaaggcggcgctggaggcggcgacccgctatatcgcccgtgacctcggccccaagggcattcgcgtcaacgccatctcggccggcgccatgcgcaccctgtcgctggccggcatttccggcggtcgaggcatgatcgcgcagggtcgcgccatgtcggccatgaaggaggacacctccatggagggcgtcgccggcgccgccctgtggctgtgctcggacctgggcctgtcgaccaccggcgagatcgtccacgtcgacgccggcttccacatgatgggcatggccgccgacgaggaataatcctcagtcgggcggcctcaggcggtcaaaggcgaagcggtcgcggatcgcctcgccgaacaagcgcccctgcgactccgcctgatcgagagcggccgcgaccttcggcggcacgtcgagataggcgtaaaccgcgccgctggtgaaggtcaccgtcagccgctggcccaccgcatcatagcgaaaccggcggatgacgctggacggcatggcgcgcctggctcagatcgcccgaacgatcttttcgatgcgcgcggccacggcgttcagcgcctcggccaccccgtcgctggcggcggggctttccagcgtcggcggcggcgcccccttcttgcgggccgcgccggtgcgggtctcgtgcagttcgtccgccagcaccagcgccgccatcaggaacaggcggatgtcgccgacgtggcccacgtcgccggccacctggcgcaccaggccgtcgaactggccggccagcgcccgcacccggtcctcctgcccgtccgcgcagccgacgttgtagggtcgcccgttcacctcaaccgtcaccgtcgccatcagcgcgcctcctgcgcatcttcgccggcttcgacggcggcgtcgtcatcaggcgcactcgcctcctgccgatcgatcaggtcgcgcaccacctcggccgcgcgtcccagcgcctcggcggcttgggcgcccgccgcctccagttcggccacgcgggcgctgtccgcacctctgggcgcgaacaggtcgtcgtcacgatcgacgccggccttggccttcaggcccgcgatcttggtctccaggtccgccagggcgcgatcgatgcgcgcccgggcggccgtcacggcatccgccatcggtcgctcctttgcgagattcgcgtatagaacgcgcgaaaccgctggggtaaagcggcgcacgcctgattttccttctgatcgcccgaaaggtttccgccgtgagcgacgccaagaccgcccccgtgaaggccacccccaagcagatggccgacgccatccgcgtgctgtcgatggacggggtggaaaaggcgaagagcggccaccctggcatgcccatgggcatggccgacgtcgccaccgtcctgttcagccgtttcctgaagttcgacgccggccgccccgattgggccgaccgcgaccgtttcgtgctgtcggcaggccatggctccatgctgatctacagcctgctgcacctgtgcggctacgaggcggcgaccaaggaggagctgtccaacttccgccagtggggctccaggaccgccggccacccggaatacggccacatgccgggcgtagaggtcaccaccgggccgctgggccagggcttggccacctccgtcggcctcgccatggccgagcgtcacctggccgcccgcttcggcgaggatctggtcgaccaccgcacctgggtgatcgccggcgacggctgcctgatggagggcgtgtcgcaggaggccatcgcgctcgcaggccgctacaggctgaacaagctgacggtgctgtgggacgacaacgccatcaccatcgacggcgcggtttccctgtcggacgccaccgaccagaaggctcgcttcaaggccgccggctgggcggtcaaggccgtggacggccacgacatgcacgcgatccgcgccgccatgaagtgggcggtcaagcaggacaagcccaccctgatcgcctgcaagaccaagatcgggcgcggcgccgccaccatggaaggcagccacaagacccacggcgcggcgctgggcgccgccgagatcgccgcaacccgcctgggcctgtcctggactcacgatccgttcgaactgcccgagaccatcgaggcggcctggagaaaagtcggcaagcgcggcgccaaggaccgcaagaagtgggaggcgcgcctggccgcccatccgcaggccggcgacttcacccgcgccatggccggcgacctgccggacggggcgttcgacgccctgaacacgaaaatggccgaactgctcgagaccaagcccgctcaggccacgcgccagtcgtcgggagcggcgctggacgaactgttcgccgcgatcccggagatgatcggcggatcggctgacctcaccggctccaacaacacctttgtcaagaacacgccgatctacgacgccccgacctatgaagggcgctacatcaactacggcatccgcgagttcggcatggcggcggccatgaacggcctggcgctgcacggcggcgtcattccctacggcggcaccttcatggtgttctccgactacagccgcccggcgatccgtctgggcgccctgatgggggtgcgggcgatccacgtcctgacccacgattccatcggcctgggcgaggatggtccgacgcaccagccggtcgagcatctggccgccctgcgcgccatccccaacctgctggtcttccgccccgccgacaccgtcgaggcgatggagtgctggcaaatcgcgctgcagtccaagacggcgccctcggcgctcgccctgtcgcgccagaagacgccggcggtccgcaccgccacgtcttctgagaacctctccgcgcgcggcgcctatgagatcaaggccgcgagcgcagaggcccgcgtcaccctgttcggcacgggcaccgaactggccctggcgctccaggccgccgagacgctggaggcggagggcgtgcccacccgcgtcgtctcggtcccctgtttcgagctgttcgagcagcagagcgccgactaccaggcctccattctcggccgcggcacggtgcgcgtcgccgttgaggccgccatcggccaaggctggggccgcttcatcggcgaggacggcgtctttgtcggcatgaccggcttcggcgcctccgccccggccgaggtcctctacgacaagttcggcgtcaccgccgacgccgtcgccgccgcagcccgctcgcggctgtaacctcaaccctctccccttgcgggagagggagaccgcgcacggcggcgcaagccgtcgttctcgcgcggtcgggtgaggggttcgccgcccgccagcccctcatccgacccttcgggccaccttctcccgaggggagaaggataaggagaacctcatgaaactcggcacgcccctctccgacaccgcggtccgcgtcatgcttctcggcgcgggcgagctcggcaaggaggtcgcgatcgagcttcagcggctgggcgtcgaggtcatcgccgtcgatcgctacgccaacgcgcccgccatgcaggtcgcgcatcgcagccacgtcatccccatgaccgaccctcaggtgctgaacggcgtgatcatggccgaggcgccgcacatggtcgtgcccgagatcgaggccatcgccaccgacatcctcgccgggatcgaggccgccggcatggccacggtggtccccaccgcccgcgccgtgcagctgaccatgaaccgcgagggcatccgccgcctggcggccgaggaactgggcctgccgaccagcccgtacgccttcgccggctctgccgacgaactggccgagggcgccgcccgcgtcggctatccctgcttcgtcaagccggtgatgtcctcctccggcaagggtcagtcctatgtcgagagccccgaggagatcgccgacgcctggacctatgcggaaggcgcgggccgcgtcgccggcggtcgcgtgatcgtcgagggccgcatcgacttcgactatgagatcaccctgttgaccgtgcgctcgcgcggcgaggacggccagacccgcaccgacttctgcgcccccatcggccatcgccaggtcaaaggcgactatgtcgagagctggcagccccagcccatgagcccggcggcgctgacggcggcgcaggacatcgccggccgtgtcaccgaggcgctgggcggacggggcgtgttcggcgtcgagctgttcgtgcgcggcgaggaggtctggttctccgaggtctctccccgcccgcacgacaccggcctggtcaccctggccagccagaccatgagcgagttcgccctgcacgcccgcgccatactgggcctgccggtggacgtcgcccagcgcgaacccgccgccagcgccgtgatctacggcgggatggaggcggccggcgtcgccttcaaaggcgtggccgaggcgctcgccgtccccaccgccgacctgcgcctgttcggcaagccggaagccttcgagcgccgccgcatgggcgtcgctgtcgcgcgcggcgccgacgtggaccaggcccgcgaccgggctcgcgaagccgcaagccgcgtcaaggtcgtccagggctgatcgcttcttgccttctccccacgtggggagaaggccctggccccgcccgcctgcagcggatgcgcaacgcagccgggctttcgcctgcctgcgccatctacgactttcgtcgattggcctcccgtggctttatgcgccaaacaggggtgcgggccgtgcagggccggcgaaggggacgaacgccatgggcaagctgacgacgccgctgatcttcggcgccatcgccattctgggggccgtcgcgctggcgatcatcgccctgcatcagggcgagagcatcagtgcggtgtggatcgtcaccgccgccgtctgcacctacgccatcgcctatcgcttctacgcccgctatctggccggcaaggtcatggggctgaacggcacccggcccacgcccggcgtgcgccgcaacgacggcctcgactatgtgccgacgccgcgaaacgtgctgttcggccaccatttcgcagccatcgccggcgcgggcccgctggtcggaccggtgctggcggcgcagatgggctatctgcccggcgtcctgtggatcctgatcggcgcggttctggccggggcggttcaggacatgatggtgctgttcatgtccacgcggcgcgacggccgctcgctgggcgacatgatccgcaccgagatgggcaatgtccccggcatcatcgcccaggtcggcgtgctgatgatcatggtcatcattctggccgtgctggcgctggtggtggtcaaggcgctggccgagagcccgtggggaaccttcaccgtcgccgccaccatccccatcgccatcttcatgggcctgtattcgcgctttctgcggccgggccgcgtgggcgaggtgtcgatcatcggcgtcttcctgctgatcgccgccatcatcggcggcggccacatcgcggccgacccgttctggggtcccgccttcacgctgtcaggcaccaccctggcgctgttgatgatggcctatggcttcatcgcctcggtgatcccggtgtggctgctgctggcgccgcgcgactacctgtccacctttctgaagatcggcgccatcgtcgccctggccatcggcatcctgatcgtgcgcccgcatgtgcagatgccggccctgaccgacttcatcgacggcaccggcccggtgttcgccggcgccctgttccccttcctgttcatcaccatcgcctgcggcgccgtgtcgggcttccacgccctgatctcgtccggcaccacgcccaagctgctggagagcgaggcgcagatcccgatgatcggctacggcgccatgctgtgcgaaagctttgtggccgtcatggccctgatcgccgcctgcgtgctggaccccgccgtctatttcgccatgaacagccccgccgccctgatcggcacggacgcggcgtccgccgccgccgccgtggcccagtggggcttccacatcacgccgatggagctggagcagctggcccgcgacgtgggcgagggcacgatcctgtcgcgcgcgggcggcgccccgaccctggccgtcggcatggcccacatcctgtccaacgtcatcggcggccaggccatgatggccttctggtatcacttcgccattctgttcgaggccctcttcatcctgaccacggtggacgcgggcacgcgtgtctgccgcttcatgatccaggacctgatcggcgtggccgtgcccaagatgcgagacacccgctcctggatcggcaacatagtggcgacggccctgaccgtcggcctgtggggctatttcctctacaccggcgtggtcgatcccttgggtggcatcaacagcctgtggccgctgttcggcatcgccaaccagatgctggcggccgtggccctgatcctgggcacggtggtgctgttcaagatgaagcgggagcggttcgccttcgccaccgcgatcccggccgtctggcttctgatctgcaccctgaccgcgggcctgcagaagctgttccacccggacgtgcgcatcggcttcctcagccacgcgcggcagtaccaggcggcgctttccaacggcgagctgctggggccagccaagacgatgggtgacatgcaccgcatcatcgtcaacgactacgtcaactcggccctgaccgccggcttcctgttcgtggtcatcaccatggtggtctatggcgtccaagcctgcctcaaggcgcgtcgtatcaaccatccgacggtgcgcgagactccggcagagcacgagctgacgcccgctgacgaggccatggacgcggcccgtgcctgagccccgatccgacgccaaggccgccctcgacctcgcctgcctgtgccgcgacacggcggtgcgttggggccgcgacgcccgacgcaccgccagcctgatgatcggtcagcccgattatcaggcctatgtcgagcacacgcaggcgcgccatccggaccagccgccgctcgacaagaccgccttcttccgcctgcacgagcagcgtcggttcggaggatcaggcggctttcgctgctgctgacttgctcttggaatgagagcgggccattccgctggccccgcgatcaaagagacgccgcatgcccatcaccaccgtcggcttggacgccgacgacaccctttggcacaacgagaccatcttccgcctgacccatgctcgctttatcgagcttctggcggatcacggcgacgagaacgtgatcgaggcgcgcctggcgggcgtcgagcagcgcaacctgcggctctacggctacggggtgaagggcttcaccctgtcgatgatcgaaacggccatggagctgacggacggaaacctgcccgcctccgtcacccgcgagatcctggccgcaggccgcgaaatgctggcccatccggttgagaccttgccgggcgttgacgaggccttggccacgctgtcgcaacgctatcgccttgtcctgatcaccaagggcgacctgctggatcaggagcgcaagctagccgcttccggcctcggcgacctgttcgccgccgtcgagatcgtttcggaaaagaccgccgacacctacagccgcgtgttcgcccgccacggcacgggcgccgaagaggccgccatggccggcaactccatgaagtccgacgtcctgccggcgctggaggccggcgcctgggccgcccacatcccctacgccatcacctgggcgcatgagctggcggacgggccggaaggggcagacaagttcggcgtgctgaccagcctggctgagcttccggcttggctacaacaacaagagcggcatggcgactgaccgacgataaccgtgtcaccaaggccacattgttagcctaccaaggatatccgggcgagaaagtcgcctccgacttgacgcacagccgtcacaaagggcttgtgcagccccatcgcggaggcctttgacgcttttcccccgagcgcctgccgcgtctttgacaccaaggagtcacatgcgtcagcatctactcgcgaccaccgtgctcgccggcgttctcgccgccggctcggccgtcgctcaaaccgccccctcgcaacaaccgccgctcgccgtcgcccccacggccgatccggaagccaccacggccgagcagctcgacgaaatcgtcgtcaccggttctcgcatccgccgcgatccaaccaacgccccgacccctctgatccaggtcggccgcgagccctgctgaacaccggtcagaccaccgttatcgactatctggcgaccctgcccgccctgtcgaactcggtcgttccgtccgacaccacgggatcgggtctcggcgacggcggcctgtcgctgccgaacctgcgctcgctgggctcgaaccgcaccctgaccctggtcgacggccgtcgccacgtcggttcctccggcggatcgctggcggtcgacgtcgacaccatcccgcgcctgctgatcgagaacatcgagatcatcaccggcggcgccgcctcggtttacggcgccgacgccgtctccggcgtgctgaacttcgtgctgcgcaaggacttcgaaggcctggagatcgacgccaacctcggcatgatcaatcaggacggccagctgaacaagcgcttctccgccctggccggcaagaacttcttcgacgaccgcctgaacgtctatgtgcacggcgaatacgaagaggtcgacgaagtcacctccaacgacatcgactggatcgacgaagcctactacctcggcgtggtcgacgctgatcgcaccgccttcccctacgatggccaggtcgaccgcctcctctacaagaacgtcctgcgcatggacacgccgcggtggggccagaccacgctcggcaacgtccagcagcccacagacctgaccaaccccaacgtcgcctatcaggactgcttcgccggcggcggctggacctattcggccaactgctacggcgtgacgcccggcaagaccttctggtatgacggaaccaccgctcgcccggccgacttcggccaacgggtcggcaacgtcggcatcaatcgtccgtacaacatcggcggcgacggcgagaacatcgccgatttcagcaccggctcgcgcgttccccgttccgagtcggcccgcttccaagccggttcgaccttccgtctgaccgacaacatcgagctgtacggcgaggccaaatacatcaccgaggacacctatgacctcggccagccgaccttctacgacatcgatctggtgaactcgtacggcgcgggtgcggtcaacccgatctacagcaccaataactttgatctgcgctggtcggacaacgccttcctgccgcagaacgtcaaggacgccatccgcaccaacacggtgacgccctacacccagccgaccctgacctcgccgggtcagccgctggcgccgatcgcggcccagttcgctcgccactcgctgtttggcccggatcgctaccaggacaacacccgcgaactgcagcgctacgtcttcggcgcgcgcggcgactgggatcagatcggcttcgtgcgcgatctggcgtgggacatcggctacaccttcggcaaggtcgaggttgaaaaccgcgaacacggcaccgacacccagcgcttctccctggcggcggatgcggtggtggacaccgccggcatcgtcaacggtcaggccggccagatcgtttgccgcgtgcagttgcttgacgcacaaggcgccgacctggacgactaccagcgcggtggcgacctgcgggacagcgaatacggccgcaactcgattgaccagtgcgccccgctgaacgtcttcggcaagggcaaccaaagcgccgaggccgtcgagtacatcctggccgacatcggcgtgaccgaggagaaccagcagcagcaggctctggcatcgatctcgggcaacctgtgggacttctggggcgccggttcgatcggcgtcgccatcggcggcgagtggcgtcgggaagagacctcggcaaccggtcgtgaccgcgacacggcgggccgcctgctgttcctgaacaccggtcccgacttcctggaagcggcctacgaaagcaaggaagtcttcgccgagctgtcggtgccgctgttccgcgacaccatgctgggcgaatacgccgaactcagcggctcctaccgttacgccgactactccacggtgggcgcgcaggacgtctatggcgtgaacctgatctatcgtccgatccaggacatcgccttcaagaccagcttcaacacctcgatccgcgttccggacctgggcgagaacttctcgcccttcagccagaccttcctgaacaacttcaccgatccgtgcacgacggccgccatcacggccgtcaacgacacgacggaacgggcgaaccgcgttcagaactgctcggccctggccgcgcagcaagggctggacttcgacttcgccggggctacgccggagaccaccgacgacttccgtccggactacacctcgggcgtcgccggcgtgctgggcggcaaccccgccctgcaaccggaagagtcggacagcttcaccttctcgacggtgctgaagccgcgcttcatcccgaacttctcgctggttctcgactactacgagattaagatcgacaacgtcatctcggccatctcggcggcgacggcggcggcgaactgcgtgaacggaccgtcgctgaacgaggcggcctgcgccaccatcttccgcaacaacccgaacattccgttcggcatcggcgcgccgcaaggcgatccggtcggcggcttcattcagggctcggtcaattacgccaagctcgagacgcgcggcctggacttcacagtcaactacggcttcgacttcgaagagatgatgggccgcaactggggtcgtctggactactcgctgggcggtctgtacctgatcgagcagcagcagttcctgaacgccgaggatgcttcggacttcgacgaactggtcagcacgcccttctatccgaaggtgcgcttcacctcctcgctgacctatacgcccaacgagatctggagcgtaaactggacggcggactggcagacgtcgcaggacatcatcgagtcgcgcgacttcatcaacaactcggaccagcggtattactatcagacgcgcacgggcaacttcgcccgtcacgacctgacggtgcgctggaacgtgcgtgaggatctgtcggtgcgcgcgggcgtggtcaacgtcttcgacgccgagcagaaggactacctgggcacgaccctgtattccaacttcgacccctatggccgccgcttctttgtcggcctgaacttccgtccgttctaagagcgtccgaaaagccacgaactgaaagggcggtccgcaggggccgccctttttcgtcggcggaccgcctccgcttgcttgccagcccccctccccctctctaaacgggccgcttaaccgacaaccggatcgatccgccgcgagcgcgtctcgcgacggcttggcgtgcgcaagggatcacaacggccgtggatgcatcggacgtcagccacgacgagcgcgacgccatggtgcgggcggcgctggcggcgcagggcgacagcggcgtgacgccgcgccacacgctgttccacttccacggcgacggcgagcacggcgacctgaacgaggtggcgcgccgggccggcttcctgacgcgcggggccgacgactacacggtgctggagaccaccatggcggtggacgaggcgtcgttctccgccacatcggcgatgatgcaatcctgggccgcggccttcctgctggactatgacggctgggaatgcgcggtcgtgacgaactagaacaacaagaggcctgatccatgcccaagcgcacagacatccgctcgatcctgatcatcggcgccggccccatcgtgatcggccaggcgtgcgagttcgactattcgggcgtgcaggcgtgcaaggcgctgaaggccgaaggctaccgggtcatcctggtcaactcgaacccggccaccatcatgaccgacccggaggtggccgacgccacctacatcgagccgatcacgccggagatcgtggaaaagatcatcgcccgcgagaagccggacgccctgttgcccaccatgggcggccagacggcgctgaacaccgctctggcgctggacgcctcgggcgccctggcccgccacggcgtggagatgatcggggcgcgcgccgaggtcatcgacaaggccgaggatcgccagaaattccgcgacgccatggacacgctgggtctggagagcccccgctcccacgcggcgcacaccatggacgaggcgctggacgggctggagttcgtgggcctgcccgccatcatccgcccctccttcaccctggccggcaccggcggcggcatcgcctataaccgcgaggagttcgaggagatcgtcgcccgcggcctggacctgtcgccgaccaccgaggtgctgatcgaggaaagcgtgctgggctggaaggagtacgagatggaggtcgtccgcgacaaggcggacaactgcatcatcatctgctccatcgagaacatcgatcccatgggcgtccacacgggcgacagcatcaccgtggcccccgccctgaccctgaccgacaaggaatatcaggcgatgcggaccggctcgatcaacgtgctgcgcgagatcggggtcgagacgggcggctcgaacgtccagtgggcgatcaacccggcggacggccgcatggtggtgatcgagatgaacccgcgcgtgtcgcgctcgtcggcgctggcgtccaaggccaccggcttcccgatcgccaaggtcgcggcgcgcctggcggtcggctacaccctggacgagctgaccaacgacatcacccaagtgacgccggcgagctttgagccgtcgatcgactatgtggtcaccaagatcccgcgcttcgcgttcgagaagtatccgggcgccgaggcgtcgctgacaacctcgatgaagtcggtgggcgaggtcatggccatcggccgcacctttcaggaatcgatgcagaaggcgctgcgggggctggagacgggcctctccggcttcgatgagatcgagatcgaaggcgtgggtggggacggcgaggagacctcgatccgcgcggcggtgatccgggcgctgggccaacccacgcccgaccgcatccgcgtcatcgcccaggccttccgccacggcctgtcggtcgaggaggtgcacgccgcctgctcctacgagccctggttcctgcgccagatcgccgagatcgtccgcaccgagggccgcgtgcgcgccgccggcctgccggccgacgcgaccgagttccgccgcctcaaggccatgggcttctccgacgcgcgcctggcgcagctgaccggccagggcgaaaagcaggtccgcgatgctcgccgcggcctggacgtgcgtccggtgttcaagcgcatcgacacctgcgcggccgagttcgcctcggccaccgcctatatgtattcgacctatgagaccggcgccctgggccaggtgccggagaacgaagccgagccgtcggataggaagaaggcggtgatcctgggcggcggcccgaaccgcatcggccagggcatcgagttcgactactgctgctgccacgccgcttttgcgttcgacgacatcggcgtcgaaagcatcatggtcaactgcaacccggagaccgtgtcgaccgactacgacacctccgaccggctgtatttcgagccgctgacagccgaggacgtgctggagctgatcgaggtcgagcgttcgcggggcgagctgatcggcgtggtggtgcagttcggcggccagacgccgctgaagctggcgcatgcgctgcgggacgatggcgtgccggtgctgggcacctccgtcgactccatcgacctggcagaggaccgcgagcggttccagcagatgctggaggccatcggcctgcgccagccgccgaacgccctcgcccgcagcgccgaggaagccgcggggaaagcggaagaggtcggctatcccgtcgtgctgcgcccctcctacgtgctgggcgggcgcggcatgatgatcgtccacgatcgcgagcagctggaccgctacgtccatgaagccatgcgcgtctcgggtgacgatccggtgctgatcgaccactatctgaaccgcgccaccgaggtggacgtggacgccctgtgcgacgacgagaccgtcttcgtcgccggcgtgctggagcatatcgaggaggcgggcgtccattcgggcgacagcgcctgctccatgccgccctattcgctgtcggccgcaacggtcgccgagctgaagcgccagaccgaggccatggcgcgcgcgctcaaggtgcgcggcctgatgaacgtccagttcgccatcgaggagccgcacggggccgagccgcgcatcttcgtgctggaagtgaacccgcgcgccagccgcaccgcgccgttcgtcgccaagaccatcggtcagcccatcgccgccatcgccgccaaggtcatggccggcgtgccgctgtcctcctttggcctcgccgacaagccgtacgaccacatcgcggtcaaggaggcggttttccccttcgcccgcttcgccggggtggacacggtgttgggtcccgagatgcgctcgaccggcgaggtcatgggcctggactggaagcgcgacggcgagacggacatggcccccgccttcgcccgcgccttcgccaagtcgcagatcggcggcggcacgacgctgccgaccgccggccgcgccttcatctcggtcaaggacgaggacaagcccttcatcctggacgccgcccggacccttctggccgagggcttctccctgatcgcgaccggcggcacccacgcctatctggtcgagcaggggatcgaggtcggactggtcaagaaagtgctggagggccgcccccacatcgtcgacgccatgaagaacggcgaggttcagctggtcttcaacaccacctcgggcaagcagtcgctgcaggacagcttctcgcttcgccgcaccgccctgatgatgaagatcccctactacaccaccaccgcaggcgccctggccgccgcccaggccatcggcgccatcaaggccggcgacctcgacgtccgtccgatccaggcctacgcctgatgaccaaagggagccgccgcatcgtcctggcgaccggcggctcccttggcgatcttcatccggtgatcgcgctgggcaaggcgctggcggcgcgcggctgccaggccgagatcgccaccgcgcgcgactatcgtctcaaggtcgaggccgaggggctggtgttccatgaggtggggcccagcctcgcccggctggaagccgacctcggcctgaacatcgcgcagctgaccgaccgcatcgcccgctcggatcgcttcctgttcgaagaggtgatgctgccttacgccgccagcagcacacgccagatgatcgccgccagcgaaggggcggccctcatcgtcggcctgtctttcgccgtcggcgccgccatcgcggccgagcgtctgggcctagcctatgtcgccgtgtcgcttcagcctacgaccgtcttctcggcctatgatccgccgttcctgccgcgtgttccctggctcaggcccgcgcaaggcggccttcagctatggctgaaccgcacgaccctggcgatcggccggcgcaccaccgcctcctggacccgcaggatcaacggcgtccggcgcgatctcggcgtcggtccggcggccggcgacatcttttttgacgctctggctggggccgacctggcgcttggcctgtactcgccggtcctcggcgagcgccagccggacgcccgcgcgaacttccacgtcgtaggctacgccccctacgacagcgaggcgggcggccctccggttctggccgaagcgctgcgccgcttcctccacgagggcgagccgccgatcgtcttcaccctgggcagcgcggtggtgaacatcgccggcgacttctatcggcaaagcctaagggccgcgcgcgcgctgggccgtcgctccgtgctgctggtcggacccggcggggacctgggcgcggcgaacgggcccgacgcgatcgccgtcccgtacgcaccctattccctgctgtttccccgcgcagccgccgtggtgcatcagggcggcgtcggcacgacccagcaggcgcttcgcgccggacggccgcagctggtcgtgccgcacctgggcgaccagcacgacaacgccgcgcgggtccgacgcctcggcgccggcctgacgctccgtcgcgggcgctatgcgccggatgcggaagccgcgctgtctctcctgcttggcgaaccgcgcttcggcctgcgtgcggacgcgctgggcgccctcacccgcgacgaggacggcgcagccgccgccgccgagctgatcgtcgggatgatcgattagatcgccgcgccgggatccggttcgggcgcctcgtcgccgccctggatgatgcgggtggcggcgaggtcggcggtgacgttgccgacggtgcgcaggatgtccggcaccacctccaccgccagaagcagcggcagcacgcccagcgggcagcccatggccaggcagatgggacccacggcggcgaaaaagctgacctgccccggcagacccacgctggcgatcgagacggcaaaggcggtcaggccgccggcgatcagggcgggcaaacccaactcgatcccgttcagctgggcgacatagaggcagacggcgaggttcgcgacggggctggtcaggcgaaacaccgccaccgccagcggcagcaccaggccggcggtcgaggcacggatgcccagcgccgtgcgtgcgcggtccaccatggccggcaggctggccagcgacgactgggtggagaaggccaccacctgcgccggtgcgaccgcctgggcgaagcggcccaggctgatccggccgaacgccgtcgcgaccgcataggtcaagaaaatcaggcccagctggctgaggcagacgatggcgatgtagtgaccgagcgtgcccgcgacgccgagccccgcgcgcaggcccacgccgagcgccagggcgaacacaccgaccggcgccgccagcagcacccagtggacgatcaccaccatggcctcggccacggcctcgaagaaggtcgacagggagcgccgaagctcggcccggagccgggtggccgcgaagccgaacacgatggcgaagacgaccaccgccagcacgccgtcgtcggccgccgcctggatcaggttggcgggagccaggctgttgaggaacgcctgaaggccgtccgtctgagccgccgccccaacctccgccgccgcctcggcggggatgcccgccaaaagcgcgcgcccggcctcaggatcgatcggccacagcgtcagcaggcccagcccggccagaaccccatagatcaccgccccgctcagcatcacgccgaagacgaccagcgcccgcaccgccagccgcccggtcgcggccgcatcggcgatggacacgatcccggtgaccagcaggccgaacaccagcggaatgacggtgatcctgagcgcgttcagccacacctggcccaactgctccaccacgcccacggcgcccagcgccagcggcgagcccgacccttgcgccagcgcgccgaccaccagccccgcgaccaggcccaccaccacgcggaagctcaaggaggacagaaacacggacaggcgtcgggaagaggtcataaggatcctggaccggcgacccggccggtcgcgtcacgccgtcgcggggaggcggcggtcatgaacggatcatgcgggcgatgcgttcatccggcaacacagaaggaaaccgatcatggccctgtcccgcatcgccaccgccgccgccggcctgctgctgtcgcgcggcggtcgtcgcttcgccggtcgtcacgccggcaagctggcgctcgccaccctggcctacgaggcctggcgcacccaccaggccaagaagaccggcggctacgcctcggcgcccaagggcggcccccgcccgcgctggagcggccgccgtccgctgtagaggctcgacagcgcgccggtcgcccggccatagtcgggcatgatcatcgtccatcatctgaacgacagtcgctcgcagcgggtgctgtggctgctcgaggagctcggcctgccctatgaggtgcggcgctatcagcgcgaccccaagacgcgcctggcgcccgccgagctgcgcgccatccatccgctgggcaagtcgccggtgatcgaggacggcgacgtccgcgtggcggagaccggcgcgatcgtcgaatacctgctggacacacatggcgcgggcctcctgcgtccgcccgcaggcacggaagacggtcgtcggttcacctactggctgcattacgccgagggttccgccatgccgccgctgctgctgaagctggtgttcggcctgctgccggcccgctcccccgcccttttgaagccgctggtccgacagatcgccggcaaggcgcagaccgggttcgtcgatccgcagttgaaggcccacgtcgccttctgggaggcggagctcggacgctcggcctggttcgcgggcgatgcgttcagcgccgcggacatcatgatgagctttccggtggaggcgggcgccgaccgcgccttcgaccgcaccgcctatccgcgcctggacgcctttctccagacgatccacgcacgccccgcctatcgccgggcgcttgagcgcggaggcccctacacctacgcgtgaacgctggggcgacccggcaaccggcgcgcgtcttgcacgtttggatcgcatgcgtatccaaaccatccagatcgttgcgggtctcctggccgccgtcgcctttgttctggccttcatggccgccggggcggtgatcgcctccagcctgttcatggtgctgggcatggcggcgctggcctggctggcctggagcctgatcaagcgggtgggtcgccaccaccgcacgtcgcgcccgaccagcggcgcctgagggggccgtccgcgcggcccttgagtttctgaacacggcgccctagcttattccccccggccgcgaccgccccgcgacctttgccgtgccgatctccaaactttccagtctccgggcgaaaacaagaaaatcacgacacaatggaaaaagtgccgatgacggccgagggctatcgcgtcctcgacgatcaactgaagcaattgaagtcggtcgaacggccgagcgtcatcgccgccatttccgaggcgcgcgagcatggcgacctgtccgaaaacgccgagtatcatgcagccaaggagcgccagggctggatcgagggccagatcgccgagatcgaggacaagatcagccgcgcccaggtcatcgacgtgtccaagctgtccggcgatcaggtcaagttcggcgccaccgtcaccgtggtggacgaggacaccgaggaagaaagccgctaccagatcgtcggcgagcacgaggccgacgtgaaggggggcaagatctccatcgcctcgcccatcgcccgcgccatgatctccaaggaagtcggcgacgtggtcgaggtgaacacccccggcggcgtcaaggcgtacgaaatcctgaaggtcgagtggaagtaggctgagcctcctgcggcggcgtcaatcgccgccccctccatcgccgccgctgtcgccgccatccgtgtgatccgcgtggtggacgaccggcgcgccgccgtcgccagcgtcagacttgctccgcttcggcttcgccgacagggccacgcccaaccccgctccaatggccgcgcccaggctcagccacagcgccatgtcgtctgtcgccgcgccgatcgccgcaccgatcgagacgcccagggcgacccctatcggcagcctctccgcaccggtgcgcttcttcatgcccgcctccgcgatgaagcggcagactagcatcgcatccgacggaatcagcgactaaatagcggccatgacccaagccgccccccgtcccgtccgcgtcgccatcatcggttcaggccccgccggctggaccgccgccatctacgccgcccgcgcctcgctcaacccggtggtgatcgccggcatccagccgggcggccagctgaccatcaccaccgacgtcgagaactacccgggtttcgcagacaccatccaggggccctggctgatggagcagatgcaggcgcaggccctgcacgtcgggacggaggtgatccacgacatcgtcacctcggccgacctgtcgcaacgcccctttcgactgacgctggacagcggcgagcagattctagcggagaccgtgatcatctcgaccggcgcccaggccaagtggctggggctggagtcggaagcggcctatcagggcttcggcgtctcggcctgcgccacctgcgacggcttcttctatcgcggcaaggaagtggtcgtggtcggcggcggcaacacggcggttgaggaggcgctgttcctgaccaacttcgcctccaaggtgacggtggtccaccgccgcgacgagttccgcgccgagaagatcctgcaggaccgcctgttcgctcaccccaaggtcgaggtgatctggaaccacgccgtggaggagatcctgggtgtcgtcgacggcgtggcgcgcaacgtcacgggcgtccggctgaagcacgcgagcgacggctcaagccgcgagatcgccgccgacggcgtcttcatcgccatcggccacgcgccgtcgtcggaactgttcaagggtcagctggagacgaactcaggcggctatctgcgggtgacgccgggcacggcctcgaccgccatcgaaggggtctgggcggccggcgacgtgaccgacgacgtctatcgccaggccgtcaccgccgccggcatgggctgcatggccgcgctggaggccagccgcttcctggccgagcaggaccacaaggccgccggacatccgatcccgcacaaggaagccgaaaagatcggggtctggtgaccgtctttggtcaccggcgggttcagccgaacagttgcagcccgaccggcgtggcgacggaagactgcccgccgcggcgtcgcagggcgtaatcgaccgcggtctgcacggcctgttcgtcggtcggcttggacagcacgccgatcgtgccggcgaccccgttgcggaccatccccggattggcggtcatgaacaggacggtgacgccctgctcctgacccagctcccgccccagatcgataccggtggcgccgtcggacaggtgtatgtccaccagggccagatcgacctccgtctcgcggacaaggtcgcgcgcggccttcgcggtcgcggcgacgccgaccacctcgtggccaaggtcctccagcacgaagcgcagctccatcgccaccagcacttcgtcttcgatgatcagaatacgcgcgggcatcaacagcgggatccagtgatcggtcgaaacgccactctggagcaatagttccaacaatcggtcaacgctctgcggcgccggcggcccgtcgccgcgccagcgccgttgccggcagatccacaagaatcctaagcccctccggccgccactcgtggctgagcttgcctccaagctgcgcctccaccgaaagcttggccagcgaggagccgaagcccgcccgctccggcgaaccttcgacgacaggtccgccggtctccacccacttcagcaggaagcgatctccgacaagggcggtgctcaggtccacccgcccgtcgccgttggacagcgctccgtatttcgccgcattggtcgccagttcatggaacagcagcgcgacggaggtggcggcctggtcgtcgaacaccgcgtcgtcgcccgagatcctcacccgggacgcgccctccccgtccgcatagggctggaaaagcgagtgcagaaaggcgtgcagtgtggtcggtcccaccaacggacgggaggcttccgtatgcggcctgacgaattcatgcgcgcgcgccagagccgcgatgcgggtccgcagcgagccggcgaacggcttggcttccggatactgccgcgcggacagagccaccagcgcgctgatgaccgcgaagatgttcttgatcctgtggctcagctcctggctgatcagctcgcgaccgtgctccagttgcttcaagtcatcgatgtcggtgcaggtgccgaaccagcgcgtgatctcgccctcaccgttgcgcaagctcaaggctcggccgagtacccagcggtatacccccgagtggtgcctcaaccgatattcgatgtcgtacggttcgcccgtctccagactatgacgccagcggctccaggcccgttcgcgatcatccggatgaaacagctcattccattcgtcgccgtcgcttgaccccgccggcacgccggtaaactcgtaccagcgcgcattatagaagtcgtgatagccgtcaggccgggtcgaccaaaccatctgcggcatggcgtcggtcaggacgcgaaaccgggcctcgctttcgctcaacgccgaggcgatctcggcaaggcgttggtccttgtgccgacgatcggtcacatcaaccgagacgccgggcaagcgcaccacctttccggtcgcgtcccgataggcccgcccccgcgccacgacccagcgcacctcgcctcgcgggtcgatcaaacgatattcgctaacgaacggttcgtcggacgcgatcgccgcctcgatgtcacgcgccagctgttcgcgatcgtcgggatgaacgtgacgggtgaagcgctcgatcggcacgcctgccccggcttcttccacgctgacgccgtactgtcgcgcgaaaccggcatcggccaccacccgatcctcgacgatgttccagtcccattcgccgacatggtcggatgcgtccagaacgcgacggctgacatcctcggccaaccgcttctgctgcagcgcgcgacgaaggcgcagttgaaccataacctgggacgccagcgtgcgcagcgtctgctcctgaagctcggaaaggccctccggcctcgggcgggtgtccagcacgcacagggtgccgatcggaagccccgcctcgtccttcagcagcaccccggcatagaaacgaagcttggcttcgcccgtgactaacgggttgcactcgaaccgaggatcgagagtggcgtcgcgcaccaccatgctgtcctgctcgagcagcgcccgggcgcagaatgagctgtccagcggcgtctcgcgcacgcccagaccgacctcggccttgaaccactggcggtccgtgtcgatcaggttcacgaccgcgatcggcgcttcgcagatgcgtgcaaccagcgccacgatgtcgtcaaaagccggctctcgttcggtgtccaggatgtcgaacgaacgcaatgcggcgacacgctcggcctcgtcccacccaggactgtcttgtttcaggtgggtcacgcccggaagtcctctcgccggcggccaatgccgctcaaccccaatgcgtccacacacatggatgttgcaagcgcaagtcgccggttcgcatcagctggccggacgcccgacttcctccacctccatgatcgccacgcccggcggaggcggagccactggtgcggctgtggggacgggggcggccttggaggcctccagcgcctgaagacgagcgttgatggccttgacctcgtcctgggtcggcaggcgacgtccccccaggctggcgacgcctaccacgcgggtctgaccgtccacctcgactgtcttcagggcctcggcggcctcgggcggcaggccgccggtggcctcgcccgcctcggggcccgtcttgatcaggcgcgggcgcgaaaagcgcgcctcgtcgatcagcggctcatgccccctgtagacggtgcggaaggcggcggtttcgccatagacgcccttccagcgatagaagatgtgcgcgccgatctgggtgatcttggccaccgtcggcgcccaccagggatgcacatagtcggcgtgatagtgggtcgcggtgccgacctgcgtcgccacatggccggacagggcgcgctccgccacgatccgcgcgcggtcccaggcccaggccaccggcgtctgggccagcgagccgtcgcaggtgaagctgaactggcagcccgtgacgcgctcggcgccttcgaacaccacgccgcagacggtgttggcgtagttggggtcccggacgcggttcagcaccacctgcgccaccgcctcctggccgttcgtcggctccagcgccgcctcgaaatagaccgcctgggtcaggcagcgcagcgcgcggcggcggtcctcggccgtggcggcgttgaagacaaagggcttggccggccgcagggccccggtggtcggcgtagccgcgttcagcctctgagcctccagcccgctgcggccgagatcgagccccggccgcccggccaggctcaggctctcccaacctggcgtaagccccagcagcgcagggtgcagcaccgacggatcatgacgtgcggccacggacagttgcgccgggtccatgcgcgacgtcagggccgagagccccttaggtcccagatcgccgccggtcagccgcgacacccgttcggcggtgcgatccacgtccgggcgcgggctcgatccggccgacatggcgacgccgagaacggcagccacggccggcgcggccgctcccgcccgcctcagcagccccttgatccggttctgatccacgcggcttttcctgggcccgcctcagcggccgcccagggtcgagcgcagcatccaggcgaacttctcatgcgcgcccaggcgctgggtcaggaggtcgacggtgacgtcgtcgccgtcctcgtccgccacctcgatcgcggcgcgcatggtggcgatcagcgtctcgtggtcgcgcatcagctcgttcagcatctcgggggcgctcttttccgggtcgccgtccttgatcgaggtcaggttggcgaaggcggcgtagccctgcggcgccaggacgccgagcgcccggatgcgttcggccacatcgtccaacgcctcccacatgtcgcggtactgctgctccagcaggttgtgcagggcgaagaactcaggcccgcggacgttccagtgatagccgtgggtcttcagatagacggcgtagctgtcggccagaaccttggtcagttcagaggcgacggcgctgcgttcggacgccgaaaggccggtgtcgatggtggcggtcatgggttgctcccctggtcgttacgaacgcccgcacaaacgggcttggccgacgagccgcagcaacgcgcaagccggcgtgatgttgcacctatatggctatggcggagccaaacgcgagtccgcccggttctcgcccggcgccatgcgcgctgacaaaaagggcgcgccgcgatgccgcgacgcgcccttgagggatcagtcaggaaggggtcagcgcttgctgcgcgccttgcgggcggcgtagcgggcgtcgcgcgccgccttctgttcttccttggtcagttgcttgcgctccttgcgggcggcgcgcttctcggcgtcgacggcttcctgggccaggcgctcggcctccagacgcgcggcttccttttccgccttttcgcggcgcagctcggccttcgccagctcgtgctgctggcgcagcgcctccttctcggccgcgcgcttctcggccagcttgtcgaactcgggatccggcgcagccgccttgggcttgaacttcgccagcagcgccttcttggcctcctgctgggcggtgatgcggtcggagaagcctgttttcagatctttcatgcggagaggtcgggtgtcctgcgatatgggccgccagggcggtcagaagggtcatgcggcgtgcagcggaccggaagcgcgccgcacaaagcggaaacgcctgccgaaatcaaggttccggccgctgatcgcatcgacggcgaaagcctctgggacggtttttccgcgtttggtgcagataggacgcgatggcgggaaatcaaccgccgggccaccggcgtcagcgcggcttggccgcttggcccgcggccgcgccggccgctccgcccacggcggcgccgaccggacccccgaccagcgcgcccgccagggctccggtcgccgagcgctgctcgttggtcgtgccgcaggcgcctagccccgccgctcccagcacaaccagggacagacctgcgatgcggaccatgaccgccccccttgctgaatcttcagccgcctcaacggtgcagcctggcccgggttccgaatcgccgttcgtgtagaacgaccgcgccgccacttccgctcagacttgcagggcctgctcgtgagaagatgattcatttgtcgatgttggtctcgacgccgtcagcgagcatccggcaagtacagcgcggaccatctgtactaagaccacgacacgcgctttgcgctgctcgacgcagcttggaaatacacaacggattccggcctttaacccgccacttgccctccgaccacattgacgccacaaaggactgtctaaaggcccgccgccaagcgccgggctcgcaagccgtgcgttagttgcggatcggactggcggcgtctctccggccgatcgcgcaagactacccgtgggcagcgtttcccgccctgctgatcaggactgagccattgtcgcatccttcgcagctccctgcgtcgccttcggtcgatcgcaagctccgcatccgtccggttgcggccgctgcgatgttcgggggggtggccgggattgcgatcggttgcgcctacctaggtggagtgacggcgcgcgctacgacggtgcgcgcccaggccgagcgcctgcagggcgcctccaacgcagggttcaccgaagaagcgctgtccgccgcggccggcggcctggacgccagcgccctggccatcgcgcgccggcatgatccctacacggtcgcgggcgccgcccagcgcgaccgacaggcggaactgctgtccgcgcgcctggagcagttgcgccccgccggcgatccgatgctgcgtcgtgtcagcctgaacacccccttcgccgactccgccggcggctcggccctgaggctggaccacgccttggacgccgcgcgggatctcgattgcctgacgcaggccgtctactacgaggcccgcggcgagggccgggacggcatgaaggccgtggcccaggtggttctgaaccgcgtccgccacccggcgtttccgaaaaccgtctgcggcgtggttttccagggcgccgcgcggtccagcggatgccaattcagcttcacctgctcgggcgtcatgcgcggacgcgtcaaccgcgccgcctggaaccgctcgcgcgacatcgccaccaaggccctttccggacaggtcttttcgggcgtgggctcggccactcactttcacaccacaggggtggcgccgggctggcgcaactccctggtccaggtcagccaggtcggccagcacctgttctaccgcttcggctccggacgcccgtcgcccgccctcacctacgcggcccgccccgctcagccggagcgtccgcgcctgatccaggctgggatcgaccctgtcgagaccgcccgacgcgccggacaggcggtcgcctattcgctggctctggctcaggacggcgtcaagccggagacaccgcccgcaaccgcagtctccacgtcggtccccgcggctgcgccggctccggctccggctccgagggccgcaaagcctgtcgagcggccgcccgaaacagcggcggccaagcccgagatcacggtcgccgccgcctcggcctagagccgccgctccgcctcaggcgtcgcgatcgcccttggacgaacggtgcgcatcgtcatggctgtgcttcaggtcgcgctcgccgccaccgcccgagaccttgctgttgcggccgttggtcgggccgccttcgcgcggatcctcgaactccggcggctcggccttggcgttttgatggcttgagccaggcccgccccagcgcttttcatcgaccggttcgggattgtgctggttgttggacatgatcaacgatctccggacttgtgctgcggggtcaggttctggttagcgttgccgaaccgcccctgctgatcgaggttcgcgtcggcgtcgcccggctgtccggactgaagcccggttgcgcggtcgcgcgcatcgcccttcgcttcggggttggcgtccgaaccgccgccggggctgatctgatcctcgggcacgtgaggcgtcttgctcatcgatggctctccttgtccgtgtacagggagaaaacccgcccgcttcgggcccgttccaaaccgcagcgcttcagagggcgtccaggccgatgtccagcaccggcgccgaatgggtcagggcgccgaccgagatgacgtccaccccggtttcggcgatccctcgcaccgtgctcagatcgacgccccccgaggcctccagcaccacccgcccctccgcgcgccgcaccgcttcgcgcaggtcgtccagagcgaagttgtccagcatgatcacgtccgggccggcgccctccgggatcaacgccagcgcctcgtccagctgatccagcccgtccacctcgacctcgaccttcatcagatgcggcgcgaaggcgcgggcgcgtcggaccgcctcccccactccgccgcagaccgccacgtggttgtccttgatcaggatggcgtcatccaggccgaagcggtggttgatcccgccgccgcaggccacggcgtgcttctccagcgcgcgcaggccgggcgtggtcttgcgggtgtcggcgatgcgcgccttcgtgccccgcaccgcctccacataggcgcgcgtcagggtggccacgccgcacagtcgccccagcaggttcagcgccgtgcgctcggccgacagaaaggcgcgggcgtccgcctcgacctcggccagcaccgcgccggcttcgaaggcgtcgccgtcgcgcaggcgcaggtcgatggacgcggccggatccgtcgtcgccaccgcgagcctgacgcagtcgatccccgccagcacccccgccttgcgcgcggtgaaggccgcccgcatccgcgccccctcggggatgcaggccatggccgtcatgtcgcccgcacgcccgaggtcctcggccagcgccagccgcaccaccggctcgatcatcaggttcggcagcgatctcattcggcggcctccagcgcccgcgcgacgtgcgcgacctgcatccggctatgtcgcgccacactgtcggtatgggggaagtcgccgcgatagtggccgccccggctctcttctctggccagcgccgcctgggcgatcagccgggcggcggtcaggaccggcgcgcccggcgcccgggtctcgatccgggcgatcagcgacaacagccgctccagccccgcccgcgtgcgctccacccccgcatgcagcgtcatggcctcgcgcagcgcctgaaggtccgccgaactcagctccgggccgatccgcgccggcaacggcacctcgccgccagtctcgcgcgccgccgccatccccgccctgcgcccgaacgcggccgcctccagcagcgagttggaggccagtcggttggccccgtgcacgccggtcgccgcgcactcgcccacggcgaacaggccgggcgcggccgtgcggccgtccgcatccgccgcgatgccgcccatgtggtagtggcaggccgccatcaccggaatcggactgacgcggggatccagcccgctccgcatgcaggcggcgaagaccgctggaaaggcctgcgggaattcgcggcccacggctcgcctcgcatccagaaaggcgccgcgcccttcgatccgcgcccggtgcaccgcccgcgccaccacgtcgcgcggctgcaggtcggcgtcctccgcttcgcccagcagaaggcgcccctccccgtccaccagtcgcgccccctcgccgcgcaaggcctcggtcgccaacggcgcgggatcgagacccacgtccatggcggtggggtggaactgcacgaactccggatccaggatttccgcccccgcctcataggccagggccatgccctcgcccttcagcgcggcgggcgtggtggtggcggcgaacagcccgccggccccgccggtcgccagcaccacggcgcgcgccgccacctcgaccagccgtccgtcgcgcgtgaccgccgcgccgacgacacggccggtcgggtccttcagcaagcccttcagcgatccgtcttcccacacctcgaccagaggctgggcgcgcacggcggcggcgaccgccgacaggatcgcccggcccgctccgtcgccgccgacccgcgccacgcgcgcgacggagtgcgccgcttccaggctgacggcgaagccgccgcgcccatcgcggtcaaagggcgcgcccagcgacgtcagccactgcacggtggcgcgtccggcctgggtcagccgcagggcggcgtcggcgtccaccaggcccgcgcccgccgcggccgtgtccgccgcatgcagctcggcgctgtcctgaaccgtcagggcggcggcgatgcccccctgggcccaggcggaagagcagccgctcagcagcggttcgggcgtcaccgccagcacggacgcgcccgcgcgcgcggcctccagcgcggcgctgaggcccgccagccccgcgccgacgatcagcacgccgtcgtgccggatgcgaatcatggtcagcgcactcccaggtagctgaggcccagccggatcgcctcgcccgtgtcgccgtcggccaccggcagcagggcgcccacggcggcggctgcacacagagcgcccgtcgccagatacagggcgaggctccgtcccgcctccggccagctcagcgtgccccaggccgggcgccacaccccgcgcttaagatggctgaacaccgccagcgccagaaaggcggccaggatgaagcgtccggtggtcagcccccaccagaccaccgcaatcccgatgaccagaagcacaagctgctccagcctcggatgcagccgcgtcagcacgggccccagcgccttggacccgtccagcggcggagcgggaaccaggttcaccaggttcagcatggcgataaagaaggccccgatcagccactctccctgccccgtcgccatccacacgcccgcgaacgggatcatggccaagaggccgaacgccggtccggccagcgacaccagcaccccgtgccattcgctctgcggctcgcgccgcgcctgggccagtccgcccaggaacgggatgatgtagacgcgcgccggccccatgccgaggcggttcatggctagggcgtgcccggcctcgtgcacgaacaggccgatcagcaccgctccggccacgatgacgctgccggtgatccaccaaaggaaggccgccatcagcagggtcgaggccagcgtccagaccaggttctggtccttctcgacaggcgcagcggcggcggtcgccggcgtcgcctcggcgggcgcggagtcgggccgagggtcccacggacccggtcggtggatgggggtgtcggtgtcgctcatggcattttagatgggcgctgcggtcggccgaaacgaggcggccgaacgccgcgtctcagatcagctccaccgcgacgtgatggcgcgcgcgcaccaggtcatagcgggccgggatggtcggaggcggcaggtcgatcatccgctgcaccgccagccttccacgctcggccacgtcctcgggcaccgtcacctcgaattgcatgtggcgcagacagtcgcggatgttcagcagggtgatgcgcttcatgtgcgggcacatgttgcatggcccgatgaactgcgtgcccggcgcgtcggcggcgacgttggaggccatggagcattctgtgatcatcaccacctggcggggctttcgctgctccacatagtcgctcatcgccgcggtcgatccggcgaagtcggcggccgacagcacctcttccggacattcggggtgcgccagaatctctgcctcgggccaggcggcgcgcatctcggcgatgtcggcggcggtgaagcgttcgtgcacctcgcagcggcccttccaggcgatgatccccacgcgggtctgcgccgccacgttgcgggccaggaactcgtcggggatcaggatgacgcggtcgacgccccactccttcgccgcccattccaccacctgcacggcgttggcggaggtgcagcagatgtcggtctcggccttcacgtcggccgtggtgttgacataggtcacgaccggcaggcccggatagcgcgccttgatcagccgcacgtccgacccggtgatcgacgtcgccagcgaacagcccgccagaggatcgggaatcagcaccgtcttgtccgggctgaggatcttggaggtctcggccatgaagtgcccgcccgcctgcacgatcacgcgcgcatcggaccgcgccgcctccttggccaggcccaggctgtcgccgacgtagtcgcccacgccatggaagatgtccggcgtcatgtagttgtgggccaggatcaccgcgtcgcgctcgcgcttcagcgcattgatctcgctgatcagggcggcctgcgccggccactccagcggggtgacgtggtccttgaccttggcccagactccggcggtctcccgctctagcgcctttgtcagcccgaacgctccgtccgccatcatgcctgctcctgaccttatgctcacattcagcataagcaggcgcaatgtaggccgatcccggagcgacgcaagcgggtgcacgctcatgaccgctgcagaccgaagcagcgagaacttcagagtctcgcaacctttggttgtctaccttggtcgatgtaatcgggggattgcatcatgttcaacgtcatcgactgtgtctggaaccagcacgacctgcggctggtggcgctcgccgccgccatctggctggtcggcggcctcgccttctttctgctgctgagccgcgcgggcgacagcggcccggctcgtcgcgatcagtgggtcgccgtggcggctgccgccggcggggtcggcgtgtggagcacccacttcgtggccatgctggcctatgacggaggcatgccgatgagctttggcccgtccctgaccgtcctgtcggtggcggtggcggtcggcatgttctggatcgcgctgcgggtgttcatggcgcagccctcgccggcggggcgtcttggggccggcgtgctgttcagcctgggcgtcgcggccatgcatttcaccggcatggcggcagtccaggcgtcggctcgtctgcactatgaccttgaacagattgccgtcgcggccctgctgggcgccgcgctgatcagcgcggcctttcatgtgttcgcccggttgcgcggcccggcgcgcataggcgttcccgcgttactcagcctgctgggcatctgcgtgatgcacttcatcggcatgtcggccacgaccctcatcccggaccccacggtggcggggccgcagggcgaggtcagccgggtgtggctgatcggggccatcgtggtcgccgccaccctgttgatcctgctgacggcggcggcggcctttgtcgaccgatgcctgaccgacctgcgcggtctgaccgaagcctcgctggagggtctgatgatcgtgcgcgacggccgcatcctggaggtcaacgcccgctttgcggccctcagcggacgcaagccggcgatgctgctgggccaaccggccgacgcggtgctgaccgtctcatccgcggatggcgtgtcctcgatcggcgccactccgatcgaggcggccctgccccggcccgacgccgagccgaggatcgtcgaggtctgcgcccacaccgtcgaatatcgtggccgcgagtgccaggtgctggccgtgcgcgacctgaccgagaaaaaggaagcccagcgccagatcgagcatctggcgcgtcacgacgccctgaccgacctgcccaaccgcgccctgctggaggaacggctggagcacgccgtcgcctggtcgcgccgcacgcgcgatccggtggccgtgctggcgctggacctcgatcggttcaaggccgtcaacgacatcttcggccacgccgagggcgaccgcgttctgtgccgggtggccgatatcctgcgctcctgcacccgcaccgtggacaccgtcgcccgtatcggcggcgacgagttcgtgatcgtccaggtcggcgcggcccagccggaaggggccaagatcctggcggaccgcatcctctcgacctttgccgccgagatggacgtgacgcgcgatccgatggcggtgggcgtctccatcggcgtggcggtctatccggacgacgcgggcgatcccgacaccctgcgccacggcgcggacgtggctctttatcgcgccaagcaggccgggcgcggcgcggcgcgcttctttgaccagcagatggacgccgaggtccggaaccgccgcaacctggagcacgacctgcgccacgccatcctgcgtcgccagctgcacgtcgcctatcagccgctggtctccaccatcggcggcgcggtcgcgggctatgaggccctgctgcgctggaggcatccggtgatgggcgagatcagcccggaggtgttcatccccatcgccgaggacaccggctccatcgtggcgctgggcgaatgggtgctccgcgaggcgtgccgcacggccgcgacctggccggacgactacgccgtctccgtcaacgtctcgaccgtgcaattcaaggtggcgaccttgccggacctcgtggccacggtgctggccgagaccgacctgcacccgtcgcggctggaactagagatcactgagtccgtgctgatgaaggaccgcgcctcggcgcttcacaccctgaaccggctgaaggccttgggcgtgcggatcgtcatggacgacttcggcaccggctattcgtcgctcagcaacctgcagagcttccccttcgacaagatcaagatcgaccgcagcttcatcggcgcgatcgaggacgacgaggccgcacgatccatcatccgcgccattgtcggcctgggccgcggcctcaacctgccggtcgttgccgaaggtgtggagaccgaagcgcagcgtcgcatggtcgccgacgagggctgcccgcaggcgcagggcttcctgttcggccgccccggctccgccccggtgttcccggagcgaagcgaggcgaaagccgcttagttcttgcccgcccccggctcggccatgccgcggtgcatttcggccagggcggtctgcggcgtgacggccgccatggcggcttgcagcttgttcttcaggcccgccaccacgtcgccgtcgccgcgcttcatggcctcatagccggtcttggcgacgtcggccgggtcggacttgtccttgctctggcccaccgaggtgtccagcatgtcggcgcgttcgaagaactcggtgtccaccgggccgggcatcagcacggtgaccgacacgtcggtgtccttcagctcgttgcgcagggcgaaggagaagctgtctacgaacgccttggtgccgttgtagaccgcctggaacgatcccggcatcaggccggcgatggagccggtcagcaggatcttgccacgcccgcgcgtccgcatctcggcgccgaccttgtagagcaggcggatggtgccggtgatgttggtgttcacgacgtgcatgacgtcgttccagtcctgatccaggaaggcgtgtcccagaccatggccggcgttggccgccagggcgtcgatcgggcggccggccgcggcggcttaaagctcatccaccgcatccacctgtgacaggtccagctgcagggcggtgacctggacgcccagcgcctccagcgactgcttggcctcgacgatggcgggctggtcggcggcgatcagcaggtcatagccgtcctgggcgaacagcctggcgagttcatagccgatgccggacgaggcgccggtgacaagggcgagggggcgggcggtttcggcggacgtgacggccatggcgggggctccagaggcagggtgtgaggtgtcttctcaagccaccgcgcgcgcgtcggttccgctttcgtcccatcaggacagcggggaacgattctgaatcctaagacttgttttgagcctcaggaggaccgcatggccaacgaccccatctcgacggacgccgacgtggcgtccaccaacttcatcgacaaggaccagcacgagggcgagcacagcgcctcctcgattcaggcggtcatgatcaacaagccgcgtgaggagctttacgccttctggcgcgatttcgggaacctgccggcctttatgccgaacgtgaagtcggtgcagcagacggacgccaagcacacccgctggatcatcgacggccctggcggcaaggacatcgaactggacagcgagatcgtcgaggacatccccggcgagaagatcgcctggcgcggaaccgaaggctccgacctcgatcacgaaggctgggtttcgttcaaggagaacccctacggtcgcggcacggaggtccgggtcttcatcagctacgacccgccggccggtgcgctcggcaaaatcgtggccaaggtcatgcagcgcgagccgcgcgtgcaggcccgtcgcgagctgcgccgcttcaagcagctgatggaaacgggcgaggtctcgacctcgcaagcccccgccgccgcgccgcgcggctgatctcctctccattcaagaaagaacaatcgcatgcgcgcactcacctggcacggcaagcacgacgtccgcgtggacacggttcccgatcccgagatcgtcaatccgcgtgacgccatcatcaagatcaccgcgaccgccatctgcggctcggacctgcacctctacgacagcatgatcccgtccatgcacaagggcgacattctgggccatgagttcatgggcgaggtggtcgaggtcggccgcggcaacaccagcctgcaggtcggacaaaaggtggtggtgcccttcgtcatcgcctgcggctcctgcttcttctgcggcaaggagcagtattcggcctgcgacaactccaatccggccgacaagtccgacatctccgagactgcctacggctatccggtggccggcctgttcggctattcgcacatgaccggcggctatgcgggcggtcaggcccagtacgcgcgggtgccctattccgacgtagggcccatcgtgatcccggaaggcattccggatgaaaaggtgctgttcctgtccgacatcttcccgacgggctggatggcggcagagaacgcccagatcgagccaggcgacaccgtggccgtctggggctgcggcccagtcggacagttcgtgatcaagagcgcgatccacatgggcgccgcccgcgtcatcgccatcgaccatcagccagcgcgcctggcgctcgccaaggccaacggcgccgaggtcctcaactaccacgaggtcaaggtccgcgaggcgcttaaggagatgacggccggcatcggcccggacgcctgcatcgacgcggtcggcatggaggcgcacggcttcgctcccgacaacatcatcgacgccgtgaagcaggagaccaaggccggcaccgatcgccagcacgtcttccgcgaggccatcatggcctgtcgcaagggcggccgcgtctcggtgcccggcgtctatggcggcatcggcgacaagttcccgatcggcgccttcatggaaaagggcctgaccatcaagaccggccagacccacgtccagaagtacctgccgcacctgctcgagctgatcatggacggcaagatcgagaccaccgacatcatcagccaccgcctgccgctggaagaagcccccaccggctacaagaacttccacgacaatcccaacgagtggcgcaaggtcatcctgtcgccgcactaggcagcggcttcgggcgtgcagacaaaggggcgagggctcgaccgtcgccccttatctatgggcgcgccaccgctgcgcgttcatgctccagcagccagcgcttgcgctcgacccctccggcatagccggtcagggcgccgcccgcgccgatcacccggtggcagggcgtgacgatccccaccggattggcgccgttggccaggcccacggcgcgcaccgcggttggttgaccgatcgccgcggccagctggccatagctgcgcgtctccccggccgggattccgcgcagggccgcccagccccgccgctggaactccgtgccgccggtggccacggtcaggccgtcgaacgccttgaggtgtccggcgaaccacgcctccagcgccgcgcgcaccggttcgggcgcggcgccctccaccagttccacctcgccgtagtgacggatcagcagccgtcgcagcctcgcctcatagtcgtggaagtcgagcgcgcgcagcacgccatccgcatccgtcgcggtcagcacctgcccgatcgggctgtccatccgccccaggatcagccgcaggggttctctcttcatctcgcctctcccgtctccatcgcccgccgccagtagagggcgccgtccgcccgccacggccgccagccctcggcccgagcaaccagcgccggattttggatttccaaccggtcgtccgccagcctgttgtcgatgatccagtcgcccggcggccgcagtcccggccgctcggccatcgccgtcgccagcatgggatcggcggacagatcgcgcgcgatcgcctccgggtcggcggctaggtcgaacacgcgccgcacccgcgccagcacgcacggcagcgccttcagcgacgacagctcgaccgagacggccaagcggcccgccccgccgtcgcgcacggagacctcgccctccgcgccgtcaaccgacatggacaggcgccgcgtccagaccccgccccgcaccgtctccccttcgacccggcgcccggccagcgcctgcatcatcgccgcgacgtcatagggcgtgcggtagccgaggctcagcgtcagtccgccggacggggttcgctcgccgcgtcgcctcagcgccgagggcgggcggccgtagagcgtctgaaaagtctcgttgaagcgccgcacgctgccgaaccccgacgccagcgccacatcggccatcgacaggtccgagtcgtggatcagcgtcttggccagcagcacccgccgcgtctgcgccacgctgaccggggccgcgcccagatgctggcggaacagccggcgaaggtgccgaccgccgacgcccagccgcgccgccaacccctccacaccgcccccgtccagcgcgcccgcctcgatcagggccatggcgcgattgaccgtgctggccgatccgcgccaggccgccatgtccggcgccgtctccggccggcagcgcaggcaggcccgtagtcccgccgcctcggccgaggcggcgctccggtgaaacaccacattctcgcggtggggcgtgcgcgccgggcacaccggccgacaatagattcccgtcgagaccacgccggtgaagaagcgcccgtcgaagcgggcgtcccgcgcctgcaccgccttccagcaaatgtccgggttcagttccacgggcggaagatgatccgtgcgtcgccgtctgtctcgcggttttcggacgcggatcagcaggcctggcgcccgtcccgtccggtgaccaggcgcaacgcggcgctgatcatgcgccacgtctcgccgatgaagcttccggcgaccgacatcatgatgatcgccgcgatcacgccttcgccggtcgagaatgccgtggtcacccgtctgacgaaatcctccaccgtgccgacccagatcacggacgacagcggcgacgccagccacagccaggcggcgaacacggcccctgcgcccgcgaacgccacgtctcccgcggccgtcaaccgcaccggcgaacccgtcgcggctcgcatcaggtcaaaggcgatgcgcgcggccatataggccagcaccggccagaagctcagcgccaccaggtcggaggcgatccgcccatagtcgaccccttccatgaccccgcccgccagggtgctgggcgcaatggatgcgccgagcgcgcccgtccaccacagcagggcgacgctccagcccacggcgctggacacggcgcgggcgctgggcgacatggcggcggcgtgcggcgcgcgatcttcacgcggtctgcgaccccgctcgcaggccttggccaactgctcgctccaggcgtccccgctcagcccgcccagttcgaacagccccaggtcctgcacccgccaccgggtcaggaacgcgggcttggtcgcctgccgttcgatgaagaagccggcgatggtcagcaggcccacgatcgtcaccgcgccagtgatcaggccgtgcagcccttgcgtgattgcctgccccaccgtcacgtcgccgacgatgctgcgcacgaccacgcctacaagcgtgatcgccgccagcaccgcaaaccccgccttcaccccgaacagccaccagggatagagctcgggccccaccagcccctgcgtctcgccgtaccggctggccaccgccagcggatggccgaagtcgcgcagcaccgcctcttcctccgcctcgttcagcggccgtcccagctcggcctcccgcgcttccatccgcgtcatcagcaggtcgcgcagttcggcgacgatgtcctcgcgcttggcggcgggcagctgcgcggccaccgccctcagatagcgttcggtcaggttcagtgcgttcatgatcggtccctcctccggcccgatgttcaaaggatgcgttcgagcgaggcgccgatgcgccgccactcgtccgccagtctggtcagcatcgcctcgccctgcggcgacagccggtagaagcgctttttccgcttctcctcctcgcgccattcgctgagcagcagcccctgcccctccagccggcgcagcagcggatagagggtgctttcctccatctcgatgccgtcctcggccagggcgacgcgcagcgaatagccgtactgctcgcttctgagccgagccagcacggccagaatcagcgacccccgccgcagctccagccgcaagctctcaaacagatccgcctcgcccatcgaagccgctcccgctgcgtcacatagtgtgtggtacacagtgtatgaactacaggttcgtagcctgtcaatgggacctccgcttgcatcgctcagacgaagtggtgaaggtggcgccgtctttgggggacgcatgagccagcagctaatcaatgcctatctaaaggaactcgccacccttcgccgtatcggcggcacgactgaaggggtcacgtcggaggcgttcaaggatcttctgaaggcttgggcgcgtcccctaggtttcacattcattccgcaacacgccttcaccaccaccgcgcgcgtcaacaaccgcgtcgatggggcgatcatgctcgagcggtttcccgtaggctactgggaggccaaggatgaggatgatgatctcaacgccgaaatccagaagaaattcaggcgcggctatcccaagaccaatatcatcttcgaggacacgcaccgcgcggtgctgtggcagcacggcaagttcgtcatggagtgcgccgtcaccgacggctccgagttggggaagctgctcgacatcttctttagctacgagcgcgaggagacaaccaacttcaagaaggccgtcgcccagttcaagatcgacctgccgccgatcctcgacatcctgcgcggccagatcgacaaggcccaggccgaggcaccggccttccaggacgccgccgcatccttcctgaaacaggcgcaggagacgatcaatccgtccgtcaccgccgaggatgtgcgcgaaatgctaatacagcacatcctgaccgaaaacatcttcgccaaggtgttcggcgacgacgaattccaccgcaaaaacaacgtggcctcggctctttacgccttggaggacaccttcttctcaggcgacgtgcgccgccgcaccctgtccaagctgtcgacctactacgctgccatcgaatccgccgccgccctgatcaagtcgcacagcgaaaagcaggggttcctcaaggcgatctatgaaggtttctacaaggtctacaacgccaaggccgcagaccggctgggggtcgtttacacgcccaacgagatcgttcgcttcatggtcgaatcgaccgactggctttgcgagacgcacttcaagaagaaccttatcgatcgcgacgtcgaaattctcgatccggccacgggcactggcaccttcatcgttgaactgctggagcagttcagcggacacgcggacaagctgaagcacaaatacgccgaagagcttcacgccaacgaagtggctatcctgccctactacgtcgccaacctgaacatcgaggcgacctatgcggcgctgacgaacgcttacgaggaatttcctagcctatgcttcgtcgatacgctcgacaacgtagccggcctcggggtttaccggaaccagcagtatgatctcttaggaggcatttcgggcgagaacgttgaacgagtcaaacgccagaaccggcgcaagatcagcgtggtgatcggcaatccgccctacaacgccaatcagcagagcgagaacgataacaacaagaatcgcgcctatcccgtcatcgatgagcgtatcagacagagctacatcaaggagagctccgcccagaagaccaagctctacgacatgtacgcccgcttcttccgctgggcgtcagaccgcatcgtggaaaacggcgtggtcgccttcatcaccaaccgcagcttcatcgacgccaagaattttgacggctttcgcaaggtggtctcgcgcgattttgccgagggatggatcatcgacttaggcggggattacaagcgcaaggaccaaggcggaggcggcaacgtcttcggcatcggcacgggcgttgcgatcagcttctgggtcaaacgctccagtgcgcgtggccgctgccgcatccgctatctcgcctgtccgccgggatcgggtgaggacaagctgtcttggattgcccagcaaaggctggcggatttgcggctggccgacatcacgccttccccagacggctactggctgaaccatcccgacgcctatcctaaggacgcgcttccactgatcagccgtgaggcgaagtccgcgaaacggacggcggagcagaacgcgatcttccggcgctactcgctcggggtctcgaccaatcgcgatgagtggctttacggacgctgacgtgatggtgtggacgacctccgcctgacgggctgttctgggtgtgtcgtcatcagggacgtcatgtgtggacgacctccaagacgcaagagtggaaacgacgttggcgctcggtcgagtgcagtcatgtgttcggcctgttgatgcagctgtttgcgctgctggccctgatgaagtccgcggaccggctccctaatcacgtcaacgcgctcgaggcgctctgaccccctgggtttcaccgatccccggctgcggccggttcgtcatcacgtctcaccactccttcgtctacggcgccggtcctgggtgaagaccggcccgatctctatgccgctgtgggcttgtagtcctcctgtcgcgccatcagggtccaggcgatgcgagccgtcttattggccaaggccacggcggcgaccttcggcttcttgcgttcgaggagattgccgacccagccctcgcgtcctcgctgccgggccattcgcaggaccgccgtggccccgacgaccaggagacgtcgaaggtagctgtcacccatcttgctgatgccgccctggcgttccttgccgccactgctattggcccgcggcgtgagtcccagccaggctgcaaactgccgaccggaacggaagagactcggatctggcgcgctggccgccatggcgctggcagtgatcggcccgatgcctgggatggtcgccagtcgccggctcgtctcatcctgccgatgccaatcgagaatccgacgctccatacggctgatctctgcgccaaggtgttcgagctgttctgccagcccgccaagcgcggcatgcgccagatccggcagggcctgaccctcttcacgcagactcttcagcgctgcccgcaccccagctggaccttgaggcgcgacgatgccgaactccccgaggtggccccgcagtgcgttgatcagcatcgttcgctgacgaaccaggagatcccgggtcttgtgcagcatcaacaccgcctgctgggccttcgacttcacagccacgaaccgcatggtcggccgggtgacagcctcggcaatcgcttcagcgtcggcggcgtcggtcttgccgcgcttcacataggccttcacgtacgccggcggcatgagccgaacatcgtggccgatcgccatcagttcacgcgcccagtggtgggctgaggcgcacgcctcgatcccgatcaggcacggcccaatcgactggaagaaggccagcacctggccgcgccgcagttgccgtctcacgacgaccgtgccgtctgtggctacaccgtgaacctggaaaacagtcttcgccagatcgagcccgacgacagcgatggtctgcatgataccgctcctagacgtgacgtccctgatgacgacacacccagaacagcccgtcaggcggaggtcgtccacaccatcacgtcaacgcgacgaggcggaggtaaccgaaaaggcgaaggcattaatcgcagcctacgaggccgttccattcaggagtgcggggtacggccagactctgaaatggtctcggaatctaaagcgcaaccattcgcgcgcgaaaagagagacgttctcatccaaacagatagtgtcggcgagctatcgcccattcacccagcgctatctctaccagtctcgagttttcaccgacgaactgggattagcggaagagctatttccaaccaccggacgcaacgaaggcattagcttcagcacgaccggacatcgggcgccctttatgaccctggcgatcgacggaatcgccgaccttcatttcggcgcggccctggatggttatcagcaggtcacccgctaccgctacgaccggcacggtattcgcctcgacaacatcacggactgggctttgaagcaattcgcggaaaggtacggcaaagccaccgcaatcactaaggaagatatcttcgcctatgtctacgccgtgctgcacgacccggtgtaccgcgagacctacgccctgaacctgaagcgcgagttcccgcgcattccgctctatcccgacttccgcagatggcgcgactggggccagcggctgctggacctgcacatcggctatgagacggtcgcgccccatcccctgacccgcaccgacgcgcccgatccgaaaagggccgagggcacgacgccggctgtcaagctgaagtccgatccagagcacggcatcgtcgtgctggacgccgacacccagctgtcgggcatcccgatcgaggcctggcgctatcgcctgggcaaccgctcggccatcgattgggtgctggaccagcacaaggaaaagacgcccaaggacccgactatccgcgagaagttcaacacctatcgcttcgccgactacaaggagacagtggtcgacctgctggcgcgcgtcgtgactgtcagcctcgagacggtggcgatcaccgacgcgatggcggccctgccgcaggccgcccgcgccgcctagcctcgcctcacgaacacagccccggccgccccgcctccaggtgcaggtggtcgtggtggacggcgttgtaatcggggctcagggtcgtgccgaagatgcggcaggcgtcgtcgcggatgcggcgcaggaagcgcgcctcggcgtcgtcgccgctccagtccgccgccactgtgatccgccggccgtcgcgcagccgcaccccggcgaagtccagggcggcggcgcggccatgggcgctgggccgcgtgctgccgcgtccgttgttcaccggccggcaggcgtagacgccatagtggtcgatctgcaccacgtccgaacccaggatctcgcgcgccgcaggctccagcgactgccggcgccagatgctcagcgccagcgccgtctcgcacgtcaccgtcacatcgcccggcgccatgcgcgccaccgtgcccaggtccggccccagcaccccggcgtccgtcaggccgcaggtctcgctgtccactcggtcgggcacagggctgaagcgcacccgcgccgccgtcagctcggctgcgcaccgctgcaggtcgccgcccgcccgcgacaccgccgcgcgcgtgccgccgtcgatcggtctgtccaccagcccgccgaccagcggcgccgggctctgcgtcggccgcgtgacgaccggccgcccggcgggcggagtccgcacacaggccgccagcgctgcgaccgccgccagaaccgttcccgcccgcttgatcgtccgcatcgccatccgccttcgcaacctccggcccgcccgccgcgctatggcggtaagtccggccgcaccctagatttcgttcatgaaccgttcctcgacgcccaaagggtctccgatcaagacggccaagccggtgcatacgcccaatcggggcctgaaagaggccgcggccgtctttcaccacgacgtcggcaagatgccgatgttcgcccccgtcaccggcccgcgcctgacgccggaggaggcgccggccgcccccggcgactggaccccgcaccgccctgaccggccgacaggcaagaagcgccagaagttccggctggagaccgcctacactcccgccggcgaccagcccgccgccatcgccgagctcgtggcccaggcggaagccggtgaccgcgaccaggtgctgctgggcgtcaccggctcgggcaagaccttcaccatggccaaggtgatcgagcagacccagcgtcccgccctgatcctggcccccaacaagaccctggccgcccagctctattccgagttcaaggccttcttccccgacaatgcggtcgaatacttcgtctcctactacgactactaccaacccgaggcatatgtacccaggacggatacgtatatcgaaaaggacagttctcagaacgagcagatcgatcggatgcggcactccgcaacccggtccatactcgaaagagacgacgtgatcgtggtggcgtcggtgtcgtgcatctacggcatcggctcggtggagacctatacggccatgaccttcacgctgaaggtcggggatcagatcgacgagggcaagctgcgcgccgatctgatcgcgctgcagtacaagaggaacgacgcgacgttcgagcgcggcatgttccgaaagcgcggcgacacgctggaggtgtttcccgtccacctggaggaccgggcctggcgcatcagcctgttcggcgacgagatcgaggccatcgtcgagttcgaccccctgaccggcaagaagacggccgagctggacgaggtcaccgtctacgccgcctcccactacgtcacgccgcgcccgacgctgaaccaggccacccacggcatcaaggccgagctgaaggagacgctcgactggatggtggagaacggcaagctgctggaggcccagcggctggagcagcgtgtccgcttcgaccttgagatgatcgaggccaccggctcctgcgccggcatcgagaactattcccgctggctgaccgggcgggctcccggcgagccgccgccgacattcttcgaatacatccccgacaacgccctgctgttcgtggacgagagccacgtcaccgtgggccagatcaacggcatgttccggggcgactaccggcgcaagtcgacgctggcggagtacggcttccgcctgccctcctgcatcgacaaccgcccgctgaagttcgaggaatgggacgccatgcggccccagacggtgcacgtctcggccacccccggcccgtgggagatggagcgcaccggcggcgtcttcgtggagcaggtgatccgccccaccggcctgatcgacccgccggtcgagatccgccccgtctccggccagacccgcaaccaggtcgacgacgtcatcgacgaggtcaaggccgtgtcgcgccagggctatcgcgccctggtcaccaccctgaccaagaagatggccgaggacctgaccgaatacatgcacgaacagggcgtgcgcgtccgctacatgcactcggacgtggacacgctggagcggatcgagatcatccgcgacctgcgcctggggacgttcgactgtttgatcggcatcaacctgctgcgcgaggggctggacatccccgaatgcggcctggtcgccatcctggacgcggacaaggagggcttcctgcgctccgagacctcgctgatccagacgatcggccgtgcggcccgcaacgtcgacggccgcgtcatcctgtacgccgaccgcatgaccggctccatggagcgcgccatcagcgagaccaaccgccggcgtgagcggcaggaggcctacaacgccgaacacggcatcacccccgcctccgtcaagcgcgacatcaaggagatcctggacagtccctacgaaaaggcccgcgtcctgatccccgccggcgtcaaggaggagagcaagccctttgtcggctccaacttccaggccgccctcaaggacctggagggccgcatgcgcgacgccgcctccaacctcgagttcgaggaggccgcccgcctgcgcgacgagatcaagcgcatgaagctgatggacctggagttcgccaacgacgccctcaccggcgccggcgaagaggtcgaccgctcagcccccaagaagtggcgcgccgaagcggcggcggagaaggctcaggcgttccggaaagggcgatagggacgaggcttcggcttatatgtagttctcaaacctgagcgagcgtaatggcaacgctccgcttggccgccgccgttcggtcgagaacctcccggcggatgcattttattagtagccacacagcgcgccgccgcttcgctcgaagcacctcttggtatggcgacaaactagatatgccgagtattgacgctcgcactcgtcggctattccttctgccggatcagtagccgcatatagcgcttaaccaccgtaatagtgggcgttagcaccgctttaacaagggagccgcacacctccagtccaacgctctagcacggtcaattctgtcgtcggtcatcagccattcgcagcgcgcttgtctccaaagcgcagctcgttgctgagggctggcaggagatcattatcttcgtcaacccgaagcatacgaaggtcggcgacaatacgcccgaaccattcgtatcggcgatccagcgcttgaaccgccattacacagcgaactgcatcagacgtctcatcaccgaagtagacgctgccttgtttacgggcaaaaccgaactcagcaaggacggtcgcgatctgcgtatagtagtgagtgttaccctcaccaaaaatggctctggctcgaacagtatcgagatcgaaggcgatggcgtacacgcgctgtttcctgtgcgttcgatgctgaggatttgtcctgacgtgcaccgagtgtttgggcatagggttcctcatggacagcagcgcgaagcgacaatcctatagacggaatcctcctaaatcgctatatataagccgcagagcggggctaacgccccgccctacggctccgtctaataaggcggcttgccacatgggattctctctttctaggcgccgagccatgccagggggttgaccgaagatggagcaggcgtgccaccgccttcaccatcagcttctgaggcgctctccggtgttgccggaagcgcctcattccgtttgggggcataactgctgacgatctggagagccttctcccgatcagccagttcccaccccgacttaccatgaccaatcacgtcagcgctccgcgaaaggagcgccccaagcgcattgatcttgttgtcgccgttgattgtatatccttgggcctcaatgatccgcacaagctcgcttgtcttcatgagactagttgttgttgtcagagcctgaagcgctagcacgaccgaagtacgggtctgcttggtgaaggcgtcgatctccaccttcggtcgagcccctgactcagatcgcgatccgacgaccggcctgctcgcaggcacttgtgggctctcaccgtagacggaaaggaagtcacgcacggcctgaagcttccgagacaggtcggcctcttcgtcgcgcatccgcttcacaatgtctgcgtccatgatcgaagtgtccctagctgctccctccatacaccacacatgacgccacgcaaaataaaaacgccggtctccatacgcaccttacctcgttagctgtacgttaatgagttccggatttgatccgtttgaacgcatgaggtctgccctcagttagccgtcggtcttggtgaagcgactaggcgccccagcactacttcaccactgatttgatcgagttgcgcgactgctcgcccgaatgccggacgtgccaaatgccaaaggcagcaacaaccggtcggcgatgtggcggtctcgggagcatctcggagattgatagcgctgcgttctcgccctgcgctgaagtgctggtccttagagctccacccttcttctccgagacgtcactctgaacgcacgcggctgactgctcgcatagatgaaggcggtgggtcggctggagttcaccctagttggactcgatgcgcatgaagccacgctggcagctctatcccggcaacgaccacgtccgcccaagattaggcagccgcttcaggtttaacaggcgcggcggttatcggcgcagggtctgagcctcgccctaccccctccgtccgcccctgacgcagcgacggtctaagcgtcgccctccaacggaggatgatcatggcgggggcgaaggcggcggggcggcggtggcgggggctggatcgggtggagcgggtcgagcagcggatgctaggcgtgctgaaggtgctcgatgtggtgaagacgatcgaggccctgccggacgggccggagaagcggcggcggatggccctggtcgaccggatggtcgccgacatcaagcggatcccgctgtgagccggcacggcgcgcccaagatccggtgccccgagacctggtcggagatccggcgggcgtgggagcggggcgagacggcggcgtcgctggcgctgcgctatgacgtggggctggccaacctgtggcggcggcgcgcggcggaggggtggcgcaggctgcgcggcgaggacccggcccctgagccgctggagggctgggcccgcttcgccgtcaccgagcgcgaggcgttcgaggcgcggctgcgggacgcgcgcgacctggccgggtgcctggagaaggccatgcgggacgagcggctgaccgaggcgccgctgtggcacatcccctggctctatcgctggcgcgccgacaacttgggctccgaggccgccgcgcgggaccgggcgcgggcgcgcgagatggatcagccctgggccgagaccttctgggacgccgagggtcggctgaagcccctgccgtggctggatgcggagatggcgcggctgcaccgcgaggagtggcgcgaggagatcggcctgccgcacggggtggagccgcatctcccttgatgcgcgcaccgggcgtgcgattcactctcacaggaacccgcgcgcgcgtcggcctttccgttccgtagagatttcagccctttccggagcatcccccatgtccatcatcgacaaggccatcgccgccgtcacccccgccccgtccgaggagcagcgcgccgaggccaccgccaaggcccgcgcctgcgccacccccggcgactggctgtccctggcgctggaccaccacgaccagatccgcgcgggcttcgagcgcggctcggccgcccgcactccggccgagcggatcgccgcctgcaaggacctgtcgatcgtgctgaacggccattcgctggccgaggagctggtgctctatccggccatggcccagtcggggcacaaggcgcaggcgggcgtcgcctataccgaacaggacacggccaagatgcagatggccgagctggagaacatcgaccccgccgacgaggcctgggccgacaagttcggccacatcaagggggccgtcctgacccacgtctatgaggaggaacacggctggttcatccacctcaagaagcacggcgagcaccaggaccgcctgaccgcgcgctataaggaggagttcgaccgctacgtctcctagagcgcctattcgtcccagcgcgggcgcgggtggccgtcgggcggctcagggatcggttcgtgccccagcccccgcagctggcgctccagcgccgccgcccgccatcgcatccggaaccacttgcggttatgcatgtcggtgatctcgcccatctcgcgatgctgggcgttgcggcgctcccagtagcgctgcttgatctcgtggtcgggatcgcgcccgggctccgagccgatcaggctgaagcgctcgcactcgttctcgtccagcagcacggcgagcttcagatccagcggcatggtgtccaccgtcatgccgccgcgccggggatcgccccgttcggccagccgggcgtaggtctcggccagcgccgccagcgccttggcctctgcccacagccgcccgtgcatggcccgcccggacgccagcgtcgccgcccgcgccagctcgcccgcatcgcccgcctgctcgttccccaccggcgccggcgaaaacagcccggccagcgcgcgcgaccccgtgggtttcagcgcccgcgccgcgccctcttcctcctccaccatccgcgcatgcgcccgcgcccgcgcatcgcccatggccttcttggtgaagccgtcacggcaggcgtagcgatagaccgaggacggcgccaccttccacttggcccccagctccttggccgtcgccccgttcttgtattcctcggcgatgatcgcccaggtctccgccgtcaggcgatagtgggtggcgggagcttcggcataggcgcgggtcatggtggggagcctagccgaagggtcagctatggcggagaagtcgggttgatcggcccttaaacgcccgcgccgccgggatcgacgacaatgagaaactctttctcgcctcctattcgtcgtcgctgcttgcgttggtttcggccacggtctcgtcagacatattcgtcagggcgccgcttcccctgagatcgtctgcgtccaacgtcgaaccgtccacgatccgcgccagcaagtccgccagcgcgggctccagcgccaccaggcgcgtcagaacccgcagcacgttcagcaactcggttgtgtattcggccagccactcgctcggctggatggctgacaggggcgagggcgggcgcttgtcacccatcggcggcttggagcggtcggcgcggcgatagctccaccactggtccagcaccaccttgcccgacacctcataggcgcggacggcgggcgagacgttgtcgatccgcccggtcggcccgaacttcagcgcccgctcggcggcgtcataaaccaggtcgtgcggcatctcggccagggtcctgggcagcgccttgcctacagtgggctcggcctcggcgggcttgacccgcaccgccccgccccggtcgccctggaaccgctcgccgaaggtgtgcagccagatcacctcgcgccccaccgccgcggcctcggcgaacagggcgccgtcggcggtgatgggaatgcgcaggcccggctgtttaaggtcgccccggaaacgttcgacataggccggatgcgccgccacggcggcgatataggccatgacgtcctcggccgagaccggcgcgccgtaagcctcccccagcgccttcagcagacccggcgagacgttcggcgtcgtcgcgtcggcatcggcccagagcgggaaaacgcggcctccgaaggagcctttgtagtgatgttgatctgggatcaaccccgtgaaggtcagtgctggaccgccgctgggcgaaaatcccataagcgcggttagatgaagctgcttgctggactctgcctcccagagtcggggacgcggatcgttcaacaggcgaacatcacctatgatccattgccgatcaaaactgcgatgaccgtaccttacggcagggagcatctcgccgtcgtcagcagttatcgaaacggagcgagccgggcgctttcccagagtctctttaacgaccttaccgacatgcctagcggcgactttgccatctcttaactgcggtcggaaaagcgtgtctttgcgaccgagttgcttctcggcgaccagttcagcccaccgtagttccaaggtggcgacatcgggtgcaatcacccacgggcggccgggcataacgcctggcccttggaactcgaagaggtcatctagcgatggatacccaatccagttggctgcgccttcgggcaggaagggcgcgcgcggatcgctcgctgcctctacccatccctcgtcgtccagcccgatccccgccaaagccgcgaacttcactgcccgcgccccctccggcagggtgcggaaccgcactcgcgccggcgtctccgggctgtccttggatttccgcagggccatgacgatgcaaacggtctgctgcactccttcgaagatgcgggtcgcggccggcggctgatatccctcgggcgaacagtcgatgacccaaatctcgtcggcgtctcggcggaggtccgcccgcatcttttggaatcccggcccattaaggaatccggcgacggtgatgaagcagacgatgccctggcgcttggtccagttggacggcacgtcttggtccgttcccgtccggaactcgtcgccgccgaacaccttccacgctgcccagcgccagaaataaacgtagaggttcctcaggtgcttggcgtgggtgcccacgccccatttgaccggcggctgccagtcatccagaggcgttttgtcgcgatcccccgcatcctcgatccaaccgcccagccccttggccttttccttgtagggcggattgcccagcacgacggtgatcgcctcgtgccgcttgacccggttcgattgcttgcgcgactcggcgatggcccgcaccgggtgcggcacccacgccgcctcctcgtccggatcggccagggtgtcggtgatatagagccgaaggtcactggcgtcggcggtgtcggcgtcggcctccgtcaggtcagcgatctcggccagcagccgcagctgcgccaccgcgaacggcccgaactgcagctcgaacccgatcaaccgcttcagcgcgtcctgcaccgccgccgggaccgagcccttgccttcggcctcctccaccgtccgcgcgatgcggttcagcacccccagcaggaaggtgcctgtccccaccgccgggtcggccagcttcacctcgggcgacgccagcccccgcgtcaggttgaaccggtcgggcgacgccagcgcctcgtccaccatccgcaccatggccgtcaccacctcgggcggcgtgtaatagctgccggtcttcttcctcagcttggtgtcgtacgactgcaggaacagttcgtagaaatacagccacgcctcgggctggcccttggacaagctcttccagttcacgacgtccagcacccgcaccagggtgttgatggacgtctccagcagatgcgcctcttccgccggttcggtcagcagcttcagcgccgatccgatcagagtgttggtctggctcagcgtcttgcccgccgcgtccagcccgcccgccagactgatgccccgcgccttggccatcagcaggccaaacgttaccgcctgggcgtatccgtcggcgaactccgcctccacggcgtccggcagcagcagctgacgccagtcctccatcaagctgaccagcgccggagccttccgatccagctgctcttcgacctcgtcgcgcagcaggcggcacagacgcgccgtggtctccgccagttgcttgggcgtgcgcggcgggatcgggttccagctgaggaagtccgcgactagggccgtcagggcgggcggagccttcagcttggcgcccgccatgtccaggtcgccgtcgaggcggacgatctcaccgaccttggtcccgtcccgccagaggctgaacgcctgcccatcggtgtagatcaggttgggcagcgacttcagcttttcccactgcgccttgtcgtgcttaccgtcgaacttcctcgggtccgcgccctttccgggcgctttgacctcgacatggccaaccaaggcgttcttgcgcgttacggcatagtcgggccgggtcatcagctccgacagggcgctttcacccaccagtacgacgtcgtcggccgccggcccgatcaggccgcataggtctgcaaccaacatctcaagcggcgctcgaagctgatcctctggctgacccgtagcgcctggattgttcagcttactcttggccgccataccgaagcgcgccacggcctcatcaagcgtcaacgtcatccacagccccctcaacaggtgccttgatcgcttggggacggcggcgatgcaaccgtgatgcgtgctggacgcttcagcgaatcacgagatgatctcaccatgtcgcaacccgaccttttcggcgctacgccgcagcccctgccgcaacctgatccggaggccgtgcgtcgaaggatgcacgatctgctgcaaacactccgcgacgccgaggcgatgcccctgacccacaaggaactgcgcttctggcgcacggtggcgcctcagaccactcgctggctggagcccgatgaacgcacctcgatcctggccgagttcgacgcccagctcgagcggctgacccgcaaggccgcttgagtcgcccggccgctggtcggcgcctcaatcttcgtccatcttcagggcggcgatgaaggcttcctgcgggatttcgaccttgccgaactggcgcatgcgcttcttgccggccttttgcttctccagcagcttcttcttccgggtcgcgtcgccgccgtagcacttgctggtcacgtccttgcgcagggcgcggacggtttcgcgggcgatgatcttgccgccgatggcggcctggatcggaatctggaacaggtggggcgggatcagctccttcatcttctccaccatgccgcggccgcgcgtctcggcgcgggcgcggtggaccagcatggacagggcgtcgaccggctcggcgttgaccaggatcgacatcttgaccaggtcgccggtcttgtagtccgtcagctcgtagtcgaacgaggcgtagccctttgagatcgacttcagccggtcgtagaagtcgaacaccacctcgttcagcggcagctcatagaccaccatggcgcggctgccgacgtagctcagctccttttgctcgccccggcggtcctggcacagcttgatcaccccgcccaggtattcgtcgggcgtcaggatggtggccttgatccagggttcggcgatgctttcgatctgcatcacgtccggcaggtcggcggggttgtgcaggtcgatggcggtcccgtcgcgcagctgaatcttgtagaccacgctgggggcggtcgcgatcaggtccaggttgaactcgcggctcaggcgctcctggatgatctccaggtgcagcagacccaggaacccgcagcggaagccgaagcccagggcggccgagctctccatctcgaaggtaaaggaggcgtcgttcaggcgcaggcggccgatggcggcgcgcaggtcctcgaaatcggcggcgtccacggggaacaggccgcagaacaccaccgactgcacctccttgaaccccttcagcggctcggcggtgggcttcttctcgtcggtgatggtgtcgccgacggcggcgtgggcgacctccttgatctgggcggtgatgaagccgacctcgccggcggccagctgatcgaccggggtgttcttgggcagaaagacgccgacgcggtccaccaggtgggtcgagccggactgcatcatcttgacccgcatgccggtcttcagcacgccgtcgaacacccgcaccagcagcaccacgcccaggtaggggtcgtaccaggcgtcgaccagcatggccttcagcggcgcgttgacgtcgcccttgggcgccggcaggcgggtgacgatggcctccagcacctcctcgatgccgaggcccgacttggcgctggccagaacggcgtccgaggcgtcgatgccgatcacgtcctcgatctgggcgcgcacgcggtcgggctcggcggcgggcaggtccaccttgttcaggaccggcacgatctcgtggttgttctcgatcgcctgatagacgttggccagcgtctgggcctcgacaccctgcgacgcgtccaccaccagaagcgagccctcgcacgccgccagcgaccggctgacctcataggcgaagtccacgtgccccggcgtgtccatcaggttcaggacgtaatccagcccgtcctgcgccttgtagtgcagcctgaccgtctgcgccttgatggtgatcccgcgctcctgctcgatctccatgttgtccagcacctggctggtcatctcgcgcgccgtcagcccgcccgtcgtctggatcagccgatcggacagcgtcgacttgccgtggtcgatgtgggccacgacactgaagtttcgaatgcgctcgacgggggtgctgctcatccgcgcgcccctatcacgcgcgggcgcggtgagccagcgggcgcggtccgccgcgttcgccccccgctcgtcacaaggcgttaaggctttgcaataaaggctttcggcgtttgagaacggttatcggacgcggtatggagatcgccctcgaacaaccggcgcaggccggcccttcgtttcgccttcaaccgaggaacatcccccgtggccaagacgacccgatccgctttgggcctcagcgccgccgccctgtgcgcattcgtgctgacgagctgcgggggccatggagacgacgaaaagggcgggccacagcctgccggcgggtcgcgccagaccgtcacggccgccaccgtcgcccaaggaagcctggatcgcaccatcaccgcgtccggcaccgtatcggcctgggaggaggtgccgatcggggcggagaccggcggcctggtcgctacggccgtctatgtcgatgaaggctcctatgtgcggcagggccagccgctggtgcagatgaacgacgccctgctgcgcgctcaggtgcgccagcagcaagcggcggtgcagaccgcccaggccaatgtggcgcgagacgacgccgccctgagccgcgcgcaggaactgcgcgagcgcggcttcctggcgcaggcggcgctggacacggcgctggccaaccagcgcgcgtccgcggccaacctggcgtcggcgcgcgcggcgctttccgagacccagacccggctgtcgcaggccacaatccgcgcgcccgtcgccggcctggtcatcagccgcagcgtcaccaagggccagatcatcgctgcgggaaccgagctgttccgcatggtgcgcgacggtcggctggagcttgacgcccaggtgcctgaaaccgaactgccgctggtgcgcgccggccagtcggccgtcgtgacctccagcgaggccggccagaccaccggcacggtccgcatcgtcacgccggaggtgaacgccgacacccgcctgggcgtggcgcgcgtttcgcttgcggccggcagccagctgcggcccggcatgttcgctcgcgccgagatcgccgtcggcgcccagcccgccgccaccgtgccgaccggggcggtgctctatcgcaacaaccaggccggggtgttcctgctgaacagcgacagttcagtgcgattccagcccatcaccgtgctgtcgcgcaccgacgcccagaccgccgtgaacggcgtcgccgcaggcgcccgggtggtggtggacggcgccggcttcctgaacgaaggcgaccgcgtcaccgtctcgaccggcgcggcgcgtccggccgcccaaccggcgccgcaacccgccgcccaacctgctgcgaagtaggaccgatcatgaaccagatctcgtcctgggcgatcaagaaccccattcccatcatcctgctgttcgttctgctgacgctcggcggcgtcgtcggcttcgccgggatgcggatcaacaacaaccccgatgtcgattttcccctggtcgccgtcaccgccgcccggccaggcgccgcgcctgcggaaatggaggtgcaggtcacccgcctgatcgaggactccctcgccgggctctccggggtgcgccacgtcaactccagcatcaccgacggcgtatcctcgaccaccatcgagttcgaactcggaaccgacaccgatcgcgcgaccaacgacgtccgcaacgccatgacgggcctgcgggccagcctgccgcaggacatgcaggagccggcggttcagcgcatcgacatcaccggcgacgccctgatcacctatgtggtccgctctccgaccatgtcgccggaagagatcagctggttcatcgacaacgagatgagccgttcgctgctggcgctgggcggcgtgggcgaggtcaatcgctcgggcggggtggaccgcgagatacgggtcgagctggacccgcagcggctgtccgcctacggcgtcaccgccggtgaggtcagccaggccctgaccagcgtcaacaacaacctgcccggcggtcgcgtgaccctggcgggatcggaacgcgccgtgcgcaccctgggggccgcaggctcggtcgagcagctgcgcgagaccctggtgccgttgggcgacggccggaccgtgcgtctgggcgatctgggcacggtcgaggacaagtggagcgaaccgcgccgcctggcgcgctacaacggccaggaggccgtgaccttcaacttcctgcgctcgcgcgaggccagcgaggtcaaggtcgccgaacgcgtccgcgaggaggtcgcccgcatcgacgaggcccacccggaactgaccatcgaacaggtcacctccagcgtgcagtacatcgaggagagctatctcgcctcgctcgaagctctgcttctgggcgccgccctggcggttgtggtggtgttcatcttcctgcgagactggcgcgcgacggtgatcgcggcgaccgccatgccgatgtcgctgatccccaccttcgccatcctgggcccgatggaccagtcgctgaacgtggtgaccctgctggcgctgtccctgaccatcggcatcctggtggacgacgccatcgtggagatcgagaacatcgtccggcacatgcgggacggcaagccgccctacgacgccgccatcgaggcggccgacgagatcggcctggcggtggtggcgaccacggccacgatcatcgccgtgttcgcgcccgtcggcttcatgccggggatcatcggccagttcttcaaggccttcgcgctggcggcgtgtatctcggtgttcttctcgctggtggtggcgcggacgctgacgccgctgatggccgcctacatgctcaagcacacccatcacgaggacaaggatccgttctggatgggcggctatctgcgcgccctgcgctggtcgctgggcaaccgctggaaggtgttcgtgctgggagtcctgttcctcgtcggttccgtgggtctgtcggtggccgccaggatgtcgttcgagttcatgtcgccgggcgacgaggcgcgcgccgccttccaggtggagcttccgccgggatcgacgctgcgccagaccgacgaagtggtgcggcgtgtcacggacatcctggaagcacgccctgaggtcacctctgtctacgccgcgataggcggtcaggacgtgaaccaggccaatgtctacgccgacatggtccccaagggcgaccgcgagctgagccagcaagccttcgcccgggtgatggtggaccagctgaagcaaattcccggcgcccgcatccgcgccggcatcgcccagcagggcggcggaccgagcgacggcaccagctacaccttctccatcctgggcgacgatccggcgacactggaaacggcggcgcgccaggtcgagagcgagatgcgcggcgtgccgggcctggccaatgtggtcaacaccgcggccatcgcccggccggagatcctggtcacgccgcgaccggacgaggccgccctggccggcgtgtcggccggcgcaatctctcaggcggtgcgggtggccaccatcggcgacatcgaccagaacctgcccaagtacaatctcggcgaccggcagatcccgatccgcctgcagctgaccgaagcggcgcgcgaggacctgtcggttctggaaagcctgcgggtgccggcgaaaaacggcgcccaggtgccgctgagcgcgatcgccgacatcagcttcggcgccgggccggcgaccgtcagccgccaggaccgctcgcgcatcgcctccatcaccgccgaactggacgggatcaccaccggcgcggccggccaggcggtgcagcgcctgccgtccgttcagaacctgccggcgggggtgcgccaggtgccggccggcgacgccgagttcatccaggagatgatcaccggcttcgccatcgccttcgcctcgggcattctgctgatgtacgcggtgctgacgctgctgttcaaaagcttcgcctatccgatcaccatcatggccgccctgcccctggcaatcggcggggccttcatcgccctggtgatcgcgggggccagcttctccatgtcggctttgatcggggtgctgatgctgatggggatcgcggccaagaactccatcctgctggtggactacgtcatcatcgccgagaaggagggcatgccccgcttcgacgccatcatggacgcggcgcacaagcgggcgcggccgatcctgatgaccaccttcgccatgggcgcgggcatggtgccgatcgccatgggcgtgggcgccgacgtcgagttccgcgctcccatggcgatcgcggtgctgggcgggctgatctcctcgaccttcctgtccctgctctacatcccggcgatcttcaccatcgtggacgacttcgcccactggacccggcgccgcctaggcaagcggttcgaaagccagcgccagcttgctcacgctccggcggagtagaggccacaccagcgatcaaggaaaagcccggccggatcgctccagccgggcttcttcttgttcgcctggatcgctggatcagtagcggacccgcagcgtcacgccataggtgcgcggctggccgagataggcgttgtaggtcgccgtgtcgcccgtcccgttcgcggggttgaacgggatgtagaagctgccgtcgggctggaccgcgttggtcgggttgttgaaggccgtgccctgcaggggggccgagaagccgacctgggtgtagtcttcctccagcaggttctgggcccacacctccagcgtccagcgctcgttctccgagcccagcatcagccggccgttcacgacggtgaagtcgtcctggaacttgtagggcagcaggtcggagccggtgttgtactcggtcgagtatctggccgacaggttgaagccgccgcgcagaccgcgtccgaagctgcggttgaagtccagcgcgcccgtcaccgaccattccggggcgaacgaggcgcgcgcgccgggcagcagcgacagctgcgggaaccggccggggctggacaggtcgcccgcgccgaactcgccgtacttggcgtcggtaaaggtcgcgccgccctggaaggtcaggccttcgaccggcgccagccagatcaggtccatgtccacgcccttggactccagttccgggatcgactcgaccacgaatgcagtgcccaggaaggtgttcagctggaagttctcgaaccgctggtcgaagtaggtggcgttgaacaggatgctgcggtcgaacagggtcgtcttcagacccagctcgtagctgtccaccgtctcggcggcgaagaacaaggaggcgtccggggtcacgcccgtctgcacccggtccatgttgtagcccgcgcccttgtagccgcgcgcgtacgagccatacagcagccagccgtccatcggcttccacgccgccttgatcgtgccggagatgttggtgtcgtcgaactcttccgcgatgcggcggttctcgtagagcgggttggaccagggcaggcacagcaggcccagcgccgcctgcggcgtccggaaggccgcgaccgggttggcctggttggccagggcgccgccgcacaccgcgccgttggcgcccaggttgtcctgaagccccagcgggcgttttttgtcatggggggcgcgcagccccgccgtgatctcgaactggtcggtgatgcggtaggtgtttttggtgaacagggcgatcgattccgaacgctggctgtagtgatcctgataggccttgccggtcccaaaggtgggcgccgcggccgagggcggcgcgaacccgaggacgcacagcggctggcccagcagcggcccgcttgttccgaccgcaaagcccgccggattggagaagcagccggtccgcaccgggctggggccgccgaatgcggcgggcacgctggccgtcagcagcaaggaggcgaaggcgttgtagtcggcgccgaacacatagctgtcgtcgcggtagatgttctcgatggtgccaaagccgcccaccagccagtcgaaccggtccgacgtgccggccagccgcatctcgtgggtcaggttggtgacgccgtagccgttggagccgtcattgtcgcggtgcagaatgtcggcgccggtgtagtcgatgtccatgccctgctggaacgaccagtcgcggaacgagctgatcgaggtcagggtcacgtccggaccgaagtcgatgttggcctcggccgacacgccgaagtcctcgatctcctgcggcgtttcgcggttcgaataggccgtgcggctatagggcagcacgccaaaggtcgcgttcggcgggcgctggccctcgccgttcgccagggcgttgatgaaggggtagctctgccccgtgcgcacctgcaccgccgcgcaacagaactcctcgcgcttggtgtagtcggcgatcagccggacggaggcgctgtcgttgggcaggatcagcagctggccccgcgtggtccagtaatcctgcgtctgatcctcggtcagggtgcgcggaccgtcgcccaggtccacgtcatagaagccgtcacgcttgcgcttggccacgaacaggcggccggcgatctggtcggtcagcggccccgtgaccgacgccgatcccccgatggcgccatagtttccgccggtcagctcggcttcgaagccgggctcgaacgaaggctgttcggtgatgatgttgatgacgccggccgaggtgttcttgccgaacagcgtgccttgcggtcctttcagcacctcgatgcggctcagctcgcccagatcgccgaagcccaccgagttgcgcgagcggtagaccccgtcgatgaccacgccgacagagctttccaggcccgggttgtcgcccacggtgcccgcgccgcggatccgcaccgtggtggaggcctccgactgggtcgaggtcaccgtcaggccgggcgtcaggatctgcaggtccttgatgtcctgcacgcccgcgccttccagcagcgcctccgacagggtggtgacgacgatgggcacctcctgcaggctctgctcgcgcttctgggcggtgacgatgatgtcgtcgacggaggtcgcctggtcgcccgcgtcctgggcgctggcggcgcccgcaagccccagaagcgaggcgccgattacggcggcggacacggagttgcaaagagagtggcggcgcatgggcgtccttcccggctagctggccggccgccgttttcatcggcgacgcagcgtttcctgttcccaatcgacccgcctctacgtggaggcggatccagtatggtgaggctacccatggattcccgcgaacgacaagcgagcgtcgttcgctgcgactatttttcgccacgatcggcccttgtgtgacaaggaagcgacagaagatgctgaccttaggtcaatctttgcgtgctgcggacaggggctccacatccggctcctgcgccgccgggtcgacaacccgcgcgcgcgacgccagcgccagcaccaccgcggccgccacggcggaaaggatggagccggcgatcacgcccagcttgacctcgatctgcacaggcgaatccaccgcgcccgggaacgcgagcacgccgatgaacaggctcatggtgaagccgacgccgcacagcagcgagacgccatagacctgcatccaggtggcgccgctggggcgcgcgccgatcctcagcgtcgaggccagccacgccgccccgaacacgccggcctgcttgcccaggaacagccccagggcgatggcgatcaccaagggcgcgaacgcctgttcgagcgacagtccggcgaacgacacccccgccttggcgaaggcgaacagcggcagcaccagaaaggcgttccacgggtgcaggtcgtgcatggcctccttcagcgggctttgcccgtcttcggcgcgcggccggatcggcacgattgcggcgaaggcgacggccgtgagcgaggtcgacaggcccgactgcaccgtcaggtaccagaccagcgcgaaccccagcacccagaagggcgcggcgatgcgcatccggtgcgcggcgaccgctccgaccgccagcgcccctatggcccagaacagcggcgtccagttcgttccttcgctgaacagcagcgcgatcagggcgatggcgcccaggtcgtccacaatggccagggtcagaagaaacacgcgaagcgacgacggaagcccccggccgacaaggccgaacacggccagggcgaaggcgatgtcggtggccagcggtatcggccatccttcatgcggcgcgccgatcaggccgcccaatgcaagatacaccgccgccggtccgaccatcccgcccgacgccgccagcaccggcgtggccagcttcctggggtcgctcagttcgccacgcaggatttcgtatttgatctccaatcccaccacgaggaagaagatcgccatcagaccttccttgatccagtcggagatcgtctcctccagccggatcggcccgatctgcagcgcgtgcacgctctttagccaggcgaagtagtcgggggcccagggcgaattggcgactgcgagcgcggcgagcgcggccagccccagcgccgcgcccgaggcggcttcggtcttcaggaaatcaagcgtcagtctgcgagccacggcggcctccggatcaaaggagcggttcgtggcgtcaggttatcgacggacgccggaccgggttcgccgcgattgcgcgcggcgccggcctggccggttggtccggcctgatctctgcgaacaagaatacggatggcgtttcaaggttcaaccccacgcggttgcgcatgcgtgggtccatccgcatctgcgcaccatgcccccgtcttcagcctaccgccccgacccgcgcttcttcgaccttggggaggattacggcgacgccgtccgcgcggccgagtttccgcaggccaccctgcgcttccgcaacgatcgggccgccggcgaggtcgggctggagaccctgagcgacgccgaatgggtcgatcatttcggccgctttacgcccctgcccggccaaccggggcccgtcgccatgcgctatcacgggcaccagttccgttcctataaccccgacctcggcgacggacgcggctttctggcggcgcagatgcgggacgcctccggtcggctcctggacatggggaccaagggctcaggccagacgccctggtcgcgcggcgcggacggacggctgacgctgaagggcggggtgcgcgaggtgctggcggcctccatgctggaggcgcaaggggtccccaccagccgcgccttttcgcttgtcgagacgggcgaggcgctggagcgcggcgacgagccctcccccacccgttcctccgtgctggtgcgcctgtcgcacagccacatccgcttcggcacgtttcagcgagcggccttctttgggcggcgcgaccagatcgagacgctggtggagcacgtccgcgccctctaccatccggacgttcctgcaggcgacgcggcggccctgctccaagcgatcgtcgaggcctcggctcgccttaccgcccgatggatcgccgcgggtttcgtgcacggcgtcttgaacaccgacaatctgaacgtcacgggcgaaagcttcgactatggcccctggcgcttcctgccgttctacgagccgggcttcaccgccgcctacttcgaccagagcgggttttacgccttcgcccgacagccggaggctgtgttctggaacctgacgcagctggccggttgcctgaagctggtcgccgaggtcgagccgctgacgcaggccctgaacggtttcggcgccgcctacatccgcgaactgcgcgcggcctttctgatgcggctgggcgtcaggagcctcggcgaggcggcggaccagcggctgctggacgcgacgctgtcgctgctgcgggaaggcggcgaaggtctgcggtgggagccgctgttctttgactggttcgccggcttctcctcctccgcccgggcgctcgccgggccgcgcaaggcgctctaccagggcgaggccttcgacgtcttccgcttcgccctgttcgaacacgagcctgatgcgcctgagcggctggagcatcccgccttcgcccggcccgagccggaggagatgctgatcgacgaggtggaggcgatctggtccgtcatcgacagtgaggacgactggacgcccttcagttcgaaactcaagcgcatcgaggaggcgcggcgcgcctacggtttcggcgccgccgacacagagcctccagccagctgaaaccatttgtcatctctcgatgactttgttcatgtcatcggctgatgacaggtcgcaaaacctttgctataagacccttgcgcaacgtcgatgccgatcagatatcgtcgctgttgcagatcacctcttttgcggctctcgggtcgccggacgtcctcccatgaccaccacgaccctctcccccgctcgcgcgcggctcgacgcgaacgcccgcaacctcgcgctctggacctttcagggatggctggcgatgttcttcatcgccgccggctgggccaaggtgtccgagcccatgaccaacttggtgacgctgatgggctggccggcccttgcgcccgagaacctggtgcgcggcctgggcgtggccgagatggtgctggctgtcggcgtgctgacgccgctgctctcctggcggctgttccgcccggctctgctgacttccgccttcgggctgatggtgctggaagccgccatgctgggcgtgcacgtcctgaaccgcgacatcggcctgtcggtcgtgaacctgctgctgctggcgatcacgattcccgtgctgctgggtcgccgccggggctgagccgcgccgagcggcagcgatcggagcaggtcttcacctgatcccagtcccgcgcccatttctttcgccatgtgaacgggcggccgcagacctcgcagggcttggtgggcaggtcgcctttcttcacaccgagcgccccgttgacgtgcttgacagccatggcgcgtgaaaaaccttccctttacgtgcgcgtcaagttattgaggcgctcatggcgaccgccgacgatcatcgcacctattcgatccgccagctctgccgcgagttcgacgcgaccgcgcgcgccctgcggttctatgaggacaaggggcttctgacccccgcccgcaagggccagacccgcgtctacaacgcgcgcgaccgagcccggctgaagctgatcctgcgcggccggcgcatcggcttcaccctgcaggagatccaagagatgctggatctctatgaccgtaaggatcacaacacccaccagatggcgatcgccctgcgccgccaccgcgcccagatcgagacgctgaagcagcagctggaggacatcgagggcgccattcagaccgccgaggacgcctgcgcctggatggagtccaagctgggcgagcaccggccggacctgctgccgggcgctcaggattacgagcaggtgctgcgcgcccggctcaaccacgaccaccaccccttcaaagcgagagcgtaaccgatggcctacacggcgcctgtccgcgacttcacctttatcctcaacgaagttctggagatcgaccgccacgccaaccagccaggcttcgaggacgtctcggccgacctggtcggccagatcctggaagaaggcgccaagttcgccgaagaggtcatcgccccgatcaaccgcgtgggcgaccaggagggctgcaagctgtccgacggcggcgtggtcaccggcccgaccggctggaaggaagcctatcagcagatggtggaggccggctggccggcgttgtcggcccataccgagttcggcggccagggcatgccggcggtgatcggcatggcgttcggccagatgacggccgcggcctccgccgccttttcgatgtatccgggcctgacggcgggcgcctatgcgggcatccacgccaacggctccgaagagctgaaggccaaatacctgcccaagatggccaccggcgagtggggcgggaccatgaacctgaccgagccccagtgcggcacggacctcggcatggtgcgcaccaaggcggttccgaacggcgacggctcctattcgatcaccggccagaagatctggatctcggcgggcgagcacgacttcaccgacaacatcatccacaccgttctggcccgcgtcgagggcgcccaggccgggatcaaggggctgtcgctgttcgtggtgcccaaggtcctggtcaatgaggacggctcgctgggcgagcgcaacggcgtggtctgcgccggcctcgagcacaagatgggcattcacggcaacgccacctgcgtgatggcctatgagaacgccaccggctggctggtcggcgaagaaggccgcggcatgaacaacatgttcgtggtcatgaacgaggcgcgcctgggcacgggcctgcaaggcctggccatcggcaccgccgcctaccaggccgccgtggagttcgccaaggaccgcatccagggccgcagcctgaccggacccaaggcccccgatcaggccgccgatccgatcatcgtccacccggacgtccgccgcatgctgctggaaagcaaggccttcgtcgagggcggccaggcgctggtgctgtggaccgcgctccaggccgacctgcagggctcggctgacgaggcgaccgccaccaaggccaaggattacatgggcctgatcaccccggtggtgaaggcctatctgaccgacaagggcttccatgtcgcctcgctggccatgcaggtgcacggcgggtcgggctacaccgagcacttcccggcctcgcagtatctgcgcgacgcccgcatcaccatgatctacgagggcaccaacggcatccaggcgctggacctggtgggcagaaagctgccggcccagggcggccgcgccatcatgagctggttctccgacatcgacgcctttgtggccgagaacggcgcggacggtccgatcaagcccttcgtcgacggcctggccgacgccaagaagaagctgcaggaggccaccatgtggctgatgcagaacggcatgggcaatccggacaacgcgggcgcggcctcgaccgactacctcaacatcttcggcgtaacggccctggcctatatgtgggcgcagatggccaaggcggcgcaagcgcaggtggatgcgggctcgaccgacccctattacgccaacaagctgatgaccggccgctacttcgtcgagcgcatcctgcccgacgccggcgcgcacctgaagaagctgaagaccggcgccgacgtcctcatgcagatgccggccgaagcgttctaaagcctcaactctcctccccatcgccgggcgatggggaggtggatcggcggcgcagccgacgagacggaggggcggacctcctcccaagctgaagagagaggcggacccaacccctccaccacttcgtggtccccctccccatcgcgggcgatggggaggagaaatcagatgaacgtcctcaacagccccgctcccgacttcatgcaggacgaggagatcaccctcttctccgacagcgtcggccgctggatcgacgagcacgcgccgcaggagaaggtgcagcagtggatcgccgactcttccgtgccccgcagcctgtggagcgcggcgggcgaggccggcctgctaggcgtctccatccccgaggcggacggcggcatgggcggcgactatcgccacgaggtggtgctgatgcgccagctgggctggaaaggcgcggaccacttcggcctgtcgctgcacaacgccatcgtcgccccctacatctggcactacggcaccgacgagcagaagcagcgctggctgccgcgcctggcgtcgggcgagctggtcggcgccatcgccatgaccgagccgggcgccggttcggacctgcagggggtcaagaccaccgccgtgaagggtggcaacggctacgtcgtgaacggctccaagaccttcatcaccaatggccagttggccaacttcatcatcgtggtggccaagaccgatccggccgagggcgccaggggcaccagcctgatcgtggtcgaaaccgacggcgccgaaggtttcgagcgtggccgcaacctgcacaagatcgggatggaggccaacgacacctccgagctgttcttcaacgatgtccaggttcccgccgataacatcatcggcggcgtcgagggccagggtttcgtgcagctgatgcagcagttgccgcaggagcggctgaacatcgccgtccagggagtcgccgccgccgagcgcggtctcgagcacaccctggcctacgtcaaggaacgccgggccttcggcaagcgcgtgctcgactttcagaacacccagttcaagctggccgaggtcaagaccaagttgacggtggccaaggtcttcgtcgatcactgcatcggtctgcacctgaagggtcagctggacgccgccaccgcctccatggctaaatattgggtcaccgacatccagggcgagacgctggacgagatgctgcagctgcacggcggctacggctacatgaccgaatacccgatcgcccagctctacaaggacgcccgcgtccagcgcatctacggcggcactaacgagatcatgaagctgctgatcgcgcggacgctgtagctgatcttgcaggaatgtacgtgaacgcgtacattatagacatgaacgcgatgtccgtgaccgatctgcgcaagaacctggcggcgactatcgaccgggtgacggcggatcacgactacaccatcatcacgcgtgagggcggcaagccggcggcggttctgatgtcgctggaggacttcgcctcctggcaggagacggactatctgctgcgcagcccggccaacgccgcacggctgcgtgaggcgatcagcgagctcgatgcgggcggcggccaggcgcgcgacctgatcgaagaatgaagctgactttccacgcccatggctgggaggattatctccattggcagcgcaccgacccgaagatgctccgaaaggtcaacgggctcgtcaaggaatgtcagcggtcaccgttcgagggaacgggcaagccggagccgctgaagggcgatctcgccggctggtggtcgcgccggctcgatcaggaacatcgcctcgtctatcgtgtcgaggatgatgcgcttctgattgcgcagtgccgccaccactacgaccgatgatccgcctccacgtcacctccgatctgtctcccggcgcagccgtcgcgccgacgctcgatcagtcgcgctatctcacccaggtgatgcggctgaaggcgggcgacgacctgctggtgttcaacggccgcgacggcgagtggcgggcgtcggtggccgaggtgctgaagaagggcgtgatcctgcgcgccgaggaacaggtgcggccgcagacccatggccccgatctcgagctgatcgtggcggtggtcaagaaggcgcgggtcgagaccattgtggaaaaggccgccgagctgggcgcgcgccgggtgcggttggcgatcaccgcgcgcaccaacgccgaccgcatccgcctggatcggctggacgccatcgccgaagaggcggccgagcagaccgggcgcctggacgtgcccgctgtcgacgatccgcagaggctggacgccattctggacggttgggaccccgcgcgccgcctgatgttctgcgacgagaccggcggcgctccggcgatcacggcgctcgcccctccccctgagggggagggggaccctgcgcaacggggtggaggcggcagttcagcatctgatagttccccctccaccgcttcgcggtccccctcccccatggggggaggatcgccggcgccttgggccatcctgatcggtcccgaaggcggcttttcgccggaggagcgcgagcggctgcgcagccttcccttcaccaccgccgtctcgctggggccgcgcatcctgcgggccgacaccgccgccatcgccgccatgaccctgtggcaggcggcggccggcgactgggaccgctgacgaaatcgtgcagcggatagaactgcgcccttgagcgttgcggttcggtcgcccatctagccgcgacacctgaggggcttcgcacatcacatggccgaccacgcgccgctgaccaaggccgatctgatcggcgccatgtccaagggcatgaagccgcgcgaccagtggcgtatcggggccgagcacgaaaagttcggcttcgacaaacagaccctgcgccgcccggcctatgagggcgaaggcggcatcaaggccatgctggacggcctgacccgcttcggctggacccccgtcgaggaaggcggctacgtcatcggcctggagcgccgcagcggcgagggcttctcagcctcggtcagcctggagcccggcggccagttcgagctttcgggcgcgccgctgcggaccatccacgacatctgctcggagaccggccagcacctggaggaggtcaagaccgtggccgacgaaatcggcctgggctttctgggcgcgggcttcgatccgctgtggagccgcgccgacgtgccggtcatgcccaagggccgctatgacatcatgcgcgcttatatgcccaaggtcggcgcgctgggcctcgacatgatgcttcgcacctgcaccatccaggccaatctcgacttcgatacggaagccgacatggtgatgaagttccgcacttcgctggcgcttcagcccatcgccaccgccctgttcgcctgttcgcccttcaccgaaggcaagccgaacggctttctgtcggcgcgggccaacgtctggaccgacacggacgcggaccgcaccggcatgctggacttcgtgttccaggacggcttcggcttcgagcgctacgccgactatgcgctggacacgccgatgtatttcgccaagcgcgagggccgttacgtcgaggcgtcgggccagtcgttccgcgacttcctggacggccgcctgccggcgctgccgggcgaacgccccacgatcaaggactggaacgaccacctgaccacccttttccccgaggtgcggctgaaggcctatctggagatgcgcggggccgacggcggcccctggagccgcatctgcgccctgcccgccctgtggaccggcgtcctctatgacgccccctcgctcgccgccgcctgggacctggtcaaggattgggaagtcgaggaccacgagcgcctgcgccgcgacgtgacccggctggggctgaaggccgaggtcgccggccgctcggtgcgcgacatcgccgtggacgtggtggccatcgcccggcaggggctgaagaaccgcgcctgcttctccggcggcatggtggacgagcgcggctatctgtccgaactcgaggacatcgccgacagcgggatcaccccggccgagcgtctgctcgacctctaccatggcgcctggggcggcgacgtgcgccgcatctacgccgacttcgcctactgaggcctcgggcggaaccggctccggcgtccggcggttcaccaagccgcccccgctgaagaaagagcccgccatgccccacgtccgcgacgacgccgatccgctgctgggtctcgccgccggccttgccggagggctggtcgccgctctggtgatgaccgagttccagtcgctgctggccaagggcggcgtcacctcgggcgtgaagggggcgccctcgacggagaaggcggccgaccgcctgtcgcgcgccatcacgggccgaggcgtgccgcgccgcaagaagcctgcggccggcgaggcggtccattacaccgtcggcgcggcggtcggcggcctctatggcctcgccgccgagatcgagccgcgcgtcaccctagggcgcggcgcggcctttggcgtcgcctccgccaccgtggtggacgaggggctggtgcccgccacgggcctgggcgatcctttctggaaggcgccgctgcgctcgcacccctattcctacgcctcgcacctggtgttcggcgtggccaccgaggcggcgcgcgccctgatccgccgcttccttgacaaggtgaaggccgggatcgccgtcgtccggcgcaaggccgagccgcgtccgccgttgaataccgaggggccgcaaggctggcgtgcgctgggcctagccttcctcttgggcgcatccggcggcaaccgcaccagcgcgcccttgctggccgtgacctgggcggccaagctgggctggatcgacctgaaggacacccgcttctcgggcatggcctccaccaaggccgccgccatcgtcacgccgctcgcgctgtatgagtccgccggcgacaagatgccgaacgcgccgcaccgcaccatgccgatcgcggtcgcggcgcgcacggccagcggcgcggccgcagggtgcgccctgaccggcggccgctctccggcggcggcgctggcgggagccgcaggctcgctcgccgccacctacatcggtcacagcatccgcctgcgcctgtcgcgcgccgccggccgcgacctgccggtcgccctggccgaggacgtcctgaccttcggcggcgcctttctggtgtgcctggcctcgctcgctccatccaggccctcggacgatcgtacggcggcctaggctcgcgcgctgcgcgctccggcccatcgcccgcggcgtgaaatcctgcgataccctcacgacttaagggagatcatccatgacgggcgcgatcagggtgggcgtgggcggctggacctatgagcggtggcgcggcgtcttctatccggaaggactgacgcagaagcgggagctggagttcgcctcgcgcgcgctgagttccatcgagatcaacggcacatattattcgaccttcaagccggacagctggcgcaagtggcgcgacgagacgccggacagcttcgtcttctcggtcaaggccagccgctattgcaccaaccgcaaggtgctgtccgacggcggcgagagtttcgaccgcttcctgtcgcaagggttgaccgagctcggccccaagctcgggccgatcaactggcagttcatgggcacgaagacgttcgaccccgaggatttcgaaggtttcctgaagctgttgccggcggaaaaggacggcctgcgtctgcgccatgcgctggaggtgcgcaacccgacctttgcgaccgagcagttccacgatctggcgcgcaagtacggcgccgccatcgtctacgccgtggacgacgaggagccgacctggccctgcatcgacgaggaaaccgctgatttcagatacgcccgcctgatgtccagccgggaggacgagccgaccggcatgaccggggacgaactggacatggtggccgagcaggcgcgcggctggagccggcgcggcgatgtcttcgcctacttcatctcgggggctaaggtgcgcaatcctgcggccgcccaggcgctgatcgaaaagctgggctgacgcttgcggacgcggcggcggctgcacacctgaacggcatccccagcctgcttgcagagacccgcccatgccgatccccacgcgcgccttcgccgccgtcgccgccgacaagccgctggagccgttcagcttcacgcgccgcgatcccctgcccgacgacgtggtgatcgacatccagtattgcggcgtctgccactcggacctgcacatggcgcgcagcgagacgggacccgcccgctatccgctggtgccgggccatgagatcgccggcgtggtcaaggcggtggggtccgacgtcacccgcttcaaggtcggcgatcgcgtcggcgtcggctgcatggtcgacagctgccgcgagtgttcctcgtgccaagcgggcgaggagcagtattgcgtgccgggcttcaccggcacctatggcaatccggacaggttcgccgagcagtcgggccagccgatcacgcagggcggctactccgaccacatcacggtggaccagcacttcgtcctgtccatccccgacgccctgccgctggacaaggccgcgccgcttctgtgcgccggcatcaccacctattcgccgctaaaggaatggaacgtcgggccgggctcgaaggtggcggtgatcggcctgggcgggctcggccacatggccgtcaagctggccgccgccatgggcgctgaggtcacggtgctgtcgacctccgaccgcaagaaggccgacgccgaacgcatgggcgccagccacttcctgatcaacaaggacaaggcggcaatgaaggccgcggccgagagcttcgacctgatcatcaacaccgtctcggccacgcacgagatcgccgaccatgttcagctgctggcccgcgacggcaccatggtgatgctgggcctgaccaccgaggggctgccggtttacgccctgcccctgctgtggcgtcggcgccgggttgcgggctcgctgatcggcggcgtccgcgagacccaggagatgctggacttctgcgccgagcacggcatcacctgcgacatcgagaccatcgccccggaccagatcaacgaggcctacgcccggatggagcggtcggacgtgcgctatcgcttcgtcatcgacatggcgaagttgccgcaggcggcctaaacacggccgcatcctgaagggggttcctgatcatcggtccgcatcggccggaatcaagaacccccttcgcccaaaatccgccgccgccctctttcatctgttgttgcatgaacttgtgggtcctcagccgcagagcgcgtccgtcgcgtcgcgtcgcgatggcgttcgccgtcgtggcgggcgtgtgcgctctggggatcctgctgtcgccgctcgcggccgaggcgcaggggcggcgcggcgcgcccgccaccggccgctatgtcgcgggctcgggccagagcttcaccctggacacctcgggatcgcgtcccttgctgcgcttcgagcgctcgaccgagatctgggtgctgcgccccacgcccgcgccgcgcggcgacatcctgtaccgcaacgacaacggcgaccagatcctgcgcgtgacgccggacggcggcatgaccctctacaccaccagcgctccgcagggctcgccggtgtcgcgcgctggcgatgcggcgtcgctgctggccccgtcgatgacggcggtgcagatgtggaactacatcgtgcggcaaagcggccgcgcctcctcggcgttgggtcggctgatccaggtggacgtcgatatccagccagggtccgaggcggtcgccgccgacgctctgtcgaccgccgtggacgccatcgtgcgcatggcgcgctcatccaaccttcgggccgaaaccaacaaggtgcggcgcatcgtggtgaccgatcagggcggcgcatcacaagccaccctgtcgcgcggcaccctgcgcatcgccgtcaatccccgcgcgggcgtggcgggccggccctcctccgcgcgcatcgtgcggctggtcgccgacgaggccctgagccgctgacggcgggccgccgaggcctcaggcggcgtccttggccgtgcggcgggcggcgaactccgacgcatcggccgccgtcaggaacggattgaagcgcgtctccgcgccgatggtcgtgggcgtggtcgcctcgccgcgctcgcgcatggcgaagacggcctcgacgtgcgcccgcatctccggccgcgcgtcctgcgtcagggcgaagcgcgcgttcgaggctgtgtattcatggccgaaccagacccgcgtctcctcgggccaggcggccaacccctgaagcgaggcccacatctggtcgggcgtcccctcgaacagacgcccgcaccccagcgcgaacagcacgtcgccggtgaaggcctcgcccgcctccgctgagcgataaaccagatggcccagcgtgtggccgggcgcctcggtcgcctcgaaccgcgtctcgcccaggtccaccacgtcgccgtcgcgcacgatccggtccagcgtcgtcacccgtgcagcctcctcggggcccaccacctcgcagccggtctcggccttcagcctctcggcgccttccgtgtggtccgggtgccagtgggtgatcagcaagaggtccagccgcccccagcctagccccgtcagttcctccagcacctgccccgcatccggcgcgtccaccgccgccgtccggccgctggcgcggtcgcggaccagatagccgtagttgtcgctgcggcagggaaaggcgtgaacatccagcgtcatgccgccatcctagcagcggagccccgctcgggcctatagtgggcgcatgcggcgcggcgtggacgagctcaggaccttttacggcgaacccacgggcgcgctggtccgccgcctcctggcgcgccgactggaggacgcctggggcgaggcggacgattgcgacgtgctgggcgtcggctacgccacgccgtggctggacgcctttgttggggcccgtcgcgtggtcgcggccatgccgggcggacaaggcgtcgaacactggcccgcgaccggcaagaaccgcacccttctggtggacgaccgccgcctgcccttcgccgccggcgccttcgaccgggtgctgctggtgcatgcgctggaggaggccgacgacgccgccgggctgctgacggaggcggtgcgggcgctggcgccggccggacgcatcatcctggcggcggcggcgcgcggcggcctttgggcgcgggccgaaagcacgcccttcggccacggccggcccttcacccgccgccagctggagggcctggtgcgcgatgcggggctggagccctcagcctggtcgcagacgctgtactgtccgccgtggagccccctgctgggcctggccgacggtttcgaacaggtcggacggcgggtcgcgcccggcacggcggggctgatccttctggaagccacgcgccaggcctacgcccgcatccggcccagcggttcggcccagcgcgtactggctcccgcccgagccctgcagccccaaccagccgtgcggaacggtccgctggcgcgccgccgcgaacgtccgtaaagctgcggtccatgcaccgactgatcctgatgcggcacgccgaagccgagaccgccgcgccgtccggcggcgacgaggcgcgtcccctgtccgccacgggtcgggccgaggccgaggggatggcccgcgccctggccgagcggggcctgcgccccgacctcgccctggtctccggcgccgtgcgcacccgcgagacctgggagcggctgcacgaggacttcggcgacgtggaggtgcgctacgagcccggcctctacaacgcctcggccgaacggctgcgccgctccgtggaggcggccggggacgaggcgggctgcctcctgatcctggcccacaatcccggcgtccaccttctggctgtgaagtatctggaggaggccgcggcctcgccgccggtgctggagcggctgtccgtcggctttccccccgccgcctgcgcggtcttcgccgtggaccccgccggccgccccgtgttcgagagcctgctgacgccgcgcgcggccggagtggccggatgaccgaggcggtcgcctacaagatcgtcgacgccgaggagtggcggcgggctcaggacgcgggtgaatacaccggctcggcggtggatcacgccgacggctacatccacatgtcgaccgaggcgcagctggccgagacggcgcgcaagcactatgcaggccgctccggcctgcgcctgctgacggtggagctcgcggtgaccgggggcgccctgaagtgggaggcgtcgcgcggcggcgccctgttcccccacctatatggtcctctgcccgtttcggccgtgacccgcgtccaggcgatgtccgtgtccgacaccggcgaggtgacgctgggggccggagcggcgtgagcctgacggagaccctgtccgactggggcgccgccgccctgcgccggctcgagcccgagacggcgcaccagctggcgatcaaggggctggcgcgcctgcccctgcccgccgccgccccagacgatccgatcctgcgcacgcggctggccgggctggacctgcccaatccggtcgggctggcggcggggctcgacaagaacgcggaggccctgcgtggcctgtcccagctgggcttcggtttcgtggagtgcggctcggtcacgccgcggccccaggccggcaaccccagcccccgcctgttccgcctggccgaggacgaggcggtgatcaaccgcatgggcttcaacaacgcggggctggacgtcttcgccggccatctgcgccgcgcccccgcccgcacggtcgtgggcgccaacctcggcgccaacaaggacaccgaggacaaggcggcggactatgtcgagggcctgcggcggctggaggggctcgccggctatttcacgatcaacatctcctcgcccaacacccccggcctgcgcgcgctgcaggggcgccaggctctggacgacctgctgggtcggatcgaccaggcgcgtccgccggtgggcgcgcccggtcgccggccggtgttcctgaagatcgcgcccgacctgtccgcggcagagatcgccgagatcgtcgaggccgccgtcgatcatgggatcgacgccctgatcgtctccaacaccacgctggcacgccccgccggcctcgcctctccccacgcggacgagagcggcggcctgtccggcgcgccgctcaagccgctggcggagcaggcgcttcgcgcggcggcggaggcggcgcaaggccggctgcctctgatcgccgtgggcggcatcggctcgggcgaggacgcgtatcgccgcatccgcctgggcgcctcggcggtgcaggtctattccgccctgatctacggcggacccggcctggtcggccgcatcaagcgcgacctcgccgcccggcttcgggccgatggctattccaccgtcgaggaggcggtcggcgccgcccgttgacggagcattagggctggcgagggcagtttgcgtcatgcgccggcgaatccagtcgcccgcagcgggaacacgcatgaccaagctcgtcgggcacgacatcgccagcggatggatcatcgccgtccggcagcgccgccgcgcggttctgcagcgggtagccgtgggtctggccagcggactggccgcgacgcccctcgtcggcgcgccgctcgccgccgcctggaccctggcctacatggccgtgcaggcgctggagatgtgggtcttcgagcccatcaacaccagccgccaggcggacgtcagccgcgaacgcaaggtcgtgggctgccttgtcctgtcgctgaacacaggcctctacggcgccctgtcgctgccgctgtggtggcacggcggagccatgggcggcatcgcagtggccatcatgctgccggccgcgatgatctactccacgctgaacgcgccgcgatcgccgctggtgctggcctgcaccgtgggtccgcacgtcttctacatggcgctgggcccctgttcatgatgagcttcggcgcctcggacgcggccgtgaccacggtgacggcggccgtggtgatctttgtggtctattgcatcaacgcctggcgccggctggccgagcgcaccgtgcaggaaggccgcgaacgccgcgccaaccagcgccgccagcgcgagatcgaacaggcgctgaccagccagcgggcctttctggccgccgttggccatgacctgcgcacccccatcggcgcgatcctgacgggcgccgccgagatgcgcgacagcggcgacagccaggtgcgcgtcaacgccgagctgatcagcgacgcgggcttgatgatgaaggctctgctggacgacctgctggaccattccaagctgggcgccggccgcatgtcggtggaggccgccgacttcgacctgcgcgccatgctggcccagaccctgcgtctgtggaaaggcgccgcgctcgccaagggcctgagcctgcggatcgaaggcgcccgtcacatgccggtcgccgtgcgcggcgactgcatgcggctgcgccaggtgctgaacaacctcctgtccaacgccatgaagttcaccgaaaccggcgctgtgaccttgcggctcaaggcctggccgaacgagcccggcggctggtcgctgctgatggaggtggtcgacaccggcgccggcatgacgcgcgaacagatggcgcgcctgttcaccccgttcgaccagaccgccgacggcgtctcggcccagcatggcggatccggcctgggcctgtcgatcagccgcgacctgatcgagctgatgggcggccggctgaccgtccgcagccagccgggccggggttcgatcttcaccatcgccctgtctctgccggagggcgagcatcagatcaccgccgagcctgcgccgctggacgaaagccgcgcggccgtcgctcgcgtcctggctgatcgtccccgacccgtcgccccgccccgccccgcgtccgtcccagaggccgcgccgccgcagccgatgtccgccgccgagtcattgctggcccagttgacggcggctcccgcgcctccgcctgagcccgaaccggaagccgaggccggcgagcggccgttgcgcgtgctggtggtcgacgatcacgacatcaaccgccgggcggtgcagttgatccttcagccgctgggctgcgacatcgccgccgccgcggacggcgtggcggcgctgaagcgctgcgaggaaagcgtcttcgacgtcatcttcatggacgtacgcatgcccgagctggacgggcgcgagaccacgcggcgcctgcgctccggcggcggacccaatgcggaaacgccggtggtcgcggtcaccgccgacacctcgcccgacgacatcgccgcctgccaggcggccggcatggcctatttcgtgtccaagccgctgacgccgccggctctcctgggcgcgctgcagcatgtgctgagcgatgcggaggccgaggtcgaagtcgcggcctgatcccgcaccgcgtcgaccagcgccccggcgaagcccggcgcgcgcatctcgcattcccacacggtgatgacgcgccagccgtcggcctgcagcgacgcggtgttgcgctcgtcccgcgcccggttgcggccgatcttggccgcccagtagtcggcgttggccttcggtcgtctcgatcctcgcgggcagtcgtgcccatgccagaagcagccgtgcacgaatacggcgacctttcgccccttcataaccagatccggccggcccggcaggccgcagccgcccaaccggtagccgatccccgccgcccgcaggatgcgtcgcaccagaagctcgggcttggtgtcgcggctccggacacgccgcatcacggcgctgcgcttttcgggagagaagacgtccgtgcctgcgcggacgccctcctctccgtccggcgtgtcggcgatcagagctgcgccagcaggtgttcggccgacgagacccggaattcgccgccctgctcgatgttcagctgggtcaccactccgtcggtgaccagcatggagtagcgctgcgagcgctggcccatgccgaagccctgcgcgtccagcaccagacccagttcgcgcgtcaggtcgccgttgccgtcggccagcatcaggatctggtcggtcttgacgccctggctctcggcccaggcggccatgacgaaggcgtcgttgaccgagatgcaggccaccgtgtccacgcccttgcccttgatggcgtccagattgtcggtgaagcccggcaggtggcgcgccgaacaggtcggggtgaaggcccccggcaccgcgaacagggccacggtcttgccgccgaagatctcggccgtggtgatcggcttggggccgtccgccgtgggcgtggacagggttgcgctcggaatgcggtcgccgatctggatggtcatgggagaggtcctttgggaacgcacgagcgcgtccgttggacagataaaggcttgttcacggcccgcaagcgggccgcttgcgcagccgctccggcatcccgattataggctgcgatgaacctcacacagtcccttaccggccacctgctcgtcgccatgccgggcatcgacgacccgcgcttcgagcacgccgtgatcctgatctgcgcccacggtccggaccacgccatgggcctgcggcttgatcgtcccgcgccgggcgtcgatctgaagacggtgctggacaagctggacgcgccggcccccgccgacagccagggccggcccgtgctgatgggcgggccggtggagcgcgagcgcggcttcgtgctgcacaccgacgactggatgacgggcggcgacagcctgccgttcggcgaggggctcgccatgaccggcacgcgcgaggccctggccgccatgaccgacaagacgggcggcccgcgccgctcggccctgcttctgggttatgccggttggggcgagggccagctggaggacgagctggccggcaacgtctggctgacggccgaggccgacctcgacctgatcttcgacgccgaccatgagaccaagtggacccgcgcccttgcacaactgggcgtcaacgccgccatgctgtcggcgcagggcgggaccgcctgacgccgttcaggtgatctggtccgggtgcgtctgggttcccgccggttttacgttcagcgggccttcggcgtcctcgtcgacctcgatcttcaggatgctttcgcccggctgcatctgcgtcaccgccgcatcgcccgcctgaatgtccgtcttggacggcacgagcagctcgcgggtggagccgccttcctggccgacggtcacgcgataggtcttcatccggcgtctcctgctgtcttcaggcacgatcaacgggcgccggcgcacgccgttccgggaacccgcccgcgcacccatccgctgtgttcctgcgaaaaggagaccgccatggacgacaagaaccagaccaaggggcgcgacgagaacggggccatccccttgggcaagcccgacgcctcgacctcggacaaggcggtcaaggacaatgcggcggtggagcagcgctcggccggcccggacggcccggacgcgaccgagatcggcgacaccttcaagcggcagccctgaggcgtcggttcaggccgagcgctgcttcagcggcgccgcgccgtccgccagcgactcggccagatagacctccgcctcctgcgccggcagcgcgggcgcatagccgaacccctggccgtagtggcactgggcctccagcagcaggcgcgccagctcggcgttctccacgccctcggccacgacctccagcgacaggtcgcgtcccaggttgaccaccgacttgacgatcttggccgagccctcgtccttgttcatggtcagaacgaagtaccggtcgatctttagcgtgtcgaaaggcaggcgcgccagatagctcagcgacgaaaagccggtgccgaagtcgtccagcgccagcgacgcgcccaccgccttcagccgcgtcagcacctcggccgccttggccgtgtcgcgcatgatgtcgccctcggtaacctccagcttcagcgcgccgcgcggcaggccggtgtcggcgatgatgcgctgcacgtcctccaccaggtgcgcccgctcgatctcgccaaccgacaggttgacgctgcagaacagatgcccggccagcggatgccgccgcagccactcagccagctgacgcgccgactcggtcatcatcagcaggccgagctcattcatcatcccgaggtcgtcggtcaagcccaggaactcgtcgggcggcaccagaccgcgccgcgggtgacgccaacgcgccaaggcctcgaaccccgccaccgccccggtgttcagattcacgatcggctggaagaagggcacgatctcgccgcgcaggaaggcgttcctgaggtccgcctccagcgccagccggctgagggagtcgctttccagcgctcgaccataggccgccgatccgccccggccggcgctcttggccgattccaccgccagttcgacacggcggagcagttccgccgcgtccggcgcgtccggcccgccttcgacctgaagcgcgcctatggacacggtcggatagatgtcgaagcccgccacccgcagcggctgctccagcgcctcgcgcatgcgcagggaggctgatcgcgcgcccctgcgcaccagcaccgcgaactcgtcctcgccgatacgcgcctgagccgcctcggcggtgaaggcggccgccagccgcgagcccagcgccgacaggaccaggtccgcccgctcatgccccagggcctcgttcagccggcgcatccggtcgacgtcgccgaccaccagctcatagtcgccgggctggaccagcatctcgccgacccgctgcagaaaggtgcgccgatccagcaggccggtcagggcgtcgcggtccgatcccgcgaacttggtctccagcgccaccacgcccgccgcacgcaggccgtcctccagccacacgccgcgccacagacaggtctccgagccgcgcatgcgcaggcgcacggcgacctccgtcccctccgcctgcggcttcagcatccgctcggccaggctgcggtcctgcggcagggccagggcgacaaagccggcggcggaacagtcgggcgccagcggacccagccccagcgaccgcgtcgcgccagtgaagcgcagctggtcctcggccggggtccacacccaaagggcggtgtcggcggctgccagcgcctcgatggaggtcgtggcgtcccaggccagcgatctggctcgcacgttcaaggcccctcgcccctcctggcggccggtcagccgccgtgatccacttcgtcctcgagcaggccgaacagcagatgatctgcccattcgccgttaattttaagataagccctggcctgcccctcatggcgaaagcctgccttttcaagcacgcggcgggatgcgtggttggtcggcaggcaggccgcctccagtcggtgcagcttcagacgtgaaaacgcgtggcgcgccatggcgctgaccgccgcggtggcgtagccgcgcccggcgaagggctggccgatccagtaacccagcgtccccgtctcggccacgccgcgccgcacgttggacagggtcaccgcgccgaacagctcgtggccggccgcgtcgaacacgaacatcggaagcgcggtccccagctccgtctcgcgttgatagatcgacagccttcgcttgaaggccgccttggacaggtcgtcctcgggccagcgcggctcccacggctgcaggtagcggcggctttcgtggcgcagcgccgaccaggcgtcgtagtcggccggacgcgggctgcgcaggcgcacgccgttgccccgcacccagccggtcccgccgtcgctcatcaagtccagaagcgccatgagggcgcaccttaagacctgtcgccccccggctccaagtcctcgttcagcaccgcctctatggctcgcgtggccaggccccgcccgaggtcgcgcggcgcctccagcatctgggtcagcacctcgccgatcaggccgtcggcgaaggccatgtagacggccgtcgtcaccaccgcccgcgcccgctcccgcgccgcctcgcccccgcccgccaggctcgccagccgctcggcctggtcgcggaccacctcggcgaaggcgtcggcccggcccgcctccccctgcatgaccatccaggcgcccagccgcgccgcgccgccctctccgaaggcgtcgaacacctgatcgagcatggcggctcggccagggttcgcgggcgcttcggccaaccccgcatccaggcgctcggccaggtcgcgcaccatccggtccatcaccgccccctgcagccccgccgccgagccaaagtgatggatcagattggcgtgccccacgcccatgcgctctcccaccgccttcagcgtcaccgccgatgcgccgccggccagcaacaggtcgcgcgcggcctccaccgcctcctctcgcgccagggcgcctctgcgccgggtcggccggttagttgacattgttgtcagttacatccatcttcagagcctgatcaggagccgacgccatgaccgtccacgcctcgcccgccgatctcgagatcaagccgcgccccctgtttatcgaccgggacgcgcccacgccacgctggtggctgaacggcgacccctacggcaccgccgtgctgaacgcgctcagcctgacgttcccggacggcgagcgcttctttatccaatcggtgcgccgcttcgccaaggatgcgccgccgcacctcgccgccgacatccgcgccttcaccgcccaagaaggcgcccacacgcgcgagcacatcgccttcaacgagatcaccgcccgcgccggctacgacaccgacgccatagaggcctatgtcaatgcacggctggacgtggctcgcgcgcggccgcccttggcgcagctggcggcgaccatggcgctggagcatttcaccgccgccttcgcccatcgcctgctggccgaccccgccttcctcgacggcgcgcccgacaacctcgctcagctgtggcgctggcattcgatcgaggagatcgagcacaagggcgtggcctatgacgtcttcatgcatgcggcgcgcaacctctcgccttggaggcgctggagcatccggcgctgggccatgctgctgaccacgctgctgttcaccaagacggtgcgcgagaccacgctgatgctgctggagcaggacggcatcaccggctggaaggcgcgcttgggcctgttccgctggctgtggctgaagccgggcctgtatcgccggatgctgggcgactacctcgccttctaccgccccgactttcacccctggcaggtcgatgaccgcgacctgatcgccgaggcggaggcgggcctgcctctccagcccgcctaggcgaacagcgcgcgagaaaaggcctcgccggccccggcgcccgccttgggccctagcacagccgtcgccgcccgtccgtccgccagcagccgcgcgccgaccgcccgcaggtcgtcggccgtgaccgcctccatctgctcgaccgagacgtcggtcggaaccggcgcgccgaagatcagcgtctgggccgccgcacgtcccgcccggctcatcggattctcgtcggccatccagagcccgcccttcagcaccgccttggcgcgcgacagttcggcgtccgtgggcccctgctcgaccagcccgcgcacctcggcggcggcgacttccgccagagccacggcccggtccgccgccgcgcccgcatagacgccgagcacgcccgtgtcctcataggcttcctggtaggcgtcgatggcgtaggccagcccccgctcctcgcgcgcgctctggaacaggcgagacgccatgcctccgccgaggatctcgccgaacaaccgcatcgccggcagcgccggatcggtcgcggccaggccgggcagttgaaacaccaggttggactgctcgatgcggcggttgagccggtcatgaccgccggtgaagcgcgcggcctccggcgccgcccgatcacccgaccgcgcctccgccccgaaccaacgctcggccagcgccagcagctcggcctcgtccacggcgcccgacgccgtgaccaccatccgctcgggcgcatacagcgcgcgccgccagccctcgatcccctcgcggtccaccggccgaaggctgtcgttcgaccccaggatcggccggcccagcggctggccggcgaaggcctgggtctgggccatctcgaacacatggtcgtcgggcgtgtcgaaggcctcggcgatctcctgggcgaccacgtccttttcgcgctcgatctcgtcgggatcgagcgtcggccgaaacagcaggtccgacagcacctgcatcgacaggccgagcgagccttgcaggccccgcacctcgaagctggtgcgctcatagccggtggcggcgttgatggagccgccctccgcctcgatccgctccacgatctcgcgcgcggccatgtcgcccgcgcccttgaacaccagatgctccaacaggtgcgaccagccggaccgcgcctcgtcctcccagcgcgcgccgcccttcaccgccgcgacgacggccagggtcttgaggcccggcatgggatcgcacacgacgcgcacgccgttggacagggtgtgaaggcggtgggtcaggggaggtctttcttcaagcggcggcgcagcagcgctgcatagaagccgaccagcgcgaccgccagcccgaaccaggtcagggcgtatcccaggtgattgttcgagaacgccgggggcggcgcggaggggcgaagggccggcgtctcggggttggcggtgctgaccgcgaacgccacctcgggcctgagcgccccctggacgcccagcgcccgcgccatggcggggccgtcacgggtgtagaagcgtccgttcgccggcggcggcgccagggccgcgggctccggcgacgtgcgcaactcgcctacgatcacgcccggcagggtggagggcagcacgcgcggccgcgtcgccaccccgtcggcgatgaacccccgatcgaccagcagggtgaaggcctcttccgccggccggcacgccgacaccagccgcacgcccgcctctccctccaggatgctctgcagttcgacgaacggcgcggtggcgaggcctgggcaggcgacgatcacgcgccggaactcgggcgcgccccccgccagcacctcggccagcggcgcgggcgggcggccctgcgccgccgccgccgcatcgatcaagccttctttccagcgcagccgctcgacctgccacacgcccagggcgaccagcacgccgaccaggggcagcaccaaggccgtcagcagccacggaaagcgtctcagcactagaacgctcctcccccctcaggggcggggaaccgcgaagcggtggagggggtctcgtcgccgcacggcgggagaaggttccccctcctccatgctgcgcatggtccccctcccccatggggggaggatcgcgagacccgccctgcgatcaaccgaagacgacgtagacgaaggcgaacaggaacagccacaccacgtccacgaagtgccagtaccaggccgccgcctcgaagccgaaatgcttctcgggcgtcagatgccccttcagcaggcgcagcaggcacacggccaggaagatggtgcccaccagcacgtggaaaccgtgaaagcccgtggccaggaagaacaccgacccgtacaggcccgagttcagcgcctcttcgttgaagaacaggttctcgtggaggatgtggttgtactcataggcctgcacgaaggtgaacagcacccccagggccacggtgatgatcagcgcgagcttggccccggcccggtcgcccacctgcaccgcatggtgcgcccaggtgacggtgcagccgctgagcagcagggtcacggtgttcagcagcggcagttgccaggggctcagcacctccaccccctgcggcggccaggtggaccaggcggcggcggtgtcggcccaggcccccacctccggcgtcagagcccggctctcgtggaacagggccatgtcgaagaacatccagaagaaggcgacaaagaacatcacctccgaggcgatgaacaggatcatgccgtagcgcaggcccagcgacaccaccggcgtatgatcgcccgcgcggccttccttgatcacgtccgaccaccagccggccatgcagatcagcacccccgccagaccggcgaagaacagggccggcttgccgtcgctcagcagctgtccggcgacgtcgtttccggcgggaaccaggccgcgcatccagaccacggcgcccaggaacatcacgaatgcggcgaacgacgacacgaacggccagatgctgggatccaccaggtgataatcgtggtgcggcttggcgtgtgcgtcggccatgcgagtccctctcccctcgtcaggcgacacagccgccttttcttttcagctataccgccggcttttccgccacgccagaggcgcgccgccagatcgccacaaacccgttcagcccgccttgggcgcgtccttggtcggatagaaggtgtaggacagggtgatctccttcacccccttcgcctcgcggtcggtggcgatttcgggcgcaacgaaatactgcacggggaactgacgggtctcgccgggcgcgatggtctggccgtcgaagcagaagcactgcagcttctggaaatacggccccgcccgctccggcaccacgttataggcggccgtggcttggatcggctggtccgaggtgttggtcacgtcgaaataagccatgccggtggcgccgatccgcacccgctggctgacctgctcggcgcggaagcgcatgggcagatcgcgcacgtttgtgtcgaaccgcaccagcaccgtctcgtccagcaccacgtccgaggccttgtccgcccgcatggtggtgccgtcgaagccggtcacctggcagaacagccgatacagcggcacggccgcgaacgccgcccccgtcatccccatgacggccagcacgcaggccagggcgatcaggttcttgcggttcaccgctgcgtctccggccgggcggcgacggactgcgtcggcgcgccgctgggcggggagaagctcgtgcccgccgccttctgggcgcgcatccgctcggccgtggccgccgcgtcgtcctggttctgatgcaggcgcagcacggtggtggtgaacaccagcacgatgaagccgaccagccccagcgcgatccacaggttgcgccgcttgcgggccgccagctcttcggggctcagcgtgatcatggcggtcagcctcccacccccggcagcgcctcgaccagaagcgccgcgaacagggccatcagatacaggatcgaaaaggcgaacaggtcacgcgccggcttggcctgcgcccgcacgtcgtacagcgccgcctcgcgcccgacagcctccgccttgtccggctcatcgccggcgcgcgagcggaacagccgccacgccagcagcaggaacgccagccctcccgcgaccgccaccgtcaggtagatcgccccgcccggccccacgatccccggcgccacggcgaccggcgtgaacagcagcgaatagatcaggatctgcagccgggtcgatcgcgcgccccgcgccaccggcatcatgggaatcccggccttggcgtagtcgccggccgaatacagcgccagcgcccaactgtgcggcggcgtccacagaaagatgatcaggaacagcagccgggcctgccagggcgccgaccccgccgccgccgcccatccgatccccggcggaagggcgcccgccgccccgccgatcacgatgttctggggcgtcctgcgcttcagcagcagggtgtagaagccggcgtaatagaccaccgtcatggccaagaggcccgccgccagccagttggcggtcatgcccagcagcatcaccgagaacaccgacaggatgacgccgaacgccatggcgtcgtggccgcgcacccgcccggccgccaccggccgtccgcgcgtgcgccgcatcagggcgtcggtctcgccctccagcgccatgttcagcgcgccggccgcgcccgctccgcaggcgatgcacaggatcgcgatcgcggcggccagcggatgcaggctaccgccgccgcgattctgggccacaatcaggccggtcgcggcggtgaacaccaccagagacatgacgcggggcttcagcagctggaagaaatcctccggctgcgcggtcgagatcgccctggtccgcccttcctgtctcgcctcgctatgcgccatgcgcgctgtctactccgatcgacccgccgtgtcgccgggaccaactgtccggcgacggggaaaaacacgccggctcgcaactgcgtcgccgctattcgaccgacaccgcccgaagaatgatcgccaacgaggtgatcaggtgcagttggagataacgatcatgcagcaggtcgctgggccggctcgccctgggaccgacgagcgtcgcgatgagccaagacagcatcgcggccactttcagccacttggtttcaagcccctccgctgcgaacgcgaaggtcgcggcggtcaaagcggccgagacaagaagaagagcggtcgccgtcgctctgcgtgacggggaccgctgcttcaaacctgtgttcggcacaggacgcctggcctcaatgcttctcggccgtgaccaccggcagttcgttgaactggtgctgcggcggcggcgaggacagggtccactccagggtggtggcgccttcgccccagggattggccacgcccttgcggcgacgcacggcggcctccagcagcatcagcaggaagacgccgacgccgacgatggtgaccacatagccccacgacgacacctgattccacagggtgtaggcctcgggatagtcgatgtatcggcgcggcatgccctgcaggcccaggaagtgttgcgggaagaacaccaggttgacccccacgaacatgatccagaagtgcgcggcgcccaggaactcgttgtacttcaccccgaacatcttctcgaaccagtagtagaagcccgcgaagatcgagaagatggcgcccagcgacagcacatagtggaagtgcgccacgacgtagtaggtgtcgtgcaggctgtagtcgatgccagcgttggacagcaccacgccggtcacgccgccgacggtgaacaggaagatgaagccgatcgcccacagcatgggcgtcttgaagctgatggagccgccccacatggtggcgatccagctgaagatcttcacccccgtcggcacggcgatgatcatggtcgcggccacgaaataggcgcgcagattgatgctcatgcccacggtatacatgtggtgcgcccacacgatgaagccgatgaagccgatcgccaccatcgcataggccatggccaggtagccgaagatcggcttgcggctgaaggtcgagacgatgtggctgatgatgccgaagcccggcaggatcatgatgtacacttcggggtggccgaagaaccagaacaggtgctggtacatcaccgggtcgccgccgccggccggattgaagaaggaggtgccgaagttgcggtccgtcagcagcatggtgatggcgcccgccagcaccggcagcgaaagcagcagcaggaaggccgtgatcagcacgccccaggcgaacagcggcatgcggtgcagggtcatgccgggcgcacgcatgttgaagatggtggtgatgaagttgatcgcccccaggatggagctggcgcccgccacgtgcagggcgaagatggccaggtcgaacgacggcccggtgtggccggtggtcgacaagggcggataggccgtccagccgcctccaaagccgcgccccggtccgccgtccacgaacaggctcaggcacagcagcagaaaggcgaagaacagcagccagaacgagatgttgttcaggcgcggaaaggccatgtccggcgccccgatcatgatcggggtgaagtagttggcgaagccccccatcgtcgccggcatgacaacaaagaacaccatgatcagggcgtgggccgtgaccgtgacgttgtagccgtgcttggaggcctccacgaggccgaggttctggatgatcgagccctcgcggaacagctgaatgcccggctcggccagctcccagcggatcaggccggacagggcgccgcccagaaggcccgcgaagatcgcgaagcccaggtacagcaggccgatgtccttgtggttggtggacatgaaccagcgggtgaagaagcccatcttgtggccgtggtcggccggatggtgctggtcagcgtgaacgtcgcgcggattgagggtcgcgtcagccatgtcggttttcgcctcttactgggcggccggcgcggcggcggccggcgcggcgggctgggccggcgcggtcgccggctcggtcgggttctgcggaatgtcggcggtcgcgccgaccggctgggtctgggcggcgggcgcctggccggtcgtgggtccggtcgtggcctggccgaccacgggcgagccggtcgtgccggccgcgttctgcgccgccgtgccgccggcgggcgccgcgcccggaggcgtcatggagccgcccttggaggcgacccagcgttcgaactcggcctgggtcaccacattgatctgcagaggcatgaaggcgtgatcgacgccgcacagctccgagcattgaccatagaagacgcccgtgcgctcggccttgaaccaggtctcgttgacccgaccggggacggcgtcggtcttcagcccgaacgcaggcagggcgaccgcgtggatcacgtcggcggcggtgaccagaaggcgcacggtccggccgaccggcaccaccatcggctcgtccgccgccaggcgatagggcacgccgcgcgcccgcgcctcctcctcgggcaacatgttggagatgtattccggcaccgcctggtccggatattcataggcccagttccactggttgccggtcaccttcaccgtcaggtcaggctcgggcatgtcgtggtaggcgaacaggagccggaacgagaacagggcgatgcccaccaggatcaccaccggcgccaccgtccagatgatctccaccgtggtgttgtggctccagcgggcgggcgtcggattggcgcgcttgttgtagcgcaccacgatccagatcagcaggcccagaaccagcagggtgatcagggtgatcaccggcatcagcacgatgttgtggaagaagatcgcgtcgtgcttcagcggcgcggccgccggctgcagatcgatgccgcccggcgtcggctggcccatcaggtcctgcgcggcggcgagacccgccatcgtcgccatcgtcgcgaaagtccccgcgccccaggccgccctgcgggctatgctgcccatccccatgcgagccgtccctcgtgtaagtcgttcttccgcaagcctttgcgaacagatcgcaactgctccgtacggcgtttgcgccgcacgctccctatggtccgtccgtatcggatcgcgtctgccttgccaagcgatcagcgacgccgatccatccgggagaacgccgatgttaaatcgatgtcatgtttcaacagctaccttgcgctacatggtacctgtcgatagtctcttcacatcacaggagacgccgaggtgcctgaaaccatcgagatacagctgaagaagggggtgctgggactttgcgtccttgccctgcttcaccgggcggacagctacgcctacgagatcgccagccgcctgtccgacgccatcggcatgggcgaagggaccatctatcccctgatgcggcgcatgcagtcggacggcctggtcgagacctatctggtcgaatcctcggccggtccgtcgcgcaaatactatcgtctgacgtccgccggccgcgaggcctttgaggcgcagtcggcggaatggtccgccttcgcccgctcggtcgacgcggtggtcgccgacaccgcttccccgtccacgtcagaacccatgggagccgttcaatgacgcgcgccgactttcttcgccgcctgaaggccggtctggtcggcctgccgacctccaccgcctccgacatcctcaacgactacgaggcccatttcgacgacggcctggccgccggccgcagcgagtcgcaggtcgccgaggcgctgggcgatcccgaccggctggcgcgcgagctcaaggccgaggcgggcatccagcgctggcgccaggaaaagaacccgtccgccgccgcaggcgccgtgttcgcggtcctgggcctgggcgcgctcgacatcctgatcctcctgccgatcttcatgggcgtggtgggggcgctgttcggcttctacatcgccgccatcggcctgttcttcggcggcggcgccgtcatggtggccggacccttcgcgggctttcccggcggaccgctggccgcgatcctgatgggtctggccttcatggccggcggggtcttcatcgccgccctgaccaccgtcttcaccatctggctggtcaacggaaccgtgtggttcgcgcgcctgcactaccgcctgctcaagcccgcgctcgagccccagtccacgacctacgttcaggagcccgcccaatgatccgcaccctgttcatcatcgccggcgcggcgcttgtgctgtgcatcgtcaccgcgggcggcgccgtcgccatcggcggtcaggacctgcagcgccacggctggtcctggaccttccgcgacgaggacggagaaagcgtccgcttcgagcgggtccggggtcccgacgaacccgacgtgagccgcaccctcccctggaccggcggccgacggctggtcaatgcgacgccctttgacgtggaataccggcagggcccgaccgcctcggtcgtggtcaccgggccccggtcctggaacgatcgggttcagctggccgacggcgtgctgcgcctggccgacggtccggtcaacgaggaggcggtgatccgctggagcggccgcaacatcaccggccggtcgttcgacgacgccgtccgcatcgtggtcaccgcccccgatgtcgccgccttcgaggtgcagggcgcgggcgacctggacatccagggctatgaccagccggcgctcagcgtcgcggtgtccggctcggccgatgtgacggcgcagggccgcaccgaagccctggaggtgaccatcaacggctcgggcgacgcggccctgaaggacctgacgacccagagcgcccgcgtggtcgtgtccggctccggggacgtgggcgtctcgcctcgcgcagaggccaatgtcaccatcaacggctcgggcgacgtcagcctcggatcccggcccgcccgcctgacttccgagctgaacggctcgggcgagatccttcaggactgaggacgccgtctcggcccggacgccgccccgcctcgcgcggggcggcgttcgtctatccggcgggcgccagccagggcgagaccttgtccaccagcgcgcgcgtcggccttctgggtcgtccatccaggtggatgcacaccgccgtcacctcggcccggcacagcacctcgccgccccgctccacgctctggcggatcaagaggcgcggtcccttcaccgcctcgtagagggtgcgcaccaccagggcgtcgtcgatccgcgcgggttttaaaaagttcaacgccatctccgacaccacgaacgccagcggctcgtcgcccttcagcagttcggcgtgtccgatccccatggcgcgcaaacagtccgaacggccccgctcaaaatagcgcacatagttggcgtgatagaccagcccggtgaagtcggtgtcctcgtaatacacccgcaccggcaacaggtgcgcgcgcccgtcgaagcgtccggcggtgggctgatcgatcatgcggacgctccttattcgaacaggccgctctgcgccggcggctgaggcggcgcggtcaggcccaggtgctcataggcgcgggcgcaggccatgcggccgcgcggcgtgcgctggatgaaaccctgctgcagcagatagggctcgatcacgtcctcgaccgcatcgcgcgcctcggcgatggcggcggctagggtgtccatgccgactggcccgccgccgtagttctcgatcagggccttgaggaagcggcgatccagcgagtccagtcccgcctcgtccacctccagccgcgccaaggaccgcgcggccaccagccggtcgatgacctcggcgccctcggcggtcgcgaagtcccgcacccgcctgagcaggcgtccggcgatgcgcggcgtgccccgcgcccgagaggcgatctcgcgcgccccgccctcgtcgatcggcgcgcccatcttcctcgccgctccgcggatcaccgccgtcagctcgtccggcgtgtagaactccagcctcagcggaatgccgaaccggtcgcgcagcggcgtggccagcagccccgcccgcgtcgtcgcccccaccagggtgaagggcgcaagatcgatccgcaccgtcctcgccgacggcccctcgccgatgatcaggtccagcacatggtcctccatggccggatacaggatctcctccacctgcggcgccaggcggtggatttcgtcgatgaacaggacgtcgcgcggctctaggttggtcaggatcgccgccagatcgcccgccttggccaggatcggccccgacgtcgcgcggaaccccacccccagctcgcgcgacacgatctgcgccagcgtcgtcttgcccaggcccggcggtccgaacagcagcacatggtccagcgcctcgccgcgcgcgcgcgccgcatcgatgaagaccttgagattgcccttggccgccccctgccccacgaactccgacagcgtctgcggcctcagcgcccggtcgtactgttcgccgcccgacgcttccggagagatcacgcggttcaccgtcccagctcctgcaggcccgcccggatcaccgccgacagctcggcctcgtcacccagccggatcagcgcctgatccaccgcccggcgcgcgttcacttccgctatgcctaggcccagcagggccgacaccgcctcgcccacgagactcggtggcggcggcgcgacctcgacatgcacgccggtggcgacgggtgcgaacaccccgtccgtcagcgtcttgcccttcagctcggtgacgatgcggagcgccagcttggtccctaccccattggcccgcgccaccgccgccttgtcctcgcgcgccaccgccgaggccagctcgcccggcggcaggacgtccagcaccgccagcgcggccttgggccccacgccttggatggccagcagcgtggtgaacgcccgccgctcgtcgcgcgagaggaatccatagaggcgcggcccctgatcctcgctccactggctgtggatgtagagaatggcctcgtcgcccggcgccggcagccgccccagcgtgcgcgcgccgcacgacgccacatagcccacgcccgcgcagtcgatcacgcagtccgcctcgccgacctcggccagcacgccgcgcagccgtccgatcacgccgcgccccggtgcatggcctcgatcagcgagcgtttgcgcaactgcgcatgggtgatcgccaccgccagcgcgtcggccgcgtccgccttgacctcgccgcaggtcggcagcagccgcttgaccatgaaggcgatctggctcttgtcggcgtgacccgcgcccaccaccgccttcttgatcagggtggccgaatattccgccacaggcagacccgccttggccggcgccagcatcaccgccgcacgcgcatgccccagcttcagcgtcgaggacggattgacgttgacgaacacctcctcgatcgccgcttcctcgcagccgtggtcggcgcagatcgcgcccacatgctccagcagatgcagcagccgctcgggaaacggcgcgctctccggcggcgcgaccaccccgtgcgcgatccagcgcagccgcgagccgtcgctttccaccacgccccagccggtgcggcgcaggccggggtccagccccaggattcggatcgggttgttcgccatccgttcccttctgcccgaaagacggttagcgagcaatgaagggcggcctcagtcgtctcgcggatcgaaccggtaggccgtgaccccttccatccgacacagggcctcggccagacgcttcaactgatcttcccgcgccgcctgcagcttccagctgcgccggatcatccgcccctgttcgatcagctcgaaccggttgtgccgcgtcgtcggatcgacgtcgcggaacaactgctcgatctccggttcgggcgacgtcgcccctcggcgccagcagacctccgcgtccaccagcgtcttgggcggcaggcgcgccgataccagacgcagccccgtcagaacacccaccgtaaccagcgtgcccgccgcgcccaggccgaacatccccgccccgaacaggaggcccagggccgaggtgatccacaacgacgcggccgtggtcagtccgtgaatggaaaagccggtgcgaaagatcacgccggcgcacagaaagccgatccccgtcagcacgccatgcgccatgcgcgtgggatcggtgacaatgttctcgtccggcaaggcctcgaacgcccactgcccctgcgacatggccgccagcatcagcaggcacgaggccaaggccaccagcaggtgagtccgcaggccagccgcccgccccctccactcccgctcgaagccgatcagtccgccagccagcacggctccaatcagaggcggcgcatagtcggcgaaacgggcgaactcgatcatgccgcccgaacggatgctccgaccacggcgttccgaaggtgcgccgatcggacgctaggacgtccgcatcaccccgcgtacttggccgcgtcctcgtcggagatgtcttcgttggaatagacgttctgcacgtcgtcctcggcgtccagcgcgtccagcagcttgaacagcgtgccgaccgcctcgcccgtgaccgggacctccgactgcggcttccacacgatggcggtggacttggggtcgcccagcaccttggacatggcgtcggccacctcgttcaggtcctcgaaggcggtccagatggtgtggccgggcgcgtcctcgtagatgtcgggcttgaccaggtcgctttcgacgtcggaggcgccggcctcgatcgccgcctccatcaccgcgtcctcagtgccggcttccgccgggtagacgatcttgccgaccttgtcccacatgaaggcgaccgagttcatctcgcccagcgccccgccgttcttggaaaaggccgagcggatgttcgatcccgcgcggttgcggttgtcggtcagcgcctcgacgatgatgcccacgcctccggggccgcgcccctcgtagcggatctcctccatcgtatcgacgtcgccgccggccgccttgttgatggcgcgctggatcacgtccttgggcaggctttcggccttggcgttgttgacggccaggcgcaggcgcgggttcagcgccgggtcgggcatgcccgacttggccgccaccgtgatgtcgcgcgacaacttggagaacagcttggaacgctgcgcatcggcgcgtcccttgcggtgcatgatgttcttgaacttcgaatggccggccatgggatcgtcttggaagtctgcgggaatcttgtgtccggcgtcctagccgacccgcgccatcctgtcacgatggcgccgcttgcgggaaccttgaccatggctggaggatttgaggcgggcgcgcggccggggcgcgcaccgttttgagaaagggcgtctccctggaccgcggaatccccaacgtcgtcgaggactatgaggacgacgcctatgacgacgccgacatcgtcgagtggtacgaggcccggcccgtcaccgttccgcccgccgtcgccgccggttccgtgatcgccgcctttgcgctgggcgccctgaccgccgccggcgtgcttctgctgctgcagcgcctggacgactgatccttcaagaaggacgaggcggggccgggaccccccccccccatcctcaccgcgccggcggcgtcgccggcgcggtcttgacgtactggtccagccagcgggtcatctcccacagcgtatggccgaccgactcgcgggcgcgatagccgtgcgcctccagcggcagggtgacgtagcgggcggtcgcccccagccccttcagcgccgcatagaagcgctcggtctgcaccgggaaggtgcccgagttgtcgtccgcctcaccgtggatcagcaggatcggctcgttcacctggtccgcataggtgaagggcgccatctccgtatagacctccgtcgcctcccagtagttgcgctgctcggcctggaagccgaacggcgtcagcgtccggttgtaggcgcccgaccgcgcgatcccggtgcggaacaggtcggtgtgcgccagcaggttcgcggtcatgaaggcgccgtagctgtgcccgccgatggcgatgcggccgcgctcggccacccccatctcgaccaccgcgtccaccgccgcctgcgcgtccgccgtcagctgctccacataggtgtcgttgggctcggccccgtcccggccgatgatcggcatggaagggttgtccaggatcgcatagccctgggtcagcaggaacaggtggctggacccgcccggccgcacgaagcggttctgcacatccaccgtctggcccgccaccgacggatcggtgaactcggccggataggcccacatcaacagcggcagcggaccgtcgcggtccttgtcgtagccggccggcaggtacagcgtgcccgacagctgcacgccgtccgcgcgcttgtaggtgatcagccgacgcgtcgcctcggccagctgcggcgcggggtcggggaagttggtcagctgcgtcgtctgacccgtcgtcaggtcgcggatgcgcaggttgggcggatccagccgcgtctcgcgctgggtcaccacccgcttgccgtcctcgtccaggaaaccgatcaccgcctcatagtcggtgtcggccgaggtccacagccgctcgcttcggcccgtcgccacgtccatcgcggccaggaacgggaactcgccctgcggcgtcgcgcccggcccgctcatcaggatgcgcccctgcccgtcaaagcggatcaccgaacggcccgccgcgttcggctgcagcaccggctgccccggattgtcgtagcgcgcctgatagttgcgctccagcagcacccggccctcgcccggattcgacggatcgaccaggaagcgggtctcgtgccgggtgttgaaccagcggctgttgacgatggccaggtcgtcgcgcccccattggatgccgccatagcgttccttcaggtcgatcagcttgaccggctcggcggtgaagggcgcggcctgcatcagcacccggtcgcggaactccgcctcgcgccggatgtcgccgccgtccagcgcctcgacccacaccagcgtcgccggcgcatcggcccgccactgcaccgagcgcggaccgggcgccaccgcatcgaaggcggtcggcacgtcgtcgcgcagcggcaggtcggccacctcacgcaccacccgcccgttcagatcggtgaccacgatctcggtcgggaacaggccggccggcacctgatagctgtatgggcgcttggcgatctcgtgcagcacgtatcggccatccggcgatgcggccgaatccagatacaccgccggctcgccgatcgtccgcgcctgtccgctcagcggaaccagcgtcagctgcgaggtgaaatagtggtcgaacagcgcctcatcggccgggttctgcagcaggtcctgataggttcgcgccggcgccacgcgccccgcggtctcctccacattggggccggtcggcgtccgatcggcgaccggcgccgccccgcgccctgcaggcacggcctcgaccagcaacgcccggctatccggcatccactcatagccggcgcccgcggccatgttgacgcgcggcccgtccagctttcgggcacgcgccgaggccacgtccaccacccacaagtccagcccggcgggcgcgtccatcaccagggccagcgacttgccgtccggcgagaagcgcgcggcggtgaagcgcgaaccctgcggcagggcgacggtcctcggctgtcctccgtccaccgcctgcaggctcagccccgtcagccaggccacccggctctcggccgggccgttgttgcgcggattgatccgatcgcccgccagcctcagcatcggctcggccagcgccgagatcgccggcaggttcgaccggtccatcagcaccagcgtggagcgatccggcgacagcatcgacgacggcgtgggcttggaatccagaatgtccgcgatcggctgcggcggctgctgatacgtcagggcgccggcctgcggcgtcgccgccgtctgcgccaacgccgttgtcgccagcaacatcgccgccagcggcaagcccgctcccatcacccgcttcatcattctggacgctccccgttccatgtagatgttacaccatacaggcgcagcccccggcgccaagccgtgatcggccggccggaacgtcgccccctcccgagggttgattccgcatccacagtgaaaaggagcgcctcatggccgacgaggaagtcaaggcaaaggatcccaccaagcagaccgagccgggcaacagcggaaccggcgaactgcgccccgaccagaacgccgccaccggacctgcgcagaagccgccctcgcccgtctccggcggtgaaggcgcggcgggcgccgggggccccgccggcgtcggcgggggcaactaagggcgccgacaaggcgcggcggttcgccgccgcgtccccccgccagcagcgcctcgacctcggcgcgctcgggcagggacggctgcgcgccggctcgcgtcgccgcgatcgccccggcggcgcaggcgaaccgaagcgcctcttccggcgccagcccgtccagcagggccacggtgatggcgccgacaaaggcgtcccccgcgccggtggcgtccaccgcctcgacgaccggggccgaggcccaagccatctcgacgccgcgctggtacatggccgcgccacgcgcgcccttggtcaccaccacccggccgccgccgcgatgcaggccgtcgccatagaaggcggcctccgtttcgttgacgacgatcaggtccgcgcgccgcagcaacatctccgacaccggcgcggcgggcgccaggttggcgcacacgaaaccggtcgcgcggcccaccgccgcctccaccgtctcgatcggcagctccaactgcacgatcagcggtccctcgatgcgttgcggcagctgttcgggcgtgacccagtggttggcgccggccgccaccacgatctggttctcgccttgaggatccaccgcgatcagggcgacgccggtgggcgcggcgacgtcggtctccacccccgacagatcgaccccgatggactccatcagcgccagcgcctcgcccgccatggcgtcgttcccgacccgcccgatcaggcagacctcggcccccagcttttccgccgccagcgcctggttggcgcccttgccgccggggtggcgctgcagcgtcgcgcccgtcaccgtctcgcccgcactgggcaggtgcgaggcgcgcgccaccaggtccaggttgatcgagccgaccacggtgatcctcaacgcccgtcctccgcaggcgtcagggcgcgcgcgatcaggtcgaacaccccgtcagcatcgaccccgacggcccagcgatgccgtgcggtcgccggatcgaccctgaactccaccgcggtatggccccgcgtcagctccgatgcggtctccacctcgatgcggcagggacgcagccggaacaggttgggccgcagccgccaggcgatggtgcaggggtcgtgcagcggcgccgcctcccaacccaccaccgtccgctccaccgcttgcgaaaagcgcagcatggccgccgccgtccgcgccggctcggtgcggatcgtctcgatggcccggatgcgcgcctcggtcgcccgcacctgatgcgtcgcgtccagccccaggcacaccacctcgcagcccgatccgaacaccaccgccgccgcatccggatcggcccagacgttgaactcggcggacgcggtgacgttgccgccctccgagcgcgcgccgcccatcaccaccaccgtcgccagccgctcggccaggcgccgctcgcgcttcatggccagggccagattggtcatcggccccatcatggcgatcgagacctcgcccgccggccgcttcatcaccaggtcgacgatggcgttggccgccggcccgtcgccgatgatgccggccggctcgaacggctggaggtcgcccaacccctccggcccgtggaactcgcccgcgtgggccggcggccgcttcaacggccgctccgccccgccatggaccgggacgtcctcgcgcccggcgatctgccggatcatgcgggcgttgcgctgggtccggtggccggggacgttgccggcgacggtggtgacggccagcacctccaactcgggcgaggcgaaggccagcagcagggccacggcgtcatccacgccggggtcgcagtcgatgatcaggggcaagcgagacaccgcctctgactagtcgccgccgcccgtcgcccgcaagcgctaaccgcccgccagacccggctccacgcaccgcagcgccggcattccggtcgtgccggtcagcggcgccgccagccccccctccctcatcccttcagatagaacaggtcttccaccgtggtcccgagcgcccgcgccagctccagcgacacgatcgtggacgggacgaacacgccgttctcgacggtgttgatggtcttgcgcgacaccccggccctttccgccagccccgcctgggtcagggcggcggccgtgcgcgcctccttcaggcgcacgcccagccgggggtcacccatggcgctcggccgcgcgatccagccaggcgaaccgcagccccgccgtcgccccgcccgccgccagcacatagggcagggccgcgacaccgaccgcgggccgccacatgcccagcaccatggcgaccgtcgcccccgccatcagcaccacgaacgccagcatcatcgcctgcgcccgcatcgactgggtcagttcgtcgtccagaaagcgcctgtgctggcgcgtgttccagtcccaccccatgacgatggcgggcaccagccagccgtagatgaccggcagcgagacttgcagatacgcccccaggccgccctctcccgccagcaccgcctgcatgccccgatgcgcctgcatcatgaaggccagcatcacgaacggaaagatcaccagctgctgggtccggccgcgctgaagccgatcgcggcgcgtttcttccccgtgggtcgccgggtcaagcggccggcccggcctcgaacaccaggccagcgccacgccggcgaacaccgccacgacccccatgccgaccgccacgccggcggccgtggccacatcgccttcgccgccggtagccagccccacggccgcgccacccacgatggccgcgacgctgacgccgacaacacccagccccagccgaaaccgccccctgcgcacccgcgccagctcttccatcaccctgccgtccgtcatgccgatcaagctcccgattcgtaacccttgggttacatatcacctatgggtgacacgcagtcaagagaggcccgcaagtccagcggcccactcggcgaactcgagccaggatgcggcttcatggccggccttggtcgatgatcatgatgatcgcacgcgtccagcgcctcgatcggatgatccgaaggccagcaaggggtgggaagcgggcgtctttaccgcgcgaggcggacaggcgcgccgtcagacgctttgttgccgactccgttcggaaccgggacggaggagttggcgtaatctgcattgatctgcagcgcgcgtccgccctcgaccttgaagtcgcgagccacgatgacggtccaaggcgtgacttcggtcgcgttgatgccgccggggacaatgatcctcaccttcggcgcatagaccacgccttccagacgccgaatttcacggaagttgaggttgatgtcgcccgtgcgcttaggatcgacggcgagagcaaacccggcccaggtgtccatctcgcccgaaccaccctgacttccggagaggtccagcatggcgacctggccatctgtgaagttgatgtccaagtctttccaaatgatcagggtgacgttctccccctcgacctttgcgcccttcttcaactgaagtttgccgttcttcaggtggtgaacgccaggtttgaaacggagggtgcccgcctcgatttcaaagtggcggcaatgcacgcccggatcgacctccacgaccgcccccgccttgtccactttcacaagattgccgaactggcagttgccgggtcccgcgccgttgaacatcgccgtgagcgggtccggaatgggcgcagcgccagttccggcattggctggcgtactgcccgttatcgaattcacggcatgcaccgccgccgcatcaacgaccgtcgatcctccaacggaaatgctcttgttggaatgaacgaggcacgccgtggcggtgatgcgggcggacggcagatcaagggcgtttgttgcagtggacccaaggctgagaacacacaagggcgccgtggcgacctgcaatgccgtcgacgcagcagaaatcacaaatccacccggcggcacgagattgccgaagaacgacatgcgacgcgccgtcagggtcacgacgacaccgctgggccttccctgctccagcaaaaacttgacgtcaggttggtcgggcgtggacgtgaggccttccaggccgctgagagcgaacgcgcgagcgcggtcaagaacgggatcgttcgcggcgagacgcatctgtccggccgcggccagcgcagtggcgtcggcgacgtctctgagccgctgccgatccacactcagcgaatagagttcgacggatgtgaccacagctagaagcagcgccggcaggccgaacgccgccatgagcgcgatgttgccgcgcgtgtctttccagaagctcttcacgtgtcacccacacttgttcccctgaggtaggcgatcagcggtgaaggttctgttacggcaacgtcctctcgctcaggatggtggggtgactttgccgttacctcgacaactccgtcgccatcgtcgcttcaaacggacgccctcaaggtctgcggcgggtatgaacccgaagtctgcgttataaccgcaagccggccccgccctcccacgtccgctcccccgatcgcgctctcgtagccgacagcccctgcgccccgccggtgtgcaggaagaccggtctcgaccgtgaaccgccccttgtctgcaggaactcggcccgatgcagccaatcgcgccctccaagcgttgccgttcacatgagcagcctggtcatcgatagggggcgagagcgccgctacctgcgcgatctcggacgtgcggtcggcggggccctgctgttcaacatcccgctactcatgaccatggagatgtggcaggctgggatctacatggaccggctgcggttgctggcctttttcgccgccgccctgccggtgctgtacggcctgtcctactatgcgggcttctcaaaggggcgcggactcaggaacgacgtgctggacgccctggtcgcgctggcggtggggtttgcggtcgcctcctgcctgcttctgctattcggggtgctgcaggtgaacgcatccccgctcgacaacgtcggcatggtggcgctgcaggccgtgcccggcgccatcggcgccctgctggcgcgccggcagatgaacggcgacggcgacggcgacgacaaggaggacgagagccgcgcctcctatggcggagagctgttcctgatgggcgccggcgccctgttcttcgcgctgaacgtcgccccgaccgaggagatgatcctgatcgcctacaagtgcacgccgtggcacgaactggggctgatcgcggtgtcggtgctgctcttgcatgtcatcgtctattcggcggggttcgcgggacaggaggagcagggccggccggttacagcgttcttccgcttcaccctgcccggctatgcgatcgccatcggggtcagcctgttcgtcctgtgggtgttcggccgcacggacggccatgcggcggcgcgcgccatggccacggcgatcgtgttgggctttcccgcctcggtcggcgccgccgccgcccggcttctggtctaggaggagacgttcatggcccgccggcccattcccgacgcctctcccttgacccagtgggtcgtcgccgcgatcggcctcgtggtcaccctgggcgcggtcggtctgatggtgttcgagctgttccagcaagagcgcccgccgaccctgatcccgcgcatcgtggaggtgcaggccacccccgccggctatgtcgccgaggtcgaggtgcgcaacgacggctccgacaccgccgcgggggtcgagcttgaaggcgtgcagggccaggcgaccgcctccgccaccctggactatgtccccggccgaggctcggccaccgcctttctgcgcttccccaccgatccgcgtagccagcctccggcgctctccatcaagggctggtcggcgccctagagccgggttatggtctcttcgttctccggggggtcgcgttcgagcggctgagattggcgtagccgcctgacccgtcgaacctgatccgggtcatgccggcgaagggatgagacacgcggaccccacgcccggagtcccgctcgccatcgtcggcggacctcttgcaaacagaggccgccatgaacatccacgtttccgccccgtccgaagagccccaatccgatctcgccctggccgacgcacgtcgcgcggtcgaggccgagaccggccgcatccccaccggcccccgcgccggcggaaacaaggtctatgtctcgggcgatatcttccccgacctgcgcgtccccttccgcgaggtgcacgtccccccgagcgccaacgaaccgccggtcacgatgtacgacgcctccggcccctacaccgacccgcacgccgccatcgacatcaagacgggcctgccgcccgttcgcggccgctggcagcaggagcgcggcgacatcgccccggtcgcccacccccgcgaggtcaagcccgaggacaacggccacgcctcgggccgtcatctcgccccccgcttcgacacctcccgccaccgcgtgttcaagggcgtgcccggccgcccagtgacccagttcgaatacgcccggcagggtatcatcacgcccgagatggagttcgtcgccatccgcgagaacctgcgccgggagcagtcggccccgtgcgtgcgcgacggcgagagcttcggcgccgcgatccccgacttcgtcacgcctgagttcgtccgccaggagatcgcccgcggccgcgccatcatcccggccaacatcaaccaccccgaggtcgagccgatgatcatcggccgcaacttcctggtgaagatcaacgccaacatcggcaactcggccgtcctgtcgaccgtggacgacgaggtggacaagctggtctgggccacccgctggggcgccgacaacgtcatggacctgtcgacgggccgcaacatccacaacatccgcgactggatcgtgcgcaactcgcccgtcccgatcggcacggtgccgatctatcaggcgctggaaaaggtcggcggcgtggccgaggacctgacatgggaggtgttcgccgacaccctggtcgaacaggccgagcagggcgtggactatttcaccatccatgcgggcgtgcgcctgccgttcgttccgctgacggcgaaccgcgtcaccggcatcgtctcacgcggcggctcgatcatggccaagtggtgcctggcccaccaccgcgagagcttcctgtacgagcatttcgccgacatctgcgacatcatgcgagcctatgacgtctccttctcattgggcgacggcctgcgccccggctccatcgccgacgccaatgacgaggcccagttcgccgagctgcgcacgcttggcgagctgacgaaaatcgcctgggacaagggctgccaggtcatgatcgagggccccggccacgtgccgatgcacaagatcaagcagaacatggacgagcagctgaagcactgccacgaggcgcccttctatacgcttgggcccctgaccaccgacatcgcgccgggctatgaccacatcacatccgccatcggcgcggccatgatcggctggttcggcacggccatgctctgctacgtcacgcccaaggagcatctgggcctgcccgaccgccaggacgtcaaggacggcgtcatcacctacaagatcgccgcccacgccgccgacctggccaagggccacccggccgcccgcctgcacgacgacgccctgagccgcgcccgcttcgagttccgctgggaggatcagttcaacttaggcctggaccccgagaccgcgcgcaagttccacgacgccaccctgcccaaggaggcccacaagaccgcccacttctgctccatgtgcggccccaagttctgctccatgaagatcagccaggacatccgcgacgccgcgcgggggcagaacgacgcgggcgcgagcctggtcgatgccgaagcgggcatgcgcgagatgtcggagaagttccgggcaggcggcggcgtagtggaggtgaaggtgtgagggcgtgagctatacacgcccgagtagcgagggttaggctcggtcctacagagtcggattttcgctgagggtatagggtggatcagtcagtttgcggatgcgccatgtgcgcgttgtcgatcgatttctcgatggacgagcatttgctgtcggaaatagaaaggcataactgcgtcatattcgccggcgcaggtatcagtacggaaacatcggatactcaccccgacactctctacgaccagcttagacatcagataaaatgcgaggattatcctcaattctgggaactagtggaccgatttgaggcgcagccaaacggacgtcaaaagttaatagagctggtcaaggaccggttcggatatatcaatggatttagagatttacggcagcaggcgacgcgctttcaccgcgctctcggaaacgctccgtacttcaaatcgatcataacaacaaactgggatcgatacttcgaagatgtaatcgaagccacgcctttcgtgtacgacagcgacatcccactatgggatacagcaaagaggccggttatcaaaatccatgggtctatcgacaactattcttccttggttgcctctagcgaagattacaaagtttgtgagaacaggctgagagaaggcgcgcttggcgctgtagtgaagcagatatttgctacaaagacgtgcattctttgcggttactcggcaaaagaccccgattttcagagcatttttcgaacgatccaagacggcttgggacgcctcgcgcggacccattacctgatatctccatacgtgaccgatgacgaggcggagcagctgagatcagagtttggtattgtggcgattcgaacagacgcgactcattttctcagaactaccaagtcacatatggaatcgaagtattgcttcgcaagcgacgactcctttgaggccatcgttgatgatctgattggatttcacgaaactcacatggatttcgtcgacaaggcggatctcaagttagaaccccatctgatattcgcaatttcatatcaagatggcgtaatacacgcgttgcaacgcttgatagatcgtcgaatgaccggcgatcactctgaccttcacagagtgcaaggtcagatatccaagtatgaagagaagatagagtcgtacaggaaggacagaaattattgggacgtcgcatacttcactggatatcgaaatggcctgatccgtctggtgctacttaactccaagatcgatgacgatccaccgtctattccagaatgttaccatccagggatcggcgagattgatctggaggaatacgataacctcgtccgcaagaatccagagattcacaagggcgccctgagagaggcccgccgccgcacgtcagacctgggcgaaggcatcgttgtccagcatctaccgtggggctgagcccgagatgaaacagggacacacgccatcctccaggaacagggacacacactctcttccgccgcttacgctggccgatccgccgcgctaatctccgtccatgcccaccctcgtcctcctcgccgggcctaacggggccgggaagaccaccttcatcaacagcttcctgcgcgagcgcgcggaggcgtttcagttcgtcaatccggacgaggtggcgcgcggcctgaccggcgtgggcgcggcgcgcgacctcgccgccggacggcgggtgcttgagcgtctggacgaccttgtcgcggcgcgcgcggacttcgtgctggagaccaccctggccacccgctctcacgcggtgcgcatccgcgattggaaggcggcgggctatcggttcgaactggtctatctgcgcctgcccagcgcggaccactccgtcgcccgcgtcgcacgacgcgtctccgaaggcggccacggcattccggaagcgacgctgcggcgtcgcttcgctatcagcctcggctatctggagagcgcctacaaaccgcttgccgacgactggaaggtctatgccagtggcggggatgcgctggaactgttagattgggggccgcgatgaacaagtcgatcttcgatcacgaaaccatcctcaaggccggcaagcgcgccgccgagatggccaagcacggcacccgcgaagagaaatccggcaagttcctgccgccgcccggctggaccggccatctggtcaccgccgacgatgccgcgccgccgcgccgtcgcaggaagggctgacctccgacgcgctacgcccggcaaggcgatcttcccccgcttgtcgggggaagtgtcagcgacgtggcgcgcagcgacacggctgacgatggggggagtttcctgttgaacttccctcaccgaccctggaccgcttcgcggtcgccgggccacctctcccgcaagcgggagagggtctgatagcgcaaagacgctgcataaaccctcgccgcatcaatcccttgcgcctctctcgccgcgacttgcgcgccgcagctgaaatccggggcatcctgcctgcggtcccgtcgcatgggagggctcgtctcggcctgcgaccttgcgagcggcgggagcggaggaaacgggaggccgcgggggttcaaacctcgcggcgccggcgtcggggatcgccccggcggtggaggatcgagggggatactcggtcgcaccggggacgggatcgccaggcccgcccgcccgtcgcaggcttatggggttaggcgataagaccgccaccatcccacgccccgagcttgcagacataatccttcgtgcggggcgtcagctttcgtcgaaacggtaaaccaactcacacagaccgggcgaaggcccagcgcccccgccctccgccgttcaaccgcgccgcgccttgatccgcgcccgcggcgcccgcacctgcgcgccccttgccggagagcccccatggccaagcccagacccgcccgtccgcgtccgcccgcgcccgaaccctggatcgactcgcgcaccggcctgccgatgacgcccgagcgcgaggaggaactgcggcgcgaactgtccgagcgctacgaccagcttgagatcttcctggcgcaaaagcgtgccgatgcggaggagcgcgcccgcatccgccggatgcaggcgcaggccgcgcccgactgatcaacccgcgcgcgggcgggaaagctgtgccacaaggcggaacggaccgacctcgccggcagcgccatgcacatcctgatcgcccatgaatcgccgatccccgtcaccgcctatggcggcaccgagcgggtgatctgggacctggcgcgcagccttgtggcgcgcggccaccgcgtgacctttctggttccggccggctccacctgccccttcgccgccgtgcagccgatccgccccggcgtaccctggcgcgagcaggtagggcgcgacatcgacatcgcccatttccagttcaagccggacgaggacctggacgtccccctcatcgtcaccgagcacggcaactgccagccgccctcgccctttccgctgaacaccgtctttgtctcggcagaccatgcgcggcgccatggcgccgaatgctttgtccacaacggcctggactggacgtcttacgcccctgtcgactggaaccggccgcgcgccggctaccattttctcggcaagggcgagtggcggctgaagaacctgcgcggcgccatccgcgtggccgagcgcgccggagagcggatcgaggtgctgggcggcgtgcgcttcaacgtccgccggggcctgcgcttcaccctttacccccgcgcgcgctttcacggcatggtcggcggccaacggaagttcgacgtgctgaacggctcgcgcggcctgatctttcccgtgcgctggaacgagccgttcggcatggcggtggtcgaaagcctgtatttcggctgtcccgtcttcgccacgccctacggcgccctgcccgagatcgtggaggaggaacacggcgtcctgtccgccgacgcccgggtcctggccgatgcggtgcgcgccaaccgcttcgacccccgcgcctgccacgcccgcgccgccgacgtcttcaacgccgaccggatgaccgagcgctatctcgcgctttacgaccgcgtcctctccggcgagaccctgaacccgcgcccgccccagctgatcgacctcgaccgcaacctgccgtgggtcaactgaggggattcacctcctccgcctcgccgccattgacgtcagagctgtggactatttcgcgtatcgcgcgtattcatgaagatgaacgcggggggcttcgtgatgcgtctctacgaattcattttcatcgacgcgcagggcggccggcccgccatggacctgtccgagtggccggacgatcagcacgccgcgcagtccgccttcagccagctggaccaacacgcctcatgcctcggcgtcgagatctatcaaggtcagcggctggtgggccggatcgagcggcctgacgatcgcaggcgcccgcccgcgaccgcctggcccgagtcgatcctgcctcagagctcctgattaaaggcgccgatctcgggataggtggccagacgcggcttgacctccttgcggaacaggtcgcgcatgtcgtcttccgagcgcatgctctcgaccaccaccaccagctccggcttgttggacgaggcgcgcaccagcacccatgagccgtcctccaggtgcacccgcacgccgttgacggtgatggcctccacgatcctgcggcccaggatggagtcgccccgctcggccatggcggaatattcggccacgatccgctccagcacctcgtacttcagctcgtcgtcgcagtgcgggctcatggtcagggaggtccaggcgtccggcagggccgccttcagctcgctgagcttcttgtccggattgcggtccagcatggccagcacggccgaggccgcgaccagcccgtcgtcgtagccgttgcccagcggcccggccatgaagaagtggcccgacttctcgaacccggccagggcgccgatctcggcggtcttgcgcttgatgtagctgtggcccgtcttccagtagacggtgttcgccccgttcgccttcagcacctcgtcggtcttgtacaggcccgtcgacttcacatcgacgacaaaggtcgagttggggtggatcctggacaggtcgcgggccagcatcaggccgatcttgtcggcgaagatctcctcgcccgtgtcgtccaccacgccgcagcggtcgccgtcgccgtcgaagccgagcgccaggtccgcccccgtctcccgcaccttttcggccatctgcatcagcatggcgtggtcttcggggttcggattgtacttcgggaaggtgaagtcgagctcggtgtccatttcgatcacctccacccccatgcggcgcagagcctcgggcgcgaacgcgccggcggtgccgttgccgcaggccgcgacgaccttgagcggccggctgaccttcaccttggcggcgacgtcggcgatgtagcgttcgcggaagtcctccacgcgcaccagcttgccgccttcgcgctcgacgccctgcccgttcagcacgatctccttcagccgcccgatctcgtccgggccaaaggtcagcggcgggttggctcccatcttgacccccgtccagccgttctcgttgtggctggcggtgaccatggcgacgcagggcgccttcagctcgaactggccgaaataggccatgggcgacagggcgagccccacgtccagcacctccatgccgccctgcatcaggccgatgatcagcgcctgcttgaccgacaggctgtagccgcggaagtcatggccggtgacgatgcggggctcgacgccgatctcatgcacataggtcgccagacccaggcccagcgcctggatgcccagcagattgatctctttttccaggatccaccgtgcgtcgtactcgcgaaagcccgtcggcttgaccagcgcctcggtctcgtaggcggccgtgttcggcttcagatcctggcggggcttcaacatggcggtccttggagacaagacgggaaaagggggcatcagggccagacgacggccagcacgaccagcagcaccgccgccaacgacaccagcggaaagaacagtcggtcggacataagcttggctatagagagcccccgatgaggcttcaacaacgcggaagctggacgatggatgcggagcccgaggacttcgcggcgaaaacttgaccgtccatccttgcgggcctaccccaaaccccccgttcgccgtcacggaaccgccatgtcccgcctgatccttcttcgccacggccaaagccagtggaacctcgagaaccgcttcaccggctgggtcgacgtagacctgacggccgagggcgaggcgcaggcgaagcgcggcggcgaactgatcgccgaagccggcttcaagccctccgtgatgttcacctccgttctgacaagggcccagcgcaccggccggatcgccctggaggcggcgaagctgtcggatacgccggtgatcgccgactggcggctgaacgagcgtcactacggcggcctgaccgggctgaacaaggccgagacggcgcagaagcatggcgaggatcaggtcaggatctggcgacgcagctatgacacgcctccgcccccgctggcgccgggcggcgagtacgacttcgcgtccgacccacgctacgccggccaggccattccggacaccgaaagcctgaagaccaccctggaccgggtccagccgtattgggacgcagagatcgcgccgcgcctcaaggctggagaggacgtgctgatcgcggcccacggcaactctttgcgcgccatcgtcaagctgctgttcgccgtgcccgacgaccagatcgtgggcgtggagattccgaccggaaatccgcttgagatcgagctggacgccgatctcaagcccaccgccgtgcgctacctcgatcagagccgggccgaagccctgccgcccctgcaatgagctggtccgacgacgaccgcgccttcatggcccgcgccatcgacctggcgaccgcccgcatgggcgagacctggcccaacccggcggtgggctgcgtcatcgtcaaggacggccgcgtcctggccgaagccgccaccgcccccggcggccgcccgcacgcggaggaacaggccgttcccgccgccggtgcagacgtccaaggcgccaccgcctatgtgacgctggagccctgcggcgcccgctcgtcgggccgcaagtcctgcgcccacttcctggccgaagccggcgtatcgcgcgtcgtcattgcctgcctggacccttcgccctttgcgtccggacgcgggaccgagcggctgcgcggacgcggcctgcaggtcgagaccggactgatgtgcgaagaaggcgagaccctgtgcgagggcttcctgcaccgtctcgagaccgggcgccccatggtgcggatcagccgtgacggccggggattcgacggccgcttcgccgcctcgccgaaagccgacctggtcaccgaactgaagcggctgggcgaggcgggctacacccggctgtggacctcagccggagagttggcggacgccttgcgcgaacaagggctgctgacggaatcttaaagcgaagccgctagcctcgtctcatggccgaggctctcgacaccacccagcgccgtcgcctgacccaggcggaagcggacctgatctgcgccaggcacgaccggctgttctccgcccgccctggcggcgcccgggcggtgttttcctggatggacctgacgggcctcagcctaaagggccgaaacctcgccgacgcggacttctcggccgcctgcctggtcggctgcgatttgtcgggcgccaagctcgacaacgccaacttctttggctcggacatgcaggacgcggtcctggccgacgccagccttcgccgcgccgacctgcgcggggcctgtctgcggggggccgacctgtcgggcgcagacctgttcgaggccgatctgcgcgaaggcaccatcgccgccgcggacgcgcgcctgggctttcgcgtcatcgaaccgcgccagcgccaggacaccgaggccatgggcgcgtgcctggccggcgccaacctgcagcgctccaagatggcgggcgtcatcgccgtcaaggccgacttctccggcgcggtcatgaaggactgcaagctggtgcgcgccaacctcaagcaggccagcttccgcggcgcggacctcgccggcgctgatctgtccggcgccgacctgtcgggggccgacctgcgcgacgccgtgctggtgggcgtgaaatcggccatgtggcgcaccgacggcgcggacatggaaggcgcgctcaccgacacccgctccgccgcccagcccctgacccgcatgccggccgccgagatgctgcgtgaccacgcccgctggtgcgagacgggcggcgccgagggccagccctcggtgttcgacggcgtcgacctgcggccgctgaagtcgatcgtgggcctgaacctcaccgccctgtcggccaagggcgcggtcttctacggcctggacatggagggggtgcagcttcagggcgcgcatctggagggcgccgacctgcgctcggcccgcctgcgacgcgccgatctgcgcggcgcccggctgaaggacgcccgattgaacggcgccgacctgcgcgaggcgcagctcggcccccttatgctcaccgccgaccgcctgctgcccgccgacctgtctggcgcgaacctgcggggcgcggacctttcgggcgccgacctgcgccgtgcggtcatggccggctgcgacctcgcccgcgccctgttccacggcgcccagacgcgtcaggcagacctcgccggcgcaaatctgacgggcgtgcgcggcctgaccgtcgatcaggccgcctagcctacgctcaggccagcgccttcagccgatcgaccagatcggtcttctcccagctgaagccgccgtcggcgtccggctcacggccgaagtggccataggcggtggtgcgggcgtagatcggcctgttcagccgcaggtgctcgcggatcgcgcgcggcgtggccccgccgatcatcgccggcagctcgcgctccagcaccgcctcgtcgatcttgcccgtgccgtgcaggtcgacgtgcaccgactgcggctgggccacgccgatggcgtagctcagctggatggtgcagcgatccgccaggcccgccgccaccacgttcttggccaggtagcgcgccgcgtaggccgccgagcgatccaccttggtcggatccttgccggaaaaggcgccgccgccgtgcggagccgcgccgccgtaggtgtccacgatgatcttgcggcccgtcaggccggtgtcgccgtccggcccgccgatttcgaagatgccggtcggattgatgtgccagacggtgttctcgtcggtgaacccctcgggcagcacctccaggatgtagggcttgaccacctcggccacctcgccggccttgcccgccgcatgctgggtcgacagcacgatggaggtggcgcgcaccggcttgccgttctcgtactggatcgtcacctggctcttggcgtccggctccaggatggtgccgccgttgtggcgcacctcggccagccgcttcaggatgttgtggctgtaggccagcgtcgccggcatcagctcgggcgtctcgttcgacgcatagccgaacatgatgccctggtcgcccgcgccctcgtccttttcgttggtcgagtcgacgccgacggcgatgtcggccgactgggcgtgcagatggcaggcgtaatccgccgtctcccagtgaaagccgtcctgctcatagccgatgtccttcaccgccgcccgcaccagcggctcaaggctgtcgatgatggcttgggtgaaggcttcgttctgctctttcgtattcccaggctgcgtcgcccgcacctcgccggccagcacgatgcgctgggtggtcaccagcgtttcgcacgccacgcgcgcctcggagtcctgcgcaaggaaggcgtcgaccaccgtgtccgagatgcgatccgccaccttgtcggggtgcccctccgacacgctctcggaagtgaagaaaaaggacgaacgagcggccaaggaaggctcctgtcagcgatcaggccgcaagacatataaagatatgcttatatcttcaagagagctttccaggatcgtcgccgacaccgctgcaccgggtgcttcaagccgcctatgtgctggagcgctctgggcgtgaacggtcgcccgacaaccgctgcgctaatgcgccgtctccagcctacggcggagaaccgactgatgattaatggaaaggtggtgccgcttgcgtgactcgaacacgcgaccccctcattacgaaatcgacggaagcgtagcggtcaaacccaggcgcggtatggctttcagcgccatctcagcactccacgagagcgtgcacccacagacctcccagactggcctgagggggtgatttaggtgttccctagtttgcgatcgttagcgtggggacgctccggaattcgacctgcgccatacctgcaccccggtctggcagtgcggtcggacggtctgttcctgtggccgtcgctgttcgatccagaagctcctacgcggtcgatgtcgggcgtttgcggaacgctaatacctcgtagcgatgctattcagcctcaactagaaataatcgtcttggggtgtatcgcggctcgcggggaacgcgtctcagggaacggtggaggggtgaatggaatacgaatacaaggtgatagatgtagcagatggagccatcagctcgctgctgctgagcgaggggcgaatcgaaactgatgtgctcgaggggtatctgaacgcgatggccgctgaaggttggcggatggtcttcatggccaaggtcatgcaacggcacctagtgatcagcgaccgcgaaaccctgatggtgacattcgaacgacgcgtgcccgaacaccaaagggaggcgcgtgctgctcgtgttctcgacgacgtgattcttgctgaagaccgagccaaggtcgtgggccgtaaggctgcagccggtacgatcggcttggccgtggggggcgcgctgttgggcgctgtgctgtcgaacggcgaggaagggtaaggcgatggatttccaggctcaggtggccgctcgtcgggcagaactggagaggcgagcgctgagcgatcagaaggtcgcagcagaacaggctcgggttcaacaggctgtcgaacaggcgcttcgcaaggacgctttggacaccatcgccgccgatctctcggatagtggtgtcgaggtagtccgtgaggggaccgccttagccatcgttgctcattcggctccagcccttgatttcgagggactgcggcgaactcagatcaggaagctactgacgcaagaagcccgaaaaatgtggacacccaaccagaactggcaggtgatcgccccaaccgccgcaggtctctgcctgcttccgttttcttggatggtcggcttgctcctggttggcgcgggaatggtacgccgactgatgcttgaagcgcgatatgaggccgaggtgcgtcggcgctacccaacgatatttcctgtcacttagggcgcgtctccgacaactctggcgaaagaagtagcggcctgaggactatccgcgcgggacttctcctgagtgaaacggatgatccgctcgcttccgcccgatcctcccaccataggcaacacgagtggttggcggacaaactcaatgacattcatcgcgtgttcagcccgagggtcaaatccttggccgctgacggctgaggcttcatcttctacgcattgtgcggacccgctttagggcccactgacgcccgggagtgtcctcgaactgatcgaccccaagcgcgcagaaactaacgcctcgcccgcgcccagacgtgatgccagcgtgcgggtaaagcgctgtctagctagctgaacggtgacctgcatagccgccgcagcttctcacttagtcaagcgactttccgctccagtgccggaaccgtgtccgccacgcgtttggcgacggccgcaagggtcgctttgtccagcttttggcggcctttaaaggtctcctgaacgaactgctccgctctctcaaggatttcggtctcggacatttgcctctcctcagattcgcgcccaaaggcggtcgatgaccagatttgtgaaatatcggtaccaatacttcggtttcaggccctttgcggccaaagcggcttgaaggtcttcgtcgacttccgcgacagcaaggagcgtcttcgctacgtcatcgtgtcggataacggtccccgtcggcaaagtggctttcaaaaagccgtgagcccgtttgagcgtcgctagccaagcggcttcgttagccaggagatatacgtcaaggccgacgttttcgagtttttgttcctcttcaagcgtcagcgccatcacgagatttccttgacggctttggtcgctacaatcgcgatccaaaacacacaggctgcaagagcgaaaagcgaaatcgcagcccaacaatcgttcatgaaaagcttggccagcaagcctgatagcgccgacccaagcgcaagcaggaagcaccacagcgcagattgcccccgcgaccggaaggccttcaccacatgcttcttctgggttggatcaactctttcgtagcctgaaacggtcgctcctaagaaaacgagaatcaaccccgctagcgtggccgccgcgccgacgatctcggtggtgatgctatagaagtttggcatggccgcccccggcttagattattgacgatctagcgaaccgcgccggatagcaaggcagctttgtcagcgatccattgcgaaaaaaacagcgccccacccgcaccccgacgtgatgccaggatgcgggtgaagcgctttggttcagaaggcgacctgcttggccgccccggcctcgacggccttcagcagcgtgtcgttggcaaggtgggcgtagcgctgggtactctggtagttggcgtggcccagcaccttgccgacggcgaagagatcgacaccgctgttgaccatgaaggacgccgccgagtgccgcaggtcgtgcagccgcagccccggcagcttggcttccttgatggcgttctgccagccgtgcttgatcgacacgaacggtaggtgggtgtcagggttcggcaccagccaagggcagtcgttgaagcgtggaagcgcctctatgatcgccacggcggccgtcgacagcgggacgtgacgcggcttgccggtcttgctggtcgggatgaaccaggaccgtcgctcgacgtcgacgttcttccagcggaggctggttgtgcttggccggtcaggtgcacttagctcttctcgataaccaccgcattaccgttggcggtcaccccgaacacgtagggcaagtacattgtcccgccacccgacgacgccgtctccggatcgagggttaggtagtcgaaatcaaccccgacgacggcgttgcacccgagctcgtaggcggcctccttaagctcagcgagagccttccgcctgatgctcgatagggagttcatgaggctttcgcctacattggttgcgctagtaaaaaatcccgacgttccgcgatcgatctgaactacatcatcacccgagatataacccgaatacttagtaatcgtataaccgtcgaagttgaaacctgacgtaattagcatgctggccagcgccttgcgcttctgttcggccgccctctccagggcttcgcgttcctcggcctcttcggcagcgctctttgtggcgtgatcttggaactgacgaaccgcgacatcaacgtctgcggggtcctcaattgatagcccgcccatcatgcttatcttgaaagggactgctcgtgatttagtgagccaagcgtcgaactgcccttggctaaggcgatatttgctcgcgatgtctttagttttcatttgggtccttacctgaaatagctttgcgcctctgggttcgacggatcgatgtccagtatcaatccggctatgcgcttcctgttgtgaggttcgtttcgacacctcagaaggagcacttggatatcatcgtagacagatataatcgattgcgcagcgggcgcactgtgcgcactcgaagtaaactttatccggcagtatgcacatacaacatactgcttctcttcgacgaggtcgttgcttccgcatttagtgcaatttacgattctcatcgaacgcttgcccgtggtcggtgcgagcccttcatagtcctagagctcgggctttggcggcgttgaactccgattgatcgatcaacccggcatctaggctcaggacccattgatgtgaggcgcgcgatctgattcaggctcctgaggagtctgattatgagtgacctgtactggctgacggacgagcagatggctcgactggagccctatttccccaagagccatggcaggccccgcgtggatgatcggcgggtgttgagcgggatcatcttcgtcaaccgtaacggcctgcgctggcgggatgcaccggcggcctacggcccgcacaagacgctctacaatcgctggaagcggtggagcgaagccggcgtgttcgttcggttgatggagggcctgtctggcgctcagaccgaacgtcgcaccgtcatgtgatcctccctcggtttggtggacacccatgctagcttttcggagctggagaggagtgtctgatgagtgttcaacgccggaactttccggattctttcaagcgcgaggccgttgaccgcgtcgccaacggcggcctgagcgtcggggcggtggcccgcgagcttgggctgcacgagacggtgcttcgtcgatggatgacgcagttcggggtgcaggcgacgggggcgtcgcggcgccccacaacgcaggcgtcgtccccgtcgccgtcggatctggcggcggaggtggcccggttgcggcgagagaacggtcagctgcggatggagcgggacatcctaaaaaaagccgcgctcatcttcggagcggcctcccgatgaagttcgggttcgtcgatgagcatcgtcaggtctggccggttcgcgtgatgtgcgcggtcctgggcttgtcggccagcggttactacgcctggcgcggtcgccccgagagccagcggtctgtcgccaatcgcgagctgaccgaggatatccggctgatccatgcggagagcagcggctgttacggctcgccgcgcgttcacgccaccctgcggcggcatgggcgtcgggtcggtcgatcccgcgtggagcggctgatgcgccgcgccggcctgcggggcttggcggccttgccgcgtcgcgcccggacgacgaacagccgccacggttatcccatcgcgcccaacaggctggcccggaacttcgaggcggcggcgcccaaccaggtctggctcgccgacctcacctacatcccgaccggcgaaggctggctctatctcgccgccatcctcgacctgcacacccgcaagatcgtgggctggtccatgcgccagaccctgcacaccgagatcgccctcgacgccctcaacatggccgtcgaacgtcagcgccccgcgcccggcctgatccatcattcggaccggggcatccaatacgcagccgaagcctatcgatcagccctggcccgatccggcatcaccccgtcgatgagccgaaagggcgactgctgggacaatgccccgatggagagcttcttccacaccctcaagaccgaacgcgttcatcaccgcctctacgccacccgagaccaggcgcggcgagacctgttcggatacatcgagggcttctacaatccccatcgcctgcactcagcactgggctatatcagccccgctgaggccgagcgcaaagcggcttaaccccgtccacttttacgggggaagatcaatgatcgacgcgacctatctgaaggcgcaccgcacagcttcgagcctgcgggtaaaaaagggggcctcgggcgactgatcggtcgcacgaaaggcggcatgaacaccaagcttcatgccgtgaccgatgcgaacgggcgtccgatcagcctgttcatgacggcgggccaggtcagcgattacaccggcgctgctgctctgctggacagcctgcccaaggcgcaatggctgctgggcgacaggggctatgacgcggactggttcagggacgccttgcaggccaggggcatcacgccctgcatcccgggccgcaaaacccgaaccgagcccattcgctacgacaagcgccgctacaaacggcgtaatcgcatagagatcatgttcggcaggctgaaggactggcggcgcgtcgccacccgctatgaccgatgcccgacggtcttcctctccgccatagccctcgccgccgtcgtgctcttctggctatgagtcctgagcctagagcccgccgcaggttttccagtactgacatcaagtcgtggttgggcagagaaccgggagaggaagctgccgccggggttttctgcatcaggtcggatagcccaatggaattggcggcaatccccatgcccaacagacctccagtgccgctgtgctccccagcagacgcgatgcccgaagccactgaagcttgcaaattggcgtttcccctggtgcccgacaatgcgtccgctcgctgaaccgtcttcagcaaatcccgcgtctgctcgtcatattcgatcccgacaattgttaccttggagagcgcgagcccgcgtgaactctgccactggtatccattctcgactgcttgtccgagagatgcagcgaagccgatggagtcctgctggatcttcgtgatccgattttctttgttgtgctcgtttgcatatatgctgaaagctgcagccagagagctgacgacttccgagaacagttgatttgcggcgtcattctcgcgatctgtgaagtcgaaatagtcttgcccctgcaggtaagaggccggaacaaactgcttggtgaagaggattgggtcaacaatccttaagctgtaggtaccccgcgtggtcgcgccaacttgtgcgttaagataggcatcgtcccagtatatctctgattgggtgccgaacttgttgtgaggaagctctttaagactgacgaacattgcgagctgctgaacgcctggccgtccgccgaacttgaatcgttcccaagactggctcacgagcgcagccgtcaccgtgctccccgcaaaaatcgactgagactccgggttctctgattgccagatgtacccgcccggctcgcttgcgaagccggttagttcaccgtcctgaaagagcagcagcccatatccttccggaacgactaggcgagagccattcgtgatgatggaccgcgagccatgaacgttggacccgcgcccggcgtttgtgccattccgcacagcagggaagagtgcggctgtgggtggcaggtttgcaggtacggtcaggaaatccttccactgatcggctaaagagccgccgacagctccgaatgctgctctaatcagtcccatcccaatccccctctaaactgaaggggttgtgacccgctccgtcggaatagggccgtcgcacagcgctccaagtgccgccggtccctgctaatacgggactatacacccatacaaggagaggcaagtacaacttgaagccctcctcgcccatggctgccccggaggccgcccctgcatgccagtggacggcacgagatgaggcttcgggcgtacgcaaggcaacctgctttgcggcacccgcctcgacggccttcagcagggtgtcattggtgaggtgggcgtagcgctgggtgctctgatagtcggcgtggcccagcaccttgccgacggcgaagaggtcgacaccgcgtgcacgagcgtctatcattgatggcagtctgctgtctcgatggctgggcccaatgggtccgcgcaatagaatgcggttgccgcttcgaacaagcaggcctccagggggtcagtttcggtggagttcggtccgagcgccgtgagcgacggcgtcgacacgaatgccactggctccgcatacccgcccatccggttacgtccattgacggtcccgcagagtcgctcatgctgggcaccgtacgtcttgacgttactgaagaccgccgacgaggggtcgaggaggagagcggccgcccgctcctccccaacgcggatcgcgtatgcttccgtgccgggaatttcatcgcacccgaccaagagcgtggaggctcccgttaatgccagcagactcaagacgcgcctactgaagctgctggtcagaaccatcctagcgacgcctgtcccagcggggcctggacggagggtcgttatcgccgccgggtgtagccacctctggtgtcgcttcttgcgagctcggtgctggttcggacatcgtggtcgtctccgccggcggaactggatcaacagctctcctcgcccctgaccgcagatgccgctcaatagcgaccatcaggaagaagaacatcacgacgaggaaagcccctaaaacctgcagggcgagcatgaggttcggaccgatctgggccctggtggcttcccgcccgtcgcgggtggcttgagcctctgcgcggacctgagcggtctgctgcgaccagagtcggaagaactcgccgtccgctcgaccgaaggcgacgcgtgggctgacgatgccttcggggtaggcggcgacgcaggtctcgactggaacgttgcgcgtgacctggcagccctgtggagcctcccaccagtagtcgcaggccgtgctgtaggaatcccacatctggcgacgttgattggttgtcgtgcaggctcgggccgtcttttcagccgccttgtactcggtcaactggacgacgaccgtcggatctcgcatcgccgccgtcaccgccgccaccgcctgctgctgatagacctcattgtcgatgaaggctgccgccttctcttcacctgccgcataggtgtctaggtcgtagccaagcgcttcgatcagcttctgctcgctgagggtctcgtcctctggctttttgtacgtctgagacgccacacgatagatcgcatagtacttcgagaacacgtcgcgtgcccactgcgcatgtcttgcgcgaacggccctcggcacctcatccgactggcgggattcggttcgggcgggcgcggcctttttcaactcttcagcgacttgcgcgcctgtcacctgaaccggctgttccttgacgtctgtcgagacgaagactcgccacgcggcgttgatgccaaacagaatcgccccgagcaggcacagggtggctaccgccaggatagccacgcgcaagctcgccagataggcgcgctcaatgcggtcgagatcgaccgactttagtctcttgattttcaaggcagtcccccaagctatgctgtagctaccatgacgcgtgaagaaagcaacttctcgtagggcgacctcatggcacgtcagatgacgggactgacaggggcaaccagccttggggctcgatacgagtcccggcgtaacttcattggccagaacttagacggtgcctggcagcggaccggctgagatggcctgcagattggagaacatgtggcacgggccacgcgcgcgggggtcgttggagcgagcaggaccgccagaaaaaaaaatagcgccccacccgcaccccgacgtgatgccaggatgcgggtgagacgcttggatcagaaggcgacctgcttcgccgccccggcctcgacagccttcagcagcgtgtcgttggcgaggtgagcatagcgctgggtgctctggtagttggcgtggcccagcaccttgccgaccgcgaacagatcgacaccgctgttgaccatgaaggaagctgctgagtggcgtaggtcgtgcagccgcagacccggcagcttcgccgccttgatcgccgtcccccaagcaccctttatcgagttatagggcaacttggtgtcggggtttggcaccagccacggacagccattgaagcgtggaagcgcctctatgatcgccagggcggccgtggagagcgggacgtggcgcggcctgccggtcttgctggtgggaatgaaccaggatcggcgctccacatcgacgttctcccacctggcgtccagcagctcgcgcagtcgcgccccggtcaggaggagcaggccgacgatgtgctgaagctgagtgttctgagacgccaccaccgccgccttcagccgcaccgcctcctcaggtgtcaggaagcgttcccgcgcgttctggatcggcgcacgtgggatgttgcgggcggggttcttctcggtgccgggtatgtcccagctcgcgcccagtacgaaagaccggccgaggatcacgcggatcttctccaccgacgccggggctaagcccttcgcccgcttctcctccagccactgcgccacagcccggctgttcatgtccgtcaggcgcgtcttcccccagcgaggcaggatgtgcacccggatgacggactccacgtcctcgaatgacttacggcccttgaacgactcgaggtgcttggccgccaactcgctgtaaaggggggtggacttcgccagcgccttcttcgcgccggggtcgccgcccatgacgacttccgagcgaagctgttgagccttcttcttggccgccgcgaacgtcacgtcttgaaagccgccgatcttgtactgcttctggccaccggcctgatcgacgtagcgtaggtagtaggtctttccgccggtgcagcggcactccagcacgaagccggtggtggtggtgcagtaccagtcggtcttcttcttgccgacttcgcaaccggcgttggcgacgaaggcctgtgtcaggttcgccttgggcatgggtggtctccttgcatgtttgatgatcggcgggcgagcgccgttaggccgccccggagggcggtcgattggggtggggtggcctggagcgggtcaggcccgcgttgccccagaggcggccgctggggccacgggtctggggcggggatggccgggccttggggagcccgaggcgggcctcagcgggccgcgtttggcgtcgctggcgtgaaggctgaggccatcgaaaccggcaaaacaggcaacctgtttcacctgtttcgacatgcccagggggagcggcaacgcaactcccccgcactcagacgccttctagtcggcgatgacctgccaagtatttcgctgagagttcgggcctgactcgatacgcatcccgttggcccaacgactccggttattcttgagataccaaccgagcttcttcgcgttgcaggtggaaccgtccatcaccccgatctcatcaagcgaatcggcaaatcgagggtctctggaggcataggggaccacctcacgcaccatcatgggatcatcgttaaacaggcgaaaccagtgcttcaagaattcgccaagctcgtcttgctcggtgtcgttctgaacctgctggattagactggtcgcgggatccggctcgcctaggctcaggacccattgatgtgaggcgctggatctgattcaggctcccgaggagtctggatatgagtgacctatattggctgacggacgagcagatggagcggctccggccgcactttcccaagagccacggcaggcccagggttgacgatcgccgggtgttgagcgggatcatcttcgtcaaccgcaacgggcttcgctggcgtgacgcgccagcggcttatggcccgcacaagaccctctacaatcgctggaagcggtggagcgaagctggcgtgttcgttcggatgatggagggcctgtctggcgctcagaccgaacgtcgcaccgtcatgatcgacgcgacctatctgaaggcgcaccgcacggcttcgagcctgcgggtaaaaaagggggcctcgggcgactgatcggtcgcacgaaaggcggcatgaacaccaagcttcatgccgtgaccgatgcgaatgggcgtccgatcagcctgttcgtgacggcgggccaggtcagcgattacaccggcgctgcagccctgctggacagcctgcccaaggcgcaatggctgttgggcgacaggggctatgacgcggactggttcagggacgccttgcaggccaaggggatcacgccctgcatcccaggccgcaaaacccgcactgagcccatccggtatgacaagcgtcgctacaagcgccgaaaccgcatcgagatcatgttcggtcgtctgaaagactggcggcgcgtcgccacccgctacgaccgatgcccgaacgtcttcctgtccgccatagccctcgccgctaccgtgctcttctggctatgagtcctgagcctagccagatgagcgagtgacggcaggctagagaccattcttcgaagcttccaattggcgggacatcggagaccggtttgcccgccagccgatgcgcctcgatgatggtgagcgcagcccgaacaatttctgaccgcttcgcgcgcacgtgggccacgggattgaacttgtacgactgcagtgtgggtgctcccccctttggggcgagtcgtatcgacaccacacgacgacgcatgtcttgggtcggttccacgttgttgcctgtgcccaagaaaagcacgttggtgcgcgcggtggcggtgcggctcctgctgaggacacgctcggtgatggtggaagttgtcagcgctttgttcatggggccgagcgacttccagcccgtcttcacctgcatgtcatcgaacaagaccacggcgggcttctcgagcagcatcgccaacagcagcttggtcgcttcctcaggagtcgtcggatagctcgcgttgtagggttcgcctgcactggccgccaacgcgatcagtgtacccatccggtgagcaccgcgacgagctgacggctagttcggctgtagaatgccgtccgtctcgatcagtctgagggcctggcggagggttttggaccggtaaaggcagtgccagaccccggtgtggcgatgccactggatgttgaagctgtccggggcgagccagtcgagacggacgaacggcgcgtcgaactcgtaaccgaggttgtcagcgaagccagagcggtagcgttggatgagccgatagcgggctccgtgccacttgccctggatattgacgggatagttgaactcagtcggacgtacgaccggcaagaaccgcggcttcaagatatcctcgatgaaccgctcgcaggtggacgtgatgtgcaccttctcagtgggtgacggcccgctcacggaagcgccacgacggatgagctggtccagttccacggcaacaactcgtcgaggcggttgctgggaaggtcattgatgcgcgccaggacgtcggccagccaggcctgaggatcgacgtcgttcatcttcgcagtggcgatcaggctgtacatggtcgccgcccgctggccgccacggtctgagccgcagaacagccaggatttgcgcccgagcgcgatgcctcgcagagcacgttcggcggcgttgttgctcaggcagacgcggccgtcctccaggaagagtgtgaaggacggccagcgcttctgcaggtagttgatcgccttgacgataccgtggctgccggtcagcggctcgcgtgccgcggccagccattccttgagttcggcgacgatgggcgcgctctgcgtctggcggacggcaagacgttcggctgggctggcgccgttgatggtccgctcgatcgcgaacagggcgtcgatcaggcgcacggcttccagcgccttgggatacacagctctgggcttctcgccgcgcgccttcttgcgctgggcggcctcaaggtcagccaactcgaagaacttgcgccggccgtgcgcccagcacgctgcttccaggatcggaccgggcggccggccctccttgtagagttcgttgtagccgccataggcgtcggcctgcagaacaccgcaccaggtctgcagatgggtctgaggatgcatccctcgccgatcccgggagtagtggaagatcgccgcgggcggcgaagtcgcgccgaacggtgcgtcatcgcgcacataggtccagagccgggcgatgtcggtcttgcccttggccagaaccgggacggtcgtgtcgtcgccatgcagtcgctcggcggccagcacatgggcttcaatgcgctggtacagcggcgccagcaccgaagcgacgccgccaacctggtccgcgagcgtcgacaggctcagtggcacgccttctctggcatagcgctcggcctgccggttcagcggctgatgctggccgaacttctcgaacatgatcatcgccagcaggcttggccccgcccagccgcgtggcagaacgtggaacggcgccggcgcctgagcgatggtctcgcagtcccggcacgagaacttctcacgcaccgtctggatcaccttccactggcgcggaatcacctccagcgtctcggtgatgtcctcgcccagtttgctcagccgctcaccgccgcagcaggcgcaggccgtcggcgtttccagcaccacccgttcgcgtggcaggtgttcggggaagggctggcgagacggcttcttacgggcgaacgccctgaccgtcgtggtcgcccgggccgccttctcggcggccagctcatcttcggtggccgaggcctccagctcttcgagctgcagctccatctgatccagcaaccggctggaacgctccgaggagacgccgaacgtctcgcgtttcagcttggcgatcatcagcttcaggtgcgcgatcagcgcctggtcttcagagcgctctgccttggcgacggcgacctcggcacgggcctcatcgcgctcgttgcgcatgctggccagcgccgccttcagcgcttcgaactcctctgcactgggcgcggtcgcggcttccatgacccgaattgaatcacagatcacgccgcttgtggcgccctaaaatgcagccgggcccaactattttcggctcagccggcgctgctcggccgccagctgtgctggggattacgccagtcgattccttccagaaggtagcccagctgggcgcttgtcagcgcgacagctccaccctcagccttcggccagatgaaccgtccccgctccaaccgcttggcgtagagcgacatgccgatcccgtcatgccagatgattttcagcagggagccgccgcgaccgcggaacacatagaggtcgccgccgtggggatcgcgcttgaggtgctcctgcaccagcagcgccagcccctgcatccccttcctcatgtccgtgtggccagtggagatccagactcgaccgcctgggggtatcatcgcagcgcccgcagcaccgcgcccacaagcaccggcgaggcggcaccggtgatgctcactcgtgccgccgccagttcaacccggatcaccggatcaccgctcggcccggatctggacccagcatccgccatgacggcttcgacgaaagccgggtcgccggtctgcgtacgcgcattacgacgccaggtgtagatcaggctcgaagagacctcgtgacggcgggcgacctcactgacgcaggcccccggcgaaaacgcttcttccaggatggccagcctctcctcgtcgcgccaccggcggcggcgttccggtcccgttagcagggtaatctggctcatctgcgcttaagctcgctcgaacgcccggtcttaagaccaggcttaagcgcagagcatcgccggagaattcagcgaaacaaggcggcccccaccggagggttaccgatcagtgccgccagaaagcttttcccgccaccggaacgcggcgcgttgatgttgatggcaggggcgagcggaagagccgctcgtactgcggcggtgaggatggcagcgatagcggccgcttggtctgcatccgacgcaaactgaaactcgcgcaagagccacttgagatagtcgagttgatgttcggcgtcctctcgcgtcggacttcccagatcgtactcggcctcgtcgaatgccgcataggtgccggttccttcatggtatccggccgtggaaaccaggagcccgtctgccccatagaacggctgcctggacaagccggtgagcgtgcgcaggtggtgccgatcctgacagtaccgaaggctttgaatgatgcttgcaggaggatcgcagcgctcccactggctccccttggcttttcgatagtagtcgatcttcgatgcaaggaatgcgctcagggtctgatcgttgacgagctccgtcgaaattgcctcttcggttgactttatgatgcggactatcggaccacgtgcgttgtagtagctgccgtccgccgccagcacccgctctgatgcagccgcagcacggtaggtttcacccgtctgcatgaagatgacagccttggcgcgcgcgacatccggggtgatgccgaggtggtctatcaggctttcagcttcgcgtttttctgaatggttgtgggtgcaacggaactgcccgatcggtctgccaaagcacggctccagatagccggcctcagacgacgattctggcggatgctccgatgcccaggggcacgtcactctgtggaacccatcgcccgcatcttcgcgatagagaccatttgccttgagggcggtcacaaccgggtttgagctgggtgcaggagtgtagacgtcatcggcaaagtccgtctccgctggcatgtcgaacagcgacgcaccgcgcgggcctggcgaaacaggcgaaaggggtgctgccagggaacgggcgggaacaggcggcctctcagtcgaggaagcttcatctgtccccggctgaccttctggtgctgcgtcctgaactaggaggtctaccgtggggcgcggcttcagaggcgggactttgatctttctcggggcaactgtgccccccctccacggctggccagacaagtcattttttaggtctgcagtcatggtgttggtcctctggtgttttgacgtggttcgactcgcgccgggattggcgtggcctcgttgcgatttcgggacagccgctgcagtcggtgtcgcgtcctcactggggacgttgtgaccccgccaaccggccgttggaaagcccttcggcgggactaccggttgcggtttttgagaggtcttcagttacgttcgcccgctggacctttccaatgtggaatagttccatgcggtggcctggaggtgtacctcggcggtcactgagccggttcaggaggcgagattttgagcgacagcgcggcagattttcagtttggcagcctgcgtgtggcgtggctggaggccttcgtgctgtccgtccgctacgggaagcagacggcggcggcggcggcgatgggggtcgcacaaggcacgatctctaagcacatcgagaaccttgaacgctggtatgggggcggcccgcgcctaatccttttggagttcaacaagtcgcctgcgacgctgaccgacgcaggaaaggtgttctttccggtcgctgaacgggcgttgcaggctctgcatgagttgcggaagcgtcccaaggttaccgagacgcctccacgacagcgcgttgatcccaagaccatcaaggtcccgaagatctagccgataacagggatcgaccacagcgacggtgcaccgatctccgtcgtcgtctcacctccgccaacgccagggctatgaccaccgctcccccgatgaaggcgagcggctgggcgacggcgaggctcgacaggatcagggtgccgaggaacaccagtgtttcccgtggtcgcgtgatgaaggtgacgagcaccgtcagcagcagcaccaccgcaagcacgatcgccaccgccctgaagaccgccagcgctacgcacaggatgagcaggaggaggagcctgctcatcaccggccaccctcctcggtccagaagtgcgtcaaacatagaccgtgaatgcccaactcagtagccgggccgttttcgacgaagatgatgatgttccgcttgacgtaggtgatttcgaaccagagcccgtggtcctccagctggtcgtagcttggctcctcggcatggtcgccggtgatggcgaagtcgagggcggcgttgatgacagccgacgtgtcgccgccctggaccacgatgatccgtgtgtcctcgctcaggtgtgacggatgctcggcataggcctgccatccgcgctgggcgatgagggttcgaaggtcgtcgtctaggtcggggtcgctgatcgcgctggcgacctcagcaagggtgttcaggcagagcatcggagggtgtccttcaggcatgaaaaaaccctcgcgacggggtgtcggagggcgtggtcggatgggtctggttggatgttcagtcggcgtcggaggccggcgggcggtcggcgaagccaaggcagttgaagcgcagggtgtggttggtgtcgggatggtcggccacgaacaccagcatcccgaagtcgtcggtgaggacgtaggccagctcgaaccatgagccgtggtcgttgaaccactcccagccgggctgctcggcctggtcccagcagatcgaaaagccgactgcgtcgtggatggtctcgggcggatcgcttggttgcacgacgacgatctggaggatttccccaaggggtcgacgtcgatcggtgtccacctgccacacccgaaggccgatcagggcgcgtatgtcggcgtccaaggtcgggtcggccagggcggcggtgaccgcgtcgcggtcggtcagtgagatcaaggagaattccttcctgggtaaagaaaaacccccgcagcggaaggccacgggggtcggtgttggtgagatttgacgcgcccttagcggaacgcagtgaacgggctcaaaggcgatgaagggtcacgacttcccgtccttcggaacgaagggaggcggaggcagccttcaggccaattgacccgctggtttaccttgccgccgggacactcggtgacagggccgaagcggcctgggaaagccgctccctcagccgtttggatcgcgacatgccggaaaggggcatggtcccgttgtgcgtgacgttgaagtagtagccgtcctgcacagagccatcacctgaacgcccccggacggaaccatggtggcgacgatctgatggctgtcgaacaggaacttgatcgtcgcctgataccccctgttggggtattcgacgcgcacgatcgggctgttgccgaactccacattcatggcgtccaccaggatctggtcggcctgagtttctgtgatcagaaacacgggttcgctttggctgacataggaaccgggcgtccttgccggtgcggatgcgcagccgcagatggccaaggcaccggcagcaagcgccgcataaacaagcgtcctcattgggcgctctgctggatagcctgcgtacgctggcgcatgaactcagccttgcggcgcagggcttcagcgcattcgttcacaacggtgtcggtgtcccattcttcctcaataatcttattctgtatctgccccatgagggcgacgggcggtgctgaactggtcgcggcgaccgtggccatgtgattgcagaactcggcgatttcctccgcctgcgttggagctttagtagtctcggccgaaccgcgaccacaggaagccaaaagggcaagtgatgaggcggcgacgatggcgtggatattcttcatgatgatgttgtctctgttttgatcggcattctgggccagaggcccgatgggtagtgctgcgtcggttagtctccagggttgtggcgcgggtgaatcgcgttcgctgaatatggaaacatttcatatccaaaagggaaaaatcgcatacgcgtattttccatataggtgggttgccggtttagactcggcggctcattggatgcccaagacgatcttcggcggcgaacatcgacacctcgtcgcggtgctcgttgaagcgcgtcaggcgtcggggctcacgcaggccgagttggccgcgcgggtggggaaggatcagtccttcgtatccatcatcgaacgcggtcagcgccgagtggacgtgctggagttcgtggcattggctagagctatggaagccgatcccgcccgactattcgagcgggtggcagacaggctatcgaaggcgttgagaatataggctccgggctctatatgccgtcctgtaggccattcatataagatggcgcgacttgcgctcgctgacggcaacgagcgccgtctggacgtgatcgagttctgtcagattgctgaggtgctggggcacaatccggccgaactgctagctgatttcgttgaccttaggggacgaagcgcgcgctgactgggttgcgccaagaccggtcattgggctccagtcgaactcgggacgtctcgttcgggtgtagacgctccttactagggtgcttccgtcgctcccaaggctgctttggcttgccgaaccctccacgcctgagacgcctcgccaagctataccttttgagacaggcatcgcccgtgagggctgatcagcatgttcgtttaacgaggataggtgggaacgttgcgccgatccgtgtgtgccttcaccgccgaagcggatccggcccaaccttagtccactcagcgcacccgcaagcgggcgaaccgtatgaataaaaggaagtcatcgccaaacgagttgacgcattcggcgcaacgatcccgcaaggagcttagccccaggcataaactggccgcaactctttccggcgcagttggtgttccacagtcaccccggtccagtccgcgaaaccgagatgagcttccagttccttcagaaggtcgaagccaatctgatcgggttggcgtgttaccttctggaagaacgactgtttgtcgatcagggcgatgtcgggcgacgccaagtaatccacggccatcagatactcttcggtatcacgccgcagcacgacgccctcggatagcacacgtttccgcaccctctgcaccagcacgtccatctgtgactggaacgttgctagatctttccgcatgcagaatgccagggagatgaaggcaaaataggtcaccctcggaacaaccagcatccgatcaagagcatcccgaacgaccgccgaggcgaggaaatcagagcctacgaaatgcgcgccgcagatcaggaggttgaacagttccacgtcgtcttcgtggccgaacttctcaccttgggcgacgatgcggtatcgaaccagtgccgtgatgtgatccgacaaaagatgttcaaccaaatcccgctgctctgggctgagcgcatcgcctgccttgtttaggatgagcgccaactggcagagggaatatgtagtccgcacccgaagatcgatggcgcagatgtagagcgcagtctccaaggcagacaccgctacgtctccaagagcctctttcgctcgcagatgacgtgatggtgtggacgacctccgcctgacgggctgttctgggtgtgtcgtcatcagggacgtcatgtgtggacgacctccaagacgcaagagtggaaacgacgttggcgctcggtcgagtgcagtcatgtgttcggcctgttgatgcagctgtttgcgctgctggccctgatgaagtccgcggaccggctccctaatcacgtcaacgcgctcgaggcgctctgaccccctgggtttcaccgatccccggcggcggccggttcgtcatcacgtctcaccactccttcgtctacggcgccggtcctgggtgaagaccggcccgatctctatgccgctgtgggcttgtagtcctcctgtcgcgccatcagggtccaggcgatgcgagccgtcttattggccaaggccacggcggcgaccttcggcttcttgcgttcgaggagattgccgacccagccctcgcgtcctcgctgccgggccattcgcaggaccgccgtggccccgacgaccaggagacgtcgaaggtagctgtcacccatcttgctgatgccgccctggcgttccttgccgccactgctattggcccgcggcgtgagtcccagccaggctgcaaactgccgaccggaacggaagagactcggatctggcgcgctggccgccatggcgctggcagtgatcggcccgatgcctgggatggtcgccagtcgccggctcgtctcatcctgccgatgccaatcgagaatccgacgctccatacggctgatctctgcgccaaggtgttcgagctgttctgccagcccgccaagcgcggcatgcgccagatccggcagggcctgaccctcttcacgcagactcttcagcgctgcccgcaccccagctggaccttgaggcgcgacgatgccgaactccccgaggtggccccgcagtgcgttgatcagcatcgttcgctgacgaaccaggagatcccgggtcttgtgcagcatcaacaccgcctgctgggccttcgacttcacagccacgaaccgcatggtcggccgggtgacagcctcggcaatcgcttcagcgtcggcggcgtcggtcttgccgcgcttcacataggccttcacgtacgccggcggcatgagccgaacatcgtggccgatcgccatcagttcacgcgcccagtggtgggctgaggcgcacgcctcgatcccgatcaggcacggcccaatcgactggaagaaggccagcacctggccgcgccgcagttgccgtctcacgacgaccgtgccgtctgtggctacaccgtgaacctggaaaacagtcttcgccagatcgagcccgacgacagcgatggtctgcatgataccgctcctagacgtgacgtccctgatgacgacacacccagaacagcccgtcaggcggaggtcgtccacaccatcacgtcacagatcctgatggtcgccgatctgtttcaaagcacgcctgacaacctttttgagccgcgacatgagccacccgctcaggttcgcgaactggacatcgtatcgcgcaacagtgaggcggatcgagcttagttgtgccttgagttgtttgaggtgccggttcagctcggacagttccgactctggcttcattgcataaagtgaagctgaaatgtccctaactcgcccagaaatctcgtcccttgctagtgttagcgccgagatgaatggtcgggcgtgggtctcgaccttcttttcgttgacgtagagcttgtaacgttgaagatggaaccgaacacactcctcaacttgatcaagaatgaccgcatcgccagcgaagagaaaatagtcgtccacatagcgtcgaatatcatactcaagaccagctctcaggccgtttttagataggtcgctctcgatgcactcatccacatcctgtaatatgatttcggcaaatatccgcgagaactctggaccgactacaatcccattcgtctcgttgtagttgcattgctgcatgagcttgtcgaagcgggactcaaagctgtaagtttccctctgctccttcgcgaatcccttgctttttaccgcccatgttactgaatgggtataaatattataaaagcatttcgagacatctacttgcctcataagtgggtagcgcgactccaatctaatatactcgcgggatgcaatgaattttcctagcaagttatacttcccatatgcgaagtatgacgacatgtgggacatgtcggcttcgtctgcttgggctaagagctgcggaatgccagatttcgcccgctcctcatcttcgatcacttcccgagcaaatggtgatgccagagctactggccttctcagggcaaatcgcccgcgcccgcagtggctgagcatgccactgccatgcagctcgtaaaactcagcgatggcgcgctgagctagagggtgaaccacactgagggtcgttttgcgcttgggatccttcgatatctggtagttgtaggggatggagtagctcgggatacctcctaccagcgacgccagcgccttcgccaagtcacccaccggctctgaagccacgctcgcgtgaaagcgatcattcgagaagatcaccggaacttcatacggcagcgtgtccgtgagcaagctccggtaggcgaatgatttgttgagacgatcagccattgcgccaagccgctttcacctcggaaagcctttcgtaagtcatgcggaccattcttcgagactcgaagccgaggcggaatgagatgcgccgcaacgcaccggcatgcgcaccgctatgtcccctgactacggcgctgaactcgctgtgcgggcttttgaggagcacatgggtgaaatcgtccagctttgagagggaagctggaacgatagggttgaagatggacccagcgtaaatcccgcaccgacggtagttgtagtacacgcccgaccgaacccgctttcccctgacaaatccaagagcaccctgacggtcgatctggtagttcgaggacagaagtttaagcctatccgtcaatagcgccgcgtcggggcgcttcacgaacgcttttagacttagtatcaccctcgacttgagacgcctgattttagcatcactgatcgtgacgcttatggcgcgaggtagtatgcccccggtccccgcctcggtcgaaatcctatagccgagatactcgaatgacttcgtgacaagcttctctttccgcgtgaaatcgacgatgtcgcactttttgcgattgaactgcatgccatccggcaagagggcctctagcgcagcggctgtgcccctcacattgacgtaggcgaacacaacgatgtcgtctgagtagcggaagtatcgatataccccgggtagcgcgcgaacctgctgatcaaacttctccattgcgagttcagccaggatagaagtgagtccgatcccacgcggcaaaccgcgaaccccacgcgggcaatgcgcgtcgaagaaggcgcccagatagtgcctgaccgacttcggaagtgaggtgtcgtagatgagccgatcgcgcagagcatcagcgtctatcgattcatagaatgaggttacgtccctccggatcacatagtagggggtagcgtccatcatcgtctcgatcacgcctgagacgacccgatcccggttggctggcacaacccgaaaacgtcttgcgagatagttcgccagagatcgtaggactaggttcgttgggtagtcgcgatatgaaacgcaacgcttccgtctgactgttccatgaaggaactggctcagtagcacggtcctagcgacagccgctgcgctgattacctcgattatcgcaggcccgttcccagccagatcctgaccgaaccgttgcgcgtcacctgaacgcaccacccgtgtgattgagcggacggaaaagactgactgaaagcccaagcaacctcccccaagtccccagagaccaaccctaggatgagaaatccagaggcacaacaggttgcgaggcagttggtcaggaaccctcgccacccaaagatatttccgcgccaaagttcagcgggcgcggtcataagccacatcagcaatcgcgccgtgagggcgacaccaccgccgctttgagtcaacaccgacccaacacgctccccaccgcatacccacgcaactcccaagcggaagcgctttccggcttatcccgaccgggcgtcaaagctagtggtgctctggaaaggtggtgccgcttgcgtgactcgaacacgcgaccccctcattacgaatgaggtgctctaccggctgagctaaagcggcccggtgcggcgggtcgggacccgcgcgagaggggctctttatacgtgcgggagcggcttgccaagcgccgcctgcagggcggcgagcagggccgtttcttccgggcggtcggcgacggcgcattgcagccggccggcgagcgggcgggcggccgccgcggagatggcgacggcgagcaaccccgccggcttcccttcgataagcgggcgcagggcgaccgccgcgcggggcgaatgaatcagcaccgcgtcgcacgcaggcggcggctccaacttcgtctccaccgtgcggtacacaggcaagcggcggatcgggatcgagccgccggccgcagccccaagatcgccggccggctgctcggcgccgggaaccagaaccgcgccctgcggcgcagccgcggcgatcagccggccgagcgcctgcacgtcgccggaggccgagcgcacctccgtgaatccgagctcccgcgccgcatccgccgtggcgtcgcccacgcagaaggtcgggaggtcgcggcggtcgctgagttcggcgaaggccgagacgccgttgatgctggtgaaggcgagcgcggcgacgccgtcgagatcgatcgggacgccgttgatccgctggaccttcagcaccggcgcgacgatcggctggaagccgagacgcctgaggcgatgcgccgttcggccggcgcccggctcggcgcgggtgacccagacgcggggcgcgcccgggctcatccgtccagggcggcgggatcgacctcttggtcgccggccatggccttgacctcggcgccgagttgttcgcccaaaaggcgggcggcctgttccgcatcctcggccgaagcgtcgaacagctcgtctgagcgccgccagcgggccgagccgtccgggctcagcatctcgacggtcagccgcatgtgaccctcggccagggttccgtgcgcgccgatcgcggtgcggcacgagccctccagcgtgcgcatggcgccgcgttcggccgcgaccgtcagggccgtgggggcgtggttcagcgcggcagcccaggcgctgtctctgtcctcggcgcgggtctgcagcgccagcgccccctgccccggcgccggcagaaaacggttcagcgacagcggctcgcggatcacggcggagaagcccagccggttcaggccggagcaggccagaaagatggcgtcgaagtcgccctcggcctcgcggcgcaggcgggtgtcgacgttgccgcgcagcatctcgatcttcagatcaggccgcagcgccagggcctgcgcctgacgccggaggctggcggtgccgatgcgggcgccggccggcagatcgtcgaaggtctcgaagcgggtgctgacaaaggcgtcgcgggcgtcttcgcgttcgggcacggcggcgatgcacaggccgtgcggctggtcggcgggcacgtccttcatggaatgcaccgccaggtcgacgcggccgtccagcaacgcctcctcgatctccttggtgaacagcgccttgccgccgatctccagaaggcgccgatcctgcacccggtcgccggtggtcgtgatctcgaccagcggcacggccgtttcgacctcgtcgcccggcacgccgagcgcccgagcgatggcgcgctgcatcatgccggactgggccagcgccagtcgggaccgccgggtgccgatgcgaaggggaaaggtcatggatacgttgcgcgcgagcaggcgggccgctacctcgaccccatggagttccatgcggactatagcagcggcgcacaggcggcaacgggacgcggcgtccgccccctgacggtgctggggctggagacgagctgcgacgagaccgccgcctccgtcgtgcgcctgacgcccagcgaccgggggggccgggccgaggtgctgtcctcggtggtccacagccagatcgacgaccatgcggcctatggcggcgtggtgcccgagatcgcagcgcgcagccatgtggagatgatcgccggcgtcacgcggcgcgccatggatcaggcgggcgtgggctatgaggcgctggacggcgtggccgcgacggcgggtccggggctggtcggcggggtcatggtggggctggggttcggcaaggcggtcagcctggcgcgcggactgccgctgatcgcggtgaaccacctggagggtcatgcggtgtcggcgcggctgggcgccgagatcgcctatcccttcctgctgctgctggtctcgggcgggcactgccagcttctggaggtgcgcgggatcggcgaggtctcgcggcttggcgccaccatcgacgatgcggcgggcgaggcgttcgacaagatcgccaaggcgctggggctcggctatccgggcggaccggcgctggagcggctggcgacgtcgggcgacccggcgcgctacgagctgccgcgcgccctgctgggccgcaaggattgcgacttctccttctccggcctgaagaccgccgccttccgcatcgcccagacctgcgagacggagagggacaaggccgatctggccgccgccgtgcaggccgccatcgcccgccagttggccgagcggtccgagagggcgatgcaggcctatgccgaacggttcgaccatcgcctctttgtcgtggcgggcggcgtcgcggccaacaggaccatccgcgcgacgctggaaggcgtggcggcccgaaacggcttcgacttcctggcgccgcccatggcctattgcaccgacaacgccgccatgatcgcgctggccggggccgagcggctggcgctggggctgacctcggacatcgacgcgccggcgcggccgcgctggccgctggacgaggcgcgcgccctgtccgatccttcgcacaaggccggccgcaagggacccaaggcatgagcgggcgagccccaggagacggcatgagctttcgcaagatcggggtgatcggcgcgggcgcctggggcacggccctggcgcaggtctgcgtgcgcgcggggctggacaccctgctgcaggcgcgcgagccggccctggtcgaggcgatgcgcgagacgcggctgaacgagccctatctgcccggcgtgactctggcgccccagatgcgtttcaccgccgacatggcggacctgtccggttgcgacctgatcctggccgtgccgccggcccagcacatgcgcgccaccctgacccgtttcgcggcctcgcatcgcgcgggcgtgcccgtggtgctgtgctccaagggggtggagcgcggctcgctgaaactgatgaccgaagtgctggccgagaccctgccggacgcgccggccgccgtgctgtctggccccagcttcgcaggcgaggtgtcgcgcggcctgcccaccgccgtgacgctggcctgcggcgatccggagctgggagaagcgctgctgaacaccctgtcggcgcccggcttccggccctatctggcgaccgacatcgtcggcgccgaggcgggcggggccctgaagaacgtcctggccatcgcctgcggcgtggtggagggccgtcagctgggccgcagcgcccacgccgccctgatcacgcgcggcttcgcggagatgacccgcctgtgcgtggcgctgggcggcgaggcggagacggtgaacggcctgtgcggcctgggcgacctggtgctgacgtgctccagcccgcaatcgcgcaacatgagcctggggctggcgctgggacagggccagacggtgcagcaggcgctggccggcaagcgcacggtggccgaaggtttcgaaagcgcgccggcggtgcgcgagctcgcggcgcggctggacatcgacatgcccatcgccacgaccaccgccgcgcttctggccggagagaccacggtggacgccgccatcgaggccctgctgtcccgccccctcaaggccgagcgcgcgtgagcgaggacgcgccggccgaacgtgcgcgggtttggaagacgccgcccggcgtcgccctgtgcgcggaaagcgacatcgccgatcccggctcgcgcggctttgtgctgcagatcggcgaggcctacttccacggcttcgtggtccgcaaggacggagaagtagccggctggatcgatcgctgccctcacgccggcttccccctggcggtggagctggaccgctacctcacgccggacggggcgctgatcctgtgcggctggcacggggcggtgttcgatccgctctcgggcgcctgcaccggcggaccgtgcgcgggcgggcgactgacgccttggccggtggaggcctcgggcggcgtgatccgcaccgcctgaggggccgggatcagtccagcggctgaggccgcgtgacgaccggtgcattcggatcattgctttgcggccgcgcggcggtcggcgccggagtggtgggcgcaggcgtgaccgtcaccaccggcggcggcgggatcggatcgatgatcggtggcgtcacgatcccttccggcgccggctggatgacgcgcggcgtcgtctcggatgccgcgggcgtcgagggccgaggcgtagagaccgccgcaggcgcgggcgtcggcgagcgcacagcggcgggcggcgggttcgtggaagccgtcgccgcgcggggcgtcgccgccggcgcgtcggatgggttctgcgcgacggtcggcgcctcatccgcagcgacgggctccggcggcaaggtcggcgtcgcggcaggcgaagacggagcaggcgtcccgatgctggaggtcacgggctcgggcgcgcctgttcgcgtcgccagccacacgccgccgccgatgatcaaaagggccgccacagccgccccggcatacagaggcaggcgcgatgagcgcgccggcttgtgcgacgccacggacgaggccgctggagccgcgacaggggcgctcggctccgtcggcggggcggcgtcggcctgagacctggccgactcattgaggggacggggccgcacagggggcgaggcgacctgcgcggcgggaccggccgaaggggccgtgatcgggtcgcgcggcaggggctgcacggtagcgccggcggaggacgtcgcgaccggcttggcggcggtcagcggtgcggcggccggagacgcagcgccgggcaaggggcgcacctgcagatcggccgaggcggcgccctgcacgggcggcgcgggcggggtcgccaccggcggcagcgccgcgggcgcttgcggacgcttctgcggcaccagcgaaccgccaaacacccccgccgacggtcgggccggcggcgcggcgggcgtcggcgtggaacggctctgcgcggatgtctgcgccgggccgggttccggcggctttggcggggtcagcggcttgaagcctgcgggcggaccgggctggcgcgcgggctgaggcaaggggccggcgtgaaaggtggcctgcggcatgcgcccccactgcaccgacttgcgggcgaagggctcgggcgatgggggacgcttgtcttcggacatggggcttcaactcgcgcgcgatctggccggtttcgtggcggggctcaggccttgaggcgatagccggtcttgaacatccacatcaccaccgccaggcacacggcgaagaagcccacggtcgccagcagactgacgccgatcgacacgtcgccctgtccgtagaaggtccagcgaaaacccgagatcagatacaccaccgggttgaacagggtgatcgcccgccacgccggcggcagcatgtcgatcgaatagaaggctccgcccaggaacgtcagcggcgtcacgatcagcatggggatgaagttcagctgctcgaacccgttggcccagaccccgatgatgaagccgaacaggctgaaggtcagcgacaccaggatcaggaagcccagcatccacaccggatgcagcacctccagcggcacaaagaagcccgccgtcgccaggatgatcagccccaggatcgccgacttggtcgccgccgcccccacataggccatgacgatctccagcgacgacaccggcgccgacaggatctcgtagatggtccctgtgaacttggggaaatagatgccgaacgaggcgttgaagatcgactgggtgaacaggctcagcatgatcaggccgggcacgatgaaggcgccgtaggctatgccgtccacctcctgcatccggccgccgatggccgagccgaacaccacgaaatacagcgcggtggtgatcaccggcgtcgccacgctctgccacagggtgcgcagcgcccgcgccatctcgaagcggtagatggcccagacgcctcttgcgttgaagccgatcacgccgccgcctccgtcttgtcgccatgcaccaggctgacgaagatgtcctccagcgagctttgccgggtgttcaggtccttgaaggcgatgcctagcccctccagacgccggatcagcgccggcaccccggtgtcgtcggcctgggcgtcgaaggcgtactccagctcctgcccctcgttgcgcaggctgagatcccattgcgccagttcgggcggcacggcggccagcggttcgaccagattcagcgtcagggtcttcttgcccagcttcttcatcagggtgatcttgtcctccaccaggatcagttcgcccttcaggatcacgcccacgcggtcggccatctcctcggcctcctcgatgtagtgggtggtcaggatcacggtgacgccgcgctcgcgcagacgccgcaccatggcccacatgtcccgccgcagctccacgtccacgccggctgtcggctcgtccaggaacaggatgtccggctcgtggctcagcgccttggcgctcatcacccggcgcttcatgccgcccgacagggtcatgatcttgctgtcgcgcttgtcccagagcgacaggtccttcagcacgccctcgataaaggctgggttcgccggcttgccgaacaggccccggctgaaggtgactgtggccagcaccgtctcgaaggcgtcggtggtcagctcctgcggcaccaggccgatcttggtgcgcgcctggcggaagtccgtgcggatatcatggccgtcggcgaccacgcgtccggtgctggccgtgacgatgccgcagacgatggagatcagcgtggtcttgcccgcgccgttcgggcccaacagggcgaagatctcacccttttcgatggtcaggtcgacgcgcttcagcgcctgcagacccgacgcataggtcttggtcagcccctcgatctcgatcgccggcatcgccacctctcagcgaccaatcgcagcgcgtctgaatatggcggctccatggccaagctcaagggcgccggcggtcagcttttccaatcaaacgccagcgtctcgcgatggccgaaccgctgaagatggtcggccacgacctgccggaagcgcgccatgtcagcgccctccccaccgtccagatcgatgcgcagcgcatggtcggaggcgctcaagcggcagacccccatcggcagttcgatgcggcccgcagccggcgtgaattcgacggggaacttgtgcgcccagtgcttggccagctgttgcagatagcggctggcgtgggcggtgggaacgtcggcatggctgtgagtcgtcatggcgccgatctgggatgtctgcgagcggctcgcaagaggaacggggagcccgccgatcgcctttgttcatcaagccttgctccgcaggatcgacatgttgaccgtccgcctcgccgttgtcgcctcgctgtttgcgctcggcgcctgtgcggggccgtcgcgcctgccggtcgatgcgggcttcggcgccgatccgcaactgccgccgccgcggcagacgctgatcccgaccgtcaagatcgcgcccgccgtcggctggccagcaggggccgctccggtcgcggccgaggggctgggcgtccaggcctttgcggacgggctggaccatccccgctggctgtatcgcctgccgaacggcgacgtgctggtcgcagagaccaacaagccgacgccgccgcccaccgttcggcgcgggctgcgcgaatgggtcatggacaaggtcatggcccgcgccggcgcgggcgtccccagtcccgaccgcatcaccctgctgcgcgacgcggacggcgacggcgtggccgagctgaagacgccgttcctgaccgggctgcattcgcctttcggaatggcgcagaccggcgaccgcctgttcatcgccaacgccgacgccgttgtcgcggtcccgtaccgttcggggcagacccgcattgatgtgacgccggtccgggttgcggaccttccggcggggcgcaaccaccactggaccaagagccttgtcgccagcccggatggttcgcgcctgtatgtcggggtgggatccaactcgaacgtcggcgaatacggcctgggcgaagaggtcgatcgcgccgccattctggagatcgatccggccacgggcgcgcgccgggtctacgcctccggccttcgcaatccggtcggcatggactggagccccgacgacgggcggctgtgggtcgcggtcaacgagcgcgacgagatcggccacgatcttgtccccgactacatgacggcggtgcagccgggcggcttctacggctggccatggagctactggggccggaacgtcgaccggcgccccccgcccgatccggccatggtcgcgcgcgccgtccgcccggactatgctctcggcgcccacaccgcctcgctgggccttgcgttcagccagggatcgctgctgcccccggacttgcgggacggcgtctttgtcggccagcacggttcctggaaccgctcgccgcgcacgggctacaaggtcatcttcgtgcccttctccgcaggccgcccggcgggtccgccgcaggatgtgctgaccggcttcctgaatgcggaaggccaggccatgggtcgaccggtgggcgtggcgttcgaccgggccggcgccctgctggtcgcggacgatgtcggcaacacgatctggcgcgtcgctccgtcgcgctgacaatacgcgtttatccgcgcccgccccttgcctgacgtcgggtcatccggcgcaatagcgccacggccgatcacaatccacgccgtcgagcccacaccgtttcgcgtcgcggttgacccgatgcgggggcttgttcattcaggatcgagcgacggcgcatccagcgccgcggcggggagacgaggcggcatgggactggtggccaacatccggcgcgacgtccggtttgcgagcggactcggtcggctcctgaagcgcatcaagcccatcgagctggacagccccgtgctgctgcccgacgacttcgaggaggcggtcgacaagttcgccgacaacgtcgccatcgaggacgagcatcgctcgctgacctatcgcgatctggatggcatggccaaccgctatgcccactgggccaaggggcgcggcctgcggcggggtgactgcatcgccctgatgatgaccaaccgcgtcgaatacatcgccgcctggatgggcttttccaagatcggcgtcgccacggccctgatcaacaccaacctgaccggtcaggcgctgggccactgcctgaccatctccggcgccttccagatcgtggcggacgaggactgctggcgcgcggtcgaggacgcccgtccgttcgtgaaccgcaacctgatgctgtgggtgctgggcctgaaggaggcggacgaggcctccgagcggcgcggtctggacaaggccgtgcgtggcggctcctccgtgcggccggccaagagcggtcgtgacggcatgaccaatcgcgacacggccctgttcatctacacctcgggcaccaccggcctgcccaaggccgcgcgcatcccgcactctcgcgcgcgcacctatatgcgcgccttcgccggctgcaccggatcgaccgagacagaccgcatcttcaactgcctgccgctgtaccactccaccggcggcctggtgggcgtcggcccggccctgttgaacggtggccgtctcgttctcaggaagaagttctcggcctccagcttctggcccgacgtgaagagttcgggcgcgaccatgttcgtctacatcggcgaactgtgccgctatctggtcaactgcccgccgaacgacgcggaacgcgatcacaagctgaagctggtgttcggcaacggcctgcgcgccgatgtgtggcccgagttccagaagcgcttcgccattccacgggtgctggaattctacggctcgaccgaaggcaatgtgtccctgttcaacttcgacggccggcagggcgccatcggccgcgtgcccaagcttctgaagagccagatcaacatccgcctggtcgagttcgacttggacaccgaacagccggtgcgcggctcggacggcctgtgccgtcccgcaccgctggggacggtgggcgaggccatcggcctgatcggccaggacgtgcgccacgacttttccggctacgcagacaaggcggcctcggaaaagaagatcctgaccgacgtgttcaagaagggcgaccgctggttccgcaccggcgacctgatgcgccaggacagcgaaggctatttctacttcatcgaccggatcggcgacaccttccgctggaagggcgaaaacgtctccaccatcgaggtcgagcagcgcctggccgaggcgcccggcgtgtcggaggccatcgtctatggcgtgccggtcgcgggctacgagggcaaggccggcatggccgcgctggtgatggagggcaagttcgacgccgcagccttcgccgcctatgtcgacgcgcagctgccgcactacgcccgtccggcctttgtgcgcctgatcgaaagcgccgacaccaccggcaccttcaagtaccgccgggtggacctggtctccgacggcttccagcccggcaaggtggagcacctctatgtccgccatgccgataaggggtacgccaagctgacccaggccgcgcacaaggcgatcctctcgggcgaaacgcgcctctgacgcctcgccggcaagaggcccttaagcattaacggcgatattcgacgtctcttcaacgcgtcgaagctcatccgtcatgttccagatcatcggcatcgtcatgctcttcggcatggtgttcggcagctatctgctggcgggcggcaagatggcggtgatcctgcactccctgccgttcgagctgatgggcatcctgggctcgggcatcgccgcctttctgatcgccaacagcatggacgtgatcaaggcgacgctggccggcttcggcaagatcttcggcggcgccaagtggaagaagcaggactacaaggacctcttgtcgctgctgttccagctgaccaagaccatgaagtccaagggcgtggtggcgctggagagccacatcgaaaagcccaaggagtccacgatcttccagaagtaccccaaggtgctgaaggaccatttcgccgtggacttcatctgcgacaccctgcgcatgatgaccatgaacctcgaagacccgcaccaggtcgaggacgccatggagaagcagctggaaaagcatcaccacgaggcccaggccggcgcccacgcgctgcagaacatggccgacgccctgcccgcgctgggcatcgtcatcgccgtgctgggcgtcatcaagaccatgggctcgatcaccgagccgccggaagtgctgggcggcatgatcggcggcgccctggtcggcaccttcctgggcgtgttcctggcctatggcatgatcggtccgttcgccacgcgcctgaaggacatcgtcgagcaggacggcgcctactacaagatcatccagtcggtgctggtcgcgcaccttcacggcaacgcggcgcagatttcggtggagatcggccggggcgacatcccctccaccgcccagccctcgttcgcggagatggaagaagccttgaacgcggcgcccaccgacgcctgatccagaccggcggcggtcatgtgacgcagggcgtcccgccggggaacagcctgcccgctggaggattgtgaagaggtcacgcggccgtgatcgccggcttgttccggcgcgagcggcggcgctagtctgctcttgggacctcgcgtcccggtcatgaacccttggaggaaaccatgcgcttcaccgttctcgccgtcgcatccgccgccgccctggcgctggccgcctgcggcaacaacaatgaatccgcggccaacgaccacgccgacaccgccgccgcggccgccgacaccgccgccgacgccgccgcgaccgccgatcaggccgccgccgacgccgccgccgccgcgggcgaggccgcctcggccgccggcgccgccccggccaacggcgccatgaccgatcccgccatgaacaacggtgcgatgaccggttcggccacgaccccgggcgcgacggctccggccggctcggccacgacgacgtcgcccgccaccaccacgcccgcgccggctcagtaagccacgccgacaaggatcaggggccgcgttctcgcggcccctttttcgcgctgtctcccgtcgaggcgtacgggatggtaagcgcgagccatgacttccgacgacctctcgccccacctgcactggacggaggcggacgagccccgctccggccgcttcggcgacgtctacttctccaaggacgacggcctggcggagacccgggcggtgttcctggccggctgcggcctgccggaggcctgggcggaacggcgccggttcacggtggccgagctcggcttcggctccggcctcaacatcgcggccctgctgcaggaatggcggcggaccagaccggcaggctcgcgactgcacgtcttctccgtggaaggtttccccctgagcgccccagaggcggcgcgcgccctgtcggcctttcccgacgtgtcggaggcggcgcaggcgttgctgtccgcctggcccgccgttacgccgggctttcaccgcatcgatctgcccggcttcgacgccgtgctggatctggcggtcggggatgtcgagtgggcgctggacgcgtggagcggatgcgccgacgcctggttcctggacggcttctcgcccgccctgaatcccggcatgtggtcgcctggggtgctgcgcctcgtgcggcggcggtccgcccccggcgcgcgcctggccaccttcaccgtcgccggtgcggtgcggcgcggtctcgctgaccatggcttcgtcgtcgagaagaggcccggtcacggccgcaagcgcgagcggctggaggcccgcctgcccgaccgcgcctcgtccccgcccgccgatccgcctcgcgtcgccgtgatcggagcgggcgtggcgggcgccgcggtcgtcagggccttgaacagcctcggcgtccgttccgtgctgatcgacaaggaagggccgggcgccggcggatcaggcttccccgccgccctcgtcacgccgcggctggacgccggagacgccctcatcgccggtctgcacgcccaggcgcttgagcgggcgcaccagctctacaccgagattgaaggcgcagtgcgggcggaaggggtgctgcagctggagcaggcgccccgcgaagccgcccgcttcgcccgcatcgccgatcaggcgatctggcggccaagcgccatgaccgtggtcgacgctcggcaggcatccgccatggccggagagctcctgcccaccggcgggctgatgatggcggacgcgctcgtcctgcatccgcgtgcggtgctcggcgcctggctgaaggatgtggacgttctatcggccgaggtccgccgtctcgtgcgcggtgacgggctgtggcgcctgatcgatgcgggcggacaggaggtcgcggctgtggacgtcgtggtgatctgcggcggctggggcgcatcggcgctgctggagggcctgagtctgccgcccatgggaccggtgcggggccaggccgactgggtccaagacgaaagccgcgccccgctcgcctggggcggctatctcgcgcccacggccgacggcctcctgttcggcgccacccacgaccggggcgacaccgacaccgcgtcgcgagacgccgacagcgcccgcaacctgcagaccctcgccgcccgtctgcccgagctggcggatcgtgtcgcccaagccgattcccgccgcagccgcgccgccgtacgcgccaccacgcccgaccgcctgccgctgtgcggagaggtcgaaggtcttcccggcctgcacctcctgaccgggctcggctcgcgcggcttctgcgtcgcgcccctgctggccgaacatgtggccgccgtgatctcgggcgcgccttcgccgctgccggccccctacgccgcgcgcctgtcgccgtcgcgcctcgcccgccggacggaaccgttcccacaggcggcggattgaaccgaaggccagacccggaggcggacgaccatgcgtgcgatcaccctgctgcccctcggcgtcctgttcggcatgctcgccgcctgcgcccccacgccgtcaggcgtcagcgacggcgtggagaccgcctcgcgtcagtgcttctacaccgatcaggtgcgcaacttccgcacggcgagcgacaacgtcctctccctccgtgacaaccgcaacaccgtgttccagctggattcggccggcggctgctgggacatcggcagccagtatgcgctgaccatcacgccctatctcggcggcggaaccagccgggtctgcgtcggcgacgatgcgcggatcggtcttgcgacctcaggccccggaccccgcacctgccgcgcccgcgtcacccgcaccctgtcggaggagcaggtcgccgccctgccgagccgcgatcgtccctgatcctcagacgtccaccgccgcgtccagggcgttttcctggatgaagtcgcgccgcggctcgaccacgtcgcccatcagcttggcgaacaggtcgtttgcgtcctcctcgtggtccaccgagacctgcagcagggtgcgggcgttggcgtccagcgtggtctcccaaagctgctcggggttcatctcgcccaagcccttgtagcgctggatggacaggcccttcttgcccgcgtccaagacagcgttcagcaggtccagcggcccccggatggtggtcgacttgtccttgcggcgatagacggcgggcgcctcgaacacgccttcgaacgcctgagcccgttcggccagacgccgcgcgtccagcgagcgcagcagcgtctcctccagcacgatggtctccgacaccgcgcggcgggtgcgggtgaacaccaccgccccctgctcgcccgtcgcgcccgaccagtcgccgtcgccctcttcggcatagaggttcaggcgcttggccgccgcggcgggatcgccgacctcttcgccgaacaggccggccagcgccgcctgttcgatggcgaaggcgggcgcgcgctggctcaggcgatcgacgcccgcccggaacgccttggcttcgcgaaccagcgactgcaggtccatgccggtgcggcgctctccgccttccaggtcgagctcggcctcggacgagccttcctcgatcagataggcgtccatctccgcctgatccttgaggtagcggctctgcttgcccttggagaccttatagagcggcggctgggcgatgtagacgtggccgcgctcgatcagctcgggcatttgccgataaaagaaggtcagaagcagggtgcggatgtgcgcgccgtcgacgtcggcgtcggccatcaggatgatcttgtggtagcgcagcttgtcggcgttgaagtcgtcgcggccgatgccggtgcccagggccaggatcagtgtgccgatcaggtccgacgacagcatgcggtcgaagcgcgcccgctcgacgttcaggatcttgcctcgcagcggcagcaccgcctggttctcgcggttcctcgcctgcttggccgagccgccggcgctatcgccctcgacgatgaacagttcggacttggccggatcgcgctcctgacagtccgccagcttgcccggcagcgagctgatctccagcgcggacttgcgccgcgtcaggtcgcgcgccttgcgcgccgcctcacgcgccgaggccgcctcgatgatcttggcgacgatcatcttggcctcgaccggatgctcctcgaaccaggtggacaggccttcggtgcacaggctctcgaccgccgggcgcacctcggacgagaccagcttgtccttggtctgggagctgaatttgggatcgggcaccttgaccgacagcacgcaggtcaggccctcgcgcgcgtcctcgccggagacggagaccttctccttcttgcccgcgcccgagctctcgatgtagccgcccatgacgcgcgtcaggctggcgcggaacgccgacaggtgcgtgcccccatcccgctgggggatgttgttggtgaagcacagcatggtctcgtgatagctgtcgttccaccacagggcgagatcgagctcgatcccctccttcttgccgcgaatgacgatcacgtccttcagcagcggcgccttggacttgtccagatggcgcacgaacgcctccaccccgccctcgtagtgcagcaggatgtcgatcggctcggcatggcgcaggtcgcgcagcttgatcaccacgcccgagttcaggaacgccagctcgcgcaggcggtgctccagcgtcttcaggtcgaagtcgatgtggctgaaggtggtgatcgacggaaagaacgtcacctccgtgccggtcagcgccttgccggtgtcctcgcggatcggggcctcgcccgtgacctccagcgacttgaccgtgtcgccgcgctcgaagcgcatctcgtggcgcttgccgttgcggtagatcttcagctgcagccaatcgctgagcgcgttcaccaccgacacgcccacgccgtgcaggccgcccgagaccttgtaggaattctggtcgaacttaccgccggcgtgcagctgggtcatgatgacctcggcggccgagacgccctcgccctcgtggatgtcggtcgggatgccgcgtccgttgtcggtcaccgtgaccgagccgtcggcgttcaggatcacctgcaccaggtcggcgtgccccgccagcgcctcgtcgatggcgttgtccaccacctcatagaccatgtggtgcagacccgagccgtcgtcggtgtcgccgatatacatgccggggcgcttgcgcaccgcatccaggcccttgagaaccttgatggaatcggcgccgtattcgggctgttcgacggattggtcggtcatagggtcagcagctctgaagtcccgcaggggacagggaggcgagcgtacggacggcgctcgagtcgagaccggcggcagaccggcttccgtgacgcaacatataagaaattatgggcgaaaagcgagactttccgccgcttcagccgggcgtcagcgcgccgtcccgcacaccgacgaactgggcccgtccatccagcccggcgaacagctcgcgttcggtgccggtcatgaaggcctgcaggcgcaaggcctcgatctcgtcgaacaacgccgcgcgtcgccgctcgtccagatgggcgggcgcctcgtccagcagcaggatcggctgggcgccggactggtcttccgccaggcgcgcgatctgcgccagcaccaggttcagcaccagcgccttctgctcgcctgaggagccttccgccgccggacggcgcgtctcgcggtgcatagccgtcaggtccgtgcgatgcggcccgaacagcgaccggccggccgcgccgtcgcgcgcgcgggaccgcagcaacccggcgcggacgcccgcggcgatctcgtcctcctccgatcccgcggcggccaacccttccgcctcgcccgccaaacccaaatcggcctgcggaaaaggccggtccgcgcgcgcatcgatcgccgcttgcagggcctgcagggccgcgacccgcgccgaggccgcccgcgcgcccgcctcgcccatccgcgcctccagcgcgtccagccagacggggtcggcctcgcgtccctccgccgcctcgttcaacaggcgctggcggtcgcgctgcgccttttcataggccgagatgctggcggcgtggtcggggtcggcggcgaacaccagccggtcgaagaacttcagccgctcggcgcgcgcgtcggaaaacagccggtcctgctcgggcgtcgcccacaccggccgcagatattccagcagccgtccgggctgcgccgtgtcgccgttgatgcggacgatccgccgggccgacggccccgccgcctgcacgcccgtgcccagccgcgccccgtcgtccagatcgaccgtcaccgcccaggcccgcccgcccgcctcgcccggctcgcgccggcccatctccgccgccgtcgcgccccgcaggcccttgccgggcgtcagcaggctgatggcctccaagaggttggtcttgcccgccccgttcggcccatgcagcaccacaggcctggaggtcatctccagccgcgcccctgcataggagcggaagtcggtgagggcgagggacgcgagggtcaagcaagccctagcgtgatgagggcggaggtcccgttcacacccgcagcggcatcagcacatactgcacgcccggatcgcccggatcgagcaccagggtggggctggcggggtcggcgaacttgaaggcggcgttctcgccggtgatctggccggcgacgtccagcaggtagcgggcgttgaagccgatctcgaacggctggtcggaatagccgatctcgacctcttcctcggcctgaccggcctccatgttgcgcacggtcagcttcacccggtcgttgtcgaaggccagcttcaccgaacggctcttctcggccgagatggtggcgacgcggtcaacggccttggcgaacagggcgttgtcgatatcggcctgcttgtcgttgccgcgcgggatgacgcgcagatagtcggggaaggccccgtcgatgaccttggaggtcaggctggcctcgcccagctggaagcggatcttctgggccgagacctgcacctgcaccggcgcattggtgtcgtccagcaggcggcggacctggtccacggtcttgcgcggcacgatcacgccggggccgccggccgccccttccggcgcgggcgtctcggccagggccagccggtggccgtcggtggccaccgcccgcagcagcggcgcgccgttctcggacacggcgtgcagatacaggccgttcagataatagcgcgtctcctccgtcgagacagcgaagcgggtcttgtcgatcagccgcgccaggtcctcccgcgccagcgaataggtcgcgccggacgcatcgttggacatcaccgggaaatcaccggccggcagcaccggcaggttgaagcgcgagcgcccggccgacaccaccaggcgcggatcgtcgccggaataggtcagcgacacctcggcgccttccggcagcttgcgcacaatctcgtacagggtgtgcgccggcgccgtgatctgcccttcgacgttcaccaccgcttccgcgtcgtccaccatctccatgtccagatcggtcgcggcgaaggccaggcggtcgcggcccgcgctcagcagcacattggacaggatcggaatggtgttgcggcgctccaccacgctctgcacatggcccagggccttgagaagcgcggatcgttcaatggtcagctgcatatcagttcgcccggcggcggcgcgccccctggcgccgctaagaagtgggtgcggacactagccgatcaggcggccggcgcaaacgcccgcgcgccgcccgatccacaagcgtcaggtcagccccgcagcttgcgcgtcagggtctcgacgtcgcgcgcgatctggtcgtcggaacccagcatctcctcgatcttgcgcacgccgtgcagcaccgtggtgtggtctcgcccgccgaagcgacggccgatgtcgggataggagcgcgtggtgtgctgcttgcacagatacatggcgatctgacgcgggcgggcgaccgagcgggtgcggcgttcgctcagcaggtccgcctgcttcagcccgaaatggtcggccaccgtcttctggatctcgtccacggtgatgcgacgctcgggcccgccacgcagcgccgcgcccagaaagccctgcgcctcctcgaccgtcagcgacgaaagccgcgatccggcggcggccgccagggtgttcaccgcgccttccagttcgcgcatcgagccaggggtgcgctccaccagttgctccagcacctcgatgcgcgcctcgccctggaccacgcccagcgcctccagcgccttcaggcggttgcgcgccaccgccaccttcagctcgcggtcgcccgcctcgaccgggcaggtcaggccggcggccaggtggctgcgcaggcgcggctcgacgtcggtcagcgccatgggcgcgcggtccgccgacaggacgatgcgcttgccgtcctcgattagggcggtcagcgtggacagcagctcttcctgggtgctcgccttgccgcccacgaactgcacgtcgtccagcagcagcatgtcggcgctgcgcaggctttccttgaaggcggcggtctgacgatcctgcatcgccttcacaaaggtggacaggaaccgctcggccgtcagatagaccaccttggcctgcggccgcaggcgctgggcctcccaagcgatggcgttcagcaggtgcgtcttgccgtagccgtagggaccgcagaagaacaccggattgaaatgcccgtcggcccaggtcgccacctggcgcgcaatggccagggcgaaggcgttgccctggccttccacgaagctgtcgaaggtcagccggtcctgcaggcccgccgcccggacggcgcgcgccccgtcggcgaccggcgccaccgtcggctgcaccagatgcggttgcgccaacgcagcgagacgcccggtcacgtccaccacattggcgccggaggcttgacctagagcgggcgcgggcgacccgacctcggcgcggcagcgcacgtccagccggcgatgttggccgtccaggcccagccacagctcgttcatgcggcgcagcgcgttcttgcgcacccagtcgcgcgcataggcggtgggcgtcaccaggatcagctgaccggcgtcgtcgacgcgcacggccgagggcgcgatgtaggaactgaaaggcccatcgccgatctcggcgcgcaggcgcagcgacgcctcgctccagatccgatccacatccgatccgcccgtcgtccggtccatcgccgccccgcccccgatcattccgtccacccgccttgcaaacccaaccaaatcaccaccctttacggggatgcgccggagacgagggcgcctgccccgaaaagcgatgctttccggcggggggccgaactcctggacagacatctccgccgacgcgggaccgaggcctcgcgccgtcttcatccgtgtcgggatggaagtgcgatagaggccaaaacttacgcggaggccgggtccggtcaacgcagattctctgcgggatcggcagttaaattgtttgactccgctaactcccaatccggcttggaattttcgcgggaaggccgctcaagaagcttggccgtgggtcgagctttccgcccgtctcgcttctgcgctttcccgccgccttagcagaaggcattgaacctgttggacttttatagcgcgtcagccgctcggctgagtcagatatgacccttatcgtcaagggggcgcgaaggaataacgtcgatctccagaccgaccctgccgccccgtttgggcgcgtcgcgcttttgcattgagccgctcgccgccatgctgtaagcggcgtttcaggatcggcgctcgcgccccacgcacccgtagctcagctggatagagcgttgccctccgaaggcaaaggtcacacgttcgaatcgtgtcgggtgcgccacttcggtttaaaactgagaactccgccaccggcggcacaatccccaccaccactggactctaagacccgtagaagttctgtgcgcgagccgataatgcgcgcctccgtcttgctgatgacctccacccgctgggttagggcgcggaggtgatcccgtcgatacccactggtccgatcccgcagcttgcgccgcgcggcgttagcgaaccgatttagtgcgtccggcgtgatcgtcggcgccaaccgatccacggatgcgctgatccgcccagcgtccgcccgagcctgatctcggatgcctgacagttcggccacgcgatccttcagtgaggcgtcgtcaggcgcgatcaggccgttctcaatggcttcgtagagccgattgagcttggcctcggcctcggtggcgcgcttgcgcatctccgcgatgtggctgcgccgctgatctgcccattcctcccgacggtcgagaagctgttccatcagcgccgctaggcgatgcggatcgagcaaacgagattcgaggtggtcgatgatggcgtcatcgagcttgtgcatcgggacagccagacctttgcagcccgcttcgcccatgcgggccttggtcgaacaggcatagtagcggtactggccgcccgcgctgccctttcccgttctcagggtcatcgcaccgccgcactcgccgcagaagcagatgcccgtgagtaggttcggaccggtggagacgcgcggcggcgtccatttcgggttccgggacgtgagacgcgctctgacggcctcgtggtccgccttcgaaacgatgggcggcacggccatgacggcgtgttccgactcgggttttggggccttcgtcttgtggtcacgtgtattgaaccggtgctcacccatgtaggtcgagcgggtcaggatctgatggacggcgctgatgccccagcgtccaccgtcgcgagtgcggacgttttgttcgttcaagcgggtggcgatggttttcagacccatgggcccttgcgagccgtcgccggtcagcgcccagcgatagatggtgcggacggtctcggcttggagcggatcgatctccagcgtcttcttgatcttggccccgcgctgctcagcggcgacgatgcggtagccgatgggcggccgggcgccgttccagaacccctgacgggcattctctttcatggctcgcagggtgtgcttggcgttctcgcgcgattggtactcgtcgaagagcgtcatgatttggcgcatcatcacgctcattgggtcgtcgcccagctcctgggtgattgagacgaggcgaacgccgttcttcgccaacttccggacgtagaactcgaactggaactggtcgcggaagaaccgcgagaagctgtgcaccacgatcatgtcgaaggcaggtggtttggtcagcgccgcctcgatcatggactggaaagatgggcgccggtcgtcggtggcggtgctccccggctcgacatactccgccgtcgcctcccaccccttcgtctcgcagtaggcttccaactgacggcgctggtcagggatcgacagatcgttgacagcctgtcgtccggtcgagacgcggaggtagagggcggcgcgagtccgaacgcctgtggtgacggctttgcaactcatgtcctgctcctctcagaggcgcggacccagaacctcgtcgagcacctcgccaagccacgcctccaccgcctgaagctcggccggggtgatcggcagatcatcagaccaggtgtcggtgacgcggacggccgattgtacgccaactggccgggcttgcggagtccggcgccgacacgcctcctgctctgatgacggctggacgtacatgtccgccaagctgatcgctctaaaactacgcgcatactcgtaaccttcccctcggaaatcttcggccgccgctttctcgcaaagcggatcgatccatcgatcacgcccagccctcagcggcggcggccgaccgggtcaacgcctgcggcgcttgccgcagcccgcagggcgcgaagcggggttgaagcgggcgggcggcgctgctccccaccccaaaaatgagggtccatacggctccgcttgtcagacaatgccggcgcaaagcctatcctgccctagaccctcatttgcgttctggatgtcggatgcgggcggctttatcgacggcgcggctcagacgaacgagcgcccctgccagacgcgcttcgaccactctcttctcgactccgaggtgctcggcgatctgctccagcggcattccggtgaagcgatggaggacaaagacatctcgatagcggcgagggagtcggcggatcgcccgcgccagaacgcggcgctcggggttttcctcgtcgaattgagatggcggagggttcacagagcggtgccgctgtcgatccctatcgcagcctcgacggcgctcagaagatcacagatgacttggtcggcgacttcgggtggaagcggcatgtccggcttgatgcccgagcgtagtgcgccggaaccataaagcggaccgagcaacgctgcgagttcggcagtgccgtcagggacaccttcaaatcccagcatcctaacgcagcggagcgccttgctcagatcgtgccggagccagacgcgtgtccagtcgtcagagaagccgcgatgcaggagataggctttgaggccaagctcaatagcgatggcggagtgataggccgactgggcacctacgcggtcatcgtctgtccaagccatcgcgtggaagcctcgggcgttacgggcgaaggcgatagccagtcggcgctgtggcggacgccgccgccaccgtcgtgaccggagtaagacgcgctgaggggttggcatgcgcagacctccgtagcgacggcgcggcatatagccggacggtgtcggctggcgtttcggcacaaggtgcgtgaagatgatcacaccgacccgactaagtcaacacggtgtactcataaaggagcacgtcgtgccgactatcacgcctttgcaagtcaagctggcccgaaccgccgtaggactcggagttcgagaactcgctgaatcggctggcgtcgccccgtccacaatccagcgtttcgaatccgggcgaggggacatgcagtctcgcacgttagacaaggtgcagaggtgccttgaagcctctggcgtgatcttcattccggctgattcaacgggcgggccgggcgttcgattgagggctcatgcggggcggggtgctgcaacggaagcaccctagagaaggcacagcgatcggcacagctcacgccgaggcggcattatgccaaacgtccatgggaacatcccagtggcattactccaacaatgttgctagtttgttctcattactcttggcgagggttcgcgaagattcttatcgtgaggtccgacttccgccgcgacgaggacgcaagaagtgctaagcgggctgccggagcgctcgcccgaaacgggaagacttggttaaatcccaagtcggtaggattaacgggagggaggaaagacgcatgtcggttcaacacatcctcgaccttctcgattcccacgccgccggggatgaggaacggctgttatcggtcgccctagccgccgccgccgcggaggccagggcgggacgtccccaggacgccgccgccctgaaggcggctgtccaagctcttcgctccgccactccgaaggccggcgcgaccgctgcccccattcccctggcccgcccgcggggcgagctgcagtcgctgatcaacagcagctatccgcgcaccaccctggccagtatggtcctttcgtccgagatggaggcccggctccagcgtctcgtgagacagcagcgggagcgcgccgccctgcgcgaccatggccagcgcccgtccacccatctgctgctgatcggcccgcccggcaccggcaagacgatgacctcggccgccttggccggtgagctgaagctccctctattcaccgtgaagctggagtccgtcttcagtcgctacatgggcgagactgctgccaagatccgactgatcttcgaccaggccgcgcagacccggggcgtctatctgctcgacgagttcgacgccatcggcgctcgccgcggcgatcccaatgacgtcggcgagatgcgccgggtgctgaactcggtgttggccttcatggaagagcccaatcagaccgacagcatcataattgccgcgaccaaccatgtcgaaatcctcgaccgggccttggcgcggcggttcgacgaggtggtcgaatacggcctgccgagcgtcgctgaggccaagaccctgctctcgacccggctgaagaagttcaagctcgacgcccgggcgctcaaggcgcttgcgcccgacctcgaaggcctcagccaggccgacgtcgtcctggccgccgacgccgcggtgaaggacgccatcctcgacggccaaagcaaggtgtcgctcgatctggtgcgcacggtgctgcaggagcgccgcgcggtcagcgctcgcttccattcctagattgcgcaatcgatgcaaccggtgatgattaacgaatcatcaccgccggatagccgatggctctcgaagacttcagccgccacaccctggcccatctgacgatcgacgcctttcgcgaggcgggtccctacacctatcccgcgcgccgccagacgcgcacgcctcagcgcgacgactatgtcgcgcacggccggcagttgctgggccaactggcggccgccctgcccgccctgccggtccaaggtgccgatccccgcctcgtgctggatggattacgaccgggcgcgatcgtctcggtggaaacccgcgcgccccagtccgatcgtcaggggccggccaaggtcccggccaccttcgagcttccggcccaggacctcatcgtcctgcgcaccagtcgacgcgatgatcgatcggaagtggctgtcgtcttcgtgcctgacgccgcccgcccggccctgcagcagaggatcgccgcctatggcgcccgggagctcggtaaccgcgaacggccgtatgtggatcagttcgagcggatcgagaccttcgccgccgccagcgcggaggacctgtttgcgggcgatcacgactcgaacgacccgcagcctcactggtgggagttgtgggtgcgcgatggcaaggccgaaggggtgcgcgtgcaggcgcgcgccgccgggttcgaggttcatgcggacaccctgatctttcccgacgtcgaggtggcctttgtccatgccgccgcagccaccctgcgcggcctgctcaaccgcatgcccggagccgtcgccgaggtccggaggtcggtcggcacgatcgagcccttcctgaccttggcggccaatgctgtgaaccagcacgacttcgtggccgagttcggcgggcgcatccgggctccggcgccggacgcgccggccatctgcattctcgacaccggcgtctccgccgcccatccgctggtggcgcctggcctggcccacgccacgacgatcaacgcggactggggaacggacgaccacgccgacgacacggggcacgggaccggcctggcgagcctggccctgttcggcgatctggaggggccgctgaacgatctgcgcgtggtccagcttggccatgcggtcgaatccgtgaaactcctcgccccgcggggggcggtgcagaccgacgtccacagctatggcgcggtgacccagtccgccatttccgtgatcgagatcgaccggcccgggatcgagcggtccttctgcctggcgtcctccaccgcgcgacacccgccgacccgcccttccagctggagcggcgcgatcgaccaggccgccgccggcgcgatgagcggcgagcgcgcacggggcatggcggccgcccagacccccaaacggctgatgctggtcgccgccggcaacgtcatcggcggatcgctggaggagatcgaggccggtgcccgcatcgaggatccggcccaggcctggaacgctctgaccataggcggggttaccgccaagacgaccgtcgagcctggagccgcacggctgcgtccggtcgcggcggccaatacggtcagcccctacagcgccgacacagtgggcttgccgaccgacctgctgccgatgaagccggaggtgatgttcgaagctggcaacatgaccgtggatgcggcgaactggtgcgacctgcatccggccttgtccctgctagccgccggccgggatgtagagagcgaacctctgtcctccttctgggccacgagcgcggccgtcgcggtcggcgggcatttcctgggccggctgaaggccgagctgcccggtctgtggccggagacctatcgggcgctgatggtgcatagcgcccgctggcccgagcccattcgtcggcagctcatcggtacgggggccagctggcggacgcggctaagcaaggccgacattcagcgactgctgcgccgggtcggttatggcgtcccggatctcgacatcgcgacgcggtcggcccgcaatgatctgacgctcctggcccaggccgaaatccagccctatgcggccggagccaacgatcagggggcggtcttcaacgaggtgcatttctacgacctgccttggccggtcgaggccctgcgcgctctcggggacgagccgatgacgatgcgggtcaccctctcgtacttcatcgaacccaatctgagtggcaaggcggccacccgtcccgaaacctaccgttcctacggcttgcggtttgcgctgaagaagcgaaccgagacggatcttgagttcaaaggacggctcagccgtctgcagaacgaggcacaggtggccgcgctagaggccggcgacgaagacgcggacgctcaaggcgaacggtctttctggctgctggggcccaaggcggtccaggccggatccctgcactgcgacctctggcgcggcaaggcgtccgatctggtcaaccacgacctgatcgcggttcatcccgtgggcggctggtggaagtcgcatctcggccagcagcggcgcagcgaccgggggcgctacgccctggccctgtccatctcggccccgtcgtcggaggtcgatctctacagtgagtcccaggccctggtgatcgacaaggacatcgagatcctgctcggctgagatcgaacgccgcggctcaggccggggcgcatccgctcggcgacgttgatttgtcctcctcgacgaacccgtaagcccctgcctatttggccgccttggtcgcgaagacgcagggttcggcgtcggtcggcggcgcgaagaccggccaccagaacgggtgcgcggtccatccgagatcccggccgccctgctgctgcagcaaggccagcgctggcttgctgcggggctcatcgaggagcttgcgcctcagcaccgtaccgacgatcgaccggccggatttgtcgcccgacttttcccggttcagccggcggccggtttcggcgattagggcgatcttgccgtcgccaccgtgcttggcgtccgagtagtagtcgatcagggcgcgcatggcgtcccactcgaattcaacggtgtcgaattccatgctgttctcgatggcggcgatgatttccaaagccatcttgcgctcgacctcgacgaactcgccggtgtctcgccaagcgggattgatcagcttctccagcttggcctgaacaaccgccatggcgttgccgccacgggtctgaaaatcggtcggcaacagcaggcttgacggagagaccgacaccatctcactcagcatcaccttgttcggcgcgcaggggcgcacccggccggtagggtcggactggataaagacaacgccggcgtcttccttcttctcgtcgaaggccgtgcggagcgcgttttccaaagcgttgatcgtgtagagccggtcgtagaccgcccgcgaggtgtagaagcgcgtcaccgccaggtcttgccgattgcggttcccgtacatgcgcgagtgctgcagcaccgtatcggcttgcatcgtccgggggtttcgcccgtagtagaaggcgatgaggttcgggatcgtgatcccacgatccagaatgttgccgccgacccatatgttgtagggcgtgcgcagcttcaactcagcgttgtcatcgagcagcttcatgacgtcgttgtcggagttcaccttctcgacgacgacctcgtcactctgcagggcgtcgatgaatgcgtcgaaagcgtcgtcgcggggtggcatcttgcccttgtcggcggtgaccgaggcctggaggtcgtcatatgcttgatcgaacattggccgcagcgcgtcgggggcgctctccgccgcctcaatgatggcactgaagatccagtcgatcacctgatcctgccaggcgtgcgccgcccgctggatatcgttgtggatgaccatggcgtatttggttggccgcaggccggcctcccgctgctgccattgccgcacacccacggccaccacgaaggtggtgatggcgcggcgcaggcccgtggtgttgggcgtatcgagcacggtgctctggctaatgcggcgcttgtcggccttgcgcagcgagtcttgctcctggtcggtaacctcgacgatcagcttggaccgcgggtcgtcatcgtcgaaagcgccgaaatagtcgtcgccaccgacataaccgccatggatcggcaagggctcggtgaacgccggccgcttgggcgtgaacacgtagctctcgccgctcgccgtctcctcgtaatcctcgggctgcaaatagagcgaatagggcgtggcggtgacctgcaggaaggcgatgccgttggacatcccgcgcagctcgtcgatctgccccgcgatcgtgccttgagcgaccgcgccggttcccttgtcacggacgaagcgcacgctggccaggtcggcctcgtcgtcaatcaggaggaccttgcggttctgcagaccctggttggactgcatgaagttgatcaggcgctccaggttcttggactgcttcttggcgacaacgacgatcttgcggcgcagctctccgcgcttaagcgtagggaggttcatgatgtcgagcaccatgatctcatcgtcggcgatgaactccttgaaatcggagctcaaccgcctgaccgtctgggctgatagggttttggtccccttagtcagcactagggcgatgtcgaagccgcggtcgaacgccttggcgatcactccgacgaaggcacgcgtctttccggactggatcttccccagcagcattcccgggctgcgcccactggtgccgttggcttcaaggcgggtgacgatccgatcgatgcaagcggcgaggccctcgtcatcgttacgctggctcttcaagcgtggatagaagttcgagccctcgtccatctcgctgagtttacggttgttgcgcttcaaccaagcgcggatctggggctttcggaaaaccggccccgaagccaactcggcaagcggggatgggaagtcagatgaacgcgcccgccaattggtgactgcttggctcgtcacgccggcgagggcggcgatttcgttgatcccgaccagatcgtgttccatttagcacctgtgtagtttgtacacattgtgtacgtcgcacacagtggagagtcaacagtcgtgagcgtgatcaactcgtcgcttggacggcggaagtcttggggcacgttaacagggcctttgaatgcgggcggcgttcggctagccaggtcggacatcaggggcctaggccaatccagatcccggtcagtgcatgagcttcgggtatgggtgccgctcctgacagccgaaggttctcgagccctcgcctcgatagccgctcataactcgtagcgtctcgcgggggcggtagggctgtgttcgccgaaccgtaatgaggagcgagctttgcgcctggctttgtgtactgcagttcgcttagcgacgggttttctcgtttcgacggtcaatcatctttatccgcctggacctgggtgatgaggtcgctcaacagcatcattcgcaccagggcggtaagctgctgccctacgaaggtttcgtagcctcgcagggtcgcattcatctgtgcggtgaaatcgagcgaaccgctatcgatcttctcgatgaagagcttaagaaacccggtgaaatcgccgacctctgagacggctgagcttaacaccaatccctccactttctcgcgggcccacgtcgcaccctccagcgtcgtctgttcaaggcttggccgcccctcgccggcgaacccccaggcgcggatgccgtcctgcacgaccaaccgcgtccactatccgcagcccattctgctggacgcgcgtgaggcggggttgcttgaccggtatctcgcgctcaagggcaagctcggctcgcgcctcgatctcgcgcttaggcggctccgctcggcctacgggcgtgtcgacgaagaggatcaactgctggacctgtcgatcgctttcgaggcgcttctgggcgacgacaagaacgaactctcgttccgctacggtctgcgcggcgcgttgcttctgggctcgggcccggaggagcgccggcggatcaggacagcgatcaagaccatgtacgcgctccggagcaagatcgtgcatgggggcacggtcacggacgatctcaggaccgtcacacgtggcgcaatcgcgcaggtggtcctgattcttcagatcttcattgggctcgggaaggagcccgactggaacgctctcgagctgggcgaaggtttgtactgacgcgccgacacgtgatgctggctggccatcagccggccaccgcgaccgctgtgcaatagttctcggcttcgtccgatgcggcgcacccacgccggcatcgctcagccacgccatacagatggctgctgtcctaggtgtctgcaccctagcccaccgcccacgggaacgcatggtgaacactctgcgttggacgaggtaggaggaagagctatgaccgaacgcgaactcaacgagcctcacaaaggcgataaacgatatcagcgtcgcaacaaagacggcacacttggcgaatccgacgatcagtcgaagtcgcttggcaaagacgttcagcagcacgctaaaacgaaaaagccgaaaaacgagggcgacaagggcgactaataatctggcttgcctgagcgcttcgctcgtctaggtgaggagtggaggcaagcatgactcgcaaactgtttatttcgtatagccacgccgacgccgatctattgggtgaactgcgcgttcatcttcgtccgcatgagcggaatggagtcatcgagccttggcatgacggatatctgatacccggcgacgacttcgactccgaggtccgcaaagctctcgcggagtcgaactttatcgcactcttagtgacgcccagatttcttgcctctgactactgcgttgacgtcgagatggaggatgccgtccgccgtcacctcgctggggaggctcgggtcgttcccatcatcgctaaaacctgcggttggaaagaaacctttctaaagaaacttctggcgacccccaaggatgggatccccatcacgaagtggcccgaccaggatgaggcctgggacatggtggccggcgatattgcaaaggcggcgcgaactccgctgggacaaaaaacgggcgccccggaatcgtacacgcgtcgcgacccagcggcgcctgctccgcgcgccatgcccgccgagccgcagcgcacaactgttgccgcccaggtcttttccattcccagaaatgcgaagccgacggatcagcagatcgacgacttccgtcatgaagctttcgagcggatcgcggagcttttcgaggcatcggtcagcgcgctgacggacgggatgtccggacggttcaggcgcgtcgacgccaaccgcttcaccgccaccctttatcgccaaggtcaaaagctcggcggatgcactgtcttcaccggcaccggccatttcgcagcgcacggcatcgcctacagcggcactgacagcggcgagaccaatggcatgaatgaagaattgtcggtcgatctgggtcccgctggccttggactgaagccgctgatgcgcggcatgcacagtggcgagcgggataagacaatctctccggaggaaagcgccaagctcctgtgggacatgttcaccgagcgcttgaggtactgagagcgaagggggatcggctacatgccctctcaatctctccgcgtgctccgacagaagcggtgatcgcgaccaaagtggagtagttctcaggatcatccacggcggcgcacccacgacgtctcgcgcctcgacagcgaagagtcccgccaatgccgtcgcaggtccgcattgcgcctggacggcaaagcccgaattcgacccatacaagacatttagccccggttcgaaacacgacattcagtgacgtgatggtgtggacgacctccgcctgacgggctgttctgggtgtgtcgtcatcagggacgtcacgtctaggagcggtatcatgcagaccatcgctgtcgtcgggctcgatctggcgaagactgttttccaggttcacggtgtagccacagacggcacggtcgtcgtgagacggcaactgcggcgcggccaggtgctggccttcttccagtcgattgggccgtgcctgatcgggatcgaggcgtgcgcctcagcccaccactgggcgcgtgaactgatggcgatcggccacgatgttcggctcatgccgccggcgtacgtgaaggcctatgtgaagcgcggcaagaccgacgccgccgacgctgaagcgattgccgaggctgtcacccggccgaccatgcggttcgtggctgtgaagtcgaaggcccagcaggcggtgttgatgctgcacaagacccgggatctcctggttcgtcagcgaacgatgctgatcaacgcactgcggggccacctcggggagttcggcatcgtcgcgcctcaaggtccagctggggtgcgggcagcgctgaagagtctgcgtgaagagggtcaggccctgccggatctggcgcatgccgcgcttggcgggctggcagaacagctcgaacaccttggcgcagagatcagccgtatggagcgtcggattctcgattggcatcggcaggatgagacgagccggcgactggcgaccatcccaggcatcgggccgatcactgccagcgccatggcggccagcgcgccagatccgagtctcttccgttccggtcggcagtttgcagcctggctgggactcacgccgcgggccaatagcagtggcggcaaggaacgccagggcggcatcagcaagatgggtgacagctaccttcgacgtctcctggtcgtcggggccacggcggtcctgcgaatggcccggcagcgaggacgcgagggctgggtcggcaatctcctcgaacgcaagaagccgaaggtcgccgccgtggccttggccaataagacggctcgcatcgcctggaccctgatggcgcgacaggaggactacaagcccacagcggcatagagatcgggccggtcttcacccaggaccggcgccgtagacgaaggagtggtgagacgtgatgacgaaccggccgcagccggggatcggtgaaacccagggggtcagagcgcctcgagcgcgttgacgtgattagggagccggtccgcggacttcatcagggccagcagcgcaaacagctgcatcaacaggccgaacacatgactgcactcgaccgagcgccaacgtcgtttccactcttgcgtcttggaggtcgtccacacatgacccccgtttctcatccagccataacgagagtcctttggtgatctgaactggggtttgtggggttggcaagaggccggtcagcgcagcccccaaccagcgcagcggaccggccgatctgtacggtgagcgcttctgcgtaagcctgcggcgtcagccatccgagcttcgagtgcggtcgggtttcgttgtagtcgcgtcgccaggcctccagcaccgcgcgggcgtgcggcagggagcggaacagcgtctcgttcagcagctcgtcgcgaagccggccattgaagctttcgttgaagccgttctgctggggcttgcccggtgcgatgtaatgccagcccacgccggcctcgtcggcccaagccaaaatggcgttggacgtatattccgtgccgttgtcgctgatgatggtgtctggtcgccctcgccgttggatgatggcgttcagctcgcgcgcgacccgcaggcccgagagcgaggtgtcggcgacgagcccgaggcactcgcgggtgcagttgtcgatcaccgtcaggatgcggaagcgccgtccatccgtcatctgatccgacacgaagtcgagcgaccagcgctggttcgcgaccagggggatctccaatggacgccgcgtgcccatggcccgtttacgcccgccccgccggcgcaccgtcagcttctcctcgcgatagatccgctgaacccgcttcttgttgaccgcatggccctcccgcctaagcaggatgtgcaggcggcgatagccgaaccggcgacgctcctgggccagagccttcagccggtcgcgcagcgcgccgtcgtccgggcgcgtcgcctgatagcgcacgctcgtccgatcgacgcccagcacacggcacgcccgccgttcgctcatctcgtaggcggcctgcagatggctagccgcctcgcgatagccggcgggcgtcaccacttttttcccagcagatccttcagcgcgacgttgtccagcatcgcgtccgccagcatccgcttcagcttggtgttctcgtcctccagcgccttcagccgccgggcctccgacacgtccatgcctccgaacttggccttccacttgtagaaggtcgccgagctgacaccgtgtcgccggcacacctctgccgtcgccacaccggcctcctgctcccgcaagatcccgatgatttgctcttccgtgaaccttgatcgcttcattctgtccgtccttcgttgggcggactctagctattcctggaggagtttcaggggggcacgtcacggtcaacggcctcgcgcttgaaagaatccggaaagttccggcgttgaacactcatcagacactcctctccagctccgaaaagctagcatgggtgtccaccaaaccgagggaggatcatgttctcgatgtagactgttccgctcctgcggccgggatgctctagcgcgttccgcatccgaacgagcggcacggcccattgctgttctgaccggataagcgtggtgcgctgatcgtcagcaccgaacctctcgacagctcaagcttccagcttcgatgcggtctccttaccgttgaggatgtagacggacgcctcgtcgaaatcggtttcgtaaaaccagttccagacgcggagggtgttccgaaggtagttcttggcttggtagaggaagtgttctgctctctgttccagttgttcgacagcgtgaaggtgaaagacgcgcgggtctctcttgttctgcccggaggcttggacggccttcaaaacatcagccgctagagcgtcccgcgtcttccagcactctatcagcaccggatagagttctttgtaatagatcgtcgcaagatcgtcccgctgacccttgctatagcttgtggctgcaaggagatcggtcgtctgcaacatcagccgcgcgacgactggattgcttgttccaacgtccgataccttcgtgaccgtccaccgcattcgctcgtccatctctgctccgtcctgacgctacggctgtggatggcctgaagccaagggttgaaaccagaacagaaccagaacattcctccggccatgagggcgaggcctccttccgaatggacacctgagaacgtcaccgcccgtgatgtcgctgcggattccaagttcgtggcgacgttccggtgtgagggatgccgcgagagccgcgagttcaacgtcttcaaggtcgggatggtgctggccgacactccccttcagagtcttcgctttcgctgccaaaagtgcggactctatccgagtgtcttggagatcggccggagaacgtcgggtatcggcgaccaccttgtgaccgtcaggttgaggccgaggtgctgggacgagggccatgagcggaagcagcgggaagctgcgtcgcggctcaatcgaagctgatctggtgcaatatgtcgcgcctgtggatgggtctgaaaccgcctgagcgtaaccgcattgtatcgggctatggggtcaacgatcagctacaaccggatgcgtgctgcgtcggcgcggcggctcgcgctcaaggctgataatcccgacgaccgttggcgcctcctgcgtatctcacaccagtatgacgcaatcaccgaactggaagcggcgacgccatcggtcaggcgcgctgaaggccagcgacggctttaagttcgttcctcgctaggacttttcagcatcgtcagagcttcagcgatctgcggtctcaatcgccacctccagtgatcactgtccggttcaaccgtgtcgatggatcgatctgcgtcgtcagcaccagtggccaaggcgaacgtccagatcgccactcctttgaagtgcggtggcgaccagcccaactgatcagccagcttcttgccgagcttaccatattggctgttcgcggcttcatagtggtcgctacccgccgccttggccaactgagtggccgtcaggatcatgtcaggagcgcgcagatgggcatggagcatcgcatcctgcccgttggagatggatatctgcttgagcgcgacgtgcacctcagcggcgcaagggaagccatctcgcgcgcgtgcttcggcgaactccctgtcaatctcgtcgatctgccgtttcagagcggctaccacctcgtccttcgtggcttcgctgaggatcgctccaaccctctcgtcgccgcgatagctcgctccccgccagaccgaaccagacggcacaaacttcaggaggtagcgcccgtatgagactgagcggtcgttgtctgtcacggattttacgacctcagacgccggaggggatcacctgaacggcgtaaagccgcaacagaccgtcgtcaatatgatgtccccatactcgacatcatatggctgtcctgccatacgatgtcgccttcagcgacatcatacgcaggaagccgtgagcgatttcggactggccgccttcaaggcatcaccactggggaagaagatcgaaccgatcatcacccaccccgaggttcgcactgagatgaaggtgctggccaagtatggcttcgcgcccgtgatcgcgcttgacgaacgactcgctcatctcagaccggaagttggggtgcgagaagtcaactcgcagatcggacgttgggtctacgaggagatcggagaggacgtatacgaggtggccgggcggaccaagctcaagggccaagtgttcagcacgggcgccacgttccggtcgctacccgaagaggcctatcgcatcgaacgtcgggagcctcgccccggtgggcccgaatacccggtgaaagggccaaggggctatgtgctggtctcacctgatctcccgaagggggaacggacccgcgatggtaacgcgatccatgtcgagaccctagctgaagctgtgcccttcctcgacgagggctaccacatccgcatgggacgaaagggcgttcgtccgtcattgatcgcgaagaagagcctgaagatcgcgaagctgtaggttgttaggtgttgtcagtgctgaaggatggccgaccggcgggcttcacgacttcgctgcgctctttgggggccgccccacagggttcttcgtcgcggaggatttcgctcgtcgcttcgcgcgctcctcagaactcggcaggatgtccctgtccgaccgaggggatttgatgcgtgcggcgggcacctttgtcgaagccaccttcaacttcttatttggcttgccagtcgctgttaggataccagcccccgtcacgggaagcaccgtcacaatccctacctgactggcgttcagtttcgttgccagatcatcggcttgcttcttggtgtagaggtagatgtcgtagtcgccaccgaaatcccgttttcgtattgccccccgcatcacgaactgaaggacgtcttcctcttcccgcgctcgttcgatctgggcatcggtgatgccggtcagggttgacgtgatggtgtggacgacctccgcctgacccaactcgccttttcgccccgccgcgtgggctcgatccagatctggaagatgcgggtggtcacatcctcggcgttccattcggagtggcgaacgcccgtgcccgcgctcataacctgtacgtcgccggcttcggtccggccctggttgcccaggctgtcctgatgggtgatggctccgtcccggacgtaggtgatgatctccatgtccgaatgcggatgcggcggaaagcccgtgccgggggcgatctcgtcgtcattccagacgcgcagcgcgccccagctcatgcgagaagggtcatgatagctggcgaaggagaaatggtgcttggcgttcagccagccgtgatcggcgccgccgagctgctcaaaaggtctgcgttcgatcatcgtgtttgtccctcgtttcatcgagccgccgagctcgtgcttcgagagccaagataagggcgatgaaccgatccgcaacagcgctcgatatcaatgcactgtgaggcgtatccgcctcgtcttcagggcgtgaactggatggtgcgctcgaaacggtgaggctggttgtcgccggcgggctcaagcgtcgcgccgttcatcagggccagcgccgcttcgccaaagcccaagcccgggcgggtttcgtgcaggacctcgcaattcgccacgcggccgtccggatacgccgtgcagcctagccgcacggcgacgttcgacaacggggcctcgggagccgccttcacgtccgtctgaacagccttcaccaacggcttggcgggctgcgccgcaaccgggttggaggcggtcagaagcagaacgagagcggaaacgagcatggcggggcggccttgaaacgacaaggctacaacccctgaccctcagacctgttccacccttgcgtgaagtatgccgctgcgtcccagcccgtgttcaggcgacgcttgctgcggtctgagactcgacgaccgcggagcggggcgtcttcgccttcggcttgcgcgcccgaagctcagccgcggcgatatagatcggcgttcccgccaccagcaggcagacgctgccgatgctgatcaagcccatgacctgcgcgatggacgatgcaaccatgcgtattccccccggagcgcataaaggtgaagcttgtcttaacacgaggcgaagctgttcgccaaccggcgttgcagtatcttgagctgcggaaggggaaaatggcgcacccgacacgagaccgggtgcgggcttggctctgcgggatttgggtgtcgtcggtcaaggggctcgctccatcgttctggagcgtccagccatcgtcacgggagcgattccgtcaacgctcttgagggcgatctcgcgacgctcacgaccggctctgacgtcaggcggcgacgctctccagacggtcttcctcgaccgtggccatcgagcgtttgatcgcggtcacggtcatgggcgaggcacgatggaggcgggcggtggcgcggatgccctgaccgtctcgcaacgatttcctgatcgcttccacacggtcgtcaggcatgggcttgcgaccgctcttcttggtcgtccgccggaggcccgagaacacgcgctccctgtgaatggccctttcgaattcggcaaaaacgccaagcatcgagaacatcatccggccggagggcgtcgaggtgtcgaggccctgcgtgtggacgtagaggtccacgttcttggtctggatgtcgccgaggaagtggatcaggtcaggcagggatcggccgatcctacagaccgagaagcaagcgatcagatcgaagtccctgcgtgcgacccctttcagcaaggcgtcgaaccccggtcgtttgtctcgtcccttggcgccggatatgccctcgtcgaggaacgtcgccgcgatcttccagtcctgacgctcggcgacggccagcagatcgcgcagttggttctcgacggtctggttcttatcggccgtgctcacacgagcgtagatggcgacgcgcttggtcagggtgttctccgatccaatgttgggagaacaggctctcatggatcggtaggccgtcaatcagatgtgggacacactttagagcaggctgacggaccttgataataacctgtcagcggcgaacgttagacactcttcccgattcagaagcgtcacgctgtccgtcacaggcgcctgttcacatttcctgacagccgcttcgtgctcgacctccaattgagcaaactgccgttgaagtgctgattggtcacggacttcgatttccgagcgggcggcacctatcattacggtcagccactcccgctcctgctcgtagcaatgggtcagcaggtggtcggccgagcttgagccgtcggttctatgattggagcaggttggacgctgtgtcgcgatagtctcacgaatctgctgtgcggcctcggctcgctcggtcggcggcggcggcgaacacgcggccaacaaaacagctaacgtcgcaacgcgaagcttgaacatctttccccccttggtttccgatccggacatagcatctggtttcgccgtcccctgaatcagatggtgtcaggcacatcgacgagcggctctgaaagcccggctcttcgggccgccggagggctgaattccgagggtgtttgggagaacggcgccaacagcgccaatagcgtcgatagctcggccagaacctgtcctcgcgtgcttggtcggccttcggcctcgtcacctgattttctggttcacgagatcaatcaaccgaaggccagtcgctggtcgaaggcgagcggctcgtccgcgaagacatcgaccaaggcgaacgatgtcgtggccgaaggacacggctcgtcccgatcaaccacatcaggctgaagcctccacaaccaccatcagcgaggcgaccgccttcggcgttcacctgcgacagggccgctcgtctcgacctcgggcctcgcctccggctcgttgccttcggtcggccgatcagcccgtcgatctctccagaaccagatcactcgtccccggagagccgaattaattatgtccgcaccttctctaagagaagcacgcgcggacagagtttcttcagaggtcgaaaggcacagcttccacacgatccagccaacacgcgcgaaccctatcgacgctgttggcgccaacgacagagggagcaggtgcgtgggggacaggacgatttcggagattgctttcgatctttgggccagcgagcaggggttgctggaccggctgggtctggctgcgccagagcgtcatgaggcgggaacgcagtgttggctatacgcgggcaccgcccttgatgttcggaagcgggaggtcgtccacacgttcacccgaggtgctgggacgcgacagtggtcattcagtccgtgggacggcgggcgacccgactttgagcccgtccttgagatcaccatccacatgctgcgaaccaaggcgaaggaggcttggcgttccgcatctgatgctctcgacgctgctgtcgccgatgggcgcgtggtgatcgccgggcgcattggatcgcctgtggccgattcgcagagctttccctcctccgcatgggccttcatcgacatcgatgactggagcgcagcaactggcgaaggtcaggggatgggagacatcttcgacctccgcgaatttgaagccaccgaggatgttcagtttgaagacagtgatgacctcgggcggtttgcctcggccgttaaggttgagttggccaaaatttatcccatgggcatccctgcccatctgactcacaaagaactgcacaacgacgtctgcaaacactacacgctggcagggatcaaccgacagccaagtttggataccgtcaagcgagcagcgggccggaggaagcaaaagtagcagaaaaagcagccgatcttgcttgattacaagccgaggttcgggctgcatatgggtctccgtctttcaccgccgcttctgcggcaagaaaatcggagagcctatgaagacccgcctgatcgcgtcgagcaccacttcggacccgacctccttcaactgggacaaccccgacacctcgctgcttgatggcgatgtggcgccccgccctgatttccccacgcacttgctcggcgaaactcgcccgctgaaggtcgtcgatctattctgcggcgtgggcggcctttcgcgtgggtttgaggacgccggatacgaggtcgttgcggccttcgactattgggagcgagcggtcgagacatatcggttgaatttcagccaccctgtcttccggttcgatctgaccgatgtcgaagcggcaaccgctcagatcagaccttttgccccggacctgatcgtgggcggtcccccgtgccaagagttctcatcagcgggcaagcggtctgagggaagcaaggccgtgacgtgatggtgtggacgacctccgcctgacgggctgttctgggtgtgtcgtcatcagggacgtcacgtctaggagcggtatcatgcagaccatcgctgtcgtcgggctcgatctggcgaagactgttttccaggttcacggtgtagccacagacggcacggtcgtcgtgagacggcaactgcggcgcggccaggtgctggccttcttccagtcgattgggccgtgcctgatcgggatcgaggcgtgcgcctcagcccaccactgggcgcgtgaactgatggcgatcggccacgatgttcggctcatgccgccggcgtacgtgaaggcctatgtgaagcgcggcaagaccgacgccgccgacgctgaagcgattgccgaggctgtcacccggccgaccatgcggttcgtggctgtgaagtcgaaggcccagcaggcggtgttgatgctgcacaagacccgggatctcctggttcgtcagcgaacgatgctgatcaacgcactgcggggccacctcggggagttcggcatcgtcgcgcctcaaggtccagctggggtgcgggcagcgctgaagagtctgcgtgaagagggtcaggccctgccggatctggcgcatgccgcgcttggcgggctggcagaacagctcgaacaccttggcgcagagatcagccgtatggagcgtcggattctcgattggcatcggcaggatgagacgagccggcgactggcgaccatcccaggcatcgggccgatcactgccagcgccatggcggccagcgcgccagatccgagtctcttccgttccggtcggcagtttgcagcctggctgggactcacgccgcgggccaatagcagtggcggcaaggaacgccagggcggcatcagcaagatgggtgacagctaccttcgacgtctcctggtcgtcggggccacggcggtcctgcgaatggcccggcagcgaggacgcgagggctgggtcggcaatctcctcgaacgcaagaagccgaaggtcgccgccgtggccttggccaataagacggctcgcatcgcctggaccctgatggcgcgacaggaggactacaagcccacagcggcatagagatcgggccggtcttcacccaggaccggcgccgtagacgaaggagtggtgagacgtgatgacgaaccggccgcagccggggatcggtgaaacccagggggtcagagcgcctcgagcgcgttgacgtgattagggagccggtccgcggacttcatcagggccagcagcgcaaacagctgcatcaacaggccgaacacatgactgcactcgaccgagcgccaacgtcgtttccactcttgcgtcttggaggtcgtccacacatgacgtccctgatgacgacacacccagaacagcccgtcaggcggaggtcgtccacaccatcacgtcatggaggaggccgtcgaaggcgatcgcgatcaattccgatagatcatcctcgaccatggcaatgggcggatgacgcaggttggcagaggaagatcgttccaagagagtcatggccgtaaactcgctgggtgatgtccggaaaagctgggaagctccggacccgccctctgcgggtccggagctacaagccttcgacgatgcgctgcgcgtggaccgaaccacgtccgcttagttcaagatccattcgatacaaatggagcctcgccgcacagtgtcaatagcgaaccgcacgtcccagcgatgaacgaggtcacgacactccgctcctttagtcgctgctagttctcgccactggaggacttgcggagctcgcgaccgcagttctctttcagcttcaacttcgtcgggaagtcagatcaccacgcgtacgtgacgcagcccttcaccaccggccgtccattgcggctcctcgtcgttgacgatgatcaagtcgtccgcgcaaccacggcgaccctgctggccgaggagcatgaagccatcgtcgagactgaagcagttgccgcagccatcgaggttcccgcccgtgagaaggttgacgtggtggtcacggattatgcgctcgtcggacaaaccggtttggacttcgtcaagcgaacgcggcagggcaggcatcgccaaccggttctttggtgacaggctatgctgatcccgtcgaaagccttccggcggacgtgatacgccaaaacaagccataccgccgtgcagaactgctcgaagctgtcgcgacggcggcaacttcttggaagtcgtaggttcctcgtcaagtctccagctcgagtcgatcaacatacggcagcgaatcggccatcgaggtcaaactgtcgaactgggaacggcccgacgttgcttcaccacctgcgcgccacgcgaagaagtacgagcgtttcgcgagtggctggacggcgcgattgctggaaacgtcggttggcgctgccacagcctgacctgttgccgtccgcaaattcctatgggaaacgccgcatcaaagcagagaggttcgatgcagctattccgcccgatcttgcctggcgcgacaatcatcgaccgcgtcatggcttgcgttggagctctcgtcggcgtcgcggcaacagggctagccgcgcggtgtacgttgggctcagagatctccgcaccgatgttgatgatcgcttcgatgggtgcctccgccgttctcgtcttcgcagttccagcgagtcccctcgcgcagccctggcccgtgatcgggggcaacatcgtgtcggcagccgtcggtgtgtttgtcgctcacctgatcgatgatccgatgattggggccggcgtcgcagtggggacggcgatcgcggtgatgtcggcttctcgctgccttcatcccccaggcggaggaacggctctgatccccgtgctggcaggcttgggcgctcccgcgtctgattggatgttccccctgctgccggttgcgctcaacgccgcgcttctccttggcgtcgcctggatcttccaccgcttctccggacacagataccccaggatcatagcgcccgctcagacgcttcaggtctcgatcaacgacgacgatatcgcccacgccctatctcaactccacgagccgctcgacgtgaatgcgggagacctccggatcattgcgacgctcgctgcggagcatgcccgcagtcgcgcgcgaaccggtcgctgatggttgtatggcggccactgcacttcgctacaacaaagcggaatagctgatcagaacaatcttccggcggttccggccatgatcttcggagcaatctccgggctgcgatgaagcaggatttcatgtctctggggactttgcgcaacaggtgacgattgaatgccaacggtcaattctgtttccacaacaacgctgctcacgcggtttttccgttaccgtttggcaggtctgagcggcgccaggagcggacgttggcacgcctacggattcgagccattcagccaagccggccgaggtcagatggagaacgcctcgaaggcatggagccgaggccgcagagcagccagcacaacttgatgggggtggccgctcagcggtgttgggaaaccgctcgccactggaacgcgacatgctacaggggctctaagcagccttacctctcgcgcatcccaaatctggctaatcggctcccgcatttagaagacgacagccgggcggccacgatccccgcttagttccggatctcaccgctttggtcggttagtttgtacgcgagaacctgtgcgtcctcgattttcggcagcccgtcgagcaattccggggttctggcgacgagcgcacgcccaaccttccccgcgagatgggcgagccgtcccgcatcactcgggaaggtgtcgaaaatggcgaagtcgtcgtggccgaagcgaacagcataccacgtggtcgtgtcccgctcctccataacggccgccaggccgtctcgcaggaaggcctcgacatcggcctccttgccgggcttcgcgcgcaatcgcacgaacagcgccttgttcacaggtgagcgggtttcagcatcggccatcacggtctcctttcgagttcttgggcgtcatggcaacgctccgcggcggtattggctgcgtccataccgaaccgaggtccgcgtcgcaccggcggtagatgactatccgcccgacttttttccgcgttccgctggtcccccggggtggagcaaggcctcggcccctccgctgcggttcggttgcatggcgccaactctccgggttcgagctcggtttgaaggatcgggaattgtggcttgaggcggcgcgacggcggccggtacatcaccaaagacaggccagcgtcgttaggacctgccggctcggcagcagacgtcgccgatggccggcttgagtcagggccggctgtagctgtcgggcgtcttggaaggcgccggaagcagctagcgacacagcggcgaaaaccgaaccttcagaccgcgcctcgttgattgaagcagctgtccggaacggaccctgggaggagctgcaatagcatggccgcgaatacagaagacgagggccgtggaggtcgtccgctctgcctgccgaggcagacctccggcttagtgaggctgggcctctgcccgagctgcgttctgcgtcaagatttctccgacttttgaggctaggtccgttagggcgaacggcttgctgatcatgtccatgccggggtcgaggaagctggtccggacagtggcgttggcggcatagccggtgacaaagagaaccggcaggttcggccggaggccgcgcgccgcttccgcgagctggcgaccgttcattcccggcagtccgacatcggtaatcaggagatcgatgacccgggcggatcgcaggtggatcagcgcctgttcgccgccagcggactgcagcgcattgtagccgaactccgaaaggagctcgacgatcagcgccctgaccgagtcctcgtcctcgacaacgagaatggtttcaccgtccccgggccgagcttcgatgagcgtgccgacattggcgtggacctcgcctgtcgcgcgcggcaggtacatccggatggtcgttcccttgccctcgacgctctcgatgagggcgtgcccgccggtctgccggacgaagccgtagatcatcgaaaggccgagaccggtgccctgcccgatcggcttggtcgtgaagaagggatcgaatgccttggcgagcacgtcggcgggcatgccggcgccggtgtcggagacggagatggccacatagtcgccagaggtcgcgtccggatgccgggccgcaccggcggcgtcgagggacacattgcctgcctcgatgtgcagttcgccgccctccggcatggcgtcccgcgcgttgatggcgaggttcaggatcgcgctctcgagctggttgacgtcgctgaccgctggccagagatcctcgctcccgcgcacgctgagccgcacctgctcgcccagggtccgggtcagcaggtccgtcatggagtccacaagggccgccacgtcgaccggcttcgggtccagcggctgctggcgcgaaaaggccagcaggcggtgagtcagcccggccgcccgctgagccgattgcagcgccgcatccatgaagcggtcgatctcgcccagcctccctgccgcaatccggctgcggatgatctcgagcccgccgatgatgccggtcagcatgttgttgaagtcgtgggccagcccgccggtcagctggccaacggcctccatcttctgcgcttggcgcagctgctcctcggccttctcaagcgcctcggcgcgttccttctccgcggtgacgtcgcggccataggcgtagacgacgccttcctcgacgaaggtgttccaggtgatccagcggtagccgccgtccttgtggcggtagcggttctcgaaactgctgaggttgcgcccggccaacgcctcccccctcgcggcgtcactggacgccagatcgtctgggtgaagcagacgtcggtacccttggcccacgacctcctcggcctcatatcccagcgacctcctccacgccgggctgacggcgcggaagttaccgtcgggtccgatgatcaccagcaggtcgcgcgaattgttccagacgcggtcgcgttcgcgcgtccgctccgtcacccgctgttccagcgtggcggtgagatcgcgcagacgggcctcggccgtcttgaagtccgtgatgtcgtggatcgctccgatgaagcgctccgcgccaccgggtccgtccttgcgatgctcgccccggcgggcgatccagcgctcctcgccagtgtcggcgcggatgatccggcattcgcggtagtccatggcgcccccagcggggagctcgcctccgccgatcagcttcggcgaccccagcgcgaccgtggcgttgaccgctctcagagccacggcgtccgtcggcgtcagccccagaagccggcagaactgctccgaaacctcaaccgtgccgaagccgctgacgtgctcgaacgtccccacgcctccggccgactgcgcgacccgcagccgttcctcaaggcgcttctgcgcggtgatgtcggtcaggacgccgctgaaggtcagcacccggtggtcgccgtcgcgctctgcctcgccggtggcggacacccagcgaagctcgccggccgaggtggcgaggcggaaggtcttggcgaagacatccgccccgtgcatcaggccggcgacggcgatgcgaatgcgcatccggtcgtcggggtggatcgcggagaagaacgcgtccgtgtcgactccgcccgccaccgcttcccgcgacaggccgtacagatcggcgaaacgggcgtcgccgtagaggcggccgtccgccacgctccacagccacatgccggcggctccggccgttagcctggcgatgcgggggttcgccgggcccgatgatccctcgagcgtcatcggagctagccgagccggccgaggtcgtcggcagtcatcacacgttcaatgaactcgccgatcaacaccttcagggcctccagcgagggcagatccatcagcatggcgatgtagccgcggatgtcgcggccgctgatcgagaaattaatgtacaggaacaggaccacgccctggtcgtcgtcccgggcggacagttcgaagaacaagtcgccgttgccgcgcatgacctccggcagcgacatgctcaggggccgcttgagcatgttggccatggtggccaggcagccgttgaggaccacgttgccggtctcggcgagcgcctcgccctccatggcgagcgcgtccttcgcgtccagctcgtctccggtgacggcctgcacgagcgccaggctgttcgactgcgggaagatcagcagggcccggccggaaaaggctccttcgaagtcctggcgcaccgcgacaagctcgccgctctcgcgttcgcggatcagggtcgcggcggacttgcggctcacgacctcgacggatgggaccgacagagtgacttgttcgccaaccatattccgcagactggcggccgcgcggcttacgccgatgttgaccagctcggtcaaagcgtcgtgttcaagctccgaaagcacgaccgtcgcgccgctcatccacgttgacgcagcttgagcgccgcgccggaaaggaagcccttcaagccgccctcgttgatcggcttgggaatgaaggtcgcattgagccgccgcgcctgtgcgatgatctcgtcctgcacgttcgccgtcgccagggcgatcggcatctccgcgtccacgccgcgaatttcgccggccagttccagaccgttccgccccggcatgttgaagtcgacgatcgttacgtcgatcccgcccgccgcgatcatggccaaggcctcgtcggcgttggccgcttcctgcttgttccagtccggctgcagcgccgctatcgctttgctgacgacgatgcgggccaacttgctgtcgtcgacgatcaggacggtcggtgtcattcggatcgctccatcacattcgcagcttccagaatcgaccctgccgtcgtcacgcaggcctcggccagcgcaggtaggacaaatcggatcaggaaaccatcctccggggcgccgtccagacgcggctggaagcgaagcagagcttgaaccacggcgctgtgcagttgtcgaccgtgcgagacgtcgacccgaagccccccccccccctccagcgcgcgcacaagcggctcggcgtcctcgaccccgcactcgccttccaggaagatgacatcgccctcgatcctcacactcatccgaccaacgcctctggatcaaggatcatcaagacctgcccgtccgccagaagggtggttccggagacaccgggcatgcccgccagcaggccgtccagcggacgcaccgccagatcggctcgttcccgtatcgcatcaacggccacgcccgcgatgcggccgccggaccgcaccaccagcactgtgcagtcgccggtcaccggtcctccagggccgccgactagcgcggcaagggtcagcaggggcacggtgcgattccgccagttgaaggcctggcccgcgcggatcgggatcacggcctcggccgggacgcgaagcgtctccagcacctcctccaggggcaggccgtaggcctcaccctcgctcatcaccaccatgatccgggtcagcgtcagactgagcggcagggtgatgcggacggttgtgccccgcctgggccggctgtcgatcaggatgcgcccgcccaggcgctgcaccgccgctctgaccgcgtccatgccgacgccccggccagagacgtcggtgagcgccctcgcggtggagaatcccggcaggaagatcaggttgaccgcctcagcgtcgccgagcgcggccagcgcctcatcggaaatcaggccgcgggagcgcgcggccgtgcggatcgcctccggatcgatgcccgctccgtcgtccgccagcgtgagttcgagccggccgcctcccgcttccgccgtcagccggatcgttccccggcgcgcctttccggcggcctcacgcgctgccggcggctcaacgccgtggtcgatggcgttgcgcaccagatgggtgagaggttcgaacagtccttcgatgatagtcttgtccgcttcgacgccgttgtcctgcgcgatgaagtcgatttcccgccccagcgatcccgccagctcgcgggcgacccggggaaagcggcgaaggaggggggcgagcggcgtcatccgcagggcggtgacctgccggtgcatccggccgaccagccggtccaggtttgcggaatggaccgccagttcccgcgacacttcggcctgtccggcccctttgtcggcccgggaggacagggctgccagggcggtttgggcggcgaccagttcatccatcatgcccgcgagcgcctccacctgcccggcgtcgacccgaagggtgcgcgcgcctccgcccccggcttcgccggaggaggcttccctgtcactggcaggcgcggccagggcgacgatctcgacctgatcgggcacgaatcgcagcgcggcgcgggcctctggcacggcggcggtgctcagggcctcaatgacaaggcggcaggtgaaagggtcgtagacgcccccctccgcctcccgcagtcccagccggagatgaaccagctccggaacggttccgatcagcccgagcggatcatcgccgctgaaataggaaccctccgccgggacgtagcggatcgccgtcacggcgtcagacccggggtgaccctgacgcaggaccgtcgcccagccggggacggcgccggaggagagggtcgtggccggctccgcctcgtcctggccgaggcgtcccgcaagccttcgagcgacctcgccggcgtcggacggaagaccgcccccaccctcaaggaccgcgagccagcgctcggtctggacaaggacggccagcagcgagtcgatatcagggcggtccgcgctccgcacgcccgaccggatcgctccgagcacgtcctcggccgtgtgcagggtcatggccatgggcggcaggtcgaacagcccgaccgagcccttcagcgtgtggatggcccggaaggcgtcgtccattagcgcccggtcgtccgggttccgctcgagggccagcagggcgtcgctgccctgctgcaccagttcgggcgcctcgatcaggaactgggcgagcagctcgtccatcaggcggacggccgctggtagacgatcgcatccgggaagcgccggaccgtgaagcggtcgctgatccgcgacatggactcggtgtgcccaaggcagatgaagccgccgggcgcgagggtgtcgtgcagatggccgaccgcctgcgcccgcgattggtcgtcgaaatagatcaacacattgcgacagaagatgacgtcaaagacaccgtgggctttcatcgactccgcgtcgatcagattggctttggtgaagattacggatttgcgcagatcatcgatgatgcgccgacgtcccttccccgcgggttcgaagtaggcgtcagcgactggctgcggcagccgactgagggcacggtcgccgtacacgccctcgcgggcggcccgcagggcatcgccgtcgatatccgacccgacgatctcgatattgtaggcgtccaccatccgccagttctcgagtagccacagcgctatggaataggcttcttcaccggttgaacagggctgggaccagatgcggatcctgtcccccggtccccgggtccgggtgatctcaggcagcaggttctcgctcagacagcggaactggtgctcttcccggtagaagtaggtttcgttgacggtgaagctgttgatcaccgtcgccgcctcgccggggtcggagcgcagcagcagcaggtagttggcgaacgacaaggccccggtcgccgccagccgctcgtgcagccgccgctcgatgtagtagcgtttggtctcgccaaactgcatgccggtgcgggcgtaaagaaattcgcagaagcgccttagctcgtccccggtcagaaccggcgcgatgtcggagggatggaccatcaggagcgccccgcgagctcgagcaggccggcggcgacccgatccagcgacaggaccgcctcggcgccgcccgcgcgcaccagttcgccgggcatgccccagacgacggcggtgtcctcggcctcagcgatggtccggccgccgccctcccgcacccgggtcatcgccgccgcgccgtcattgcccatgcccgtcagcagaattccgacgaggtccgtcgcttcgacgtgatccaacgcgctgtcgaccatccggtcgacgctcggatgccagcggaaggcggtgctcgacggggcaggcagagcgactaggtccccgccgcggcggctgatgatcagatctgcgtcgccccggccgatgtagacgcagccgggctcgagcgtcgtgggccgggccacctcactgactgcaagcgcgcaaagccggtccagccgaccggcaagggctccggtgaagctggcgggcatgtgctgcgccactacgatcggccacgggaagtccgccgggagcgggctgaggagcgcgtccagcgcgggcggcccgcctgtggaactgccgaccagaaccagccggccggctccggcgccggccatcggcgatagacgagtgcgtctcgccggcgccggccgggccccgggaggcggccggagcttcgggacccaggtctcgctccgggcgcgcacccgctccgacaggcggtggctgcggggaagccgcgcctggaacgccgcgcgcaccttctccaccagaaccggcccgaattcgtcgatcttcagcgaaatggcgccgcccggcttggcaacgaaatcaacggcgcccagcgacagggcctccagagtctcgcgggccccgtcagcggtcagggcggagaacatcaccaccggacagggtcgctcgagcatgatccgatccagacaggccagcccatccatgcggggcatgtgaacgtcgagagtgatgacgtccggactgaactccgcgagcatcgccagcgcctcgacgccgtcgcgcgcgaaacggacatcaaatccctcctcgtccgcgaacacctcgccgatcagccgccgcatcagggcggagtcgtcgacagccagaagtcggatcacggctggtccgacaccccggcgtccatgccggccagcaggtcgcgctcggcgcggtcgagcatttcgcgtggctcgatcagcaggatcagcctctcgccgccgtcgagggtcgcgacccggctgaacagccggccggcgtcggcggccatccccggcgtcggctccatctggcgccggccgatatcgacgatccctgacaccccgtcgacaatgaaacccgcctgccggcgattaacggtcgtgaccacgattcgggggcgcgcgccggtcgtcgccgcctccgcctggaagcggctgcgctgatcgatgatcggggtgacccggccgcgcaggttcaggacgccctcgacgaaggcgggcgccttgggcacgcgggtcagccgctcaggcaggcggaccacctcgtcgaccgcggtcagcggcaggccgtactcgtcgcctccgatccggaagatcagatagcggtcgcactcgtcggccaccgcgttctcgtccatctcgccaacctcgctgcggccgtcggccaggatgcgcgcgaccttctcgtcgcggaagagtcgttcggcggagaggagggcgaccagtccgcggccgtccggcagtcggcagatcgcctgaacctgcgcctcaccctcgccgcggttcagcacggcgggcgcggcgtcgatgtcggtttctgacacccggaggatggcgtgcaggcgctccaccgccagaccgacgatcgcgtcgccgacgcgggtgaccacgatgcgtcccgcctcgtccgcccctgccccgaggcccagcagccgccgcaaggagaccaccggcaggagtcggccgcgcaggttgtgcacgcccagcaccgcgtcgtcggagccggctacggcggccagccgctccggcaaggtaagaacctcgctgacctcttccagcggcagggcgtaggtctggcccatcaggtcgaacgccagcagcgcggtccacgcttccgcttccgcttcggcttggtccccgcccaccgtcggatcgaccgccgcacgccgctctgcgggggcgcgggcgaactcacgacgcagcagaccctcgagatcgagcacccgcagggcggaatcctcgaccgcatacaggcgcccgaacgccgctccggcccccacattcttcggcgccggcaggtgggcgagcgcgccgacacggtcgacggaaaggccgatagcctcccggccggacagcagaaggaggcgggactccggacccggcgtctcctgccgcccgagcaggcgcgccaacgaggccaccggggcggccgcgccgcgcaggccggcgatgccgagcaggcccggcggcccgcccggcacacgggtgatccgcggccgacggaagatctcggacacgtccgccgcgtcaacggcgtactggtcctccccgacgaagaaggtgatatagggactggtctccgcggcgctcacctaggcctcgcggctccgcagctcgtcggccagggaggcgatctcctcgatggcggcggcgagatcctcggcgccgcgggattgctggcgcgcggctgctccggcctcggcggccgaactggtggcctcctcggcgaccgaggcgatctgggcgacccccgccagcacctgctcgaccatcgagagggaggcgtgcgcagcctccagaacttcctgcccgccggccttcaaatcgtccgcgacgctcaccacggcggccagacgatcgtccagcttgcggttcttctccgcctccgcccgggtgacggcgccgatctgctccaggtccctggacacgagggcaatctgcccctgcatctggcggacgatgtcgccggcgcgggcggcgttgtcgccggacgcccgagccagattgcggatgtcggtagacaccaccgagaagccgcggccctgatcgcccgcccgcgccgcctcaacggagccgctgacggcgagcatcgtcgtctgcaccgccaccagcgccatgccgtcgatgatccgctcgatcgcgtgcgcggaactctcgagcaccccgaccaggtccagcagctcgccgatctcggctccgccaccggcgacgccctccgccagcttcagcaccgcggcgcggctgccgcccagctgcgacagagatcgctcgatctgctgcacggactcatcgcccgcgtcgcgcgtggccgcgaccgacctctggatctgcgccatcgctgcattggcctgctgggtcgccgaggcctgaatctgagccccgcggccgatctggtcgacggcggtgagaatctctccggcggcgccggccagctcttggattgtcgcagaaagctcctcggcggctgtgcttacctgttccgccagtccggcgtcggcggtgtcggaccgaagaccctccgccagctccgccagcgactcggcggtggcttggctctcatccagcgaggcgctctgctgctggaccgcgcgctgggcctccgcggctccggcggcctgctcctcggcggcggccgcgacgctctccgagcccgcctgggcctcccgcgccgccgcctcgatctcaacggcggcggtcaggatcgtcttgctgccgctggcgatgacacccagcccggcccggacctcttgcagatcgcgctcgatgacccgccccgcccgcgcctcggccactgcggcttcggcggcggtcgcaatccggcttgcgatcgtccgcacgtcctcgacgatccgcgtcgtcagtcggccgacctcgcgcgaccgctgctcggcgacctcggccagacccctgacctcgtcagccacgacggcgaagcctcggccgtgatcgccggcgcgcgcggcctcgatggctgcgttcagggcgagcaggttggtttggtcggcgatgtcggcgaccgccccggccacctcgccgatcgacgaggcgtgctcctcgagccgtcgggtcagttcgatcgatttcagctggcgttcggcgctggtctcgatcgcctcgagcgaggcctcgacgagcgcggcggcctcccccagctgtccctgcaactgcaggctgcggtcgtgcgaacggtcagcccgggtccgggcctgcacgaaggtggaggccagagcggtgatggcggccagggactcgtgcgaggcgccggccgcctcctcggccgcggtggagatttgctccatcgatcggcgcagctcctccgccgcgcttgcggcctcggtgagtccgctggccagttcctgagtcgcggcggcgagccgctcgggggcggcctgacgcgagcgcacccgctttccggacttcgcgaccgcccgcgccggcgccggcctgacgtcctcggccagcttcaccggggccttggaccgccctctccccgccagcgcagaggtcttcaccaacgccattcatcgcctcgccgcatgtcccctgaccggcacggcgccgcaagaggtggatgtcggaacggtagaggcttgcgaaagggcccacaaggggcggttcacgctccgtcgggcggggcagcttggggcgccgtacgccatttcgatcactgcgcgctcaccctcaagggctcggcaccccaccaagacctcatccgctcctcaccaataccgggcgcgcactacactcatgttcctgtgccggccgaagagcggaccttccgaacgtccgtcatgagccgataccgttgaaaaagtcggcaattgccacgggcggcgagtgctgattcactctggtcattgaggctggaggcagcgcgatgatgggcgagcggcgggtcgatcaggcggccctgttctatactttctcgctggaagaccacgtccctgcgaaccatctgctgaggtcgatcgaccggttcgtggagttggaaggtctgagagggcatctggcgccgttctacagcgccatgggtcgcccctcgatcgaccccgagttgctgatccggatgctgctggtcggctattgcttcggcattcgctcggagcgtcggctgtgcgaagaggttcacctgaacctggcctaccgctggttctgccggctaggcctcgaaggtgccgtgccggatcattcgaccttctccaagaaccgccacggccgctttcgcgacagcgatctgctgcgccagttgttcgacacggtgctgcgccgctgcatggctgaaagcctggtcggcggcgaaggctttgccgtggacgccagcctgatcaaggccgaggcgaaccgggaacgcagcgtgcctggcgatccgggccttccgcccgaggcgtcgagccgggccatcgacgagtatctggcggtgctggacgacgcggcgttcggtgcggctactccggtgacgcccaagttcatctcgccggtggatccggcagcgcgctggaccgccgccaacaaggggccggccttcttcgcctatgccaccaactacctgatcgacctgaagcacgccgtcatcgtcgatgtcgaggcgtccaccgccgtgcggccggctgagctgacggcggcccgcaccatgatcgagcgggttcaggataggcatgatctccaccccgaccgccttgccgctgacaccgcctatggctcggccgagatgctggaatggctggtcaacgaccaggggatcgcaccccacatcccgatcatcgacaagtctggccggacggacgggaccttctctcgagccgacttcacctatgatcccaccgccgacctttatcgctgtccgggcggcaaggcgctgaagcagtatcggcgtgccttccgagccgatcatcccgagacgccgccggatgacacctatcgctatcgcgcctccaagatagactgcgacgcctgcgctctgaagccgcgctgctgtcccaacacgcccgcccggaaggtcacgcgctcaatccacgaaggtgcgcgggacttcgctcgcgacatcgccaggaccgacgcctacgtcgtttcacggcgcgagcggaagaaggtcgaaatgctgttcgcccacctgaagcgcatcctcaggctggaccgactgcgtcttcgtggtccctgcggcgcccgagacgagttcctcctcgccgccaccgcccagaacctgcgcaaaatggctcgactgatcccgcaaccgaccgctcccacgcccgcctgaaggcctgaagcgtcacgatcccatcacagcctgaccacgcagccgtgctgtcccgtcagccatccgactttttcaacggtatcagccagaagcggctatcgcgccaacaaatgtccgagtcacacgcgcataaaccgcgacccgcgggctcaagcgacgctttctggctagtttctggttagcacttctgaagcggtcgagctaagtgtctgaaaggaatggtggatgcgacagggattgaacctgtgaccccctcggtgtgaacgaggtgctctcccgctgagctacgcatccggccgcttgggaggcggcgacatagcctgatcgcgcgagacgcgcaagcgccgcgtcaggaaagcgcttgctccggcgccgtgcatcgtgtggaggaacgactgtttccttgcttgccgatccgagttcccgtgaccgcatccgacaatccgcatctcgatcgccccttgcgctcctttgggcgcatcaaggcgcggccgatcaagccgcgtcaggcggccttgatggacaccctgctgccggcgatcgccgtgcctgatccgaaggccggcgcggtcgatccccgcgccctgatgccgcacgcaaaggaagtctggctggagatcgggttcggcgggggcgagcacatggcggcgcaggccgcacgccgtcccgacgcgctggtgatcggctgcgagcctttcctgaacggcgtggcctcggcgctgcgacacgtcgaagaaggcgatctgaagaacgtccgcatccacgccgacgacgcccgcgacctggtggacgccctgccggacgcctcggtcgaccgggtgctgatcctgtttcccgatccctggcacaaggcgcgccacaacaagcgccgcctgatccaggacgagaccgcccaggccttggcccgcatcctgaaacccggcggtcggctgcgcttcgtcaccgattggaaggactacgccgactgggcgctggagcggctcggccgcacgcccggcctgcgctggctggcggaagaggccgacgactggcgcgtcgccccgcccgaccacgtcgtcacccgttatgaggagaagaagctcggcgacacgccgccgatctttctggagttcgagcgggagtgaccaaaacctccggcaggatcgacgcccttcgctttctgatctgcgccctgcttgctcccgggacgtcggtcatcatctgcgggcttctggcgcacatgctgccgcaagacgccgagggattgagggcgctggagccggcgctgctgctgaatcccttcgcctttctgctcgtctcggtgctgggcgcgccgtccagcgtcatcttcggtctggccgggcgccttctggcggagcggcgtctccagggccgccccctttggctctggggcggggccggcctcgtcgccgccggcgtctatgcggctctggggacgctgctgcaccggatcccggcctttgatatcctggcgccctgggccggcatgttgcgcgagcctgagccctggagcgtcgacgcctgcatcatcgcaagcatcctggcgtccggcctgatcgcgggaaccgcctaccggctggccagccgagaagtctaggtcggcttcacccgctcatagattccggtcagcacccccttggccagcaccgacttgacgatggcggtcttcacctcgtccttgccgggcttgtcgtcccagtcgaccacgcggttcagggcgaagacctgaaacaggtagtggtgcggaccgtggccgggcggcggatcgttcggcaaccagccgacgccgcccatggagtgcttgccgagacgtgcgaggctggagccgtccttcagcccgccttcgcccacgctcgtcaccgcggcgtcgaacacggcgatcaggtgaatgaacggttgaggcgccggtatgtccggatcctcgaccaccaccagcacctgctttgtcccctccggcaggttggaccaggacaacggcggcgacgttccctcgccgtcagcggtgaatcgcaccggaatggcgccgccgtcggagaaggccgggctttcgacctggatggtttcgggggcctgggcgccctcctcgttcagcagcagcttgtccacgcccgcgcgcacgccgcccagcgccttgccgaggctcgccggtatcttctggaacatgaggtcctcacgtctgatggtgcagaccaagagaacccggccacggccgttcggttcgccgcaaccgcgcgaacaacagggctgacaacccgacaaaagccgcctataagcgccctacatcgttagaccggcgtccgacgagacgccgtttccaagcggcggcccggacggctcgccgctttttgtttggacctgaccttgcgcgcaaagaccgccgaagaccgcgccctgctggagctgatcgaccctgtggccgagagcctgggtcttgaggtcgtgcgggtgcggctgatgggcggaacgctgcgtcggcgcctgcagatcatggccgagcgccccagcgaccacgacatcgccgtcgaggagtgcgcgcgcctgagccgcgccgtctccgaggtgctggacgccgccgaccccatcgccggcgaatacctgctggaggtgtcgtcgcccggcatcgaccgcccgctgacccgtccgatcgacttcgagctgttcgacggcttcgaggcgcggctggagaccgaccgcatgatcgaggggcgcaagcgcttcaagggcgtgttggccggcgtggacggcgacaacatcgccatcgatctggacggagaggacgaaaccgccctgatcccgttcgactggctggccgacgccaagctggtcatgaccgacgccctgctgaagcgcggcgccgcgatccgcgcccagcgcggcgaacctgaagacgacggcctgcccgagggttcggccgaccaagacaccaccacgaccccctctgaggacaacgcctgatggccgtcaccggtatttccgccaaccgtctcgaacttctgcagatcgccgactcggtcgcgcgcgagaagaacatcgaacgcgagatcgtcatcgaggccatcgaggaggcgatccagaagggcgccaaatctcgctacggcgcccaccacgacatccgcgccaagatcgaccacaagaccggcgagctgatgctgacccgccacgtcacggtggtcgaggacgactggcagccggaagacgagctggaggagttcaacgacagcgccatggtgcgcctgcgcgacgcctccaagcgcgatccggaggccgaggtcggcaaggaatacgtcgaggtcctgccgccgttcgagttcggccgcgtccagacgcagatggctcgccaggtggtgaccggaaaggtccgcgaggccgagcgcgccaaccagtacgaagagttcaaggaccgcgtcggcgagatcgtcaacggcacggtcaagcgcgtcgaatacggcaacaccatcgtcgacctgggccggggcgagggcgtgatgcgccgcgaccagtcgatcccgcgcgaggtgttcaacatcggcgaccgcatccgcacctacatctatgacgtgcgtccggaggccaagggtccgcaggtgatgctgtctcgcgcccaccccggcttcatggccaagctgttcgcccaggaagtgcccgaggtctatgacggcgtgatcgagatccgcgccgccgcccgcgattcaggctcgcgagccaagatggcggtgctgtccaacgacagctccatcgatcccgtcggcgcctgcgtcggcatgcgcggctcgcgcgtgcaggcggtggtcgccgaactgcagggcgagaagatcgacatcatccagtggaacccggatgagccgaccttcatcgtgaacgccctggccccggccgaggtcgccaaggtggtgctggacgaagaggccggccgcgtggaagtggtggtgccggacgaacagctgtcgctggccatcggtcgtcgcggccagaacgtgcgcctcgcctcgcagctgaccggctggcagatcgacatcatcaccgaatcccaggactccgagcgtcgccagcgcgagttcaccgagcgcaccgccctgttccaggaagcgctggacgttgatgaggtgatcgcccagctgctggtcaccgaaggctacgccacggtggaagacctggcctatgtcgaagcctatgaagtcgccgagatcgagggcttcgacgaggacacggccgaggagctgcaggcccgcgcgcgcgagttcctggatcgccaggcggccgagctggacgccaagcgcaccgaactgggcgtcgaggacggcgtgctcgaggtgccgggcgtgaccttggccatggcggtcgccctgggccaaggcggcgtcaagacggtcgaggatctggccgacctggccaccgacgaaatccgcggcggctacgaggtgaagaacggcgaacgggtcaaggtcccgggcgtgctggaaagcttcaacctggcccaggaagacgccgagttgctgatcctgcaggcgcgcgtggcggccggctggatcgacgcctcggaactgcctcagcccgagcctgagtacgaggacgagggcgaatacgccgagggcgaatacgacccggatcaggtgttcggcgacgcgcctgcggccgatgcgggcgacgacgcggaggccgccgacacctccgagccgacgcgcgacgcgtgatggagaccctgaccgttcatgagcctgcgcgacgcaacgatcgatagggaacgccgggatctggcttcgcaccaggtcatggacgagtctcgcttgatccgttttgtcgcggggccggatggtcaggtggtccccgacctgggacgcaagctgccgggccgcggcctgtgggtcgcggccgaccgcgcctccgtccagacggcggcgaagaagaacctgttttcgcgtgcggccaagactcggctcgcagcatcggacgacctgccggacctcgtcgaacggctgctgcatcggcgctgtctggaccagctgggtcttgccaggcgcgaaggcgtgcttatctccggcttcgaaaagtcggcggcggcgatccggtccggacgcgcggcctgggtgatcgaggcctctgacggctcggccgatggtcggggcaagatcctggccttggcctctcacggaaccgcacgaatctgcggcgccttcaccggcgacgatttgagtttggcccttgggctggaaaatgcgatacatgcggtcctgcttgcgggcggacgcgccgatcgctggaccgtggaggtcgaacgactggccggcttccggccgcttcgaccgatccattgggaccatcccggaggcgaggacgatacggctggagcgcgcccgacccaggcaacgggatcaggggcgagctgaggatttcggcgggcatgggcctgtctccagggacggagacgggctcacgcccgtttatgtgcattgagcgacggcgggcttttccgccacgagtaaagcgaccggatgagcgacgagaacgacaagaccaacgaaggccagggcgccaacaccggcggaacgccgtcccagtcgggaccgcgcgcaccgctgagcctgaagccgcgccagacgggatcggtttcgaccggcaccgtcaagcagagcttcagccatggacgctccaagacggtggtcgtggaaaccaagcggcgccccggcgcggccggcggtccgcagcggccgcagggcttcgatgtcgcgcgtccgcgccctgaccaaggccagccgcgcccgcagggccaacggccgcaaggctcgcccgccggcggcgccctgtcgcccgaggagcaggaggcgcgccgccgcgccatcgcgctcgccacccacgcccaggccgagcgcgaaaaggccgccgccgccgacaaggcgcgccgcgacgccgccgcccgcgaacaggcagaggccgccgaacgcgccgccgccgccgcccgcgccgaagccgccgccgccaaggccgccgccgacgccgcgcgcgccgaagccgccaaactggccgccgccgcacccgcgcccgcccacacgcgtccggctgcgaagcccgccgccccgctgcctcgacaccggcgcccgcgccgacgcccgccccgcctcaagccgccgctcccaccccgccggcgcgtccggccgcgccgccgcgtccgcaggtcaacttcggccagcgcacgcccaagccgaacaatccgcagcgcgcaccggtcgaacgccccgccttcggcggtcgctcggctcgcgaacaggccatgggcggcggcgagcgcgcctattcggaccgtccgcagggcgcaggcgccggtcgcccgcaaggcgccggtgcaggtcggccccagggtggccccggcggtcgcccgcagggcgctaagccggctgagcccgtccgctattccgcattgaacccgcgcccggcgcccggcgccgcccgtccgggcggtccgcgcaccggtcccggcggccgtcccagcccgaaccagccgccggccgagcccaacgtcgcccgcccggtccgctcgggcgcaggtttcggccgtcctgtcggccgcgaggacgatcgcgacaagcgcttctccgacgccggtcccggaaaggcggtcagccgcacccgcggcgagcccaagcgccgcgaaggccgcatgaccatccagtcggtggtcggcgacggcgacgccgccgagcgcatgcgctccctggcctcggtccgccgcgcccgcgaacgcgaaaaggaaaagcgcaagggcggctcgaccgacgcgccgaaccgtccgcgcgaggtggtcatccccgacgtcatcacggtgcaggagctgtccaaccggatggctgtgcgcggcgtcgacatcataaagttcctgatgcgtcagggcctgatgatgaagatcaacgacgtgatcgactccgacaccgccgagctggtggccgacgaatacggcatgaccgtcaagcgggtgtccgaatccgacgtggaaaccggcttcatcgccgaggccgacgacgccgaggcgtccgagacccgcgcgccggtcgtggccatcatgggacacgtcgaccacggcaagacctcgctgctggacgcgctgcgcaccaccgacgtggcgggcggcgaagccggcggcatcacccagcacatcggcgcctatcaggtgcgcctggaagacggccagcgcgtcaccttcctggacacccccggccacgccgccttttcggcgatgcgggcgcgcggcgccaacgtcaccgacatcgtggtgctggtggtggccgccgacgacggcgtcatgccccagacgatcgaggccatccagcacgcccgtgcggccgaggccccgatcatcgtggcggtcaacaagatcgacaagcccggcgcgacttcgcaaaaggtcgtcaacgagctgctgcagtacgaggtcatcgccgagagtctcggcggcgacacccagatcatcgaggtgtcggccaaggaacgcatcaacctggaaggcctgatcgaggccatcctggtgcaggccgaggtcatggacctgcgcgccaacgccgaccgttcggccgaaggcgtggtggtcgaggccaagctggacaagggccgcggcccggtcgccaccgtcctggtcaagcgcggcacgctgcgtcgcggcgacatcgtcgtggccggcggatcttggggcaaggtccgcgccctgctgaacgagcgcaacgagcagttgcccgaggcggggccgtcggtcccggtcgagattctcggcctggacgaggcgccttcgcccggcgacgtcttcgccgtggtggagtcggaggcccgcgcccgcgagctgaccgagtaccgtcagcgggtgaagcgcgaaaaggctcaggtctccggcggctcggtgtcgctggtcgacatgatggccaagctgggctccaagaagatcagcgaactgccggtggtcatcaagtcggacgtccagggctcgggcgaggccatcgcggcttcgctggagaagatgggcaacgacgaagtccgcgcccgcatcgtcttctcgggcgccggcggcatcaccgaaagcgacgtcaacctggccaagtccgccggcgcgccgatcctgggcttcaacgtccgcgcctccaagcaggctcgcgacctggccgagcgcgaaggcgtggagatccgctactactcgatcatctacgaccttctggacgacatgaagggcgtgctgtcgggcatgctggcgccgctgcagcgggaaaccttcctgggcaacgcccaggtgcttcaggtgttcgacatctccaagatcggcaagatcgccggctgccgcgtcaccgagggcgtggtccgcaagggcgcgcgcgtccgcatcatccgcgacgacgtggtggtgctggaactgggcgtgctcaacacgctcaagcgcttcaaggacgaggtcaacgaggtgccctcgggccaggagtgcggcatgcagttccagggcttccaagacatcaaggaaggcgactacatcgagtgcttcacggtcgaagagatcaagcgcactctcgactagaacagctggaaggcccggagctcaggttccgggccttttttctgggctactcgtcagccgtggaaacggtcttcgataatggcggcgaacaggccgggatcgacgttgccgcccgacagcacgatggccgtgatctggccccgcgcctcgatcttgccggcaagcagcgccgccagcgaaaccgccccgcccggctccaccaccagcttcagctgacgaaaggcgaaacgcaccgcttcggcgacctccgcgtccgaaaccgtgatcgcccccgcgagccgccggttaatggcaaaggtcagctcgcccggcatgggcgccatcagggcgtcgcagatcgagggcgcgcccgtcggatggccgacgcgctctccggcccgcaatgaccgggcggtgtcgtcgaacgcctccggctccaccacgatcacgcgcgtgtccggactgcgctcggccatgaccaggttgatgccggcgatcagcccgccgccggacgcaccacacagcagctggtccagcggtgcatccgcctgctccagcaactccagccccaccgtgccctgaccctctatgacgaagggatcgtcgaacggcggcaccagcacgcagccgcgctcccgagccagggccgcgccgatctcctcgcggctctcgctccagcggtcgtacatccgcacttcgccgccgaagctcagcaccccctcgaccttcacgcgcggcgagtctgacggcatgacgatgaccgcgggctctccgaccaaggccgccgccgccgccacgccctgcgcgtgattgccggacgaaaaggccacgaccccacgctggcgctcgtcctcggtcaggcggctgatgcggttataggcgccgcgaaacttgaaggcgccggccctctggaccgtctccgccttcatcagcacccgcccgccgacacggtcgttcaacgccgggctctcgatcaggggtgtgcggacggcgacgccatcgatctggcgggcggcgtctaggacgccctggaagctgggaggtgtcatgcgcatccctccccttaccgcagcgccgatcccacgcgtaaggtggccgacagggagaaacgaaatgagcctgatcctcgccatcgaccagggcaccacctccacccgcgccatcgccttcgaggtgcggggcggagaccttcagccggtggctgtcagtcagatcgagctgacgcagcatttcccacgctcaggctgggtcgagcatgacgccggcgagatctggcgggcgacgctgcagacctgccgcgaggtgctggcgaccgccggcggtgcggcgcgtttctcctcgatcggcctgaccaaccagcgctagacggcggtgatctgggatgtcgccacgggcgagcccctgcatcgcgcgatcgtctggcaggaccgccgcaccgccgacgtcaccgcccgcctcgccgccgaaggccatgagcccggcctgcaggccgcaaccgggctgatcctcgatccctacttctccgcatccaagttcgcctggctgcttgatgcggttccggatgcgcgggcccgcgccgaggcgggcgaaatcaagctgggcacgatcgacagctggctgatctggaagctgacgggcgggcgcgtccacgccaccgacgccgccaacgccgcccgcacctctctgatggacctgcggacgctgcaatggcgagcgaacctgtgcgccctattcgacgtgccgctggcggcgctgcccgacatccgcccctgcgccggcctgatcggcgagaccgagccgtcgctgttcggccgctccctgccgatctgcggctcggccggagaccagcaggcggcgctggtcggccacggcgcgctccaggccggggacgccaagatcacctatgggaccggggcgtttctcgtggccaatgtgggaccgtcgcccgtcgcctccacacgccggctgctgggcacgctcggctaccaggccaacggcgtgaccgcctatgcgctggagggctcgatcttctcggccggctcggcgatccagtggctgcgcgacggcgtgggccttctggacgagtcccgccagtccgaggccatggcgcagggcctgcccgacaacggcggcgtctatctggtccccggcttcaccggcctgggcgcgccctggtggcggccggaggcgcggggcgtgatcgtcggcctgacgcgcgacgccggcccggcccacttcgtgcgcgcggcgctggaggcgctggcctatcagacgcgcgaccttctggacgccctggcggaggacggcgcaccgccgctgaccacgctgaaggtggacggcggcgtcaccgccaacagcttcgccatgcagttcgtcgccgacatctgcgaggtcgaggtggtgcggccggcctttcaggagatgacggccctgggcgccgcccggctggcggcgctcggctgcggcctcctggacgatctggaggcgcgccctcgcgaggcgccggcgatctggcgtccccgcatgggcgccgaggagcgcgggcgtctgctccggggctggcgccgcgcagtgcgggccgccatggtcgcggccgaagacgatggagaggccgcccgatgaccgaggctcaagacgatgcccaggccgccttcgccggcgtccgcccggtcgatccgcgccatgcgctggacgaggcggcgctcggccgctggctggcggatcatgtcgagggctatgccggcccgctgacggttcatcagttccgaggcgggcagtcgaacccgacctatcggctgaccacacccgaccgaacctatgttctgcgccgcaagccgtccggcgccctgctggcgtcggcccatgcggtggaccgtgagtttcgtgtcatatcggtcctgcacgcccaagggtttcccgtcgcccggccctacgccctgtgcgaggacgagggcgtgatcggctcggtcttctacgtcatggccgaggtccagggccgcatcttctgggacctgaagctgccgggcctgcaaccggccgagcgccgctccatctaccaggcccaagtgaacacgctggcgcggctgcacgcctttgatccggcggcgatcggcctttccgactatggccggacaggcaactatttcgagcgccaggtgtcgcgctggaccaagcagtaccgcgcctccgagaccgcgcccacgcccgccatggacaggctgatcgcctttctgcccgaaagcctgccgcccgagggcgagacccgcatcgtccacggcgacttccgcctcgacaacctgatcctggcgcccgagacggccgaggtgcgggcggtgctggactgggagctgtcgaccctgggcgatcccatggccgacttctcctatctgctgatcgcctgggccattccggcgtccttgaggaacggcctggccggcgccgatctggaggcgctgggcgtcccgtccgtcgcggagatggtggagctgtatgcagcgcagacaggcgcgcgaccggtcgatctgccgtggctgttcgcctataatctgtttcggctggccgcgatctgccagggcatcgccggaagggtgcgcgacggcacagccgcctccaaccacgcccgcgccatggcggcgcaggtccagccgcttgcggacgccgcctgggattgggcgcgaaaagccggcgcctgagcggcgcctagcggctggcggcggcgcccaggatgcggcggtcggccttgccctgcaccacccccaccgtctcctcccccgtcgcccggacgggcagggcgaacagcaccggccgtccccgccaatcgcccaggcgcgtgacttcgcgcaccacgttcatgtgccgcacggcctcgccgcgattgtcgccggccgcgacctccaccacctgcggtcccggccgataggtgacggccaccacctcggcgccgcccgtcggcgcgcggccggagccgacgccgacctggcggccggtctcgcggaactctatctggggcggccaagactcacgcctggcctcgcgctgaatggcgcttcccagctcgacttcccgcgcgccggtcagctgggtgcgcccggcgatcaccacctgcggcgtcgacaccccccgcagccgcatggcggagcggtaggcccgctgccgcgcgctgaaggcgggcttggcgaaggtgtcgcgccagccgagatagtcccagtagtccacgccataggtcagggcgatcaccccgggcgtttcggccgcctgctcgacggcgaggttcgcttcgggacagccggcgcagccctgggcggtgaacagctccaccaccaccggccgttcggtcgtgcggcggggcgcggcctcgcccgaggtcgccagcatgccgatcgcgcaagcggccgcagccgccatccagccctttgcactcataatcgccattctagcgacggcgcggatcggcggcggtcacggtcgcgtgacaccgcctcaggacgatggaggcgcggtcttcgacgaagggggcgcatgcttgcgcttggtcaccttgttggcgatgtcctcggcgtgcttcatcgtgaaggacagggcggcgggattgccgcgccgggcgcccacggtgtcggccacggttgcgccgcgtccgcccagcggctcgggctggccggtggtggtgtccaccgccgtctggtgctccacctcggcgttcagctcggcgcccatcaggatcacctgagccgagatccagatccacagcagcacgcccatcaccgccgccaggggaccgtagctgtcggtcttgacgaaattcgccagataccagctgaacagcagcgacaccgtcacgctgatcacggcggcgaagatcgcgccgggtgtcagccacgaccagcgcgcccgctgccggcagggaccgaaccggtagatcagcgccagaacacccatgtagccgagcagcagcaccggccagcgcagccacgccagataggcccactcctcctccaggccgaacagcgacagcaccaccggcacgcccaccaccagacccgccagcgtcagcaccgccagcattccgcccagcgtgaaggccaggcagatcaggttgtatttgacgatgttgcgcttttcgacctcgtgataggcgacgttcaacccgtagaacagggtcttgaccgcgccgttggcgctccacaacgacagcgccagcgtccagatcagcgtcagggtcagctcgctgctggagttctcggccagccgctgcatctggtcgccgacaaaggtggcgacgttggcgggcagcagcccgttcaggaactgcagccggtcccacgcccccgcagggtcggcgaacagcccatagatggtgacaaaggaacccaggatcgggaacagagacagcagggtgaagaaggtcacgccccccgcgacaaagcccacgcgatcgcccgtgtaggccgcgccggtccgccaaaggatgtcgatccagcccttcagcggaatgtggtcggggcgctgcgcaagccgtccgcgtcccggctcgtgcgcatcatagtcgtgcggctccatagcctcgggcgcctctggcggagcgaccttctcacgcaggtcgagaccgatccggtggccttgggtgtacagcaggtgcgcgacgccggcgcccgccgccagcccgccggccgccgcgcccacgaagcgggcgacgccgggtccgcgtctcggcggcgccccgaacgcgcgggcgcgcagacgcaggctgtcgatgatcgaggaagggcgctggctcatggaggggcgaacggccaagcctgcgccctgttccagtcctgtcgcccgccgcgcttgaaatcaccgccggggcgggcgattgaccgatcatgaccgacgccgcaccctccgccgccccgaccctcctgaccgcctggaaggcggcgcaggcgcgcctgaaacagggcgcggtcgacagccccgccatcgacgcccgcctgctgctggaggcggcggccggggcgacccgcaccgacatcctgaccgatccctatcgggtgatcggcgccgatcagcaggccgcctatgacgccatgatcgagcgccggctgcggcgcgagcccgtgtcgcgcatcctggggcgcaagggcttctggaagatcatgctgaacgtcacccccgacgtgctcagcccccgcccggacaccgaaaccatcatggacgtggccctggccgccttcccccagggcgaggcgttccagatgatcgacctggggaccggctcgggcgcgatcctgctggcggtgctcagcgagcggccggccgcccgcggcgtcggcacggacatctcgtccgaggcgctggccgtggcgaaagagaacgcggccaatctcgacctggacggccgcgccacggtcctgcgcacggaatgggcgacgggctttgcggaccaaagcttcgacttcgtggcgtccaacccgccctacattccgtcgggcgacatcgccggccttgatcccgaagtccgggaccacgaccccgtgctggcgctggacggcgggccggacggcctgcaggcctatcgcgacctggcgcctgaaatcctgcgcatcctcaagcccggcggcgtcttcgccgtcgagatcggttgggaccagggcccggccgtgaaggctctgttcgaagcggcgggtctccagggcgccaaggtggtcaaggatctgtctgaccgcgatcgcgtggtcaccaacggcccagatccgcgcacgacgccgatccccaaggcctagcgcctgccgcggcgaagccccagcagtcccggccagccgccgctgctcagcaaggccacatccagaagcgccaccggcagcggcgtcgagatcggcgcggcgatgaagcgcggcttccagtccggaaagaacttggccttgtagctgcgcaggccctgaaagccgtagagagccccgccctcctcgaacaccagggcgccgacgcgggcgaacacgggggcgaggcgacgatcctcaagccccgccagcggcgccatgccgaggtccagcgcctccagcccttccgccttggcccactggatgcagcgcacgaacagatagtccatcaccccgtgcggcccatcggggctgtgccgcatcaggtcgatggccgcctcgcgcgtcgggccctcgcccatcagcaggttggcgaaggcgacgatccgtccctcctcgcgcaccaccgccagaggcgtcaggtcgagataggcggggtcaaaccggccaagcgagaacgccttttcctcgccttggtgcatcgccagccaggcgtcggacaccagccgcagttcgtcggccagggcgctggccgagccgggcgggagcacttcgaagctcgctccctcgcgttcggcgcggttcacggccgtgcgcaggttctgcttgcccttgccttccgtggtgaaacgggcggcgtccacccgcgccgtttcgccgaccttgcgcaccgcgaagcccatggtggcgatgtcgcccagaaggctttcgccgatggagtagaacaccgccgacccgccgtaggagtccgccagctcggcgaaggcccacaagagctcgcgcgcctccgcccgatcgcccgccggtccgcccatggcgatccagcgacgcccgcgcacgcgataggcgatgaagctgcgccccgacgggctgaacaacagcgccttgtcgcccagcatggcgagccaggcctcgggcgtcgactgatcggccagctccagcgcagtccgcgcccgcgccagatcaagcgcggaggccgggccgtggctgctggcgcccggcgccgccatcagcgacagggccgccgccaccagcgtcagcagcgcgagcgccgtgccgtcgcgcacgaagccggacgcctgccgatcgatcagaaaggtccaccacagctcgttggagtagtcgacgccccggtaggcgaacaggcccagccaaagcatcgccagcaccgccagacacaccagcatcagccatgacggccgaagcggctcggccaggcgcgagcggcggcgaaacgcctcccgacagggaaacagcaaaagggcgatcgccagaagcgccgccgcctcttcccagtccaggcccttgagcagcgaaaagacggcgccgccgaccagcaccaccaaggccgcccagtaggccccgcgcctccggcgccacaggccggccgacaggatcaacagaagaaagccggccacgctggccgcgaagtgcgacaggtcgatcagcagcggcggcgccgcgcccgacagcaggcgcaggcggtcggcgaaggccggcgtcatggcagacgccagcatcagcgcgcctgcgagaaaggccagaaccgcgaacaccagaggcgtcagctcgaaacctagtccgacgatgcgccgcagcaggctggctgcgggcaggggcttggctgccgttttggaggtcagcgtcgaatctcctgaatgtccagccgcagcttagcctgattttcggcggatcggggcggggcgaaggtcatttcggggcggccgaaacaaagcaaaacatgaaggattgttcatctgcgggcgacacgcccgagcaaccggggatgatcccatgacgatcaagaccgccttcctggccggcgccgccgccgtgctgatgacctccgcgcccgctctggcgcaggacgcgcccgcatcgaccccgcccgaggcttccgccgcccagccgcagagcctgacgctggcgcccggcgcgacggtgaagggatccgacggcgcggagatcggcaagctggtcggcgtccagaacaacactgcgggcgagcaggagctgacggtgcgcggcgccgacggccaggtgcgcgccgtgccgctgcccggcatccgccaggacggcgcggacgtcgtggtcggctggacggtggccgagtatcaggccgcgcctgcggtttccggctctacaagcccggccgctccggccgccgaaccgacgagcccggcgccctccgagctctccgagccctccatggcgcccgacgcctccacgccgcctgaaccgaccacgccgcagtaacccggcgcatcaggtatagaaaaagggcggctccatcggagccgccctttccttttggtgtcgatctgggatcaggcgcgacgcttgatcaggcccagcaggaacagcaggatcaccgcgccgatggtggcgacgatggtggagccgatccagccgccccagtcgaatccgagcgccctggcgatgaagccgccgatgaaggcgccgacgataccgacgatcaggttggtgagcagcccgtggttgcggcccatgatcttctccgcgagccagcccgcgatgatgccgatgatgatccaggcgataatgcccatggtgatatcccttccagtgaatagctaagccgggacataaatgcgcatcccgcctccgggttgccgcactcccgaacagcttcgcttgtgaggcgaagtcggcacgcgccttgccgcgtctcaggcgaaccgtcccgccatgggacgacctcggacaaggacgcggcgcatggccaccgacatcgatcttcacctcggccgccggctgcggcgccgccgccgcctgctcggcctgacccagcagcagttggcgctcaaggtcggcatccgctttcagcagatccaaaagtatgagtgcggcgccaaccgcatctcggccgcccgcctgtgggaactggcggaggcgctggagacgcccgtcagctacttctacgacggcctggccgaagccttggagcgcaaggaggccgccgccaacggcgactccttctcgcgcaaggagacgctggacctgatccaggcctattaccagctgggcgaacgcccccgccgccgcctgctggatctcgccaagtctctgcacaccgaaagcgacgcggcctgacgcgcgagcgcccgtgacttgtgcggctgccgccgctatggccggcggatgaccgaacacgaagccttcgccgtcgagctggcgcacgcggccgccgccgagaccctgccgctgttccggggcgactgcgaggccgacaacaagctggcggacggcggtttcgaccccgtcacggctgccgaccgcaacgccgaggccgccatccgccgcctgatcgccgaacgctatccgcaccacggcgtgatcggcgaggagtacggcgaggaccgcccggacgccgaacacgtgtgggtgctggacccggtcgacggcacgcgcgcctttatcgcgggcctgccgctgtggaccacgctgatcgccctgcgcacccaggggcggccccgcatcggcttgatcgcccagccctatctggacgaggtcttcatcggcggtccctccggcgcgtggctgatccgcggcgagacgcatacgccgctgaagacccgcgcctgcgagcggctgaccgaggcggtgatctccaccaccgacccagacatcttcaacggcgccgaactgggggcctggacccaggtgcgggcgacggcgaagctggcgcggctgggctgcgacgcctacgcctacgccatggtggcggccggacgcatggatcttgtggccgagaccagcctgaagccctgggactggtcggcgctggtcccggtggtcgaggcggcgggaggccgggtcgtcaactggcgcggcgcggcgcccgacgacggcggccaggttctggccgtgggggacgccagcctgatcgatcaggcgctggtcacgctcaggcgcgcggcggtctagctagccggcggcttcgagctcgacgcggttctgctccgcaccagccggcgccaccctttctgccaaggcctcgaattcccggaaggcctcggcccgcaggtcgtcccgctccatcagcacctcgtgctgggcgccgccgatctcgacatagcgaccgtgcggcaggcgcttggtcgcccagcggctggtctgcttccagacgcggtcgtcgtccgccgcctgcaccacggtcaccggaatccgcaccgacttcagcgccttcagcttcagcgcccgctccccggcgtccagcgcgaacgccagccagccccaggtcgtgccgccgatcgccagatgcgggcaggcgtacatctgctggcgccacagttcgtatcgcccctcgtccgaggtcagggcgtccttttcgaaggtgtggccgaacggatcgtccggttcgtccagcacatagtcgcccgccttgccgtgccggatattccagcgcaccgccagcttgaccgaccacatcgaatgcttgccggtcttgacccgcagcatggggctggacagcagcgcgcccgcgaaacgggtctcccccgcctgcaggctcagcaggttcagcgccgcgcccatggagtggccgaccatgatccacggcttggggcatcggtcttcgaacacggtcaacaggcgggcgtagtcgtcgaggaactcctcgaccgcacgggcgtgacccttcagccggtcgggcagcagccgcgccgacaatccctgcccccgccagtcgtgcgccagcacgcaccagccgcgcgccaggaagttgccgatgacctcgaaatatttctcgatcggctcggtgcggccggggctcagcaccaccgtgccgcgcggctctccggccgccggcgcggacggcgtccacaaggcggcgcgcaggcgcaggccgccggctccgcgataccactcgccctggccgccgggcggggacgcggcgtccggcgtgcccatcaggggcgcttcggcggcataggcttgggcgcggttcactcgggcttcctgaacttcaaggtcatgcggtcggattcgccgatggcgtcgtacggcgtgcggtcgaactcggggtcgggcggctggcccgccggcgcggtcagccgcaccggcggcagggtgtcgacgccgaacggatggtccttggtgtcggcctcattggcgttgatctcggagccggcgacgaactggaagcccgcctcttccgccagctgacgtacaaacgcctcctgcacatagccgttggcggcgacgggatcctgatcctcctccggctcgagccggtgctggacgatccccagcacgccgcccggcttcagcgccgcaaaggcgtcggcgaaggccttttcggcgatccccgccgccatccaggcatgcaggctgcggatgaacaggcacaggtccgccgttccaggcggtgcgacggcgcccgtgctcgccccgaactgggtgaactggatgtctccgtagaggtcccggtcggaggtgaagcgcgcctgaaaagccgcgttcagcgccgcctgcgcgggatcggccgacggcccctgcgcgaaggtggcggcgaaatagcgccccccccccttggccagatagggggcgatgatttcggtgtaccagccgccgcccggccagaactcgaccaccgtcatggcgggctgaagaccaaagaagcgcagcgtctccatggggtggcgggcggcgtcgcggcccttgtcccggtcgcgccaggcgccggcgaccgaccattccagcgagccttccggcggtcccgcaggcgcggtgtccggcgcaggcgcggtcggcgtcgcctcgtccctgcggccgcatccgcccaggcacgccgtcagccccaatcccgcgcccgccagcagcaggccgcgacgtgacgcgaacggaaagccaggcgcatgatcagccatacaatatccttgccggacgtgcggcgccccgcaggccgccatcctcgacccctcgcttagacagcttcgcctcaccggtcaaaacgggagcggttacgtttgttcgagcctattccggcttgcgcagccgcagggtcatccggtcgctttcgccgatggcgtcgaaggcggcccgctcctccggcgtcagcacgcgcccggcctggtcgccgcgcccctgtgactggcggatcggcggcagggtccagacgccgaacggatgatcgtggtcgtcctttggattggcgttcagttcgctgcgcgcctccagcacgaagccggcgttgcgggcgtcccggatcacgtggctttcgggcacatagccggtgggcgccacatcggcgacgttcagcccgtcttcgctgcgatgctgctcgatggccaggattccgcccggcttcagcgcccggaagaaggcttgcagatagggttcggtgcgcccgtcgcgcgcccagttgtgaaaggcgcgggcgaccagcaccatgtcggccgatccatcctcgacccctatcgtctccagcggccggttgacggccacatagcgcccgcccgtcgcctgcagataaggctgcaggatcgcactccaccagccgccgcgacccggctcgatctccacaaccgtcatgcgcggctgaagaccccagaaggtcaggctttcatagggatggcgtgcggcgtcacgggcgcggtcggcttccgatcggctggttgacgccaccgccgccttcagcgcctcgtcctcctggaacaccggcggcgtcatggcgagccccgagcgggtctgaagcggggcctgggacgtggattggggcgtcgattgggcgaccgccgaaccggcggctcccgccaacaggacggcggcgacggcgggggcgatcaggcgcatgaaacaagctccggcgggggacaccgccttcctgcccgtggaaggccgaccacgccagagcggatcgtcgttcgcgaccatttcacgcgctgatccgcaccctcttgaaccgcgaaaaccgcctcccacattccgtttcgaaggcgccggtttcgggccttccagccaggcggcgccggtttcgggccgctcgactgcaatcgttgtgaccttgctgatcctcaggaggatgcttccatgcgtacctatgacttctcgccgctgtaccgttcggccgtcggcttcgaccgtctggccaacctgctcgaaagcgccgcgcgcacgagccaggaaggcggctatcccccctataacatcgagaccacgggcgagaacgcctatcgcatcgagatcgccgtcgccggcttttcgcccgacgagctgaacatcgaggtgaaggagaacctgctcaccgtctctggccggaagaccgccaacgacgatgcggcgacgcagaggacctatctgcatcgcggcctcgccgaacgcgacttcgagcgccgcttccagctggccgactatgtgatcgtcaccgacgccaacctgtcgaacggcctgctgtccatcgcgctgaagcgcgaactgcccgaggcgctgaagccccgccgcatcgagatcggcacgggcccggccctgatcgagggcgaagccaaggcggcgtaatcgcccctggcctgctggactgacgggagggggcggcgcttcggcgtcgcccctttttctatgccgtcaggtgggcgaaggcgcggaccacctgggcgtaggcgtcgcgcttgaacggcacgatcaggtcgcacgcctcgtccagccggccccagcgccaggcgtcgaactcgacctctccgtccgcgccgacatggctctgcagatcgatctcgctgtccgggccgatcaggcgaaaggcgaaccagcgctgcttctggcctttgaagccgcgccaggccttggcgttgttcgcggcctcgggcggaaagtcgtacaggatccagtcgtcggtcgaggccagacgttcgacggagtggacacccgtctcctcgcgcagctcgcgccgtgcggccgcctccaggtcctcgccctcgtccacgcccccttgagggaactgccagttccagggcggcggcgtcgcgtggcgttggccataccagacaagaccgtcccggttgaacaggaccaccccgacgttgggccggtaaagccggaggtccgtcaacggccgggacgctgggtcatggcggatgcgggcgccagctgcagggcgcgctgctccagcccggcggtccaacgtgcggcggcctcgaccgtgaccggataggagaagccggttccgagcgccgagccgcgaatcttggcctgggcctccaggctgttcagggcggcgatgatggcggcgggcgactgggtctggtcgatcaccttgtcggcgctggcgcgggcccaagcgccgggccggcgctggaacgacccgtcgtccaggaaggccacgccacgctggcgcagcgtggtcagaaaggcgttcatgcccgcatccgacgccgcgaaccggtcgcccaggtagttggtcacgccgaagtagccggtcgcgcggcccagcagccagttcatcttggcgccgatgtcgtccgccccgccgtcggccagcagggtgtaggggccgggatcgttgttgggatagccggtcggctccatcggcatttccagcatgacctcatgcccttgagcccgcgcctggtcgatccaaccctgcaggttctcggcatagggaacgaagctgagggtcacatcggccggcaaccgctcgatggccgccttggtggtcaccgcattcagcccgaggcccccgacgatcagggccacgcgcggcttgccgttcgaccggaatggccgggcgtaggcctgcgccggcacccgcccgtccggcgcgatcaccggcagcagcccattcggccccggccccgacaggcccgccagcggcgccttggcgagcggagacgcgacctgcatcggcgccgaatagctggacccgccgcccgcgaccgtggctccgtccggcagggtgatcagcgcctcgccgccagccgcgccgctcagcggatcgccggttccggtcaggtcctggtacagccccatagcgcccatggaaaaggcgtcaaagccggagggcgccggcgcctccgccgccgcctcgcgcttcaaggcgatgcgagccgacggcgcgcccgcgcgggggtcgcccagcaccgtcagaaacagcgcgcccgtcgacagaagcagcaggcccgccagccccgcgatcaccggcggcttgcgcacggcggccttcagcacctcgaccggcttcaaggcgcgagggggcggcgggctgccggcggcggcggcgagggcggactggcgtttggcgaacatggtgcggacttgggacccagcggaatccttcggccgccactttcgcgcaaggcgggttaagaaaccctaacgcccgttcaccacgttggccttatcgctgcggctccggccgtggctcgttgcccggcgtgatctccggggtgcgggcgggcggctcggccgggtcggcgggcggggtcgccggcgcggcgtcgtccgccgcatcctcgctcttttcggtcaccaccacggtcgagggcggcgccgacaccctggacacgtccccgccggcgcgcagcacgtccagcgcccgctccagctgatagtcggtgtccttgtcatagttttcgcccggcgcctcacgcgggatgtgcggtcccttgcgctcggccccgatggaggagtccagcgccgtggcgtaggcggcctccgaatagatgaagctggaacgcgagacgatgcgcgcctcggcctccgagcgggcgacctccaggtccggctcgatgccgatcttctggatggaggcgccggacggggtgtagtaacgcgccgtggtgatcgacaccgcgccgtcgcggccgccgcgcagcgggatcactgtctgcaccgagcccttgccgaagctggtcaggccgacgaccgaggcccgctcgtgatccttcaaggcgccggccacgatctcggacgccgaggccgagccgtagttgatcagcaccaccagcggcaggccgccgatcaggtcgccgggcttggcggcgtagcgctcgatgtcgtccggcttgcggccgcgctggctgacgatctcgccgcgctccaggaaggcgtccgacacgtcgatggcggcgttcagcagccccccgccgttgttgcgcagatccagcacatagcccttcacgcccggcttctcggccttgatcttgttgatcgcctccgtcagctcgcgcccggtgttctcgttgaaggtcgagacgcgcagatagccgaagtcccccttcacctcgccggtgaccgactgcaccttgatgacctcgcgggtcagggtcacctcgcgcggctcctcgccgtcgcgcaggaaggtcacgcggacggaggtgcccaccccgccgcgcagcttctccgaaacctggctgacggtcagacccgaggcgctctgaccctcgatggcgctgatgacgtcgccggcctgcacgcccgcgcgcgacgccgggctgttgtccatcggcgagatcaccttcaccagtccgccttcggaggtgatggtcaggccgacgcccgaatactggccctccgtgcgctcgcgcagctcgtcgaagttctcgggcggcagatagttggagtgcgggtccagcgccgtcatcatgccctgaagcgccgcctcgatcagcttcttgttgtcgacgggcaccacataggcctgctcgacgatcccaagaacgtcgccgaacagctccagcaggcgaaaggtctcgttgcgcggggtctggctggccacggccatggccgatccgccgagcgccagggcggcgcagccgacaacaagcagtttacgcattcggtctctttcgatgggctcgctcatcgacgccctgcggtgaaggaaggccttgagaccacgacgaaatcgaggccgatcggcgttgtttccgatgtaagccgccgcgagcgcagttgcaaagcggctattgcagccagggacgcgggtcgatcggccgttcgtcgcgccgcagctcgaaatagacctcgccgtcacggccgctgcggcccagcgcctggccgtccgcgacgcgctggtcggcctggacgtccagtgtctccagccccgccaccaccgcgcgccagccggggcccagatccaggatcaccacctgcccccagccgcccagcggtccggcgtaggccacgcgggacgccgccggcgcgccggccaccgcccggtccgcccgccatctccatccgctggagccgtcgccgaaacgctccgccggctctgcggacaggggcgggcgaaggcgcgcgccgcccgcgggccggcttgcggtctcgggctgcgcggccgccggcggcgtgctgacctgtccgcccagcgcccggatgcgcgcctccagcacctcggccgagcgctcggccgtttgcgcctcggcccgaagcaccgcgaccagcgccgtcttgcgggccgtcaggctctcgatttcagcgccgcggtcgccttgcgcgctttctgtggtcagcagccgctcgctggacagcacggccagccggcgaatccggccgatctcggcctgctggtcggacagggtcttggcccggctttgcagctccggcgctatcgccttgatcaggatggctgcgcgcaccgtatccaccgccttgtcggccgggaccagcagcgggggcggaggtctgcggctcatcatctgcagcgcgctgagcagccgcccgtgacgtccgcgctcgcgggacagttcgcccaccagccgcccctcgcggtcgccgagctccttcaggcgcgcccgctgcgcctccagctgcacgtcctcagccgaggcttcgcgcctgagatcggccagacgcccatccagatcgcgcagctcgtcacgggccgcgtccgcgtcggcccgcagcctttgcgcccgcaccgcctcgtcgcggtattcggcctggaggcgcgccagctccgattgcggcgcgcgacggccggcggcgggcgtggcggccgccagcgccagaacggcgacgcccgcgacacgcagcatgccgctcttccgcatcgccttcagtcgcggtgatagggcgagccggacaggatcgtcacggcgcgatacagctgttccgccagcatggctcgggccagggcgtgcggccaggtctgcggcccgaacgcaagggtcgaggcggcggccgcgcgcacgctgtcgtccagaccgtcggcgccgccgacggcgaacaccacccgccgctcgccccgatcccgcagggtcgcgacgtggtcggcgaaagcgcgggaggaataggtccggccccgctcgtcgcaggcgatcaggtgcgcgccctccgccgcctgcaggatcagttcggcctccggcgccttgccgctctttcgcggttccaggtcgatcagttcgagcggacccagaccgagcgcccggcccgccagactggcgcgccgggcgtagtcgtcggccagcgccgcctcaggcccgcgtccgggcttgccgatggcgacgacggccagcctcaccgaaggatcagacgctcgcggggcggcggtgggcgctgtcgacggcccagatcttttcgatgttgtagaaggtgcgcacctccggccggaacaggtgcacgatcacgtcgccggcgtcgatcagcacccagtcgcagtgcggcaggccctcgaccttggccttgcccaggccctggtccttgagctcgcgcagcaggtggtcggcgatggcgccgacgtggcggtgcgaccggcccgaggccacgatcatggcgtcggccatcgggctcttgcccttgaggtcgatcaggacgatgtcctgcgccttgtcgaaatccagcttggccagaagcgcttcttccagcggggtcgaaccgaccgggcgcggcgtctcctgaccgatcggtccggcggaggcttcgtcgtcgaagtcgtcgtcgccgaactccagaccggcgaagtcggagtcggtttcggctccgtcctcagtatggaggggttcgatgggatccatctcgttcgccaggttcgaaacggcggcgtcttgcgcatcgtgcgcgggagagggggtcagcgtagggctccaggagcgtttatctaatccggacatatagcacgcccggcgccgaacgtcacccgaccacgcgatccgccatccgtcccgcccggatcgcggtggaggagcgcgcgttcagcggcgccgccagatacgtccaggccggcgcctggagcgtcgccagcagcccggcctgggcgtccggcacgcgaaaggccgagaagcgtcgcgccgccggagcgctgcggctgtccagctgcgaccccggccgcgccaccacggccacgggcgccatccgcatgatgtcggtccagccgcgccagcggtgaaagctggccaggttgtccgatcccatcagccagacgaagtgcacgcctggatgccggctcctcagcgcccacagggtgtccaccgtccactgcgtgcccgcccgggtctcgaaatccgagacaatcatggcgggcccttgcgcctgcgtccgcgccgaggccatgcgctcggccagcggtgcgctgtggcgggcgtccttgagcggggtctgcggcgacaccagccagaccacccggtccaaccccaaccgtctcaacgccgtctcggccacatgggcgtgcccgtcgtgggcgggattgaacgagccgccgaacagcccgaccttcatccccgccgtgatcggcaagccgtcacgcagcgccccgatgcgggggccagagcctcgcggcgcgggaccggcgtgaaaaaaggacaagagggcggcggctcggagaaacggttatgctcgccgacgccctatcaggcggcgggaggcgtgtcccgcgcgaaatccgtcagactgcggcgtccagcagcgcgcttcgcaccacttccggctgcgtcatgggaaacaggtgacgggcgcccggcacgacctccacccgccgccgcccgtcgtcggatgcgaccgccggcacatggcaggtcgatccgatctccgccttcacgatgcgcgtccggccgccgtagcgccgcagcgcccgccagggatcgtggctctgggcggcgtagttggaggcctcccactccggcgtggcgctcagcgcatagccgccgtcaccctccaccagcccatccgacagatagtcggccagcgccgcatcgggccagccgcgaaaggcgccgcgaccacgataggcggccagcgcctgctcgcggctctcaaaggcgctgcgtcgacgcctcgccgtcttcgccagcggattgttgtacaggcccgcccgcatcaccggcaggcggaacaggaggctggtcgcccggctccagatcacgggatcgaacagcaccagaccggccgtccgctccggccgctcggccgccgccagcagggccgaggttccccccatcgaatggccgctcagcaccaccggtggtccgtccacggcgtcgagcagggcgatcaggtcgtcgcggtgatcgcgccagtcccaacgccgccgcgtgcggatcggcaggtttgtccgcccgtgcccccgcaggtcgggcgcccagatgcgcagcgaagccgacagcggcgccagcacgctgcggtaggtcgccgcgttgaagccgttggcgtgggcgaagaccacgtccaccgggcgttcgggcggaccgaagtccagcaccgccatctcgccgccgccccaccgattttcgatggcgatgctcagacggcgcggcgcgtcgagcccggacgggtccatggatcaggcggcctctcgacaggcggcgcagcgtccgtgcgcctcgatggttgtgcgctgcaccgcatagcccgcctcgtgtgcggcctgatgcaggcggtcgtcctcgccgatcgcgacctcgcgcgtcgcgccgcagcagtcgcagataagaaaggcggcggcgtgcgcgctctggtcgtcgccgctgcaggccacataggcgctgatggaggcgatgcggtgcgccagccccagtcgctccaggaaatccagggcgcggtacaccgtcggcggcttggccgcttggccttcggcgccgccgaagcgggcgatcaggtcataggccttgaccggctctccggcctccagcagcagcgtcagcacgcgtcggcggggcgcggtcatccgctcgccggcgtcggcgatgcggcgctcggaggcgcccagcgcgcgctccagcgccccgccgtgcaagccgccgtgaacatgatcgtgatcgcaggctgcgcccatgacccacagctaatgcctgcggtctcccgccgcaacacaacgcgcacagcatggcgaacggcgatgtttgccgcgtgcctgcccttcggctagaaggcccgttccttacggcttctcagcgatcctgcttacccatgaccgacgcttcgtcctcgccgctttcgggcaacgtcctgttctacaaccagcccgagccgctggatcccgcccgtcacggcggcctgggcgtcaacgccgccgacaagccgtacgcctttgtgggcgcgaccaacttcgtgccgctgacggtgaccgagttcgccgccgccgccctgtccttccccgtggtcttcatgggcgaccagaagcagccggtcgcggtcatgggcctgcgccagggcgagaacctgtatgtctccaatgagggcgactaccgtcccgacgcctacatcccggcctatgtgcgccgcttcccgttcgtcttcgccgacgacaagcagaactcgcgactgatcctgtgcatcgaccgcggcgcgccgatcgtcacggaaggcggcgaaacgccgctgttcgtggacgggcagcccagcgactacacccagatggcgatggagttctgcaacaacttcgagcaggagcgcctgcgcaccgaggccttcgtgcagctcctgggcgagcttgacctgttcgagacccgcaccgccaacttcaccccgcgcaaccccgacggcagcgccggcgagccgcagcgcctggccgagtatttcgccgtctccgaagacaagctgaaggccctgccggccgagaagctggctgagctgcgcgacaacggcgccctgggccagatctacgcccatctggtgtcgctgctggggtgggaccgcctgatcgccctggccttccagcgctcggcgcagacgccttcggccgccaacaactaaggcgcttgatcgtaaagaaaggccccgccggctctcgccgacagggccttttttgcacctgacggcgagattcaccacaagcgtcaacaaggtcgaaaggctgttgtcggcataacagcgttcatgaccgacacgcccttcacccgccggcctgtcacccaggtcgatcccgcaaaggaccgctcgcaacagctgcgagacgatgtccagatccagagccggccgcagacgccgtccgcgcgcgccgatcacgccttcagccgctcagaccgcgacggcggttccggcttcggcgccctgttctagcgcctggagaacaccgcccgcgtcaggcaggcgaacaccagacggccgctctcgtccaggaggtcgtgcgaggcgatgacgatgcccttttcgtcgccgaccggatccttgcccatcaccgtcatgcggccgcgcagcagctcgcccgccggcggattgcgcataaagcgaagcccgtccaccgccagcaccttggactgggcccagctcgccgccttgtccgcgaacagacggctccacagggcgtagaccatggcgtccggtgcgccataggccgtgtcccagcccggcgcgaaccgttcgacgaagacgtccagcgcgccggcatcgaccgcacacgccccgagcggcgcaacctgtccgacatccaggtcctcgaaatgggccagcagcggttcgctcatgccggtggggtcctcaggccggttcgtcggagacgcggaccagcagcttgccgttgtggtcgccggtgaacaagcggttcagcgagccgaccgcgccttccagcccctcgtcgacgtggaccttccacttgacccggccgtccgccagccagggccccatctcggccaccatctcgcgggcgcgatgggcgtagtccagcaccagaaagccccgcacgtcgagccgatgggtgatgatccgggcgaagttcggcgagggcggagccttggtcgcattgtaggacgacaccagcccgcacacggccatgcgcccatggaccttcagccggttgaacacggcgatcatgatgtcgccgccgacgttctcgaagttcaggtcgatgccgtcgggcgccagccggtccagcgcctcgcccacgtcttcgttcttgtagtcgacggcggcgtcgaagccgagttcgtcgaccagccagcggcatttgtccggtccgcccgcaatgccgatcacccgcgcgccgcgctgcttggcgacctgtccggcgatcgagcccaccgccccggcggccgccgagatcaccagcgtctcgcccgcctggaccttgagcacgtcggtgacgccaaaataggccgtcagccccgtcatgccgagcaccgacaggttggccgtcagcggcaggccggcggcgcggtgcaccggccgcaacgcctggtccgacaccacggcgtaatccgcccagccgccggacagcggcgtcaccacgtcgcccgccttgaagcggtccgagcgcgactgctccaccacccccagcgtcagcccgcgcatcacctcgcccaggcccaccggcggcagatagccttccgcgtcgttcatccaggtgcggtttgtgggatccagcgacaggtagacggtgcgcaccagcacctccgactccttgaggtccgggatggggctttccaccagctccaggtcgccgggctggaccatgccgcgcggacgctggcgcagcacccactgccgattgatccttgtcatcgtattctccgatccgctggcgttgatctcatagtggccaagcgacgcgagcgggtcgagcccggcgaaaaagaaaagggggcccggggggaccgcctttcagtggcattgtcgagaatgaggcgcggaggcgacaggccggcagggccggcctggagtcggggggcgtcgccgcctccgcccaccaacaacggcgcggatcgaacacggttccgcgccttatctagtttacccgcatcgaccgatcagcggtctacggaacagcgaagctcggatcggcgttgatggagccaagcggcaatcatcaggacagacggcggccatgacccatgaagatcccaatgttcgcgcctcgaacatcgtcgacgccgaacagacggcgggtgcgcaagacacgcgtcaggggcgacccggcaagcgcatcctctggctgctgatcgtctccgccggcgctgcggccgttctgctgctgggcctgtggttcgtcagccaaaacggcatgtcgcagaccaacgccaacgacggcggccaggtcgtggacgcccaggcctttcagggcgacagccagaccgcgccggcggccgatgcgcccacgacctcgaccggcgaaccgaccgcgccgccgaccggggaggcccccaacgtcaacgcgcctacgacctcggcccagccgtcgaactgacgccggcgcggccagcctcagtcgaagatgtcaaagatgctgtcgcgcttctttttcttgtaaccgtgacgatgatcgtcccggtagcgatcgtccttgtagcggcgatcgtcatcgcgatagccgccacctcctccccaaggttgggagtgggattgcggatgggcttgcggaggcggcgccgcatagccgggctgcggcggcggggcgtaggcggcgggcgcgctggcgcggccttcgtccatcgccgcctccatcagcttttccagctctccccgatccagccacacacctcggcatttggggcacatgtcgaactggacgccggagcgttccagcgtctgcatcggggcgtcgtcgttggggcacatcaagaggggcatgatgggaagctaggcgcagcccccgcgcgcgcaatgcggccgaccgccgcaagcgtcgcctagcaggcctgaccggccgcccaacccgacgaccaggcccactggaagttgtagccgcccagccagccggtgatgtccaccgcctcgccgatgaagaacaggccgggcgtggtcttcaccgccatggtggtctggtccagcgccgccgtgtccaccccgcccagcgtgacctcggcggtgcggtagccttccgatcccaccggcttcaccgtccagccgttgaccgccgcatccagcgcccgcagccgcttgtccgacaattccgccagcttgcccgaggcgcccttgcgctgggcgaggctttccgccaggcgacgcggcacgatctgggccagggcggtgtgcaccgcctgtttcccgttctcctcctttgccgtcttcagccgtgcgaagacgtcctgccccggcgccatggtcacggtgatcggatcgccttccttccagtaggagctgatctgcaggatcgccggacccgacagcccgcggtgggtgaacagcatcgcctctgggaaccgcgcgccgcccgcctccgccacaacatccaccgccaccccggccagcggcttcaactgctccagcagccccgcctcaaacgtcagcggcaccagcgccggtcgcgtaacggtgacccgcaggccaaaccgccgcgccacttcataggcccagccggtagcccccatcttgggtatggacttgccgcccgtggcgatcaccaccgaggccgcgcgcacgaccgatccgtcggaaagccgcgcctcgaaccgctcgccgacacgctccagcccgtcgatcgagacgcccagcttcagctccacgccgcccgcccgcagatcgtccgtcagcatacggacgatctgcttggcgctgtcgtcgcagaacagctggcccagcgtcttttcgtgccaggcgatacccgcccggtccacgcgacgcacgaaatcctggtgggtgtagcgcctgagcgccgaggtcgcgaaccgcgggttttcgcccaggaagttggccggacttgtgccggtgttggtgaagttgcaacgaccgccgcccgagatgcggatcttctcgccgggtgcgcgcgcatggtccaccaccagcacccgccgcccgcgccgccccgcctcccccgcgcacatcatgccggcggctcccgcgccgacgatcaggacgtcgaaggccttcgttgatccagcgctcaatgcgcctcgtcccagttggcggcggcgcgcgcttcgaccaccaggggcacgctgagcgccgcggcgggttcggccgcgccctccatgatccggcgcaccagggcgatggcggcctcggcctcggcctccggcgcctcgaacaccagttcgtcgtggacctgcagcagcatccgggtcttgagtcccgccccggcaagcgcgcccggcatgcggatcatggcccggcggatgatgtcggcggccgcgccctggatcggcgcattgatcgccgcccgctcgccaaagctgcgctcggccgccgacttcgacccgatcgccggaatgtggatcttgcgtccgaacagggtggagacgaagcccgtccgcttcacctcggccttggtcttgtccatgtaggcgcggatgccggggaagcgctcgaaataggtcttgatgtaggccccggcctcgccctgatcgatgcccagctggttcgacaggccgaaggccgagatgccgtagacgatgccgaagttgatcgccttggcccgccggcgggtctccgggtccatctgctcgaccggcacgccgaacatctcggacgccgtggccgtgtggatgtcgatcccggccttgaaggcgcgcttcagctcggggatgtcgccgatgtgggccagcaggcgcagctcgatctgggaatagtccgccgaaatcagcacgtgccccggcgccgcgatgaaggcttggcgaatctggcggccgatctcgttgcggatcgggatgttctgcaggttcggttcggacgacgacagccgcccggtcgtggtcgccgccagctgataggaggtgtgcacccggtccgtgttcggatcggccgccgccgacagcgcgtcggtataggtgttcttcagcttggacagttggcgccattccaggatcgcgcgcggcagctcatggctcagcgccagttcgtccagcacgctggcgtccgtgccccactggcccgaggcggtcttcttgccgcccggcaggcccagctctccgaacaggatctcgccgatctggcgcggcgatccgatgttgaagggccgcccagccagctcgtgcgccttgccctccagctcggccatgcgcaggccgaactcgctggacagcgacttcagccgctccggatcgatgcggacgccggccagctccatgtcggccaacacgcccggcagcccgcgctccagcgtctcatagacggtggacagcccctgctcggccaagcggggcttgaggatgcgatagagccgcagcgtcacgtccgcgtcctcggcggcgtagcaggtcgccggcttcagctcgacgtgcttgaagctcttctgcgacttgccggtgcccgccaccgacttgaaggtgatcggcgtgtggccaaggtgcaggcgcgccagctcgtccatgccgtggccgtgcagcccgccctccagcacataggagatcagcatggtgtcctcgacgggcgagacgcggacgccccgacgcgccatcaccgccatgtcgtatttgatgttctgaccgaccttgaggacgctggggtcctcaagcagcgtcttcagccgcgccagcaccgtgggcttgtccagctggttcaacggctcgcgcgacgcatcctcgccgccgccaaagtccagccccccgccctcgaccggcggatgctcgtgcgtcagcggaatatagcaggcgtcgttcggccccagcgccagggacacgccgcacagtccggcgtgtgtcgccgacagcttgtccgtctcggtgtcgaaccccaccacgccggcctcaagggcgcgctcgatccagcgatccagatcggccaggtcgcggatgcagcggtaggcctcggtgtccacgacttgcgcctcgacctccgccggctcggccggggcgtagcgcggcgtcagcaccggcgcgctaggctggcgcgtgaaggccgagccctccttgggcggcgccttgccgtcgcccacgcggcgctgcaggccccggaactccatccgctccaggaagtcgctcagggccgccggatcgggatcgcgcaccgcgaagtcctcgatcgcctcggacgccggcgcatcgcacgtcagccgcaccagttcgcggctgagccggatttggtcggcatactgaatgagggtgtcgcggcgtttcggctgcttgatctcgcccgcctgctccagcagcgtgtcgaggtcgccgaactggtccagaagctgcgccgcggtcttcggtccgatgcccggcgcgcccggcacgttgtcgacgctgtcgccgatcagggcctgcagatcgaccatcttgtccggacccacgccgaacttctcgaccacctcgggctcggcgagacgtttgtccttcatggggtcccacatgaccacgccgcgcccgatcagctgcatcaggtccttgtcggacgagacgatcaccgcctcgccgcccatgtcgcgggccttgcaggcgtaggtggcgatcaggtcgtcggcttcatagccgggcagctccacgcaatggacgccgaacgccgccgtcgcctcacgcaccaaggggaactgcggcgcaagatcctcgggcgcgggcggccggtgcgccttgtactggtcgtagaggtcgttccggaacgtcttctccgaatgatcgaagatggcgaccaggtgcgtcggcccgtcggcccccttcatgtcgcgcaacagcttccacagcatgttgcagtagccctgcaccgccccgaccggcaggccgtccgacttgcgcgtcagcggcggcagggcgtgataggcgcggaagatgtaggccgaggcgtcgatcatccacagccgcagcgcgggcccatcctgggtcagcgggcgctcggtctcgggcggggcgtctgcagcgtcggcgggggcgtcggtcatgcgccgcaacataggggcggacgccgcctgcgtcagccgtttccgatcagaaggcggtccagctctgtcccggatcgcgctcgcccggctgggcctgctgctggccccaattgatcaccatcagcacctggtggctgcggatgcgatagcggccgatcatcggcgtcaccgcacccagcggcgagccggtctgggcgtcgtagagaaagcccgagaactcggccacgccgacccggtcacgctggctgtagaccgacagctcgggcacggagacgaagttccattcctcgatcgggatgcgcatggccgggatgccgaccacacggcgcatctgctccagcgacagggcgccggcgcgcacttcgaagatcacgctggcggtgttgcgatcgcgcgccagcgcatagccggcctccgacagcgccgcgcggatcgcgcccaccgcatagcgcgcgctttcggcctgaaagtaggtgtcgtccacgaagatgcgcgcccccaccgggatcggcagcaccagcccctccaccgccatgtcggcggcgcgcgacacaagcagctgctcggtggcggtgcgtcccggattggtttcggtggtcgaggcgcaggcggacaggacgcccgccagcatcagcgtcatggcgacgccgaggcgcgccatcaccacacgcccgtgttcggcatggaggcccagggctcggccggcgcgagcggcgcgccttcctgcagcagttcgatggagatgccgtcgggcgagcgcacgaacgccatgttgccgtcgcgcggcggccggttcaccaccacgcccgcgtccatgaaccgctggcaggcggcgtagatgtcgtcgaccttgtaggctaggtggccgaagttgcggccgcccgcgtaatcctcagggtcccagttgtaggtcagctcgacctccggcgcgcgctcggccgccgactgctccaggttcctgggcgccgccagaaacaccagggtgtagcggcccgcctcgttctcagtgcgccgcacctcctgcaggcccagcaggtcgcagtagaagcgcagggacgcgtccaggtcgcggacgcggaccatggtgtgaagataacgcatcacgggaactccgaagaagaggcggaaggagggctcagtgcgcctcggacccgcgcaccgccgggctcagatactcgttctcgtcatgggcgtcggccgacaacacgaagcgccggtcgcaatagccgcattccacgtggtcgtgcttgcccatatcgaggtagaccagcgggtggcccagcgccccgcccccgccgtcgcaggccacgcgcttggtcgagaccacgatctcttcgggcggcgggatgatcgcatccggatgacgtggcggcatttggcgctttgaccttggcgggaagaggtgcggcgcatacctatgcggcccgcccggcggcgtcaaacgtggccgctgcacttccgcgagagctcttttaagccgatgaccgacgccgcccgcctgcccgacaacgccatcgaggtgcggggcctgaagaagacctatgccggctccaagaaggcggcgcccaagacggcgctgcgcggcgtcgacttggcgatcccgcgcggctcgatgttcggccttctgggtccgaacggggcgggcaagtccaccctgatcaacatcctggccggcgtggtcaagaagtccgaaggctcggtctccatctggggccgcgacatcgatcgcgagccgcgcgacgccgccgccgccctgggcgtggtgccgcaggagatcgtcgccgatgtgttcttcaccccgcgcgaggcgctggaggttcaggccggcttctatggcgtgcccaaggacgagcggcgctcggacgagctgctggctgcgctgggcctgtcggacaaggccaacgcctatgtccgcgccctgtccggcggcatgaagcggcgcctgatggtggccaaggccctggtgcacaatccgcccatcctgatcctggacgagcccaccgccggcgtggacgtcgagctgcgccgccagctatgggcctatgtgcgccgcatcaacgccgagggcgtgaccatccttctgaccacccactatctggaggaggcccaggagctctgcgacaccatcgccatcgtcaatcgcggcgaggtggtggcctgcgaaccgacgccccagctcttgcgccgcctggacacccgcaatgtggtggtgacgcccgagacgcctgtgggagacttgccgatcctttcgggcttcgacgtgacggcgcgcccgaacggcgcctttgcggtcacctacaagaagggtcagtcttcggtcgagcaggtcatcaacgccgtgcgcgaggcgggcgtccacatcgccgacatcaccaccgaggacccggacctggaggacgtcttcctggccctgacctatggcgacctgtcgcgcgccgatccgacgcgggactgaagccgcgcgttgcaaggcgcaacgcgaagtgagtctggcggatttggtccgaacgaccccttttgatacaggggcggccgacatggtgatcgctcaagcgaccgccgcctttctcgaacggagagcgccatgatcccctttatcgacctccaggcccagcgcgtccgcctcggcggcaggatcgaagccgcggtggccgaggccgtgaccggcggcgcctgggtcatgggtcctcaggtgcgccagttcgaaaccgacctcgccgcctttggtcaggccaggcacgcgctgggctgcgccaacggcacggacgccctggctctgccgctgatggcgtgggggatcgggcggggcgacgcggtgttcgtcccctccttcaccttcgccgcgacggccgaggtcgtgccctggttcgacgccgagccggtgttcgtcgacgtggacgaaaagacctacaacatgagcccggccgcgctggaggcggcgatcgacgggatcaaggccgaaggccgcctgacgccgcgcgtcgtcatcgccgtggacctgttcggccagccagccgactatccggccatcaaggcgatctgcgacaggcacgggctgaagctgatttcggactcggcgcaaggcttcggctgcacgatcgatggggcgcatccgctgaagtgggcggacgtgaccaccaccagcttctttccggccaagccgctcggctgctacggcgacggcggggcggtgctgaccgacgacgacgaactggcccagctgatggattccatccgcgtccacggcaaggcggtggcggtggaccttcaggaccgcaccttcgatcacgaccctaaatatctgaacatgcgtatcggcctgaacagccgcctggacaccatccaggccgccgtcctgatcgaaaagctcaaggtgttcggccaggagatcgagtggcgcaacgccgccgccgcccgctacaacgcgggcctgcgcccccacgtctcggccgtgccggacgttcccgccgggaacatctccaactgggctcaatacacgatcgagcacccggaccgcgacgacctggccgcgcatctgaaggcgcacgacatccccaccgccgtctattatccgatcccgctgcacctgcagccggcctatgaacactatccgcgcggcgcgggcggcctgccggtcaccgaacggctcaaggacgtggtgatcagcctgccgatgcacgcggatctggacgcagcgacccaggaccgcatcgtcgccgccgtcgccgcctacaagggctgatcctcatgccgaaccccactccgctgaagatcggcgtcgccggcgcgggcgtcatgggccgcaaccatgcgcgggtcgccgccgagatgcgcgacttcgacttgaccgccgtcttcgatccggacgccaccacggccgaaggcgtggccgccgcctatggcgccgcccctttcacctccgctgaagacttcgtggacgccggtctggatgcggcgatcgtatcgacgccgaaccgcttccacgccgaagtgggcgtggccctgctggagcggggcgtccacgtgctggtggaaaagcccatcgccgccaccgtcgccgacgcccagcggatgatcgatgcggcccgggccaacagccgcgtgctgatggtcggccaggtggagcggttcaacccggcggtcgagaccgtcaagcgcgccgtggccgacgacgacatcatctccatccaggtcacccgcgtcggtccgttcccgccccgcatgggcgaggtcggcgtggtcatcgacctggcggtccacgacatcgacatcatccgtcacctgaccggctcggagatcgtcgaggtccagcctcagctggtccgcagccgcgccgagcgtgaggacacggccctgctccagttccggctggctgacggggccatcgcccacatcaccaccaattgggtcaccccctacaagacccgcacccttcaggtcgccaccaagaccaagttcgtggtcgccgatctgatcacccgccaggtcaccgaatatttcggccagcagccggacggctcctactccacccgcatgctgaacagctggccggccgaaccgctaaaaaaggagctggaggctttcgcccacgccatccgctcgggcgagccccccgccgtcaccggcgaggacggcctgcgcaacctcgaggtcgcgctgaggtgcctgggcgaggtctgaagccccgccgccttggcgaggccgcaaaccgctggaaccttgccgatcatgcgcctgtccgccgctctcaccgccctgtcgcttctcgccacagccacgcccgcgctggccgatgtgcgctacctcgccttcgacgccggcgaccgcctgacccagtcgctgacgcgcggcgtgacgctggaagtcgagcgcggcctgttcggcgcgatccgcgtcaaccgcctgttctccaccacctcgcgggggtcggcgacgttcgagcgcggcggcccggccgaggccctgtcggtgctgcccgacggcgcgcgcggcgatctgtatgaagtccggcaggtcggcgacggccggggcctggcccgcgccctatgccccgccgcgagccaggtctggctggccatcggccgcgtccgcgccgcgcgccccctctccatgcaggcggtgggtctctggcccgacggcaagtatcgtcactgcgccgccctgtcgtacgaatggcgcggcgaatgggcgacgcggccgcccggcggcggcggcaacccctgacgcggccctgacgcggggtcgtgacgcctcgcaggcgaaggcgcttctggacgcccgtcccgcgcgttatgctcgggtcatgagcgccgcctttcatccatcgccgcgtcgtcccgccctcggcccgaccgtggcgctggcgctgggcggcctggcggcggtgctgagcggcgcccttctggtcgagcccatgctgaaccgcctgaccgagagcggcgccctggtccaggcctatgacgccgcccgaggcctcgcgggacgcgccgtcgagcagacgcgcgctctggatgtcgtccccgcccccgacgacggccctcgccccgtcaacgacctgtcgccggatggcgtctggaccgctgcggatgaaccggctcgcgcgctctccgatcagctgacgttcgagggcgcgaccctgcgcctgtcgggacaggcgcccctcgccaccacgccgcaccgcctgctggaggcgcgcgagccgctgcccggcggcgacacctacgcccgcgccctgcgcgtgcaggccaacgtgcaggtggaggtgcgcgacctggctcagccgcaggcgacggcctccctatgcgacggccgcaccgtccagcggatcgccctggtgcagacggcgcgcgagttgatcctgctgccgctggcgacggacggcggcgccccttgcgcccgcctgctgtggcgccgctgaagccggtgggcgtcctgcgtttttctctggtccttatgctcgcggccctgttcggcgcgggcgcggccctgtggacctggacgcggccgggcgaccccgccctggccctgtcggcggacgagccggcggtggtcgtccacctgctggacaacggatttcacaccgatctggcggttcctcgcgcccttcttctccagcgcggcgacccgctcgctgaggccgtccggcagctcgcgcctggagagtgggtcttcatcggctggggcgacgcccgcttctatgtggaccagagcccgatctccagccgcctgcccgacggcgcccgcgcctttttcggcccgaacaatccgtcggtgctgatgctggacccggagacccgcgacccggccgaaatgtatccgaccgagggccgcgccgcgcttcgtctgtcgcccgccgccttcgaccgcatggcgggccgcatcgaggcctcgctggacctgtcgtccgtcgcgccggagatcgcggcgcaacgacccggagacgacgcccgcttcttccggagccgcgagatcttttcgatcgcgcacctgtgcaaccactggaccgcccaagtgctgcacgccgcaggcctccaggttcggcccgcccgcagcctgacctccggtgaggtgatgcggaccgtccagcgcgccgctccgctggacagcgacgcccccgccgcctagaccccgccccttcgcttttccggccgggcccgacccccggcgagcggcacgaaaggacggctctcatggccaggaaacaacacacccgcaacgcctccggtcccgccggcccgagccagcgccaactgcgcgcgggcgagctgatccgccacgccctggtcgacatcctgcgcgaggaggagatccacgacgaggctctggccggcgtctccatcaccgtcaccgaggtgcggctgtcgcctgacctgaagcacgccacctgctttgtcgaaccgctgggcgccggcgtcgaggccgcctccacgaccggccatgagagcgagatcatcaaggcgctgaacgcccacgcccgattcctccgcggccgcctggggcccaagctggacatcaagttcacgcccgacctcaagttccgccacgacgaaagcttcgacgccgccagccgcatcgaccgcctgttcgccgacccccgcgtccgcgccgacctcgaggcaggcgacgaggacaaccagtgaccgcatcaatcctcccctctgggggggggaccctgaagcgtggagggggcttccccatgcaccggcctcgagcttgccccctccaccacgctgcgcgtccccctcccccgcgacgcgggggaggatttagaatggcgcgcaggaagaagggcgaggtcgtcaacggctgggtgtgcctggacaagccatacgagatgggctcgaccgacgccgtcagccgcatccgccgcctgttcaacgcccagaaggctggtcacgccggcaccctggacccgctggccagcggcgtcctgcccatcgcgctcggcgaggcgaccaagaccgtgcccatgatgatggaggcgcaaaaggtctatcgcttcaccatcgagtggggcgtctcgaccgacagcgtggaccgcgagggcgagatcatcgcccgctccgacgtgcggccgacgcccgaccaggtgaaggccgccctgcccgccttcgtcggcgagatcgagcaggttccgccgcgtttctcggccatcaaggtggacgggcagcgcgcctacgacctcgcccgcgacggcgccgagttcgagcttcagggccgccgcgtcctgatccattcggcggaggtgaccaatgcgcccgatcccgaccacgtcgaactgaccatccgcaccggcaagggcgtctatgtccggtcgctggcccgcgatctcgccgccgccctgggcgcggagggccatgtttcggcgcttcggcgcgagcgcgtggggccgttcagcacggaaaacgccgtcacgctggatttcctcgaggatctggtgcataggggcgccgcctcggaaggcttgcttcccgtcgcgaccgccctggacgacatcccggagttggccgtgacgaccgaagacgccttttcgcttcggcagggacgaccgatcgttctgctcccccgccaggtggaaaccctcaaggatcgcctttccggcggttcccggacggtttcagcctttcagggccagaccctcgtcgcgctatgtcagttgcgggccggccggttagaacccgaccgcgttttcaatctctcctgatcgcctgatcaggggactccaacccggcctcaagcagcgcgaagcgcggtaggccaccaaggggagactctacgatgtcggtcactgctgaacgcaagcaagagatcatcgccgataacgcccgctccacgggcgacaccggctcttcggaagtgcaggtcgcgatcctgtcggaacgcatcgccaacctgaccgagcacttcaagacccacaagaaggacaaccactcgcgtcgcggcctgctgaagctggtgtcgcaacgccgtcgccttctggaccacctgaacaagaccgacgccgaacgctaccaggcgatcgtcgccaagctgggcctgcgccgctaaggcgctcggttccgagcacaaatgcatcggcgaggcgcgggcggtcacgtccgcgcctcgttgtgcaactagagcctgcccgttctgaacgacccgggcgccgcgggactgaaacggcgcaagagacgcgagggctgaaacggctctcaccacccgcccggcatgtcgccgggctcaccgggaccgagggactgaacgcctgacgctccgcacaccccccgacgggaatacgcccgcgggagacgaaagacgaaacatgttcgacatcaaacgcaagacgatcgagtgggccggacgcccgctgacgctggaaacgggccgcatcgcccgccaggccgacggcgccgtgctggcgacctatggcgagactgtggtcctggccaccgtcgtctacggccgcgcgcccaagcccggcctggatttcttccccctgaccgtcaactaccaggaaaagaccttcgccgccggcaagatcccgggcggttacttcaagcgtgaaggccgtccgaccgagaaggaaacgctggtttcccgactgatcgaccgtccgatccgcccgctgttcgtcaagggcttcaagaacgagacccaggtcgtcgtcaccgtgctgcagcacgacatggagaacgacccggacatcctgggcatggtcgcggcgtccgccgccctgaccatctcgggcgtgcccttcatgggtccgatcggcgccgcgcgcgtcggcctgatcgatggcgaactggtgctgaacccgtccatcgacctgatcccgacctcggacctcgacctggtggtcgccggcacccaggacgccctgatgatggtcgaatccgaagccaaggagctgtcggaagagaagatgctcgaggccctgatgttcgcgcacgcgggcatgcagccggtgatcgacgccatcatcgacctggccgaacacgccgccaaggagcccttcgacttccagggcgaggaccactccgacgtggtcgcctcgatcaagggcctggtcggcgaggacatcaaggccgcctacacccaccccggcaagtacgaccgtcgctcgggcgttgatgcggccaagaagaccgccgccgccaagctggtgaagaccgacgacaaccccgacggcgtcgactcgtccaagttctcggccgccttcaaggagtgcgaagccgaggtcctgcgccgcgacatcatcgagaacagccaccgcgtcgacggccgcgccctggacaaggtccgcgccatcgtgtcggaagtcggcgttctgccgcgcacccacggctcggccctgttcacgcgtggggaaacccaggccctggtcgtcgccaccctcggcaccggcgaggacgagcagtacatcgacagcctgtcgggcacctacaaggaaagcttcctgctgcactacaacttccccccctattcggtgggtgaagcgggccgcatgggctcgcccggccgtcgcgagatcggtcacggcaagctggcctggcgcgcgatccgtccgatgctgccgaccaaggaagacttcccctacaccatccgcttggtctccgagatcaccgagtcgaacggctcgtcctcgatggccacggtgtgcggatcgtcgctggccctgatggacgccggcgtgccgctggtccgtccggtctcgggcatcgccatgggcctgatccttgagccgtcgggcgagttcgccatcctgtcggacatcctgggcgacgaggaccacctcggcgacatggacttcaaggttgcgggcaccagcgaaggcatcacctcgctgcagatggacatcaaggtccccggcatcaccgaggagatcatgaagcaggccctgacccaggcctcggccggccgcctccacatcctggacgaaatgtccaaggccatggacgcgccgcgcaccgagctgggcgagcacgcgcccaagatcgagaccgtcaagatcgccgtggacaagatccgcgaagtgatcggttcgggcggcaaggtgatccgcgagattgtcgaaaagaccggcgccaagatcgacatcggcgatgacggcaccatcaagatcgccgccaacgaccaggacaagatcgacgccgccaagacctggatccagtccatcgcctccgagccggagatgggcgtgatctacaccggcaaggtggtcaaggtcgtcgacttcggcgccttcgtgaacttcttcggcgccaaggacggtctggttcacgtgtcccagatcagcctggagcgcgtcgccaacccggccgacgtcctcagcgaaggccaggaggtcaaggtcaagttcctgggcttcgacgaccgcggcaagaccaagctgtcgatgaaggtcgtcgaccaggaaaccggcgaggacatcaccgacaagatcaacgccgagcgcgccgaacgcggcgaggccccgctgtcggaagacaccggcggtcgtcccaagcgcgagggcggcgaccggggcggcgaccgcggccgtcgccgtcgcgactgatcgccgtcgctgaacgcctgacatgaagaggccccgccggatcgctccggcggggcctttttcagtgttgaacctcgcttaaccaacagcggcgcaccctctccccaatcgcccttgagggaggacggccatgtcgaccaagctgaccagcggcgcgcgccgccacagcgatcacttcgagccgcaggacacggacccgcacgagcagcgccgcctgcgcggccagctggaggccatcgactacgccgcctacgtcgccaacaaggaggtgatcggccagaccctccccccgctggacgccgcctcgctgcagaagctcgccgtcctgaccgccggagcccgcgcccgctgggccgccgaggccctgcgcgcccactccggctcgcccgccacccccgaccagaccgcccgcctcaccgccgcccgcaccgccttcgacgaactcaccgaagcctacgaagccatccgccgcatggtcgagcgggggtacgtgagtctgaagggctgatatccaagaaaaaccgcctggtggagccgaggggacggccgtgtggtcgctttcgtcggtcatggtggcagtgcgcgactcggttggttaggagatcgccaaggctctgatcggacggggagaaggtcaacgtgtggaagctggatcatgtcgtcccggcgtccgatgttgacgccgaggagcagcggctcgccgatgtgctgtccaaggcgggctacgacgtcaggaagctgtcgctgaacgcgctggcgcagcaggtgctggccgagcgggcgaaggcggtagtgatggctatcggtatccagccgtcgaactggccgcactacccgctcggcaatggcggcgtcgaggtgcgcttccagttcagccgcgaggaagatcaggtgaacgcaaagctggcgctggcttaggcctacggcaggggcacgatagtccgcccatcaggtcggcctatcgctgatctgtcccgccaatctgcggctctgcatcttggtcgagcacttcggctttctcgcgcagatggctcgcagcggcatgcatgagcgcatcaacaccttgcctccagacgggtggaattttggaacttccttgaagtgcggcgattttcaaaccgcacgttatcaggagaaaaaccgtggccgacaaaacccttgacgaccttttccacgacaccctcaaggacatctattacgccgagcggaagattctgaagtcgctgccgaaaatggcgcgcgcggctcaacatccgcaactcaaggccgctttcgaaaagcacaaggatcagactgaaggccagatcgagcgccttcagcaggtgtttgagatcatcggaaaagcaccgcgcggcaagacgtgcgacgccatcgagggcatcctcgccgagggcgatgagatcatggaggaatacaaaggcacgcctgctctcgacgccggtctattggccgccgcgcaggcggtggagcactacgagatcactcgctacggcacactgcgccgctgggccaacgtgcttggtttgaaggatgcggccaagctcctcgaagagacgctcaacgaagagtcgcagacggacgaagacctgaccaccatcgccgatgcggcggtcaacaaggacgccctcgcctccaagtcctgatctcgtgggtggaggagggggcggataaaacgctgccttctccacgcccgactgacttccgatccttgcccggagggtcagcccccaagggtcgcccgaccggtctggaggttctggttaggctccaaactggtggcgaacgtcacgcgacgactacatggtcgttgaaacgcgattggacggccgctggtctggtcgtcgaggtttcattcccggttcagcccgtggcctcgtccgcctgacggaagttcgaccggcagagcgcacgcaacgcattggtcagcgaccgaccctcaagctgcgcccggatgcccgtgaagccttcgcgtttgagggctgcggcgatctcgcgaaggtcacggcacgaaccgctttcggcgagttgataggcacgttcgaggcaggtgggtcggcttgacatgacgtgatggtgtggacgacctccgcctgacgggctgttctgggtgtgtcgtcatcagggacgtcatgtgtggacgacctccaagacgcaagagtggaaacgacgttggcgctcggtcgagtgcagtcatgtgttcggcctgttgatgcagctgtttgcgctgctggccctgatgaagtccgcggaccggctccctaatcacgtcaacgcgctcgaggcgctctgaccccctgggtttcaccgatccccggctgcggccggttcgtcatcacgtctcaccactccttcgtctacggcgccggtcctgggtgaagaccggcccgatctctatgccgctgtgggcttgtagtcctcctgtcgcgccatcagggtccaggcgatgcgagccgtcttattggccaaggccacggcggcgaccttcggcttcttgcgttcgaggagattgccgacccagccctcgcgtcctcgctgccgggccattcgcaggaccgccgtggccccgacgaccaggagacgtcgaaggtagctgtcacccatcttgctgatgccgccctggcgttccttgccgccactgctattggcccgcggcgtgagtcccagccaggctgcaaactgccgaccggaacggaagagactcggatctggcgcgctggccgccatggcgctggcagtgatcggcccgatgcctgggatggtcgccagtcgccggctcgtctcatcctgccgatgccaatcgagaatccgacgctccatacggctgatctctgcgccaaggtgttcgagctgttctgccagcccgccaagcgcggcatgcgccagatccggcagggcctgaccctcttcacgcagactcttcagcgctgcccgcaccccagctggaccttgaggcgcgacgatgccgaactccccgaggtggccccgcggtgcgttgatcagcatcgttcgctgacgaaccaggagatcccgggtcttgtgcagcatcaacaccgcctgctgggccttcgacttcacagccacgaaccgcatggtcggccgggtgacagcctcggcaatcgcttcagcgtcggcggcgtcggtcttgccgcgcttcacataggccttcacgtacgccggcggcatgagccgaacatcgtggccgatcgccatcagttcacgcgcccagtggtgggctgaggcgcacgcctcgatcccgatcaggcacggcccaatcgactggaagaaggccagcacctggccgcgccgcagttgccgtctcacgacgaccgtgccgtctgtggctacaccgtgaacctggaaaacagtcttcgccagatcgagcccgacgacagcgatggtctgcatgataccgctcctagacgtgacgtccctgatgacgacacacccagaacagcccgtcaggcggaggtcgtccacaccatcacgtcaatagatcggatcgttcgccgctcaccccacagtccgaccgtcagttcgatgaggttaaggtagtggaggtcagtctttcgggtgcgctgtttcgcaggatcggacctgaacagttcgaacacttcacgcatcgtcttttccgttgggacggtcgatgtcacggagaaaggctctggccagatggcagagcgagccgggacgctcacagagaccccggaggcttcgatgtttctccaatccgcttcgaacgcggcagcgaccatccgagccttacggatagcctcggctcgatagcctgtcccgagagacttcacgacgtgcgtcttgccgatcacgcccgccaatgagcgcggaacacgaagtcgaaggtagtaggtcgatccccggacgatcaggccaaacgactgccgccgaaattgaggagaccgtggaggcggtgggacgagccgtttggacggtgtgtgcgccggtgtggtgctacaggcgcgggagcctgaaccgactgtagaggaacgctttttcgacggtcgctttggggccgtgtgacacagcgtggtgtcagaattctcgcctgatcctgtccaaacccctgtggaacaaggatttggtggagccgaggagtcgaacccctgacctcgtcattgcgaacgacgcgctctaccaactgagctacggccccggttccagcgggctggtcgggcctccaggcaggggcgggacatagaaggcggggggcgggtgtcaaccggcggatgcggcgaaagcgccccttccgctccgcccgggcgcaaaacattgtccacccggccacggccgcgctaaaagccgctccacgcgtcatcaaggagagcgttcatgagcgaagccattgtctggctggtcaacgccgtcatcaccctgatggtctgggccatcatcggctcggccatcctgagctggctgttcgcattcgacgtcatcaaccaccgcaaccggttcgtgaaccagctggcgacgttcctggacacggtgacccggccgatcctggagccgttccgccgcatcatcccgccgctgggcggcatcgacatctcgccgatcgtggtgctgctgctgctgcagttcgtgcgcatcctgttcaacaacatggcggcgccgtcgctgatcatgctgctgggctgatccgttgacgccgggacacggccgcgcgggaatctggcggggcgtcggccttgcggccttgcgcgccgcccccggcctgcccaaggtggccggcccttcacgcagcaggtccctccgggttcgccctttatgagcacgatcaagacagtggccgtcatcggcgccgggcagatgggctcgggcatcgcccaggccgtggcgctgggcggctatgcggtgcgcctgttcgacgcctcgccggagcggctgccgcaggcgcagggactgatcgccgccagcctggcgcgccagaccggccggggcctggtggcgcccgacgcggccgacgccgccctggagcgcatcgcgcccgcggcttccgtcgccgaggcggtgtccggcgccgatctggtgatcgaggccaccgtcgaggacgaagcggtcaagaaggccgtctacgccgaagtcgtgccgcacctgtcggccggcgcgctgatcgcctccaacacctcctccatctccatcacccggctggcgtcggcgacggatcggcctgaccggttcgtgggcctgcacttcatgaagcctgcgcccgccatgcggctggtagagattattcgcggcatcgccacatccgccgagacccacgccgccgccgtcgccttcgccgagagcctgggcaagaccaccacggacgccgaggactttcccgcctttatcgtcaaccgcatcctggtgccgatgatgaacgaggcgatcttcgccctgtacgagggcgtcggcaacgtcgcctccatcgacaaggcgctgaagctgggcgccaaccatccgatgggcccgctggagctggcggacttcatggggctggacgtggtcctggccatcatgaacgtgctctacgacggcctcgccgacagcaagtaccggccctgtccgctgctggtgaagtacgtcgaggccggatggttggggcgcaagagcgggcggggcttctacgactattccggcgacacgccggcgccgacccggtgatgcggatggagctgccgggccaggtcgccgtcgcgccgcgccgccagacctcggcgcacgtggccgcggccgtggcgggcgccgcctggcctccgctgatcctcaccctgccgttctggccgccgaacacctggatgcccggccccgagatggattggcgcctgatgatcctgctggtgggcctcatcgccacgcccctgtgcctgtggcggctggggcgcgagcgcgagcgtcacgggcggccggcgacgcggctgggcgtggtgtggcgctttgtcttctatggcgggctgctggccgcagggttgcaggcgctggtggcgctcgccatggccgtcgcgggctggctggaggcgggcgatcccgcccaggcgctgggcttcaccgagaccacgcttctgatcttcggcgtcggctttctgccggtcgcggtgatggtggggatcagctacgccctgtgggccggcctgtgcgcggcgttcatcgcctatgagcctcagggcgaggcgccggatcgcatgaacagggtggtgcgccgcaccatctgaccgccggcctggccggcgccttgttgggggacaaggacgatgaccatggacgcttctgctccgccgccttcgcgcgaacgcatcgccaccctggacctgatccgggggctggcggtgctgggcattctggcggtcaacgccgaagggttcgccgcgaccttcagcgcctatggttcgcccggcctgtggcccttcccgaacgagggcgcgtcggccgcggcgaagtggatcgtggacgcctttttccatcagaagttcatcagcctgttctccatgctgttcggcgcctccatctttctggtgggcggcgagcgggacgagcgcggcgcggaggagcgcggccggcgcctgcgtcgccggctgttctggctgttcgtcttcgccctgttccacggcctggcgctgtggtggggcgacgtgctgctgctttacgcctggtcgggcgtgttcgtgatgctggcgcgctcgtggtcggtgcgcaggctggcgatcgtgggcggcctgctgttcggcctgttcgcggccctgcagatcctgggtgggcttgcgctgcagttcgcgccggccgaggtccagacccaggtcgccgccgccaccggcgccacgcccgaacggctggccgccgtccgggccgagatcgcggaggcggccgggtcgctggccggcgcctatcgccagaacacgtccggctggatgtcgcttcaggcgcccagcgtcatggcctttgtgtttcccaccaccgggctgatgatgatcggcctggcgctgttcaagtccggctttctttccggcgcccgatccctgcgcgcctacgccgtcaccctgtccatggccgccgccgccctggttgtggtggcctggctggagtgggggcaggtgatgaacggcgcggagtcgccgctggccagcggcgtcgacttcctgctgaacccgctgatcggcctgggctacgcctccatcctgatcctgttgtggaaggcgggtcgcgcccgcgccctgtcgccgctggcggcggccggtcgcatggccttcaccaactacctgacccagtcgctcatcatgaccaccctgttctacggcggtcgcggcttcggcttgatgggccaggtggaccggccggccctgtgggggatcgtcgtggccgtctgggcgctgcagctggtctggtcggcgctgtggctccggcggttccagatggggccgctggagtggctgtggcgttcgctgaccgagggacggcgcctgccgatccgccggacggcctgatccgccttttccccgccggcttcacccgctaacgacagggcatggccgctcccgacacgcccgccgagaccttcaagcgcgccctgtcccacgccgcccgcgccctggccgagcagccggagctggaggtcctgttcggcgcggacggcccgcgcctggcgaacggcgtcctgaccctgccccatccgccgcgcgacccgtccgccccggagagcgcctcgctgaggggacaggccgaccggctggcgctgcggctggccaatcacgacgcaggcgtcaacgcccgcctgcgcccgatcgacactgcggccgccgaggtgttcgacgcggtcgagcaggcgcgggtcgaggcggtgggctcccacgccttggccggggtgcgcgccaacatgaccgccgccctgctgacgcggctggagaagaccggggccctgcgcgtcaacgatcccgaccgcgtgccggtgtccgaggccgtggcgctgctggtgcgcgagcgcctgaccggccagcgcacgcccgacggcgccggcgccatgctggacctggtgcgtgagccgctggagctcaaggccggccgccagatcgacaccctgtccgaggtcgccgccgatcagaccgccttcgccgcccgcatgcgcgaggtgctgcgcgcgctcgacctcgatcccggcgacggccagggcgaggacagttccgacgatcccggcgaggaggagcccgacccgcaggagcccgaagcccaggaccagcccgacgaggacgaggagcaggacggcggcgaaggcgaccaatcgatggagggctcggccgacgactcgtcctccgagcaggagcgcgacagccgccccgagggcgcgcccgccgatccgagcggcgaggcgtcggaggacggccccgaactgaacgagggcgaccagcccaaccgccagcaggcgcgcgacgacggccgcccggtggatttctaccgcgtcttcacccaggcctatgacgaggtggtggacgccgccgacctgtgcgacccgatggagctggaccggctgcgcagcctgctggacggccagctcgcggtgctgtccagcgtcgtatcgcgcctggccaacaagctgcagcgccgcctgctggcccagcagaaccgttcctggatcttcgacctcgaagaagggatgctcgacaccgcgcggctgacgcgcatcgtcaccgacccgtcggcgccgctcagcttcaaggccgagagcgagagcccgttccgcgacacggtggtcaccctgctgctggacaactcgggctccatgcggggacggccgatcatggtggcggccgtctgcgccgacatcctggcgcgcacgctggagcgctgcggcgtcaaggtggagatcctgggcttcaccacccgcgcctggaagggcggccagagccgggaggcttggatcaccgccggcaaacccgccaatccgggtcgtctgaacgatttgcgccacatcatctacaaggccgccgacgcgccctggcgacgcgccaagaagaacctcggcctgatgatgcgcgagggcctgctgaaggagaacatcgacggcgaggccctgctgtgggcgcatgaccggctgctcgcgcgcaccgagcagcgccgcatcctgatggtgatctccgatggctcgccggtggacgactcgacccagtccgccaacgccgcgctttacctcgaccagcacctgcgccgcgtcatttccgacatcgaggagcgctcgccggtcgagcttctcgccatcggcatcggccacgacgtcacccgctggtatcgtcgcgccttgacgatcgtcgatgtggagcagctggccggcgccatgaccgagaagctggccgagctgttcgagaccgaaccggctggcccaagtcgcgcgcagggccgcacacgcggtcgtcggcgcatcgccgcatgatccgcctgcgtcgcctgctgggcctgggcgccgcgctggcgctcgccgcctgcgccgcggtcggcagcgcccagcgcccgatcctgcctgcggaggacggctggacgcctcaggtgatccagacccgcgccgtcagcctgggactgccgggcggcgccgagcttgcgccgggcgtgcgcttcatgggcggtctgcagatcagcgccccgcccggctcgccgatccacagcctgtcggatctgaagcgggtcggcgagcggggcctcgtcagcgtctccgacgtcggagacctggtccgcgccgagcttcggctggacggctccggccgcctgatcgggttggaggggatgcgcagccgccgcctgcccgggctcgacggcctgccgatcaccgacaaggcggccggcgacgccgagggcctgctgctgacggacgatggcgacctgctggtctcgttcgagcgcgaccaccgcatctggagctacggcccgctcgcccgaccggcttcgcgcccgatccccatgcgccggcccgacgcggcgttcgaggggaacgccggcatggagggcctggcgagcacgccgggcggcggctggcgcgtggcgggcgaaggcggcggcgtctgggactgcgatccaagcgcctgccggaccgtgcaggcgcccccggccacacccctgcccgacagcgcgtttcgcatcaccgccctcgaccgcgatccttcaggcgacggctggttcgtggtgcagcggctctaccgcgcgcccatcgacatgcgcgcccaggtgcggcggatggcgcccgacggcggcctcggcccggtgctgatctcgctgaagcttcccggcacgaccgacaatttcgaaggcgtctcggccgagcggctgaacggccggacgcgcctctacattctttcggacgacaacttcaatccggcccagcgcaccttgctcttgggcttcgacgtggactgagcctgctcgcgcgcgcgctccagcgtcaccccgtcgtcagagacgggcgccccgaccagcgccttgacgaaatcatcgcgccagaccgccacgtcggtcttgcgcaccacgtccatcagcgcgctccacttccggacgcgttcggccagcggcatggtcagggccttcttgatcgcctccgacagctcctcgcggctgtagggattgaccagcagcgcctcgcccatctgctcggccgcaccggcgaaccgcgacaggatcagcacgccgggatcatccggattctgcgccgccacgaactccttggcgaccaggttcatgccgtcgcgcaagggcgtcaccagcccgacccgcgcggcgcggtagatgcccgccagctggtcccggcgataggtgcggttcagatagcggatcggcgcccagtccatgtcggcgaaggcgccgttgatgcgcccggccagcgcgtccagccgcgcgcgaatgtcctgatagctgtcgacgtcgtcacgcgagatcggcgtgacctgcagcaggaacacctcgccgcgctggtccgggttgtcctgcaggaactgctcatagcccagcagccgctcctccagccccttggagtagtccagccggtccacccccacgatcatggagcggaacagggccgaggccgccatccggtcataggtgcgcgtgcccagcgtcgagttcctggcggccatgaagccgtccacgtcgatgccgatcgggaacacgcccgtctgcacatgacgcccgaagcagtccagcccgccgcgcccgtccacctcgccccgcgcctccgtcaccacatagtcggtgaacaggtccatccactcgcgcgtgtgaaagccgatcaggtcgaagtcgaacatcgactccaccagccgccgatggtgcggcagggtgaccagcagttgccgcgtcggccacggcgtgtgcaggaagaagccgatgcggttggtgatgcccagccggcgcaggtcccgcgccatcgggatcatgtgatagtcgtggatccagatgatgtcgtccggctggatcgccggcgccagcacctcggcgaagcggcggttcacccgctcatacccctcgccgtaggaccgctcgtactgggtcaggtccacgcggtgatggaacagcggccaaagcgtcttgttggcgtagccgttgtagtattcgtcgacgtcctgcggctccaggtcgaccaggccgacggtgacgcccgcacggtcctcgaccttcatctcgccggtccagtggtccaccgtctcgccggaccagccgaaccaaaggccgtcgtacttccgaagcgccgccgacagcgccatcgccagccctccggccgagcccgccgccgggtcggcgggggcggacacgcggttggatacgacgatcaggcggctcatgacttcacttcaggcggcgctccagccccggagcggacgatcaacgcacgtccgtccaggaacggctcagcagcaccgcgcaattgatgatccccacaagcgaataggtctgcggatagttgccccaaagctcgccgtcatcgacggaaatatcctcgctgagcagaccggccgaggtccgccgggccagcatctcgtcgaatatctggcgcgcctcgtcgatgcggccgttctgggccaaggcctcgatgaaccagaaggtgcagaagttgaacgccgtctccggctcgccgaagtcgtccggctcgacatagcggaacaggaacgctcccttcttcaggtcgcgctcgatcgcgtcgaacgtcgccacctgccgcggatcatgggcgtccaggaagcccaggtcagtcatctgcagcagggatgcatccagctcgcgattgccgaagctggcggcgaaacggccctcgtcgggcaaaaaggcctcccgctcgatccgttcacggatgatcgccgcccgctcgttccagaactcgggccgatccgccagccccaggtggtccgcggccttggccagccggtcgcaggccgcccagcacatcaccgacgaataggtgtgcacccgcgcgatggtgcggaactcccacagccccgcatcggtctggtcgtgcatggcgaaggcgcggtcgccgaccttttccagcgcgtggaagtcgtcaacggtgcccggccgcagcaggcgctggtcgtagaaggcctgcaccagcggcagcacgatctgtccgtacacgtcatgttgcaggtgctcgtgcgcctggttgccgatgcgcaccggcttcatgccgcgatagccttcgaccgtctcgacgatgctttcgccgatgccgggctccagaccgacgccgtagaccggctggacgtggccgccggccgagtcgtccaccaggttgcgcagatagacgagatagccttccaggatgtccaccgcgcccagccggttcagcgcacgcaccgtgtaataggcgtcgcgaatccagcagtagcgatagtcccagttgcgcccgctgttctggaactccggcaccgaggtggtcatggccgcgacgatggcgcccgtctcctcataggcgcagagcttcagcgtgatggccgcgcggatcaccgcctcctggtagtccagcggcaggtacagcttgcgcacccactcctgccaataggccaccgtgcgatccagcgccgactgcacgcccgggcccacgtcctggtcgtagccctcgtccgggccgaagaagaaggtcagttcgcgctcgagccggaaggtgcgctcgttcagcacgtgcgacaccggacagtcggtggtcagccggaacgtcacctccgggcaacgatagcggatgtggttggagccggaggtgtgctcggcctctcgcgcgccccaatcggcgctgggcttcagccggatggccacgcgcggcgtgcccttcagcggccgcacgatgcgcccgaacgccagcgggcgataggtgcgcgaatgcttgggatggcgcggggcgaagtcgatgatctcgacctgggcgccgtccttgtcggtcagcaccgtgcgcagcaccggcgtgttgcggacataggcctgctcgacgctttccagcccctccagatcgacggcccagaagccatgctccgggtccgagccgttcatcagggccgagaacaccggatcgccgtccacgcgcggcgcgcaggcccagacataccggccctgccggtcgatcagcgcgctgatcgagcagttgccgatgggaaagaggtcgaggttgggggtcatgctcacgccttggtcaccgcttccagccagtccagaaccgcatcaacgcccgacaatccatatcgagccgccgtttccctgacgggccccaccaggacgccgaagccgccgagcgcctcggccgcgcggaagccgtgctcgtccgtcaggtcgtcgcccagcatgatcggcacggccccgttgaacggcgcctcggccatgaaggcctgcaccgccgtgcccttggttgcgcccggcgtcttcaactccagcaccatgtgtccgggctggagcgacaggccggtgtccgcctccagctgttgcgccagccgcgccgcctcgccttcggcgtcgggcgccaggcgatagtgcaggccggcggagacccccttgtcctcgacgatcacgcccggccgatccgcggcgaaggccttgaaggcgcgcagcgcctcgaccacgccctcgtcggccggcgggcgcaccaccgagccgtcgcgccggcgccgctccagcccgtgcacgccggacgccgtcggcatggcgcggtccgcgatgcggtcgatctcggcgatggtccggccgctgacgatggccacccgtccctccagccgctggtccagcgcgcgcagcaccgcagtccggcgcgaggtcgggaccaccgcgtcgggcgtcggggccatcggcgccagcacgccgtccagatccaggaacagggccacgccttcggcgcgaatgggcggcggcggcaacaggaggtcgactccggcgaaagagggcatcggcaactcgggtgtgcgacggggggaggacgcccgccttctaacacccaaatacggtaaaggttgacggcgaaacgacttgggcgttcagaaagcgccccacattcgccgccgagcctgtggaaggggctcttcatgctgtcgaacatcgttccgtcctctcccgaccagatcgcctccatgagcgagcgcgcccgcgaggtcgtgcggctgaacatcgaggcgctggaggcgctggagcgctcgatcgacgtgtcgctggcccgcgcgtgcgacatcatcatgggccgtccgggctatgtggtggtgaccggcatgggcaagtcgggccacatcggcaacaagatcgccgcgaccctggcctccaccggcaccagcgcctttttcgtgcatccgggcgagatgagccacggcgacctgggcatgctgcggccggacgtgacgctcttggccatctccaactcgggcgaaagccgcgaactgcgcgacccgctgctgtactgccagcgcaacgacattccggtgatcggcctgacccagcgcgcctccagcttcctgggccgtcactcggccgtgtgcctgaccatgcccagcgtcgccgaggcctgtcccaacggcctggcgcccaccacctccaccctgatgacgctggcgctgggcgacgccctggccatggtgctgatggaccggcgcggcttcaccgccatggacttcggcctgcaccacccgggcggctctttggggatgagcctgcaaagcgtgcgcgaatggatgggcgacaacgccgccgcccccgccgccgtcccgcccgacgccggcttcagcgaggtggtctcggcggtgacggaaggccgcaagggcgccgtcgccgtgatcgagcccaacggccgactggcggggatcgtcactgacggcgacatccgccgggcgttccagcgcgacatctcaggcctccaggcccgcgacatgatgagcacccacccgatcaccgtctcgcccgaggcgcgcatgagcgacgtggtggacctgctgaccgccaacaagatcgccaacctgttcgtggtcgaggacgaacgccccgtcgccatcgtgcacatcgccgaactgatgcaggccggctacgtctcctgacatgaccacccgcgtcctgttcgacgtcagccggctgatgagccggatcgagcgcggctcgcccacgggcgtggaccgcgtctgcctggcctatgccgaatggctgtcgaatcgtccgggcgtccagatgatcccggtgcgcggtcgcaaggaccggcttgtcgctgtcgatcccgcctggttcgagcgcaagatgcgcaccttgcgcgcccgctggagcggcggcgaggcggaccggcccgagaccgagcgccagcgtcgcctgttcgccgccctgctgtcgcccacccgacccgccgcctccgtgatcgacgagccgcccccgccggagtccgccacgccgcgcaaggcggcgccctggcgggtgtggcgccagtatttccgctctgagccgacccgcgccccctcgccggtcggcgatctctacgtcagcgtcggccacaccggcctgcacaccccggccatcctccaggatctggaggcgcggggcatcgcgcgcgtgatcctgatccacgacctgatccccgtcacccatcccgagttctgccgccccggcgacggcgacaagcaccgcgcccgggtccgcaacgtcctgcgccacgccagccgtgtgatcgtcaactcggcctacaccggcgatgaactgcaggcctttgcgcggacggagggcctgctgtgcccgcccgtccatgtcgcccacctgggtctggagccggacttcctccaggcccgcgaacctcggcccgccgtccccttctttgtgcacatcggcaccatcgaggcgcgcaagaacctggcctttctgctgaccctctggcgcaggctggaggaacgcaacggcgacgcctgcccgcgcctggtgctggtcgggcgctacggctgggagaacgaggcggtgctggaccacctccagcgttcccccaacctgcagggcctggtgcaccaggccgagaacctgccggacgccgccctggccgccctgatgcgcgacgcccgcgcggtcctggcgccgtcgtcggtagagggcttcgatctgccggcggtggaggcctcggccatgcgctgcccgctgatcgcctcggacatcccggcgcaccgcgagctgatcgggcacgcgcggctggtcgatccgctggacggccccggctggatcgaggcgatcgaggcgctggccggcgcgcccgccggatcgggacccgcctatgacgccccgacatggaaaagccatttcgcggttgtggagcaggcgcttgacctgcccccggtcgaggtcgcctgacgcttgcctatggccgtcgtccgctaagcccggtatggacacaagcagcacggaaatcagagacttcatgcacacgcgcgcgcttcttccccgcctttcgcttcgggtctcggccctggccctgaccgcggtcctcgccggctgctccaccctgccccgcgacgggccgtcgggcgcctccgtcaacgcaggcgcgaccacccccgaggcgttgggcagctacgccctggtgccgctgacctatgaggtgaccgagcggatcaaggcggtgccgccgcagttcttcggcaccttggcgctcgcctccagcgaccagcccgccgacgtgatcggcgagggcgacaccctggcgatctcgatctttgacccgtcgggctcgctgttcggcggttcgctgggcgcctccagcgccaaccgcgccgccacgcttcagggcggcagccagaacttcaccggcgtcgtcgtggaccgcgcgggcaatgtggcggtgccctttggcggccccgtgcgcgtgcagggcctgacctcgacccaggccgccgccgccatccgccgctcgctggtcggcaaggtcgccaatccgcaggtgctggtctcggtcgcgggcaacgtctccaacaccgtcaacgtcctgggcgacgtgcgccagccgggccgcgcgccgctgggcgtcaacagcgaccgcatcctggacgtcatcgccgcggccggcggctcggcccgcaccaacgacgacctgatcatcagcatccagcggaatggcgagaccttcaccgcgccgctgaccgccgtcaccacccagttcgtcgagaacgtgcggctgcagcgcggcgacgtggtcaacgtccagtacaagccgcgccgcatctcgacgttcggggcgctgaacgcggtgacccagatcgacatgcccgccggccccatgaccctgacgggcgccatatcgcgcgtcggcggcctgaacaccaacaccgccaatccgcgccgtgtgctggtgttccgcttcgagcggcccgaggtcgcccaggctttgggcatcagccagccggccacgccgcgcggcgtgcctgtggtctatgagctcgacttcaacgacgccgccaacgtcttcgccgccaccaacatggagatcatgcccgaggacgtgatctatgtgccgctggccggcgcggccgagatgcgcaaattcttcgaagtcgtgcagagcctgacgcgcgtcgtctacgacgtctcggtcaccagcacgctgaacaacgactgatccgacgatggcgggccgctggcgcgcctggctgccccgccgccggagcgcgcctccggctccggtggaggcggatccgttcacgccgccggccgacttcgagccgccgcccgaggacgatcccctgtcgctgctgctggcggagatccaggcaggcgcgctggccgtctatgatcgtcacggcctgccgacgcggcttggccactatgtccgcgatccggctgacggcgaatggcgcttcatcgccgaacggctgtcgccgacccggcgcttcgagctgatgctggagcatccgccggaagagggctggcgcttcgcccggctggaggatctgggcgcgcgtcaccgcgaccatccggaggtcgaggtcgcctccgaactgctgaacgccgtgtctcgccttcgccagaaccgcgcctcggccagcgccgacgacctggccgaggccatccggctgggccaggcctggcgcgctctgaacgcgcccagcccggagctcgagaccctctccgccgcgcccgaggcgatcgcccaggcgtccgattcgacgcgcgcgccgctggcgcttcgcccgccggacaagcccaagcgccgccgcaagcgctgacagccgtcccacgccgcgctagaggacgcgcctcctccccgacctttcgagcgcctttctcatgtccgacgcccttccccagcccccagccggccagccggtcggccgcgtcatcgccatgccgggcgacaccaatcccgagggcgacatcttcggcggctggctcttggcccagatggacctggccggcgctacgcccgccttcgaactcgcctgcggccgctgcgccacggtggcgctggacggcatggtgttccaccagccggtgtcggtcggcgacgaggtgtcgatctacgccgaggtggtggggacgggccgcacctccatccgcgtccacgtcgaggcctggaagcggtcgcgcaaccagcctcaggccgcctccgtgcgcgtgaccgagggcgtcttcacctatgtggccatcgacggcgagcgcaagccccgccccctgcccggcaaggcgtgaaatcttgacctcgcggcggggcggccctacgtcccgacaatggccgtccgtcgcatcctcaccatcgacaatcccgccgatctggcgatcctgaagcaggtgtcccagccggttccggcggtggacgacgccgtccgcgccctgatggacgacatgctggagaccatgtacgccgcccccggcatcggcttggccgccgtgcagatcggcgcgctggaccgggtcatcgtcatggatctgggcgaccgcgacggcgacgttcccgaaaccgaagaggaagaggcggagaacgccgaggcgcgtcgcaacccacggttcttcgccaatcccgagatcctgtggtcgtccgacgaactgttcgtctacgaggaaggctgcctgtcgatcccggagtatttcgacaaggtcgaacgcccggcccgcgtgcgcatccgctatctgaaccgcgacggagaacaggtcgaggaagaggcgtcgggcctctacgccgtctgcatccagcacgagatggaccacctgaacggcgtgctgttcatcgaccacctgtcgcggctgaagcgcgaacgcgccgtgaccaaggtcaagaaggccgcccgcgaaaggatcgccgcctgatgcgcctgccctccgacgaactcgccaaggaccttccgcgcaccgccgctcgcatttcgcgccgcggccgttcgctggtgatcgacaccaccggccgtcgccgtttgacccgcagccagaaggccggcgtcgcgggcgtggcgacccttgccggcgtcgccctgctgggggtcgtggcgggtctgctgctcgatcgcctgctggacttcgacgacgcgctggacgccggcggcgagtgggacgagggcggcggcgtcttcacccgctggcagtaacctctcccgtcctctaaaggcgtgcccatgcgcctcgcctttatgggaacccccgacttcgccgtgccgtcgctggccgagctgatcgcctccggccatgaggtcgtggccgtctattcacagccgcccaagccgaaggggcgcggccggaagctgacgccctcgcccgttcacgccttcgccgagaccatgggcctgccggtcttcactcccgcctccatgaaggccgccgacgccattgaggtgttcgaaagcctggatctcgacgccgcctgcgtcgtcgcctacggccagattctgaagcccgccgtgctggaggcgccgcgcctcggctgcttcaacctgcacggctcgctgctgccccgctggcggggcgccgctcccatccaacgcgccatcatggccggggaccggcagaccggcgtccagatcatgcgcatgagcgagggcctggacgaagggcccatcctgctgggcgaggtcatggacatccgccccgacgacaccgccgccagcctgtccgagcgcatggcccacaccggcgccgccctgtggccccgcgcgctggccgccatcgaacgcggtggcgccaccccgaccgaacaggccggcgagccgacctacgcccgcaagatcaccccggccgaggcccgcatcgactggagccgccccgccgccgagatcgacgcccgcatccgcggcctatcgccctttcccggcgcctggttcgaggcgccgtccgccgaaggccccgtgcgcgtcaaggcgctgctgtcgacgcccgccgacggatcggccgcgccgggaaccgtgctggacgatcgccttacggtcgcctgcggctcaggcgccgtgcgcctgctgcgggtgcagcgcgagggccgcgccgcccagtccgccgaggacctgctgcgcggcttccccctgcccgccggcgccgtgctcggctgatgccgcgctatcggctaacggtcgagtacgacggcacggcctacaacggcttccaggcccaggccgaccagccgacggtgcagggcgcccttgagaccgccatcaacgccttttcgggcgagcgcatccgcatcaacgccgccggccgcaccgacaccggcgtccacgccacgggccaggtgatccacgccgacctccagcgcgactggccggccgcgaccgtcatgaacgccatgaacgcccatctggcgcgcgaaggcgtctgcgtcctggactgcgcgcccgcccccgatccggaatggcacgcgcgcttttcggctgtgggacgcgcctaccgctaccgcatcctgaaccgtcaggcccagccggtgctggagcgcaaccgtgtctggcacgtgcgaaagccgctggacgccgaggccatgcatgcagcggcgcaaggcctggtcggccagcacgacttcaccaccttccgcgacgtgggctgtcagtcgaaatcgccgatcaagacgctggacgtcgcccgcgtcgagcgccacggcgaggaggtccacctggtgttcgaggctcgcagcttcctgcaccgccaggtccgctccatggccggcaccctggtcgaggtgggcctcggccgctggacggacgaggacgtgcaggcggcgctggacgcccgcgaccgcagcgcctgcggccccgtcgcgccgtccgccgggctttatctgactggcgtccgctacgattgacgccctcgcgccgtcaccctcgggcttgacccgagggccggatgatccgccgtattgcgccaaccgcttcgcacgcgcgccttcgcccccgatcctcgggtcaagcccgaggatgacgggcaaggcggttacaccttcgagaacaccaccgtgccgttggtgccgccaaagccgaagctgttggacatcacatgggtcagttcgccgtccttgcgttcgcgcaggatcggcatgccttcgaacgccgggtccaggttctcgatgtgcgcgctctcggccgcgaagccgttctgcatcatcaagaggcagtagatcgcctcctgcgccccagcggcgcccaatgagtggcccgtcagcgacttggtggaggagatcatcggcatccggtcgccgaacacggcgcgcacggcctccatctccttggcgtcgccgaccggggtcgaggtgccgtgcgggttcagatagtcgatcctgggattgccggcctgttccagcgcgatcttcatgcagcgctgggcgccctcgcccgaaggggcaaccatgtcgtagccgtcggcgttggcgccatagcctgtgacctcggcgtagatggtcgcgccgcgcgccttggcccgctcgtattcctccaagaccacgatcccggccccgccggcgatgacgaagccgtcgcgatccttgtcataggcgcgcgaggccgctgccggcgtgtcattgaagttggaggacatggcgcccatggcgtcgaacatgttggacatggaccagtcgatgtcctcgcagccgccggcgaagaccacgtcctgcttgccccactggatctgctccacgccggcgccgatgcagtgggcggatgtcgcgcaggccgaggagatcgaatagttgatgccgcgcatcccgaaccaggtcgacagcgccgccgacggaccggacgccatggccttcggtacggcgaagggcccgacgcgcttcggcgagttcttctccacggtggtcgccgccgcctgcaggatcacctgggtcgaggggccgccctctccgacgatcaggccgacgcggtcgtccttgatctcgtcggcgctcatgccggacgacttcagcgcctcttcgaaggcgatgtgcgcccaggcggtgccgttggccaggaagcgggcggcgcggcggtcgaccagttcctcccacgggccgatcttgggcggcgcccagacctggctgcggaagccgtatttggcgtgatcgggggcggcgacgacgcccgagcgggcctcgcgcagcgattgggtgacctcttcggcgccgtggccgatggaggagacgatgccgaggccggtgacgacgacacgacgcatgatgcttccttctggtgctgcagcccctcccggagccggccgcgttgcttcgcggtctagatgggggctctaaccgcccgccgcttggtccttggcgccgaaaaggccgacgcgcatgtcgttgcaagtgtagatgacctcgccatcggcctccagcacgccgtcggcgatgcccatcaccagcttacgattgatcacccgcttcagatcgatcttgtagacgaccttcttgatgtcgggcgtgacctggcccgtgaacttgacgtctccaacgcccagcgcgcgcccacggcccggaccgccgatccagccgagatagaagccgaccagctgccacatggcgtccaggccgagacagcctggcatcaccggatcgccgatgaagtgacactggaagaaccaaaggtccgggtggatgtcgagctcggcctccacatagcccttgccgtgcgcgccgccgtccgcgttgatctgcgtgatccggtcgaacatcagcatcggcggagccggcagctgggcgttgccgggaccgaacagctcgccgcgtcccgaggcgagcagcgcctccttgtcgaaggacgaggggtattgggactggctcaaggcgtttccgtttctaaactgttgttgcagcgggttacacgaccccgccggacggctcaacagcaggaacgaaggcctccggtcaggtgcgtccccgtccggcgggccgcgcggcgttgcacaacgcacgctcctgggcgccgaacaccgcccgctggctgacccagccgcgcgtctttctggcccgcacccggcaccagccctcttcgcattcgtccagcgacacgatggagcgcggctgaaggcgcgcgcgcacgccggacgcctcggtgcggcccgcgtggatcatcacctcctgcgaggaggcgttgaagacgctgcggcggcccgacgccaccgtgcggtggatccacgacaccgacccttgcgcgtcgcacacctttcgccactcgcgcgtctcggcgatcacctgaaccggcaggccggcggcgcggtattcccacaggatcggataatccagccccggcccctgccgcgcccgcacgtgcgaggacttcagcgacacccagcgcggcacctccagcccggtcggcgtcggccgcccgtccggcatggtgttccccgccgccgccatcagccccgcgccgacggccgccgcggcgaccaccgcccttctgatcctgttgcacatcgttctggacaccgaacccctgccagcagcgccgggtttgttgcgaaggcctgagggccgcgagtgtcgcccgaggagcttaagagcggattaaccaagccgggcggcgggggtccgatctaaacgcggtcttaagtcgccctgtgaaaggtgggcgcctcaggggcgcgaaaggggggcgagcgggcgtggacagagtgccggacaagcccttcgatatctgggacggcctggccttcgccgcgtcggtgctggtcgtgctgctctacgggcagatctggttcgcgcccctgaccggctatggccaggcttcggccgacccgctgaaggccgtcttctatcccgcctacatgctggctatcgcgctcgtactgctgcggccgggagaaacgttgcgtatcctgaagcgctcgccctggctgctcgccctgatcctgctggtgatcgcctccaatgtctggtccatcgcgccggacaagaccctgcgccgcacccttgcgctggtctgcacctccctggcggggatcgccctggccgctcgctggagctggcctcgctttctggaggtgctggcgaccgcctttgcgataatgggggtgctgtcgctgatgctggcggtgctgaagccggactggggccggatgaccgagttgttccccggcgcctggcgcggcgtgtgggtcgagaagaactcgctgggcagcgtcatggccctggccgcggtgacgcagatcgccgccgccgtcctgacccccaggcgcgccatggtctggagcggcgcggccgccctgtcggtgttcctggtgctgatgtcgacctccaagacttcgctggtggtgctgctgctggcgctggcggccctcagcttcatggccgtgttcaagggcggcccgctgcgcgcggtggtcgggggctgggtcgcggtggtgggcgtcgcgggcgcggcggtggtgctgaccctggcctggcggatcgccttcgacctgctcggcaaggacgccaccctgaccggccgcacaaaggtctggagcggcattctgaaccagatgccgtctcattattcgaccggcttcggctacggcgcggtgtgggacaatgaatccagcttcggcccggccatgcacgtcgcgcgcgaggccctgttcctgcccgcccatgcccacaacggctggctggaggtgctgctggcgctgggcgtgcccggcgtcgtgctgatggccctgtggctggccgagacgtggctgcggtcgatctggtcggcgttcacttcaccggccggatggttcgccctgcccttcaccctgatctacagcgtcaacatgttgaccgagagcgtgacgctgaactggcacgatctctggtgggtgatgttcgtggcggtcgccagccgcctggtgctgggggtcgatccggatcccgcctaccgcccgtctccccgtcgcgcggcggggcgtcgccgcctcggagtccgccccgcgccggcctgagcctgagcctgggcctgcgtcagccgccgcacaccgggcacgtggggtccgacgccaccctgaccgtccgcgcctcgcccgccagcccgtcgtacagcatcagccgccccgtcagcggctcgccggcgcccgtgatgatcttgaccgcctccagcgccgccattgtcccgatcaccccggccagcgcgccgaccacgccgacgcgggcgcaggtctcggcgtccggcggagtctccggcaccaggcactggtagcagggccgtcccgcgaacaccccgacctgcccgctccagcggcccagcgcccccgacaccagcggcttgcccgcctcgacacaggcgcggttcaccagaagacgggtatcgaagtcgtccgtgccgtccagcgccaggtcgaagccgccgaccacctcggccgcattcgcctgcgtcagccgccggggaaaggtctccaccgccacatgcgggttcagggcgcgcagccgtccggcccccgcctcgaccttgagccgaccctgatcgacggtgtcgaacagcacctgccgctgcaggttggacagggacacgacgtcctcgtcgatcaggcccagcacgccgacacccgccgccgccagatacagggccgcagggcttccgacgccgcccgcgccgacgatcagcacccgcgcgcgggccagccgctgctgtcccggcccgccgacctcgcgcagcaccagatggcgggcgtagcgttcgacttcgtcaggggagaagggcacccctcctcctagcccgccccgaacctccaggcgagaggcgcagagccttagggcgcgacggccatggagcggctggctttgctcagcaggctttcgacgcggcggcccgcatcggcgccgttcatggcgtccgtcgcctggtccaggaacgcggcgacttccggcgtcggatcgacccgcgccatgccccagtcgggaaacagccgggcctcgatcggctcgtcgctgaggatgcggatgccggcgtggcgggtgtctccgtccagccgcttcatcaggcggtccagatcggcgcgcgtgccctcgatcacctgcaggaaccggccttcgcagcgcatcagcacgcccgtcaggtgatcgcgccggttgttgcggtcggacgcgccgacgatgtcgatcagcggcatcaggccgtcggcggccgcgcccacggcgtcgctgacatagacgatgcgagacaagggcatgggcggtgtcgtccttgaaggtgtgaaaaacaccttggcggatcaggactgaataaaagcctccgaccggctgcggcggccggtcgcggaggcaaggggacggcttgatgggcgaggccttcgtcgccatctggcggacatgaacaccgcctccgacaccgcctcgcccggctggcacggcaccaccatcctggcggtacgcaagaacggccgcaccgtgatcgccggcgacggccaggtctccatggggccgaccatcgtaaagggcgccgcgcgcaaggtgcgcaccctcgcgaacggccgcgtgctggcgggcttcgccggggccacggccgacgccttcaccctgatcgagcggctggaggccaagctggagcagtatccggaccagctggcgcgcgcctgcgtcgacctggccaaggactggcgcaccgaccgctacctgcgccggctggaggccatgctgctggtggcggacgcccattcgatcttcaccgtgaccggcgtcggcgacgtgctggagccggaacacggcgtcgcggccgtcggctcgggcggcaacttcgccctgtccgccgcccgcgccctgatcgaggaaaccgatctggacgccgaggccatcgcgcgcaaggccatgaagatcgccgccgaggtctgcgtctacaccaacggcaatctgacggtggagacgctgagcgcctgaccgggcgctgaaccgaaggccagcgtggccgtttgaccgggcgtcgccgaccctgcgatggatggagcccgcacatgcgcgcctgcacgccccttcttgtctcgtcgatcctgctcgcgacctctctcgcggcttgcggagaccgacaccgggagacggagccttcggcgcccgcgcccgggacgccccccatcccggccgagaacgtcgccgcctcggacgcctccgccacgccgccgtcggcgggacaggccgcgcccgatcagggtcttcagggcggaagcgccgactggcgcaccgtcgcgcgcgccaccgacgccagcctgctggggcggctggaccaggcctggcgcctcggccgcgccgaggccgaggactcgggcttcgccgcccaggtcgaggcgctgggtcccttggtcgatccgaacgccgccagggccggccagcttcagccgcccccgggcgcctatcgctgccgcacgatcaagctgggccgcaaggtcgagggccaggggctggcctatgtcgactatccgccgttccgctgcacggtcgagctgacgcccggcggcgacctggtcctgaccaagaccaccggctcgcagcgcacccgcggcctgctctatccggacggcgaacgccgcctggtctatcttggcgcccaggctctgggcgacgagacgggtttccccgcttacggggaccgcgccgaccgcaaccaaatcggcgtgctggagcgcgtcggccccgaccgctggcgcctggccctgccctggccgcacgcggaggccaagctcgagctgctcgagctgacccgctgatatcgcctcagacccgcgtcagccgcaggtcctgatagtcgtaggagaagtcgatgtcgggcgacacccccttcatcgtcgccgtctccggccggccatcccgcagcgcaaaggtgatgaaggcgtcctcctcgcgcttgtccgggaagcgggtgcggaaggtctcgccgtcatagggctccagcggccccttcagcgccggcgtgtgggtgaagtccagccacaggccgcgcccccgccgcgagacgacgatgtcgccgtaccagggatcgcgccaggtcccgacgtagcggtccagcggcagcgacggccgggtccccgccttctgcttcgcgtcgatctcgacggcggcggccagcgacttttgcgttccctccgcctccagccgcttggagtcggcgatccagtcgaagccggacttgctcatgcagatgtcggctatgcccgagcgcagcgcgcgcagcagcaggctctcttccgcattggagaagatcgaaaagccgatgccgcgccccggcagcagcacggtggccgagatgccgcccggcgagccgccgccgtggctgatcagcctctcgccgcggtaatcctgcacctggaaccccatggcgtaggtcgaggcgatggcccgccccggcagctcggccgtcggaccgggcgaggagcccacgatgatgttaggccgcaacatttcgcgcgcggcggcttcggagaacaggcgcgagccgtccggcagcacgccctccttcagccgcagcgtcatccacttggcccagtccgtgggcgtggtgcagatgccgccggccgccgccgcggaatcccaattccacacctccacgatgctgtcggcgatcgggaccatgcggccctgataacgcagcggcggcccgacccgcccgtgcggcagggccgagcgcgcgggcgcggcgcggctggccagggggacggtctcggtcatgccgacgcggtccaggatgcgggtctggacgaagtcctcccaccgctgacccgacaccgcctcgatcaccgcgccggccaccacgaacatcagattgcagtagtcgtactcggcccgaaacccgttctcgatcggcacgaacgccgcctgctggatcacctcggcgcgggtgcggtcgctgttgggccagaacagcaggtcgccggcgcccagcccgaacccggcccggtggctcagcgcgtcgcgcaccgtcgcatgttcggtgatgtaggggtcggccagccggaagttcggcagataggttttgatcggctcgtcccacttcaccttgccttcgtccaccaggatggccagggccgcggctgtgacgttcttggtgttggaggcgatcgcgaacagggtgtgctcgtcggcgtgttcggcccgcccctggcgcttgacgccgtagccgcgcgccagcaccggccggccgtcccggaccaccgcgatccccagcgccggctgctcgggccaggccgccatgcactgtcgcacaaaggcgtccaccgtctcggccaagcccgcgtcgtcgttggcgggcgtctgcgcccaggcggggcgggaggccagcgccgcggcgcctcccgatgcgaacagggcggaacggcgcgacaggcgaacggacatggcaggcggcttccccgaggatagatgcgcggacgctaaggcgccgctcgcccgccgccaagcaaaagccccgcgccttgcggtcgcggggctcggctcaggtctcggtcgcggctcagagggtgcagcgcgccgtctggcccgcacgcggcacaaaggtgtcggtgcgcggattatagctcttgtagcgctgctggcaggcgcggacatgggcgtaccagttgctcgtgttcgcatagcccgagggcggcgccggcggctggggtccccagctcgtctcccagcggccataggtcgaagcttgcccttgcgtgcccgagccctgcatgccggagccctgcattccgccctgcacgcccggctccgacatataggggcggggcgtggtgttcatgccgggcgtgttcgccgatccaggccgcgtcgcggcgccgctctggccggtcatcgggcggttgggcatctgcggggcctgggccgccgggcggttcgccggggtggcggtggtcgagcccgtgcccggctggttcggccgcacgtcgggcgtcgcaggattggtggtggtctggcccggattctggcccggcgtcgtcaccggctcgcgggccggatcgcgcggcagggtcggcggcgtggtctgggccagcgcaggcaggctggcggtggtcagcagcccggcgagggctagggcgagggtcttggtcatgacggtttcctccatctggcgttgtcccccgcagatgaaccggccaaccgccgtttggtctcagcttgacgataaggaatctcgcgtccgcccgccccttgtgtggccgccgggacacgcccacttcatcgctcaagagccggccgcccgcttcagggggccggcgccgacctccgcctgatccaggggaaacagaagaaccgatgaacctcgacctctattccgaccgcgccaaacaggccgtccagtccgcccagtcgctggcgctcgcccgccgccaccagcagttcgcccccgaacacctgctgaaagtcctgctggaggaacgcgacggcctcgcccgcaacctgatccagtccgccggcggcgatccccgccgcgccgagaccgacatcgaaaccgccctgtccaagcgcgcccaggtcaccggcggctcgggccagctgtatctcgacggcgacaccgcccgcgtcttcgcctcagcggaaagcgccgctaaaaaggccggcgacgcctttgtcaccaccgagcgcctgctggccgccctggcccgcgagggcggggtggccgcgaccgtgctggccgccgccggcgccaaggccgaggcgctggacgccgccatcgccgagatccgcaagggcaagaccgccgacagctcgggcgccgaagacgcctatgacgcgctgaagcgctacgcccgcgacctgaccctggccgcccgcgacggcaagatcgacccggtgatcggccgcgacgaggagatccgccgcaccatccaggtcctggcccgccgcaccaagaacaaccccgtcctgatcggcgagcccggcgtcggcaagaccgccatcgtcgagggcctggccctgcgcatcgtcaacggcgacgtgcccgaatccctgcgcgacaagaaggtgctgtcgctcgacatgggcgccctgatcgccggcgcgaaataccggggcgagttcgaagagcgcctcaaggccgtgctgaccgaggtcgccgccgccgagggccagatcgtgctgttcatcgacgagatgcacaccctggtcggcgccggaaagggcgacggcgccatggacgcctccaatctgctcaagcccgccctggcccggggcgagctgcactgcgtcggcgccacgacgctggatgagtacaggaagcacgtcgagaaggacgcggccctggcccgccgcttccagccggtcatggtcgaggagcccactgtcgaggacacggtgtcgatcctgcgcggcctgaaggagaagtacgaggtccaccacggcgtgcgtatttccgacagcgccatcgtcgccgccgcctcgctctccaaccgctacatcaccgaccgcttcctgccggacaaggccatcgacctggtggacgaggccgccagccgcgtccgcatggccgtcgactccaagcccgaggcgctggacgagatcgaccgccgcctggtgcagctgaagatcgagcgcgaggccctgaaaaaggagaccgacaccgcctccaaggcccgcctggagaagctcgaggacgagatcgccgatctggagggccagtccgacgacctcaccgcccgctggaaggcggaaaaggacaaggtggccggcggcgcccagctgcgtgagacgctggaccgcctgcgggtcgaactggccaacgcccagcgccagggcgacttggggcgcgcctcagagatcgcctacggccagatcccgcagatcgagaagcagctggcagaggccgaaagcgccgaggccgacaggtccggccctctgacgcccgaggtggtcgacgccgagcagatcgccgccgtcgtgtcccgctggaccggcgtgcccgtcgacaagatgctggagggcgagcgcgaaaagctgctggccatggaggatgcgctgcgccgccgcgtggtgggccaggaggacgccctgatcgccgtctccgatgcggtgcgccgcgcgcgcgccggcctgaacgaccccaaccgcccgctgggctcctttctgttcctgggccccacgggcgtcggcaagaccgagctgacccgcgccttggccgagttcctgttcgacgacgaggcggccatcacccgcctggacatgagcgaatacatggagaagcacagcgtctcccgcctgatcggcgcgcctcccggctatgtcggctatgacgagggcggcgccctgaccgaggcggtgcgccggcgtccctatcaggtcgtgctgttcgacgagatcgaaaaggcccaccccgacgtcttcaacgtcctgcttcaggtgctggacgacggccgcctgaccgacagccagggccgcaccgtcgacttcaagaacaccctgatcatcatgacctccaacctgggcggccacttcctggccaatcaggacgagcacgaggaggtcgagaccgtgcgccccttcgtcatggaggcggtgcgcgctcacttccgccccgagttcctgaaccggatcgacgagatcatcctgttccagcgcctgggccgcgcccagatgggcggcattgtccgcatccagcttgcgcggttcgagcgcctgctcgccgaccgccgcctgtcgctgacgctggacgacagcgccctgcaatggctcgccgacaagggctatgaccccgcctacggtgcccgccccctcaagcgcgtgatccagaaggaactggtcgaccccatcgcccgcaaactcctcgccggcgacatcgcggacggctcaaccatcgccgtgacgacgagcccggacgggctggagattgggtaggggcggatttaatcgggcgattgtggctctaagttcgagaacaagtcggcttcgggcgcttccggtaatggaagcgccctgagcggaacaacggacagacctaaccgctcggcgaatttggccaagttcctatcgtcggagtagatcactgatgcactatttactcgcgctatcgcaatgatctgacgatcaactttcaccttctgccaaggcgcatccgatccgtcgaatttatctcccttgcggagcgcttcccgagtcatagctgcaacttcgaccgctgcacgaacatcgaagtcggctacctttatgcgagaagatcgtgaaatacggtcaagcatcgcaggaccagcatcgtcggccaagactagtacttcacttagagccggagaaggtacaatcagagtagtcttctcacgatcaagctgcacaattaaatgctcgatgcggtccttcgctctggaaacctgctcgccggtagctgggtcgattggagctctgccgtctggcgtgatcagatacgcaagcgtggtagcatcaatcaccgcgttcaatgaatttctccatcactcgcgcggatactcataagctccgtgaatgctgtcgtcgtatccgggattgacccgatacctcgcaaatcatcgagaatctcgacgagccccctatcatccaaaatctcgaatcggtcgactttgaagtcgagcagcttccaagctccatcgggatgacgttcccaacgcccttcgcctgacagccgcacctttggtccatagagatgctgcgcaagctgccgcgcgaggtcacgggtcaaagtacaacccgaaaaggttgtacttccatcctgaaggatgacatgtgcggagctgtcccggccaccaacacttacaacctgaccgtcgatcgtgcctacctggcggaaggctgggaaggtcagtggcctaggacgagtgcgccctggaaaggggatgattaccgctccaaacctcgacagctctccaaccgcgttgtcatcagccagcagatcatcaagggtcttgaaagctcgaacagcgtccttcggcccggcaccctgagctacgtcgccaagccgccggtcaaccttcggaacgtcaggtgcctccactttatgaaccaacttagcgctaccacgctcgatggcgacgaagtgggtcgaatctgcatgtcccacgaggtcggcaagcgcagcaagatacttcgccaaccgggccatcggcaaagtgtcaggagtgaagacgtcgatcttgaatgtgtattcagcgtcttgcacgtccacctcccttctctgacatgatgttctaaaactctttcataatgtcaaatgagggtaaggcgatcaaacgcttctgtcacgagagggatagcttgtccctgcggcgaatttggacatagccatgcgacgtccgcttccttggacggaccgtctgaaccctagcgggtcaacaccggcatcacctccaccccgtcgcagggccagatcgtcatgtgcgggtagccttcgaacaggcgggcggcggcgtcgtgggatggggcgcgcacgaccatgaagacggtcagcagattgacgatgtccgtcagcccctcttgcgtcagccgcttggtcgggcccagcgcgccgccgctatggacgatgctgtcgcgatgcctggcctcccatccttaatggcggccatgccggcggcgtcggtcgcgcgctgctcctcctccgtcatcgcataccaggcgcgccagcgcgggccggtcttgtccgaggtgaagacggccagatagtgagcctggtcggtcatggcgggctcctcgcagcgacgcctccagattagcgccaccgccgttcttccggccagcctccgcgtcgcacggcccggttcaacgatcttcccccgcttgtcgggggaagtgtcagcgcgtggcgcggagcgacacggctgacgatgggggaagtttcctcttgaaggagactcccctcaccgaccctggaccgcttcgcggtcgacgggccacctctcccgcaggcgggagagtaataatgcgcctgctctcctatcaacggcgaaaaaccccaaccggatcgaggccctggccgatcctcgtaccgactggcgcgccgcagcacggagacgtgcgatcctgcatccgtctcgtcgctggggagggctcgcttggcctgcgcccttgcgagcggcgggagcggatggggcgggagggggtcggtcaggtcgatcgaacccgccggcgtcggggatcgccccggcgcggggggggcgggggggatactcggccgcaccggggagcgctgtcgcagagcgccccgcccgccgcaggcttatggggttaggggataagaccgccaccatcctccgccccgagcttgcagccaaccacccgcgcggggcgtcagaccttcgtcgaaacggtacacaaccactcacactccgggcgaaggcccggcgccccgcccgccctccaaccggatgcatctcgcagaccggggctttcgcgcgaccgcaatccgccgacatggcggacagggtgggattcgaacccacggtaggcttccacctacggcggttttcaagaccgctgccttaaaccactcggccacctgtccgggagctgtgttcgagcgccggaggcggcgtcgtagcagcccggccggtcttcgccaacctttcggctcagccgagctcgcggtggaaaaaggcggccatgtccgccagcaccggagccttgcgacggaacaggggcgagaagctggcgagggtgtcggtgtggctgaggccggggtagagcctggcctcggagcggcctccggcggcgcgctggcgccggttcaggatgatcgtatcctcggcgtggaccacggtgtcggcgtcgccatgccccagccagatcgacggggcgtcgccacgcacgaacgtcacgggctgggtcagggtggggtcgggcgcgcgaccgaaagcgttgatcgaggccggcacgtcgaacggcagaaagtcgtagggaccggacacgccggcggcggcgcggatcaggcgcggccgccccgccgcctccatgtagcgccgatccagggtgatcatcagcgccagatgcgcaccggccgagtggccgcatactccaaggcgggccgggtctccgcgataggtcgaagcgatctcgccagcttttgcggtcgcggcggcggcgtcctcgatgaaggcgggaaacaccacctgcggcacaaggcggtagtccggcaggacgaccacaaagccccgggcggcgatagcttgcgcggcccagccgtagacgtcctttgatcccgagctccagctgccgccatagaagaagacgaccaccggccacggcccctcgcccaccggcgcatagacgtccagcgtctgacgcggatcggggccgtaggcgatgtcgcgccctacgcgacgcacgccgccgtcgcggggaccgacggcgttcagcaccgccagcggcgaacaggcggccgtcaaagcgccgagcgccggcgcgaaaaaacctctgcgggtcaagcctgacgatccctcttgccgatcaacgcgcgctggcgatcaactggccgcagttggcgtcctcggcaagacccggatcgacaaaggcgaacagggcggcgaccggggcggcgaccgcgccgacgatggcggccaggcccccttgcttgacaacctcgcccacatccacgccggggcggggagacgtgaacgtgccgccgatggtgatcggcgcccacacccgcaaaaggcgcggcttcttggagtcgccgtcgatgcgcaggttcagcgtctcctgccccaggttgaacgagccggagccgcgggccagcaccacgccggtgtcgatcacaaaggtcttggcgctggccacgccgcccgcgacgttgaagtcggccacggcgcaccggatctgtgtctggccctggtcgccgctgagcagcttgatcaggccggcgctggcgttgatgcccagcagctcggcgaaggcctcgcgcatccggccctgcggcaccacgacgctgagcgagcccttggaggcggcggcgaaccggtggatcgacgatccggggccctccaggcgcacacggcccagcatgcgaccgctgatcggctggacaccccctcgggccggcaccagcgattccagcggatagccgccgaggcggaagtcgatggcgctgtagggggtgtcgcgcgtggcgttgatcttggccgtgccgttcagctcgcctcgattgaagttgaagctgacgggatcgaggttcagcaccccgccttccagttcggcgcccaggttcacggcgcgcacgtcgaagtcgttggccttgaccgaggcggcgcggtagctgagcgagccgtccatggtgcgcaggcgctcgacctgcaaggtggcgtcgggcagcagcttgcccggcgagccgctggtggtctcggtgttctcgcccgaggtgcgcggctgcgcgccgacaacggccagcaggtcgtcgaggtcgaggcggcgggacgtcagttgcgcctcgacgcgcagccgctcggccgcatccaccttgacgtctccggacaggtcggaggcgccgacgcgcccgtcgaaatcgttgaacgtccagacacggtcatcgcgcgtcagggcgcccgacaggcgataggcgggtgtgttgggcagggtcacgccggtcagcaggtaaagatcggccaggttctggcctttcaggctcagcgtcgcctggaactggcccagatcgaacgggcgggtgatggcgccgtccgccctcagccgcgaccccgccccgtccactgcggcggtgaactgatacggccgattgcggcgcatgttgataaagggcccgccctgaatccgcagcgtcaggggcgagccgttgatgctgccgcggccggccagaaggaagccggcgtcgccgtcgttcgcgggctcgcgcgcattgacctgggcgtccagcgtgaggtcgcgcctctgctcgtcgacggggagacgaccgtcggcgatgaccagttgctggatgaccggcagcttcatgccctcgccatgatcgggcttgtcaggctccagctcccagctcttcctgccgtcggcggttgcgatcagcaccacgttcggtcgggtgaaggacagcagcggcatctcgatctggccgccgaacagcttgcgcagccgcacggaggcctcgattcgaccgacgttggcggtgtcgcgttcacgcgcccagtcgggtccgccgaatttcaggtcgttgacgaccaccgaaggcgtccagctgaacaggttcacgtccaggtcgccgcgcaaagcgacctcgcggtcatacttctgcgacgcccatcgtccgatcggaccccgcagccagttccagtcgaacagcaacaggaagatcaccaccgctgcgaccagcagcagggtgacgcccgccgccatcttctccgcgcggcccggacggcgtgcggcggcgtagacgggatcgttggcgcggacccaatcgcggccgcgacgcaggcggtcggccactccagacgcgccgttgcgaaggccgtccttaaaatccttagcgttcaaggtcgtggccaagctgcgcccctccgttcgctcactaacgcacaaggtcgcggttggagccgaagaggctatttgtcacctcgatgacacctctctgtcttgaaacctttacattcctggagatcggcgcatggtgaggctcaagacccgcgatgcggcgggccacgggagatccagccatgaagcgtgcagcccttttcgtcctttcgatcgccacactcgccgcggtccagacccccgccagcgcccaggcgccgacacggaccgcctcgcccgagagcgcctccagacaggccgtgatgatctgcgcgtccgacagcgccacacgacgggccttccagcgcgagcatggctccacaccggtgttcgtcaccgcacgcgaggtgatggaggctcagcgagccggcgaggcctggagcacgccgcgctgtatgaacgagcaggagtatcgacggctggtccttatcgccaacacgcgcgcctcgctctgaggtcatcctgacgcaagaaagaaggggcgcggggatcacccgcgtcccttcttcgtgtctcccgacggttgaggtcagcgcgtctcttcgaggtgcttgttcagccagccgaacacctcgtcatgccagcgccggctgttggccggcttcagcacccagtggttctcgtctggaaacaccaccagacggctgtcgatcccgcgccgctgaagcgcggtgaaggtggacagcccctgcgccgtcgggatgcggaaatcgaggtcgccctgcaccaccagcatcggcgtcctccagttctcgacatggttggccgggttgaagcgctgatagccctcgggcttgtcccagggcgtgccgccgtactcccactcggtgaaccacagctcctcggtcgaatagcccatggcgaaggtgtcgaagacgccgtcgtggttgaccaggcacttgaaggcgtcgttccagcggccggcgatccagttgatcatgtagccgccgtaggaggcgcccagcgcacaggcgttgtcgccgtccaggaacgaatactggcgctgagcataggcccagcccttctgcaggtcctccagcggccggtcgccccaatgctggctgatcgcatcagtgaagccctggccgtaaccggtcgagccgtggaaatcgatcatcaccaccgcatagcccgcgcccgcataggtctcggggttccagcggtaggaccagctgtcgccgaaagacccttgaggcccgccgtgaatcaggaaggcgaccggatatttgcggccctcgacgtatccgaccggcttgatgacatagccgtgcacggtttcattgttccagccggggaaggagaactgctcgaactcgccaaaggccttggtgtccagctgcgggttcacattggtgatccgacgcggcagttcgcggcccatgaaggtcttcacgaacagctcggtcggacgggtcaggctgtcctgggccaggacaaagcccgagggcgtcagcccgaacgcagagacatggccgtcgccggtgatcggcgtcaccacgccgttgcgcgcatccacggcgaacagcttggtccgtccggtgtcgccggcgatggcgtacagggtgttgccgtcctttgaccactgcagggtgtcagccgagcggtcccagtcggcggcgatctcgcgcgtctgccccgtcgccacgtccatcagcttgatttggtagcggtcggcctcgaagcccggccgcgccatggcgcggtaagcgagcgtgcggccgtccggcgagaacacggggcccgcgtcccaggcgtcgttggcgtccgtcagattagtgaaggtgccgtcacccgacaggccgttggtgcgccacaggtcgaagttggtgctccagggttcggtccggcccgccagccgcgccgagaacaccagggcgtcgcccgcaggcgtgaaaacgaagtcgctctcgtcgccgaacggcttggagggtgtgtccccgtcaaagcccttggtcgcccacacgggcgcatccacagcgcggccgttcgcgccgatcgactgcacgaagaggtgattttgggtgtggtcgttccaggtgtcccagtggcgcacgaacatgcggtcgtagaccttggccgtggtcttctgctcggcgcgcgactgcgccatggcgaccgaggcgccgaggtcggccgcgtcgggatagacggccagcgacaccgccagcttgtcggcctgcggactaagccgataggcgttgacgtccagcggcaggtcggtgacctggaccggccgggtcccgtcggcctcggcccgccacacctgactggatcccgacttgccggacaggaagtagatgcggccgtccgagccccagcgcgcggtgttggcgccctggtccgagatcggcaggcggcgcgcctcggcgtcggacgacaactccttcaggaacagcgcgcccgagcggcggttggcggtcacgtcggtggtggtcagcgaatagatcacccagcggccgtccggcgacacctgcggatcgcccagccggttggccgagatcatgtccccataggtgaaggcgtcgggcgtcgccgccggggcgggaacgggtgcaggcggaacctgggccagggccggcgcagccgccgcaagggcgacggcggcgcaggcggccgaaaaaagggtgcgatgacgcatgtggaggctcctcaaccgacgctgtggcggcaaggcgtagcaccggcgttccggcggcggaagttgatccttgcccgcgcccgcgcgaccggcgacaagcggtttgtccatgccgcccgcctccgcacccgttcggtccccgccgcacatcgtcgatgtgctgatcgccgagcgcgcgccgcggcaacgcgctcgcccgcctggccgctggtcaggcccggcctctatgcgcttctcggctacggcaaggcgcgccgcatggccgacgccatcgcgcctatgtcgggcgcggagacgctgcgtcacgtttccgacttgcttcacctgaaggtggaggccgcccatctggagcggttgcccgccgcgggccgctgcatcgtggtgtgcaaccatccgaccggcgtcgcggacgggatcgccctgtacgacgcgatccgtcggcggcgctccgacgcggtcttcttcgccaacgccgacgccttgcgggtttcgccgcgcctgtccgagacggtgatccctgtcgagtgggtgcacgacaagcgcacgcgcgacaagacgcgcgccaccctgcaggcggcgcgcgaggcgttcgaggccgaacgctgcatcgtcatgtttcccgccggccgactggcgcgcgtcgagagtgacggcctgttgaccgacccggaatgggcgcccaccgccgcctccctgtcgcgcaagttcgacgcgccggtgatccccatgcatgtgaccggcccctacagccggctgttccacctgttcgacaaggtttcgcgggagttgcgcgacgtgaccctgttccacgaactgctcaacaaggccggaaagcggttcacggtcacggtcggacgatcggtttcgcccgaaagcctgccggcggacgcgggcgaggcgacggcggcgttgaagcgcttcaccgagcgcaccctgtccgcagacgccgacgcggtgttcgcatgagccggatcgtgctgcccgacacagaggcgaccacgcggctgggtcaggtcatcgctcccctgctggaggcgggcgacagcgtgctgctgtatggtccgctcggcatgggcaagtcgacgctggcgcgcggcctgatccgcgccttgaccacgccggatgaagacgtgccgtcccccaccttcaccctggtgcagttctacgaaagcgatccgcccgtcgcccacttcgacctttatcgcctgaaccagcccgaggaggcgtgggagatcggcctggacgaggcgctggacgacggctgcgcgatcatcgaatggcccgagcggctgggcgaggacccatcgggtttcctgcgcgccgaccggctggtcatcgtcatcgcggaagagggccagggccgtgttgcgaccgtttccggcgcgggccggtgggaaaggctgatcgatcatgtccatccctgaccgagaggaacaacgtcgcgcgtttctggccgcgcacggcctgggcgacgccgtgcgcgcgcccctgcccggagacgcctcgacccggcgctacgagcggctgacccggccctccggcgcgaccctgatgctgatggaccagcctccagccgccgagagccagccctgtgatcccctctggtcgcccgacgagcgccgcgcccagggctggaacgcgcttgcgcgcctgtcggcgggcaggatcgaggccttcgccgctgtcgccgctcacctgcggtcgctgggcctttcggcgcccgagatcgtggcggtggatgcgccggcgggtctggcggtgatcgaggatttcggcgacgacctgttcgcccgcgtgatcgaagggggtgcggacgaggcgcctctgtatctcgcggccgtcgaggccctggcccggctgcacgatgcgccgacgcccgagacgctgagcggtctcgccggcgactggccgctgctcagctatgacgagacggcgctgcaagggggggccgacctgttcatcgaatggctgcccaaactggaactccgcctgagcttcgacgacgcggcggttgcggagtggcgcgcggcctggggaccgaccgtccgcatcggtgcgcagggcgccgtggtgatggcgcaccgcgactaccacgccgagaatctgatccggcttgaaggtcgggacggcgccgtgcgcgtcggcatgatcgattttcaggacgcggtgcgggcgcacgcgtcttgggacctgcattccctgctgcaggacgcgcgccgcgacgtctcgccggagctggaggcgctggcgctcgaccgctacttcgccctgcgaccgcaggtggagcgcgagccgttcatgcgggcctatgccgggctcgctgcgctgaacgaggcccgcatcctgggtatcttcgcccgtctgatcgcgcgcgacggcaagtcgcgctatcgtcagttcatgccgcgcatgtgggcgcatctgaacgccaacctcgccaagccggggctggaaccggtcgccgcctggttcgaccgccacgtccctgcggagctgcgccgatgagcgcgccccggaccgcccccaagacggcgatggtgctggcggcggggctcggcacccgcatgcgtccgctaaccgacgatcggccaaaggcgctggtcgaggtcggcggccgcgccctgatcgaccacgtgctggaccggctggcggacgcgggcgtcgagcgcgccgtggtcaacgtccactggttcgccgatcgcctggagacgcatctgcagggccgcgcccgccccgccatcgccatctcggacgagcggctgcagctgctggagaccggcggcgggttgaagaaggcgcggccgttgctgggcgatgatccggtgttcgtggccaacatcgacagcgtctggatcgaccgaggcgacgccttgggggacctcgtccggctgtgggatcccgaacggatggacgtggtgctgctgctggcgcggcgcgagggttcgatcggcttcgaaggcgatggcgacgtcttctgcgacacggacggacggctgaccttccgaggcgacgcgcccagcgccccttacgcctatatgggcgtccacatcacgcgtcccgactatgccgacgaagggcccgccggcccgttctcgctgagctcgctgtggcgcaagtcggcggaggcgggacgcctgttcggctgcgtgctggacggcgagtggatgcacgtcggcgacccccaggcccgggacgaagccgaagcccgcctggccgagagcgaatgagcggcttcgaccccttcgcggacacagaaccccgctggtacgccgtcccggcgcaccgaccgttcctggaagatttggcggcgggcgtgctgtcgtggctgggcgacctgccgcccgagaccctgtcggacgccaccatcctgctgcccaaccgtcgggcggcgcgcgccttcaccgccgccttggcgcgccaggcgaacgggcgtgcgatgctgctgccccaggtccggccgctgggcgatctggaagaggatgagccgccgttcacgcccggcgcgctcggcctggacctgccgcccgccatcgcccccatgcaccgccgcttcgagatcgcgcgcatgatcgcagaggatttcgaccgcgacctgacgccgctgcgcgcgttggagatggccgatgcgctgggcggcttcatcgactcctgccacctcgaggaggttccggatcccggccgcgtcgcgcgtctggtggacggcgagatggccgcgcactgggagcgctcggccgagttcctgggcatggcggtcgaggcctggccccggcggctggaggcgatgggcctggtcgatccgtcctggcggcgcgcgaccctgctgcgccggctggccgaggcctgggaccggacgccgccgacccagccggtgatcgccgccggatcaaccggcaccgtgccggccgccgccgacgtgctgggcgccgtcgcccgcgcgccgcagggctgcgtcgtcctccccggtctggactgcgacctggatgaccgggtctgggacctgatcgacgagaccaacgagggccatccccaacgcgccctgaagcggcttctggaacgacacgatctgacccgcggcgacgtgaggccctggtttgagccgcccgcggagcccgcgctccgcagccggggtctggcgcgccaacggctgctgaacgaagccctgcgccccgccgacgccaccgacgactggaggcgcgagatcggccgcatccgcagccgcgccgccgaagcgggccagtccgccgatcccatcgccttggggttggagggtctgtcggtgctgacccttcggacggaggaagaggccgccgccgccatcgccctgttgatgcgcgagacgctggagacgccaaacgcggacgggtcgccccgcacctgcgcgctggtcacgcccgaccaggcattggggcgccgggtcgaggcgcggctggagcgttggggcgtgatcccggactcttcggccggacgcccgctgtcgcgcatgccggcgggggcgctgatcgatctgtgcgcccgcttcatcaccgatccgctggacccgcacgtgctgctgggcctgatcaagcatccgctggtccgcctcgatgcaggcggggcggaccagcggcgcgcggtcgaggcgctggagcgatacggactgcgcggcccccgctcgcgcgacttcgcccgcttgaaacggcgcctgctggaggccgcccagcccgaccgccgcggcaaggcgccgccctaccgggcgcagccccatctgatcgcggcgcaagcgctggtcgatcggctggagacgctggcgggcgaggcccaggcgccgttcgccgaagacgccgccgcgctggatcaagccgcgcgcgcgctgacgcggctggccgagaccctggcgggtcagaacctgtgggcgggaccggacggagaatgtgcggcgacgacgctggccgggctgatcgagggcggcgcgccgctgggggcggtgtcgcgcgcggacttcgccgctttgcttcacagcctcttgcaggatgcggtggtccgcacgggcggcgcgacccatccgtccctgcgcatcctgggcgccatcgaggcgcggcttgtgcgcgccgaccggatgatcctggccggcctcgaggaaggcgtctggccgcaaggccccgcgacagaccccttcctgtcgcgcccgatgcgcaagagcctgggactgccgccgcccgagcggcgtctcggccagacggcgcaggacttcgtccaggccgcctgcgcgcccgaggcgatcctggtccactccgaccggcgcgggggtcagccggccgtacggtcccgctggctgtggcggctggagatgctgacgcgcggggcggacagcgaggcgacgccggtcgtgctggagcggccctccgccgccgtcgattggacccgcacgctggacgcgccgccgcccggcccgccggccctcgccccgcgcccgcagccccgcccgcccgttcaccgccgcccgcgcagcctttacgtcacgcgggtcgaacgctgggttcgcgacccttattccgtatacgcacaatccatcttgaggctggaggcgatggagcggccgggcgcctctgccgaggctctggcgcgcggcgatgcggtgcacaaggcgatcgagctgctgacgctggagtggccgaacgatctccccgacgactgcgaggcggtgctgcgcgaccatctgctgcaccaactgggcgcgcacgggttcgaggacgccgccatggcgcgcgaggcgccgctggcccgcaactgcgcacgctggctgaccgcgttcgagcgccgccgccgcgagcgcggcgtgaccctgctgatcgaacagaggggcgcaatgaccttcgacgccccggccggtcccttcaccctgaaagctttcgccgaccgcatcgagctgtccggcactggcgcggcggtcatggatttcaagacgggcgcggcgccgtcgatgaagcaggtcaagaccggcttctcgccgcagctgaccctgaccggcgccatcctggcccacggcggctttgcggacaccaacggtccagtcgaaccggacgagctgacctatgtccgcgtggtcgggcgcaaggtggcgggcgaggtcgccgtgcggggtcaggggcttgaggcggcggagctgtcgcgtggcgccttggagggcctgaagcggcgcatcgcgcgcttcgacgacgagaccaccccttacgtctcctgggcggcgccgcagttcatgggcaaccagggcggcaactacgaccatctggcgcgcgtgtgggagtgggccgtggccggcggcgacgaggaggcctcggaatgagcggagccgcccaccagatcctcgccgccgacccgaacctgtcggtcttcgtcaccgccaacgccggctcgggcaagaccaccaccctggtcaaccgcgtggcccgcctgctgctggccgaggcccggcccgacgccatcctgtgcgtcacctacaccaaggccgccgccgccgagatgcaggcgcggctgttcgatcagctgggcggctgggccgtgatggacgatcgcgagctcgccaaggccgtggccgcgctggacgacggcgatcccgccgcgctcagcgaagcgcgattgtcggaggcgcgccgcctgttcgctcgcgcgctggagacgccgggcggcctgaagatccagaccattcatgccttctgcgaaaagctcttgaggcgctttccgcttgaggccggcgtgtcgcccgccttcacggtgctggaggaccaggcggcggcgctgctgtcgcaccaggcgcgcgaggatctggcccgctacgccctggcggatgcggaggggccgatcggcgcggcctacagccactttgctgtcgagctggactggccgcggttccaggccctgctggcgatgatcgaggcccggcgcgatgcgctgaccgcctataccgacgcctgggaagcaggaaccgcaccctcgccacacgcgctgaccggcgccgatccgcaccagaggccggaggagatcgagcgcgacttcatccgcttcatcgatcccggcgagtggagccgcatggccgaggcgatggcggggggcgccaagaccgacgccaagctggccgacgccatgcgggccgccgcaccgcctgacgtcgccttcgccgccctggccgtcgtcttctgcaaggcggacggcgagggccgcaccggcatgggcaccaagtccgctccgaccgatgcggtgggctggctgacggacctgcaggccaaatacctggcgacgcgcgacgtcctgcgggcggccaaggtcgccgacgacacggtcaaggtgctgacgctcgcccgcgcccacgccgccctctacgaacaggccaaggcggcgggcggcgcgctggacttctccgacctcgtggcgcgcaccgttcggcttctgacccggaacgcctccgccgcctgggtgctgtacaagctggacggcggcgtggaccacgtcctgatcgacgaggcccaggacaccgcgcctcagcagtgggagatcgtccgcgctctgaccggcgagttcttcgcgggcgaggtgtccggccgcaccgtcttcgccgtgggcgacgagaagcagtccatctactcgttccagggcgcccggcccgagcgcctgcgccaggaaagccgcgtctatcagcagctggtcgaaggcgccggcgcggtgttccagcaggcgccgctggagacctcgtaccgctccaccgaagaggtgctgcagttcgtggacgccgtgttcgaaagccccgagcgcacccgcgccctggtcggcaaggaaggcgacattcctcgccaccagccggcgcgcgtcggtcagcacggttcggtcgaactgtggcccctgttcgtggacgagccggcgccagagcgcgacgcctgggacgcagcggtggacgaggaggccgcctccagcgcgcgcaagcggatggcgatgacgctggccggcgagatccgccgccaggtcgaaaccggcgtcgccgtgttcgaccgcaaggaacgcaccttgcgccccgccggctacggcgacttcctgatcctggtgcgccggcgcgacgcgacctttgaggaggtgatccgggcgctgaagaccgcgggcgtgcccgtcgccggcgccgaccggctgaagctgtccagccacatcgtgttcgacgatctggtcgcgctggcccgcttcgccctgttttccgacgacgagctttcgctggcctgcatcctgcgcagccccttctgcgacgtggacgagaacggcctgtatgcgctggcgggcggcgagacgcgcaagggcctgtggcgcgagctgcgggcgcgggccgacgagcggccggagtggacgcgcgcgcacgacctccttcggttcgccattgaccagcggggacgcgacccgttcggcttcttctccgccctcttgaaccgggtggacgacaccggccgctcgggtcgcgcgcgcatcctggcgcgcctcggccgcgaagcggaggaggccgtcgacgagaccctgaaccaggtgctggcggccgaaaaccgcggcgggctggatctggagacctgcgtcgccctgctggaggccgccgacgtcgaggtgaagcgcgagctcgagggcgcgcgcggcgaagtgcgggtgatgacggttcacggcgccaaggggctggaggcgccggtggtgatccttccggacaccaccatgaaggcaaaggcgcagggccccagcctcatgcccgtcgcgctggacgaagacggcgcagaggcctggctcatgtgccccggttccaggaaggacgactgcgcggcttccgccgccgcgcgcgacgcccgtcaggcgcgcaccgacgacgagacgctgcggctgctctatgtcgccctgacccgcgcccgtgaccgcgtcatcgtcatgggccgcgcctccagccgtgggcccgaggccggcagctggtggtcggtgatcgaagagacctttgagcgtctgggcgagcgggtgcggaggacggacactggcctacgccgcttcggcgtcgatcccgaacagcggccgcaaggcgcggcgattgtgatcgcggagacgacggcgcccgactgggcccgccgcgccgcgccggtcgaggcctctgcacgcttcgcctcgccgtcgcgcatggaaggctcaatccgcatccccgcgccctcgccgctggcgcagtccggcgcaaacctgggccgcttccgacgcggcgacctgatccaccggctgcttgaccgcctgccggaaatcgcaccaccggaccgcgccgacgccgcccgccgcctgctggccagggagacggatctggacgaggcccagcgtctggagatgatcgaggccgccttcggcgtgctggacgacgcccgctttgcgccggtgttcggccccggctcgcgcggcgaggtcgcactgacgggcgcggcggccgacctgccgccgggcgtggtcgtctccggccggatcgaccggctggtggtcacgcccgagagcgtcttggtcgtcgattacaagaccaaccgtcccgcccctgagcgcgtagaggacgccgatccggcctatgtgctgcagctcgccgtctatgcggcggtgctgaaagacctctatcctgaccggccggtggaggcggcgctggtgtggaccgacgggccgaaactgatgccggttccggaggccctgatggggcaggcgctgcaccgcgcgcgttgatttccgcccgggcctcgcccacatctgcgccagcgcctctggcgacaatggagagattgaacatggccaccgtcaaggtcactgacgacagcttcgagaccgaggtgctgaaggcctccacccccgtgctggtggatttctgggccgagtggtgcggcccgtgcaagcagatcggcccggcgctggagcagatcgccgacgaactgggcggccaggtcaccgtggccaaggtcaacatcgacgacagccccatgacgccctccaagctgggcgtgaagggcattccgaccctgatgctgttcaaggacggccagatgacctccatgaaagtcggcgccatgcccaagggcaagatcgtcgaatggctggccgaagccggggtcaaggccgaagggtaaggcggcggcgcccgctctcgtggcaagacaagaggggcggctcggagacgggtcgccccttttctttcccgacgtctcagatcggccaagtctccgggctggcgcccagcacctcgcctccgaggtacagcgagccgcagatgaccacacggccagctcccaagcgcagggccatgtccagcgcctcggccgccgatccagccggcgtggcggccagcccatggccgcgcgcgacggcggcaagggcctggggttcggccgccgcgccgtcgaagccgacggtgaagaccgcggcgccgctccccttcagcgcgtcgaagaagccgccggcgtccttgttccccagcatgccgcagatcagcgccagcggacgcggcgcgcgcgcctggcgttcggccaggaatgcggccagagcacgcgccgcatgcggattgtgcccaccgtccagccatagctcggcgtccgccccgcgcgccgcctccgcataggggccggcggtcagccgctgcagccgggcgggccagcgcaccgcctgcagcccctgggcgatcgcggcctccggcaggtccagctccagcgccgcggcgatggcgacgccggcgttgtcgatctggtgcgcgcccaccagcgccgaggcgggcaggtcgaggaaacgctcgccatcctggaacgccacgccgccgcgctcggcccacgcgtcgaagtccacccccatcacggcgaggcgggcgtggacccgtgcggcggcgtcttcgaccgcgcgcatggcggcctcgctctggcgcgcgatcaccgccggcgcgccgggcttcagcaccccggccttttcgcgcgcgatcccggccaggtccgtccccaggaactcggcgtggtcgagatcgacgggcgtgatgacgctgagcagcggccggtcgatgacgttggtcgcatccagcgacccccccagcccgacctcgatgatcgcgaggtcggccggcgtctcggccatggcgacaaaggcggcggctgtggtgctttcgaacacggtggcctcgccgcccgccgcctcgacgcggtccaggatggcgttcagcgtcgcatcgtcgatcagccgtccggccaggcggatgcgctcgttgaaccgcacaaggtgcggcgaagtgtaggcgtgcacgcgaaggcccgccgcctcggcgatggcgcggatcagagcgacggtggaccccttgccgttggtgccggccacatggatcacgggcggcagacggttctgcgggtcgcccagcgcggcgcacagccggcgcatccgctccagcgacaggtcgatcttttgggggtggcgcgcgcgcaggcgctcggagatggcgtccatggcgcccaactagaccaccgatagcggcctcgccatggcgggcgtgctaggaaggaggcgatgacccgtcccgcaccccgcgccgtcgcccgcctcgtgctggcgctcgcctacttcgccgcgggcgtgctgcacctagttctgcctgagcccttcctgaccatcacgcccggctgggttccggcgcccgaacaggtgatccgcctgaccggcgtggtcgagatcgcgggcgcgatcgggctgatgatcccgcgcctgcggcgggcggcggggatcggcctggcgctttacgccgtctgcgtgttcccggccaacatcaagcacgccatggacaatctgagcacggggaacggcctcggcctcgcctaccacctgccgcgcctgatgctgcagccggtgatcgtctggtgggccttatgggccggccttgtggtcgactggccgttccgaaggaggcgctaggccgcctgtcgcgttccgcccatcagcatggacaggatttggccgagcacgtgcggcagctccccgcgcgtgacaacccgatcaaccatgcccttctcctgcaggtattcggcgcgctggaagcccggcggcagcttctcgcgaatggtggcctcgatcacacgcgggccggcgaaaccgatcagggcgccgggctcggccaggtgcacgtcgcccagcatggcgtaggaagcggtgacccccccggtggtggggtcggtcagcaccaccgcatacggcagcttggcctgcttcagctcgtcgatcgccagggtggtgcgggccatctgcatcagggacagggccccctcctgcatgcgcgcgccgccggcggcggtgaagcagatcaatggaaccctgcgcgccacggcctcgcgcgccgccttgatgaaggcctcgcccgccgccatgcccagcgaaccgcccatgaaggtgaagtcctgaacgatcaccaccgccggctggccgcccacagagccgaagccgatggccatcgtgtccttgcggccagaggccttgcgcgcggcgttcagccggtcgcgataggagcggccgtccgagaacttcagcgggtcttccggcacgtccggcgtgtcgatcgactcatactcgccgccgtcgaaggtgaagcgcagccgcgtcggcgcgtcgatccgcatgtggcggccggacggcgtgacccacagcgaaccctccagctcggaccggtacagcatgtcgccggtgtccggatccttgacccaaaggttgtcgggcgtctcgcggcgcgagacgatcttgcgcacgcccggggcgaagcggctgagccagccgccgggcttgtcggattgcggcttgttcttgtcgaccatggacgggctcttagacggtttcgaccgatcgtgcagccctgacggcgtcgcccagcgcgcggaccttcgccagaacgcgcggggcgggggcggcgttctcggccagcgccgccgccacctcttcgaccagggccgagccgaccaccaccgcatcggccacgcgcgcgatctcggccgcacgctccggcgtcttgacgccaaagccgaccgcgaccggcagcttggccgcgcgccgcacgcgctccaccgccggggcgacggaagcggcgtccgcctccttgacgccggtcaccccggccaccgccacatagtagacgaagccggaggtgcgctcggcgatgatcttgaggcgcgcgtcgtccgaggtcggcgtcgccagccggatcagcgagatcgacactgcgtccagcgcgtcggtcagcggcccggcctcctccggcggacaatcgaccacgatcagaccgtcgatcccggcgtcggccgcagcctgagcgaacgcctcgtagcccatgctctcgatcggattcagatagcccatcaggatcagaggcgtgtcggcgttgccgacgcggaagtcacgcgccagctccagcgtgccgcgcatcgacagcccggccttgagccctcgcagcgccgccttctggatcggcgggccctcggccatcgggtcgctgaacggaaagccgagttcgatgatgtcggccccggcctctggcaggccgcgcagaatctccagcgcttcgccgcgcgagggatcgccccccatgacataggccacgaaggcggctcgaccctcggccttcagccgggcgaagcgggcgtcgatgcgggcggtggtcattgggcgggagcggcggctggcgtctggccggcgcagacgtcgccggggatggtggcgaagccgaggtaggcgggggcttcggcgatggcgggcttggccgtgtcgtagaaggcgaccatctgcagtccgtcgcagccgcccgcctcacggcgcttgacgaagacgacgcggttgtcgtcgccgccggccggcagccagccgcgcgttccgaagtcggcgatgtaggcgtcggccagggcgccgatcgagctcagcggcgcggtgatgcagaaggcgcgaccggccaggttgttgagcccgccgcagtccggcgacgcctgcgcgcccgtcaggatcggcgtgtccgtcgccggcgcgccggccgccgccgcgacaggggccgccgttgtcggggccgcgccctcttgcgcgagcgcgggtgcgcagacgcttcccgccagaaaggccgtgacgatcagggtcttcatcattctagagctccacgcccaggtgacgcgccacctggaagatgtccttgtcgccgcgtcccgacatcagcagcaccacgtcgccgcccttgccgacctcgcgcgccacctcggcggtccgggccagcgcatgggcgggctccagcgccggaatgatcccttccagacgcgagcagagctgaaacgcctccagcgcctcggcgtcggtggccgagcggtattcggcgcggccgatgtcgtgcagccaggcgtgctcgggcccgatgcccggataatccagaccggccgagatcgagtgaccctcgacgatctggccatgctcgtcctgcagcagataggtgcggttgccgtgcagcacgcccggccgtccgcccttgaggctggctgcgtgggcgggcgtgtccaggccgtggccggccgcctcgacgccgatcagacgcacgccctcatcgtccacaaaggggtggaaggcgccgatggcgttggagccgccgccgatgcaggcgaccaccgcctccggcagcttgcccatctgggccttcgactggaccttgatctccttaccgatcacggactggaagtcgcgcaccatggccggataggggtgcgggcccgccgccgtgccgatgatgtagtaggtgtcggcgacattggtgacccagtcgcgcatcgcctcgttcatggcgtccttcagcgtcgccgcgccggcggtgaccgggaacacctcggcgcccagaaggcgcatgcggaagacgttgggctgctgccgctccacgtccaccgcgcccatgtagacggtgcagggcaggtcgaagcgcgcgctgacggtggcggaggccacgccgtgctggcccgcgcctgtttcggcgatgatgcgggtcttgcccatgcggcgggccagcaggatctggcccatgcagttgttgatcttgtgcgcgcccgtatggttcaggtcctcgcgcttcagccagacgttggcgccgccgaaatgctcggtcagccgctcggcgaaatagagcgggctttcgcgccccacatagtgggtcagatagccgtccagctcggcctgaaagccggggtccgccttggcttcggcataggcctgatccagctcgtggatcagcggcatcagggtttcggcgacgaactggccgccatagggaccaaagcgacccttcgcgtccggccaagcgtaggtgttggggagtatggcgttcacaggcagcatcctggcgcgagcaggcgtccgaattacgaccggcgcacagcctgcagaaaggccgcgatccgggccgcgtccttaacacccggcgcgctctccacgccagaggagacgtccgccatgggcgcgcctgtcaaggcgagcgcttcggccacattgtcgggtgtcaggccgccggccaggaaccagggcttgtcaaagatgcggccggccagaagcgaccagtcgaagctgtgtcccactccgcccggcagcaccgaaccctccggcggcttggcgtcgaacatcaggtgatcgacgtgcggcgcccacgcttcagcggcatcgaggtccgccgccgtacggaccggcagggccttgatcacgcccgcccctgtcagcgcgcgcacggcggccatgcgttccggcgtctcgcgaccatgcagctgcaccaggtccggcctcagcatgcggccgatgctctccagcaaggcgtcgtccggatcgaccaccaccgccacgatccgggcccgtccgcgcgccgcctcgaacagctcgcccgccacatccggcgcgatgtgccgggggcttgggggaaagaccaccgcgcccacgaagtcggccccgccgtccagagcggcagccagggtgtccgccgtggtcaggccgcagatcttgatcgccggggtcatggcggatgcaggtgtgcccggcgggccgtccggtcaagccggctcgacgaagatcgaggcgatctcgtccggcgtcagcagccgccaggcgccgggggcgagatcggccggaagcgtcagcccgcccagccgttcccggtgcagcgcttccacatggttgccgacggcggcgaacatgcggcgcacttggtggtagcggccctcggtcaccgtcagcagcgcctcggtgggggagaccacctccagccgggccggcgccaagggtttgctttcgccttccagcatcagctcgcccgaggcgaacagcgtgtcctcgcccccctccagcgggcgggccagagtcgcgcgatagactttggcgacgtgacgcttggggctgatgacgcggtgcagcaaatcgccgtcgtcggtcagcagcagcaggcccgtggtctgcttgtcgagccgtccgatggtggagaccgccgggtcgcgccggcgccagcggtcgggcaggacgtcatagaccagcgccccatcctccttgtgcgaacaggtcatgcccagcggcttgttcagcaggatgaccaggcccggcgcgggatcgagcggctcgccatcgatctccatgcgcgtggacaagtcgggcgtgatcggaatgcgccgcgacacgtcggccacgtcctcaccgtccagcaccacgccgcctgcgcgcgccagccgggcgatctcggccctcgagccgtagcccatggagcccagcagcttgtcgatccgggcggtcggggtcttcttcatgcgctaccgcccttcgggctaagtgagcgcgggttcacttcaccgcctcgaacaccttgtagccgccttggtccgcaaccggacgcacgcgcgcgaaggcggcgttcaactcggcctcgtagggcaggtgccgattggcgaccagccacagcaccccgcccttcctcagcatctcggccgccttgcggataaaggcccaccccagccgccggtcctcggcgccgccgtcgtggaagggcggattgctgaccacgaagtcgtagtcgccgttggtcgccagcgtgcgcacgtcggtccactgaaccttggcgcgggcgtcctcgatgttgcggcgcgccgcctggatcgcgcgccggtcgatgtcgaccagcttgagcgaaacgaccttcggcgagcgcaggatcacagtagccagagcgccgtagccgcagcccaggtccgcgcccttgcccttcagcgcgggcaagtgttgcgccagcagggccgagcccgcgtcgacgcggtcccaggcgaaaatccccggctgcgaccaggcctccagtccgggcacaagctgctgcgcgcccgcagcgatcgcctcgtccaccccgatcacgacgtccgggcgcagggcgatgcaacgcctgtggtgcgccttggcggtctcggcgacctcgagcccgaaagccttcagctccttggccaggcgcgagccgcccttggccttgggcgccatgacgtccagccgcccgccgaccttgagcgcccgcagcgccatggccagggtgtagcgccgctccagcacgcccggcggcgcatagaccgtcacgtcgtcgaccgagcccggctccatggcctccagcgccgccgattccgggatcagcggcgaggtctggatcgcatcggcgggcgggtcgaacaccgccggcgggcggccatatagaagcgtggtcatgcgcggctccttagctcgcgcgccccgaatcgccaaaaaggccgcctctggcctttcgacgcgtcccgctgtatgaggcgcccgcctcccgaaccgtcgcttctttattcacgcggcccgcccggacctcctggtccgctcgccggccgcctcgcacgtctgatcctgaaatgaacctgcgcaacgtcgccatcatcgcccacgtcgaccacggcaagaccacgctcgtcgaccagcttctcgcccagtccggcgtgttccgcgccaatgaggcgacgaccgaacgcgccatggactccaacgaccaggagcgcgagcgcggcatcaccatcctggccaaggccacctcggtggtctggaacggcaaggcgggcgagacccgcatcaacatcatcgacacccccggccacgccgacttcggcggcgaggtcgagcgcatcctgggcatggtggacggctgcgtcatcctggtggacgccgaagagggcgtgatgccccagaccaagttcgtgctgaccaaggcgctgaagatgggcctgcgccccatcctgtgcatcaacaaggtcgaccgcgcccacgccgatccggaccgcgtgcaccttgagaccattgaactgttcgaggcaatcggcgcgacgcccgagcagctcgacttcccgcacatctacgcctcgggccgtaacggctgggccacgctggacatgagccagccgtcggacaccctggccccgctgttcgacctgatcgtcgaccacgtgccgccgccgccggtcgccgagaacaaggacaagccgttccgcatcctgaacgtgctgatcgagtccgatcccttcctcggtcgcatcctcaccggccggatcgaaagcggcagggccgtgccgggcatgccgatcaaggcgctggaccgcgacggcaagcagatcgagcagggccgcatcaccaaggtgctggccttccgcggcctgaagcgccagccgctggacgagggctcggaagcgggcgacatcgtcgccatcgccggcatgtccaaggccaccgtcgccgacaccctgtgcgcgctggaggtcaccgagccgctggacgcccagccgatcgacccgccgaccatctccatgaccgtgggcgtcaacgacagcccgctggccggccgcgaaggcgacaaggtgcagtcgcgcgtgatccgcgaccgcctgctgaaggaggccgaggccaacgtcgccatccgtgtcacccagacaccgggcgccgacgcctatgaggtcgccggccgcggcgaactgcagctgggcgtgttggtcgagaacatgcgccgcgaaggcttcgagctgtcgatcagccggccgcgcgtggtctatcagaccggcgagaacggcgagcggctggagccgatcgaggacgtcatgatcgacgtcgacgacgaatacaccggcgtggtgatcgaaaagctgtcgacccgccgtgccgaactgaaggacatgggtccctccggcgccggcaagacccgcatccagctgatgtgcccgtcccgggcgctgatcggctaccagggcgagttcctgaccgacacgcgcggttcgggcgtgctgaaccgcgtgttcagccactatgagccgcacaagggtccgatcgaaggccgcctcaagggcgttctggtctcgaactccgacggcgacaccgccgccttcgccctgtggaacctggaggatcgcggcgtcatgttcgtgggcgccggcgaaaagacctaccagggcatgatcatcggcgaaaacagccgctcggacgacctggacgtcaacccgatcaagggcaagcagctgaccaacgtccgcgccgccggcaaggacgaggccgtgcgcctgaccccgccgcgccgcccgtcgctggagcaggccatcgcctatatcgaggaggacgagctggtcgaggtcacgcccaagtcgatccgcctgcgcaaggaggtcctgaacccatccttccgcaagaagcgcgtccgcgccgactgatttgctcttggaatggggcgagacgcgcgctaagtctcgccctgtctcccactcaaacgcagcctgtcgggccggtcgcccggtgatctcgcgccttgagcacgcatgacggtcggccgccgtggccggcgcaccatgccgggcggcgacggctttcctgcatttcggccccggggatcggccccgatccggcctggaggcgaaggaaagacggatcaggacacgcccggcgtcttccctcgcccggcggcgtcgccccacagaacggttatggttccatgagagacttcaagggcatgaagcgtcagcgcggacgcaacaggaagcccggcggcgccaacaacgccaacaacgccaatccgaaccgttcgtgggactcgcaggggcccgagaacatcaaggtccgcggcaacgcgcagaccgtgtacgagcgctatcagcagctggcgcgcgacgcctcgtcctccggcgaccgggtgttggccgagaactaccagcagcacgccgagcactattatcgcgtgctgcgggcgctccagccgcagaagtccttctccgacatcgccgcgcgcgagctgtcgcaccagggcttcgacatcgacttcgaagacgagtcgggcgctcaggccgccgccttcatcgccgctcagcaggccgccgaaaaggccgaggccgaccgggcggagcagcagcgtcaacgcgaggatcgcgccgagcagcagcgccgcgaacgcgaggaacgcacccgtcaggaacgccccgagcggtctgagcgccaagaccgcgacgccgaagagggcgaggctcgagccgaaggcgaaggcggcggtcgccgcgaaagccgccgcgagcgctgggagcgccggcgcgaggagcgcacccgccgcttcgaggcgcaagcgtcgggagacgtcgagaccgaggcccagccccccgtcgaaacggccgaaccggaaccgaccgcgcccgccgaagcgacgccgccggcggagttgatggaacccgcagcggtccaccaggacgcggaaccgccggcccaacggcccgcgcgtcgcgcacgcacgccgcgggcgatcgcggaagacgggtccgctgcaagcttgccgagctttctgacccgctccacccgcacggaaggctcggatgaggccggggaagaagcgcctcgccgccgtgcgacgcggcgcaaggccgagcccgccccgcactccgaagaaccggaaacaacctaggcgagaaaattcaccgtccagcaactctcgaccggcatgatcccatcgaactgggggatggtgcatggaacgggtggtgttggtcggagccttggcgctcgccgcggcgacggcgggctgggcgatggcgttggggtctcgcggccgggcggaacgtctgctgcgagagaacgaaacgctggagcaacgggtgcgggaacgcacgcgcgcgcaggcgctggagctgtctcgcgcccaagcgcttcgactttccgaagccagccagtccaagtccgacttcctcaacggcctgggccatgaactcagaacgccgctcaacgccgtgatcggcttcgccgaactgatgcggatgaatgcggcggccgagccgttgacccgtcggcaggatcaggccgtgcatcagatcctgggcgccagcgccgaactgcgggacctggtcgatcaggtgacggccttcgcccgccttcaggcgggacgcgtgtccctgtcgatagagcgtgtggatccgcaggtccttctgcgtcaggtctgcgaccgtctggcgtcgctggcgcaagccagaggcgtcaccctggaccttcccacgcccgaggccgggatttgcgtcgccgccgatcgcgggcgcctgcacgagacgctgacgacgctgatcagccacgcgatcggtcgaagctcgtccgacgccgtggtctcgatcgcgtttgaggccgatgacgacgccgaactggtcgtgcgggtgtcggacgcggcgggatcgccgacgtcggcggagctggggacgctgttcaagccgtttgaaacctttagcgaccccgccctgcctcggggcgaagtcatgaacctggcgctggcgcggggattggtcgaggcgatgggcggccgactgaccgccgcagtgggcgccgacggtctggacatcgtcttgaccctggcgcgagcggctcggcgggacatgccggtcgtcgccgcgccggacaggccgctcccgccggcgaccctgctgtacgtcgaggacaatccatccaacatcgccctgatgcgccaggtgatcacggccctggggcctctggcgctgcatgtggccgagacgggtccggaaggcctgaccttggcgcgcgacctgcggccggacgtggtgatcctggacatcaacctgcccggcatggacggaatcgaggtgaaggcgcggctggacggcgatcccctgacccgcgacatccctgttatcgccctgtccgccggggccctgccggatgatctcgcaaaggtcggggcctccggcttctccacctacctcgccaagccgctgcatgtcccggccctggctcaggcgctggagcgggctctcgccgaagctgcggaagacccgaggggcgaacagatgcgggcgaccggctcggcctgcgcataggcgtcggcgaacaccgcccttgacgcggccccgttgttccgggtcaacacgggtcttgttctgcaaggagccgccgcttgcgtctcgttcgttcccgatcgatcatcgcctccctgctcatcctggccgccgcgggttgcgccacgtcgccccccgccacgccgccggtcgagaaggcgtccccagcgccagctccatctgcctggcgcgccgaggccagcgccgccgatcaggaccgccatgaccgtctgggcgaggcctggacacgggccctggatcaggcccgccgcctgccgggatcgggcgacctgacgcgcgtgggcgagttgatcgcgccggatgcggcgcggccgggcgtggcgccgccgccgggcgcctatcgctgccgaacggtgaagctgggctcccagtcggagacggccggcgaagaggccgggttgggctatgtggtctatggctggttcgcctgccgcatcgagcagaccccagagggcttgcgcttcatcaagctcacgggatcgcagcgcccgtccggccggctcttcgccgacaccgaccggcgcatgattcttctgggagcgatggcgcttggcggcgagacgacctcgcccgcctacgggcagtccgccgaccgcgacatgctggcggtgctggagcggatcggcgagcggcgctggcggctggtcacgccctggccgcaggcggaatcgacgctcgacctcattgaactggtcccagccgcctgaggcgcgttgcggcggcgagggcgatggcttaatcgcccgccatgagcaccgacacccccgacgacgccaccgcccgcccgctcgcccgcaacccgcgcggcttcggcgacaagcgcggaccggacctgctggccgagcgccggatcgtggccgaggtgtcgcgcgtctaccaacgctggggctttgaggcgctggagacgccggcgttcgaatacgccgacgccctgggcaagttcctgccggactccgaccgccccaacgagggggtgttcgcgcttcaggacgacgcagggtcggacacgcccggcgactggatggccctgcgatacgaccacaccgcgcctctggctcggttcgcggcgcagaattgggagaccctgcccaagcccttccgccgctacgcctatgggccggtctggcgcaacgaaaagcctggtcccgggcgcttccgcgaattctggcagtgcgacgccgacaccgtgggctccgaccggcccgaagccgacgccgagatcatcgccatggcgggcgaaggccttcgcgcggccgggcttgcggacggccaggcggtgatccgcgtctccaaccgcaagctgttcgacggcctgttcgacgccggaggcgtgtccgatccggcgcagcggctgaccgccttgcgcgccgtggacaagttcgaccgcctgggctgggagggggtcgcggccctgcttggcgaggggcggctggacgagtccggcgactataccaggggcgcccgcctgccttcgtccgtcaccgacgcgatccaggcctttttggcgtccgcatcaaaccccgacatgacgcgggctgaaacgctgcggacggtcgcgaactgcggcgcgccgctgggggcggccggcgaggcggcgctcgcggaactctccgccatcgacgaggcgctgaaggccatgcgggtggaagaggcggcggtgcgtttcgatccgaccattgtgcgcgggctggaatactacaccggcgcggtgttcgaggccgaacttctgctggagaccacggacgacagggggcggccggtgcggttcggctccatcggcgggggcggtcgctatgacgacctggtggcccgcttcaccggccagagcctgcccgcgacgggcttttcgttcggcgtgtcgcgcctcgcggccgccttgcgcgccgcaggccacggtgcggcgggcgcgacgcgggggccggtggtggtgatcgccttttcggacgccgacacgccccattatctgtcggccgtcgccgaactgcgcgccgccggcgtcgcggccgaactctacctgggtcgggcgggcatgaaggcgcagatgaaatacgccgatcgccggggcgcacccgccgccgtgctgctgggcggcgacgagatcgcccaggggctggtcacgatcaaggacctggacgcgggtcgcgctgcggcccgaggcatcgcggacaacgaggcttggaaggccgaacgtcccggccagcaaaccgtcccacgcgaccagctcgccgccgtcatccaggccattctcgaataggcttcgataacgagacaggctggagaggtgttttcgacgttttttcgaagaaaccctgtcgaggcggcgaggcggcgttgacttggacccagttaaggcgtcatttggtctcactcgagaagccagacgcaaacgcggtgcttcttgaaggcgtttcggggaggaaacgtccgctcagtaagagcgcaaagagcccgctgcgatgtatcccccgcagcgggctttttcgcgtctgaagctctggagtctcgttacgggcatgaaaaaggccgcctcgcgggaagcgaagcggccttgtcgacgaggttcgtgcgcctagggttcaggcggcttccttctggcgcgaaggatggaagaacagcgcctggctgatcgccgccttcaccgtctcgggctggaacggcttggtgatcaggaaggtcggctccggacgctcgcccgtcagcaggcgctcggggaaggcggtgatgaagatcacgggcacgtcgatgctcttcaggatgtccttgaccgcatcgatgccggacgatccgtcagccagctggatgtccgccagcaccagacccggacggtgacgcgaaaccgcatccaccgcttcgtcgtgagtcgtggccgtgccggtgacccggtggcccagctcccgcacgaggctttcgatgtccgccgagatgatggcttcgtcctcgatgatcagcacatcggtggcgagctcggcgtcgatgtcggactgagcgtccgagatcagccgctccacgtcgcgcggatcggccgacaggatttgcgcggcctcggacggggtgaaaccttccagcgccgtcagcagaaaggcctgacgggaccgcggcgagatgcgcatcagccggcgggacgcgtcctcgcgcccgtccaggccgctttcatcctccagccgggctccggtggacgaccagatggcgtgaaacacatgataaagcgcgacgcgcggcgtcatctccggaggcagctgctgctccccggccgccagagcctccagcgccacgcgcacatagttgtcgcccgtcgactgatcgccggtcagcgctcgcgcataacgacggacatacggaagatgcggcgctagcctggccaagagactcatggatattccccgacgaaaatcgccctcccgatcagatcgggaaagcgctacagcgttgcagaacgtgcgcacaccaccacggttccacgccgtggcgcaagacctgcaacaaagtgcggacgtcgccggaaccgccggaagggggcggcgtttaggccgcttgattatcacactgcaagttgggggcggtgtcccgtacatgactgattcatcccacgcctcacggcgggaccctgtcgcgcctgacgacgaggctggtctcgaggaggcgcgactgcgccagcaagccatcggcgtgaagctgcggcacatgttcgaccaggtggtcaatgaacctgttccggacgagttcctggatatcctgcgccgcgccgacgcccgtgcgtcgcaaggcgaccaatcatgagcaccgcacgcctgggcgccgccccaaaaccgccctcggccgacgacgcggccttcaagaccgaactggtcacgctgatcccgcacctgcgcgccttcgcccggaccctgaccggcgatccgaccgcggccgacgatctggcccaggacgccatgatgaaggcctgggacgcgcgcgcctcgtaccagatgggcaccaacatgaaggcttggaccttcatgatcctgcgcaaccagttctactcggaaaagcgacgctcctggcggcagtcgcagctggatcaggaagccgccgaacgcaccctcgtcgccgtggacgaccccgaggcgccggtcgctctggacgaattgcgtcaggcgctgaagaccctgccggaagagcagcgagaggcgctgatcctggtgggcgccggcggcttcgcctatgaagaggcggccgagatctgcggttgcgccgtcggcacggtgaagagccgcgtcagccgcgcacgtcgcgcccttcaggccaccctggagaagggcggctacggccgcgacggcaaggcggccggcgacgccatgcgctcgattttggccgacgcggaccgtctgagcggcgcccggaactgacatgaggcgtctggcggccgtgggccggagcttcgggcgcggctcgccccgctttcagggcatccggttcaggctcggcgtcgccatggcgctggccctgctgccgatcttcatcgtcagcatcatccagacgcaggaccatttccgcatccaggccgaagagcgccgtcgcgatctcgagctcgcggtcgaacgcagcgccgcggcggcccggggacggctggacagcgctcaggtcctgctcagggctttgagccccgacgtggacgatccggactgccaagcgcggatgtcggcgctggtcgggcggctggagggctatgaggggctttaccggctgaccgccgacggccgactggtgtgcgactcctcggctccgccccctccggtcgatcccgcacccgatttggacgccgacagcgccgccattgcgtcgcccgcccccccgacgcccgccatcaacggccgcagcagcgcgggcgaggcctggttccaaaggctgcggcagggcgacgagctggtggtgacgcgggccccgcccagcgtcttcgacgggcggccgtccctgatcgtcgcgatccgggccgagcggccgatgggcgggttcgacggggccatggcggcggtcattcccttgcagacgctgcagccggacatcgacgaccccgcgcttccagaggattcccaggccgccctgacggatgcggccggacagcttctggtggccaccgacgccgacaccttccgcctgtcgggacgccagacgctgaacgggtgggtggcccgcgccgcggacggcccttcggtcttccagggcaaggatgcgcatggagagcggcgctactacgccgggtcggccctggcggggaatgacgtttacgccctgctgtcggcgcccgcgcccggcctcttgtcgtgggcgcgactgaacccgatcggcacgctgctgctgccgctaggcgcgtggctgaccgccttcgcggccgtgatgctgctgtccgagcgcatcttcatccgctggctggattacctggagcggatcgccgccatctacgccaaggggcgcttttccgtacgccctctgcaggccatgaacgcgccttcggaaatccgcaccatggcgcgcacccttgacgaaatggccgaggccatcatcgcgcgcgaccgctcgctgaccgaaagcctgatggagaaggacgcgctgatgcgcgagatccaccaccgggtgaagaacaacctccagatcatctcgtctctgctgtcgatgcagcagcgggcgctgaccgacgcccccgcgaaggcggcgctgggcgacacgcgccaacgcatctcggcgctcgccctgatctatcgcaccctttatcaaagcgaggacatccggcacgccgacgcccgcgagttcctgacggaactggtgggacagctggtggccagcgaggcggcgcggggtcccgtcgtcgtgtccaaggtcgaggccgactctctcgtggtcgatcccgacaagctggcgcccctggccctgtggctggtcgaggcggtcaccaatgcgcagaagcacgccttcgccggccgcggcgggcggctggacgtgcgcttccgcgtcaacggcgagcgcagcatcctggaggtcgaggacgacgggccgggcgcctcggccgccggcgcccagtcgggcgtgggccgcaccctgatgggcgccttcgccaagcagttgcgcggcgatttcgaactggtcgccgcgccgtcgggcggcgccatcgcccgcatgaccttcgccacgccggaggcgctcagccccgtggatccggccgatcagccggtgcggccgttcggaaccccggctcgccccttgcgttgatgcggcttggccgacgacgcgtcgccggcgcttcatcggagctgtcgccatgcgcaagctgtttgttttcgtcgccgccgccgccgccctgaccaccgcggcctgcaacaccatttccggcgtgggccgcgacacccaggcggcgggcaaggccgtcacggaatgcgctcagggccagacctgctgaggcctgcccgccatcatcatcgacgacaacgaagaggctcgccctgcggcgagcctttttgctttgtggagccgacgccatgacccttgatccacgccaggccggcctcgccctgctgcgcgaacacgccctgatcggcggcgagccgtcgcgtggctcaagcgaggtcatcgccgtcgacgatccggcgaccggcgagatcatcggccatgttcccaaactcggcgcctcggagacggagcaggccatccgggcggccgatgaggcgtttccggcttggtcgcaggacgatccgcatgcgcgcggccgcttcctgcgcgactgggccgggctgatcgacgaccacgcggacggcctggccgccctgatgtcgatggagaacggcaagccgttcgaggaggccaggggtgaggtcgcctacgccaacggcttcatcaagtggttcgcgggcgaggccgagcgcctgacgggagaaacgcacgacagcccgctgggccatctgatcttgaccttccgggaagcggtcggcccctgcgccctgatcacgccctggaacttcccggccgccatgctgacgcgaaagctgggaccggcctttgcggccggctgcaccgccgtggtcaagccggccagccagacgcccttcaccgccatcgcgctggcggagcttgcctacgaagccgggttgccgccgggtgtcctcagcgtcgtcaccggggaggcaggcgagatcggcggcgtcctgaccgcctcgcccctgatccgcaaactgtccttcaccggctcgacgcccgtgggccgcacactggccgagcagtgcgcgccgacgctgaagcgggtgtcgatggagctgggcggcgcggcgcccctgatcgttttcgacgacgccgatctggatcttgcggttgccgaaaccatcaagggcaagttccgcaactcgggccagacctgcgtctgccccaatcgcgtctatgttgagcgttcggtcgcgcgcgacttcgccgaccgtctggcgtccgaggtcgcgaagctcccggtcggcggcggcttcgacgacggcgtcaaggtcgggcccttgatcgaggacaaggcgctggacaaggtcgaggcgcatctggcccgcatcgtcgcggacggcggcgaggtgctgacgggcggcgcacggcacgaacgcggcggccgcttcttccagcccaccgtgaccttcggcggcgacgacgccctgttccgcgaggaggaaacctttggtccggtcgtgcccgtcttcgccttcgacggcgaggaggaggttctggacaaggccaacgccagcgacctgggcctcgcctcctatctgttcacgcgcgacctgaaccgggccatgcggctgggccgtcggatcgaggccggcatgtgcgggatcaacaccggcatcatctccacgacggtcgcgccgttcggcggcgtcaagcagtccggctacggccgtgagggctcgcagcacgggatcgaggagtatgtgaacatcagggccgtgaccctggcgctcggctgaaaccgcaaggggcgggcgctttcggcgcccgcccctccgcttgacccttgaaggctgaggctcagtcctcttcggcggcttccgcctcttccttggtcttgtgcgacacgccttcttcttcggccggcggcgaatagacggtgaacagcttcagcggctcctcgcccttgttgatgatgttgtgcaccgcgcccttggggatgaccacgatgtggttcggcgtcaccttggagcgcgagccgtcgaccacgacctggccctcgccggccacgaaaaaggtcgtctggtcggcgtcgtgcgtttcttcgccgatgtcgtcgccgggctcgatgctcatcatcacgatctggcactgctcgtcgtaatagacttccttctggaagtgcttgttgtccgtggtcagcttgatgatgtctttgttgaagacggccatgatcgttccttctgcaattgagccgactcaacacccatgcgcgcacgcggttcggccgcaggctcgaaaaagccgcgcatctgcggcataagccggcaatgaagttccttgatcaggccaagatctatatccgctccggctccggcggcgcgggctccgtgtcgttccggcgcgagaagttcattcccaacggcggccccgacggcggcgacggcgggcggggcggcgacgtctggatcgaggctgtggaggggctgaacaccctgattgactaccgctaccagcagcatttcaaggcccagaccggcaaccacggccagggccgccagatgcacggcgccaagggcgaggacgtggtactgaaggtgccggtcggcacacaggtgttggacgaggacaaggagacggtgctgctggacatggacgtggccggccggtccgaactactgctgaagggcggcaacggcggctggggcaatgtccgcttcaaggggcctgtcaatcaggctccgcgccacgccaatcccggacaggacggccaggagcgctggatctggctgcggctgaagctgatcgccgacatcggcctggcgggcctgccgaacgcgggcaagtcgacctttctgtccgccgccagcgccgcccggcccaaggtcgccgactatcccttcaccaccctgacgcccaacctcggcatggtggacctgtctccgaccgaacgcttcgtcatcgccgacattcccggcctgatcgaaggcgcgtccgaaggcgcggggctcggcacccgtttcctgggtcacgtcgagcgttcggcctctctgatccacctgatcgacggcacgcaggacgacgtggccgaggcctatcgcattatccgcggcgagctggaggcctacggcgaagggctggccgacaaggccgagatcctggcgctgaacaagatcgacgccctgacgcctgaactgcgcgaggaaaaggttgcggagctggaggccgtcgcgggccgccgacccatgctggtgtccggcgtctcgggcgaaggcgtgccggagctgctgcgcgcggcctgggcggaggtcagaaagacgcgcggcgaagtcgccgaccccgacgccgaggtcgcgcagaccaccggctggacaccctgatccgcgcctgcgggacaacggtttgccgccggctgcgttcacgctaggaacggtgaagctgaggagacgccggtgaccgccctgagacgcgtgctgatctggtcgatcatggctcttgtggtcggggcgctgctggtcgcggcgggctactgggcctactggaacttctattcccgcttccagcccgtgacgatcagccgcgccccggccgagatccaacgcctgctggacgaggcgtcctgggtgtcgccaggcgggggcgacacgccgctctatgtcgtcgcctaccacgacaacccggccgcgcgccgcttcgagcgcgaggcggcgccgcaactgcgggcggcgggcgtcgatgtgcgcgctatcgccttcgcgcgccccgaccaggacggccggattcagtccacagcggccgagcgtgcgaccgtcgccgagctttggctgacgcgcgactggtcgctgtacgagcaatggagcgcgacgccggcccgtcagtggcgcgccgagggcctgcccagcgcggaccgcaacctggcgcgcgcggccgtggtcgacgccggccgcgtctttgtggagcgcctcacgacgctgctgcgtgacgcgggggtggagacacagtatccgatcatcctgtggcgcgatcgccaagggttcctcaaggcctgcgcctgcgcggacgaccggtcctgggcctttgtccgcgacgacctggacgcctcgggacgctcggcgccgccgccggtcgagaccgaagcctcgtccgaggaggcgccggagaatgggcgagcggcccccgccgatcccggcctgccctatccgagcctgcccgccatgccgccatcgccgtcgggcgtcgccccggcccggcctctgtccccgcccggaacatcgacgccccggacgacgcctcagacctcgccccaggcgccgccgaacgtccagcctcgggcgcccgccgccacgccccgaccgcaacggtcgacgccatcgcgtcagccgcccgaggccaagcgcggcgacgacaccaccttctactgaccggctagagccgagcgcaggccgcgatcaggtgctcgacatcctccgtattctgataaaggccaaatccgaagcggatcacgtcgtcgcgcacgtctgtgacgatgtcgccggcgagcagctgttcgcgccagcgcgccgcctccgggtggcgcagcgccagaaagcgcgcacgggcgccgtcgcccgccagcggattgagcaggaccgcctgagacagggggccggcgcggccgtcctccaccgcatcctggaacagctgcatcagcgtgcgggcgtgatccgccaccgcagccgtgtcaagcccagtgtccgccagcattcggcgcgccgcgttgaagcgatagagcgccgaacagtcgaaggtcgctccccagaaccgcccgccgtcgctgcggtactgaaccccgcccggcggccccgaaagatcgccgaactccgcgaaccagccggtgatcgccgggcgcgggcagaagccgtctggcgaatgcaggaagcacgcaccctcgcccgccatggcgtatttgtagccgccggccatgtagaagacgcggtccgccacgcgcgacaggtcggtcggcgtggccatgaagccgtgatagccgtcgatcagcacccaaggtccctcgggccgcgccagttcggccagagcctcgaagcggtcgaacacctgaccggtgcggaaaaagacatggctgaccacgatccagtcgtggccgccctgttcggcagcctgaaggaagcgctcgccgaagctgctgaacggctccagcgggacgcgcgtgaccagcgcctcgcccgtttcgacccagcgatcggcctggcgccggaacgagtggaactcgccgtcggtggacaggatgcggaccggccgccgctcgaaccccgagaaaatcctcagcaggaagtcgtgcgtgttggacgagaacaccacgctgtcgggcgacggcaggttcagctcgcgcccgacatgcgcctgcgcctcagggatgacttgtccgaacaccagatcccacttgcggtccgcatgagcgttggcgtcgatccacgcctgcgtctgcgcctcgaagctggcgtccggccacaggtggtggctgtgcgcggcgaagtgcaggcgctcgggcgcaagcgatagggcgcgggagaacagggctttgtggctcatgcaggcacattaggcgcttgccgccgtgcacccaagacaagaggcggaccacattgcgatccgcctccaggtcccatcagttaagtctgcgcctagaccaacgccccgtggcaatgcttgaacttgcggcccgagccgcaggggcaggcggcgttgcggccggtcatctcccagccgacgggaagcgcctcgaccggcaggcgagcgcggtcgtcgccgatcagctggccttccgggttctgcgcggccgtattcgccatctcgttctcgccggtgccggggttcaggtggatctcctggaactcgggtagttcgggcggcggctggaagcggaactccaccgtcatcagccagcgcgtcacattgtggcgcagctcgttcagcaggttctcgaacagggtgaaggcttcggtcttgtactcgttcagcggatcgcgctggccgtagccgcgcaggccgatgacgccgcgcaggtggtccaggtggaccaggtgctcgcgccactgcatgtcgatcatctgcagcatgaactgcttttcgagcccccgcgtctgatcggctccgatcagctccagccgctcggccgcacgcgcggcggcggcgtcttgcagccgctcctcgatctcctcgttggacacgccctcttcggccgcccagtcacgcagcggcagctcaagtcccagcgtcgagcggaccttttcgtccagaccctcgatgtcccactgctcggcataggccttgggcggcatgtagcgctcgaccaggtcggtgacgacctcgcggcggaagtcgccgaccagttcggacaggtcctcggagtccatgaactcctggcgctgctcgaacaccgccttgcgctggtcgttcacgacgtcgtcgtacttcagcaggttcttgcggatgtcgtagttgcgctgctcgacgcgcttctgcgctgtctcgatggcgcggttcagccaggggtgggtgatcgcctcgccctcggccacgccgaacgtcttcatgatcgagtcgagacggtcgccggcgaaaatgcgcagcaggtcgtcctcgcacgacagatagaatttcgacacgccggggtcgccctgccgaccggtgcggccacggagctgattgtcgatgcggcggctttcgtggcgttcggtgccgagcacgaaaaggccgccggcggcgagagccttctgcttctgtacggcgatgtccgccttgaactcggcttccttggcggcttccgcctcgggcgtgacctccagcgccatgttgcgctgctccagcatccacttctgcatcctcatctcgaggttgccgcccagctggatgtcggtgccgcgtccggccatgttggtggcgatggtgaccgcgcccggcaggcccgcgtccgccacgatataggcttcctgctcgtgctggcgcgcgttcaggacgttgtgcggaatgccgcgcagcctggtctcgtaggtgatgtcataggcggcgtcgccgaccttttccgcctccttggcctttccggcgtattcggctttcagcgtgcgcgcggtttcgaccttgtactcatagcggctcaggagatcggacagctgctccgaccgttcgatcgacacggtgccgaccaggatgggctgaccggccagatggcactcggcgatctggcgcgcgatcgcctggttcttctcggcgtgggtgcgatagacctcgtcgtcgtggtccttgcgctggatcggccggttggtcggcacctccagtacgtccatcttgtagatgtcgccgaactcctgcgcctcggtcgcggcggtgccggtcatgcccgacagcttctcgtacaggcggaagtagttctggatggtgaccgaggccagggtctggttctcgggctggatcttgacgccttccttggcctcgatggcctgatgcaggccttcggacaggcggcgccccgtcatcatgcggccggtgaactcgtcgatcaggacgatctcttcgcccttgatgatgtagtccttgtcgcgctggtacagggtgttggcgcgcagggcctggttggtgtggtgcaccaggctgatgttggcggcgtcatacaggccggtggtgtcctcggcgaaatggccgccctgctccagcgcctgctcgatccgctcagacccttcttcggtcagcaggacctgcttctgcttttcgtccagctcgtaggtcgacttgtcggtgatcagctctttgatcaggccgtccaggatcttgtacaggtccgagcggtcctcggtcgggcccgagatgatcaggggcgtgcgcgcctcgtcgatcaggatggagtcgacctcgtcgacgatggcgaagttgtgcgggcgctgcaccatctcgcgccggtcatagaccaggttgtcgcgcagatagtcgaagccgaattcgttgttggtgccataggtgacgtcggcggcgtaggcggcctgacgctggccctggctcagaccgttgacgatcacgccgacttcgaggcccaggaagcgatagacgcggcccatggtctcggcgtcgcgtcgcgccagatagtcgttcacggtgatcacgtgcacgcccttgcccgccagcgcgttcagatacaccggcgccacggccaccagcgtcttgccctcgccggtccgcatctcggcgatgccgccttcgtgcaggatcatgccgccggccagctgaacgtcgtactgacgctggcccagcacccgcttggaggcctcgcgcaccacggcgaaggcttccggcaggatcttgtccaggctttcgccgcgctccagccgatccttgaaggcgtccgtcatcatccgcagctcgtcgtcggacagggcggcgaacttgggctccagcacattgatgcgctgggcctgatcctggaaagccttgaccttgcggtcgttggaagagccgaagagtttcttggcgaagccgagcatgttggatccggtaggcggtcaggcgttttggagcttgagcggctctgaaatcccgagtggggcggcggtgatgcgggtcggccggcggtcggaccggcggcggccccgtcgccgcgaaacgggcgcacgcgaagggccgcgcggacgatcaaaacccctcgccttgggcgcaggcgggacttaagcaccgcctctacccctgtcaacgcaaggggttttcacgccccttcacgacggagcgcgcccccatgagccccatccggcggactcccggtctggtcgcgatcctgctggcggtcggcctgacggcctcgggctgcgggcgcgacggcgacgaccgcgcgcctgagccgaacgatcgcgccgtggccgaggtgcagggccagaccctctgggcctccgacgtcaagcgcgaggcggtggctcaagggctggtcggcgagggcgagacgctggacgtcacctccgacctgttccggcgcgtgctggacgaggtcatcgaccagaagctgctggcccgcgaggccgagcgccgcaagctggacgactctcccttggcccagcgccggctggaggccacgcgcgagcgcatcctgggcgacatgctggtggagacggtggtgaacggcgccgtgtcggaaaaggcggtcgagacgctgtacaacgagcagttgcggttggcgaagacgtccgaagaggtgcgggtgcggctgatcctgtcgcggagcaagccggaggccgacgcggtgctgggcatcctgggccagggcgcggcgttcgaggcggtggcgggcgagcgctctatcgacgaggcgacgcggttctccggcggcgacctgggctactccacgctggatgtgatgccccagacctacgcagacgcattgcgcgaccggccggccggctcggtcgtggggcctttccagaccgagggcggctgggccgtgctgcgggtcgaggaccgtcggcgcgagacgccgccgacgttggagcaggcgcggccccagatcgtccgctatctgacctatgaaggcgtgcgccagctcctggaacagctgcgcggcaaggccgaggtcgatgtgctgctgcccgccgacacgcctccggcgccgcgtccgagcgcgccggcgcctgcggcatagacccagcggcatagaccatgagcaagacgccccctcgccccgcctccaccagccagaagatcgaacaggcgcttgaaaaggcgctggatcccctggcgtcggcgctgaagcgcgccacgcgtacgccgacgggcggcgccgtgccgccggacgcgccggcaggcaaacccggtctgaaggtctcgcccctggccgtgccgttcccggccattccgcccatcggcggggtggagatcgcgaccgcccgcgccggcttctacaagcatgagcgcgacgacctggtggtgttccgcttcgccgagaacaccaactgcgccggcgtcctgacgcggcacaaggtcggctcggcccccgtcgactggtgtcgacggcgcctggaggcggcggacggcggcaagggcgtgcgggcgcttgtggtcaacgccggatgcgccaacgccttcaccggcaagcagggcgccgacgccgcccggcgcacggcctcggaggtcgccaaacaattcggctgtcgccagcgcgacgtgatgctggcctcgaccggcgtcatcggcgtggtgctggacgacggcaagatcgcggcgcgcctgccggagatcgcgggatcgctccacgccgacaactgggcggcggccggtcgcgccatcatgaccaccgacacctttccgaagggcgcctacgccgaggccgagatcgagggacacacggtcaggatcgccggcgtcgccaagggctcgggcatgatcgcgcccgacatggcgaccatgctggcctttatcgtcaccgacgcctgcatcgcgcctccggtgctgaaggcgctcttgggcctgcacgtgcgcaccaccttcaactcggtcacggtggacggcgacacctccaccaacgacacctgcctgatgttcgccacaggcgcctcgggcgcgccgcgcatcggccgggtcggcgaccggcggctgaaggacttctccgccgcgcttgaccgcgtcatgctggatctggcgcaccagctggtgcgggacggcgagggcgccaccaagttcgtgcgggtccaggtggacggcgccgcctctcccgcctctgcccgcaagctggccaagtccatcgccgacagccctctggtgaagaccgccatcgccggggaggacgccaactggggccgcgtggtcatggcggtgggcaagacggaggagcccgtcgaccgggaccgcctggccatccgcttcggcccccatgtcgccgcgatcgacggcgcgccggccgccgactacgacgaggcgaccatgagcgcctatatgaagaacgccgagatcgacatcagcgtggacgtcggctccggccgcgcctcggccaccgtctggacctgcgatctcaccaagggctacatcgagatcaacggcgactatcgctcgtgaccgcgccgttgaagacggtctttgtcgtcgccgtcgcgctgatcgaccccgacggtcgggtgctgatcgcgcagcgcccggagggcaagcagttggccggcctgtgggagttccccggcggcaaggtcgaggcgggcgagcggccggaacaggcgctgatccgcgaactgcgggaagaactcggcatcgacgtcaacgaggcttgtctggcgccgttcgttttcgccagccacgcttacgattcgtttcacctgttcatgccactgtacctgtgccggcgctggtcgggcgtggtcatcgcgcgcgagcacgccggcctggcctgggtgaagccgaaccggctgtccgactatcccatgccgcctgcggacgaacctctggtcgcctggttgcgcgacctgctttgatgatcgccacgaggagggcggacatgcgacgaccttcgctttccctcttcaggcgcctgacgcgtgaccggaagggcgccacggccatcgaatacggcctgatcgttgcaatgatctccctcgccatcgtggctgctgtgggcgggatcggcgacaagatcagcgcggccctgggccggcttgccgaggcgcttagctaggccggttcctcgccggactgctccttgacgccgagcgcgtccgccagccgcatcttggccgagccgcgcggcagcggcttttgctggctttcgtgcggcgcccatccggccagatggatgatctcgaaactgaccggaatgcgtccgtcggcgtcgccgtgacgctcggcatagagcgacgccgcgcgcgcgatcacagcccggctcaagggccggacggcgccggccagcgcattggtctcccccatggcccgcaggtcccggatcagggcgaacaggtcagggtagcgcacggtgaagcggtccacgtccgatacgggcagcgcaaagcccgcccgctgaagcagcgccgccccgtcataggcgtccgcgaacggcgagattcgcgcctgcgccccgccccgttcggcaagctccgcctccgtcagcacgccccgcagctccttcagcgtgcccgccccgaacagtgcgccgatgaacaggccgtccggctgcagcgcgcgtttgatctgggccagcgctcccggcaggtcgttggcccagtgcagggtcagcagcgacacgatgaggttggcggacgcgtcctccaccggcagcgcctcggcgcctggcgcggcccgctgagagagagtcgtcggccggacgaccggtccgatccgctgggcggcgtcgctcatgcgaaccgcctcttcgaacacgccgccttgcgccgacaggtcgacggcgagggggaaatcccgcaggatcgcctccaggctgcccgccgcgttatcggccgcccgccggtgcaggaagtcggccccagggaaggtcgcggcggaccggcgcaggcgggcttcgcgccgcacggggtcgaagatgcggggcgggccggaggcggctgacaaggttggggcggagggggacggtgtcatgcgcgatcaagatggaggctggcggaccgcctgcaaagcggcggggctgcatttgcgcgatgcgggccgcggcttggccgatctgatcctgccgccggtcgcccccgacagccgcgaagccgccgcatcggccggtctctcgccgggcgcctggagccgcatcgtctttctggaggcgccggtgtgcgacggctgcggcgccgcgttcgagttcgacggcggccccttcgcctccgaccggtgtgcggcctgcatcgccctgccctacgccttctcgcgggcgcgggcggcctgcgtctatgacgacgcctcgcgcgggccgatcctgcgcttcaagcatggcgaccagcagcagttcggccctctgttcgcgcggtggatcggccgctcggcggctgatctgctgtccgaggcggacgcggtcgcgcccgtgccgctgcaccggctgcgtcttttgtcgcgccgcttcaaccaggcggccgagatcgcccggccgctggcacgtcacgcccgcctcgactacctgcccgacgccctgatccgcgcgacccacaccgccagccagggcggcaagagcgcgcgcggacgccgcctgaacgtcaccaaggcctttgccgtcaccgaaaacggccgcaggcggatcaagggtcggcgcatccttctggtggacgacgtgttgaccacgggcgcgacggccgaggcctgcgctcgcgccctgatcgaggccggggcgagggcggtggacctggcggtcgtggcccgggtgcgaaccgcccggcagctgactatctagacgccatcaacttcaggagttctcccttggccgacatcgtcatctacaccaagcctggttgcccctattgctcgcgcgccaaggcgctgctggagcgcaagggcgcggactatcaggagatcgtcgcctccaacgacccggcgctgaaggccgagatggtcgagaagtccggcggcaaggccaccttcccgcagatcttcatcgacgggaaacacgtcggcggctgcgacgacatccacgccctggatgcgcgcggcggcctggatccgctgctggccgcctgaagcctgcacatggacggcggcctcgacatcgcgctggtccagctgcgcacgccggcgacggcggacgcgggtctggcgcatgtcgaaccgctgatccgccaggcggcgtctgaaggcgcccgcctgatcctgacgccggaaggcaccaaccttctggaacagcgccgcgaccgccgctcggccgcgctgtcgagcgaaggcgaggatgccgccgtgatcggccttcgtcgcctcgcggccgagttgggcgtctggctgctgatcggctcggccatcgtgcggtcggatcgccagggcgacgaccgggccgccaaccgttcgctgctgatcggtcccgacggggcgatcgtcgcccgatacgacaagctgcatgtgttcgatgtcgatctgccgaacggcgagacctaccgcgagagcgccggcgtccgtcccggcgacagcgccgtggtcgcggagacgccgtggggccggctgggcctcagcgtctgctacgacatccgctttccgcacctgtatcgacagctcgccaaggccggcgcacggatgatcgccgtgcccgccgccttcaccgccccgacgggcgaggcgcattgggaggtgttgctgcgcgcccgcgccatcgagacgggcgccttcatcttggcgccggcgcagggcggcctccatgaggacggtcgccgcacctggggacgctccaccgtggtgtcgccttggggcgaggttctggcccgcgccgaccacgacgagccttgcattgtgacggccaagctggacatggaggcggtcacaaaggcccgccgggccatcccctccctgctgcacgaccgcgacttcagccccgttccatgatccgctacgcccttcgctgcgaccacgaccacggcttcgaggcctggttcggctcgtccgccgacttcgacgaccaggccggacgcggcctggtcgaatgccccttctgcggttcgcgcgccgtcgaaaaggcggtgatggctccggccgtcagcggcgcgcgcaagtccgccgccgcgcccgaggcggcgcgccagatgcagaccatgatgatggaggccgcgcgcgaggttcgcgcccatgtggaggccaacttcgactacgtcggcgaccgcttcgcccgcgaggcccgcgacatccacgaaggccgttccgaaaagcgcgagatctatggcgaggcgacgccggccgaggtgaaaaagctgaaggacgacggcgtgcccgtgtccgccctgccctcgccgccgcctgagccggagaagctgaattgactgcgctgggctggcggtcgatgcgaacggcggatctcgacgccgtggtcgagatcgcccgcctgtcctttcccgaccatcctgaagaccgcgcctgtttcgagaaccggctggccctctatccgcacggatgcttcgtcttggcgcccggcgacggcaaggccaggggctatctgatcgcctacccctggacggcggatgcggcgccgccgttgaacagctgcttttcagatctgccgggggacgcggcgctgatctacctgcacgacctcgccatccacccggaggcgcgcggcggcggatcgacgccggcgatcatcgagcgcctggctgagcggtcgcgcgccgccggctggccggcgctggccctggtggccgtcaacgccgccgcgcccttctgggcccgccaaggtttcgagccgcgcgatccgccgggcatggcccagaagctggcgacctatggcgcagacgcccgctacatggttcgcccgctctgacccctcagtcgcgcaaggcgaccatcatgtagtttacggccgcatcgtcggtctcgctccaacggtcggccagcgggtcgtaggccaggccataggggccatgcagggaaagcggctcctccgacagcatcaggcggatctcgtccggccgcaggaactggcgccagtcgtgcgtgccggcgggcacccaacgcagcacgtattccgccgccaccttgcccagcagcagcgagcgcaccgtccggttcagcgtcatcaccatcagcagaccgcccggcttcaccaggcgcgcgcaggtgcggataaagctttcggggtcggcgacgtgctcgatcacctccatggtcagcaccacgtcgaacggacccgcgccctccgcctccatctgctccaccgtggcggcgcggtagcggatgtcgagacccacctgatcggcatgggcccgcgccgtgccgatgttctcggacgaggcgtcgatggcggtgacgtcgaaacccatccggcgcatgggctctgccaacagcccgccgccgcaaccgatgtcgatcaggctgaggccgccaaagggctgacgcgccctggaatcgcgcccgaaccgcgccgccgcgtggtctcggatcagcttcagccgcgcaggattgaaccggtgcagcggtgcgaacggacccttggcgtcccaccattcggcggcctgcgccgagaagcgcgccacgtcggccgggtcgatcgaggcgccggaggcgatctccgcctcgcttgcggaaaaaccctcctgcgggcggggtatgcgaggcgtcgccgtatcgttagaagcgctcatgggcgggagggatgaaccctcgcgcccgctcacgcaagacaagccaagaggcgacacgcgacgatgacgcggccggacacttcgccacagacgacttcgcgcctggtgatgaagttcggcggcacctccatgggcgacctggagcgcatccgccgggccgcccggatcgtcgcggccgaggccgcctctggcaagtcggtggccgtggtggtctccgccatggcgggcaagaccaacgaactggtggcctggacggacggtgcgggaccctcggccgtggaggacgcgctgtctgacgacgaatacgacgtggtggtggcgtcgggcgagcaggtcacctcggggctcctggcgctgacgctgcgcaacatggggctgaacgcacggtcgtggatggggtggcaggtgccgatcctgaccgacgaggcccacggccgcgcgcgcatcgtcgacattcccggcgaggctctgggcgcggcgctggacagcggggagatcgccgtggtgccgggctttcagggcgtgacgccgggcggtcgcatcaccaccctggggcgcggcggctccgacacctcggcggtggcggtggcggcggcgcttgggtgctcctgcgacatctacaccgacgtggacggcgtctacaccaccgacccgcggatcgagagccgcgcccgccgtctgaacaaggtctcctacgaggagatgctggagatggcctcgctgggcgccaaggtgcttcagacccgctcggtcgagctggccatggccaagcgggtgccggtgcgcgtcctgtccagcttcattgaacccgacgcgaacggcgtcatgccggacaagggcggaaccctgatctgcgacgaggaggaaatcttggaaaagcgcatcgtgtccggcgtgaccatgagccgcgacgaggcccgcatcaccctgctgggcctgtccgaccgggtggacgcgccggccgacgtcttcacccgcctggccgaggccaacgtcaatgtcgacatgatcgttcagagccagtcgaggacggcggggacggtgaacctcaccttcaccaccggtcgccgcgacgcggttcgcgcggccgagctgatgcgggcggccaaggatcagctgtcgtttgaagagatccgcgtcgatgaggacgtggccaaggtgtcggtcgtcggcgtcggcatgcgcagccacgcaggcgtcgcccagaccatgttcaaggcccttgccgacaagggcgtcaagttccaggccatctcgacgtccgagatcaagatcagcgtcctgatcgacgcggcctatgcggaattggcggtgcgcgcgctacattcggcctacggcctggaagcggtctaaacaaacaacaacggcgcgacggtcgcgcctgaggagcaggagcgaggatgccggcgggcggagcgatgacgagggggccccgaaacctcctgcgccagatccgcgaggcgctgggcggggcgggcgcgggcgcgaccccggcgcaggaccggctgaacatggtggtgcggatcatcgcccgctccatggtggccgaggtctgctccatctatctgcggcgcgcctccggcgagcttgagctgttcgccaccgagggccttaatccggaggccgtgcacaacacccgcctgcgcgccggcgagggcctggtgggcgaggtcgcgcggctggcccagccggtcagcctgtcggatgcgcccacccaccccagcttctcctaccggcccgagacgggcgaggacccctatcacgcgtttctcggcgcgcctctgctgcgcggcgggcgggccatcggcgttctggtggtccagaaccgcaccgagcgccgctacgacgaggacgaggtcgaggacatccagaccatcgccatggtgctggccgaaaccgtggcctccggcgaactgctgggcccggacgaactccgagacgtggagctggcgccccatcggcccgagcggctgaagggccaacggttcgccgagggactcgccttcggccacgtggtgctgcatgaggcgccgctgccgcccgagcgcctcttgtccgacgatccggccatggaggaagcgcggctgaagctgggcctcgcggcgctgaagtccggcctcgacgccatgctggagggcggccagggcctggccggtccctcgttcgaggtgctggagacctatcgcatgttcgccgacgaccggggctggaaccggtcgctggaggaggcggtgcgcaacggcctgaccgccgaggcggcggtggaccgggtgcgcaacgagcaccgcgcccgcttcgcccaggcgcgcgacccctatatccgcgagcggctgcacgacttcgaggatctggccaaccggctgctgcgggtgctggcgggcgacaagccgggcgagcgcgaacttccggatgacgccatcctggtggcgcgcaatctgggtccagccgacctgctggaatatccgcgacacaagcttaaaggcctgctgctggaggaaggctcggccgccagccacgccgccattgtcgcccgcgccctgcagatcccctgcgtcggccggctggccggtctgcgtgaccgcctgtccgagaacgacatggtcatcgccgacggcgagaccggcgaggcctatctgcggccccgtcccgacatgctggaggcggttcggtcgcgcatggcggtgcgggaccagcgtcgggccgagttcgccctgctgcgcgacacgccggcggtgacgctggacggccagcggatcacccttctgaccaacgcgggcctggccgtggatctggagaacctgaacgagacgggcgctgagggcatcggcctgttccgcaccgagttccagttcatggtgtccgacgaactgccgcgcctggatgcgcagacggccctctatcgactggtgatggactcggccggcgggcgacccgtggtgttccgcaccctggacatcggcggcgacaaggtgctgccctatctcgaggcagagcgcgaggagaaccccgctctggggcggcgcgccatccgcctgggactggaccggccctccctgctgcggcttcagctgcgcgccttgctgaccgccgccgccgggcgcgagctgcgcgtcatgttcccgatgatcgccacggtggacgagttccgcgccgcccgcgaactggtcgacatcgaatgcgcctgggcccgccgtcgcggccgcaccctgcccgccctgctgcgggtgggcgccatgatcgaatgcccctcggtgctgtggcacctggacgccctgttgccgctgacggacttcgtctccatcggcaccaacgacctgttccagtacatgttcgccgccgaccgcaccaatccgctggtctccgaccgctacgacccgttgtcgccgccggcgctgcgcgccctgcagacgatccagaaggcgtgcgccgacaccggcacgcccgtttccatctgcggcgagctggcggggcggccgctggaggcctttgtgctgatcaccctgggcttcacccgtctatcggcgcccgccggcggcgtgggcccggtcaagcgcatgatcctgtcgacggacctttcggccgcgaagcgcggcctgaacagccttctgggcctgtcgtcgagctccatccgaggcgagatcgagtccctggcgcgcaagctgaacatcgccgtctgaccacgaggccgcgcctccatccgcgttgagcgctcggggtcgatcggctatgtctgcggcccatgacgcaatcggctgcggaccccgttcccgcacactcctctggcgagatcgacccggtcgatgcggccccttcgctgggcgacgccctgcgccaggcgcgcgaagtttccggccggtctatggctcagctgtcgatggagacccgcgtccatccgcgtttcctgatcgcgctggagcagaacgactggtcgacgctgccctcgcgggtgttcgccgccggctatgtgcgggcctacgccagtgcgctgcggctggacgaaaccgcggcggtggagcggttcaagcgcgacagccccgacacctccacgccgctgaaggcgcccatcggcatcgccttcgaggacgtgcgccggcagtcgccgcgcgtgatcgcggccgtggcggtgctggccgtcgccgtgatcggctggaacatctttcagcgcgccagcctgcgccaggcgccgcacccctccgacatcgtcgccgtgcccaagacctgggctgaacaggacgccgccgcccagctcaaggccgtgaccctgaacgcgccgcgtcaggcgccgcccgaccagaccacgccggagctctacgtcacgccggggctggagatgcagctgacgggcgtcgacccggccgatccggccgctgtcgccgccgcggccgccctgaaggcccagccggtgcagcgcgccttcaacccgcgcggcgcggtctacggcgccccggccaccgcgtcccaggtggtgctgcaggcgaacaagcccaccggcctggtggtgcgcacgccgagcggacaggtgctgttcgcacgccagctggccaagggcgagtcctggcgcgcaccgctgaacacctcggccgtggtcgacgcctccgagcccgccgccttcgatgtctatctgaacggcgagcacgccggagcgctggagcagccgctgacccccttgcagaccctgaacacccgcgccgtcgccatggcccgggacgtccaggctcaagccgccgcccagaccgcgcgtcaggcgcaggccgctgcgccgcccacaccgatcggctgacgcgcgggccgtggttccgccgtcatggaagtcctatatgctggcggcatgagcgaccacacccacgtccgtccctggcgccacatcgagcgccgcaagagccgcaaaatccgcgtgggctccgtcgaggtcggcggggacgcgccgatcagcgtccagtccatgaccaacacgccgaccacggacgcggcggccaccatcgaccagatccgccagctcgaagaagctggcgccgacatcgtgcgcgtctcctgccccgacgaggagtccaccgccgccttccgcaccatcgcgcgcgaggccaaggtcccgctggtggccgacatccacttccattaccggcgcggcatcgaggcggctcaggcgggcgccgcctgcttgcggatcaatcccggcaacatcggcagcgctgagcgggtgcgcgaggtggtccaggcggccaaggactatggctgctccatgcgcatcggcgtcaacgccggctcgctggagcgcgaactgctggagaaatacggcgagccctgccccgacgccatggtcgagtcagcgctgaatcacgcccgcatcctccaggaccacgacttccacgagttcaagatctcggtgaaggcgtccgatccgttcctgaccgtggccgcctatcagcagctggccgaggcgatcgactgcccgctgcacctgggcgtgaccgaggccgggccgcttcgcaccggcaccatcaagtcggccatcggcatgggctccatgctgtgggccggcatcggcgacaccatccgcgtgtccctggccgccgatccggtggaggagatcaaggtcggattcgacatcctgaagtcgctgggcctgcgccatcggggcgtcaacatcatcgcctgcccgtcctgcgcccgtcagggcttcaacgtcatcgagacggtggcgctgctggaggaacggttggcccatgtcgccacgccgatgagcctgtcgatcatcggctgtgtcgtgaacggcccgggcgaggcgctctacaccgacatcggcttcaccggcggcggcaagggcgcgggcatgatctacatgaacggcaagatcgcccataagctctccaacgacggcatggtcgaccatatcgtcgccctggtcgaggaaaaggccgccgaactgaccgccgcccgccaggccgacgtccaggacctcgcccgccaggtggcctgagggcccttaggccagcacccccgccagctgcagcccctggaacagcgacagggccagcagcaagccgccgacggcgaaggtcaggacgcgctgcggggccttttttacgatatagccggcgaagggagcggcgatcaggccccccgcgaccaggccagccaccgccgcggcgtggtcggtcagggcctcggcgtcctcccagtggccggtgaccaaggcccagacgaaggtggccgagatggcgaccgtcagaaagaactcggccgtgttgacggtgccgatggcgcggcgcggctcttctcccgccccgaccatggccgaggacacggtgggaccccacccgccgccgccgatcgcgtcgaagaagcccccgatcaggccgagcggccccgtggtccaggcgggcaggcggcgcggcttggcctttcgaaagccgcgccacaggatgtagaggccgatcagcgccagatagaccacgatgaacggcttgatgatatcgccgtcgatcccgctgagcacataggcgcccaccacgccgccgacgatcccggcgacggccagtggcagaaacagccgccattcgacgttcttgtgcagcacgtggcttccggccgaggccgccgtggtgaagacctccgcgccgtgcacgcttgctgaagcggtggccggcggcacgccgaaggccagcagcaccgaggatgaaatcacgccgtaggccatgcccagcgcgccgtcgatcgcctgcgccagcgcgccgaccagcagaaacatcagaaaggtgtccatcgcccctgtccgcgccgcatgtgaacaacgccgcagcggcaaaggcctgagccttgctgttggttgcgtggcttgtctgacatttgcgtcaccgcgccttcgcatcgacacgaggcgggcgggccgctaagcctccgcgtcttcaaggagaaccccggctttgcgtctgccccaggcccgtctcgatcaggtgctcgaccgtttccacgaggtggaggcgcgcatgggcgcggcgactgacggggccgagatcgtgcgcctgtccaaggagcacgccgagctgaagccggtggccgacgcggtggcgggcctggcccgcgcgcgcggcgagatcgaggacctgcgcgccctggccgaggatcctgagatggcggccatggccggcgacgagctgcgcgccctgaacgagcgcctgcccgagctggagcgcgaggtcgcgcttctgctggcgcctcgggacgccgacgagaacgcctccgcggtgctggaggtgcgggccggcaccggcggcgacgaggcggccctgttcgccggcgacctgttccgcatgtactcgcgctacgcctccgcgcgcggctggcgcgtcgaggtggactcggccaccgagggcgaggccggcggctacaaggaggtgatcgccacggtcaccggcgacggcgtgttcggccggttgaagttcgaaagcggcgtgcaccgcgtccagcgcgtgcccgcgaccgaggccggcggccgcatccacacctcggccgccaccgtcgccgtcctgccggaggtcgaggacgtggagatcgagatccgcgaccaggacatccgcatcgacacctatcgatcgtccggcgcgggcggccagcacgtcaacaagacggactccgccgtgcgcatcacccacctgcccaccggcatcgtggtgacgtcgtcggagaagtcccagcacgtcaaccgcgacaaggcgatgaagaacctgcgggtgcgcctgtacgacatgcagcgccaggccaaggacgcggcgcgttcggacgcccgcaagtcgcaggtcggctccggcgaccggtccgagcgcatccgcacctacaactttccgcaagggagagtgaccgaccaccgcatcggcctcacgctgcacagcctgccgcaggtgatggagggtgagatcgatccggtgctggacgcgctgatcgccgaggaccaggccgcgcgcctggccgacctggaggccgagttcggctgatcagccggtctgttcagcctcgagcgcgcgctgcaccgctgggcgcgcgctcatgcgggcgaagtgatcggccacgcgcgggaactcggcgaggtctacatcgtcgtgcccgagccagccggcgatggtgaacagataaggatcggccacggaataggcgtcgcccatcacccaaggtccttccaggccgctttcgatccgggcgaatccgtcgcgcatgttcgcggggaccttggcggacatggccgcctgcgccgcctcgtcgtcggcccagcgcgaggcgcgtcggcgatgggcgtgcgccacatggacggtggacgcgagataggcgttgaacgcctgcatactggcgaaggcgaagggctcggttggcgccagggcgccgggcgcagacagcgaggcgacgtaggccaggatcgccggcgtttcggtcagcacgcctctatctgtcgccagcgcgggcacgcgacccttcggattcaccgccaggaactcgggcgtgcgctgctcggccttgccgaaatcgatcagccgcacctcgaaggcgaggccggactcctccagcgcaatatggctggcgcggctgcatgcgcccggcgaggtgaacagggtcagcaaggtggagccctccgtaaaaacagaaagggcggcggaatgatccgccgccctacttccttacaggtccagcagaacgcgctgcggatcctccagatgttccttcagccgcaccaggaaggtcaccgcctccttgccgtcgacgatgcggtgatcgtaggagagcgccagatacatcatcggccggatcttgacctcgccgttcaccgccatcggacgctgcacgatgttgtgcatgcccaggatgccggactgcggcgcgttcaggatcggcgtcgacatcagcgagccgtaggtgccgccgttggtgatggtgaaggtgccgccctgcatctggtccatggtcagggcgccgtcgcgcgccgccttgcccaaggccgcgatgcccttctcgatgcccgccagagacagcgcatcggcgtcgcgcagcaccggcacgaccagtcccttgtcggtgccgacggcgatgccgatgtcgtagtggttcttgtagatgatgtcggtgccgtcgatctcggcgttgatggccgggatctccttcagcgcggcgaccaccgccttggtgaagaagctcatgaagccgagcttggcgccgtgacgcttttcgaaggcttccttgtactggctgcgcagcgccatcaccgccgtcatgtccacctcgttgaaggtggtcagctgggcggccgtgttctgcgactccttcaggcggcgggcgatggtctgacgcaggcgcgtcatcttcacccgctcttcgcgggggccggtctggcggggcgcggcgggagcggcggccggcgcctgagacacggcttgagccgcctggccgatggcggccagggcgtcggccttggtgatgttgccctttggaccagacgcctggatcgacttgggatcgaggttgttttcgcccaccacgcgctgcaccgccggggacagggtggcgttctgcgcgggcgcgacctgggccgagccggtgttggcggaagccgtcggctgggtcgcaggcgcgggcgcgccgccgtagccggcgttcgagctgaagccgccgatggtggcgatggcctggcccggagtaacggtggcgccctcatcgaccgagatggtcagcacgccgtcagccggagacgacacctcgaccgcgaccttgtcggtctcgatctcgaccagcagctcgtccttcttgacggtgtcgccgctcttcttggtccacttgccgatggtgccctcggcgccgctttcgcccatggtcggcaccgccaccgtcaggctctcgcccgccccgccggacgccatgggggcgtccgcccgcaccggctcgtccgccttgggagcctcggccttggcggccggagccgtcttcgccgcttgggaagccgtcgtcgctgcggcgcccgcgccgccttcggacaccacgcccagcaccgcgcccggcgtcaccgtgtcgccctcggcgaccttgatttcgcccagcacgccgtcggccggggccacgacctcgagggagaccttgtcggtctccagctcgaccagcatctcgtccttcttcaccggctcgcccgccttcttggtccacttggcgatagtggcttcggtgacggattcaccaagggtcggggtcaggatgtcggccatgtcgggtccagctgcgctctagtcgttcagtcttagggtatcaggcgaaggcttcggtggtgaaggcttccagttccttcaggtggcggctcatcaggccggcggcggtggaggccgagccggggcgcccgacgtagcgcgcgcgcttggcggcgacgtccagcttgtccagcgtcagctccagccacggatcgacaaaggtccagccgcccatgttcttgggctcttcctggcaccagaccaactcggcctgcgggaagcgcgccagttccttgcgcagcgactggatcggccacggatagaactgctcaagccgcaggatgtagacgtcgtccaccttttggccgtccttggccttcttctcgcgcgcgtcgagcaggtcgtaatagaccttgcccgagcacaggatcacgcggcggacgtccttgtccgccttgatcttgatcccggcgacgtccggacgcgtctgggcgtcgtcgtgcagcacgcggtggaaggccgagccttcggccaggtccttcaggctggacaccgccttcttgtggcgaagcaggctcttgggcgtcatcaggatcagcggcttgcggaacggccgatgcatctgccggcgcaggatgtggaaatagttcgccggcgtcgtgcagttggcgacctgcatgttgtcttcggcgcaggcctgaaggaaccgctccagccgcgccgacgagtgctccggcccctgcccctcatagccgtgcggcaacagcatggtcaggccgctcatccgcagccacttgcgctcgcccgatgagatgaactggtcgatcaccacctgggcgccgttcacgaagtcgccgaactgggcctcccacagcaccagggtgttgggatcggccagcgagtagccgtattcgaagcccagcaccgcctcttcggacagggccgaatcgatcacctcgaagtcggcctggccctcgcgcaggttgttcagcggaaaatagcgctcctccgtggtctgatcgacgatgccggagtgccgctgcgagaaggtcccccgcaccgagtcctggccggacagacggatggggaagccctcgtccaccaggctggcgaaggccagactttcggccgtggcccagtccagcccctcgcccgaggtgatcgcctcgcgccggccgtcgatgacccgcttcagcgtcttgtgcatgtcgacgctgttgggaatggtcgtcagccggtgacccaggtccttgagcgtctccatcggcacggccgtgtcgccgcgcaactcctccttgggcgcctggaagccctgccactggccgtccagccagtcggcgcgctcagccttgaaggtcttgccggcctcgaactgctcgtcgaggaaggtctcgaagcgcgacagttctgcgtccacctcggcttgtgtgatcacgccctcggccaccagccgctgggagtagatctcgcgcgtcgagggctgggcgcggatcttggcgtacatgatcggctgggtgaaggtcggatcgtcgccttcgttgtggccgaagcggcggtagcagaacatgtccaccaccacgtccttgtggaacttctgccggtactcggtcgccaccttggcggcgaacaccaccgcttccggatcgtcgccgttgacgtggaagatcggcgcctggaccatcagcgccacgtccgacggataaggcgaggagcgcgagttgcgcgggctggtggtgaagccgatctggttgttgatgacgaagtgcagggtgccgccggtgcggtagcccttcagccccatcagggcgaagcattccgccaccacgccctggccggcgaaggcggcgtcgccgtggatcaggatcggcgcgaccttggcgcggtccagcgcctgctgcgcatcgccctcgccgcgtgcggcgtcgcgcaggtcgaacgcctgcttggcgcgcgccttgcccagcaccaccggattgacgatctcgaggtgcgagggattggccgtcagcgacaggtggaccttggcgccgtcgaactcgcgattggacgaggcgcccatgtgatacttgacgtcgcccgaaccctcgatgtcgctgggcacggtcgagccgccctggaactcgtggaagatggcgcgataaggcttgcccatcacggcggccagcacgttcaagcggccgcggtgggccatgccgaatacgacctcgtcgacgcccagagcgccgccgcgcttgatcacctgctccagcgccgggaccatggcctcgccgccgtccagaccgaaccgcttggtgccgggaaagcgcttgtgcaggaagcgttcgaagccctcggcctcgatcagcttgttcaggatggccagcttgccttccttggtgaagccgttctgctcgaacttgtcggcgccctcgaaacgctgctgcagccaggacttctcctccggctccgcgatgtgcatgaactgcacgccgatgttgccgcaataggtgcgcttcagcagcgccagcacctcgcggatggtgccggtctgcagccccagcacgccgtccaggaagatcggacggtcgaggtcgcccggaccgaagccgtggaattccggcgtcaactcggggttctcgatcggctgttcgatgcccagcgggtcgagcttggcctgcaggtgaccgcgcacgcggtagctgcggatcagcatcagggcgcggatggagtcgtgggcggcggcgcgcacgtcctcggccgtgacgcccgacgccgccggagcggacggggcgctcgccggcttggcgctcttggcgtcaggcttgggcgccggccagcggccgtcgaacacggcggtctgttcagtgggctcggtcgccgtcgaacggccccaggcgcccgcttccgcattggccttcaccgaggcggcgttgtcgcgaagctggtcgaagaaggcgcgccattcgcccgagaccgaggccggatcacccgcccatttctcgtgcagttcctcgatataggcggcgtttgcgccgtaaaggaatgaggtctcggcaaagacctggttcagccgacccgcatcgtccgccatactgcttcgtgtccgtctctgaagcccttgcgcacacaaccgcgtgaagggcgcgcccgtcatataggcccgctttcctggcgggtcatgaccgaaagggggcgcccaagcgagaaattggtcgcatggacaaagaaaaacgcccccggcgcgaaccgggggcgttcatcctcagggagagaggcgaaatcagcccttcagcacgtccaccagcgtcttgcccaggcgagcgggcgacggcgagacgcggatgccggccgcctccatcgccgcgatcttggattccgcatcgcccttgccgcccgagaccaccgcgccggcgtggcccatggtgcggcccttgggcgccgtgcggcccgcgatgaagccggccatcggcttcttgcggcccttcttggcctcgtcgatcaggaactgggcggcgtcttcttcggccgagccgccgatctcgccgatcatgatgatcgactgggtctcttcgtcggcgaggaacatctccagcacgtcgatgaactcggtgcctttgaccgggtcgccgccgatgccgaccgccgtgctctggcccaggccctcgttggttgtctggaacaccgcctcataggtcagggtgcccgagcgcgagacgatgccgacgttgcccttcttgaagatggagcccggcatgatgccgatcttgcactcgtccggcgtcatgatgccggggcagttggggccgagcaggcgcgagttcgagcggtccagccgcgccttgacccgcaccatgtccagcaccggaatgccttcggtgatgcaggtgatgaaggggatctcggcgtcaatggcctcgatgatggcgtcggcggctcccgccggcggcacatagatgaccgaggcgtcggcgccggtggcttccttgccctcggcgacggaagcgaagatcggcaggctttcgccgttggcgcccgtccaggtctcgccgcccttcttggggtgcacgccgccgaccatctgcgtgccatgataggccagcgcctgttcggtgtggaagctgccggtcttgccggtcagaccctggaccaggatcttggtgttcttgttgaccagaatggacatgaggtctcgcttctcgggttaggcggagaggaaggggttttcgacccggaccgacccgtaggtctgcccatggttgaggtcttcggaatagatgacgcgggcgcgaaggcgctcagcggcggcgatgatggcgccgtcccagtaggacagctgatagcgtcgcgcgtgatcaatgcccgacaccaccacttccggcgtgatgggctggcacggcttcatggcgacgacgcggacccattctcgggcccggtccggcgtcagcggtgacgcccctttgcgagtcgcgttgttgtagaactccgccaagacctgcccagaggtgcagtaatcctccgccagcacgatctctctcgcccgctcccagcgatggccggcgtgatcccggcccagagcggcgtagagcaggacgttggtgtccaggaagacctcagaactcgcgatcaaaccgaggctccccgctataggtctcttcccggctgaaccgccagtcgcccatgcggccttcggactcgtcaatcagcttcagcagggcttcccgcgcctcgtcctttgactgctcgtcctcgaccagccgggtcaggaagccgcgcaccatttcattgacactggtccgcttcatggcggccagcacccgcaccttgtcgagcagggcgtcgtcgatggcgagggtgaggttgcgggtcacagccctcgtctacacgggttatgtggaacacacaatccgtgtgagcgaggggatcaaagccggaagttagcagacaacccgctcttggtacccggctcatcgcgaccccgtaccgcttggacatactggacatccaagacttgcgatccgttcactcgccatttgcgtgtccggaaatctacgccatggtcgatctcggaaagctggcggccgtcaactgtcaactgttcaatctgattcaagacgtcgtcgtcagcttcgtcgaagtcgatcatgcaaatcgctgtggccggggcctcgcggagcacctgcgcgccctttgatggagcccgcccagaacgaagcagcgatcgcagggcctcgccagtaggcggcgcatccacccactcactgactgcgtcgaacacctcaagccgaattgtcaccgcgcctgccgaataaacaagaacgccatcggcgtcctcgaacatcggcgcctcatcagcatgacgcgtccagccgcggatctccgcgagcgcttcaagacgtgaagcctgcccggcagtcgccagacaggcttcatagaacgtctgcacaggtccctgacccgtagattggctaaccagaagcgctgaaaacagcgccgtcagcatcagccgaccgccgcgacgatcttctgggcggcgtcgtccaggtcgtcggcggccgtgatggccaggcccgactggttcaggatggccttgcccttttcgacgttggtgccttccaggcgcaccaccagcggaaccttcaggcccacctccttcaccgcggcaaccacgccctcggcgatcacgtcgcacttcatgatgccgccgaagatgttgaccaggatgccctgcaccttgggatcagcggtgatgatcttgaaggccgccgcgaccttctccttggaggcgccgccgccgacatcgcagaagttggccggctccttgccgtacagcttgatgatgtccatggtcgccatggccagccctgcgccgttcaccatgcagccgatgttgccgtcgagcgcgacataggccaggtcccacttggaggcctcgatctccttggcgtcctcttcggtctcgtcgcgcagtgccttcatgtcgtcgtggcggaacagggcgttgccgtcaaacgagaccttggcgtccagcacgcgcaggtggccgtccgtcatgacgatcagcgggttcacctccagcagcgccatgtccttctcgacaaaggccttgtacagcgccgggaacagcgacttggcgtcctcggccgccgcgcccgacaggccgtaggcgtccgagatggtcttgacgtcggcctcggtcacgcccgcttccgggtcgatggcgacggtgatgatcttttcaggcgtgtcgtgggcgacggcctcgatgtccatgccgccctcggtcgacaccacataggagacgcggccggtcgaacgatcgaccagcagcgagcagtacagctcacggtcgatgtcggcgccgtcctcgatgtacaggcggttgacctgcttgccggcctcgcccgtctgggcggtgaccagggtgttgcccagcatctccttggcgtgggcgacgacctcttcgatcgacttggccaggcgcacgccgcccttggcgtcggcgccgagttcggtgaacttgcccttgccgcggccgcccgcgtgaatctgcgacttcaccacatagagcggacccggcagctggcgggcggcggcttccgcctcgtccgccgaggtgatggcgacgccctgcgccaccggagcgccaaagcccttgaggacctgcttggcctgatattcgtggatgttcatggggaggaaccgccgcaatcgctgctgggagaaggttgcggggcttataggcccccgttctttgcaggcgcaaccgtctggcggatcggccttagtcgacccagtcgcgcttcagcgtgcgcgaggcgccgatcagcaggacggacgccagcacatagaagcccatgccgctgtagatggcccagcgcaggctttcctcgccgaagcgcggcgccagcaggtcgctcatccagccgaagtaggaaaagccgacggccagtcccaagaggttgttgatcagcagaaacagggcggacgccgtggagcgcatgggcgcgggaaccagcgactgcaccgccgccgtcaacggacccagccacgtcaggttcagccccgtcggaatcagaaagatcagaaacgccagcaccagcgcctgagcctgagttccgccgcccggcagcagttgaccgatcagccaatgcgagttcatcgccagcacgaaacacggcgccgagatcagaaaggcgatggcgggcgtcagcggataggcgcccttgctcttgcgcgccagcctatcggccacgaccccgccgccccatatgccggccagtcccccgatcagggcgatgccggaatagtaccagctggtctgcgccaaagtcaggtcgaacgagcgcataaagaacagcggcagccagcccgcgacgccatagccgcataccgatgacgatgccgcgcccagcgccagcagccagaagctgggctttgggatcaccaccgacgccgcctgcttcgccaccctcagcgacaggccgatcaccagcagcagcccgccgccgaaagccaggaccgtccagccggccccgccggacgctgcgacgcccgccgccgccagaagaaccgcccccagcccgatcacgaccgtcgccgcgcgccgtccgacccggtccgagcccggcgggttcgttggcgcgatccgcggccgggcggtcgtctggcgctcacggcgcggctcgcgcacggtgaacaggagcagcggcgcgaccaccaggccgagcagccccaccaccacaaaggcggtgcgccagccccaggtcgccgccagcaatccaccgaccagggttccgccggccatgccgatcggtatgccgaaggcgaagcccgccagcgccctcgcccgctgctccggcggaaagtagtcggcgatcagcgcataggccggggccacgccgcccgcctcgcctccgcctacgcccatgcggcacaggaacagctggcggaagccgcccgccgctccgcacagggcggtgaagcccgaccacaccgccagcgcccccgtcatgatccacacccggctggtgcgatccgccagccacgccagcggaatggccagggtcgaatagacgctggcgaaggcgatgccgcccaacaggccgaactgggtgtcggacaggtcgaactcggccttcagcggcgcggccaggatgccgatgatctgccggtcgatgaagttcagcgcatagacgacgatcagcacgcccagcacatagaagcggtaggccgagcgcgggcgcgacgagggttcaggcatcgacatgggagcgtcccggcggcggatcagccggccgcctgttcctgcaaaagggcggcggcgggcgccgcgcagccgttcagccgcgtctcgcccatctcgaccagggccgtcagcggatacagccggtcgctcatgccgtccgaacattcggtggccatcagggtgacggtgaagggctggccttgcgccggctggacgctccaggtcgcggtggtgccctgcaccaccactccgtcgttcgcgcctcgccgctcggcctggtcgacgccggagtagaccacggcctccgtatcgatcgacacgccccagaacggctcggtccccaccgcccgcaccggctgatccaggttcaccccgccgagcaccgcaggctccgccgccggagcctcgaccgactgcggcgcttcattgtccgagcaggcggccagcgtcagggcggcggcgaggccgatcgaaaggcgaaacacggcgaactcctcctgcgctgtgcgatgtcgcatgctgcgctatagctgaatacatgtcgattcgaccggtcgcctatgagttcttcgccggcggcggcctggccgggatcggattgtccggcgatttcgacatcggtttcgccaacgacatcgacccgatcaagacggcggcgtttgccgccaaccatccgcaggtcccgctgcatcaaggcgatgtgtgggaactcgagcccgacgacctgcccggccgccccgatctgtgctgggcgtcgtcgccgtgccaggacgtgagtctggcgggcgcccggggcgggctggaagcgcgtcggtccggcgccttttggggcttctggcggctgatgcaggggctggacgcgcaaggtcgtgcgcctcgactgatcgtgctggaaaatgtggtcgggctgctcacctcgggcggcggggcggacttcgccgccgtgtgccgggcgatgaccgatctgggctatgtcgtcggcgcgctggagatggacgcggcgctgtggctgccgcaatcccggccccggctgttcgtggtcgccatgaagagcctcgagggtccggtctcggctgggccgcgcgcgcccttccactcgtcccggctggttggggcgcagcaggctctgcccgaccaagtgcggcggcgctggcgctggtggtcgctgaccccgccgccgttgcgcaatccggatctggcttcggtgctggagccggagacggactgcgcctggttcgactgggagcgcgccaacgctctgctggctctgctttcgccgctccaccgacgcaggctggatgcgatgtcggcgtcgggcgagcgccgcgtcggcgccgcctatcgccgggtccgccgcgaggcggacgggaagcggcaaaggctggagcttcgcttcgacggtctggcgggatgcctgcgtacgcccgccggcggctcctcacgccagtatgtggtggcggtcgaacagggacaggtgcgcatccgctatctgaacgcgcgggagggcgcgcgtctgatgggcctccccgacgactaccgcctgccggcgcgggaatcggccggtctgaaattggtcggcgacgcggtggccgtgcccgtggtgcgcgcgctgagcgaaggcctgctccgtcccgcgctgggagccgccgcacgcgccgcctaacgatcctcctcttcgggacgccccggatcgcaggtgttgtcgacggcgtcgtcccagccttcgcggctggagcgaaaggccagggtcatcaggccccaggttagacccagcgtgccgagaacgcccagccccagagcgatccagccgtggaccgacatggcgccgccgccgatcagcgtccagaaggcgccgagcgcccaggtcgcgccggcgctgatcgccaccgccaacgccagccggatcaggaagcgacgcgccgggccgggcaccgcctcagcccgccggccttaacgctggacccaccgcccctgggcgttgcgataccactggcccgacgagatgcgcggcaggagctggccctcgaacatgcgcgcgccggccacgtcggcggtggtcccggcttcggacgcgctgcgggcgtaggcctggcgacggccggcgttggtggcgtccaccgccgcacgcagggcggggtcgctgctggcggtgcggaagccgacatagccgtcggcctgctcgcccacgacgccctggctcttggcctgatcgatcagcgccttctgggcgccggtctgggcgagggccgcgcccgccacgcccagcgcgagaacggaagcggcgatcacaaaggtcttgcggaaggtcatttcagcctgccctttcagaaaagacggcgtcaaaacaggttcgggttgtcctggagcagctgctgcagctcccgatccaggcgaacgcgcacgtcggcgtcgagttttgcatagatctggatcggcgccacctccagcttgatggtgggggcgcaggcgacgaccccaccggtcaggagactggcgcccagaaggacgagagcgagcgggcgctgggtcatggcggcgggggctccggttcggttcggttgaggcgatctagcacggctgtgggtgaacgccgcctgaatgatcatggcgtcggcgcatccgactgtccggcgcgcgcgcggttcagcgccaggatgtccgacaccagctggttcaggttcagcgtcgtgtccagcgtcaggtcgatgcccgtgtcggacggcagcggcagctggcgcttcaggaagtcgcgcgtgatcaggtcgcgcagcgtcagccgcagctcctggcgctggggcggatcatggcggcccttgatgtggaagacgacggaggcgcgcccgccgtccaggctgttgacctcggccgtcagcatgtcgaaggccaggttctccatcgcctgatacgccaggtcctcgaccgtgcccgggggcacgtcctcgcccgccccgccggcgctgacatcgctcagcacctcccgctggatcgacaggcggcccggctgcaccgcctgcagcgtcccgccggcgatgcgcacgccggcgttgggatcggacacgaacggcaggcgccccgacaccaccgcatccagctccaccttgtcgtccagaccggcgtcggagaccacctcgcccaactgcacgcgctccagcacgatgaccccgctgaacggctgcgtcgggtcgagcgggatcgacaacggctccaccgagatcacgccgccgccggccgcgacccgcgcgccggccaccgtcacggccgtctcgtcgagcccgaaggtcagatccagatcggtgatgtccgcgcccgcatccaggctggcgacgcgcagccgctggttcggcgcggtgatcaggggcgcgaggctggtgaagtcgatctcgcccgtcagtcccttcaccggcccggccgggctggtgaagtcgaggttcgggatcaccagccggccgctgctggttccctcttccggcgtgtcggtccagccgaagcggccgtcgaagcggaccgagccggtcaccggggactgcacaaaggcgtccagcagcggcgtcagcgtctgcggctgcagcccgttctcggcgaaagtcagttccggcgcgctgatctccagcccacccgtgcgcgtcgcgccgtcatgctggaaggtcagccgaccgatcgaatgaggcccggacgccagttcgaagccgccggtccatcgctccgaccggagccgggccgatcccgtcgccgacagggggttgaaccggcgcggcgtcacggcgtcctcgacccgggccgacctcacgtccgcatcggccgacagtccggcgcgcgcgccgtcgaccgtcacgccgcccgtcgcctcctcgaaacccatgcccaggaacggcgcctggcctctgacctgtgcaaatccgccgacgacgcgccagcggccgttctgcgccgccagcagcggccgggcgtcagggcacaggttcccggccacggccgtgacgtcgttctcgcccagctccaggcgctccaaggtgaaggccgaacagccctgcggcgcataggtcaggcgtcctgcggcgttggccagccgtccgcgcgtctcaacggtcaggccccgcgcgagatcgaagtccagcgcggcgcgcgcatcgacctcggccttgaagccgttcggcgtcagccgccaggacggcacgtccgcccgcatctgcggcagtccccggccgcgcgtcgccgcaagggtcagggcgccgccgcccagccgccccggccgggcctgatagacgggcgtacgcgcgggctggaccgtcaggacgccgccgttggccggccgcagggtcgcgttctggttcaggctgaccgaaacaccggcccggcccacctgcaccgcccagcgcggaaccgacagggccaaggaccccagcgcccgcttcatctcgcgcaggtccggcaggtccttcggctccggcgcgccgaacaggggccaggcgccgtcacgggcggacaggccgcccgccgccgtcagcctcagccctccgtcctgcaccagatccaggtcgaagccggaccgcgcctgcgacagccgcaagtcgccgaagacgaagcgatccgtctcggcttcgaggcgccccgtggcctccaacgcggcaccgcgcccgccgaccgccagagcgcccgaccgggcgtcgaacccgtccatcgacacgcccgacgtggaaagacgcgccgacctcaaccgcatcgggccccgcacgctccagcgcagcggcccttcggacgcgcggcggagctcggcgtcgccttcgatgcggatgtcggcgccccgcgcctgaagcgccgtcccgccgatctcgtccgcagtcagcgtcgtggtcgtgcggcccgccaggcgaaaggcctcaagccagccgctggtcgcgccgtcgaagcgggtccgcacggccgcctcggtcatgcgcgtcccgccgaccgacattcgatccgcctccagcgccgcctcaatcaccgcgcggccgtcgcccttgcggcccttcaggtcgggatagggcaggtcgccggagaagctgaggcgcgcgccgtcgcccccggccccatcggcgccgaacccggccgccgcagcgttcagcctcaaggcgatccggtccccgcgcgtggtcaggtcgatgtcgccggacaggccgcgggcctccgtcgatccgcttttcagcgccgccgccggcatgcgagcgaccagccgcatcagcttgccgtcctccattcgggcgtcgccgcgcgcctcgaccgggccgtattcggtatcgagcctcagccgtccctgttcgacgatcaccagcggggcgcgcgaatccgggcgcggcggccggccggtgaagcgctccaccaggggatccagcgatccgagcgacagctcgccttcgcgccagctcgcccgcaccactggccgcaacaggcgaatgcggctgggcgtgacgccaagaccttcgcgcgaccagggcgcgccgacggcgtagtcgacctccacccgctcgaccaccacgtcggggtcgcggggatcgccgatgcggatgcgaccgacaaagccgtccagctcgatcctctccacctcgacttcggcgggcacgccctgacgttccagccatccgaccagcacctcgcgcgcggcgatccggcggttcagataggccagcgccagcagcacaagcagaaccgccgccgccgtggcgatcgcggtcagcgcgcgcgggggcgggggcgtcgggcggctgggtcgccggcgtctcggtcaacacgcggcctttctcaggggcgacaggtcttcggcgtcgtcgtgacggcttggagctcacgacagggactctgtcgctaggacgtaacggtttgcaaagcgttgccgccaagcgcggcgacatcgggcgcccggcggagctccgccccgaaccgcttcccgaccgggctcgtctcgagtgaagaccggcgtcttaaccctttgtaacgatctgcttcccaaagtgagacaggcgcgatataggacgcgtctcgcgctcggggcctgagttgagcgcgtccttgatagtgaccgattgggcgccgcgcggcgtcgcaaaccgacggggaccgatggctcagttcgacccacgccgccagccgacgcgcctcgcgccgcatctgctcaccacagccgccgcggtcaccgtggccttgctggcgggacgggcttatgaacccgccaaggccgaagaagttccggtcgtcacggccgcccagatggacagcctggaggcccaggccttcgccgccgccggtgcgccgcagggcctgaccgctccggaagccgtccccgtccagatccgtcgcggcgaaagcttcgaggacgccgtgcgccgcaccggcgtcacctccgaggaagccagcgccgtcgccgccaccgtggccggcgcctttgacctcgccgatctgcgcgccggcctgaagttcgagaccgccatcgccaagccgcgcgacggccgcggcgacgcccgcctgatcggcctgaccatgcgcacgggccccgccagccagctgacggtgtcgcgcagcttcgacggcgccctgcgcctgcgctcgcttgaggaaaaggtcgctcacgagacggtggtgctgaagggcgacgtggagcgttcgctgtcctccagcgcccgggagctgggcgccacgtccagcatcgtgcgcgccgccagccgcctgttcgccaccaagttcgacatgcagcgcgacatccgcgcctccgacgaattcaccctggtgttcgaccgcgagatcaccgaggccggccgcgtggtcgcggccggcgacctgctctacgccgaactgcgcggccgcaccttttaccgcttccagccggccggcgcgaaggaagcccagttcttcgacgccgagggcaagaacctgcgctcggccatgatgcgcacgccgctgcagagcttccgccgcgtgtcgtccaacttcggtttccgcactcatccgatctccggctacaagaagatgcaccagggcatcgatttcgcggccgggaccggcacgccgatcgtggcgccggccgacggcgtggtggtcgaggcccgccgctggggcggctacggcaactggctgcgcattcgccacgccaatggtctggaaagcggctacggtcacctgtcgcgctacggctcgggcatccgcgccggccagcgcgtcagccagggccaggtcgtcgcctatgtgggctccaccggcgcctccaccggcccgcacctgcactatgagctgtggcgcaacggccaacggatcaatccggcgggcgtgaagacgcaggaaggctccgaactgtcgggcgccgatctcgccgcgttccgcgccgaaaagtctcgcatcgaccgcatcatcgccgccggcggccagaagcgtccggcgctgcagcaggcctcggccgacggcctgcgcgccgcccgcggctgagacccaggtccttcatccgaccagcaccggcggcgccgcgccgccgcgcgggcaggacacgccggggaccgtcacgtccgcctctccgagatgcagacccaagagcgccagcacgctgttcagcacgccgtcgagcacgggccccagcggcgtcagcagcagcccgaccgcctggctgatcgcgcccatttacccccaggcctagcgccgtcacctccaggtccagccgctgaagcaggctggtcacagccccgctggcgaaggcgcgcgactgaaccgtgcgcacgcgctgccgggcgatgtcggcggcggagaaggtcgtgggttgaaagccggcgtccgccgccgtcacctccgcgcgccccttgaccgtggcgatgccggccagcgacgccagctgggtcgatcggctcgacaggggcgcggagaagtcgcgcagggcccttgcgtccgcccggcccaccatcacccgcgccacgcccggccgcacgtccagccgcacctcggcatcgggcgtgcagcggatatccgccagccgcgcctcggacggcgccgcctcgatgatcagcggcagttccacccgaccgagcagcgccaaggcctggctggtcgtcgccaccacggacagccggacctgcgccgtgcggatcgtcggctcgcccctgtcgctgaccgtgagccatgggctgttcaccggccgttcgcctatggccagcatgacgcgaatgtccgcaaggccggacgggaccgccagatccagcgccgcctgccgctcgccgccgccgatctccagcatggccatggcgaggtccagggccgagacctgcgcgctcgccgcgcctttcagaccgtgcggcgcggaggcgtccacaccgatcaggtcgccggctttcaaccgcatgccgcccgccgccgtggccagacggttcagcgccgaagcggcccccggcggcgtcatcgccgccagccggcgcagcaccgggcccgcctcgatctcggcgtcggcgagccgggcgtagtcgccgacccgcagatccgcctcggtcgccagcgcgtccaaggcgtccggcaggctgatccgcgcctccgccagcgagcggtagtccgccgccgacagcgacaccttggcgccggtaagcgcgtgcagcagctggttggcgaaaccgccgtccagccgcgccagacgcgagccgatggaaaaggcggcggtttcccgatgcggcctcgcggccgtggcctgacggctcagcatcacgctgtcccgccccaggatcacccgtccgaaatgcagggacgccggccccgagagccgcacccgcgcggcgttgggcgagcccgccccggcgcgaaagcgctggcgcggaggggttcggggatcgggatcataggcgccggtggtcgtctccaccgcatgggcgtcgcgcaggggtcccgaaagattgtcgcgcgccgtggccgccgccgccgccgccgcgcggtccaggtcccgcgccgccgacagggccgccagatccgcggcggactgcaaccggcgtccctccatctccagaaaggccaggtcgaccaccatcgctgcgagaaggctcagcagggccagccccgccgcccccatcatccccaccccgccgccttggtccgccagccaggacccgccgcgcccgctccgccgcctcactcagtagccgcccacgcgcaccaccgcgcgtcgctcgatccgccgcgacggtcccggcaccaggttcatcagctgcaggatcgggtgctcgctggcgtcatagaccagcaccacctccacgcgctggtcgtcgctgatgatgcgggtgctgaggtgatcggcgtccagcacccgggaggcgtgggataatccttcttgcacctcgctctgcgccagaagcctacgctcctcgtggtccagtcccgccaccgccgcccgcgcggcttcggacgccaccgactgcacggactgcgccagccacagccaaccgccgtagaccaccacccccgccagaagcagcacgaacaagggtccgatcagcgcgaactccaccgccgccgccccgccgtcgtccgccagacttctcttccaaatcctgacgcgcatgaccttctccccgcaccacctgtggttgtgcatggaagatcgttaaacaccggtttgcacgcagccgtttcgccgagcctcggccggacagcacacgacaccctgcgcctctcagcccgtgctaactctggttgtgtggagaatgtgggcgcgtcagggatcgacggcgtgttggccgacgcctgaacgagggttggatcgcggggcccagccgaattgcgagcgtcaaagaggaacgcccatgaggcctggccatgcgtccgccttcaccatcaggcaggagagcgcatcccttaggcgtcacggagtcgaggatcacccatcgtaaggagcgtcttcgaggacgtcgctttgcaccatgtcactcagagataatgtctcggcggacgacgctggcgcttagctgttgaacagctgcggtgctcgaaagcttgcggcggtgctcacaggtacttgagccaggcccgttggctgttgcgcttgacgcctgcgaaccagcggcatgcaaaccagcagggaacggccaggatcgccgcaacaagccagagccatcccactgcgggcacgccgaatgtgtcgccccgattggccccaagcagcgaaagcgcggcgaggtggagcaggtgcagagcgtacaggtggatcagatagaagaacaagggagcgccgccgaagaccgccagcaggcgcaccacacgcacggaggtccgctccagcgccgcaaggaccagcacgcccacgcctagggtcagcaagaggaaatctgctgagggcggatacttggtcaggttcaggtaactcatcgccgagcgaagcgcgtccggctggacggaccagggcgtcggatcgccgtagaggttgacgcagcgcagaaccacaaacatcccgagcatgatggcgcctgcggtcagcagccgccgccgacgcgacgcggcttcgcccgcgaaccaggggccgaccgcgtaacccagcgccgccacgccgatccacggcagcagcgggtacgaggtgcgcgcctgcccgccccatggcaggtcgatgaagcctcgatcgtgcaggatggcccatagggtgtgaccaggctgaccctcgacgaagttgatcggatcaagaaggttgtggcccagcacgatgatcacgccgacagcgatcagccagccgcggggcagatgcacaagcgccgccagcgcaatcatcgacaggccgatcacccagatcacctgcaggaacacggtcggcggcgtcagcgagaacgtccaggcgaagttgaccgccgtcaactccagcaggaccaggaacaggccgcgcttgaacagaaagccggaagctgcagccgcgccgcccttcttcgatccgtaaagccaggcgccgagccccgtcagcgccacgaacaccggcgcgcacaggtgcgccgccaagcgcgtgaagaacaaggccggcgcggtcgtgcccacgtccatggggtccgagacctgggcgtggatgaagaagaactcccgcgtgtgatcgaccagcatcagcaggatgaccagaccccgcagcgcatctatggactggatgcgtggggcgagcgttttagcgcctggagcggaacaggggtcggcggcgacaagcgtggcgggtgttgacatcatcacgaccgagcgactagccgatacaggataacatttcaacggagcctccccttgttcctcctgtcgagctgcgctggcctgtgcctgctgaccgccgccgcgccttcggcggcggtccagccgcagggcgggcgaccccaggcgcaggcccttgatgagatcgtggtgctgggccgacgcgcggggcggagggatgggaccttgggagcaggagcggtgacggagcggatgtcgccgtccagccgctcgatcgaagcggatttgctgcaggcggtgggcgccacgcgccttgtggatgcgctggagctggtcagcggcgtcagtcagcagaacaaccgcggcggggtcatggacaacttcgccattcgcggctttctgggcacgccggacggcggggccgagtactacgtcgacggctttctggcgaaccggggcatggcgccgccgagagacccagccacggctgaacggatcgagattctgaaaggaccggccggcgccttgttcggcgacatcgatcccgccggtcgcgtcaacatcgtgtccaagacgccgcgcttttccaatgaagccggtctgacgctgacggcgggatcgttcgaactggcccgcgccgagcttgatctgacaggggcgctgaacgacgtcttggccgggcgggtcgccgcggccgtggaaaccagcgatggctggcgcgaccatgtggggctgagacggatcgcccttgcgccgtcgctgacctggcgtcccagcgatgacctgcgcctgacctatgtgggcgagttcacgaccttcgacaccttgttcgaccgcggtcttccggccgtggacggcgacgccctggccttgccgcgcttcagctacttcggagagccgaacgacggcgtgacccgattcatcaacgaacgacaccaggtcacgggcgaataccgcatcaccgacgactggagcctcaacggcggcctcgcctggcgcggcggcacgctgaaaggctactccagcgatcactcgcgactggtcggcgacaccctgtggcgccagcgccggggccgcgacttcactgtcgaggatctgtccgggcgtctggagttgaacggtcgggtgcaggcgggtgcaagcctccaccggctcggcttcggtgtgaaggcctatacgttggagtatggcgagcgctggctgcggatcaatccaacggccgaacggccctacggcattgacatctataatccggtgtacggctccccggcgccggatccgctgccgttcaccgacaatctggaagggcgcaaggtcgtcactctatacgctcaggatctgtgggaggcgacgggccgcctcagcctgctcgccggcgtccgctacgacgacttcagccagacgatccgaaacaaccggaccgaggccgtcggagaggccgctgacaaccccgtcaactatcgcttcagcgcacgttaccgtctgacggagaccgtaggcgtccacgccagctacggcgaatcgttcgtgctcaattcaggcacgggccgcagcggaggcggcttcgcacccgaaacaggctccgggtacgaagtcgggatcaagggcgcttggccgggcgtcgacatcgctgcgacgctgttcgagatcgagaagagcaacatcctgaccaccgatccagtggatgcgaactacctggcgccggtcggcaagctgatcagtcggggcgtcgagttcgacgcctcggtgcgagtcagcgagacgtggcgggtcgtcgccaactacgccttcaccgaggcaaaggcagacgacaccgcctttgcgaccgacgccgtgctgaacgtgcccgatcactccggttcgatgtacgccatgggccggttcacgacgcctgccggccgggactggtcgctcaccgccggcgcggcctacaccggagatcgcgtcgcgggcctggacggaagcggcgttcagcttcccgcctactggaaggtcaaggccgcggtcgattacaccctgacggatcgcgtggccgtgcggctcgaggcggacaacctgttggacgagcactacgccgccagctcctatagccgcctgtggatcttccccggagcgccccgctctctgcgcgcttcgatacaattcaccctgtgacatagaacaagatgaccacacgaccgggccgggcgggatcgaccgagcccgcacacggcctggctgccgcaagaggcggaacgccttgcccatcgcctcgctccctgcggttgcgccgagagaatcaacgtcgagctgtggctggctgggaactccgcgcgtccgtcagagggcgcgccggagcaacggctggccagagccgagcgcgtgagtggagcagcgctgctcgtggacaaggaggcgctgttgagagccagcacggtgaacatgcttgcaacctcgcgcactgactacatcagccgcgaccgataggttcgagcaacggactttagctggtggctggtcagcacttccagcgcccgtcgagctaagcgcttgaaagaatggtggacgcgacagggattgaacctgtgacccctacgatgtcaacgctgacatctatagcgaattcaatgacttccagttctccgcaccagaaaaagacaaacgaaaacagcccgctcgcccagggtattatgggcgtttcttgggcaggacgtttcttaccggccgaactggagccccctccactagcctgttgttagtggggcatttctgcgccttcagcacaaggctgacgtgaagttgccggtcagtgcttccccgccccggtgcaacatccgttaaagatgtgacaacgcaaccttattgcgctaaggacccccatccaaggcgcggcggcgccgtctcgagcgcctttgtctatgtgcggcatcatcggcatcaccggcgaaggtcaggtcgttccgcgcctgctcgacagcctgaagcggctggaataccggggctatgactctgcgggcgtcgccgccgtggtcgatggtcgcatcgagcgccgccgcgccaagggcaagatccgcgcgctggaagaggtgctggcggacgagccgctgaaggccaccgtcgggatcggccacacccgttgggcgacgcacggcgcgccgaacgtgcccaacgcccacccgcaccgggccgggcgcgtgacgctggttcacaacggcatcatcgagaacttcgccgagctgaaggctggactgacggctcagggccatgtgttcgaaagccagaccgacaccgaggtggtggcccatctggtggatcagaccttgtctgaaggcgcggcgccgctcgtcgccttcaaggcgacgctggaccgactgaccggcgcctatgcgctggcggtgctgatcgagggtgaggatggcctgattttgggcgcccggcgcggcagccctctggtggtcggctggggcgagggcgagatgtacctgggctccgacgccctggcggtcgggcccttcacccagaagatctcctatctggaggagggcgattatgtcgccgtcgaccgttctggcgcgcgcatgttcgatgcgagcggcgccgccgtcgaacgcgcgatcgtccaggtctcggcttcctcggccatggtcgagaagggcgagtaccgccacttcatggaaaaggaaatccatgagcagcccgacagcgttcagcacaccctgtcggagtacctcgacctcgtgaccggcaaggccaagacgccggcggtggacttcgccgccatcgaccgcatccagatcatcgcctgcggcaccgccttctacgccggccagatcggccgctatgcgttcgagcgcatcgccggactgccgtgcgacgtcgagatcgcgtcggagttccgctaccgctcgccggcgctgtcgcagagcgccctggccgtcgccgtcagccagtcgggcgagaccgccgacaccctggccagcctgacgtggtgcaagcgcgaggggctgaagaccgcggcggtggtcaatgtccactcgtcctccatggcgcgtgaggccgacgtgctgtggccgacgcatgcggggccggagatcggcgtggcctccaccaaggccttcgccctcacaagaagtgccaatgcctacgccgacctatatgcgaggcatatatcggagattaggtggtctgacgttgcgttcttccacgccagacgagcgctttcctctgtccaccgggcctgccgccgtcgggcagcatgaaagtgctggacgagtcgtagctgtgggctctcaagcaatggagcatatatgcacctcgcgatttacttcaccacgctcggaggcgggggtaccgagcgggttctagtgcggctggcggatgaattcgttcgtcggggacaccgcgtcgatttcgttctcatgcggcttggcgatgcggcttatacacgcgggattcatcctggagtgcactttgtagacctcgccgccacgaagctcagcgcgagcttgcctgccctttggcggtatctgaggcgtgagcgtcccgatgtggtgatttccgctggtgatatggctaatggcttctctggttgggcaggcagtctgctccatccgaagccggtgctgatcttcacccatcaccacggcgcagctacgatcttcggcaatctcgcgggtcgaaggtgcgggctgctaacctggctcttgcgccaatcacaccgtttggccgacgctgttgtgggcgttagtgagggcgtcgcctgcaacatccggcgcatgccgagcttttcgccccagcaggtctactgtatatataacccctcctggcatccgtcgattgaagaagaggcgcgtaagcttcctcggtgtgcatggcttgaacgatccagcacgcctgtgattctcggcgtgggtcgacttgaacaagagaaggacttctcaaccctgctcagggcgttcgcccttttgcgcgcgcgccgggaggcgcgcctactcatcgtcggagaaggatcggaacgccggaggttggagaacctcgtcaccgagctccgcttggatgaagatgtttaccttcccggttggacggataatcccttctctctcatggcgagcgcctccgtcttcgctctctcttccgcgcatgaagggctgcccaccgtgctgatcgaggcgatggcatgtggcacccctgtcgtcagcaccgattgccccccctccggccccagtgagatccttgacggcggtcggtttggctcgctggtgcccgttggagaccagaaggcgctggcggtcgctatagaagaacaacttgacgatccgactgctgccgatgtgctgcgcgcacgcgctcgtgagttctctgcagaggcgtcggccacagcatatttgaacctcgccgaaacgcttctcggtcgcaagacaagacgatcatgaagttaggctcaggactcatagccagaagagcacggtagcggcgagggctatggcggacaggaagacgttcgggcatcggtcgtagcgggtggcgacgcgccgccagtctttcagacgaccgaacatgatctcgatgcggtttcgccgcttgtagcgacgcttgtcataccggatgggctcagtgcgggttttgcggcctgggatgcagggcgtgatccccttggcctgcaaggcgtccctgaaccagtccgcgtcatagcccctgtcgcccaacagccattgcgccttgggcaggctgtccagcagggctgcagcgccggtgtaatcgctgacctggcccgccgtcacgaacaggctgatcggacgcccattcgcatcggtcacggcatgaagcttggtgttcatgccgcctttcgtgcgaccgatcagtcgcccgaggcccccttttttacccgcaggctcgaagccgtgcggtgcgccttcagataggtcgcgtcgatcatgacggtgcgacgttcggtctgagcgccagacaggccctccatcatccgaacgaacacgccagcttcgctccaccgcttccagcgcttgtagagggtcttgtgcgggccataagccgctggcgcgtcacgccagcgaagcccgttgcggttgacgaagatgatcccgctcaacacccggcgatcgtcaaccctgggcctgccgtggctcttgggaaagtgcggccggagccgctccatctgctcgtccgtcagccaatataggtcactcatatccagactcctcgggagcctgaatcagatccagcgcctcacatcaatgggtcctgagcctaggcagcatggattaagttagccgtatgtgtgtgacgatagggatcccggtcctcaacgctgaactttatctcgtcgatgcattgcgttccgtcttcgcgcaaacgcacgaggattgggagttgatattggttgatgatggatcgacggaccgatcggtggacatcatgcgggccgtcacggacccccgggtgaggggggtgtacgatggcaaacgacgagggctccctgcgcgattgaaccagatccacggtatggcaaaacgaccattcattgcgcggatggacgcggacgatctcatggcacctgatcggctggagcgtcagctagtttacctgaaagagcgccgggatctggatctgatatcaacaggcatctactcagtcgataacgatctcaatgtggttggtgtccgaggtaggatgagcgccgatttcacagtgcacgaccttctgttcggacgaaagggagttgttcatcccgccgtgatggcgaggactgagtggttcgtgagaaataggtaccgggaggatatcaaggggttcgaagatctcgaactttgggcccgcgcgatcacccggggggacttccgcgcggagacgctggaggagccattgctcgcctatcgagagcaaggaaacatcacgcccgagaagatgttgcgtgcctacgcaggggagagaggggtcatggcgcagttcctgccggatcgggcggagcggtgggcgtatatcgggcgctcgtggctaaaaactgcaagggctaagattatgagctcccgccgtattcatgaaagcagaaaccgcgtgctgctgtcagcagctgaacggaacgggtacgcccgcttgatcgaacaggtgaaggcgacgcgtgtaccggggctttgattgcggcaatggcgatgaatggctcacggtatcgaactcaagggacgggatcacgattatcagcgatacgccgcagtgtggtcccgcgcgggaacaactgttcagccgcagatcgtctgcctctcgccggagtcgaacggtcgcttgtcgcaccggcttgggtggtcccgcagggcccgactgccgcatgcttctccatcgagcgcatggtggacaactatcgctcaatctggtttggcgatgaggagctgcgcgcccatcgcgcgcagggccggagctagcgtgcatattcttctgactggcggggccggctacatcggttcgcatgtcctggtctgctgtctgcaggctggacatgaggtgacggttctggacgacttctccaacagttcgccggaggcgctggcgcgtgtgcaggccctcaccgggtgtacggtaaaagtgcaacgcggcgacgttcgtgataccgcactgcttggccgcatttttcgggatagttccatcgaggcggtgatgcatttcgccgggctcaaggccgtgggcgagagcgtgcagcagccgctccgctactatgacgtaaacgtcggcggcagcatcgctctgggtcaggccatggcggaggcgggcgtgttccggcttgtcttcagctcgaccgcttcggtttatggcgatcagacgcagatgccgctcgacgagagcagtcctcttgggcgaccggccagcccctatggccgctccaagctgatggtggagcaggccctgtctgatctgtgcttgtcagatccgcgttggtcggtggcggtgctgcgctacttcaatcccgtcggggcgcatcccagcggccgtatcggcgaggacccgcaaggagagcctgcgaacctcgtgccgtacctcatgcaggttgcagtgggccagcggaaggagctgtcggtctttggcggcgactatccaacgacagacggcacgggcgtgcgcgattacatccatgtcatggatctggcgcaggggcatctggccgcgatggagcgcgtctcgagagtctcgggcttcgatgtgctgaacctggggaccggtcgaggccactcggttctggaggtcatcaaagccttcgaacgagtcagcggacagcagctgccctatcgtgtggtggaccgccgtcccggagacacggctcaatgctgggccgacccggcgcgggcggagcagagcctcgggtggcgcgctcaacgcggcctcgacgaaatgcttgcggatcactggcgatggcaggcggcaaatccgcagggctataggaacaccttagtatgaggatcgctgttgtttcgcagcacgccggatccctgagtacctttcgcggtccgcttctttctgagttggtccggcggggtcatgaagtccttacttttgcaccgaactttgatgaagagtcttgagcggcgatgatcaggttcggcacccagccgatcgactggcccctgtcacgcaccggcatgaacccgctccaggaccttagctccgttgacgtgatggtgtggacgacctccgcctgacgggctgttctgggtgtgtcgtcatcagggacgtcacgtctaggctcaggacccattgatgtgaggcgcgcgatctgattcaggctcctgaggagtctgattatgagtgacctgtactggctgacggacgagcagatggctcgactggagccctatttccccaagagccatggcaggccccgcgtggatgatcggcgggtgttgagcgggatcatcttcgtcaaccgtaacggcctgcgctggcgggatgcaccggcggcctacggcccgcacaagacgctctacaatcgctggaagcggtggagcgaagccggcgtgttcgttcggttgatggagggcctgtctggcgctcagaccgaacgtcgcaccgtcatgatcgacgcgacctatctgaaggcgcaccgcacagcttcgagcctgcgggtaaaaaagggggcctcgggcgactgatcggtcgcacgaaaggcggcatgaacaccaagcttcatgccgtgaccgatgcgaacgggcgtccgatcagcctgttcatgacggcgggccaggtcagcgattacaccggcgctgctgctctgctggacagcctgcccaaggcgcaatggctgctgggcgacaggggctatgacgcggactggttcagggacgccttgcaggccaggggcatcacgccctgcatcccgggccgcaaaacccgaaccgagcccattcgctacgacaagcgccgctacaaacggcgtaatcgcatagagatcatgttcggcaggctgaaggactggcggcgcgtcgccacccgctatgaccgatgcccgacggtcttcctctccgccatagccctcgccgccgtcgtgctcttctggctatgagtcctgagcctaagtcgcgatctcccgcgacgatgcggaagtcgaactcgtcgcctagctgatcgaccatgttggcgatcgagcggattggcccgcccgccttgtagcccggcaggtaatgtcccgcgaaggagagaatgatcgggcggggcatcaggcgtccgagtcttcaagtgagttcacacaggccaagaatcgatctgccattacctgcgtattataaagcttatgagccatgatgtatgatgaagcggacatctcattgagtagctgctcatcatctactatccccgctatcgcgagcgctaaagaagccggatttccttcttggaaggcgagcccgttctttccgtcttggaatgcagcgatctcaggcatgtggtgctgacggttgtcgtgcacgacggcgggcaatccataggccatgccatgaagcaagctcaatcctacagagccagggtagatgaacatacggcagcgattagcgacggcagcgatgctcgcctcttcgatcgtccctgcgtgccaggtgatgcgttcgtcgacgctcagctcccgcgccagctgctgcagcctcccccgtttcggtccgtccccgattatgtgaagatgaaagttgacgagagcaggctctgccaaggccgtgattagcagcgccacacagctcttgtccgttaatcgcccaataaataaaccggtacgatctcgctcacgagcgttgtacctgactagcgcctcacttatgaaggttgtgtctagaccgttattcagcgcggatatgattcgacggtctcgacggccgacgccgttacgataatgctcaacctcgtcgtccgtgtaaaacagtactgcatcagccagtttcatcagccatatccgcagaaaaaggcggtgcttcctggtggtgctgcttcgatactgaccccaccatatcgtctttgcgcgaagcgcctttgccttcagcagaagggcgacgttagacaaacacctaggtccgccagatacgacgactatgtcacctcgccgaacgtgcacagatagtgcccccacctgccactcaactcctgcaatgggacggaggatcgggccgattatccgggcccatcttgcgcccgaggccttgcctgtcagaacccccatgctctcaggagaatggtagaccacaaatggatcgcctagcgcagctgcaactcgatcaaagaagtcgacccggtagtgggggagcgctggctgaaccgcgataatgcggcgttcggagaaatcgaatccagacacagacaaacccctattcagactgcagtcgggatatcgatcagatcagtaaaggtaatcggaacgtccctcacaccagatacacgcaataatcaagacgtgtgataatgatccatgcccctgtgaggtgaaggaccaaccgagcgtcggctggatgttacaccaggcaacatcgagactttcaacataacagccatcaaatcctgtcgtattaaagaacgacccgaatggaaagccgggctcaagcaaggatatcaccaaaccagcagcgatagctccgccaacaccgacagcccctctgtgcctcactccttcgcgagataccaggatcaccagacgatacaaaagggctaaggacggcaacagcccgatcattccacttgctgcggccgcagcgatccaggcattgtgaacggccagtcgcccatgcaatctggactccagcagaccgactccatggatcgggctgtcgaggaaggatacgactccatgcctccaagtctcgtaccgatcagatgtaattcttgctaggctcaggactcatagccagaagagcacggtagcggcgagggctatggcggacaggaagacgttcgggcatcggtcgtagcgggtggcgacgcgccgccagtctttcagacgaccgaacatgatctcgatgcggtttcggcgcttgtagcgacgcttgtcataccggatgggctcagtgcgggttttgcggcctgggatgcagggcgtgatccccttggcctgcaaggcgtccctgaaccagtccgcgtcatagcccctgtcgcccaacagccattgcgccttgggcaggctgtccagcagggctgcagcgccggtgtaatcgctgacctggcccgccgtcacgaacaggctgatcggacgcccattcgcatcggtcacggcatgaagcttggtgttcatgccgcctttcgtgcgaccgatcagtcgcccgaggcccccttttttacccgcaggctcgaagccgtgcggtgcgccttcagataggtcgcgtcgatcatgacggtgcgacgttcggtctgagcgccagacaggccctccatcatccgaacgaacacgccagcttcgctccaccgcttccagcgattgtagagggtcttgtgcgggccataagccgctggcgcgtcacgccagcgaagcccgttgcggttgacgaagatgatcccgctcaacacccggcgatcgtcaaccctgggcctgccgtggctcttgggaaagtgcggccggagccgctccatctgctcgtccgtcagccaatataggtcactcatatccagactcctcgggagcctgaatcagatccagcgcctcacatcaatgggtcctgagcctagcctgttgttagtggggcatttctgcgccttcagcacaaggctgacgtgaagttgccggtcagtgcttccccgccccggtgcaacatccgttaaagatgtgacaacgcaaccttatggcgctaaggacccccatccaaggcgcggcggcgccgtctcgagcgcctttgtctatgtgcggcatcatcggcatcaccggcgaaggtcaggtcgttccgcgcctgctcgacagcctgaagcggctggaataccggggctatgactctgcgggcgtcgccgccgtggtcgatggtcgcatcgagcgccgccgcgccaagggcaagatccgcgcgctggaagaggtgctggcggacgagccgctgaaggccaccgtcgggatcggccacacccgttgggcgacgcacggcgcgccgaacgtgcccaacgcccacccgcaccgggccgggcgcgtgacgctggttcacaacggcatcatcgagaacttcgccgagctgaaggctggactgacggctcagggccatgtgttcgaaagccagaccgacaccgaggtggtggcccatctggtggatcagaccttgtctgaaggcgcggcgccgctcgtcgccttcaaggcgacgctggaccgactgaccggcgcctatgcgctggcggtgctgatcgagggtgaggatggcctgattttgggcgcccggcgcggcagccctctggtggtcggctggggcgagggcgagatgtacctgggctccgacgccctggcggtcgggcccttcacccagaagatctcctatctggaggagggcgattatgtcgccgtcgaccgttctggcgcgcgcatgttcgatgcgagcggcgccgccgtcgaacgcgcgatcgtccaggtctcggcttcctcggccatggtcgagaagggcgagtaccgccacttcatggaaaaggaaatccatgagcagcccgacagcgttcagcacaccctgtcggagtacctcgacctcgtgaccggcacggccaagacgccggcggcggacttccccgccctcgaccgcatccagatcatcgcctgcggccccgccttctacgccggcccgatcggccgctatgcgttcgagcgcctcgccggactgccgtgcgacgtcgagatcgcgtcggagttccgctaccgctcgccggcgctgtcgcagagcgccctggccgtcgccgtcagccagtcgggcgagaccgccgacaccctggccagcctgacgtggtgcaagcgcgaggggctgaagaccgcggcggtggtcaatgtccactcgtcatcgatggcgcgagaagccggggtgctgtggccgacacatgcgggacccgagatcggcgtggcctccaccaaggccttcaccgcccaggtcgcggcgctgttggcgctggcggtcgcggcgggcgtggctcggggccgcatcgacgccgccgaggaggccgagctggtcaaggccctgttcgaaagcccgcgcctgatcgccgaatgcgccgagcatcacgccgacatcgaagctgtcgcccacgacctggccaaggccagagacgtgctgttcctgggtcgcggcgccatgttcccgctggccatggaaggcgcgctgaagctgaaggagatcagctacatccacgccgagggctacgccgccggcgagctgaagcacggccccatcgccctgatcgacgaggaaacgccgacggtagcgctcgcgccgctggacgacgtgttcgaaaaaaccgcctccaatcttcaggaagtctccgcccgcggcggtcccgtgatcatgatcgccccggagaccgcccccgctccgcacggcgccgacatccgccgcatccacgcccccgactgccaccccctgatcgcgcccctggtctacgccgtcccggtccagttgctggcctactacaccgccatccacaagggcacggacgtggaccagccccgcaacctggcgaagtcggtgacggtggagtgaccatgctggaggttcgctgaatgccgcaccgtttcaaagcgccggcgcggttcggagtcaccgacgccacgaagttcgccctgcatgtgggcgtgctgtttgtcgcgtttctcgcggcctatgaaatccggcgcgccctgccgctggagtggtggctgacgcaaagcgatgcgatccgggtcctgggctgggcggcgctgtatgccgggataggcggtgcggtcgaactcgtcgccaagactgaacggtccgcctggcgctatacgtctctgggcgagctgctggccctggcgcgcagccttgtcgcggccatggctctgttcctggtactcgtgttcgcccttgatcggggtctgcaactgccgcgctcggttctagttctcgcccttctgttcagcctgctgggactggcgggcttgcggctgtgctggcgcctggctcacgatcctcacctgcttcgtcgatcggtcgcaggcggcctcaaggccggagagctccacgccgctcgcaacacgcccctgctcgtagtgggagacatgaaggccgcagacgcgcatctgcgccacctcctggccgatgcccggtcgccgcaccagccggtcgggatcatcacgcccaacgggggcgaggtcggcctgcgtcttcatggcgtgccggtgctgggcatggtcggcgagtggcgcctgcccgagacggcggatgggccgcgttacgccatccttttcctcgacgatccggttcaggcctggaacgtcagtccggcgcgcatcggcgaggtgcgcaaggcgggccatacgctgcttcggccgcggatgctggtggacctggcggcggcggatggggatccccagacgctcaaggaaattccgttggaggagttcctgccgcgcagcccggttcggctcgaccccgcgcgcgttcgccagcttgtgcagggcaagcgcgtgctggtgaccggcgcgggcggcagcatcggctccgaaatctgccgccaagtcgcggctttcgactgcggtcatctggcgctgctggatcactccgagttcggcctgttcaagatcgaccaggagatcggtcaagcctatccccacctgtcgcgccgcgagatcatctgcgacgtgcgcgaccgccgccgcgtcgcggcctgggtgtcgcaagaagcgccggacatcatctttcacgccgcggcgctgaagcatgtgcccatcgtcgagcatcacccggccgagggcgtgctgaccaatgtggtcggcacctggaatgtcgccgaggcggcgcgagaggcgcgcgtgccgcagatggtgatgatctccaccgacaaggcggtcgatcccgccaacgtcatgggcgccaccaagcggctggccgaggccgtggtccgggggctgcacgacccagcgggcgacaccgcctttagcgtggttcggttcggcaatgtgctgggatcggccggatcggtggcgccgatctttcaggaccagatccggcgcggcggcccggtgaccgtcacccacccggacgtcgagcgctatttcatgaccatcccggaggcggtgcagctggtgctgcacgccaccgccgagagcgccgcgcgcgagctgtctcgccccagcgttttcgtgctggacatgggcgagccggtgaagatcgtggacatggcgcgcaacatgatcctgctccacggcctgcagccggatgtggacgtccccgtcgtcttcaccggcctgcgcccgggcgagaagctgacggaggagctggtggactccagcgagcgcgtcgtggcgcggctggattcggtgatggaggtagtggagcacggagcctcggctgttgtctctgaagaacaggttgcatcactcgaggcgctggcgaggcgaggcgacgaggtcgaggtgcgtcgggtcgtctatgatcacgtaacccgcttgcggggcatcgccgatcagcgagccgcgggttgacgtcatgtccatgcgccctcacagcccctccggcatggccggaaccggatcaggactgaaggcgtcgcatgtcgcgttgcgttggctgccggccggggttcgcgcgcggctcgatcggtccgagaccctgcgtcgctttctgaagctggccagctggagcctggtcgccttcgccctggacaaggcggccatgctggtgatcgtcttccttctggcgcgcattctcggcgcggccgattacggccggctgacgctggcgcaaggggcggtgaacacggggcagatctttgtggtcttgggcgccgggaccatgctggcgcgctacattccggcgatgcgggaggaaagcgtccggcgcgccgtggagctggtgaacctttgcgccctcgtggttctgggcacggccacggccttcactatcggcggcgttctgggcgcgccgcggatcgcgacggcgatcctggacctgcccgcacactccccgataccctactgcatggtggcctgggtgctgctgacggcgctgaacagtctgtcgctgaccatcatgctgtcgttcgaaaagggtcgagccatgggcctggtgtcgctggtcggcggcctgctcacgatcgcggctgttcccgcgttggcggtgcaatggggactgccgggcgccgtggcggccttgctcgtcgtcgaagccgccaagggcattctgctgctgaccctgtatcggcggctgatcagggcggaaggtgttgccatgctgacgcccgtgcgccgcagcgacgcgccgctgctgtggcgcttcggcctgccggtgttcctgaactccgccttgtggggaccgacgatgtggctggctcagatcattctcaagacgcgggcgcccgacggcttggtcgccgtcggcgtattcggctttaccaacagtatcctcggcgcggtgatcctgatcagcggcctgaccaatcgcgccgccttgcccatcttgtcgtcgatcgatgcaagagggggacatcaggttctttggagaacaactcgaaagatggcgtgggtgcaaacaggtatagcggctctcattggcgttcccatagccgcggcagctcctatgatcatggagttggcgggggcggagtttaaggcctcatgggctgcaatcccggtgatgatcgccgtcggggttgtgatctccggacagacggccttagggaactttttgctgataagagggcgagcgtatttcattttaggcacaatggctgtttgggcggcagttgtactcggcgtaaccacttggtttagtgcttacggcgtgtttagtcttgtgtgggcgttgttcacaggggcgcttgtccgcacaggaatgatcggcttgacatcgtttcgggaagcccgttcggaattcggcggaacgaaagttgcacagaacggcggagcggcggacgcgtgaactaccctgcgctcccatctccccgtcggaccgcagtcgcgccagatcgcggtgccctgctcatctatttgccattggccctgctgctcggagtgaggctcgcgtcgccgtcggcggcgctgctcgcctatgtcggcttggccgcctacgccctgctggggcgcaggcaagcgatctatgctctggctctgtcgtggctgttgaccataatcaaccctggccttgtcctcggcggcggggccatggtcgccggtgttgcctcggggggcgctcaattctagacatgtctctgcaaacacaggaatttgccgtcttcgcaggtgcgctcacgccctacaatggcgtcgacgttctggcgcgagcttgggcaagccaaggtgtaccgtatgatcttcacatattcggcaggggggctctcgagagggatctagaagcgctgtcgagggaccatgaccgtatccacgttcacggatttgttcctgagcaggatgtagcctgttggttgacgcgcgctcgttggaacttttgtttccgattgagtcgtgggatcgatcagcgatacttttttccttcaaagctcttcaccttggcttgcacgtctggggcgatagttacaaacacatcttttgatgcgccagccgacctgaaatctcatatgcacgttgtttctgatgacgcgagcggactcatacagcatctccacgtcgcgcgggacacatgcggtgaattagcagtttctgagcgaaaacggcacgtcatcacaaagtatacctggaagcaagaagtggcggccattctacaagagctaagaggcgtttaggtgttgtctcgtcagaagagtgcacttgacgtcgatcctgcattgagtggtcgtcaggaatcgcgaagattggcgacgtttctcgcctacactcttgcgacggtcgtggcgttctggatctcgtggatcctcctcgggatgtataccggaggcgataacaagttttatggtgcattgtacatcgctcttgcgagcgtggatttgagcgaagtgccgcaaatccagaggggtatggtgggtggttccgaacctctatacggcgcgatcatgtggttgggtgctcatcttggcatcgatcggctgatatatttgagcgttttcaacgccgtactccttgttggctctcttctgctggcgcgtagatttggcgcagggtggatattttgcgttcttctgctgtcaaacttctatgttctggttctcgtctgttccgctgagcgactcaagttcgcctatatcgtagtaatgctgggatttttatctggcggatctcggcgatggcttctcctcgtgtcggcgccattctttcattttcagacgataatcggttacgtggcagcatctctgccggtcctgcggcgtgttgcgctcaccgcgatgcgatcgcaaagcgtgtggaggcctgtgattgtcagcgcaggcgcattggcggcaggtgcgctgctcgcgcctttgttccccgctatcggtgggaagctatcatcgtatgccagagaagggaccagcgttttggagttggccaatctgctggtgctttggacgagcggattgatagtaacgcataggcgtcttgacctttccatcatgatgtttgcgactatcgtcgctgcagtgatcctgggacctgaacgcgttaacatgatcggggtgacgctgttcatcggtcatcttctcgcggagcggcgcgtgaacaatggcgttgtctatttgatcatggcctatctgtcggctaagtcggtgggctttatctacaatgtggtccagtacggcgacggctttgtgaactccgtctggggaggcggcgggtttcaatgagggttgagcgcttcgacgtccgaatcgccgccattcgccactcgctcggctatctggcgaccggtcacgaaaccgccgactggctggtggcgcggggcgcccgtgcggaccgggtgttccccttcgcctatttcctgtcggacgggatcgggcgcggaccggcgccgtcccggccggccggcggctttcgcatcctgttcgccggtcagttcattgaacgcaagcggctcgacctcctgatccgggccgtggcggcgctcgggcgcgaggatgtcgaactccaggtgatcggatcgggccctcaggaggagacgctccggcgtctggctgccgaggccctggggtcgcggcttcggtggatcggccgggtcccctcgggcgatgttccgggccggatggcgcaggcggatcttctggttctgcccagccgccatgatggctggggcgcggtggtgtcggaagcgatcatggtcggcacgccggccgtttgcagcgaccgctgcggctcggcgggcgtggttcaggccagcgggcgaggcggggtgtttccggcggacgacctgggcgccctgaccgccttgctgcgccgtctggtggacgaagggccgccctcgacggaccagcgcgctgccctggcgcagtgggggcggcgattgggcgccggcgccggcgcggactatctgaaggcgatcctcgccttcgcggacgcgggtggtgatcgcccggcgccgccgtggatgattcctgcggggatatgtcagtgacccgccccgttatcctgaccttcacggggcattacctgcccggctacaaggccggcgggccgatccgcagtctggtcaacatggtcgagcagctgggggacacgtttgacttccgcatcgtggcggcggaccgtgatctgggggacgcggcgccgttcgagggcgtcgccgtcgatgcgtggaacacggtcggcgacgcgctggtgttctatcgctcgccgggcgcgacgggttggcgcgccctgctgcagagcctggacgagacgtcgttcgacctgatctatctgaacagctttttctcgacgagcgcggccttgcgcccgctggcctatcgtcgaacggggcgcgtggcgcgaaagccggtgctgcttgcgccgcgcggcgagttctcggccggcgcgctcgccctgaagcccttgaagaagcgcctgttcatcgcgctgtcgaaggggatcggcctgcatcagggtgtgatgttccaggcgtcgtctgagcatgaggcggccgacattcgccgggtgctgggcgatgtgtccattcacgtcgcctccgacctgccgggccgttccggatcaggcgtcgccgccgacgtgcccgctctggtcgccaccgaccgaccgctgcgcgccgtcttcctgtcgcgcatcagccccatgaagaacctgctgggcgcgatcgagattctcgcgcgggtcgcgacgccggtgacgttcgacatctatggggtgatagaggatcaggcttactgggcccgctgcgaggccgccattaccgccttgccggcccatgtccaagtgcgatatcgacggcctctacggccggatgaggtcgccgacgtcctagcggcgtatgaccttttttttctgcccacgctgggcgaaaactacggccacgtcatccgtgaagccctgtcggctggattaccggtgctgatcagcgaccgcacgccctggcgcggcctggccgcccagtccgcgggcgcggacctgccgctggaggccccggacgccttcgtcgagtggatcgagcagttcgccaggctcgcgccggccgagcggaacgccatgtgccgcgccgcgcgggcgcgaggcgacgatcctgcgatggcggcggcggctgtcgaggccaaccgaacgatgctgctgtccgcccttggcgcggctgccgcctaagacatcttttcaggactcccagaccatgttcaaggacaagaccctgctgatcaccggcggcaccggctcgttcggcaacgccgtgcttcgccgatttttgtcgtcagatattggcgagatccgcgtcttcagtcgcgacgagaagaagcaggacgacatgcgtaagcgctatggctcgtccaagctgcggttctatctcggcgacgtgcgtgacgaccgcagcgtggcggcggcgatgcagggcgtggacttctgttttcacgccgcggcgctgaagcaggtgccttcgtgcgagtttcacccgatgcaggcggtgcgcaccaatgtgctgggcaccgaaaacgtgttgaacgcggcgctgcacagcggcgtgcggcgcaccatctgcctgagcaccgacaaggccgtctatccgatcaacgcgatgggcgtctccaaggcgatgatggaaaaggtggccgtagcgtcctcccgcagcttcgccgagacgggcctcacggtttgcggcacgcgctacggcaatgtgatggcctcgcgcggttcggtgatccccttgttcgtcagccagcttctggaggggcggccgatcacggtgaccgaacccgccatgacgcggttcatgatgacgctggaagacgccgtcgaactggtgctctacgccttcgctcatggggacaacggcgacatcttcgtgcagaaggcgcccgccgccacggtggagaccctggttcaggccctgctggaactgttcggccgaccggatcacgaggtgcgcgtgatcggcgttcgtcacggcgagaagcagtatgaatccttgctcggcaaggaggaacgggcgcgctccgaggatctcggggactacttccgggtgccgccggacggccgtgacctcaactacggcaagttcgtcgatcagggcgacgcctgcctgcacgaaggcgaggaatacaactcgcacaacaccgagcgtctggacgtcgagggcatgaaggccttgctgctcaagctggagttcatccagcgcctgctgagcggcgagcgggcctcgctggaggactgagccatggctgttgttgtcaccggagcgcgaggattcattggccgcaacctgatggtgcggcttcaggagaccggagtggagcctcttccgctcggttcggatgcggatgaggccgccattcgggccgccgtggcgcgagcggagttcgtcattcacctggcgggcgtgaaccgacccgttgacgagacggatttcgtgaccggcaatgtcggctcgaccgaagggctggtgaaggccctcaaggacgcgggcagaccgattccggtcctctacgcttcgtcgatccaggccgagcgcgacaatccttacggccgcagcaagcacgcggccgaggacgtcctgttccgctattcggaagagacggatgcgccggtgcgtgtctttcggctggctaacgtcttcggcaaatgggcgaggccgaactacaactcggcggtcgccaccttctgccacaatatcgcgcgcggcttgccgatcgccgtcaacgatccctcggcgtcgcttcgcctggtgcatgtggacgatgtgtgcgacgcgatgctggacctgatccgtcatccgccgtcgagcgccgcttttgctgaagcgggacccatccacgaaacaacggtcggggcggtggccaacgccatcaccgactatgccgccagccgggagaccctcgtcaccaaccgcgtgggccaggggctcgaccgagcactttacgccacgtatctcagctacctggagcctgagagcttcgcctatgacgtgccgcggcacgccgatccgcgcggcgttttcgtggaaatgctgaagacgccggactgcggacagttctcctatttcacagccggcccgggaatcacgcgcggcgagcactatcaccacaccaagaccgagaagtttctggtcctgaccggcaaggcgcactttggctttcgtcacatactgaccgatcaacggcacgagatcgtcgtcgacggcggccagggtcgcatcgtcgagaccatccctggctggacccacaacatcaccaacatcggggatggcgagatggtcgtgatgttgtgggccaacgagatattcgatcgggcgcggcccgacaccgtggcgcagaaggtctagccgtgaagaagttgaaggtcatgacggtcgtgggaacacggccagaactcatccgcctgtcgcgcgtcatcgctcggctggacgatcatacgcagcaggtcctcgtccacacgggccagaactacgactatgagctgaacgaggtcttctttcgggacctggaaattcgcaagcccgaccatttcctgaatgcggccggcggcaatgcggccgagaccatcggtcagatcatcatcgccgtggacaaggtgctggcgacggaaaatccggacgccctgctggtgctcggcgacaccaacagctgcctgtctgtcattcccgccaaacggcgcaagatcccgatcttccacatggaggctggcaatcgctgctttgatcagcgcgtgccggaagaaaccaatcgtcgcatcgtcgatcacaccgccgatatcaacctgacctactccgccatcgcgcgggattacctgttggttgaaggcgtcgcccccgaccgcgtgatttgcaccggcagcccaatgaacgaggtcttgagctactatcgtcccgccatcgaaggctcgcgcgttctggaggaagtgggggtccgcgaaggaggctacgtcgtcgtcagcgcccatcgtgaggagaatgtcgattccgagcgccaattgcgacgcctcgccgactgcctgaatgctgtggccgatcacactggcgagcccgtcctggtaaccacccacccacgtacgcgggcccggatcgaagcttttggggtcagcttcgacaaccgggtgcgcctgctcaagccctttgggttcctggactacatcgcccttcagacgaaggcgcgggcggtgttgtcggacagcggcacgatcaccgaggaatcgtccatcctcaacttcccggcgctgaacttgcgcgaagctcatgagcgcccggaaggcatggaggaagcgtcggtgatgatgaccgggctcaaccccgagcgcgtgctgcaagccatggcgatcctggaaacccagccccgcggggacgaacgtctgctacggttggtgcgcgactattcgccggacaatgtgtcggacaaggtgctccgcatcatccttagctacaccgactatgtgcgccggaccgtctggaaagagtactgattgtgtcgcgtcggattctatatctcagccagtggttctggccggaacctaccacgcgtggcctgaaggttttaaagggcctccaggctagaggctatgaagtcgaggtcctgaccggcttccccaactatccctccggcaagctggcgcaaggttatcgtctcgcgccctataagcgcgagcagatcgagggcatggccgtccatcgcgtcttcctttatcccagccacaatcgctccagcctcggacgggctctcaactatctgtccttcttcctgtcggcgttcgtcttttgcctggtccaggctaggcgctttgacctgatctacgtctatcacccgccgatcacgacaggcttggccgcagcgcttgctggtctgatctggcgcaaacccttcattctggaggttcaggacctatggcccgatacagtggcggcttcgggcatgtcagccaccggcaccttagcacgcattctggatccgatctgccgcttcgtttataagcgcgccgccctggtgttgggccagtctgagggcatggcggcgcggctggttgagcgcggcgttgatcctcgccgcgctcacgtctttttcaactgggcggacgaagacgccgcacgcgccaatggcctctacgatctggcttccctgaacttcgaaggacgcttcaactttgttttcgccggcaacatgggaacggttcaggcgcttgaggtactgatcgacgcggcacacagcttggccaagatcgcgcctcaaatccagctgactctgatcggagagggtgccgagcgcgcgcgcctcgagacccttgtccgtaaacaaggagcccgaaatgttcagattctgccgggcgtgccgccgtcccacatcggcgatgttatggctgccgccgatgtgcaggtggtccatcttaaagatgatccgctgttcgaaatcaccatcccgtccaagacccagttctatctcgccatggggcgccccatcctgatcggtgtccgcggcgaggccgcccgaatcgttacagaggctggcgccgggatcagcacgccgcccgagaacagcgccgccatggctgaggcgatgctgcatctggccactctgccgaaaaccgacctccaagccatgggcacccgcgcccgctccgcttatgattcccgtttcgccttcaaggccaccatggatcgcatcgctgcccatgtgggtggggtcctggagaagacgtgacggtgctcttgtcattgatcccaagagaagctgaaagaagcgaagacagtgccagttccgcctgaatccgtttcctctacagtgtcgatctgaacatgttccacgacatctccgctttcgcgcccggatggcagcgcatcggctggtttccgacgaggtactaattgtgagcaaaggtagtcatcgggatcaggtccctgtcggtgtggcgagaggatccacgcttcaatcgacacttatccgcgccatcgacttggtggcggcgatctccggcggggtggtgactttgccaatcttgctgatcctcgcgtttctggtgcggcttaactcacccggtcccgctcttttccgtcagagccgagtaggtcgaaacgaagccctgttcgtgtgctacaagttgcggacgatggttgaggggacacctggcgtcggcacacacgagatttcggtcgcccacgtcacctcgattggtcgctggttgcgccgcttgaagctcgacgaactcccgcaactttggaacgtggttcgcggcgagatgagtctggtggggccgcgcccgtgcttgccctcgcagcttgaactgatcgaggcgcggcgggcgcgtggagtctatggcgttcgccctggggtgacagggctcgcacaggtcatcgggctggacatgtcgacgcctcgcgaacttgcggagaaggatgcgatctgggcgcgcgccccaaatctcaaggactacgtccgcttgatcatattgactgttttgggaaaggggcagggtgatgccatcggcgcttgatcgtgtcgggattgtcggagcgtcgggctatgtcggcggggctctagcgcaagcactggtcgcggatggtggctctccacggctgtttggccggtgtgctgcccgagtggcaggccttgatgtgagagcgctaacctccgatccggcacagttcgaggggttggactgcgtcgtacatctgtccggcatcacaacgagtcgggcgtctttggacgatcttcgtcgagccaatgtcgaactggctgtgaacacggctcgcatggccgcgaccgccaacgtcaagcggtgcgtattcacaagttcgctgcacgtgcacggcaagtcctccgaagaggccatccgacccgatacgccgatcaatcaagccgcgaacccctacgggcgctctaagggcgacgccgagaaggcgctgacggagcttgccgccaaagccgggcttgaactggcgattctacgtccccccatgatctatggggctggatccaagggcagtttcccgttgctggtgcgcttggtccgaagtggtttgccgctcccctttgccacggctcgagcaaaacgcagcttctgttccatcgacaatgtagtttcagcgctccgccattccatcgcggcaccggtctccgtcggggttttcttgccggctgatcccgaggactttgataccgcaaccctggtgagagaagtagcggcggccatgaaccgcagaatcctgctttggccagcgcccaaggcgctcctggcggcgccgcttgctgtcatagggcgcgcggaaatggtggccagcctgttcgatcccctgcagattgatcgcacacactggagcagattgggatggcagcccatcgagacaggcgcgcaggctgtccgcaaggcggttcgctcacgctgagcagaaggttggaactcgggtcgcttcgggaggcgcagattcaagcgaggagcgccaaggggtcgcatgatcgccgtgtgctgtatctgccgaagagaacggctgagcctgtggggctagatcgcctataatcaggccaccgccgcctatgcggctgaatcggtcgtcgatcctacgcttctacgcacaaccattctcgctccgcctctcgccaggctgcctagcagcagcgccagaagcacctgaagcgcaggggtgcgaagcggatagtcaacgagcgaggccgctaggagcacggcgacggcgagaagaacaagagcgctatacgggcccttgtgtagccacgcctttcggagcagcagcacaagaagggctgcgggcaagagcgcgagcaggccatattcgatccccacctccagccagtcattgtgcgcctggttggtgaagccggcggtcagatcgtccggcgtttcgacgccggcgaagaccgcgctaaagctgccagcgcccgtcccgaacggcaggtgggcggccgcgatgcgtcctgcgtcggcccagatgtcgaaccgcagatcacgaggcgcatcggcgaagcggtccgcagcgacccaagacccggcgacggccaggccgagaccgaccaccagcagcaggccgagcagaaggaggcgacgccggtccggtgtccggcgggctcgcagccctggcagcagtccaagggtgcaaagcagcagcagcccggcgccggccctggagccggaaatcgccacccctgctagaagggcgagacaggcgacggcgccaagggcgagtgcgacgccggagcgccctcgatccgccgaggcgcggcgctgaaagctccacgcccccacggcgggaagggaggcgaccagaaaggcagcccagtggttgcggttggcgaagaagccagtcgctgcgcgtccggcatccggcccatagagacgaaacgggctggacgggccgccacccagttgaaaaccgcctaagccgacggagatgaccgctatcaccgcgacgagcagccacaacgtctcggcttgcgagcgacgaagcgtcaatacgccgaggaagacggcggcaaagggcgtgaggccgagcagcgcgtctatcgtggcgccgggcgccaagctgaccggccgccaggtctcgccggcaccaactgcaacgagatcattcgccaatgcggctcgaccaggcagagcgctccagagcgctgggggcagggggatcaactgcaccagcggcaacaggaaaagcgagccgagaaacagcagggccgggcgagagacgtcccctctcgtcagcagccgcagagcgcccatagccagcagcggcaagccggccagccggagaacgaggtcgaagccgtcgttgtcttgagacgccccgccaaggaccagcgccagaacaaggtacaagcccaaggctgcagtgtaccaaggatgggcgtcttcgccggttcgcgcatgtgcggaaagcgggttcatcggagacccgtcggttcaatgctcagttcgtcgaagaccgcggtacccggcgacaggctcgcgcccggtcgtgtctccagcgcaagtcgctgtgcagggcaggcctgtggcgtttcgaaagtgacggagaagaggaaggcgccctccccgcttccgcgtagggtttgagttgcctctatggcaggtccgttctcacagcgcatcgtccacaccagggcgtcttcgcgtgtatccgcttcacgccacaggcgtccctgcagccgataggatccgggcgcgagcaccagcagctgttccgccagcctctgccgctttagtccgccaagcgccgtcgcctggagtacgcggccctctcctgtgggcgagccgatgatctcggccgcccccccgtccgccgccagcagtcgccatccgaagggcggcaggctgttatcggcctcaaagccgccgtcgatcagcaagccggcggccgtctgtgggcgctgttgttgccacgcaaccagcgcggcgacataggcgcggtcgcggacaagacgatcgatgtaggcgccggcttcctgatcggtgggaggcgccggaccatcccgcagcaactgatagagatggtaggcgaaggcgggttgagaggcggatcgagcgtagctcgtcagcagcatcgatcgccatggcggcgtcagcgccagccgttccgccagggcggcgcgcgcgcccggcgcggcgtcgagcaaggggaacagcacggggaacagcgtctcgttcagctccggacggcgtcgaagcagaacatccagagagcgcatggcggcaggatagtcctggcgatctaaggcgcgggcgaaaagccaggtttggctgggcgcgtcgcgcaggctgcgacgggccgccgtttgcatcaatgcatcggcgtgctggagctcgcccttgaagacggcggcttgtcccagcacggacacggcgcgcaccgacagcggggcgtactctagcgcgctgcgtgcgtgagcttcggccagcgagacgctcgcaggtcccgcagcgcttcccagggcgtccgcagcaagattgaggtgcgcctccgcctgccacggccataccctgagcgctcgatcgggattatcctgcgcccatagtctgccgaggccgaacgccgccgtgatcacgcccaaaccgacggtggcgccgacgatgagaactgccgcaagaggagatgcccgcagctttccctgccggcggctttcacgagcgccatgctgcgacgtgcggcggaccatctcagagacgtccctcagcgcttgcgtcgacgcgccttgccgccggacgtctcctccatcccatagtcataggaataggtgtactcatagccgtagccgccgaggttcgcccgcttggagtcgaagcgctccaacacaccgcccaggatgtcggcgcccgcgcctctcaaccggtcaagggcgcgcagcgccgtgcctcgccgcacgatgcccgcgccgctgatgaagagcacgccgtccacggcattgccgagcaaggtggcgtcggccaagcccatcaccggcgggccgtcgatgatcaccagttcgaaatgctcagcaagcctgcctagaacgtcgggcaaggcctggctggagagcaggtcggcggggcttggcggacgcggaccgctcggcagcagggtcaagtgttcctgctccgtcggctgcagcaggtcgttcaggtctgatcccgccagagccgacgagaagccagcccggttggcgccgcccagcatcttgtgcagggacggattgcgaaggtcgccgtcgaccagcaacacgctcttgcccatccgtgcaaaggcgcgggcgatcgcaaccgacgaggtgctcttgccttcgaccggctgggagctggtcacaagaagggtgcggaccatgccgccaggccttgcgaactgcagcgccgaacgcacggagtgataggcttcagagaagccggagcgagggtcccgctcggcctgcgccaaagccgcagccgacggcaacagcggaacactgccaagaaggggcaggttcagcttcgcttcgatatcggccggcacacgcagcgattcatccaggaattcgagcacgaagatgatcgcagcgcccagcagcaaacccagaagacccgcgagtgcgaggttgatcagcgggcgcggcgccacgggcttcaccggaaggtcagcccgatccaccaccgacacattgttggtgcccacacccccagcgatgccgatttcacggtagcgctgaagcaggccgtcatagagggtgcggttcgtgtccaactcgcgctgaagaatgttgtagcggatgctgcgttgatccagatcgagcgcctgcgccttcagagcgtcgatttcgccctggatcgagcgttcggcggccgccgccgacgcatactggccttgaagcgagcgacgaacgtcgcccgcctcggccgccaactgccgatccagctccgtgatctgggcctgtagctgctgaacgctggggtactctggttgaaagcgttccagaagctcctgccgcctcgcggcaagttcggcacgctgttcgcgcagagcctgaatggtggggctggacaacacctcgctgagccccaatccggtggacgcttgcgctgcgcgccagcgctcttccgcggcgatgcggctggtgcgcgcctcggcaagcgaggcgttgagcgcctccagcgaggaagcgatcaacgagcggccgcggttggcgcccccgtccgatgtggcgctggcgctggggatgttgatgatctgctggttggaggcataggcgacgagctcgcgctcggactcctccaagcgggcgcgcaactgctcaatccgttcttcaagaaagcggcgggcgtaggaggaggcctcgaagcgacgctccaggttggtcgcgataaaggtctcggtgatggagttgaccaccgcctgcgccagcgccggatcggcgctgtcgtagctgatcgtcactaaccgtgagttcacgaccggggtgacacgaagattggcgagcagttgattgaccgcctgccgattgcgttcggccggtgagccgccatctttgtcagtagacgactgtgcgttggcggggctgcgtcggttcgattccagaaactgagcatcctgcgccagtcgcaggcccgtcaccacgcgctgggccaatgagcggctcttcagcagctcatattgggtttcgtagaactcctgtgccgaatacatgccttccgctgggagaaccccttctacgtcgacaacctgcgcggcttcgcggtcgatctgcagcgtggcgctggcgcggtagatcggtgtcgaaagcaaggtgaccacgacgccaaggaccaacgccaccgctagcacgccggcgagcacccaccagcgcttcaatacaatgtgccaaagacgccgcaggtcaatcaggccttcgccatcctgaccgaacaggggacgggaccccgcggccgaagaggttgcgccgccctcaggtagcatggtggtcatcggctttatttcagtacgttgaagatgccgaccaggaagccgcctagcggcgccaggtcgcgaatgaggcggcgcgcgcgcgccgtgtcgacgatcactgtatcgccaggagccagctcagggtcggcaagccgacccgcttgaatctcccgcagatcgaaacgagcagccgtttgttggcctcctgtctggcgcaagacaacaacgtttccggcgtttgcgttatcgctcaggccttgagcctgtgcgatggcctgaaccagggtcagccgcccctgcaccgggaagacaccggcctcgcgcacttcaccggacacaaccacccgttggctttgcggcgtggtgatctggatggtgacattcgggtcgcgaacatagcgcgcagcataggcccgctccacctgagccgccagttgcgggggggtgcgccccagggcgtccacagcgccgacgagcggcaggttcaactgcccgtctccatccacctgcgcggcgccggatagttctggcacgccgaagacgttgacctgcaattgatcgaaaggcccgatgcggtagctgggctgcggcgtggtttgaacaaccggggcgggcaaggcgacgggcagaggcgcttcgcgcgtcgcacaggcgctcaacccgctgcagaacagcaggacagcagcacaagctgcgcttgacgtgcggatcatccaaaacctccaaaccagcgccgacgcgcaggcctgccagcggacgcctgcgcgggtgcgagcgcaggcatggttgctggcggctgatcaagcagcacgccatgaggccgaaccgacaccatgtccagcgccgcctctcttcctaagcgatcagccactcgttcgcgtgcttccgaaagcacgggccggcgacggcgaaggttgtgcccatcgctggcgaggatgtgcacgcgcccctcgtccagcatccgatccgaccagtattgcgcacgtcggccaaacaggcctgtgacggaaccgcccgtcaactggatccaggcgcccgcctcgaatacatcgcagatcgtctggtagcggtcttcaatccaggtcagccgctcgggatgggtgatgatcggaacaaagcctgccgcgagaatgtcgaagatgacctccgccatccggggcggcgccacgtgatgcggcggctcgaacaggaagtagcgcgacccgccaagcgttggaatgcgcccagtctgcaactgctcaagcatgtcaggggtgagctgcgcatccgcgccgactgtcaaggtcagcgggatgtcggcctgagccaactgctcgcgcagccgggtgaccccatcatggatgatctcggcggtgttgttgtacaggccagggtagatgtgcggggtacaggcaagggtggtgatgccgtccgcgcacgccacacgcgccatagccagggcttcttccaggtccggggcgccatcatcgatgccgggcaggagatggcaatgcagatcgatcattgagtggatacgctacgccccccggcgccggcacaaaccgcaaaaaaagagcggccgaagccgctcttcttgacttccgtgatcagggcttagcggctgatcggctcgtcttcgtcatcgtcggcgacggtcgccacaacggccaccagaccgccggccgccagaccgccaaccaccagacccgtggtgctgatcgctgccagccccccagcagatgctgatcccgccgcgacgccagcgccggtctcaacggcctggccgccgccggccacctgagcggcgcagggcgaaaccgaaggaaccgtaaaggcctgacccgcagcgatcggcagcgcgcagccgtcggcgaagacaacctgggtggccgcagacgtccgaaccacgtcaccggcgcgcaggatcgaggctgcgtccgacgaaacaaagccttggccgcggtccaccatcacttgaccagcagcacccgacaggcgcgcggtcggcgtttgagccgaaacgcccgactgggccgaagcgcctgcggaaaccgcagcgacggcgagagcggcggcgacgacgctcagggacttcatcatggtggacctttcgaacagacggctaccgcaggttgccaagacgcatagcacggtggagatcgcgtcagcaaccccgattacgtcaaatgagatgactgcgaggttaaagggcggatcaggcaaaaggttcatatcggcgacgcgtctcgtaactcagagggcgcgcctcagcggtgatccgagccgctatgcgggccgccggcttggcgcctcacagctccaatcgagataaccagaaacacagctgcgacaacagccgaatcccagagggcttcaagaacgctggggcctcggttcacgccgggcaggccctggatcacttcaatcaagattccaagaagcgtcaggccccaccacagccgcagaagcgacgttcggggcagagccgcggcggacagagccgccagcaccagaaaggctgcaccgtggctcagccaatccgagccaagcgagggtgcggacgagaccggcagaaaggcggccgccagcacacccgcgcccgagacgataagcgcaaggcggcttaagagaacaacaaggcgcgagtttgaaaaggcgggagaggctatgttcacgcgctgtcctagccgactggccctcaggcccgcaacgaccagcctcccggcttgcatcgggatgtgcggggatggtgcaaaggccgaccccttggcgctgaatgggcgcaacggcatagacctcggtcggtggagaacaccacgactgggggcggcggacatacgatcaacctcgagcagggtgtcgaggcagaattgctgatccgccgcgcccgcgggccgctcaccattcaggtgcagatgatcagccaagtcgaggtggtctcgtcgagcggacctgcgcccggcggcaggtgaagggttcaccttgcgccaacagggtcgatggcaagcgcaaccgggtggacatagacagccgcacgggagcacgaatcttacctcgccgaatgcgcacgccagcgggttgatgaccgtcttgggcgccaggttgccgggacatgatcagcggccccgcgaaaacaaacgctccaacgcagacgccagctccgcccagacctcgccttcgcggccgtcgcgcctggccttgatccgcacctcctggagcaacagctcgcgctctacgtagcggctgagcttcaggtatgcgtcgcgctgctcgcccttggcgccacgggcgcgggcctccagctgatcaagcgtcagatcgctcttgaggcgattggcggcgtcgcacacgacccgaacattgccgggaacatagccgcgcttaggctcgacacggtccagcgacggcgaggcccccgagcgcggctgaccaacaaccaagggggtgccgaaggcggggcaggttggcggcagcacgatgtcggaacggtcaagccgaaagcggatgcccgcccgcttggcgcgacgcctcgcccgctccagcaaggccagcgccggttcgctgcgtcgtcgacggcgctggtaggccgccatgtaaaccgcattacagcgcaagcacgtagctcgcttcagcttcgatccgtggatgggacaaacaggggtggttagctcagtctctgacatgctagtctcctacatcaagacgagtccactaattcaaactgagtcgaaagagtcaaattgatgatgaggccgccccgcaagaagccggctgaccacccgaccggcgcccagcttcgtgcggcgcgcggcctgctgaacatgagcgttctggagttgtcagagcgcacggggctggccgtgaacacaatcaagcgcgcggaatcggtcaacgccggcgccccgatcaacgccgccaatgccaagctgttggtcacgacgctgaccgccgcaggcgtcgccttcattgcgccgtccgacggcctgggtgcgggcgctcgtcttgttgacgacgctcaaccggcgctgagccgtaagcgcagatcgacgtcggaaagcgaaggcgactaagggcccttgcgcaggcggtcgcgcccggaggcttagcagttcgcgcatgtttgtgtgcttaccggccttctgagcaccaagagccagcttcataaaggcagcgcttcggcgccaccgcactcttggtccccttcacggtggtgcaaagaaggatatgggctctacgccgagggccacagcgaccaggacggcggacgtcttaggcgaagcgcatgcgacgcaaaccagaacgaccggcggggcaaaggctgctggccgcgtccacgcaggcgccctgcgtacgcaggacgcccacaatcatcaacaaggccgacgcccacaacagcggcgtcacgctgcatttcaaagtgcacgggatgaacaacggccaagtgctgagcatcgacgtcctgcaggcgaatcggctcgctgatcgcatcatccaggacgcatccgccaaacccgtcagggtcaggaagccggctgagcagcacaacacgaagaacggccggggcgccgctttggcggacccaaagggacggcgccagaacggcattgagcggtccttctcgacgccgcgcctggccatcatgttttgacgcgggcgagtccggacctgtcaaagcctgcccgccggcgacaggcgtctggctcacgccgcctgccccatcagatcttccaggtccgcatccgggtcctgcagcacagccagagcggcggcttgcagcaccactacgcgcttgttctcgtccccatccaacgccagggcggcgctgagttgcagcgtggcgcaatcctcataggcgagctggtaatcgatcgcagtcacgtcgcccgtatccgatcgggtgaacatgcgctcggcggccgcaggcaagccttcgttcgccatctcgtggagcgtctcgatcgcgacggcgacctcatccaccgccagggcgctcaacaggccgttcatcaaccaaaaccgaccttccgaccgggggtgagccgccgcgatgcggcaggcttcagccaggcgcgacagaatgggcggcgtcgcggtcgaggcgcacgtcggcacgtcgccttggacgcccgatgccggggatgcgcgccaggcggcgcaccaggcttgaccttcagccgtcaacgcccaacgcgtttcgccttgggcgccggtgaaggactgcaccattccctcctcagccaattgctgaagggcggcagggactatgcggtgctcgatggaggcgttcataaggaggctcgctgttgtgcggcgcctttttattcgacgccgcctatatgggattgtggttcaagagccgctggagagcgcggcattgaccagcaacagcccacacgcgtggggacctcgccgctccgccagggcgcagccgcaaatcgtgttgattgtcgatgccgctgaccgaagcggttggaacaagagacgggaacgccacgtcatcttgttttcagatcctgccacaaaggtcggaggttgtcaagatatcgcccacgccgctccagtctcaacgccggaacgttagcccgtctgtcaacactctcgcgccaacctataactatcactgtccctttttcttcttttgaagcgacagccgactccatcaccatggacctagacggcgcatggttgtgaaggggactcgtctctacccgttccttgatgctgtctgctatttgctcggactgcgtttgttgacagaggagacatcaatccagctgacgaagtccgagttgcatgcggcgcatcccctttcggccaagccctgcaacagggcgcagccgttttgccggcccaagcagcgccaccttggcgccgccgctgctgtgctcctcagacctgttcgcgaagagggatccaaacgccggccgcgagccctccgggagcttgttccggaagacctcttgctgagcatgaccgaagcccttcagcggcggcgaacagcgaatacgcctttgagttggagacgcttacagacgcagtcacggtttccaccgggcgtgacagccgggcagtcacgaaaggtggtcactttagccctcgaaggtgactgcttaagcgtttgttggggcgccagtcacgttttccaccaacggtgactcgtcccaggccggaacgagccggtcctgagcgggcgcggctggggctgggaggggtcacccccagccgcgcccctcagcgtcgacgcttccgcggctcccgctccgcattgctgggcgcgaggtcgccgtggcttcaggtgaagccggtggcggcgttgaagggcgctagagcagcggttttcaccgggtgaccttgacctgagacgacgcactgatccgccgactctatagcggctgcgcctgcagttggcggctcaggctgaagcgcctcgtcccacccccaggtattggaagccgtgcgcctgaacagcgtcaggctcgtagacgttgcgcagatcgagcagcaccggccgccgcatcaggctcttcaggcgctcgaaatccagcgcgcggaaggaatcccattccgtgacaatgaccaccacatcggcgccctcggcggcatcataggcgccgcttgtcatctcgacgtccggcatcagccgggcggcctcgggcatgccttccggatcgtagccgcgcaccctggcgccggcggcgatcagggcgggtgcgatgtccagcgccggcgcgtcgcgcatgtcgtcggtgtccggcttgaaggtcagacccagcagcgccaccgtcttgccggccaggccctcatcgaccgccgcggccaccttgtccgccatggccttcttgcgcgcatcgttcacctcgaccgtggtctcgatcaggcgggcgcgggcgccgtgatcctgcgccgtccgcaccagggccagggtgtccttggggaaacagctgccgccgtagccggggccggcgtgcaggaagcgcgagccgatcctctggtccagcccgatgccgcgcgccacctcctgcacgtccgcgcccgtggcctcgcacaggtccgccatctcgttgatgaaggtgatcttcatcgccagaaaggcgttggcggcgtatttgatcagctcgctggtgcggcggccgacaaagaggatggggctctcgttcagggccagcgggcggtacagctcgctcatcaccatccgggcgcgctggctgtcctggacgcccaccacgacgcggtcgggccgcttgaaatcgccgatggcggcgccttcacgcaggaactccgggttggagacgacggcgaagtccgcatcggggcgtacgcggcggatgatagcctccacctcgtcgcccgtgccgaccggcacggtcgacttagtcacaacgacggtgaagccttggatgaggccggcgatctcttcggccgccgcatggacataggacaggtcggcgcgaccgtcgccgtgccgcgacggcgtgcccacggcgatgaacacggcgtccgcttcacggatcgcgtccgccccgtcctgcgtgaagaacagccgttcctcgcgcacattgttggcgaccagatcctccagtcccggctcgaagatggggatctcgccccggttcagccgctcgatcttggacggatccttgtcgatgcaggtcaccacatggccgaagtcggcgaaacaggccccggacaccaggcccacatagccggtcccaatcatcgcaacgcgcatctgcatcgatcccctttggcggcctgccgcttagctggccacggacctgataaccagcctttgggttgatgctctctgggacgaagacgacctccaggggcgccggaacgccctagacctgcaggaaacgggttcggggtttttgaggctgccgtggcatgagtttgggccccgaagggcctccacgggccggaaaatgggcttgtccgaagtgtttagcggcccagtcacgttttccaccgggcgtgactcggtttttgtcacgaaaacgggcgcgccagtcacgaaagcggaggggttcagtcacgaaacgtggtcacgttacacaccatctgtgactccttaaccgtttgttggggcgggcctcgccgtgggttggggcgggcttaacttttcgttgaggcctcagtcacgttttccaccaacggtgactggacagggggtcgagcaggggacggcgtctgcgcttttcgtgactacgctgatgattctgggcacggcctttggatttcgtgactcggtcagtgacccgactgagtcacgattgccggggcgattttgctgtaaatgctgaggattttccgggggtgttcggacgggttggaggcggggcgcggtgtgaaacaatggtgaacgctgttcgcccgcgactttcccgaaacgtgacaggggtcaaacggttgaaaaggttcttcttttcagcggaggccaatccctctgtcacgttacatacgaagggtgactcacaaatgcggtcttaaatagcaactttgtgcatttggattgcgcgcgtccggacctgcctcaatgagataagcagcgccgggacggtggggcgcggctggggctggggggttcacccccagccgcgccccctcgcggcgagaactgttggcgcggttcttgcgacggcggttgtggtgaacagggagggtttggctatgcggtctgaaagatgcggcgccgggatcacctatcgcgcgatccgccaagcttttgccgacgagctgaaccgcaacgccctccttgttgctcggatagagaaggcggcaggtcacgcgtctacgcagtcgttcgaaggcgcgttcatgaccaaccatggcacggaccttcgtatgatcatcgtcacggccgatggttcagacgaccagatccaccttaatgtgcagatcgactccggcagccggtccggcagcgccatcgacgtcaacaccaagcctaaggtgcgcattcggcgatcaggcgatcaccgccacgtcaccattgcgccgtccctgtggttccaggatcgcgtaaatgcagcggaagcggagaacatggtgacgttcgaagccctgatgaaactcgcctcaccatccttcaaggacgcccttgaggagggcatagcgcgcgcgaaaaggacgttcgctgatcgcatgagaccgaaatctccttacccctattggatgtcagcccggcggcggcctctttaggaacagcggccggagccacggggtgcaggtggttcacgtcccagagctacgaaagcgatggcctctccaccagcttcgcacccaagagcgtcagcggaaacgcaatagagccggcgcagctaggcgcggccttgtgccggctgaacagcatcatcagcatgagcagcgatgggaaaggacctcaagcgccgtcgcggccgccacaagcgcagcccttcaccaaagcgcagtcagaaggtgtttgcggcgccgacagtcagggaaagacgacgccttctgagcgaccgtgatcggtgcgcgcatcatagtcgccgttggctttcaggatgtccgaccgccagcggtccgagacccgcaccatgtcgccacatgaagaggcggagcgcatctcggtctgcatctgcgctgcgcccatggcgaccaagtgggcatgctgacgttcatgaacttcgagacgctgcaagtaccgcgtccaagcctgtcggaggcggccggtgcgacggtgttcgtcctttaaggacggcagagtgatcgagatcactggcaagacggtcaccgtcgccggcacgcaatcgccacttgcatctgtcgaccagtcgatttggaagcgccatgacgtcactgcatcatggcgcgcaccggaggcgtccgccggccggcgctgattgagcgacctgcgaaaatcacggggcgttcgcccatcgacctggtaagtcgtcacgctgacctgcgccgcggcggatgcgtttgcgggaagatcagccagactggcgatcattggaccttagcctccccaggcgagactgagtctcaaggtatggacgcgggcgggactcggatcgcttctgtcctgtgtcgccatgggagcctagcgccccaggccttctcgcttcgtggcgaggcccaaagccaccatgagctacgagcgccttatggcctagcgtttcggcggcacgagggtgaacagcggccggggcgtggcgtcggcgatcgctgccgccaccgcccagagattgatcaagcccgccgcttccaccgtttcgtccgcggcgtcttcacttagtgcgtgaagcaacctgcattctccgttctcgataacagcgtgccggtagacctggctcatgccctcgagttcagccaagatcagcaggtgggcgtggtcgccggtctgctccaaagcctcgatgtatgcggcggcttcatccgccgcaccttcaacagccaaggtccgacgctgatgttcggacaaggcggcgaacaccactcctggcgcggcttcgacggccgcacgcctggaggccggaagcgacacccccagtccccgcatacgcatcatcaggcgcatttcagccagttcgcgcggagtgaaactggcgcgcccgccttggcgagcgcgcagcaacccctgaccgcgccaatcgcgctgcaggtgaagcggcgtgccggtgatggccgccgcctctgacggcgagaactggctttcgcgatagcgcagcgagatctgagcgcttgacattcagcctattccgtgtgacccaaccacattccgtgtcgaagacacgcttttgaatgacagatacgttatgccccgcgtcggagcatcgcgcaagcaccatacaggattgaaccgaatggctgccgagcacatcacaagcgagactaggcggcctgacgacagtggacagccgcctcctgaagtcctcgccttcccctgcccaccgggcatcggtctcgatacgccgctgcgtctgtccaaggcggcggccaccgcctttccggatggctcggtgaagcccagcaccttgatgaccgaacatcagcggggaaacttagttctggagaaaatcggaggccgctggttcgtcaccctccgatccattatcgaaatgaggaagaattgccgcgtcgtcgtgaaccgccccgattatggctccgagagcgcgcaggccgcgcgcccgtatacgtcatcctcgacggaggccgtgaggtcggcacgggctgcggccttgatcgcagccgagaggctcaagaagcgcttgcgcgctacttaaccgccaaacatgaacccgcctttggcgagggggacccccgccgcatcctcgtcgccgattgcctgatctactacttgcagagcttgagagacgaccaccgcgggcccgagcccacccacgtgccgtggctgatcgggcatttcggcggcatgacgtgcagccaagtgaacatcgacacctgcaaggcctacgtcaccgcccgcatcagcggcgccatcgggcacaagccggtcagggaggcgacggcaaagcgcgagctggagacactctcggccgccctgaaccgtgcgtggaaggccggcaagatggatcgccctatcgccgtgtggaagccggacgcgaacccccaggaagcccggtggctgacccgcgacgagtccgcccggctgatccgcggcgccctgggcttcacgccaaagggcttcgacgcggaagggagggtgaccggctacacccgcgtcgccaagccgaactaccatgtggctcggtttatcctgatcgctctctatagcgctacccgccacgcggcggtgctcggattgcagtgggaacggaacgcccactcgggctcgatcgacctgaaggagaagcgcatctatcgacgcggaacggaagagcgggaaacacgcaagcggcgccgcccctgcccgatccccgaccgcctgctcccgcacctgcggcgctggcggcggctcaccgtcacaggcccagccgaatacgcgggcgagaccatccagcggcaaaagacggggttcgaagccgcgcggcggctgtcgaagttggacaaggacgtgacgccccatacactcaagcacacctgcatcacctggatgcttcaggcaggggtgccgacgtgggaggtcgccggcttcagctcgaccagcgagaacctgatccgtcagcgttacggtcaccattgcccggaccatatggagaacgcccgtaaggccctgagccggcggcgcagcgcctagcgcggcgaggaagggaaggcttcgctgcgggcgggccattcctcaccatcgtcatcttctccgccatcgtctcgggcggcgttgcggccgacaacggcggcacgctcagtcatgtcctgcacaaggccgtctaggaaggcgctgccgccggccggcatggcggcgaccgcctcggccgccccattgatttcgcgttggaggcggtcggtcagggcgatgacccgccgcacggtggcggccggcgccaaaccgcaggcctcggccattcggcgccagtgccgggcttggatgtggcggccgcggacctgaccgccgatggcctgagcgtggttctgggtaattccgggccaaggcaggccggacatcaggtcgtagagcggcgccagggcggccccgtctgcggtcagcaagatcgagtagttcttggcgtgcgaatcgacattgcctacggcgatgttgaagatcactgcgtccaacaggcgggtgatgtcgacggccgtcatgtgccggcggaccagggcgaacatttcagccagcgagggtccgcgcacaccggtttggttgcgctcgtatttggagccaggtggaattcccaaagcctggcagaagtcttcctggtgacggcgcatggcggttggcgcctggccgtctcggtcgtagcgatcgaccaggagataggcgcggccgccggccagtcctgtggtgacgggggccgcgggcaggcgacagcgggcggccagcaccatgcacaaggcctcgttctggacgctgcccggcaggcgcggattgtcaggcttcaggatgtgggtcgaaggcgcgccgtttacgggaacggcgatctgaccatccagcagcgcgaccggcagcttgtcctgggcgccggccagactcatggtcacgccctcgtccccgacaaggaagggtttgcgaggcaattgctcgatgatccgctccaggtcgtctggcgtgggcacgagccggtagtcgccctggtcttttctcgggccgccgacacgcagcgcgccggcgaggtcgccgccagtggccgagatcaggcccaacacgtcctcttgagctacaccaagcgcgcgctgcatagcgcgcatcggttcgccttcggggagcaggttcatcagccacggcagcaccacctctggcggacaggcttcttgggccagcggcatcgacagcgacacagggaaagcgtccgacgaggcgcgccaggcgtcatcataggtcagcaccggccccgtgggcgaaggcgtcacctcggcaaccggcctgtcgccgtggaacagcgtcggcatcagcgacgccccgcggtgttctctaagcggatgccgaccgccttggcggccgcgagcgccttgccgagttgggcggtggccttacccgcctctagttcgacgatgaaccgctcgccggttccaatagccagggcgaggtcgcgctgggtcaagccgagggcgcggcgcgcctcggcgacctgtcggccgaaatcctctgcagtgacgatcatagcgcttcttgccgatcgggaagatcgcagcagagcacgactttcgtcaaggctattcttaccgatcgggaagatcggctcgccccaacctcatcacgcacagaatcttaccgatcgggcagatccacgttttatgggctaatcatgggcaggctcctgcggagcagacccaaacatcaactaagtctttgaaaataatggtggacgcgacagggattgaacctgtgacccctacgatgtcaacgtagtgctctcccgctgagctacgcgtccgccgtggcggccctggacgcagggtccggggcgggaaggggcggtctataacccggggggttcccgaaccgcaaggggcaaaacgccgacgtcccttcggggcgcggtcaggcggcgaccatgcgctcgacctcgttgacgaggtcgcgcaggtgcacgggcttggacaggaccttggcctggggcgaggcctgggcggcagacagggccacggcggcgaagccggtgatgaacatgatgcgcagacccggctggcgggcggcggccacgcgggcgacctcgatgccgtccgcgcccggcatgacgatgtcggtcagcagcaggtcgtagggcccgtgctccagcgcgtcgatggcttcgtcgccgttctcgcagtcgatgacctgatgccccgcgcgctccagcgcgcgcgtcaggaaaccgcgcagggatccgtcgtcttccgccagaaggatgcgcgccatgaccgaatgcctcgtcgaaaacaggcgcggacgctagcggcggaacggtaaaccgcgcgtgaaaaaccggcggcccggctatgccgccggtggagaagcagcctatggcgacgggcatgagcccgtttggagaggtctgtcgcatcagtcgcccggaatcgggcgcggcttcgatcccgctggtgttcgcgtctgcgcactcgggcgatgtccatccgccctgcccggccgccgcggacctgcccgcccggagcctgcgcagcgccgaagacgccctgatgcagcatctggtcggcgccggacccgcccaaggcgcggtgctgatcgccgctgtgatcgcccgctcctttgtggacctcaatcgtgatccggacgagcttgacccgctgacggtggagggcgcgcccgcggaactcctgtccccgcgggcgcgcgccggctatggcgtcattccccggctgagcggcgacggtctggctctgcatcgacggcggctgacgcgcgaggaggcgcaggcgcgtctggacggcgtgcaccgcccctaccatgtcgccctggccgatctgatgcatgagacaagggcgcggcatggccgggcgatcctggtcgactggcattccatgcccagccgcgccggcgacatggacgtggtgctggggacgcggcacggcgccgcctgcggatcggcgctcagccgacagatgcaggggctgatggagaggcagggctggcgggggtcgctgaaccacccctacgccggcggttactccacccggaggtgggggcgccctgacgaaggcttcgaggcggtgcaggtcgagatcaaccgccgactttacctcgacgaggacacgcttgagccgtcgcccggctatggcgcgctcgcgaaggccctgtcgcgcattatcgcggaactgtgcggatcccaccggtgagcgcgggcaaaaaaaagccgcgccagaccggcgcggctatgtaaagtctatagggaggaaacgcccaggaagggcaagacgcccgaaggcgtcgaggagcaatctagatacccaggcccagctcgtcaagcctgaccactgataagttattcacggtaagttacaccgtgcgacgagacgacgcacgaaacgtgcgttctcacggggtggcgccgctcaaagcggaaaactcgtctattccagcagacgacgggctgcgcggatcgcacgcgctgcaggcgaagcctcttgccgccacagcagcagcgcgaaggccgagaacacgccggcggccagccacaagggtccaaacagccaggccgcggcggccagggcgaaatagtagccccgcacgccctgactgaacgacgacagcgccggattgatgagattggccgccgcctcgccgaaagccgtgttctcgcgctcgtcctcgggcgcggcgccgatcagcgccagggtgtagttcagctggcgcagcgcccagatgaagtccaggaacccgcgcgccaggcagatcagcaccagagccagcttgccctccagcatgcgcagcggcacgtcctcggcgcccacggcggcgaacccctgcagccggctttcgcccccgaacaggatgccggccacggcggcgatcagcagcaggttggtggaggcgaagaaagacgccgagttgatggaatggcccatcaactggctgtccacgagccgcatctcgcgtcgcgtcatcgcctgcatccagatgcggcgcacgtgcagcatgtcgtcgttcaaggagccgctcttgcggccgatcagccccaggagagggccgtagccgagccagcacacgaagaagagcgcgagagccgccccgtccagaaaggtcatgaccctcttcctgccgtgcgccgggccgccggtgcaagggccgccgcaggcgccgctgcttgcccggaggcctgcgccgtcctatcacgccagccgcttttccgctcaaagacatacagccaggcagacaccgccatgaacatcgacgccatctcggtcgggcccaagcccccctacgacatccatgtggtgatcgagatcccggccggcggcctgccggtcaagtacgagatggacaaggagtccggcgccctgttcgtggaccgcttcctgaacacggccatgtactaccccggcaactacggcttcatcccgcacaccctggccgacgacggcgacccctgcgacgtgatcgtgatcaatccgacgccggtggtgccgggcgcggtgatccgcgcgcgtccgatcggcgtgctgctgatggaggacgaggccggccgcgacgagaagatcctggcggtgccggtcgacaagctgaacccctactattcggacatccagagctacacccagctgcccaagatcctgatcgagcagatcgagcacttcttcacccgctacaaggacctggagaagggcaagatggtccgcgtcgacaaatgggccgaggccgacgtggcggcggagctgatcgagaccggcatgaagatgcacgaggaggccaaggccaagggcgaaaagacgctctgatcgtcatcccgccatgaggctgaagaggcgccctccggctgcggagcggcgcctttttcgtgcgacgccccgccctctcccgcttcgcctgcgcgcctcctatgtgcggggcatgacagacctttccccccgcgagatcgtctccgaactcgaccgcttcattgtcggccaggacgaggccaagcgcgccgtggccgtggcgctgaggaaccgctggcgcaggaagcgcgtgcccgacgacctgcgcgacgaggtcacgcccaagaacatcctgatgatcggacccacgggcgtcggcaagaccgagatcgcccggcggctggccaagctggcgggttcgcccttcctgaaggtcgaggccaccaaattcacggaggtcggctatgtcggccgcgacgtcgaccagatcatgcgcgacctggtcgaaagcgccctggtgatggtgcgcgaccgacgccgggtcgaggtgcgcgcccgggccgaggccgccgccgagaaccgcatcctggacgccctggtcgggccgggcgcgggccaggccacgcgcgacgccttccgcacccgcctgcgcgccggcgagctggacgacaaggagatcgagatcgccctggccgacaccgcctcgccgatccaggggctggacatcccaggcggccaagtcggcctgctgaacctgtcggagatgctgggcaagatgggcggggggcgcaccaagaccgtgcgcctgactgtgcgcgacgccacgggtcccctgaccaccgaggagggcgacaagctgctggatggggacagcctgaccaaggaagccctgctgctggccgagaacgaaggcatcgtctttctggacgagatcgacaaggtggcggggcgtcaggatcgcggcggcgccgacgtctcgcgcgagggcgtgcaacgcgacctgctgccgctgatcgagggcaccaccgtctccactaaatacgggccggtgaagaccgaccatgtgctgttcatcgcctcgggcgcctttcacgtcgccaagcccagcgacctgctgcccgagcttcagggccggctgccgatccgggtcgagctgaaggccctgacacgcgacgacttcaagcgcatcctgaccgagccggaggccaatctgatccgtcagaaccaggcgctgctggcgaccgaggacgtgacgctgaccttcaccgacgatgcggtggaggcgctggcagacgcggcggtggccgccaactcggcggtcgagaacatcggcgcgcgcaggctgcagacggtattggagcgggtgctggaggagaccagctttcgcgcctccgacctgggcggccagacgatcgccttcgacggcgaggcggtgcgcgaaaaggtcggcgacctggcgaagaacgccgacctttcgcggttcatcctctagcggccgtcaatccatcagctgctgggccaggtagacgtagtgccgggcccagcggcgggcgttggccaccggatcggcgtcgttggagtggccgcccgccgtgtcctcgaaatacaggtggtcgtggccctgctcgcccagacgcgcggcgaacttcctcgcatggccgggatgcacccggtcgtcgcgcgtgttggtggtgatgtagacgcgcggatagtcgacctcgggtcgcagctgctgataggccgaatattttgcgatccaggccgcctcttccgggatgcgcggatcgccgtattcgccgatccaggacgcgccggccggcagctcgtgatagcgcagcatgtcgatcagcgggctttcgatcaccgccgcgttgaacagctccggatgctgggtgatcgacaccgaggtcagaaccccgccgttggagcggccgtaaatgcccaggcggcgcggcgaggtgatccgccgctgctgcaggtcgcgcgcaaccgccgcgaagtcgtcgaaggctttttgccgctcgccgtccagcgccgcctggtgccagtccggcccgaactcgccgccgccccggatgttggcctggacgaagacgccgccgttctccagccacagcttgcccatctcgggcttgtaggccgggttcaggctgccctgaaaaccgccgtagccgaataggatggtcggcgccgaaccgtccatcgccaggtcgcgcgggcgggtgacgaaataagggatcctggtcccgtcgctcgacgtcgcctcgaactgctccaccacatgggtcgaggcgtcgaacttggccggcgccgccttcagctcggtcagcgaagccgcgccgacatcggcgaggctcagcgtctgcggcgtcaggaagccctgagccgacacgaaaacgcgtcctgtcttcttggatcggtcacccaggctgacagtgctgttttcaggcacctgaacctggcgctcttcccagggaaactcgccggcaggcctgaagctcgacaaccggctgcgcacgttgtcgctgacgacgaccatgagcctgtcgtcgaagacggcgacgtccgccaccgactgccgcgcggtcggcgtgaacacgatcgtgtcctcatgcgcgggtcccggcttgcggggcggatcgccgatccactcctgcagggaaccgatgttgatcgccagcaggctcccggctttgatgtcgtcgcccgcgccatagcggttgaacggctcttccggcgtgaagatcaaccgctcacccatcatgccgtgcaaggatacgcgcgacggcagcatcagcttcaccggctcgctgtccaccagccgccaggtttcggagcggaaggtgtccagcgggcgggtgatgatgacggccagcacctcgccgtccttgtcgcggtacaccgacgggctgacgccgtagccgccgtcgccctgctcgccacgatagacctctgtcgcgtccgccagcgcctgaccgcgcttcaaggtcttgacgatgaagggatagcccgactccgtcatggtgccggctccgaagtcggtggcgaccagcagggtgtcgcggtccagccattcgatgcggtgcttgccctcgggcagcacgaagccgttgtcgaggaaggtcttggtggtgatgtcgaactcgcgcaccgtcaccgcgtccttgccgccgtccgacagcatgatcaggcagcggtcgtcgtcgggcgccaggcaacttgcgcccttgaacacccagtcgcggccttccgccctggccagggcgtcgatgtcgatcagcgtgtcccaccggggcgtttcggtgcggtagctgtccagcgtcgtgcgccgccacacgcccttggggttcgtcgcgtcctgccagaagttgccgatcccgtcgcccaagaagctcggctgcgggatgcggtcggtggcggtcaggatcgcctcggcctcctggcggaacggctcatagcggcggtcgccgggcagtgtcgccagcgccttgcggttctcctcggccacaaaggccatggcctcggcgccgtccacctcttccagcgccagatggtcgtcggcggccttgaccccctccaccgtcaggtcgcgcggatagtgcggcggcggcggggtcgcggcggccgatgcggccgtcggcgtctgggctcgggatgcaggcgcggccgcgagcaacagggccgggatggcggcagacaggatcaggtgacgcatggctcaactttccgctcatccccgcgcaggcgggatccagacctttgggcgttcgacgtcgccagttcgtactcagttccgtcccagccgccgaactccacgagagaactgggccccgcctgcgcggggatgagcggttctgtagaacctattcctgcgccggcgtgtccatcaggcggcgcgacagataggtgtactccagcgccagccgccgggcggtctcgcgaagattggctcccgctgcgtggccgccgtcggtgttttcatagaacagcaccggatagcccaactcctccagccgcgccgccgccttgcgggcgtggccgggatggacgcggtcgtccttggtcgaggtgtggatgaacacctccggatagggctggccggccgcgagcttctgatagggcgagtactgctcgatccaggcgcgctcttccggcacgtcggggtttccgtattcgccgatccagctggcgccggccaaaagcttgtggaagcgcagcatgtcgaacagcggcacctggatcaccgcgccgttgatcaggtccggccgctgggtcagcatcgcccccatgaacagcccgccttgcgagccgcccatgatcgcaagcttgggctgtgaggtgatgcggcgagccgtcaggtccagagccacggcctggaagtcctcgtgtgcgcgctggcggttctcttgcagcgccgcatcatgccagcgcgggccgaactcgccgccgccgcgcgtgttggcgatcacataaacgccgccccgctccagccacagcttgccgaccgtgggcgaatagccgggcagcagcgagttctggaatccgccatagccgtacagcagcgtcgggttggagccgtccagcgcgatgtccgccttgtgcaccacgaagtaggggatcatcgtcccgtccgccgagcgcgcctcatactggtccacggtcatgccggaggcgtcgaacttggcgggcgtcgacttgacctgctcgacctgcccgctcgcggcgtccgccagatacaggctggacgggttcagatagcccgagacgctgacgaacacgcggtcgtcggcctccgaggccgatcccacgccgaccgacacattctgcggcagatccagcgtgctgtaggcccactcgccctcgcccggcgtatagacgcgcaccgcgcccttcacgttctcgaacagggcgacgatcaggcggttgcggctggcggtgatcccctccaccgcctggcgctcggtcggacgcagcaccagctgggcctgaacgctgggatcgtccatccacgccttgagcggataggcgatgacgtcgccggactggaaggtctggccggatggcgcggtccagtcctccttggtggtgaacaccagccggccgtccaccagggcgttgatgtccgacttggccggcaaggtcagcttggtcagctgtccgtcgtcccccaggctgaagacctcgctggagtagaagtccaccgcacgggtgatcagggtcgcctggatgttcccatcggcgtcgcgcagggtcgagccctgcaccgacacgtctgtcggctggccggtgaagagggtttcagcctgctccatcggctggccgcgcctcatgcgcttgaccaccatgggatagcccgagttggtcaggctgccttcgccgaaatcgcgcgcgatcagcagggtgtccgcatcgatccaggccgcattgcccttggattccggcagcacgatgccgccgtccacgaacgtcttggtctcggcgtcgaactcgcgcagcgtcaccgcgtccttgccgccgtccgacagcgacaccaggcacagccgctcgttcggctgcaggcagttgacgcccttgtagacccagttcttgccttccgccgcggccagggcgtcgatgtcgaggatggtctcccactcaggcgtttcggtgcgatagctgtccaccgtggtctggcgccacacgccgcgcacatgctgggcgtcctgccagaagttgctcagcgtgccgtcgcggttgaagccgacgcccgggatgcggtcgcgcgcctgcacgatctccagcgcctgctggtgcagcggctcgtagcgggcgtcggcctgaagcacgcccagcgacttttcattgtggtcgcgcacccattgcatggcgcgctcgccctcgacctcttccagccacagataaggatcggtcgcatcggtcgttgcgaaggcggccgtcgccgacgaggaagagggtgcggcttgcgccatggcgatgctcgacagcgaggtggaggcgagcagcgcaacgagcgctgcggcggaggtgcggatcatgtgcgtctttccccgaaaatctggggcgcaccttaaacggcggacttggctcggcaagccgcgcacgcattttgtcacgtcgggccgtcagccctcatccggaatgcacaggaggtttccgcaggccttgcagtggacggcgtccggatcgtggttctgcaagccgcatcgctcgcaagggtgacgcaccttgtgcggcttgatcactgtctgcgccaccctgaggaacagggtgatgcccgtcagcatgatgacgatggacagcagcttgccgagcggaccgggcaaggtcacgtcgccgaagcccgtcgtggtcagagccgccactgtgaaatacagcgcgtcgatgtagcccgcgatgccgtcgtgccccctgaacaccgcataaacaaagccggtcgccacaaacacgaaggtcaccagcccggccatggcgcgcacaatggcctcgacccgagtatcgtcgaacttctggcccaccgtgcgccagaagagttctgagttgagcagcgtccagagccgcagcatgcgcagaaagcccaggttggacacccaggcgggcaccagcagggtcaacaggatgaacaggtccacccagacgatgggccgcttcagccaatccttcacatcagaataggcccaggcccgcgccgcgagatcgacggccagcagcgccgcgacgatgccgtccaacacataaaaggcccaccccgcctccctcaggatcggagcggccagaaaaaaggcgatgatcagcacgtcgacgacgatcacagccatgcggaaccggacggccggcggctgggagccgtggtagagatatcgcagtcgcgcccgcaggcgcaggccctctccgttcccgtggctcggatttccagacttcacgcggttctccgaaggcacgggcggcgctatagcacgggcatgacacgccccttcgtcaagatgaatggcgccggcaacgatttcgttgtggtcaatgcgttggaagcgccgttttctcctacggcggaccgggtgcgcgcgctcgccgaccgctcaaccggtgaaggtttcgaccagttgatcgcgattgagccttcggacacggcggacgctttcatgcgggtgtggaacgcggacggctcgcttgtgcagacctgcggcaacgccctgcggtgcgtcggctggctgctgatgcaggcgaacggctcggatcgggtggtgatcgacactctcggcggcccgaccgtcgccgtgcgcgccggcgaccgcagcgtcaccgtggacatgggccggccgcgtcttgactggacggaggtgccgctggccgaggagatggacacgcgcggcatcgagcttcaggtcgggcccatcgacgatccggtgctgcacacgccgggcgcggtctccatgggcaatccgcacgtggtcttcttcaccgaccggcaggacgacggcttcgtcaccggttcgggctctctggtcgagcatcacccgcttttcccggaaggggtcaacgtcggcttcgccaatgtgctggaacgcgatcacatccgcctgcgcgtatgggagcgcggcgccggactgacacgggcctgcggcaccggcgcctgcgcggcgctggtggcctgcgcccggcggggtctggcggagcgcaaggcgcgcgtgaccgtggacggcggcgaactggtgatcgactgggacgaggcgtccggccatgtcttcatgaccggcccggtcgagatcgaacgcaccggaacgctggccctctgacgccgggctgtcggagatcgggctcgcctgagcgcacggcgttccgtcgggtaaactgttgttacggccgccgggcggttctaggactggcggacacccgccgcctgcgcctggaccaccaatgcccgacctgaccgacaaacagaccttttccgacaacgaggcgctggacttccacagcgagccgacgccgggcaagatctccatggcgccgaccaagccgatggcgacgcagcgcgacctgtcgctggcctattcgccgggcgtcgccgtgccggtgctggcgatcgccgccgatgcggacaaggcctacgactacaccgccaagggcaacatggtggcggtgatctccaacggcaccgccattctaggcctgggcaacctcggccacatggcgtccaagccggtgatggagggcaagagcgtgctgttcaagcgcttcgccgacgtggacagcttcgacgtggaggtgaagaccaccgatccggccgagttcgtcaccgtggtcaagaacatcggcgacacctggggcggcatcaacctggaggacatcaagtctccggaatgcttcgtgatcgaaagcgagcttcaggacctgctggacattcccgtcttccatgacgaccagcacggcaccgccatcatctccaccgccggcctgatcaacgcctgccatgtcgccggcaagaagctggaggaggtcaaggtggtgctggcgggggcgggcgccgcggggctgtcctccatcgccctgatgaaggcggcgggcgtgaaggccgagaacacggtcatcgtcgatcgcgacggcgtggtcttcaaggggcgcgcccacggcatggcccagtggaaggccgcgcacgccactgacacgccgcaccgcaccctggccgaggccatggtcggcgccgacgtggtgctgggcctgtcggccaagggcgccctgaccaaggagatggtggcctccatgggaccgcgcccgattatcttcgccatggccaacccggatccggagatcacgccggaggacgtgatgagcgtgcgctcggacgccatcatcgccactggccggtccgactacgtcaaccaggtcaacaacgtcctggccttcccctatctgttccggggcgcgctggacgtgcgcgcgcggcgcgtgaaccacgagatgaaggtggcctgcgcccgcgccctggccgcgctcgcccgcgaggacgtgccggacgaggtcgccgccgcctaccggggcaggaagctgaagttcggtcccgactacatcatcccgacgccgttcgacccgcgtctgatctggtacatcccgccgttcgtcgcccaggcggccatggacacgggcgtggcgcgccggccgatccccgacatggacgcctaccgcaccgagttgcgatcgcgcgtcgatccgtcggcggctttgatccagaagatttcttcggccgtgcgcagcgggccgaacaagcgggtggtgttcgccgagggcgaggagccgtcggtgatccgcgccgcctggggcttcaagcaggccgagctgggcacgccgatcctggtcggccgcgaggacctgatccgtcagaatgcccaggaagcgggcctgaacttcgacgaactgggcatcgagatcaccaatgcgcgggtgtcgggccgcaacgtcgaatacaccgactggctgtacgaaaagctccagcgacgcggctatctgcgtcgcgacgtgcagcggatgatcaaccaggaccgcaactatttcggcgcgaccctggtggcccagggcgaggccgacgccatggtcaccggcgtcacccgcaacttcaacatggccctgcgcgaagtgcagcgcgtgctggaggtcaaggagacgctggtcggcctgtcgatcctgctggccaagggccgcaccctgttcgtcgccgacacctccatccacgaactgccggacgccgaggagctggccgatatcgcgtgtcaggccgccgcgtcggtgcgtcgcctcggccgcaatccacgcgtggcgttcatgtcctattcgaccttcggcaacccgccgggcgatcgcggcgagaaggtgcgcgaggccatccgcatcctggatcgacgcggcgtcgatttcgaatatgagggcgagatgccgccggagatcgcgctggatccggccgcgcaccccgcctacgccttcaaccggctcagcaagcccgccaacgtcctggtcatgcccgccattcactcggccgcgatctcgaccaagctggttcaggcgctgggcggcgccaccgtgatcggcccgctgctggtcgggttggagaagtcggtgcagatcgttccgctgggcgcctcggtcagcgagatcatcaccgccgccaccttcgccgcctaccacgaaggcccggtgttccacggcgaaggcgtctcctcggcccccaggccgcccgcgcccttcatcgaggactgagcggaagcggcttgaggcggcggggtccggctggcacggtcgggcgatgaccgacaccgcctcccctttcccgcccacggccccgcccgcccggcgcgtggggcccggcctctatctggtcgccacgccgatcgggaacctgcgcgacatcaccctgcgtgcgctggatgtgctggccgccgccgaccttgtgctggccgaggacacgcgggtcaccgccaagctcctgcaggcctacggcctcaaggctcgcctcgagcgctgcgacgaccacgcctccgcgcgcgccgccgagatcgcgctggagcggctgcacgccggcgaggtcgtggccctggtgtcggacgccggcaccccgatgatcagcgaccccggcttcgtggtcgcccgcgccgccatcgccgccggactgccggtgcacccgatcccgggcgcgtccagccttctggccgccctgtgcatcgccggcctgcccgccgaccgggtgctgttcgcgggctttcttccgcccaagtcggccgcgcgccgcaccctgctggagagcctcaaggcgcccggccagacgctggtcttcttcgaaagcggtcctcgcctggccgacagccttcgcgacatggccgccgtgctgggcccccgccccgccgccgtcgcccgcgaactgaccaagctgtacgaggagtgcgtgcgcggccccctcgacgccctgtccgccgatccgcgcctgcaatcgcccaagggcgagatcgtggtggtcgtcgcgcccggagaggccgaagcggtgtccgaagccgacgccgacgccgccctggccgaggccctgacccgcctgccgccgggagaggccgcgtccgaagtctcgcgcgccctcgacctgccgcgcaaggcgctctaccgccgcgccctggacatgcagggacggtgaagccacagcgcctccgtcccgccgcccggccgcccgcgcccaagaggccgtggcgtcaggcgctgggcggacacgcccgtcggcagggacacggcgccgaatggatcgccgccgcctggctgatgctgaagggctaccagatcctcggctttcgcctgaagacccgcgccggcgagatcgacctcctggcccggcgcggctccgtcctggcggtggtcgaggtcaagcgacggcgcaccctggtccaggccgaggccgctctggccgccgaccagtacgtccgattgctggcggccggcgaggcggcgatgcgcaatcgcccggcgctgcaggcccttcgcctaagaatcgatactgtggcgctggctcccggtcgttttccacggcatctttgtggcgttgaccgctccgcgcccggagaccggaggatcaggtgacgcgagaggaagccgaggacatcctgacgcaggcgggtccctgtgaggacggcgacttcccgctgctggaagcggccatcgcctgcgccctccacgactatcctcttcgcgactgcgaaccggtgcgggggctggcccgcaacgccggcgagcggctgaaggagcggatcggcggcgaaagccccgacgacgccctcgccgagaccatggccgccgacctgcggctgaacggcgacctgatcagctacgaccatccctgcaacaccgacatcatcgacgtggccgagcgcaggcggggcctgtcggcggccctggccatcttctacctcgacgccgcccggcgcgcgggactggaggctgcgggcgtcgatttccccggccacttcctgatgcgggtcgagacgccggacgggccggtcgccctggacccgttcagccagggccggctggtgctgcccagcgagctgacccgccgcgcgctgcgggccggcctcacgccccatgtggccgaccggctggacctgctgatggcgcccgtcagcgaccgtcacgccctgatccggctgcagaacgtgctgttcagccgcgccatcaaggccagcgactacgaggcggccgaacgatccgccctgcgccgcgccctgctggacccgaccgaccaccgcccgtggctggatgtcgccgccgcgcgtgagaagcagggcgcattggccggcgccctggacgccctctcccgcgcccgcagcctggacggtccggccgaggccctgcgctcgaccagcttcgatcgcgtgcggatgcagctgaactgacgcatccgtccgggcgaggcggtcgtaaatacctcaaccattcccgtgggttgcctgaagccggaacggctttgttcatgtcccgttcaactacgaagcgcgataacggtcgccttaggagatcatccatgaaaaccccctcgctgaagaccctcgcgctggtcgcgacggcgggcctgatgctcgccgcctgcgccaccgcgacgccctatcaacccgccggcttcaacggccagcgcaacggctacgccgagcagcggctggagagcaatcgcttccgcgtcagcttctccggcaactccctgacctcgcgcgagcaggtcgagatgagcctgctgctccgctcggccgaagtggcggccgagaacggctacgactggttcgccacggtgaaccgcgcgaccgagcgcgacacccgcttctactccacgcccgaccccttctatgaccgcttctacggtccccgcttcggcccctactggagcccgtcgtggcgcttctaccgtcgcggctactggagcccgtggggtccgacctggggcaacgacttcgacatccgtcaggtcgaccgctatgaggccaacgccgagatcatcctgggccgcggtcccaagcccgccggcgatcccaacgcctttgacgcccgcgaggtgatccagaacctcgccccccgcgtgacgcgtccgtcgtaaggacgatcatctcctccccgtcgtcccgcgatggggagggggaccgcccgcgcagcgggtggtggaggggttcctgacggctggcaacccctccgtcgcggcgcaggcgcgccgcgccacctccccacaggtggggaggagagttcaacccgccttaaccaacgcgcggggtcttcagacggcgcttgttggcgtgggtggcgggcgcctggcccatggcctcgggcaactcgcccttgaagtagaagcgctgccacgcctccttggccgcgtccgggtcgccggaggccaggcggttgttgaaatcggtgcgctggcggttccaggcgtcgaactggtcgcgcatggtggggttggaatccaggctgcggatcaccggctggaactgctccaccttcttgtgctcgatcagattgatgaagcagaagggctcgcccttttcgaacttgatccgccctggccgggtgaagatccagttcatggtgaaggggaacggcagccagtcggtctcgatcaggccgaccagcggctgaatgccgtccttcacatggttcggcgagcccgagcacgtcatcccccagcccggcggcgtgcggaacagatactgcggatgcatcgtcaggacgccgcgcgagaagtgcgaggtgacgaagtggtccagatccgcctgcggccggtcgggtgtgatggtgatgtcctcctggcgcggcccgccgttccattcggcggcgaagccgaacgggcacaggatttcccatcccgtggtgttggccatgttcagcggcaggcagcgataggggtggcggctggcgaaggcgtccatccagttgcgcgactggcggcccggcaccaggtccggcggccgcgccgacatcggatagcactccagttccaacgggcggttttgaacgctagtgaccatggcctcttcgtaacgcgccgccgatgaccgctcaaccgatgcccgctcccttgttcgaccgcacggcgctggaagcctggctgacggaccacgccatccccttccacacggtcgaacacccggccgtgttccgtgtcgaggagggcctggacctcaaggccgacctgcccggcgcccacaccaagaacctgttcctcaaggacaagaagggccggctgtggctgatctcggcccgtcaggacacgctcatcgacctgaagcgcacgcccgaggccatcggctcggaccggctgtcgttcgcaaacgaagccctgatgcacgagacgctgggcgtccgccccggctcggtcacggcgatggccctgatcaacgacacggacgcccgcgtcacctttgtgctggatcagcgcctgtgggaggccgacctcatcaacttccaccccctcaccaacaccgccaccaccgccctgtcgcaggacgcgttccgccggttcctgagcctgctggggcgggagccgctggtggtggacttcgatcagcttcgggccgagtccgctggcggggagcggggcgacttccgagttcgacccgttgcggcccctcgacgacggctgcttacgaggagggtgctagaacgcggtcaatccgttgcgcgcaaagcgatcttcgttaatcatgagcatctcacttgagggttgagaatggctgggttccgcgtcgcgcttcgttctgtgaaaatagccactcataccgccttgtatctggtatcggcctttctgctcgtgaggcttggacaaggcttcatcgacggcctattcggcggctaacgtccgctttccacccccagtcgaagttgcgaagttccgctcctcggcattgggggcgcggttggcggagtgggcgtttgctgcgcctacagcttcgtcctgagcgaccacagctcgggaaaacagcggcgggtcagggtggaggacagatagccgacgccgtcggtgccgccggtgccgcggcggcggccgatgatgcgctcgaccgtgaccacatgcttgtgccgccaagtcagcagggcgtcgtccagatcgaccagcttctcggccagctgatacagcgcccaccagcggtcggtgtcgcgatagacctcgagccacgccgcctcgacggcctcggaggccccatacgggcggctgacgtcgcggtgaagcaccgcgtccggcacgggcaggccggcggccgccagctgatgcagggcgtcgtcgtagaggctgggctcgcgcagcgccgtcgtcagggcggcgtgggccgccggccgctcctggtggaagcgcaggaagctgtcgtccttgagccccagcagatactcgacccggcggaactgatcgctctggaagcctgaggaggcgcccagcacgcctcggaaccgcaggtagtcggccggcgtcatggtggccaggatgtcccagctctgggtcatgaccgactggatgcggctgacccgcgccaggctcttgtaggcgggcaccaggttccctgcgcgcaccagcgtcttggccagggcgatctcgtgcaggatctgcttgagccacagttccttggtctggtggatcacgacgaacagcatctcgtcgtgctggtccgacagcgggtgctgcgccgccaggaggtcgtccagcgccagatagccggcgtaggtaatgcccgagggcgaatggggatcggcgctcatggcgagaggcctaacgcgtcggagcgcgccgttgcaagcgtctgcgcctcagggctggccggcgcccagggtgttctcggccatttggcgcgagccgccaaaggcgtcgcgatcgcctttgtagatgaatccgtaggtcggatagatcgtcgagcccaggtcgttggagggcttgtaccagaccttgacctgcgaccagtcgttggaggtcgagacgtccaccacggtgacgttctcctcgaccttgccgcggctgccgccccagttggcgtgggtcacgcgcacgacgcggtcggtcaggatgtcggagacgacggcgacgtggccccggctcatgcggccctcggggcggaacaccagaacggagccggtctcaggcgccttgccggtgcggaacttgtctgcggcctggcgccaccaggtccaggcgtcgccgaagatgttgatgcccgagaacatgcgggcgaaggtgacgcactgccaatacggatcatcggcccgggcggcggcgggcgtgacgctcaccgcaaaaaatccgagactcgccgcaaccagagcggtcttgatccgtttcgtcatgctgtgcctgcgtgaagacgtccccgtaggaccgttgctaaccgatacaggcggagtgttgaagaactgtttcagtgtgtcacaacggcacgccgacgggggttgacgcgattttccggcgcctcgccatcgccttcaaagccttgcgggccgggtgttcgaccagatggtacgacgccgccgcgacgaccggcaaaagcgccagaacggccaaccacacaaaaagttgaagctgcttgtccggcgcgcccgtcgcccgcgcggcgaggttcacggccaggagcttccacggcacgcagaccatatagaccgagtagctgatctcgccgagatacacggccgggcgcgaggccagccagcccgcccgcgcgttcggcagtgaggccagagacaggatcaatccgcccgccagcaggaccgtgatcccgtcccacagctgcagcgcggcgcttgtgaccagcaggaccagaaagacggcggccagcagacccgccggccgcgccggctggcggcggtagacgaggtaaagcgcgcagccgaacaggaagggcggcacgatccgcaacgcgccccagcggatcgtcgcctcggtcagcgaaaagccggccagccgctcgaacacgacatagaggagggccagaaagccgcccgccaggatcactgcgatcagcgggcgctcgcgcattcgccaggcgacataggcgaaggcgggaaagcacagataggcgaaccactcggccgagatcgaccaggacgggtggttccagcccgcgaccggagccagaccccaggcgtgcaccatcagaaggttcgccggcagcgacgaccagctcagcacattggcgtccacgttcagcccgacgacaagcgccgctccggccagcagccccaccccgaccagcgtcgccagatgcagcggatagacccgcgcgatgcgcgcccacagaaagccgcgataggagaaccgtccctcccccgccggcgccagatagacgtggcaaaggatgaagccggaaagcacaaagaacagctcgaccccaaggtagcccttggccaccaggcccggcatggcgcccgctccggccaggttctcccagaaggtgtagacggccacccaggcggcggcggcgaagcgcagggcggtgatcggccgaaggtcggcgggggtctggaccggggtcatgtccgaacctgtaagcccccaccggttccgattccgtgaatcgccggtgtgcggaggaacgctagtccgcgtccgcctcgatcgcgtcgatatcgtcgtccgacaggccgaagtggtggccgatctcgtggatcagcacatgggcgatcagatcggacagggtcacgtcgccgcgctcgcaccattcatccaagatcgggcggcgatacagaaagacgcgcgacggctcggccgccggccccaggccgtcgcgctggccgatgtccacgccgtgatacaggccggtcagctcgaagggatcctcaatgccgagatcctccagcgtgcgctcgtcggcgaagtcgtcgatgcggaacaccacctcgcccgccgcctttcggaacggctcgggcagggcgtcaaaggcggcgcgggcgagacgggcgaagtcgtccagcgacggcgcgacctgatcgagcgaggcgggggtgttcatgcgccggatgtaggatcattccgcacagcgccacaaggcgaccgaaggccgccgctcatccatctgcgggcgcatcgcttttcacctgtccggggtatggtaaacgccgaatcgggcgcacgccgccttctggagacaccgaacgtccatggccgaggccgacatcgcctatgtcgcaaccgcgggcgcggccggcctggcccttgcggtcagcgcctgggccgtgcgcctgcgcgcgcggctgcaggcccaggccgcctccgacgcccggcggctggagacgctgcaggccgagctggccggccgcaacggcgcgctggcggccatggacgagatcagcctgtccctgacgcccgagggcgacgccgacgccctagccggaccgccggacgcggccgccgccctgaccggagacgcctgggcctcgccggacgccgtgctggcgctgctggcgccgacgcaggacgagcgcattcgcgccctggtgcaatccggcgagccgttcgacgccctggttcaggcgccgggcgacggccggccctggcgcgtggcggggcgggtggccggcggcgcggcctggctgcgcctgtcgccgctggagaacgccctgcccggcctggggagcggcgacgcggccgagagcggcctgggcgttctggccgacgcctcgcccgtgcccacctgggtgaccgacgccgccggacgcctggcctgggccaaccgcgcctggctgagcgaggtgcgcgccgccgacctcgccgaggcgcaagagaagggcctgacctttgatcgcggcgcagacgccctggtggccgaggccatgcggctgggcgttcgtcaggaaggcttccgctggaccacggggggcggccggcgtcgcgcctggcgcatcctggccgagccggctgcgggcggaaccgacgccgttctggcctttgcgctggacatgacggaggccgaggagacccgcgacaccctgcgccgccacgtcgaggcgcatgacgagacgctgaaccacctggcggacgccgtggccatcttcggccctcagcggcggctggcgttccacaacaccgcttttcagaccctgttcgacatcgatcccgcctggctggacgagcgccccacccacgccgagctgctggaccggctgcgccagcgtcgccaactgccggaggtcgtggattacgccggctggaaggcgcgcgagctggagttctacgaggcgtcggaggccgcgccggacgacagctggtccctgcccgacggccgcacgcttcgggtggtgcgccagccgcacccgctgggcggcgtcctgctgctgttctcggacatcaccgatgagctgaagctgcgcagccgcttcaacgcccagctgcaggtccagaccgcgacgctggacaagctgaacgacgcggtggcggtgttcggctccgacgggcggttgcgcctgcacaacgaggcgttcgagaccttctggaacctgtcgggcgagcggctgtcgcaggcgcgcgacttcgacgccatcgccgagctgtgcaaggcggttctgcccgacccggccctgtggctggggctgaaggcgcgcgtggccgatcccgatccggaaagccgcgtcgccatctcgggcgagagccgcaccgccgacgggcgcatggccgcctggcagacacggccgctgccggacggcgccaccctggtcgccttctccgacgtcaccgcccgccgcaagctggaaaaggccctggccgagcgcgaggcggcgctggccgaaagccaggccctgaagcgcgagttcgtgggcagcgtctcctatgagctccgcacgcccctgacgaccatcgtcggctattccgaactgctggagacgctgggcgacctgcccgagcgcagccgccagcacgccggcgccatccgcgtcgccgccagccacctggcgcgctccattgacgacgtgctggacatggcccagatcgacgctggcgagatggagctgtcgctgggcgacctgcgcgtctgcgacctgctggacgaggcggcggaaaaggtccgcgcgcgggtcgagggacgcggcgcgacgctgaccgtctcctgccccgagagcctggcgccgatccgggccgacgccgcacgcatcggccaggcgctggatcacctgctggacaacgccgcgcgcgcagtgggcgaaggcggggcggtgtcgctcagcgttgagcgcgggccctcggaggtgcgcatccgcatctccgataccgggcgcggcattccctatcacctgcaggcccacgtctttgaccgcttcgtgcgccgcgagcgcggcgggccgggcgtcggtctggccctcgtcaaggccctggtcgagctgcacggcggcggggccgaggtggagagcgagccgggcaagggcgcgaccttcatcctgcacctgccgctccgcgccgatccggtgaacgccccgcccgagctggtgctggaggacggcggcgccgtctgatcgcaagcgtcgcgggcttcagccgctcgccggccgatccagccacgacagcacgcccgccgccgcgaccgcacccgaggcgaagctcgcctgcagcagatagccgccggtgggcgcttcccagtccagcatctcgccggcgacgaacacgcccggccgcctccgcagcatcaggttctcgtccagctggtccagccgcacgcccccggcggaggagatggcgcggtccagcccctgcatggcgaggagccgcagcggcgtcgccttgacccgttcggcgagggccgcaccctgcgccggcggatcgcccgcctcgcgcatcagggcgatcgccagcgggtccagccccgccgccttgcgcaggtggttcgacaggctggccttgccgcgcgggcgctgcagccgctcggtcagacgacctaggctcagatccggcttcagatcgacggtcagcaccgccgcgccgtccgcctcgatggcgtcgcgcagcgcggccgacagggcatagatcgctccgccctcgatcccgtaggtcgagatcaccgcctcgcccctcaccgtccggccgccgaaggaaaaggcggccttcagcggccgaccggcgaagcggagcttgaaggcgtcggaccaggccacgtcgaagccggcgttggcgggtcggaacggcgcgacctcgacgccggcagcctccagccacggccgccaggcgccgtccgatcccagccgcggccaactggccccgcccagcgccagcacgacggcgtcggcctgctccagccgctcgccttcaggggtttgcaggaccagggcgccgtcgcgccacccggtccagcgcgagcgcgtgcgcacctcgacgcccatcgtctgcagccgctccagccaggcgcgcagcagcggcgaggccttcatcgcgcgtggaaagacccgcccgctggagccaacaaaggtcggctggcccaggccttcggcccaggcgatcagctcggcaggagagaaggcgtcgatccaacgcgccacctcgcgcggctcgtcgccgtagcgcttgaggaacgcctccagcggctcggaatgggtcaggttcagcccgccgcggccggccatcaggaatttgcgcgccaccgagggcatgcgctcgtgcaccgtgacccgcacgcccgctccggccagccgctcggccgccatcagcccggcggggccggcgccgatcacggcgacatggcggacgggagaggaaggatcggtcatccgtccagcctttgccctgccgcgcctgcgctggccataggcgacgccggtcgccatatgacggcgatgagcgtagccttcacccgcgaagaagatctggaagccaccgccgcggaccttccggaccggccgatctcgccgcatccgaatctggtcacccccgagggtctgcagcagatcgaggctgagctggcctcggcccgcgccgcctatgcttcagcccaggcgaaaggctccatcgagagcgaccgcaccgccatggcgcgggcgactcgggatctgcgttattggtccgcgcgccgcggcacggcccagctggtggagccagtcgagggtgacggggccgcccgcttcggctcgcgcgtgtcgatcgtgcgcgaggacggccgtgaacagacctggcggatcgtgggcgaggacgaggccgatccggcgcagggcacggtcagccacgtgtcgccgctggcgcgcgcgcttctgggccggcgcatgggcgacgaggtgtcggtggccggtcagacggtggagatgaccgccgtcgactgaacgggatcagtcctgctcggcctcggccggcgcgacgcccgccatctcgcggatcatctccagcaccagcttctgcttgcgcaccggcagctgcggcgccaggcgcgcgatctcgatggtgtgccgcgtcgccgggaagtcgtggtcgaagcccgaggcgcggccgtcgccctcgtcctcggccatgcccgggttgaggccctcgtagaaatagccgggctggacgccgaaaaagcgagagatgtcccagagcttggacgccgagatccggttggcgcccttttcgtacttctgcacctgctggaaggtcagccccagcgcacgacccaggtcgctctgattgtagcccaggctgatccgcttttcgcaaaccctgcggcccacatggcgatccaccggatggggaccgtcttcgcctgtgcctctggccattctcgcctcgttcgtctcgcgcgttggcgcgccttaacagctttgccttatacggtcacgcttgtcgggcggtttcatggccctttcaactttcacgtgccggcgggcgcccagcgcagctttttgcgggcggccggaaccccgcctgcgacgccggcgacgagcagcatcaaccagaacaaggcgtcgccccagcggccaaagggcgtcacgccggtcggctccggcaggggcgcgtcgatcacgcccatgacgccgggctccagcctctggccgtccacgatccggccccagggatcgatcatggccgacacccccgtgggcgtggcccgcacgatcggaaggccggtctcgatagcgcgatagctggcgaggttcaggtgctggcgcgggccggatgtcttgccgaaccaggcgtcgttggacgcattgacgatccagcgcggccgatcctcgccgcccgccgtgaagcccggatacaggctttcatagcagatcagcggctgcacgcgcggcgcattcggcagatcgatgggcgcaggcgtcgggccggcgctgaagtccgagggcacatgcaccagactgcgtacgcccagcgtgctcatcagcccgcccagcggcagatattcgccgaaggggaccagccggtgcttgtcgtagacggaggcgatgcgcaaggcggcgccctcgtcgtgcagggcgaacaggctgttgtagtagcgcgcgccgtccggcgcatcggacgcggcctcgccgcgcgacagccccatgagcagcgtctggcccggccgcatcgcctcggccagcgcctggccgtcggcggaggcgaacacgtcgttggccgtggccggcagcgcgccttccggccacaccaccacgtcaggcaaggtctgaccaggctgcgacgtcagcgtgagatagcgctggacgatcgagcgataactgtccggcgaccatttggattcctgctgcacatccgcctggacgatgcgcacggtggtgtcggtcagccgcagctgcgcgcccgacagccgcgccatccccccggcgaccagcgccagcaagaccacggcgcccgcccccgccgagatccaccgcccgcgccgcccgcccggaccgatcagcagcgcaaaggcgcaaacggccgcgacggtcagcaggctgaggccatagaccccggcgaccgaggcgaactgcgacacggtgccccctgcacgccagctcgcgcccgccgggttccacggaaagccggtcaggatgttgccgcgcagccattcgaacagacagaacagagccgcgaacagcagcacccgccgcgcgcccagcggcgcgaacctgcgatagagggcgcaggcgcatccccagaacagccccagccccgccggcaggaggctggccgcgaagggcgccatccaggcctgctcgggattgacgaaaaaggcctcggccacccaccagcagccgatgaagaaataggcgaaacccgccagccaccccatccagaaggcgccgcgcggcgtgtccgagcgctcgctcaggatcatcagcagcggatagcctaagaggcccggcagcacgccgaacggcggatgcgcaaacgccgcgcccgcccccgccagcagcgccaacccgatccgcagccagcgcaggaacaccgtgcgccgacgctcgggccacgccctcaccctggcctgcaccgcctcaaacggcatggtcgccccggtacggatcggcgaccccgaggtcggccagaatggcgcgctcctcgccctccatctcctcggcctcggcatcgtcctcgtggtcgcgccccagcaggtgcagcacgccgtgcaccaccagatgcgtcaggtggtcggacaggcttttgccctgagcctcggcttccgtggcgcagacgccatgggccagcaccacgtcgcccaggtgcggcgcggcgctctccgcggccgggaaggacaggacgttggtcggcttgtccttgttgcggaaccgggcgttcagcgcctgcaccgccatgtcgtcgctcaacagcaccacgacctcgcccttgaccttgcccagagccgcctcgcccgcgcggcgcaccctggcctcgacgtccggcagggcttccagccaggcgtcatgctcgatctcgacgtcgaccgtcatccggcgtcttcgaggtcgggccccgggcggctgcgggcggcgtcggcgtcataggccttgacgatccgctccaccatggcgtggcgcaccacgtcggaggccgcgaacttcagcacccccacgcccttgacgccctccaggatacgaagcgcatgcggcaggccggaatcgcgcgcgttcaacaggtcgatctgcgacgggtcgcccgtcaccaccatgcgcgcgccctcgcccaggcgcgtcagcaccatcttcatctgcaggcgcgaggtgttctgcgcctcgtcgacgatgatgaaggcgtggctcagcgtgcggccgcgcatgaaggcgatgggcgccgcctcgatctcgcccttgtcgcgccggcgctgcacgtcctcaggccccaggatctcgttcagagcctcccagatcggcgcaagataaggatcgaccttttcgttcaggtcgccgggcaggaagcccagcttctcgcccgcctccaccgccggccgggtgatcacaagccggtccacctggccccgacgcagcagcgatgcgccgtaggccgccgccagaaacgtcttgccggtccccgccggcccgacgccgaagctcagctcgcagcgccccagcatgtcgagataggcggcctgcgccggcgtcttgggcacgatggcgccgcgcttgccgaccggcagcgacacgccggccagcgccatgccggcgcccttgccgccccgcacgttcgcaagcgccgtgcgcacgtccgcctccgtcacctcggcgcccacctcggagcgcttggccagatcctcgatcacggtgcgcgcatcctggcggtcgcgcgcgccgccgttgatggagacgccgccgcccggcgcctcgaccagcaccttgaaggcgtcctcgatcagcgcgacgtggcggctgttcggcccgatcaccgcccgcagctcggcgtcgttcaggggcaggaattcggagtctctcgccattcaggctgctttgctttctgcattgaggacgttcatcgtaagccgcccggtcagactgttctgctggccgctgacgatctcgaccggaacgatccggccgatcagatgatccgcgtcctcgacgtgaaccgactgcagatagggcgagcggccgatggcctgggcgccgtggcggcccttcttttcaaacagcaccggcagcacgcgccccgcctgggatgcgttgaaggcgacctgctgctccagcagcagcgcctgtagccggtgcagccgcgccttggcgacctccggctcgatctgcttgcccatgccggcggcgggcgtgcccggccgcggcgaatacataaaggagaaggccgaggcgtagcgcacctgccgcaccagatcgagcgtgtcctcgaaatccctgtcggtctcgccggggaagccgacgatgaagtcgccggacagggccagatccggccgggcctcgcggatgcgggcgatcaggtcgaaatacttctggcggccatgcttgcggttcatcagccgcaggatgcggtccgagcccgactgcaccggcaggtgcagatagggcatcagggcctgaagatcggcgtgggcggcgataaggtcgtcccccatgtcgttggggtggctggtggtgtagcggatgcgatccagccccggcacctcggccagggcgtaggccaggcgcgccagggtccatggctttccgtccggcccttcgccgtcataggcgttgacgttctggcccagcaaggtgacctcgcgcacgccgcgcccggccagcgccctcgcctcctccagcaccttcatgaccggccgcgaccattcggcgccgcgcgtatagggcaccacgcagaaggtgcagaacttgtcgcagccctcctgcacggtcaggaaggcggtgacgcccgagccgccgcgctcggccggcagggcgtcgaacttgtccaccggcgcgaagtcggcgccgatccgctcgccgcgggcgcgcgccgtgcgggtcagcagctccggcagctggtgataggcctgggggccgacgaccagatccaccgccggctggcgacgcatgatctcctcgccctcggcctgggccacgcagccggccacggcgatggtcatggcggcgccggtcgcctgcgccttggcctgcttcaactcctttagcttgccgagttcggaatagaccttctcggccgccttttcgcggatgtggcaggtgttcaggatgacaaagtcggcgtcgtccggcgtgtcggtctcggcatagcccagcgggcgcagcacatcggccatccgctcggagtcatagacgttcatctgacagccgtaggtcttgatgaacaggcgcttgggcgcgtgctcggacccggcgggaacgagggtgtcggtcatgtctcggcttatgatcgccgaaacgggcgcgggcaaggcggccgagacagccctcagggaacctctacgtcggccgggttcacgcgcgcggcgtggcgggtgaagatcagaccctcgcgcgacgacggctcggccccctcgatcggcacgccgtaaagctccagcttgtggccgatcagctcgaaacccagtcgtttggcgatctcggacttcagccgctcgatctcggcgtcgaagaactcgatcacctcgccggtgcgggtatcgataaggtgatcgtggtggtcgtcgcccgcctcttcgtagcgtgagcgcccgtcgccgaagtcatgcttctcgaccacgcccgcttcctcgaacaggcgcacggtgcggtagacggtggcgatggatatgtgcggatcgatggaggaggcgcggcgatacagctcctccacgtccggatgatcctcggccgaagacagcacgcgcgcgatcacgcgccgctgctcggtcatgcgcatgccgcggtcggcgcaaagtttctcgatccggtccatggcgcaggagaataggggctgatcgcccgtcagggaagaaccggagacgagagatcgaggctcatcaccaccgcatcgacgcgccggccgtccgtcgacggataatagcctttgcgccgtccgctcggaacaaagcccgcttggccgtagagcgccatggcggccgtgttggtctcggccacctccaggaacatccgccgggcgccggcgcgcgccgcctccagcgccccccgccccgtcaatcttgcgccgacgccgcgccgccgcgccgccggccgcaccgccagcgtcaggatctcggcttcgtccagcacgacgcgcagcatgatgaagccgtcgtcctcggcgaccaccagcaccccacgctgggcggccagggcgtcgagttccgcttcactccagggcgtcgcaaaggcttccgcatggatggcggccagccggttcatgtcggacgcgcccgtcttcagcgtcacttcaccgccgcctgccgtggttggccgggcaggcgcgtgggcgccgtggcgtcgggcgcgcgcagatacaggggccggggcgggtgcgcttctggatcgagcgcgagggtcaggcgcgccagggcggcggggctcggagccgacagcggctcaaccttggccgcgacctgcggatgggcttgggcgacgaccggcccgcccgatcccaccagccgccagtctccgtccgccagccgtgcggcggcttcggccaggggcagggcctcggcctcgccttgcggcgcctcgtcgcggaacaggcgcgcatagacctggtcgcgccgggcgtcgatcagggcggcgacgggtccgtcgctggcgaccgaggcggccagggcgtctagcgccgatacgccgaccaccggccggtccagcgcctcgccgagccccagcgcgaacgccagccccacccgcagaccggtgaacgatcccggtcccaaggtgacgccgatccgctcgaccacgtcgaagccgatcccggcgtcggccatcgcatcgcgcacgaagccgcccagccgttcggaatggcccttgctcatcggctcggagcgcacgccgagcggccgcgggccgtcgaacacagcggcggtgcaggcgcccagcgccgtgtcgatcaccagaacgatcatggcgacggctttgtgcgcgctacagcgtctgctcgacgcgcgtcacctcgggcacatagtgccgcatcatctgctcgacgccggccttcagcgtggccgaggacgaggggcagccggcgcaggcgccgcgcatgcgcaggctcaggacgcccgtctcctcgtcgaaggcgtcgaacaggatgtcgccgccgtcctgggcgacggccgggcggatgcggctgtccagcagggccttgatctcggccaccacctcgctgtcctcgcccgccgcctccggctggtcgccgccgccggctcgcagcaacggctggccggacacgaagtgatccatgatgacgcccaggatcggcgccttcatctccgaccagtccgggccccgtgcgtcacgcgtcaccgaaacgtagtcgccgccgaagaagacgccgccgacgccctccagctcgaacagggcctcggccagcggcgaggccgtcgcctcgtcgaccgtgcggtactccagcgcggcggccggcgagacgtcgcggccgggcaggaacttcagcacattgggattgggcgtgggttcggtctggatgaacatggccgggagatgcgctcgcgctaccggcggcgcaagccccccagcacgccgcgcagcagctcgcgcgtcagggtcgatccggcggtgcgcaggaccgatttggtcagggcctccatcggcgtctggcgattggaggcgcgggcgcggggcttcggcttttccgccggagcgcgcgggggcggcgccccggcctcggcctcggcccgacgttcggccagccgttcggcggcggagtctcgatcgatccgctcgtcgtacaggccccgtaccggactttgcaccatgacctgcgcccgctcggccggcgtcgcgggaccgacccggctgttgggcgggcggatgcgcgtgcgggcgacaacggtcggcgcgcccttctcgtccaggacggacaccagcgcctcgccgacgcccagcccctggatcgcctgcgcggtgtcaaaggcgggattggcgcgaaagctttgcgccgcggccttcaggcccttctgctcggcgggcgtataggcgcgcagggcgtgctggacgcggtttcccagttgggccaacacgggatcggggacgtccgccgggttctgcgtcacgaagtagacgccgacgcccttggaccggatcaggcgcaccacctgctccaccttgtcgcgcagggccgcgggcatgtcgtcgaacaagaggtgcgcctcgtcaaagaagaacaccagtcgcgggcggtccaggtcgccgacttccggcagctgctcgaacaactcggacagcagccacaacagaaaggcggcgtagagccgcggcgtgttcatcaagcggacggcgtgaagcacattgatctggccccgcccgtccagacccgtgcgcagcaggtcctccagccgcagcgccggttcgccgaacagggcctgtccgccgtcccgctccagttgcagcagcgcgcgctggatggcggagaccgaggcgggcgagacgcggccgacctcccggccgatgcgctcggcgttctccgccacatagacgagcatgctgcgcaggtcgtcgaggtccagcagcagcaggccttcctgatcggcgacgtgaaaggcgacggacagcacgccttcctgaacctcgctgaggtccagcatccgggccagcagcaccggcccgacctcggacaccgtggtccgcacgggatgtccggcctcgccgtggacgtcccagaacaccacgggcgccgagcgaggcgtcagcggcccgccgagctcgacggcgcggtcggcgagcggaccttcggacaggcccgaacagcaaaggccggaaaggtcgcccttcacatcggcgcagaacacggccgttccagcgtcggaaaaaccctcggccatcagttgcaaggtcacggtcttgcccgttccggtcgcgccggcgatcagcccgtggcggttggcccggcgcagccaaagggactgggcctcgcctccgtgttccggcggggcgcagcccaaaaacaacgcggcgtcggacattcgggcctctccgtggcggtgcgcggaccggtctagcccagcctttcgacgacgcaagcgtccgctgcgaccgcctgccgcgcgacagtttcgcaaatcaggcgatccggctcttgcggcttcggcgcaggggcctatctaccgcccatcgtcgcgggcccatcccctcctgttcgcggcgctgaaccggcgccaccctccctccccctcggcgccggccaaagcaggccgtcggactcccccagtccggcggccttgttgtttgcgacgttcctgccacggtttgtcgcaggtcggccgcagacgggaacgctcggttggggtcgtcgttgatcgcgcggacgggctgtcgcctacctcctgccgctcacggcgattgatcctaaggacctccccacgatgacccttcgcacgacggcggccgcgctcgccctgatgaccaccgcagtgtccgctccggccatggcgcagaccacccccgactggaccggcccctatgtcggcgtgttcatcggcggcaaccaggccaacgaccagggcgacgagcgcctgcgcttcgaccgcaacctggacgggaactatggcgagacggtttccacggccgccggcgccgacgccttcagccccggcttctgcgacggcgcggccaacacggccctggccgccgacggctgctcggacgacaagaccggctacgagttcggcgttcgcggcggctatgactggcagttcggcaacttcgtggtcggcggcgtgggcgaatacagcgccggcgcggccgaggacacggtgaccggcttctccaccacccccgccaactatgtgttcacccgcgagctggagcagctggccgccgcgcgcgtgcgcctgggctatgcagccggtccggccctgatctacgccaccggcggcggcgcctggggcaaggtcaagaaccgcttcttcagctccaacaccgccaacagcttctccgaaaccgtcgatgaccaggacgcggacggctatcagtggggcggcggcgtcgaatatgcgctggcgccgaacctgtcggtcaccggcgaatacctctacacctcgctggacgcgggcgatcacgtggtgcgggtgacccaaggctccgcaccggcaaccaatccatttgtgctggcgccgaatacggcgggcacggacatgatccgctccaacagcaagttcgggctgcacgcggttcgcctcggcatgaactaccgcttctaggcgagatcgcggctcgtttccgcctccttctcgactgaacgtcgataatccagaccgggttcgtcgaaagacgggcccggttttctctttgggggttttcgccgcttcggatcgggcctagtcaggtgatcacggcggcgttccggcgtcacaggacgacgggctcgccgcgcccctcgcggcccagccgcgccttgcgagaccgttcttcatgtccgccgtcgacctgcgttcgaagccctccgcgcctgctgatctggacgccgtcagccaggcgtattcccgtctgggcggcgatggggcgaaccccggggccgtgcgcgccttcctggcccaggcctttgaggactattccgccgacgaaacgccgcagatcgacggcgaggacttcgcctgccttctggtcgacgcatggcgcgcggccgaggcgcaggcggacggcgccgcgcccacgatcaccgtgggaccgctgaccggcgcgggaggccgcgcggtcggctatgatctggtgcgcatcgttcaggcggatgcgcctttcctggtcgacagcgtgctgggggaactggccgaagcggacgtgtccgtgcgcgccctgttccacccggtggtcgaaatgggcgatgggcggcgcctgtcggtgatcctgctggttcttgatccgatcacccaggagcggcgcgacggtctgggcgaggggctcgccgcaaccctggcggatgttcgccaggcggtggccgaccatcccgccatgctggacctgatgcgccgggcgatcgcgcagctcgaagcgggcgccccggtcgccgaggaggccgtggccgccgagaacgtcgcctttctgcgctggctcaagagcgatcacttcgtcttcctgggcgcgcgggactatgactatccccgcgcggaggacggcgactacgaggccgaggcgccgctgagccagtcgggcgaaggcctgggcgtgctgcgcgaccccgagcgccgagtgctgcgccgcggcaacgagccggcggtgctgacgcgccagatgcgccgccagatggacctgtccgaaccggtcaccgtggccaaggccaacctgcgctcgcgggtgcatcgccgcgcctacatggactacatcggcgtcaagaagtacgggccggacggccgcgcctcgggcgagacccgcttcgtcggcctgttcacggccgaggcctatgaccacgtcgccgccgaggtcccgctgatcaggcgcaaggtggcgggcgttctggcgcgcgcggacaaggcgccgggcagccacaacgaaaagcgcctgcgcaacatcctggacaactatccccgcgacgagctgttccagatcaccgaggacgagctgctgtcgatctcgctgggggtgctgcacctctatgaccggccgcgcatccgcatcttcacccgccccgacccgttcgaccgtttcgtttcggtgctgtgcttcattccgcgcgaacggttcgacgcggcggtgcgccagcgcatcggccagatcctggcgcgcgcttggggcggccgggtctcggcctggtatccgcagctgtccgaagcgcccctggtccgcgtccactacatcatcggcgtgacgcccggcgaccatccgacgccggacatgcagcagctggaagcggacgtggccgaggccgggcgcggctgggtcgaaaggttcgagaccgcgctgcgccgcgacggcgtggatgaggtcgaggtcggtccgctcagcgcgcgatgggcccgggccttcggcgccgcctaccgcgaccgctacgacgccggggaagccgcgatcgacctggaggcgctgaccacggtcggggagggcggggcgccgctcgccgtgcgcgccttccgtcacgccgacgacagtccgctgcagttccgcttcaagctgtatcggcggggtccggcggtgccgctgtccgacgttctgcccatcctggcggacatgggactgaagacgctggaggaatacggctatccgatccgtccggccggcgacgccgagatccacgttcacgagttcctgatggaagacccgcgcggcgaggcgctggtgttcgacgagatccggcgcccgttcgagcaggcgttcgccgcggcctggagcggcctgacggagagcgacggcttcaaccggctggtggtcgaactgggcgtctcctggcgcgaggcggcgctgatccgcaccctggcgcgctatcgccagcagacgggcctggatccgtcccaggcggtgcaggaagaggccctgcgggaatatcccgatgtgtcgcgcgccctgctgaagctgtgggaggccaagttcgccggtgagggcgatgcggccagccgccaaggcgccgtggccgagcaggaagccgccatcgccgcccagctgcaggctgtgaagagcctggatcacgaccgcgccctgcgccgcctcgccgccctcatcggagcgatcaagcgcaccaacttctaccagacggatgcggacggcgcgcccaagccgcacatctcgatcaagatcgcctcgcgcgagctggacgacctgccgctgcccaagccctatcgcgagatcttcgtctgggcgccgcacgtcgagggcgtgcacctgcgcttcggccccgtggcgcgcgggggcctgcgctggtccgaccgccgcgacgacttccgcaccgaggtgctgggcctggtcaaggcgcagcaggtcaagaatgcggtgatcgtgcccgtcggctccaagggcggcttttatcccaagcagttgccgcgcaccggcgaccgcgaggcgatccagggcgaggcgatccgcgcctatcgcaccttcctctcgggcctgttggacatcaccgacaacatcggcgcggacggcggcgtggtccgccccgccaacgtgatcgcctgggaaggagacgacccttatctggtggttgcggccgacaagggcaccgccaccttctccgacatcgccaacggcgtgtctgcggcctacggcttctggctgggcgacgccttcgcctcgggcggctcggtcggctacgaccacaaggccatgggcatcaccgcgcgcggcgcgtgggaggcggtcaagcgtcacttccgcgaaatgggcaaggacatccagacagagcccttcaccatggtgggcgtcggcgacatgtccggcgacgtgttcggcaacggcgccctgctgtccaaggccacgcgcctggtggccgccttcgaccatcgcgacatcttcatcgatccgagcccggaccacgtgaccggctggaccgagcgcaagcgcctgttcgacctgccgcgctcgtcctggcaggactatgacaaggcgctgatctccgagggcggcggggtgttctcacggtccgccaagtcgatcccgctctcgcccgagatcaaggccgcgctggacatctccgaggacagcctggatcccgtcagcctgatccgcgccatcctgaaggcgccggccgagctgctctacctcggcggcatcggcacctatgtgaaatcggccgccgagacggacgctcaggtcggggacaagtccaccgatcccttgcggatcaacgccgacgagctgcgggtcaaggtggtgggcgagggggccaacctcggcttcacccaggcggggcgcatcgccttcggccacgccggcggccgcatcaacaccgacgccatcgacaactcggcgggcgtggacacctccgaccacgaggtcaacatcaagatcctggtcggctcggcggtgaccaacgggaccctgccggcggatcagcgcacggacctgctggcctccatgaccgaagaggtcgggctgaaggtgctggcccacaactacgaccagaccctggcgctgacgctgcagcaggcggaaggcgccagggcgctcgacagccagcagcgcttcatgcagacgctgtccgcgcgcggaaagctggaccgcaaggtcgagggcctgcccaatgacgcccgcatgcgcgagatgacggcttcgggcacgccgctcagccggccggagatcgcggtcctgaccgcctacggcaagcttgagctgtcggacgacatcgtggcctcctccgcgcccgaggatccggctttcgagcaggtgctggtccgctacttcccgcaagcgctggcccggttcgagccggagatgaagagccaccggctgcggcgggagatcatcgccacggtgatggccaacgagatcgtcaacatgtgcggtccgaccttccccgatcgcctgcgcggcgccgccgaatgcgacacgggcgccctgaccgtggcgttcgaggccgcacgccgcatcttccgcctggacgaggcgtgggacgccgtgtccgccctggaccacaagatttcggccgaggcgcaagtcgccctctacaacgaaatctccgtagtgctgcggcgccagaccttctggatggcgcggcgggccaagaccggcctcggcgtccaggcccttttcgacgcctatcggccggtggccgaagccatccacgccgaaggcccgacggttctgtcgcggttcgagcagaagtgcctggaggaccgggttcgccgtttcgccgacaagggggcgcccgaggccctgacgcagggtgtggccatcctgcgcccgctggtcgccgccttcgacatcggcgacctttcgtcggagaccggctggcccgtggcggccatggcccggctgtatcaccaggtcggagccgccttcgacttcgaccggctgcgggcggcggcggggtcgatcccctccgtcgatcacttcgaccgtctggccgtgcgccggctgatcgaggatctgatgggcgagcagcgcaccctgacccgtgcggtggcgcgcgcctccgacccgtcggtcggcgtcagcgaagaggcggcggaagcggccgtcgacgcctggatcggagcccgtcagggcgtcgtggaaggcgtgcgcgcctcggtcgacgagatcgagggctccggctccggctggaccttcgccaagctgaccatcgccaacgccaccatccgcgacctggcggtctcggccgcgcagcagggctagggccgggccatggcgcgcaaattcctggtggtggccgacgacagtcccgagttcgcggccgccctgcgcttcgccgcgcgtcgggcgcgctcgaccggcgggcgcgtggtgctgctgcggatgctgccggacaacaccgacgcccattggtccggcgcccgcgaggaaatcgagcgccagcagcgggaggaggcggaagcgctgctgacccgtctgggcgaagaggcggctgagcggtcgggcgccgcgccggtcttcctgatcgagaagggcgacgcccaggccgcgatcaagaaggcggtggcggacgacccggagatcaagatcctggtgctggcggccggctccggctcgcgcgggccggggccgctggtctcggccatcatcaagcacggcgcgcagctgggcgggcgcaagctgccggtcaccatcgtgccgggcgacctgaccgaggccgagctggaagacctggcctagacgacgggcctcaggccgccgggcgcgggaccagccgccacatgcgcaagggatggcggaccgagcccgcctcggcgcccgccgccgggccccggcccatatagagatcggcgcgcaccgggccgcggatcgccgagcccgtgtccagcgccatgaccagcccgcgataactcgagcgcgcgccgcgcaggtttccgccgtccgcctcgacccaggccaggtcgccgtatctccagctggccggatcgatcgcaatggcgcgccgggccggcaggggtacgccggcggcgcccgccggatcgccgccgtcgtccggatcggtcctgaagaagatgtagcgcgggttgagcgccatcaccctttgcgcctgcgcgcctcggtgatccgccagccagcggctgatggcctcgccagaggttccgtttgcgggcagaaggccctgctgcgccatcggccgggcgatgccgacgaacggcttgccgttgtcggcggcgtaggccgcgcgcatccggccgccgtcctcgaacgtcagatagcccgagccctggatctgcataaagaacaggtcctcggcccgcatccaggccagggcctggtccgcgcgcgcgccggcctcgatcgtcgcccggtctcccgcactctcgggattggccggagcgggcaggacgggggccgaaaattccgcatcgggccggcgacgcgccgggtattcgggggcgaagtaggcggtcagcagactggagcgatccggcgacgggtcggcctcgacggcggtgaaaccggcttccagaaaggcgcgggcgtcgctgggcgtgacccggccggcggccagctccttggcccggtcgcacagccggcgcgcggccggctcgcgcgacacgccgcagccgcgaagataggcgttgaaggcgccgagatggtcttcctcggcccagccgggcagggcggccgggctcacgcccgaacccggctgcggcggaacgggcggcgtcggcgagggcgccggagcgggataggcgggccgtgtcggcgcgggagccgggggcgtgggcgagcaggcggccagccaaaggccgagcaggcccacggcggctccggccagggagcgggagcggccccgacgcaccgccgcgatgcggctcatcaggccgaggccgcctcgacgcgggccagcacccagttgggatcggaggcgcccagcgtccgctcgaacgtccagtgctcggcggtgcgacgctcctccgtagccggttcgccggtgacctggtcggccgactgccccgccgcgttgacgatcttgctgcgcagttcggccaggaagcgcaccttggtcaccgcgcggtcgccctcgaccgtgccgctctccaggtcggcgcggggcggataaaggaactcgacctgttcggtctcgccccgggtttcgcgcgcggcgatgccggcctcgaacgactccatcacagcgggggccagcagcggcttcagcgtcgcgcggtcccccgacgcataggcgcgcacgatggtctcataggcctgtcgcgccccttccaggaaccgaaccggatcaaaggcgggatcgcgcgccttcaggccggcgatggcggcaagcgtcgcggcgtccacgcccggcgtcttcggaaccgccggctggtcagcgccgggcgcggcgggcaggggcgtgcgcgacttgttgtcctcgggctgacggcccacgcgcctgcccagcacgttatagagctggaacagcacaaaggccgcgataagggcgaagatcacgatctggaacgaaaccggcaaggcgtctgtcctgtccttggaacgagccggatgtcgccggccacaaacgattaggcacacatatagggcagagcaaggcgatccgctcccttccgcccgcgcgcgacgttgcggccaagcgtcccgccatggtagtcgcccggcctcctttccgccttcgggcgcttccatccacggccccacaccatgaccgacgccccaccgcccgccgatctgccgcaaggcggccagccgcaagatccggctctgcaaggccagccggtcggccccggcttccgcatcctggcgcaatatgtgcgcgacttctcgtttgaaaatccgcgcgcgccggaatcgctgcgcatcgacggcaagcccgccatcgatctcggcgtcgagatggccgcgcagggtcgcccggacggcctgttcgagctggacctgaagctgtcggtcaaggcgacgcacgagaaccagccggtgttccacgtggaactggtgtatggcggcctgttccagctggccaatgtgcaggagcgggacatcgagccgctgctgctgatcgaatgcccgcgctatctgttcccgttcgcccgcgagatcatctccggcgcgacgtcggacggcggcttctatccgcccttcatgctggacccgatcgacttcgccgccatctacatcgcccgccagcagcagatcgcccagggtccggccgaagccggaatggcgtaagcgttactgatacgcttctccctcggggagggagagggtcgttcaggccgcggcgtcttcctgaacgacctgaacgccctgcgccgcccacagggaatggtcggacagcaccgcccgcagaaactcgatatgcgccgcgcgctcggcgggtgtcgacaaaggcgccagcggccgggggcgaggcggataggcggtcgccgccaccacggcggacgcccccccggctcgggcgccggacaggtccagcacccgctccttgccgccgcgcagctccagatagacttcggccagcagccgggcgtcgatcagggcgccgtgcaggctgcgctcgaccagcgagatcttgaagcgcttgcacagggcgtccagcgagttggccatgcctggaaatcgcttctgcgccagctgcagcgtgtcgatccagcgcgcttcgccggtgatcggatggccgcaacggccgcattcgtggtcgatgaagttgcggtcgaacgcggcgttatgggcgatgatctgcgcatcgccgatgaagtccatcaggtcgtgcacgacctcgtggaacttgggcgcgtccctaaccttgtcgtcagtgatgccgtggaccttgatggcgtccggcgggatcagccgctcagggttgacgaagcggtgaaacgtccggccggtcggcagcaggtcctcgatctcgatgcagccgacctcgatcagccggtcgcccgtcttcgggtcgaagccggtggtttcggtgtccagaacgatctcgcgcgccatggccccttaatgggcgtcttcgccgatttccgaaagagtcaggggcggcggcgcggcgatgtccacaagggattgagcaccttttcgaccacggcgcgcacctgatcccgtgcggcgtccagccctccgcccgtatcgatcacgaagtcggcgcgggcgcgcttttcggcgtcgggcgtctggcgggccaggatggcgtccagccgctcgcgggtcatgccggggcggcccaggacgcgggcggcctggacctcgggcggggcggtgaccaccaccaccgcgtccacggccgcaccgcccccggtctcgaacagcagagggatatccagcaccgccagccgcacgccggcctgctccgcccttgcgagttcctccaggcggccccgcatcaccagcgggtggacaatggcctccagccggcgaaaggccgtctcatcccgccccagcgcctcggccagtcgcgcacgatcgatccccccctcgacaaccacgccagggaaagccgtttggatcggtccgaccgccgcgccgcccggcgaatacagggcgtgcaccgccgcatcggcgttccagaccaggccgccctcgttcgcgaacatggcggcggtcgtggacttgcccatgccgatcgacccggtcaggcccagaacgatcacgcgaccgcctccagatgccggatcaggagcatccgcagatcaagcggtggcggggcctggccgaaagccgcctcgaacagaggcgccgcctggccgatcagcatggccaggccgtccacagtcacgagcccgcgcgtgcgggcggcctgcagaaggggcgtgacgaccgggcgataggtcatgtccatcaccacggcgtcggcgcgcaggcgggcgaggtcgaaatccggccggatgctgagggcgttgatcaccaggtcggcgtcgtccggggcctcgtctccgcagacctccaccccccgtccgagatcggccacgagcgcctcggctcgttcgcgcgtgcgattgacgatgcggacctgcgcgcccgcctgcaccagcgcccccgcgccggcccgcgccgcgccgcccgcgcccagcagaacaacgcgggcgccattcagcacaaggtccggcgcctgcgtctgcaaggcggacagcagtcccgccccgtccgagctgtcggcgtggatgcgccctttctcgaacagcaggatgttggccgatccggtcaggcgagcggcgtcactgacctcgtccgcgccggcgaaggcctgttccttgaacggcgcggtgacgttcagcgcccgaatcatgccggcccgtcccgcggcgacaagcgtctggaatcctgcgtcatccggcggtgcgaacggaaggtaggcggcgtccagccccgccgcctcgatccaggcgttgtggatcaccggactgagcgaatgggctaccggccgcccgacgatgccgagcaccgtcgcctcgcccgtgatgcgagccctcatgccggcagggctccgacgcggcgcaactggtccagcaccgcccatagcggcaggcccagcacggtgaagtagtcgccctccaccttctcgaacagctgggcccccatgccctccagccgataggccccgacgcacgacagcagggcctcgccctcgttgtcgagataggcgtcgaggaagctgtcggtaaagggccgcacctgcatcgtcgccgtatccgcgcccgaccagaccgcctggccgccgcgcgccagggtcgcgcccgaatgcagggcatgcgagcggccgcgcatggccccgagccgcgccctcgcttcgtggagggatttggccttggacaccagcccgccgtcgaaggccagggtctggtcgccgcccagcacccaggcgtccggatggaggcgggacacggccagcgccttggccgtcgcaagttcgaccgccagttgatcgggttcgatcgcgccaagttcggcctttaacgcctcttcgtccaccggagcgacctccacgcggaacgacacgcccgcacccttcagcatctcgcgccgcgcggcgctgccggacgccaggatcagttcgggcgcgctcaccagctggcgcccaggcgctgggtgcggcgctcgttcagcagattgacgatggcggcggcggtttcctcgaccgagcggcgggtcacgtcgatggtcggccagccgcgccgctcgaacgcgcgccgcgccttgacggtctcgtcgcgcaccgcatcctgatcggtgtaggtggagccttggtcggcgttcaggttgtcgatgcggttgcggcggatctgcaccaggcggtcgggcgacaccgtcaggccgatgacgagcggattcttcagccccgtcagccgctctccgtcctcctgccccggcaccagcggcacattggcggcgcggatgccccggtgcgccagatagatgcaggtcggcgtcttggaggtgcggctgaccccgcacagcaccacgtccgcgccctctagctgttccgccgtgccctggccgtcgtcataggccatggcgaaatccagcgcggcgatgcggttgaaatagtcgtggtccagcgcgtgctgggccccgacccgcttggacagcgaggcccccagatagcgggacagggcgcccaccagcgggtccaacgcgccgatctggggcatgtccagccggcggcagccctcctccagctgttcgcgcagatcgcggtccaccagggtgtggagaaccacgcccggcgcggtctcgatctcctccagcacccggtccagctgcctggacgagcggaccagggcgtagatgtgctcgatcgggatcaccccgtcgaagcgggccgtcaccgccttggccatggcgttcaacgtctcgccggtcgaatccgacaccagatggacgtgaaaataggtggcgagacgaagcggcgccgccgttctgccgaggcctctgccgggacttgcaactgggctcatggcgggcctcatctggcttgatcgactgtggacatccggtgggcgctcgcggccggaaatccctccgcatcctatagcgccggcttggcgccggagcgagcaggggaccatgaggatgactccgaacccgcgcggtcaaactatccagactggaaaatccggatcggccgcacctgtggattttcttaccaaagggttaacacgtgttagccgtcttccgggcgtcaaaaccctcaaacccgctcgccttaagggttcgttaaggatcagcgagcggcgccgacggcctcgacaggcctctggatgttccggcgtgcgacgtggatatccgcttttgttctcgggatggctggtgaatcatcctcgtcattccacggtcctacctgcttccacgaatcttctaattcttcttttgattagggattgagcacgggagatggggaccgtaagccttccgaccatgaccacgcctgcgccgaccccgcctctgctgctcagagccttgcaaggcgagacgctggatcggcctccggtctggttcatgcggcaggcggggcgctatctgccggagtaccgggctctgcgcgcccaggcgccggacttcatcgccttttgcctgaaccccgacatggcggcggaggcgacgctgcagccgatgcggcggttcggcttcgacgccgccatcatcttcgccgacatcctgctgatcccccgcgccctgggccaggaggggtggttcgaggcgggcgaggggcctcggctcggccgcatgccggagccggatcagatggcctcgctggcggcctcggccggcgagcatctgtcggcggtgggcggttcgctcagccgggtgcgagcggccttggagccggagcgggcgctgatcggcttctgcggcgcgccctggacggtcgccacctacatgctggacggcgaggcccgcacaatcggcaagggcgagcgggcgcaggcgcgaacctacgcctacgccgaccccaggcgggttgcggcgacgttggaggtgctggtcgaggccagcgcccattatctgaagatgcaggccgacgccggcgcgcaggtgctgaagatattcgagagctgggcagaagggctgccggacgacctgttcgaaaccctggtgctgcggccacaccaggcgctggtgcgtcgcgtgcgcgaactgggcgtgaccacgccgctgatcggctttccacgcggctcggcggccctggccgagcggtatgcacaggaggtcgaggtggacgccgtggcgctggacaccgcctgtccgctggaggtcggacgtcgcgtccaggcgatcaagccgatccagggcgcgctggatccgctgcttctgcgcgcgggcggcgaggcgctggaccgccgagtcgatcagttggtggaggcctgggggcagggcccctggatcttcaacctgggccacggcatcctgccggacgtgccgatcacccatgtggagcgggtcctgacgcggatcggcgcgcaatgagcgaggggacggttgacgcgggcgtgggcggacgccgcatcgcggtggtgctgttcaacctgggcgggccggacgaccaggcgacggtaaagccgttcctgttcaacctgttcaacgatccggccatcatcggcctgcccggcttcgcccgcacgccgctggcccggctgatctcctcgcggcgggagaagacggcccaggccaactacgccctgatgggcggcggctcgcccctgctgcccgagacccgcaaacaggccgaggcgctggagagcctgctgaacgatcgtctggacggcgacgaggcgaaggtgttcgtcgccatgcgctactggcggccgctgacggaggagacggcggccgatgtcgcggtgttcggccccgacgagatcgtgctgctgccgctgtatccgcagttctcgaccaccacctcgcagtcgtcgctgaagctgtggcacgagacctacgccggctcgggccggtcgcgcaccgtgtgctgctatccgcaaggcgccggctggatcgaggcccaggtcgaagccgttcgtcagaagctgacggaggccggcgaccgcccggtgcgcatcctgttctcggctcacggcattccggaaagcctgatcgagaagaagggcgatccctatcaggcgcaggtcgaggccaccgtcgaggcggtggtcgcccggctggcggtcgagggcgtcggcatcgatcacggcctctgctatcaaagccgggtgggaccgatgaaatggctgggcccctccacgcccgaggcgctggagcaggccgcgcgcgacggcgtcggcgtggtagtcgtgccgatcgcctttgtgtccgaacacgtcgaaaccctggtcgagctggacatcgaatacggcgaactggcgcataggctgggggtcgcgccctatctgcgggcgccggccgtgggcgccgagcccgccttcatcgccgccctcgccgacgccgtggccgacgccctgccgcgcacgggcgccgcgccgttcgggccgggctgccgcaaggcgtggaaggcctgtccccatctctgcccgcaggaggccaaggccgcatgaccgtctatgacatcgcgcgcggactgcacatcctggcggtgatcgcctggatggcgggtctgctgttcctgccgcgcctctatgcctatgacgccgaacaggccgccaagcccgagcctctgcggggcgagatgcaggcgctgctgcggagctggcagacccgcctgctgcgcatcatcgtcaatccggccatgatcctggcctggggcttaggcctgtggctgatccacctggacacggtggcgcgcggcgcgtccttcctgctcgagccctggatggtgaccaagcttctgggcgtgctgctgctcagcggctggcatggctttctcgccggccagcggcgcaggatcgcggccggaacgtccaaatactccggccgcttctggcgcatgaccaacgaggtgccgttcgtgctggccatcatcatggtgctgtcggtgacgacggaatggcggttctgatccgctccgcttgacctcgccggcggcctgtggttccgctggcgtgagccgtgcggcgcgcttcgcctgcggtccctctctcttcgtgacgcctgccgatcgaccggcgggagcccgtcacgtctccctgcctgcggcccccggccgacaatctggatacaacagcgcccgcgcgggctcgccagcgcgtgtgcgaccgtgagctcccccatgaccgacgtgcgcgacaccgacatcaccacgcccgaagctgagaccttcgagagcgaccaggttcaggacagccagccgaccggcgacgaaggcgtggttgatcaggaagcccacgaggaagacggcgagcctgtcgttcccaacggccgcatcaccctggccgagctgaacgagaagacgcccgcggatctggtcgccttcgccgaagggcttgaggtcgagaacgcctccaacctgcgcaagcaggacctgctgttcgccatcctcaaggccctggccgaggaagaggtggagatcatcgccgacggcgtgctggagatcctgccggacggcttcggcttcctgcgcagcccggacgccaactatctgcccggccccgacgacatctacgtgtcgccgtcgcagatccgccgcttcgggctgcggtcgggcgatacggtgcacggcgcggtgcgcggcccgcgtgagggcgagcgctatttcgccctgctcaaggtcgacacgatcaatctcgaggaccccgaggcggtcaagaccaaggtcctgttcgacaatctgactccgctctatcccgaagagcgcctgcacatggagatccaggatcccacgctgcgggaccgctcagggcgggtcatcgacatcgtggcgccgctcggcaagggccagcgctgcctgatcgtggccccgccgcgcgtcggcaagacggtgatgctgcagaacatcgccaagtcgatcgagcgcaaccatcctgaagtcttcttgatcgtcctgctgatcgacgagcgtccggaagaagtcaccgacatgcagcgcacggtgaagggcgaggtcgtggcctcgaccttcgacgagccggccacccgccacgtcgcggtcgccgagatggtgatcgaaaaggccaagcgtctggtcgagcacaagaaggacgtggtgatcctgctggactccatcactcgcctgggccgcgcctacaacgccaccgtaccctcgtcgggcaaggtcctgaccggcggcgtcgacgccaacgccctgcagcggcccaagcgcttcttcggcgcggcgcgcaacgtggaacagggcggttcgctgaccatcatcgccaccgccctgatcgacaccggcagccgcatggacgaggtgatctttgaagagttcaagggcaccggcaactcggaaatcgtgctggaccgcaaggtcgccgacaagcgcatcttcccggccatcgacgtgctgaagtccggcacccgcaaggaagacctgatcacgcccaaggagcagctggccaagacctatgtcctgcgccgcatcctgaaccccatgggtcctcaggacgccatcgagttcctgttggacaagctgcgccagtccaagaacaacgcggacttcttccagtccatgaacacctgaggcagtcggcgcgagccggcgtttcacgtggaacaagaaggaggatcgggggccggcgatgaccgacaccatcttcgccttggcgaccccgcccggacgcggcgccatcgctgtgatccggctgtccgggcctggggtcgcggacgttctggatcgcctcggcgcgggcgatctcaagccccgcatggtggcggtgcgtcatctctcccatgggggcgcgcagatcgaccaggctctgatgctgcgcttcgtcgcgcctggttcctacaccggagaggacgcggccgagctgcacctgcatggtggacgcgccgtggtggaggccgcgcaaaaggccttgttggctctgggcctgcgaccggccgagcccggcgagttcacccgccgggcgtttcagaacggacgcatggacctgacccaggcggaggccgtggccgatctcatcgatgcggagaccacggctcaggcgcgccaggcgctgggccagctggagggtcggctcagcgaaacctacgccggcttccgccgtgatcttctgcaggcgctggccctggtggaagccgagatcgacttcccggacgaggaggtgccggacaatctggcgctcacggcaggaccggtgctggagcggctcgccagcgatctgcgcgacgccatcgcgacgggtgaacgcggcgaacgggtgaggagcggctatcgcatcgtcctgatcggggagaccaacgccggcaagtcgtcgctgttcaacgccctggttcagcgcgaagcggccatcgtcacgccgatcgccgggaccacccgcgacgtgctggacgccgatctggtgatcggcggctatgcggccaccctgtcggacacggccggcctgcgtaacagcgacgatccggtggaggcggagggcgtccgccgcgcccgcgcccgcgccgaggcggccgaccttcgcctgtgggttcgcgcgccgggcgatccgtccggtgcggcggcggactacgtgcggccgggcgatctgatcgtcgccaacaaggccgacctcggagatgtgagctccagcactgaccttgaaacgatcaagctcagcaccgcatccggggaggggctctccgctttgcaggactggctcggcgcccgacttcaacgtgatctctccggcgccgactttccggctgtgacccaggcgcggcaccgccaccgcctgggagaggcgctccaggccgtcgaggcggctcggcgtattctggggcagtcgccggaaatggccggagacgatctgcgtcgcgcaggcgaagctctcgcgcgtgtcacgggggcgatcggcgtcgaggacatactcggagaggtgttctcgaccttctgcatcggaaagtaataccgacgttccacgtgaaacacgccgcgctaggagccgcggccacgctggcgattggcgacgttttcccctatgtggcggcgcatgcgcccagcttcggatctcagcttcgacgtcatcgtaatcggcggcggccacgccggctgtgaggcggcggcagcctccgcccgcgcgggcgcgcgcaccctgctgctgacgcagaggctcgagacgatcggcgagatgtcctgcaacccggccatcggcggtttaggcaagggtcatctggtccgggagatcgacgcccttgacgggttgatggggcgtctggcggacgtgtcgggcattcagttccgcctgctcaaccgttccaagggtgcggctgtgcgcggcccgcgcagccagatcgaccgtcgcctctaccgtgaagccatgcaggcggaactggccgagaccccgaacctcaccctcaaggcgggaacggcggagcgcctgctaatggacggcgagcgtgtggtcggggtggtgacgggcgacggcgagactctgacggcggcggcggtggtgctgaccaccggcaccttcctgaacggcgtgatccatcgcggcgatgagcgcatccccgcgggtcgctttggcgaagcggcctctacaggtctggccgccgacctgcacgcggcagggctggcgctggggcggctgaagacggggacaccggcgcggctcgacggtcgcaccatcgcctgggaccggctggagatgcaggcggcggatgaggagcccgtcccgttctccttcctgaccgaccagattcgcgtgccgcagatccagtgcggcatcacccacaccacggccgagacccaccgcatcatcgctgaaaacctgggcgagagcgccgtctatggcgggcggctgtcggggcgggggccgcggtactgtccatcaatcgaggacaaggtggtgcgtttcgccgacaagtcgagccatcaggtcttcctcgagcctgaggggctggacgatcccaccgtctatcctaacggcatctcgacctccgtgtctgaggcgacgcagatggcgttcttgcgcaccatgccggggctggagcaggtggaggtgttccgcttcggctacgccattgaatacgactacgtcgatcctcgagagctgacccccgcgctggaagtcaagcgccggccgggcctgtatctcgccggccagatcaacggcacaaccggctatgaagaggcgggggcgcaggggctgatggcggggctgaacgccgcacgcgcggcggcgggccgggagccgttcatcctgggccgcgagcaggcctacatcggcgtgatgatcgacgatctggtgacgcgcggcgtcaccgaaccctatcgcatgttcaccagccgcgccgagtatcggctgacgctgcgcgcggacaacgccgaccagcgcctgacgccgcttggcgtccaggtcgggctggttggcggcgagcgtcgccggcggttcgagagcaaggcgcgggccttgaaggcggcgggtcaggtcgcacgggagcgtctgttcacgccgggcgaggccaacgcggtcggcgttcccgtcaatgcggacggtcggcggcgttcgatgcgcgacctcttggcttttccgaacgtttcgctcgccctcttcgaaagcgtcgtgcccgagatcgccggctggtcggcggaggtgcgcgagcagatcgagatcgacgcgggctacgcctcctacctcgatcgccaggccgtggatgcgcaggcgctgcggcaggaggaggctctgaccctatcgcccgatctggactatgacgcgatcggcggcctgtcgaacgaggtgcgcgagaagctggcgcgcgtgcggccccgcacgctggggcaggccggccgcattgaaggcgtgacgcccggcgcgctgaccgcactgctggcccatgtgcgtcgctcgaaatcggcggccgccgcctgatggatgcgcaggccttcgccgcctcaacgggtgcgactgcggcccagatggaggatctggacgccttccgcgcgcgcctgatcgaggccaacgccgtgatgaacctggtcgggcccgacaccctgccggacttctggaaccgccatgctttcgacagcgcgcaactgatgcggcatgcccgcaacgcccaaacctgggctgatctcggcgccggcgcgggctttcccggcgtggtgctcgccatcctgtcgaagggcagggcggatgcgcatgtctggctgatcgacagcttgggcaagcgctgccgcttcctgcaggaggtggtggacgaactcgccctgcccgctaccgtcatcaacggccgggccgaagcgcagtcggtcaccgtcgacatcgtcaccgcccgtgccgtcgcgcctttggagaagctgctgggttatgcacagccatacttcgagcgcggggcgcagggtcttttcctgaagggggaaaaggccgaaacggaagtggcggccgcacgcagttcctggcggttcgacgcgtcgctgtcggtgtccgagagcgatccgcgcggccgcatcgtctatgtccggagtcttcgccgtgcccgcccagcgtaagcccgcccgagttctcgccatctccaaccagaagggcggcgtcggcaagacgaccaccgccatcaatctgggcaccgccttggctgcgatcggcgagaaggtgctgatcgtcgacatggacccgcaaggcaatgcctccacaggtctcggtgttccacgtgaaacgcggcgagtgacgatctatgacgtggtggtggatggtcgctcgatccaggacgccgcagtcgacaccttggtgccggggctgtccatcgtgccggccgatgcggatatgtccggggtggagatcgaactcagccaggcggaccggcggtcctaccgactgcgcgacgcgctgcgggcgcatgatctgggcgcagcgccgtatgactatgtgctgatcgactgcccgccgtcgctgaacctcctgacgctgaacgccatggcggcggcggatgctgtgctggtgccgctgcagtgcgagttcttcgcgctggagggcctcagtcagttgatgcgcacggtggacatggtccgccagagcctcaatcccgttctggagatccagggtctggtgctgaccatgtacgaccgccgcagcagcctgtcgggtcaggtcgccaatgacgttcgcgcccactttggcgacaaggtctatgacagcgtcattccccgcaacgtgcgggtggccgaggcgccttcgtacggcaagccggcgctgatctatgatctgaagtgcaccggcagtcaggcctatctgaagctggcgcgcgaactggtgcagcgcgagcgcaagcgattgaagcaggcagcctgaagcggacggacgaagacgtggcggaacgacaaagaggattggggcgcggcctgtcggcgctgatgggcgaagcggcctccgaggcgcctatcgcggcgggatcgcccgcgccggccggcgtgcaacgcgtgccgatcgagagcctgaagcccaatccggaccagccgcgcaagctgttctcccgccaggacatggaggagctcgccgcctccatccgcgacaagggcgtgctgcagccgatcctggtgcgcagccagccggatgagcccggcgtgtggcagatcatcgccggcgaacgccgctggcgcgcctctcaagtcgcgcgcctgacggaggtgcccatcgtcgtgcgcgagatggacgacgtcgaggtgttcgaggtcgccatcatcgagaacgtccagcgcgccgacctcaatccgctggaagaagccaatgcctacggcctcctggtcgaacgccacggccgcacccaggacgagatcgccggcattgtcggcaagagccgcagccacgtcgccaacacgctgcggctgctgcaactcccgatgggagtgctgaaccacgtcatcgacggcaagctgaccgccggtcacgctcgcgccctgatcaccgccccggacccgcaggccttggccgaacaggtcatccgcgacggcatgaacgtgcgccagaccgaggcgctggtgcgacgcgcggcggaggggccgctgaagccgaagggcaggggcaagccggctgcctttagcggcggccgcgatgaggacatagccgcgctggagcaggacctgctcgatgtcttggggctgaatgtctccatcgcctacaagggcgacggcgcgggcgaggtggtgctgaggtatgcctcgctggagcagctggatgacatctgccgccgattgatggggtcctgacccgctctccgtggtagggtgcggcatgtccgacgaacctcaaccgcaaaccgagtccctcaccgccaccgaaaagctcaggcaggcggtcgccgccaagaagggggcccagtcggctccaggcgccgcgcacgacagcggtcgtttggctgagaaggtcgtggcccagcgcaatcagacgatggccaagcccgccttccgcaaggcgtccaagcgcggctgatcgaccgttacagcccgaggcgccgcgcccgtccggcgatctccagcagcagccgttcggcgatcagctggtccggcaggccggtcgtcttggtggcgacatcggcggtgttgatgctgtccagcacctcgtccagcgcctccagccgccaggcgcgggcctgacgcagcatctccgcctcctgcttccagaacacgccggcggccttggcggcctccttggcgttggcgccgctggcctgaaggatgtttatgcgccgcagcttgccgagatgcagcgcggcctgccgcaccgccatgacggaagactcgccctccgccagcgcccgtcgcaggccggactgcgcgggacccgcccgcgcgccgaaggcctgaagggccgcgtcctgcagcgaggcgtccggctcgacgcccaactgcttgtccagctcctcgctgtcgatggtcttgcccgagcccggcccgatgaacagcgccagccgctcgatctcctgccgcatcagaccccgttcgcgcggcagtcgcgccacgaaccggtccagggcgtccgacgtcaggcccaccttgtcggcggcgagggcctcgcgcgtcatgcgggccacgtcgccggtctcgtcctcgtagcagacgatgccgaccgcgccggcttccttctcggcggtcttgcgcagcgtggactcccgccccagctggccggcttcgatcaccagcatggcgtcgggattgaagccgccttcggcatgggtcttgagcgccgccgccagcatcttgtcgatcgacgccttgtcggccgacagccggacacggaccagccgccggccgcccatcatcgacagggcggtcaaggcctcctccagtctcgcctcgtccccgtcgatgtcgctgtcggtcaggaccgtgacgttgaacgggtcgttaaggtccggcgtcaccgtgcggcacaggatctcggcgcgctcggccacacccgagcggtccttgccgtggatcaccgccgcccgaatgccgcgatccggcgccttcaggaagcgctcgatctcgggccgcttggagaggatcaccgcccggccggcccttggttcaaggcctgggccaggtccagccggatcatgcgtgacagctcggccgccgcgcgctcctcgccgtcctgctgggcggcgatggcggcgtagggctggtccgccgcctcataggtggtggtgacggtctcgtcgccgttcagcgccgggcggccgtccagcggcgtcagcacccagacggcccgcaccgtcagctcatagcgggaagcggtgtcgtcgatgcgccgccccagcgcccgccgctcctgctcgaccgaggtctccagccaatacaggggaggggaggccctgtcgaaccccagcgcatcctccagctgctcacgcagccgatagccgagccggttgtccggtgtcgacacggcgatccggcgcagacccgatcccgtcaaaggttcggcatacatgggcgtgaagccgcaaccggccgctccgaggggcaggccgaccgccagcagaaacaggatcgccgcgcgccgcatcagccggccaccagattgacgatacggtccttcaccacgaccaccttgcggatgctgagcccctcgagtcgggccttcaccgtctcgtcagccagtacgatcgcctcgacctccgccgcctctgttccacgtggaacacgaacctcggccttgcgcttgccgttgatctggaccggcaggaccacctcgtcgtccgccgccagctccggatcataggcgggccacggcgcgtccaggatcatcccgtgctcacccagccgcgtccagcactcctccgccaggtgcggggtgaagggggcgaccagccgcgccagcgccgacagcgcctgagccttggcttcgccaccggcccggtcgtgcgccttcaccgtggccacgaaggcgtagagcttggcgatggccgagttgaagcggaaaccctccaccccctcggtcacggccttgatcgccttgtgcgtctcgcggaccaggctcttgttctgcgcctcgtcgcctgcggcgtcggcatcgtgagtgtcgaactcggtccagacgcgaccgacaaagcggctggcgccctcgaccccgccggtggtccactgcacgtcgcgctcgggcgggctgtcggacaggacgaacaggcggccggcgtccacgccataggcgtcgacgatctcctgcggcgcgaccacgttcttcttggacttggacatcttctcgatgtcgccgatggtcagggtctcgccggtcgagagccgccgcgccgagcgggcgccgccgccgttgggcagttccacatccgtcggctcgacccattggccgcccttggtgcgataggtctcgtgcaccaccatcccttgagtgaacaggccggcgaacggctccttcacgttcatcagcccggcgtcggtcagggcgcgggtgacgaagcgggcgtacagcaggtgcagcaccgcatgctccaccccgccgatatactggtccaccggcagccatcggtctgcggcggccgtgttgatcgcctcgtccgccgtcggatcggtgaagcgggcgaagtaccacgagctgtcgacgaacgtgtccagggtgtccgtctcgcgcaccgcgtccgcattgcacgaagggcatttcacctgcttccacgtaggatgccggtccagcggattgccgggcgtgtcgaacgtcacgtcctcgggcagcacaaccggcagctgatcagccggaaccggcacaggaccgcaggaggcgcaatggatgatcgggatcggacaaccccaataacgctggcggctgacgccccagtcgcgcaggcgatagatggtcgcgccctcaccctgtcccgcctcttcgatgcggcggatggcctcggccttcgccgcctcgatctccagcccgtcgaggaagtcggaacggaagatcaggcccgggccggtgtaggcctcttccgccacagcgaagtcgtcgcccgcgccatccggccgcaccaccgggatcaccggcaggctgtattttcgggcgaaatccaggtcgcgctggtcgtgcgccggacagccgaagatcgcgcccgtgccgtattccgacaggatgaagttggcgatccagacgctgatctcgcgcccgtcgaagggatggcgcaccgtcaggcccgtgtcccagccgatcttgggcgcctgctcgatctcggcctgcgaggcgccgccctggcggcactgggcgacgaaggcggcgacgtccgggttcgcgtcggccagttgcttggagatcggatggtcgggcgcgaggcccaggaagctggcgccgaagagggtgtcgggccgggtggtgtagatctccacgccgtcctcgaagccggccggaggctcgcccgcccacttccaggtcatgcgcaggccctcggaccggccgatccagttctcctgcatcagtcgaaccttgtccggccatcggtccaggtccttcagcccgtcgatcaggtcgtcggcgtagtcggtgatgcgcaggaaccactggttcagcttgcgcttctcgaccactgcgcccgagcgccagccgcggccgtcgatcacctgctcattggccagcaccgtgttgtcggccggatcccagttgaccaccccgtccttacgatagacgaggcctcgggcgtacagctccaggaaccaggcctgctgcttgccgtagtattcgggatcgcaggtggcgaactcgcgcgaccagtctagcgacaggcccagcagcttcagctgttcgcgcatcgccgcgatgttggaataggtccagcccttgggatggatgccgcgctccatggccgcgttctcggccggcatgccgaaggcgtcccagcccatggggtgcagcacgtcgaaaccttgcgcccgcttcgagcgcgccaccacgtcgcccatcacatagttgcgggcgtgtcccatgtggatgttccccgaggggtagggaaacatttcaagcacatagtatttcggccggccggtgtcccgggtgacgaaggcgtcggcttcggcccagcgggcctgctggcggggttcggcggtcttggggtcgtatcgggccacgggcgtcctgaagaaggcagaggggctcgcgcccctcgcactccactagcccgaagggcggcgtcgcccaagaagatttggcgcggcttcgacggcgcgccgcaggggtcagcccgcgttggcgaggttcagctggcgcgccttggtcaggatggcgttctccaggtccgcctcggtctgggcggcgacgggggcgcccgtccactggccgtcggccccacgcacttccttgaccacggtgacgttcagcgcatcggcgcgcagacgggtgtcgaggatgaacaccgtggccttgaaccgctcgttcggcgtctgcggattgatgtaccagtcatagttgatgactccgccccagggatcggcggtcaccagcggcatgaagctgagggtgtccagcgacgcgcgccacagatagccgttgacgccgatgccctgctgcacgtccgcgcgctgggcgcggggcttgccgccgacgaacgggatgctggagcagccggccagcgccacgcccgaggcgaccaaggcgaccgtcgcgccgcgaaccaaagccttgttgaggcccatcgggatagtctccaaaccatgtgatcgcggacggaccgccacgcacgcgatccatccggcgcaccgtgaccgcagcaaccttctataacacggccaaaaggggcgatgacaaggcgaaggcgggaaggggccgatcgcccgccgtccgctttcgccgcatcgccgtgacgcttgcgccacacggcgcgggcaacctgccgaggaaccggcgcccaaagctgacgttgcgttgaccgggcgagccgcgggtgtctaatccaccggctcacggcgaacacgccggttcaggatgttctgcgtcgcccgtgcggcgccgaagggttggaaatgcgcgtaggcggtctgtcgatatcggccctgagccttgctgtcctgctgagcgcgggcggcacggcgcacgcccagtcgaccagtcgcgcccagacgctgaccctgtccgaagccgccaacgcccagcgtgcagcacccagccagcgccggggcctgcgcctgaacgaccggggccgctggggtctggacttcaacctgaaccagccggtcggccgcgagcaggactggagcgacgtggaggccggggcctattatcgcctgaacgaccgcctgcgcgtaggggccgccgcgggcctggccgcgcccgagaccgatccggcgcgcgcgccggaaacggccaatcgcacccagccgcgcgtgcgcctggaaagcatcttcaagttctgaccggccggaacgccgtctggacggcgtcgatccccgcgatcccgcaggcgccgctcttgtgcagctcgttgccacgatccgcattgatcccgcccagcgcatagaccgggcaaggcgccgcgtcggccctcttccggaacgcctccacgccgagcgccggcttgcctgccgacacgccgccggccggaaacaccggcgacagcacaagggcgtccagtccggccgcatcctgcgcaagaggcccgccatgccaggcggacgtgagcagccactccgggcaccgccggcgcaaggccgccgcctccgccatcgcgcgctccggcagatgcactccgtccgcgtccagacgtgacgccagctccgcgtccagtccaatcagcaggcgcacgccacgccccgccgtcgccgccctcagccgccacccgacctccagcgcgtcggcgcggccgaatgcgcggaacaccaggcctgcgcccgccggcagccgcgccgccgtctcccacggccggggcgttcgctccggatcggtgaagaacagcagcggcggcagacgcccggccgccgggctgacagcggcggcgacgcggtttagatcaagcgccgttccccagagcgcgcgcgcctcgtcgctgtagtctttcgccaggatcatgaccgcttcatcccccgccgcccgatccgcgtccatcgccgaacgcatcgcaaccgtgcgcggtcgcatggaggcgagcgcccgcgccgccggccgcgacccggcgggcgtcgtcctgaccgccgtgtccaagacccagccgccccaggcgatcgatgcggcgctggccgccggtctgcgcgtgttcggcgagaaccgggtgcaggaggcgcaaggccgctgggcctcccggcgcgcggacctgaccgatcgggagctgcggctgatcggtccgttgcagaccaacaaggccgccgacgccctggccctgttcgacgtgatcgagagcgtggaccgcgaaaagctcgcccgcgccctggccgaggccggtcagaaggccggcgtccagccccgcgtcctgatccaggtcaacaccggcgccgagccgcagaaagcgggcgttcatccccgggacgccgacgccctgatcgccgccgcccgcgccctggccctcggggtcgagggtctgatgtgcatcccgccggccgaggaggccgcaggaccgcacttcgccctcctggcgcgcctcgcccggcgcaacgaccttcctgtcctgtcgatggggatgagcggcgatttcgaaaccgcgatccggttcggcgccacccatgtgcggatcggatcggccctgttcggggaacgaaatccgccgcttacgccctctagcagcacccccgcgccgtaacgccgcgggatttcccttctccaagccttggcgtagccgtcaagcctcgccattctccggtcatgcccgccccaaagacaatcctgatcatcgacgacgacgacgacctgcgcgaggccctggccgagcagctggccctgcacgaagagtttcgcaccgttcaggccgccaccgccacggacggcgtgcggatggggcgcgaggtgcgggccgacctgatcctgctggacgtcgacctgcccgacatggacggccgcgaggcctgccgcctcctgcgcaaggatggcgtctccaccccggtcatcatgctgacggcccaggcggcggacgccgacaccattctggggctggacgccggggccaacgactatgtcaccaagcccttccggttcgccgtgctcctggcccgcatccgcgcgcatctgcgcagccatgagcagtcggaggacgcggtcttctcgatcggcccgtacgagttccgccccgcggccaaggttctggtggactcaaaggaccgcaagatccggctgacggagaaggagaccaacatcctgaagtatctctaccgcgccggggccaagccggtgtcgcgcgaggagctgctgacagaggtctggggctacaacgccggcgtcaccacccacacgctggaaacccacatctatcgcctgcgccagaagatcgagcccgagcccggccaggcccgcctgctgctgaccgacgccgggggctaccggctgcagccctgaggctcagccgcctcgccactcgctgagcaccgcgccctgcgcgtcctcgaaggccacgcggtcgagttggacggcgccgatgcagatcggtcgctggtcgggaccggcggcgcggcagcggacggcgcggccgtcggcgaaggcggccatgcgtccttccagcaccaggcgatagccgccgtcgggaatggcggccggccgatcggcgtcccctctgaccacaaagctgtaggcgcgaccgttgcgtcggcccaggcgagacccgtcggcttcgaacaccgccgccagccccatggtctgcggcgatggcgggaccggctcgtcggcctgtgaggcggccgatgcgacgggacaggtctccgcccgcatccaggggcgtgtcagccagaacccctccgccgcctcccaggtctcgccggagccggcgacgagcggcgactccgtccagtcgcccggcgccagcgacaatcgaagcccgcggccctcggccgcctgcacgacgacggccagaccttccgacgccgcctcgtcgctgtcgctcgagcctgtgcagccgaaagcctggcgcacgacaaagcgacggccggccagggacgcgtccgcctcctcagtccgcccggccgcaaaggcggaggcggcggcgtcgagaccctgcagcagttcggcgcgaccgatcgtcggcgtgggagcaagcgtcgcaggggcgggagggggagcgctggcgggctgcggcggtccggccgggcgcggctcaggctgacgctcgcaggcggcgagaccgaggatcgccgcaatggccagggtcgctgaagaggtcgcggtcggcttcgacatgcaacccttctagcatgggagtcgctcaaaggggggacgtcgcccgaaacggttgacgtcaactgatgaaagcggtctgcaggcgcttatgactttcgaccaggttgtggcgctagcggtgcttgtcgccgtggtcggcgtgctgatccacggcaaggcgcgcgccgacatcgtggctctgaccggcgccgccgtgctgctgctgctgggggtggtgcggccggtggaggtgcagggcgccttcgccagtccagcggtgatcgccctggccggcctgttcgtgatcgcctacgccattgagctgtcgggcctgctgggcctgctgatccgcaacgccacgcggctggcggcgcgcatcggcgcgaccggcatctggatcgtgatcggcctgtgcggctcggtcggcggcttcctcaacaacacgccggtggttgtgctggccgcgcccgtgatccgcgacgtggcccaatcgctgaggctgtcgcccaagcggttccttatgccgctcagccacgtcacggtgatgggcgggctgctgaccctgatcggcacctccaccaacctgctggtcaacgacatggcccgcaacgccggccagccggtgttcagcctgttcgagatcacgcccgtcggcctgtgcatcgcggcgacgggcggcctgtggctgtatttcgtgggggcgcgccagctgggtcgctccgtcgccatggacgaagcggaggccgcccgcctggccgagctggaggagtcgcgacgaaaggcggccatggaggcgtcgcggcgacgccggcgcgttctgccgttcaacctgcctcggctgggcgaggcccgcaatctggcggacggctcgggcgacgccaatctcggcgacgtggagctgtacggcgccgccgaccggccgttccgcctgcggccggcgctgatttcgctgggcgtgttcgtcctggtgatcgcggccgccgggttcggctggacgcccatcgccgcggccgcctttgcgggagcggtggcgctgatcctcatgcgggtcatcacggcggaggaggcctacgccggcctgcgccccgagatcctgcttctgatcgccggcatggtggtggtgggcacggccatcgaagtcaccggcctggcccaggcgggggccgagcggctgatcgacgtaatccggccgttgggcccgatgggcgcgctgatcgtgctctacggcgtgacgctgatcgccaccgagcttctgtccaacgccacggtcgcggtgctgatcacgccggtggctgtggccctggccgagagcctgggtgtcgatccccggccctttctggtgtgcgtcatgatggccgcctcggccgccttcgccacgccgttcggctatcagaccaatgtgctggtcttcaacatggccggctacagctacatggatttcgtcaaggtcggcgcgccgctgaacctgatcacctggctggcggccatggtcgccatcccgatattctttcccttctagaggtccaggtccaccgtcaccggcgcgtggtcgctgggccgctcccactcgcgcacgtcgtcgtggatgcgggcggtctccggaaccaccgccggcgtcaggccgggcgaggtccagatgtggtccagccgcaggcctcgattggacttgcggaagtcggcggcgcgatagctccaccagctggccagcttctgcggctcgggatagcggtcacgcagcacgtcggcgaagccgccggtctcctgcagccggttcagcgtctccacctcgactggcgtgtggctgacgaccttggacatgtagcggtggttccacacgtcgttctcgcccggcgcgatgttgaagtcgccggccaagacaagcggcgcggccttgtcccggcgggcgatctcgtcagtcagccgttcgtagaagtccatcttgtgatcgaacttggggttcagcgcgcggtcgggcgtgtcgccgccggccgggatgtagaagttctgcacgtccatccccgcgatccggccggagacgcagcgcgcgtgccccagcttgcagacctcaagcgtcgcattgtcttcgatcggcaggcgcgaggcgatggcgacgccgtgccagcctttctgaccccgcacccgcaggtacggcaggcccatctcttcgaacgcggcgcgggggaactggtcggtggtgcatttgatctcctgcaacagcaggacgtccggagcacgctcggtcacgaaccgcgccacctggtcgatgcgcaggcgaaccgagtttatgttccaggtggcgaggcgaagcgtcatggcccgcgccttagcaggccggacgcttcgcacctagccggcgctcaagcgacgagcggccgcgtcgcgagcgtagcgaccctagttccggcccggccggcgggtggggtcgcgcagttggaacaggctggcggacagtccggacgcgggctgcaggctggtcagctgggtgcgcgtgcgctggccctgcgcatcggtgatggtccattcgcgaagccgcatcgggctgccggcaaaggcgagaatgacctgaccgtcattcggccggcggctgtcgcgcgcggtgatggcgaaggcgccggagtccatccgcgtcacccgctcgatccgcacgccttggtccagcctgacgttgcgggccaggaaggtggacagcggcgtggcgctgagcggaacctggcggaagacgttcaggcgcgggtcgtagcgcttgacgttggatccgtccgacacgaccagcagaccctgtgggttggtgtattcgaaccgcatcttgcccggccgctgcagatagaagcggccctcgcggcgctgattgccgctggtctcgacaaaggtcccctgggcggcgctcaggttctgcagataggtctgagcctgctgcagggcggcgcggtcttgggccgacaggttgctttgcgcatcggccggcaaggccgagcccagggcggccaggcccgtcagggcgcccatgccgagcaggagggtgcggcgggcggcggcgtgctgttctacggcgatggcgcgggctgaagcgcgggtgggggcgcgttggggcatggtgttcttctcgctcccattcgggattgtgggtgtcgccttcatgccgggtccgcttggcgtccgcatgacgccagcctgaccatattccggcgctccgatgaagcggcgttcatcgaaaacggccaagcttggcgtggaggcgggagaagaacgtggcgggggcgacaccgttcctctccctccggacttgggaaagaggaacggcgctcaagccgcgagcgaccgcgtcgcgagcatagcgcccctaaacgatgggcggcggtccagccaggacctcgcgcttgccggcgtggttggcggggctgaccacgccttcctgctccatgcgctcgatcagggtcgcggcgcgattgtagccgatctgcagccggcgctggacataggaggtcgaggccttgcggtcgcgcgtcaccacggccaccgcccggtcgtacaggtcgtcgccggtgccgccgccgtcctcgccgcccatcgcgccgtcaccgtcgccgtccggctcgtcggtgatcaggtcgagatagtcgggctcggcctgcaggcgcaggtgcttgcagacctcctcgacctcgtggtcgcccacgaacggaccgtgcaggcgggtgatgcgaccgccgcccgccatgtagagcatgtcgccctgacccagcagctgctcgccgccctgttcacctagaatggtgcggctgtcgatcttggaggtgacctggaaggagatgcgggtcgggaagttggccttgatggtgccggtgatcacgtccaccgacgggcgttgcgtggccatgatcaggtggataccggcggcccgcgccatctgcgccaggcgctgcaccgcgccctccacgtccttgccggccaccagcatcaggtcggccatctcgtccatcaccaccaccagatagggcatgggttcaggacggattttttcggactcatagaccgggcggccctggtcgtcgaagccggtctgcaccgtgcgttcgaaatgctcgcccttcttctgcgcctcgaccgcgcgctcgttgtaggaggccacattgcgcacgcccagcttggacatgcggcgatagcggtcctccatctcccgcaccgtccacttcaaggcgaccaccgccttcttgggatcggtgacgacgggcgccagcaggtgcgggatgccgtcatagaccgacagctccagcatcttggggtcgatcatgatgaagcggcattcggccggcgaatggcgatacaggatcgacaggatcatggcgttgacccccaccgacttgccggagccggtggtgcccgcgatcaacagatgcggcatgcgcgcgaggtcggccacatagggctcgccgccgatggtctcgcccagcgccagcggcagcagatggcccttcttgtcgtattcggcgctggccaggaggtcgcgcaggtagaccgtctcgcgcttggcgttgggcagttcgatgccaatggcgttgcggccctggaccacgctgatgcggcaggcgcgcgccgacatcgagcgggcgatgtcgtcggccaaggccacgacgcggccatgcttcacgccgggcgcgggcaccagttcgtacagggtgaccacggggccggggcggatctggtcgatctggccgcgcacgccgaactcctgcagcacgccctccagcatcttggcgttggccttcagcgattcctcgtcgaccgaggcggtgcgctgggccggcttggccagaatgccgagcgggggcaggtcgaactcgccctcgggccgggcgaagtcgaaggcggtctggtccacgtccgtacgcgccggcttgggcgccttgaccgccgccacgcgcggctccggggccgaggcggcgcggggcgcgggcgcagccggaacgggcatcagcggcgcctggtcgtcgtcctggtcatcttcccatggcggcggggcggcgaaggtgtcggcgtgcgcctcggccgccgcttcacgtgaaacggcgagagcgtcttcgtcgagagcaggctcgggcgcgggggccgggcgcgacttgggcttgcggacggccttgggggcggggggcgcctctgccttggccggcgtcggcgcgcgacgcaacgaccgcccccagtgcaaggcatcgccgaggtctgcgatcctcaggcccaccgcgtatccgcccgcccacaggcccgcgcccaggaacagcaagccggcgatccatcggccccctgagattctcagcgccgccacgcccgaggcgaacaggccggtgacgccatcgccccacagcccgcccagacccgtcgccagcggccacgccgccggcgcgaccggagccgacaaggccgccgacagcgccagcaccgaaccggtggcggcaagcgccttcagcggcgtcggcgtcagcctctgacccagggcgtcgcccaccgcacgcgccagcccgaaagcgatcagcagcagggccgccggccaggcggccagccccagcgtctgcatgaacagatcggcgaacagcgccccgttcattcccagccagttggtgggcgcatccgtagacgccgcgttcaggctgggatcggccggattccatgacgccaatgccacaagaagcagcgccgccagcagcgcctgcagcacgccccggaaccgcaccacgaagggcgcgccccacagcacgcgggcgctgatccaggcctgttggccgatggcgagggcggtggacatgacggagcggacacccttggcgcgaacgatccgccccttgtcgcgccaacagggttaagaggcgtttaccagacgcccgtctctcctcccgatcgctgcgcgacaaggagccgagagggtggacgaaagaggcgtgcggggcgacaaggccgcatgacccaggctgaagatcacgacatcatcatcgccggcgccgggctggcgggggcggcgtttgcgctggcggcggcgcagggcgggctgaaggtcgtgatgatcgatccccagccgttcgagctgcagttggcgccgacctttgacgggcgctcgacggccatcgccttttccaccttccggatgctggacgccttggggctgggcgaggatttgcgcccgcacgcctgccggatggaccgcatcctggtgaccgatggacggcggccgggcgccgccagccgtcaggcgtcgcccgcatttctccgcttcgacgccgacgagatcggggggcgcaccggcggcgagccgctgggctacatggtcgagaaccgccgtatccgcgcggccctggccaaggcggtcgaggcaacggggctggaggtcatcgctccagcctcgctggcggcggtcgatgccggaccgggccgcgcaaccgtgaccctgtcaaacgggcggtcactttcggcgccgcttgtcgtgggggctgaggggcgcggctcgcgcgtgcggtcggcggcggggatcgacacgatcggctggggctatggccagagcggcgtggtggcgacggtgcggctggcgcgcgaccacggcaatgtggcgcacgaatacttcctgccaggcggtcccttcgccatcctgccgctgacggaccagcgcgccagcctggtctggaccgagaccacccgccgggccgaggcgctgcgcgacgcctccgacgaggccttccacgcccacctgctgcgccgcttcggcgacttcctcggcgacgtggccgtggaggggccgcgcttcgtctatccgctgtcgctgtcgctggccgaacggctgtatgcgccgcgcatcgccctgatcggagacgccgcccacggcgtgcatcccgtcgcgggccaggggctgaacatggggctgaaggacgccgccgccctggcagaggtgctgaccgacgccgcgcgcctgggcgaggacatcggctcggaaacagtgctggagcgctacgcccgctggcgccggttcgacaacgcggctctggccgccggctttgacgcctttgtgcgtctgttctccaacgacatcggcccggtccggctggtgcgcaacctcggcatggccgccgtcaaccgcatcgcgcccctgcgccgcgccttcatgcacgaggcgggcggcgcgaccggcgacctgccgcgcctgttgaagggcgaacggctctagtccagctgacgcgcctcttccgccagcatgatcggcacgccctcgcggatcggataggccagcttggcgcccgccgagaccagctcgttggcggcccggtcataggtcagcttgccgcgcgtcaccgggcacaccagcacctccagcaggcgcggatcgacggaggcgggcgtgtgaaaggcgtcggacatggtttgtggcctatcgcgcagtcgcgctacttgaggccggtgttctaggacgtatcgcgtggtcgcgctacttgaggccggtgttctaggacgtatcgcgtggtcgcgctacttgaggccggtattctaggacgtatcgcgtggtcgcgctacttgaggcctactgcatcgaaggcgaggcgtcgtcgccggcgtcggcggcgtcgatgcgcatcagggcggtcagcgcctcgccgcgccccagcaggtcgccggcctcgagcagcgcctgcttctcggccggttcgaacggcagggccatggacaggctgttgatcagggcctcgaccggcgcgccctcggccgtgtcccagtcgatctccagcgcccgatgctccagatagacccgtagggcgtccaggaagccatgccgatcgaaggccgcatcgtccgcatccggcgcgaccagatcggcctcgaacggagcgaagtcggctcgcaccgtgcgatacggcgccttggacggcagttcgctggtgatccggaaccggctgacgcccgtcagggtgatcagatagcgcccgtccgaggtctccgcgaaagaggtgatccgccccgcgcagccgaccggcgacaaacccggcagctcgcgcgaaccgccgctgggctggaccatgccgatgatccggtcccccgccatggcgtcgtcgatcatgttcagatagcgcggctcgaagatgttcagcggcagctggccgcgcggcagcacgatgaccccgccgatcggaaacaccgggatcacctgcggcaggtccgccgccctgttgtagccttgcgccatcgatttccaggtcatgtgatgcggagggagcgggtcacgagaacaggatcgacgacagccggcgtcgtccctccttggccacgtccgacatggcgcccgcggcctcgaagacggtcaaaagctgcttgcgcgccgcctgttcgttccactcgcggtcggcctgcacgatcgtcagcaggtggtcggccgcgcccttcatgtcgccggacgccgccagcgcctgcgccaggtcgaagcgcgcctggtggtcgttcgcatcggcggcgagccgcgcctccagctcagcgttctcgcccgaggcgggcgcggaggcggccagcgccagctgggcgcgcacgctctgcaccgtcggctccttggagtcctcgggggccatggcgatggtctggcgcgcctgctccacgtcgcctcccgccagatacacgcgggccagaccggcgatggccttgggattctccggctcgatcgacagcacatgggcataggcctgcgccgcgccgccgaagtcgttcaggcccagcgactcctcgcccatggccagcacctcgtcgatctcgggcgaggccccgcccgcgccgccggtcagcttttcgataaaggccttgatctggctgtccggcaccgcgccctggaagccgtccaccggctggccgttgacgaaggcgtagaccgtggggatcgactgcacccgcagctggccggcgtaggcggggttcttgtccacgtcgatcttgaccatccgcaccttgccgccggcggcgcgcaccgccttttcgagcgcgggacccagcgtccggcacggcccgcaccaggtcgcccagaaatccacgatcaccggcgtggtgcgcgacgcctcgaccacgtcggtcatgaagctggcgtccgagccgtccttgatcaggtcgtccttgggggcggcggggtcggcgaaggtcatggatcggtccctgttccggtgggtaacgcgcgagcgagagagatggtcgcgcaggcgccgcgactcaagcgcccccgccggaaaccggctcaggtctggggtgtttcatcgttgaagaacaaggaccctccccatgacgaccgccaacgaccacgacatcaaggtgctgaacggcctgctggagtccacgctggacagcgtcgacggctaccgcgaggccgccaaggagaccgaccagacgcgctatcgcggcctgttcgaacagcgggcggaggagcgcggacgcgtggcctcggacctgcaggcggcggtgcgcggcctgggcggagaaccggaccacgaaggctcgatcctggccaaggcgcatcgcgcgttcctggacatcaaacacgcgctgttgcgtgacgatcagtcggtggttgcttccgtggagagcggcgaggaccacctcaaggcgcgcttcgaccgggcgctggaggacgagcgcatctccgccaccacgcgtgacgtgatccgccgcgcctatgtctccgtccgccaaggtcatgacgagatgagcgcgctgaagcacagcctggagggccagcgcgacgcctccagcccgctctatccgcagtagaacgaaaaaggccccggcggttcgcgccggggccctgatcgtgttgctgcgctgagggatcagccctcggcggtgtcggccgcgccggtttccggcacggtcgcgcccttggccggacgcacggtctgacgctcggcgatccgcgccgatttgccgcgacgatcgcgcaggtaatacagcttggcgcgacgcaccacgccgcgacgcttcacttcgatggactcgatgttcggcgacaggatcgggaacttgcgctccacgccttcgccgaaagagatcttgcggacggtgaaggtctcgttcacgccgccgccgtcgcgggcgatgcagacgccttcaaaggcctgaacgcgctcgcgctcgccttccttgatgcgcacgttgacgcgcagggtgtcgcccggctggaattcgggaatggtgcggtcgccgaggacgcgcgccttttcttcggcagcgagttgctggagaaggttcatggttttgtctcctgggctttagcgccctttagctgtcatttggcggggcgaaccccgcgtggtccgcaaggtcaagccttgcgggggttggcggttctggcggcccagaggtccggacgccgttcccgcgtggtctcttcccgctgcgcctggcgccaccgttcgatccttgcgtgatcgcccgacagcagcacctcgggtatctccagcccctcgaacgtccgcggtcgcgtgtactgcggatgctccagaagcccgtcctcgaagctttcggtgctcaggctcgcggcctggcccagcactccggggatcagtcgtacgcacgcctcgatcaccagcatcgccgccgcctcgccgccggcgagaaccgcgtctccgacggagacctcctcgaacccgcgcgcgtcgagcacgcgctggtccaccccctcgaaacggccgcacaggacgacgacgccgtccgcccccctttcgggagagacccattccttgacgcgcgcctgggtcaggggctgaccccgggcgctcatgtacaaaagcggccgccgcgaccggtaagcgccctcgacgaaatcaagagcgcgggccaccacgtccgccttcaatacggctcccggcccgccacccgcgggggtgtcgtccaagaagccgcgcttatcggtggaaaagtcgcgaatgtccactgtttccagcgcccacagccccttctcccgccacgccgtgccgatcagcgacacgcccaaggcgccgggaaaggcctcggggaacatggtcagggcggtggcggtgaaaggcatggcgcgcgctcttagcgcaaaaggaccatccgcgcgcgccggaacatcacgcctgcggcgcgcgcgggatcagggcgtcgtcggcggccgccgcgcgcctgtaggcgtcgcgcgccgtcagcctggccgcataggcggcgaaggcctcccgctgcggcagggtcttgaattgaaggccccagatcacctgcgcgccgagatagacgtcggcggcggtgaactgctctccgcacagccacggatcagccgaggcgacggcgccttccagcgcatttaccatctgctcgaacgagccatagcccgccatcccggcgcgctcggccggcgccaggaggttcagcgccttggccgtgaccgccgcctccacggggccggccgcaaagaacatccaccgcagataggccgcgcgtcgcggatcgcccggcgccggcgccagtccggcgtctggaaaggcgtcggccagataggcgcagaccgcgcccgtttccgtcaccacggccccgcgatgaaccaccgccggcaccttgcccatcggattcacggccagaaactccggcctcttcagctggtcgaaggcgcgcacctcgacgcggtagggctggccggtctcttccagcatccagcgggcgatgcggccccgcgacatggggttggtgtagagtacgaggtcgtcggtcatggcgtgtgtctctccgtatcgtcaggcctggggcgcggcgccgcccgcggcgatccatgcgtccacctgttcctccagcacgtccagcggcaccgagcctgagcccagcaccacggcgtgaaaagccttgatgtcgaagcggtcgcccagcgccgcgcgcgccttgtcgcgcagctcctcgatcttcagctcgccgatcttatagctggtcgcctgacccggattggtgatgtagcgctcgacctccttgacgatgtcgcgttcgctcaagagcgagttccgccggaagtagtcgatggcctgttcgcgcgaccaccgcttggcgtgcaggcccgtgtccgtcaccagccgcaccgcccgccacagctcggtcgaaagccggccgaagtcggaatacgggtcctggtagaagcccatctccttgcccagaccctcggcgtagagcccccagccctcggcgtaggcgccatagccgccgaaccggcgaaagcgcggcatctcgcccagctcctgcgcataggcgatctggaaatggtggccgggcgcgccctcgtgatagctgatgccctcgatctgaggcttcagcacctgggtcatgtccgacaggttgacgtagtagatgccgggccgcgagccgtcgggggccggcgcattgtagaaggcgatggaggcggtggcctcgcggaacggctcaaccgcccgcacctcaagctcggccttcggcagggtcgagaaccactgcggcgcggcggccatcacctgggcgatgaaggcgcgcgcgtccgtcagatactgttccttgccctctggcgtgttgggatactggaagcgcgcatcggtcttcaggaacacaaagaagtcctgcagcgagccggtgaagccgacccgcgtcttgatcgtctccatctcggcctggatgcgcgcgacttccgccaggccgatgtcgtggatccggtccgccgtcaggtccgtggtggtcgagagctgcagccgcgcgttgtagtaggcctcgccttgcggcagccgccacacgccgccgtccttgtccggcatggcctcggccttcgcctgcagctcgcccagcgccgccagcacggtgtcgtacccgcggcggaacggcccggtcagggcctcccggccttcttccagcagccgggccttggtggcggcgtcggcgtccagcgcctcgacctttccggtgaagtcggcccagaccggattggcctcaccgtcatcgaacggcgcgccggcgatcacctggcgggtgttggcgatggacggggcgaacacgaaggccggcgagatcacgcccttgtccgcgcgcgccttcagcacggtggtgacctcgcccatgacgcgctccgcctcgcgaatgcgcgccacataggcctgggcgtcctcgacgctgtccaccgcatgttcgttgatcaggaacaccggaaggctggtggtgggattgcggttggccgcaaacagatagccccagtcacgccagcgctcgcccagccgcccctgcaccacgccgtgctcgaacagccgccagctgacctgactctgaggcgacagggcgtcgtagtcgaagcgcgccttcatctcggccagctgccgctcggccagcgcctgcccctcggccgatcccgcgtcggtgtagtcgtccagcttgtcgtagtcggtcttgaggcccagcgaggtcatgctttcggggctcagcgccagcgattgatcgaaggccgtctcgaaccaggcggcgaggcgggcgtcctcgctctgcgcggcggccagggcccaggcgggcgtcgcctgcgcccacgccggtgcggccgacagggtcgccagcacggcggcggtgatgattgaaatcctgcgcatcggcggctccctccaagaacggctaggggcttcacagggcgacggccgcgaagcaagtgaccgaagcgtcagatgcgcgggcgcaacacctcgatcggcttcatcatcgtcatgcaacccgatccgggggtcggcgttttcagagcttcaccattcagggatacccacaatgcgcaagatcatcgctctgtccgtcgtcgccgccgccctggccgtgtcggcctgcaaccccatctcgggcgccggccgcgacgtccaggccgccggttcggccgtgagccaaggcgccgagagcgccaagaactaagtcgatccttcgacggttcggatcagggcccgccggtcgccggcgggccctttttcatgtctgcgccggttcgacccgcgccgtgtcgctctcggcctgatccgacagtcgggcctgaagcgcggtctgctttcgcgccaccacgaacgccaggatcacggcgaaaacgccgatggcggtggagtagagaaagaacgtcacatagccggcgcccagggcctcgcgcgtcacgccgctggtcgccgcgcccgccgccagcgagccctctctgccaaaagtgatctagctattgaattgagaaagccgcggactccacctttcgctgccgcagcagaagcgcccagcataacagcacagcaggtatgcccactgcagccgttgcggcgaagaacactgcgtaggcttccataagcggtctcccttgttcgagtcgctcaacgattacgcctgaccaccccttcaagaacttgccgagcagagcgtagaaggagctcagcagcgcgtattgtgtggctgtatatccaatgctcgtcaggctggccatgtaggcgactagcgccgcgccggcaaaaccttcggaaaagttctctacgaacaggacgctgccgaaaaccggcgtcgacatgccgacgaccgccatagtggtgtatcccaggttggacaggggcccgatcagtgcgcccagcaacagggtcttgccgaagccgaaccgcacggcgaacagtccgcccgccgcgatgcccaggaaggctgcgatcagaccgacgctcagccgcattgcgccgatggtcggcttgtcgaggccgaggtcggtatagaagggtccgaccatcggccccatgacgaagtccggaagccggtagagactgatcgcggccagcatcaggaaggcagcggcgccgtgagttttcaggaaggtcaggaacgggccgaaaatggagtcgaataggccatgcggggacagcagcgagacctgacctgttgcttgggccaggtcgcgacgatcgacgggctccttggcgaacagggtggcgatgatcgccaggctcatcgccgcgccccagatggcataggcgccgttccatcccagccaggtggcgaagaacaggatcagggcgttaccggcgagaatagcgaagcggtatccgagctggaacgcggaagtcagcagcgcctgatcctcgtcgccttcggcgctttcgatccgccaggcgtccacgacggtatcctgggtggccgaggcgaaggcggtgaccagggcggcgacgcccagcattgtgagaccgccctcgggtccgatgatcgccatagtgatgagcgacaggccgacgaggccctgggacagcagcatccagccacgccgccgcccgaaccggccgaggaagggcacgtcgaaccggtcgactacgggcgcccacaggaatttgaacgaataggccagaccaacccaggagatgaagccgatcgcggccagctccacaccgccttcgcgcagccaaaggcttaaggtcgcgccggtcagaaggaagggcagaccggaaccgaaaccgatcaccaaggcgatcagaacccgtgcttgaccgagcgctttcagcacatccatagagcctgtagcctttttctcggtcggaccttccgacatcggcacagggctggcgctctctgcgccgcgcgattcggcgttgatcgggctactgggcggctggttagtcattgcgggcggcctctctcgaagggcgcccgatctgatcgccgggtcgccctatccgaaggcgaccttggcgcgaacggcgccgctcgtccagcgggccagggccgcacgcagcgcctcgggctccagcggcttggccagatggtcgtccatcccggcctccaggcacaggcggcggtcctcggcgaaggcgttggcggtcagggccaggatcggcgtgcggtcgccgcccgcgcggatcaggcgcgccgccgacggcccgtccaggcccggcatccgcatatccatgaagaccaggtcgtagcgcgcgcgcttcaaggcctcgaccgcctcgtcgcccgtgccggcggtctccaccacgcagccctcgcgccgcagaagcgtgcgggccagaagcgcgcccaccggattgtcctcggccagcagcacccgcaccccggcgaagcggaccggctggacgcggtcgtcctcgatcggggcggagggcgccgcttccgacggctggcgctgcgccgccagcacccgctcggccagcgaggcgcgccgcaagggcttgatcagatagccgctgaagccgagggagcgatagcgcgcgatcagctcgcgctcgcccggcttcagcagcacgatggcgcgcgcgccgaccggcgcctcgaccagcggccggcccccagccggagccagggtgtgatcgaccagaacgacggaggcgtcgtccgccacccgtccgccggacgcttcgatctgtgcggcggcggacgcccggaccagcggatcggcgacgcgcagcgcgacggcgcagccggtcaggggacggtcgcgcgcgatggcggcggcctcgaacgcggcctcgaagcggaaacgggcgccggggccgtccggacggtcctcgaccgaaaccttgccgtccatggcctcggccaggcggcggaccaccgccaggccgaggcccgcgccgtccacgcgcaccgcgtccgaggcgtctgcgtggccgaactcctcgaagatgcgggcgcgcgcctcgaccggcacgccgggaccggtgtcctcgaccacaaaggccaggcgcggccgcgcgcgcgtgccgccgcagcgctcaacggcgatgcgcaccccgccggcctgcgtgaacttcaccgcattgccggccaggttgaacaggatctggcgcaggcggccgtcgtcggcgatcacgtccggcgcgtcggccgcgaccgaccaggcgatctccagccccttgtcgtgggcgcgggggctgagcagttcggccaccccgcgcgccagcccctccagatccaccggcgccaggtcgaactccagcctgccggcctccagacgcgcatagtccagcaggtcgttgaccagccccagcagatgctcggccgactgcagggcgttgtcggcgtaagcgcgttgcgccccgtccagccgcgtgcgctgcaagaggccgatcatgccgatcacgccgttcaggggcgtgcgcatctcgtggctcatcagcctgaggaactgctggccggcgggatcgaccgcgggcggcgtcgcggtcttgcggggcttccgggcggcctgggtcatgcgcgtctcccacgtgcggggccgagcatggacaaggaagcgttaaggatgccgtaagcgcaggcctagtggacgaagggcgtctgggcctcctcgcgcacgccgagactgcgcgccgccgacgcccggtcgaagtcgccctgagcgtccacggtggtgcggcgatagatcagggcctcggcgatgtggcggcgcagcacgcccgccgatccgtccagatcggcgatggtgcgcgccaggcgcagggtgcgggtccagccgcgcgcggtcaggccgccggcctctcccgcgcgcatcagcagcgcacggcccgcctcgtcgggcgtcgcgaaccggtcgagcagctcgccgcccgcgcgggcgttgaccaccggatcaagcccggcctcgcgcatccggtcttcggccatggcgcgggcggcggcgacacgggcgcgcgcttcggccgtgccttcggccggcgggggcaaggccatgtcggcggcggtgaccggcggcgtctccaccgtcaggtcgatgcggtcgaacatgggaccggagatgcggttctgataaccgcgcgggcagcgcggggcctggccgcaggcgccgcgtcccgccccgcccatgccgcagcggcaggggttcatggccgccaccagctggaaccgcgccggatagcggacatgggcgttggcccgagccaccacgatctcgccggtctccaacggctggcgcaggctgtccagcgcctgggccgaatattccggcagctcgtccaggaacagcacgccgttgtgggccagcgacgcttcgccgggcttggccttggcgccgcccccggtcagggccgccatggaggcggaatggtgcgggctgcggaacggccggtcgcgcgtcagcgtcccgcgctcgatcaggccggcaaccgaccagaccatggaggtctccagcagctcctgcgaggtcagcggcggcagcaggcccggcaggcgctgcgccatcatcgacttgcccgatccgggaggccccatgaacaggatgttgtggccgccggccgccgcgatctccagcgcgcgcttggcgctttcctgacccttgacctcgcgcaggtcggggacgaccccgccctcgaccatggcgcccggctcgggcggccgcagcacctgggttcccttgaagtggttgaccaggccgatcagcgaacggggcgcgagaatgcgcgcatcaccggcccaggccgcctccggcccgttcgcttcgggacagatcaggcccagccccatgccgtccaccgccacagcggcgggcagggcgccgcccacgcgcgcgatctggccgtccagccccagctcgccgatcgccgcccagccgtccagcgcatccggcgccacaacccccatggccgccatcaacgccagcgcgatcggcagatcgaaatgactgccctccttgggcaggtcggcgggcgcgaggttggcgatgatccgctgcgacggcagggccaggccgatcccggcgaaggcgccgcgcacccgctcgcggctctcggccaccgccttgtccggcaggccgacgatggtgaagatcgtctgctggttctggccaaccagctgcacctccacgtccacgcgccgcgcctcgaccccgtcgaaagccaccgtcaccacccgcgcgaccatgcgttcctccctcagccaagaagaacgaaccatgaacccagatcgattgcaagagcggcgctatgcggcgcgcttggcctcgatcgcgtcccacgtcagggcggcggcgtcgacgccggagaagcgcttcagctgctgggcgccggtgggggaggtgacgttgatctcggtcaggtagtcgccgatcacgtcgatgccgacgaacaggaggccccgctcacgcagcgtcgggccgatggcggcgcagatctcgcggtcgcgcgcggtcagctcgaccggcgcggcggtgccgccgacccgcaggttggagcgcacctggtccttggccggcacccggttgatggcgcccaccggctctccgtcgatcaggatgatgcgcttgtcgccggccgagacggcgggaatgaacttctggatcaccagcggatcgcgcgatcccgcggcgtggatctcgatcagcgcctccaggttcggatcatcggccttgagccgcaccacgcccgagccggccgcgccgtgcaggggcttcagcaccacgtcgccgtggcggcggtggaaatccaccagggcgaccggatcggacgagatcagcgtcggcggctgaagacccggaaagcgcgtcgccagcagtttttcgggcgccgagcgcacctcggccggatcgttcaccaccagcgtcctggggtgcaccgtctccagcagataggtggcggtgacataggccatgtcgaacggcgggtcctggcgcatcaggatcacgtcgacgtcctccgacaggtccagccggacctcttcacccaaggagacatggtcgccttgggtctggcgcagggtcgcggggcgggcgcggcagaacaggcggccgtcctccagcgccagggtgcggaagtcgtagatccacagggcgtggccgcgatcctgcgccgtcgtggccatcagccaggtggtgtcggactcgatgttgacggactcgatggggtccatctggatggcgacgcgaagcatgcggaggtcctggcggcgggggtcagcttcgctaatgggtccgccgctcgcggggcgcaaggccgcgccggaggatcagggcgcctcgggcgcttccggagcctctggcgcttgcggcggctcgggcatgtcctccagcgactcttcgacctccgccagggcgtattcggtcatcagcttgtaggtctcaagctgctccgggtccggattggtccaggcgctgttggcggcgatgcccgttcccatggccgaggcctgctgcagctgggcctgcacctccgggtcgttcatggcctcggccaccacggcgtccacgtcgatctcggccagggcctcggcggcgatggcgccggcggaggcggcggccatggcggtgaaggcggtgacctccggctggtgctcggcccacagggcggcgacgcggccggaacgctcgctttcgctcagggattcgtcggcggcgatggcctcggcgcgggcgccgaaggcctccatgcgtttttcgaacgcctcggcggccgcctccagccgggcttcggcggaaggggcgggcgtcgtctgctgcgccagggcgggcgtggcggcggacaggatggctgcggcggaaaggagggcgcggatcatggcgggcttccggtgtttgaccggctgaagcgtccgccgaacacggcccggcctcaagtgaaatcgcggtaaggcgaggctacagccgcagggcgatcagcaccgccgcggtcagcagaagcacgcccacgaagacgttgaagccccggcggaagcgcggctcgcgcatgcgtctcgacagggcggcgccgaacagggcgtaggtgctcatggccagcgtatccagcccgatcatggccacggcgaacagcgcaagctgcggccacaccggccgggttgtgtcgataaacggcggcagcacggcggtgaagaacaggatcgccttggggttggcgatctgcaccgcaaaaccgtcagcaaaggcgttgcgcccgcgccggaccgcgatctcggacggatcggaggggttgcggaacgcgccgtgcagcgccttcaggcccagccaggcgacatacagggcgccgccgatggcgatcagccggaacaccgccggaaaggccgcgaccagcgcgcccagccccagcgcggcggcgccgaaccagaccaggctggcgctgttcatgccggccacgctgaccagggccgaggcgcggccccgctgcacgcccgaggccacggcgaacaggttcgccggaccgggcgtcaccgccatcaccgccatgatccccagaaaggtggagaacaggtgcggatcgacaggcaggacgggcatcgcggcggtgtcgggcccgccgccgcctgcgtcaagcggggatcagtgctggtgcggcgcggccgccggcgccgcgggctgagcggctgcggcgccttgagccgcggcctgttcgacctggccgcgcacctgggccggcacggccttgatggtgggaacggcggcggcgatgccgctggtgatggcggcgcgctgttcttccggcgcgagcgcggcctgcgaggcgccgaagctctccaggtcggcggcgaaagtgtcggcgtcggcctgatagcgggcctgaatggcgtccaggtcggtcttggccttggcctggtcgccggcggcggcggtgaccgcggcctgcatctcgccggccatggcctccatgcgctggccgaaggcctcgcccttggcgttgaaggcggcctcttcagccgagggggccggagcggcggcggcggcaggcgcggcgggggtctggaccggcgtctgggcgggagtctgcgccagcgccggggcggcgacggcgagggtcaggatggaggcggcggcgatcaggcgcatgggacaggctccggaaaaacaggaccgccaccgtgacgcgggatcacggcggcggcaaggcgtgcttatggttcccgggcgggcgtcagccctcgcgctggtcccggcgcgccagcacccgcaggcgcagggcgttcagcttgatgaagcccgccgcgtcgcgatggtcataggcctgcacgccttcctcgaaggtcaccaggtcctgatcgtagagggagaaggggctttcgcggccgatcacctggacattgcccttgtacagcttgacccgcaccgtgcccgagaccttggcctgggaatggtcgatggccgcctgcagcatctcgcgctcgggcgagaaccagaagccattgtagatcagctgggcgtatttcaccgccagctcgtccttcaggtgcatggccccgcgatccaaggtgatcgactcgatcccacggtgcgcggccagcaggatggtcccgcccggcgtctcatagaccccgcgcgacttcatgccgacgaagcggttctcgaccaggtccagccgtcccacgccgttgtcgtgccccagctggttcagacgcgtcaggatctcggccgggctcatcgcctcgccgtcgatcgagacggcgtcgccgcgttcgaagcccagggtgaagacggtgggcgcatccggcgcgtcctccgggctgatggtgcgctggtgcacgaactcgggcgcctcgaccgccgggtcctccagcaccttgccttcggacgaggagtgcagaaggttggcgtcgaccgagaacggcgcctcgccgcgcttgtccttggagatcgggatctggttcttctcggcgaagtccagcagggcctcgcggctgcggaactcccattcgcgccagggggcgatgacgtggatgtcggggttcagggcgtagtagctcagctcgaaccgcacctggtcgttgcccttgccggtggcgccgtgacagacggcgtcggcgccgacctggcgggcgatctcgatctggcgctgggcgatcagcggccgggcgatggaggtgcccagcagatactggccctcgtagacggtgttggcccggaacatcggaaacacgaagtcgcgcacgaactcctcgcgcaggtcgtcgatgaagatgttctcgggctttatgcccagcttcagcgccttttcgcgcgccggccccagctcctcgccttggcccaggtcggcggtgaaggtcaccacctccgcctcatattccgtctggagccacttcaggatgatggaggtgtcgaggccgccggaataggccagaacgaccttcttgatcggcttagaggagctggaggacatgggcagggtctttcgcggccgctcgggggaggaggcggggaaggattggatcgacgcgcgcataagacccgcgccgccctgatgcaaattctacggtcgtggacgggccgtcagcgggtcaggtcggaccagcgccagcggtcgcgccccagcgccacacgcggcccgccgggccggtcggtcagagagatcaccaccagcccccgcaccggcggcgcccggcaggcggcgggcgcgaacgccacctcgaccgccaccgcctggcgcacggacgccaggcccttcccgtcctggcctcggctgcgcagccagtcgccatcccagatcagcagggcgccgccgggtccgaattcgtcctgagcccgctcggccgccgccagcacggccggcgcgtcgcgcaaggcgtcctgcagccggcccaccatgtcgcagccgccgttggagccggagcccgagcccccgccgatcccggcgcccgatccgccgccaaccccgccgcccgaaccgccgcttccgctgcctgcgcccgcgcctcccgccgcgccaccggccgtgagggcgcccgccagcgcgccgtcgccgatgcggcggatcaggtcgctcggctctaccgccacggcgatgggcggaacggacgagggggccggcctcagcgccggacggggccgcacgggcgtgggcggtgtctgaacgggcgatgtggccggacgcctcaccggcgtgggcgcagggttcggctgggggcgtctcgggcgcgggcgcgggcggcgtggggctggcggcgtcggcggcggctcggggcgtcggcggccggcgatccgccgccgccggcctctccgtcgggcccctgaacgggcgtgaccggcggcgtgggcggcggaacaatcgtcacctccaccactgcgggcggggcgagcgtggcctccggcgctcccggcagcagcatcagcgccagcaccgacagatgcagcagcacgctcgccgccagcgcgcccgggcgacggtttcgcggcttggcgggggataggcgttggggagtcatccagcctccggtgacggggacgacgctcccgatcggcacagcatcaccggcaaggcgtccgcatcgtggcggaacttacggccaagctgccggtttctggcctcagacgcgacatgaggaggccttgtgccgccgtccagatgacgatcgtgtgatggaccgggcgttcccccgcgccccaacaggagaaaacaccttgaaccgttccaagatgagaaccgcttccgtggccgccgtattgctcgccgtcggcgtcgccgccagcggctgcgccagccaccgcttcgtgcgcgatcaggacgcgatcgtgaacagccgcgtcgacggcgtcgagcagcgcgtcggccaggtcgaaggcaccgcaggagaggccctgcgccgcgccaccgccgcccagcagctgctggagaacaagttcctgtacgaagtggtgctgtcggacgactcggtgaagttcccggtcgagggcgacaccctgtcgccggaagccgaggcgcgcctgcgcgagctggtccagcgcctcaaggccgagaaccgcaacgtctacctcgaaatccagggccacaccgacgccaccggcgacgccaaggccaacgaagcgctgggcctggcccgcgccgaggccgtccgccgcttcatgagccgcgagggcatcgccctgaaccggatcgccaccatctcctacggcgacaccgcaccggtggcccccaacaacacccgcgaaggccgcgcccagaaccgccgcgtggcgatcgtcgtcctcagctaggacgtcgcttcactggacacagaagggggcgaggcgccttggcgcctcgcccctttttcgtgcggccatgagaaaaggggcgggacctttcgatcccgccccttccattcaagcgatgagcctggcgtggcttagaagtccatgccgcccatgccgcccatgccgccgcccatgtcgggggctgcaccggcggaggccttcttcggcgcgtcggcgacggcggcttccgtggtgatcaggatgccggccaccgaagcggcgtcttgcagggccgtgcgcaccaccttggccgggtcgatcacgcccatctggacgaggtcgccgtactcttcggtctgggcgttgaagccgaacgaggcgtcggtgttctccagcaccttgccgaccacgatcgagccttcgacgccggagttctcggcgatctgacggatcggagcctgcagggcgcggcgcacgatggcgacgccggccttctggtcggcgttgtcgccttccacgccgttgaggaccttggaggccttcagcagggcgatgccgccgccgggaacgatgccttcgtcagccgcggcgcgcgtggcgttgagggcgtcgtcgacgcggtccttcttttccttcacttcgacttcggtcgagccgccgacgcggagaaccgcgacgccgccggccagcttggccagacgttcctgcagcttttccttgtcgtagtccgaggtggtgtcctcgatctggcgcttgatctgggcgacgcgggcctcgatgccgtccttttcaccgacgccttcgacgatggtggtgtcgtccttggtgatcgagaccttcttggccttgccgagcatgtccagcgtgaccgactcgagcttgatgccgaggtcttcggagatgacctggccgcccgtcaggatggcgatgtcttccagcatggccttgcggcggtcgccgaagcccggagccttgacggccgcgacgcgcaggccgccgcgcagcttgttgaccaccagggtggccagggcctcgccttcgatgtcctcggcgatgatcagcagcggacggcccgactgcaccacggcttccaggatcggcagcatggcctgcagcgacgtcagcttcttttcgaacagcaggatcagcggctcttcaaggaccgcctccatcttgtcggcgttggtgatgaagtatggcgacaggtagccgcggtcgaactgcatgccttcgacgacgtcgacggtggtgtcggcggtcttggcttcctcgacggtgatgacgccttcgttgccgaccttggccatggcctgggcgatcagctcgccgatttcgctgtcgccgttggccgagatggtgccgacctgggcgatctccgaattgttggagaccggcttggagttggtcttgatctcctccagcaccagggtcacggccttgtcgatgccgcgcttcaggtccatcgggttcatgccggcggcgacggccttaaggccttcctgcacgatggcctgggccaggacggtggcggtggtggtgccgtcgcccgccttgtcgttcgtcttggacgcgacttcgcggatcatctgggcgcccatgttctcgaaggcgtcttccagctcgatttccttggccaccgagacgccgtccttggtcgagcgcggggcgccgaaggacttctggatcacgacgttgcggcccttgggacccagggtcaccttgacggcgttggcgaggacgttgacgccgcgcagcatcttgtcgcgcgcgtcggtgttgaagtttacgatcttagcggccatgcgggctgctcctatctaatggattgagttgaagaaaacgtcgatgcgtcgggtgcttaggacagcacgcccaggacgtcggattccttcatgatgatcaggtcgtcgccgtcgatcttgacctcggtgcccgaccacttgccgaacaggatgcggtcgccggccttcagctccagcgcgttgaccacgcccttgtcgtcgcgggcgccggggccgacggagacgacttcgccttcctggggcttttccttggcggtgtcggggatgatgatcccgcccttggtcttggattcttcttcaacgcgcttgaccagcacacggtcgccgagcggacgaaacgccatcggtctctctcccttgatgccccggtgggggcgaggtgaacggtttcgcgggcgctccccctggtccctggcaatcgggacgggagagtgccagcgcgagcgggaggtaggcggaggcctcttcgccgtcaaggccgcgcggatgaacgcccgatgaacatttcccaacagggtcgttcagcctgacccctctagaagggacgcaacggatcaacaggaggacgccatgtccaacaccatcaagatcacttcggccgttgtcgccccggtcatcgccctgggcctgatggcggctccggcatcggcccagagctggcgcgaccgcgatcacgaccgcggcgagcgcaccacccgcaacgcggtggtgggcgcggtggtcggcggcatcgccggcgccctggtcggcaacggcgacgggacctacatcgccggcggcgccctggcgggcggcgccctgggcgcgctcagcgccaacgaccgggatcgccgctacgacaatcgctacgatcgtcgctacaacaacggctacaactaccggtacgacaaccgctacaacgccggctacgaccgtcgctactatgaccgcgatcgtcgcgattaccgccgcgaccgcgactaccgctacgaccgtcgctggtaagccggtcgcagcctgaaggcccgaggggcgtcgccggaaggcggcgccctttctttgttttagcccatcagccggttcagcagggccgccgtggacggatcgaggtcgtccgaaggcgcacccgccttcacgtcggtcaggatcgccttggccagcaccttgcccagctcgacgccccactgatcgaagctgttgatgtcccagatcacgccttccacgaacgtcttgtgttcatagagcgccagcagcgcgcccagcgtgcggggcgtcagccggtccatgacgatggcggtggacggccggtttccgggaaaggcgcggtggggggccaggcgatccgcctcggccgcgtccatgccgcccgccagcatctcgtcccgcgccgcctcggccgtcttgcccagcatcagcgcctgcatctgcgccagggcgttcgaccacagcgggctttcgggcgcatcggcgtgggtgctgcggaccaccacgaactcggccgggaccacctgcggcccctggtggatctgctgaaagaaggcgtgctggccgttggtgccgggttcgccgaacaccacggggcaggtctggcgctgaacgtcggagccgtcgcgccgcacccgcttgccgttggactccatctccagctgctgcaggaaggacggcaggcggcgaagcgcatgggcgtagggcgcgaccgtccgcgccgggcgatgcagcccgtcgacgttgaacacctgggccagcgccatcagcaccggcgcgttccgctccagcggcgccgaaacgaaatgcgcgtccatctcggcggcccccgccagcatcgcctcgaacacgtccggccccagcgccaccgcgcacgacaggctgaccgccgaccacagcgaatagcgacccccgacccaatcccggaaggcgaacgtccgcccgcagccgaattccgccgccttctccggcgcggccgtgacgccgatgaagtggttggtcatcccctccggcggcagggcgtcccgcagccacgccttggccgcctcggcgttggccagggtctcctgcgtcgtgaacgtcttggacacgaccaccacaagggttgtcgccgggttcaacccggtcagggcctcggccatgtcgcgcggatcgatgttggcgacgaagcgcagatcgatctgcggctccagcgggcgcagcgcatcccaaaccacgcgcggccccaggtccgatccgccgatgccgacatggacgatggcggtgaaccgctcgccggtcgctccgcgcaggtcgccggatcgcaccgcctcggcataggcgcggatgtcggcgcgcacctggtccacctcggccgacaccggctcgcccagcgcgtggaagtccgcgccctgttcggcgcgcagggcgggatgcagcaccgcccggccctcggtcaggttgaccgcctccccggcgaacagggcggcgcggcggccctccacatcgacggcgcgcaccagatccaggcaggcctcgaacgcttgttgcgtccagctttgcttggacaagtccagatggaggccggcggcgtccgtcgtcatgcgcgacagccgctcgggatcggccgcgaactgatcgacgatgcgggccgacgcggcctcgctcgcggcggcgtcgaaggcgctccaggcctgttcgggcgtcttggtcatctgcgtctccggcgcggcgtcatggtcaaggcctcgtttacggttgaggcgtaagcgggttctaacgcgaaaaggaacaatcgccatgtcctgcggcctcgccctcgccatcgccctgatgaccgccgatccgtcggtcgcgctcgcggccgcccagccgccggcccaggccggagctccggtctccgtcgcggccgagcccctgttcgccgacatcatcgcccgctcgcagcggctgaaggcccaggtcgacggctgggccgcctcgggcgcggccaatgcgccgggcttcttcgccgccgagccctacacagtcttcaggggcgaggccgaacggctggccgccctggacatgcaggggcacctgatcctgaaggagcggggcaccgacggcgacctgaagtgcatcctgcgcggcatctccgaggacatgccgaagaagatcgcggcggtggaggcggcccgctcggacggcggccgcgccaccgccctgtcggagctgtcctacctgctgaacgacaacgtcgaagtcatcaccgccccgcccgcgccgccggtgtagactcagctctctccgcccccgtgttcgtcatcctcggacctgtcccgaggatccagactcccggtgggtgaggccgtgaaccgccgggtgaaccgggagtctggaccctcgccacaagggcgagggtgacgggagtgcgggaccaaaggcgcgaacaggccgccttcactccgctttcagcgcatccacgaccaggccttcggtcagcagctgcggcagcacgcgcggctcgccgccgcccgccggatacagcagatacaggggcacgcccgagcggccgcgcgcctccagctcccgcgtgatggcgtcgtcgcggcgggtccagtccgcaaccagatagactccgtccgccgcctccagcgcctcggcgaccttgcgcgacgacagggccgcgcgctcgttgatcttgcaggtgacgcaccagtcggcggtgaagttgaccagcaccggttggccggcggcgcgcgcttcggccaccgctcccggcgaccacgggcgggcgtgcagcggcccggattccgacaccgccggcggctcggcttgcgaggcggccacgccggcgacgccgacgcccagcgccagggccgccaggccagcggcggcgaggctccggctcccgcgtccttgcgcccggcggctctgcacccgtccggtgagccacaggccgacggcggccagcaggctcgcggccagcagcaggatcagcgccgtctgaccgccctggcgcgcgaacacccacagcagccaggcggcggcggcgtacatcggcagggaaaggacctgtttcagccgctccatccacgggccggggcgcggcaggcgccttagcaggcggggcgacaggctgaccagcagatagggcagccccagtcccagccccagcgccagaaacaccgccagcgccgccggccacggcatcaccagcgcggcgccgagagccgcggccatgaagggggcggtgcagggcgccgccaccaccaccgcaagcgcgccggtcagaaaggcgccgcccgcgtgatcgccgctccagcgcccggcgcccagcgactgaagacccgcgcccatgtggaagacgcccgacaggttcagcgccaccgccagcatcaccagcgccagccccgccaccaccgccggcgactgcagctgaaagccccagccgatcgccgcgccgcccgccctcagcgccagaagcagccccgccagcagcagaaaggtcaggagcacgcccgcgacaaaggcgaacccgtcgcgccgcgcccggcgaggctcgtgcgccgccgccgacagcgccgccgccttcatggccagcaccggaaagacgcagggcatcaggttcagcaccagcccgccgagaaaggccaggcccaaggcctgaagcaccgcagccgcgccattggcagcgggctgggtcggctcgtcggaccagggctgaaggtccggcccgccggctgcgccgggcagcgccacgccgggcgtcgccgtgatttcccaagccccgcgatcggtggccaaaacgcccgacagcggcgcatcgcccctccgcttcggcgtcagcgtcaggctcacgccgtcaggtcccgcccgtccgggctggggcgcggcgtggtcgatggcgtcgagatcgtagggaaagaaccaggcctggcgaatggcctcgccggccagggcgccgccggtcgccgtcagggtcaggcggccgccgtcgcgcgtggcgcgggcggtgatggcggcggggcggggcgcggcctccaccgcctgctggatcgcggcgccccacggacgcgccagcggcgccgcgccgtctcgcaccggcagggcgaggctcagcaccagcggctcgggcacgcacagggtgtcgctgcacaccagaaaggtcgccgtcaccgacaggttcagggtcgagccgacgccggcggacgccggcacgctcagcgtcacgggcaggaagacctcgccctcgtagccgtagttgaccaggctcatcagccgctggcgcgtcggcaggggccacaggatcgggcccgcctcgacaccgggcggcaggcgccacgccagcgtcgtggccccgcccgagtcgcccggattgcgccaataggtgtgccagccctccgcgatgttctggcgcaccgccaccacgacggtcgagccgggcgcggcccaggcgctcatggggaccagttcggcctcgatccgctcggtgcgcgcgggctgggcctgggtcggcgcagcgaagcccaggaccgccgtcagcagaccgaaaagaagaagcagcaggcgcaaagacaggaaccggacgcgaggaaacagaccctcaacctagagcccccgctcccgccgcgccaccggcggcggcgtcgcggctcagcgcggccgtgcgtcaatcacgatctcggtgcggcgccgcaggggctcggccgcgccggcgtcggtcaccgcattctggtcgccgcccgccgccacgtcgaaggccggcgcgggaaggccggccgacgccagcgcctgcgcggtggtgcgcgcccgctgctgcgacagggacaggttggcttccgacgcgccggtggcgtcggccaggcccagcacccgcaccgtctcgatccggcagggccgcatccgctcgcccgccagcgcgatcgcctgcgccgcatccggcgtcagccgcgcctgcccttccgcgaaatagatgtcgaagcggtgcgccgcgcactgcggcgtctccgccaccagcgcctcgcgcgtcggcgcccctgtcgcgcaccccgacagtacgcccgccgccagcatcccgcccatgacaatgaaacgtctcatgtaagcccctcccgccaacccctggcatgaaaagggcggcccgccgcaacgacgagccgccccgaaacctcttcgcgccgtcagccgacgcgccggtcaacgatcaatagcggcgctggccgttgtcccagtagcattcgctctggcggttatcgtagcagtagtagtaccggccacccgagtcgcgatagcgttgctggttggcgcggtcctgcgaggagccgcggatggcgcccgccgtaccgccgatggccgcgccgatggccgcgccctgagcggtgttgccgctgccgttgccgagcaggccgccgacgaccgcgccggccgccgcgccgatggcgccctggcgaaccgtctcgttggtgccgtagttgttgccgccgtaggggtcgctggcgcaagcagaggccagaaggccggctccggcgatggcgataatggcctttttcatggtgtgatcctctgctcttcctgttcgccccgagccacaaacgccgcagccctgctggagttccgcgataaggcgaagcttctcacggccggtcggaacgtctgaacggcaaggcgcgttcgacggccatggacacgcaaaccgtcgacacgtcggacgccgtcgccgcgccggcgccctcttcgctgaaggcgctcagcccgcacgcgccgatgaagcgggtggtgatgctggtgaaccccttgtccggcagcgtggggccgcgagcggcggctgaggccgaggccatccttaaggagtacgacatcgaggcggaggtggtgacgctggagggcggaaagttcgacgcccagatcgacgccgctttcgccaagaggccggacgtgctgctggttctggccggcgacggaacggctcgctcggtcgcctccaaggccaagcccgacggtccgttgatcgctcctctgccgggcggcaccatgaacatgctgcccaaggcgctgtacggcaccaccgactggaagcaggccctgacccgcgccctggaggagggcgagccgcagcctgtgtccggcggcgaggtgcagggcgagtatttctactgcgcggccattctgggctcgcccgccctgtgggcgccggcgcgcgaggcgatccgcaccggcaagatccgcttggcgtggcagtatgggcggcgggccttgaagcgcgccttttcgggacggctccgctacagcctggacggggcggagcggcggcgcagcgaggcgctggtgctgatcagtcccatgatctcacgcgccatggacgagccgaacgggctggaagccgccgccatggacccggtcgacgcggccgaggcgttccggctcgcggccaatgcggtgttcaacgactggcgccaggacccttccgtttcgaccaaaccggcgcggcgcatcgaggtgcacgctcgctcgcgcattcctgcggtgatcgatggagagcccatgctgttgaagcctgacgcggtggtgcgcttcacgcccaaggcgttcaaggcgctggtgccaagacctccagcggcggaggattcgatctgatgggacgcgtgctgcagttctcggacgtccacttcggatgcgagcacaagaaggccgtggcggcggcgctggaatacgcccatgcgacgccgaacgacctggtgctgatcaccggcgacatcacccagaagggctatccggtcgagttcaaggcggcgggcgaatggatgcgggccatgcccgagccgcgcttcgtcatcgtcggaaaccatgacgtgccttactgggacgcgctggcgcggatgttccatccctggcgggcgtttgagacggcgaccggctttcccgcgcacgacggccagttctgcaacgagacggtgatggtgcgcggcgtcgtcaccgcgcgcggctggcaggcgcggccgaactggtccaagggcgtgatcgatctggaccagacccgacgggcggccgaggcgctgcgtcaggcgccgataggggccctgcggatcctggcttgccatcacccgcttatcgagatggtcgggacgcccatgaccggcgacgtcaagcgcggcgacaaggcggcgctgattttcgccgaggctggggtcgacctgatcatgtcgggccatgtgcatgtgcccttcgccctgccgatcgacctggcggatcgctgctcctacgccatcggctgcgggaccctgtcgcatcgggagcggggctcgccgccggggttcaaccaggtggactgggacgccaagagcatcacggtcacggccatggcctgggacggagaacgctacagctcgcaccagacctggcgtttgccgcgccggcaggacacccgcaaggcggccaccgcccccagtccggttcagcccggcgcgctggagaaggcggcgacctgagcgtcatgctccgccgcgctcgagcgtcgcgcgcggcgccagacgggacgacatgggaaaagggccggatcgtgcgatccggccctttcttgtgtctggctgttcctgtggctgctagagccgcggcgagccgcgtccgcgaagaccgcccgcgaccagggcgatcacgaacaggataatggcgatcacggcgatgaacttggcgatctcgaacgagaagttggcgatgccgccgaagccgagaacagccgcaatcaacgccacgaccaggaaaataatagcccaacgcatcatgactggggtccttcctgagagttgatgttcgacggcttcggaagtgtccttggcctgtcaagtcataaacgtggcgatgacttgcgcgttccggcggaagtcgagattcgactccgctcagcgacgccgacgatagccgcggcgctccattttccgctcggtcacgaagctggccacgatggccgccagcgccgggttgcgaagcagcaggaacagggcgcccagaccgccgaccgcgccgatcatcgggcggtccttgatcaggtgcagcgccttggccgccaggccttcgggctcttcgtcctcgtcatggtgatcgccggcgtccttcttgaggaagaccaccgcgacgatcgccgccatcgccgcgaacagggcgaaggtcagggccgaggcgccggcgggcggcaggaccagaaacagcaggtgataaacggtgatccccaggaagatcacggcgaccaggcccgcggcggcggcgaccgcccccgccacgaccttgttgatgaggcccttcagcatcagcgacgacgacccgacagcagcaggccgatcaccacgccgacgcccagggcgatggcggtggactggaccgggcgctcctgcacgcgctcggtgatgtagcgttgggcctcatcgacgcgctcggcggcgtcgtcgtagtactcgcggccgcgcacgcgggcggtgtcatagtagccgcgcgcctgctggcgcacttcgtcggacttctcggacagcttggcctgggcctgggcggccttgtccttgaggcgctgggtctcttcgcgggcgccggtcttcagatcctccttgagggtcttgatgtccgccttgatgtcgtctttcgccttggtggccatatgcgcgctccgtctaagcttggctttaaataggggaccccgttcgccaacgccaaggaaccggcgcggttccattcccgccgcgggggctcgcgccctcgtcagcccgcccgacgcgggataagctcgcctgatgcccgattggcttttcccgccccgcccgcaaccgtccctgcctgtcgagggcgacgaccggcgctttcccgtgcgtcgtatcctttgcgtgggccagaactacgccgcccatgcgcgcgagatgggatcgaagctggaaggccatgcgcccttcttcttcaccaagcccgccgacgccctggtgagcgacggcggcgatcccgcctatccgtccgcgacagcgaacctgcaccacgaggtcgagctggtggcggcgatcggcgaaggcggtcggatcgtcggctgggccgtgggcgtggacctgacgcggcgcgacctgcaggccgaggccaaggcggcggggcggccgtgggacgccgccaagggcttcgaccagtcggccccctgcggcgcgctgcggctgggggacctgccggacgtcgatgcggagatcacgctgcgcgtcaacggcgaggtgagtcagtccggccggctcggcgacatgatcctggacccccaggcggtgctggcggcggcgggcgcactgtggagcctgcaaccgggcgatttgatcttcaccggaacgcccgagggcgtggggccgctggtccggggtgatcgggtgcaggcggccatcggaggcctgccggacctgcggttcaccctggcgtgacccggtggcgccggcctgttaaccccgccgggtaaggttctcgcaaggtctcactgagggtcccttaagctttcggggcgcagggtgcgcccgtgacgaatctctccgcctccgccgacaaggccgcgccgattgaccgattggcgatcgccgtggtcaccgagcccgaacgcgtccgcggcgcggtcatttcggcgccggccggcgcgcgcgaggacgccatgcggtttctgttgcagacggcggcggacgccggcgtccgcaccgtggcgaccaagccgcagggcgacgccgagcgcctgctgggccaggcttggccgtttccatctccgttcggggtgaccgttcgaaccgtgggtctggccgaaggcgccgaccgtgtggaggcgcgggcgcgccgttcgctggaacgactgggcctaccgcgcggcgacgttctgctggtgtccagcgccgccgaccttctgggcgcggaggggcgcgcgctctggagccgtctggaagggttgaaggccaaggggctgtttcgtcggctcggcttttgcgcctccgccgaagaagcggcggacggtctggcgcggcgcctgggcgcggatgtggtgcaggtcggctgcaatctgctggaccagcgcgcggcccgcagcggactgctggaccgtatcgcccagacgggggcggaggtgcatctgtcgtcggtgttcgcgcgcggcctcctgttcgcgggcggcgaggacctgccggcgcacatggccgatcaggcgcagggcctgtcgcggatgcggcggcggctggccgagggtcgatgcgatccgatgcaggcggccctggcctacgccttttcgctcctggccgtggacaaggtgatcgccagcgtcagctccgccgccgaactcagggcggtgatcgccgccgcccatgcgccgtgcccgaacctggactggtcatcgctggcgctggacgcgccggccgccattgcgaccgacgcgccccgttaccggatcagtagcgcagcctgatcccgacatagccggacaggcccggctcgccgtaatccagcacttgctgatagcgttcgtcgaacaggttctcgacccgcgccgtcagcgtcacctgttcgctcagcccataggccgcgtttaggttggcgaccacgaagctttcgcgcgtcgcccgcgcgaaggtgaggttgtcgacatcctcctgatcgccctcggcccgaaccgtcagcgcgccggacagccgctggccggtccagcccaaggtggcggagcctgcgtgctcggccacgcgctgcaggcgaaggccggtggtgcggtcctcagcgtccgtccaggcgtaggccagcgtcaggtcgaagccgccgcccagcagggcccggccttccaactccaccccgtccgtgcgggtctcggcgatgttgacgtagcggccgccgacatagctgatctggtcctcgacgttcaggcgatacagggtcgcgcggccgtccagccgtccatcggcggaggcccagcccagggcgatctcgccgccgtcggctgtttcggggttcagccgggcgaccgggggagtgtagcagaagtcgcacaccgcctggctgatgctgggcgccttgaagcccgtgccgtaggcgcccgagacgatgaagccgccgtccagccgataggccgccgagacccggccggtggtctccgagccgaagtcgtcggtgtcgtcatggcgcagggcggccgacaggttcagccgctcggaggcgtcccagccgccggtgacgaagacggaggtgacggccagatcgtccgcctcgcccgacgacagctcgccggagctttcctcgcgctcggccccgaaggcgtaggtcagattgaggtcgggtcgggcgccgtccgcctgccagcggtaaagctggcggtcgcccgagaaggtcgagccgaagccgccgctgaatgaggtgcgctcgacgtccgatcccgacacgctgaactgatgcgccagacccagggcgttcagacgcaggcggccgaagccggaccactgctccgactgctgggtgtcgaaggtgtcagccagatcgaaggagggagcgggaaagccgtcgatctcggcgtcgccgcgtgaccagcgcaccgagccgtccaccgtagccgccggagacagggcgtagcggccgcgaacgccgatcgtggtgttctcgaagccgtcgtcctccgcattgccgtcggcctcgtcggccgctgaaatcccgtcggtgtcgaagcgcgagacataggcgcccagcgcatactggtcggtggcgacgccggccgacacgcggccgcgcagggtgtcgtagctgccggcctcggccccggcgcgcaggccgtcgatctcgcgcgtggtgaaggcgatccccccgccgatcgcatccgacccccacaaggaggactgcggcccgctcagcacctcgatgcgctggatgtcgcccagctcaaagccggagaagtcgaacgcgccgttgggctcggtcgggtcgttgacgggcacgccgtcgaccagcaccagggtcttgccgggcgtggccccgcgcatgcggacctgcgccaggccgccaaaggcgccggtgcgggtgaccgacaggccgggcacgtcggccaggatgtcggccgcaaagacggcgccgcgctgctgaatggcgcgctcgtcgatgacgcgggcgccgggcgtttctgcgacgatcgcctcgatgcgggtggcggtgaccacgacctcgtcgagttggtcggcggtctgcgccagcacgggggttgaaagaacggcgaggccgagggcaggcgagcagagaagaagggatcgcttcatggagcggggttccgttttgtcgcctccgcgaatgcgcgcgaggaggcggaaaaaagcgagccgacccgccgggccttggggctcggacggcgcaagatcgggtcgcttcgacggaacctgggtccccgcgcctctgtctggtcccggacagcggacgagcgacgtcggcggccaggtctcctggcttgcgggtcctgagccgccgtcctcgccttcccggtgttcccagtggcgccggaatcgcttccggatttggacaacggcctcgccgcctacagttgcgggcacagccgcggtgtctgaccgcgttcccttaaccgccgggcgcggctatcgcaggcgcggtcgcccggcgcaaagccgggcggatggcgcttgagacgacgggcgcgatccgtcaccctgcggccacatgaacgcgcccgtctcccacccgccgaaactggaggtcgatcccgccctgctggagggcgcgacccccttcatggcccagtatctgacggccaaggcgacgcagccggacgccatcctgttcttccgtatgggggatttctacgagctgttcttccgcgacgccgaggtggcggcgggggcgctggggatcacgctgacgcggcgcggcaagcaccagggcgaggacatccccatggccggggtgccggtgcacgccatggaaggctatctcgcccggctgatccggctggggcacaaggtcgccatctgcgagcagctggaggatccggccgaggccaagaagcgcggctcgaaggcggtggtgcgacgcgacatcgtgcgggtggtgacgcccggcacccttaccgaggactccctgctcgatgcacgcggagccaaccggctggcggcggcggcggtgcgccggggtcgggcggccgtggcggtggtggagctgtcgggcggcgcagtggacagcgtggcctgcgggctggaggacctgggcgcggtgctggccgcgttccggccgtcggaggttctggtcaccgaccgcctctacggcgatgaggcggccaagggcgcgctggacggctcgggcggggtggtgcaggcgctggcgcaggccctggccgagccccaagccgcgcgcgcaagggtcgagcggctgtacggcgtcggctcgctggacggctacggcgctttcgaagaggccgaggtctcggcgctgggcctgatcgccgcctatctggagacgacgcaggcgggcaaggtcccggccctgtcgccgccgcgccgcatgggcgaggccggcttcctcgccatcgatccggccacgcgcaccggcctggagatcgaccgcacccagcgaggcgagcgcgaggggagtttgctgcactgcatcgaccgcaccgtgacctccggcggggcgcgcgccctggccgagcggatcagccgccccttgcgcgacgtgcgtgcggtcaacgcccagctggatgcggtggagtggctcaaggaccggcgcgacctgcgtcggagcctgcgcgagaccctgaaggcttcgtccgacgtggcgcgggccactgcgcggctggcgctggggcggggcgggccgcgtgatctggcggcgattcgatcggggctgaagacggccgagatcacgggcggcctgttcgtgggcgctttcgatccgctgacgggcgcgcccgaacgcatcgcctcggtgctggagcggctggcgcccacgtccgacttggcgggcctgcgggctcagctgaccgaagggctggtggacgagccgccgcacctcgcgcgggacgggggctatgtgcaaccgggctttcggcccgagctggacgaggcccggcgcctgcgcgacgacagccgccgggtggtggccgagctggaggcgcgcgcctgcgccgacagcgggatcgccttcaaggtcaagcacaatgcggtgctgggctacttcctggagacctcggccaaggcggccgaggggctgcttcgcgccggccctgacagccccttcatccaccgtcagaccctggccagccaggtgcgcttcaccaccgtggagctgtcggagctggacgcccgcatcagccaggccggccaccgggcgctcgccatcgaagccgacaccttcgagggctggcggcgcgaggtcgcgcggctggcgcaatcgctgcaggcgacggccgaggcgctggcggaactggacgcccatgcggcgctggcggaatgggccgaggaggtcggcggcgtgcggccggtggtcgatgacagcctgtgcttcaccgtggacgcgggccgccacccggtggtggaggcggcggtcaagcgcgaggggctgccctatacccccaacaacgcccggctcgacggctcgggcgacagacgcgcgcgcctggccatcgtcaccggacccaacatggcgggcaagtcgacctttctgcgccagaacgcgctcctggtgatcttggcgcaggccggcgcctttgttccggccaaggccatgcggctgggggttgtggaccggctgttcagccgcgtgggcgcgggcgacgatctggcgcgcgggcgctccacctttatgaccgagatggtggagaccgccgccattctggtgcaggcgaccgagcgcagctttgtggtgctggatgagatcgggcgcgggaccgccacctacgacggtctggccatcgcctgggcgacggccgaggcgctgcaccagaccaatcgcgcccgcaccctgttcgccacccactaccatgagctggcgcagctggagacgcggctggaccacgtctgcaacctgtccatgaaggcgcgggagtggaacggcgagctggtgttcctgcacgaggcggcgcccggcgcggcggatcggtcctacggcgtgcaggtggccaagctggcgggcgtgccgccggccgtggtcgagcgcgcgcgcgaggtgctgggccggctggaggggcaaaaggccgccgtcgcccgcctggacgacctgccgctgttcgccgtcatggagccgccggcgcccgcgccgtcctcggcgctggacgatgccgtgcgggatctggatcccgacgcgctgagcccgcgcgaggcgctggagacgctgtatcggctgaaggcgctggggcgatgagccgccggtgctgacgctggacgaacggctggcgcaggcggcgcgggacgccgacgtgcgcgccgcgaccgcggccgtgctgcgcgagaccttttcggccgggcgcgcccgagccgagcgccggctggaggcgggcgggcaggggcgcgaggtcgcgcgtctttatgcggcggcggcggacgagatgctgcaggccctgtggacccaggcgacgcaggccttgtggcccgtatcggcggtggaggccgagcggctgtcgctgctggcggtgggcggatacgggcggggggtgctggcgccgttctcggacctggacctgctgttcgtgcgctccggccggccgacgccgaggggcgagcaggtggtcggccatgtgctgcacgtgctgtgggacctggggctcaaggtcggctcggccttccggtcggtggacgaggcgctgtcgctggcgcgcgcggacatgacggtgcgcaccaccctgctggaggcgcggccgctggcgggggacgccgggctgtcggacctgctgatcgcacgcttccgcgacatggcggggcgcgccgatccccggcccttcatcgccgccaagctggaggagcgggccgcgcgccacgaaaaggcgggcgccgtccgctacaaggtcgagcccaacgtcaaggacggcaagggcggcttgcgcgacctcaacgccctgttctggatcgcgcggtcgctggcgccggaaagccggcttggcgcggccgtcatggacccgctgctgaccgcgcgggagcggcggaccttcgacgaggctttcgacttcctgtggagggtgcgcatccacttgcacctgctggccgggcgggccgaggagaagctgacgttcgaccgccagccggaggtggcgcggcgcatgggctggcgcggacgcggcgacgagccggcggtggagcggttcatgcgacgctacttcctggtggcgcgcgacgtgggcgccctgacccgcgccttgtccgccaagctggaggcgcgccagcacaagcagccgcaagggctgtcgcggctggcggcgtcgctgctgccggggcggcagaagcggatcgacgcgccgggggtctccgtctccgacgggcggctgacggtggacgggccggaggtgttcgccgccgatccggtcatgctgctgggcctgttcgtgctggccgaccggcacgacctggatctgcaccccgacgccttttcggcggtgacgcggtccctgtcgctggtgacgccccggctgaggcgggacccgcgcgcggccagcgccttcctggatatactggcgcacgggcagcggccgtatcgcgcgctgacggtgatgaacgagaccgggctgctgggccggtttctgccggagtggggacggatcgtcggccagacccagttcaacatgtaccacgcctatacggtggacgagcacacgctgcaggccatcggcatcatcaatgacatcgcgcgcggcaagctgaagaccgaccatccggtggcgtcggagatcgtgcacctgatcgccgacatggaagcgctgatgctggccatgctgctgcacgacgtcggcaagggcggggagcgcggacagctggaggacggcgccatcgccgcacgccgcgcgtgcgagcggctgggcgtcgatccgcgccgcatcgagctggtggtttggctggtcaggaaccacctggcgctgtcggactttgcgcagaagcgcgacctgggcgatccgcagacggtgcgggactttgccgagctggtcggggatcccgagcggctgcggctcttgctgatcctgacggtggccgacatccgggcggtggggccgggcgtgtggaacggctggaagggccagctgatgcgcaccctctacaaccaggtcagcgcggtgttccggggcgaggacgtgcgacggcccgatcccgtcagcgagcatcccgccctggtggagcgcgctcgggccgagggcgcggcggccgaggccgcgcccgtcgcgccggtgcaaggcctcgcggtgcaggcgaccgagctgcgggtcgccgcccaggaccggcccgggcttttcgccgacctggcccagaccatcgccgccgccggggccgacatcaccgacgcgcgggtggcgaccacggatcagggactggtgctggacgtgttccgcatccaggacggggccggcgcgccctacggccaggccgagccgcgccgtctgtcgcgtctggtcgaggcggtcgagcgggcggcgcggggggaggggcgcatcgccaaagcgccggagccgatccccagcgcccggcgcgcggtgttcgaggtccggccggtcgtgatggtggatcaccacgccagcgagtccgccacggggatcgaggtttcgggggccgaccgtcccggcctgctggccgccctgtcgcgcgccatcaccgagcgcggcctgtcgattcgctcggcccatgtggccggctttggcgagcgggcggtggacagcttctatctggtcgacgcgcgggggcgaaagatcaccgacgaaggggtgctgtccgagctacgcgacgccctgcacggggtgctggagccgccgcgcgcccagccgccgggccgccgggtcacagccgcccgcgccagcgcccgcgacgtctccgacctcggccgccgcagtccgcgcgccaagcccgtttcgcccggcgaacaggcgcgctaagcgggggcgtgcggcgccccgccgcgccccaggaccttttcccgcgtgaagccttccgattccttcgagccggccgctccggtcaaccaggccgtcgccaacggcgagccggtggtgcagccacccgccgcctcgaccatgacggagagatccggcggcgtcatgcgctcgtcagccatcttctcgggtctgacgctggtcagccgcctggcgggtttcgcccgcgacgtggtgatctcggcggcgctgggcgcctcgtccagcccggcggcggacgcctacaacacggcgctcagcttccccaatttgttccgacgcatcttcgccgaaggcgccttcgccgccgccttcgtgcccgcctacgccaagacgttgaagaccgaaggggacgcccgggccgaccgggtggcgaccgacgcgctggcggcggtggcggcggtcacggtggtgctgaccatcgccgctcagctggccatgccgtggctgatgacgatcatcaacgtcggcttcctggacgatccggcgcggttcaagctggcggtgatcctgacccagatcaccatgccctatctgccgtgcatggcggtggcggcgctgctgagcggggtgctgaacgcgcgcggacgcttcatcgtctcgggcgcctatccgatcctgctgaacctgatcatgctggcggtggtgatcccggcgcgcggcggccaagtcggggcggcgacggcggcgtcgtggggcgtgctggtcgcgggcgtggcgcaggccggcctgtgctggtggggcgcgcgcaaggcgggggcgaacatccgcctggccctgccgcgcctgacgccggcggtgaaggccatcgtcatcaccgccattcccgccgcgatcggcaacagcgcgacccagatcaacgtcttcatctcgggcaacctgtccagcttcgtccccggcggccggacgtggctggcgacggcggaccggctgtaccagctgccgctggggctggtgggggtcgccatcggcatcgccctgctgccgcgcctgtcggcggcggtggcgtcaaaggaccacgcccagcagcaggcctcgatggacgaggcgctatgcctgtccatggccctgacgctgccggccgcggcggcgctgatggccatgccctattttctgatcgacgccctgttcacgcgcggcgcctttctgcaggtggatgcggtgaacacggcccaggccctgctgcacttcggctggggcgtgccggcctttgtgctgatccgcatcctggcgccggcctttttcgcgcgcggcgatactcgaacacccatgaccttcgccctggtgtcggtggcggtgaacgcagccctggccatcggtctgttcaacctcggcatggggatcgccgggatcgcggcggcggtgtcggcggccgcctggagcaacgccctgctgctcgcctccaccctgtggcggcgcggcgactatcggccgagttccgccgccgtgtcgcgtctattgcgcatcgccctagccagcgcgggactggcgctggtcgtcggcgtcgcctcctgggcccggccgtggatcgaggggccgacggcggacctgctgaacgcggtgcagatgtcggtgggcgccaaggaggtgtccctgttgctggtcacggccgccggcggcctggcctatgtggctctggccttcgccacgcgggcggtgacattggctgaggtcaagggactgctgcggcgcggcggacgctgatccgcttgctctggaggcccggctcgggcattgccgcgccatgtccgacgccgcccccgccgatcccgccccctacgccggtcctcgccgcatcctgtccgggatccaggcgtccggggccctgcacctgggcaactacctcggcgccctgaagcggttcacggcgctgcaggacacgggtgcgccggtgttcgtgttcgtcgccgacatgcacgccatcaccgtgtggcaggacccgcagaagctcgccgaccagacgcgagagatcgccgccgcctatctggcctcgggactcgatccggcgaaatccatcatcttcccgcaatcggcggtgcgcgcgcacgccgacctcgcctgggtgttcaactgcgtggctcgcctgggctggctggatcgcatgacccagttcaaggagaagtcgggcaagcacaaggagcgcgcctctgtcggcctctacacctatccggtgctgcaggccgccgacatcctgctctacaaggcgacggaggtgccggtcggcgaggaccagaagcagcatctggagctgacacgcgacatcgccgccaagttcaacaccgacttcggcgtgcccggcttctttccgcagcccgagccggtgatccaggggccggcgacgcgggtcatgagcttgcgcgacggctcggccaagatgagcaagtccgacccgtcggaccagagccgcatcaacctgaccgacgacgccgacgccatcgccgccaagatccgcaaggcccgcaccgacgccgagcccctgcctgacagccttgccggtctggtcgaccgggcggaggcgcgcaatctggtggccatctatgcggcgctggcgggaaccagccgcgaggcggtggtgcagcagttcgcgggccagggcttcggcgccttcaagccggcgctggccgaactcgcagtcgaggcgctggcgcccgtcaccgccgagatgcgccggctgatgaatgatccggccgagatcgaccgcgtcctcgccgacggtgccgaacgcgccgccgcagtcgccgacccggtggtcgacgaggtcaagcgcatcgtcggcttctggcgcgcctgatctagaggttcggcgacacgtcctcgagaaaggcggcgaagcggcggatcgcctcgtcggccagggtcgggtcgtggcgcatggggccgatgttggacggctcgtcgaaggcgtgggtgccctcggcgatccagctttcgacctcggcgccgcagttgcggatcatggcgttgacgtgctcggcgttccggaccgtggtcaggtgatcgcggcggcaggtcacggccagcacgcgcggacagtgccgccaggccttcagccggttgaaggcgaagggtccgacgtaggggtaggccagccacaccgccttgacgcccttgagcgcacaggcgccggcgtcggtcagccccagagcgccccggcggtccggatcggcggtcatggcctccatgatcgaccagccgccatggctccagccggccagcacgacccggtcgggatcgacgtgggggcggcgtgagataccgtccagcgccgccaggatgtcgccgccgcgctcgtagccgcgaagggtcaggccggtgcagacgcccatgacggccgccgcccggccgatgccgcgatggctgtaggaatccaccacgaacgcccgccagcccagcgccttggccgcctccgcatagcgcggcaggtgcgcgcgcaggccgccgcagccgtggaacagcagcaccgccggccgcggccggtcgtcgtcaggaccgaccaccgcgacatgcggctcaaggcgcgcccagcggctgtgcaggctgtccatcggcccgtcagtgccggaaaacgcgcacgccggtgaaggccatggcgatgtttcgctcgtcggcggcggcgatgacctcgtcgtcgcggatcgagccgccgggctggatcaccgccgtcgctccggcggcgaccgcctccagcaggccgtcggcgaaggggaagaaggcttcggacgcacaggctgacccttgcgccagcgaatgggccagacccttggcctcgccggcctccttggcgcggatggcggcgatgcgcgctgaatcgcggcggttcatctggccggcgccgatgccggcggtctggccgtccctggcgtagacgatggcgttggacttgacgtgcttggccacggtgaaggcgaacagcatgtcggcgacctcggtcggcgtcggttgtcggcgcgtgacgatcttcaggtcttcgggcttgatcaaggaccggtcccgcgcctgaaccaggaaccccccggcgaccgagcggaacacctcgcctgcgcccagcggatcgggcaggctgtcggtgatcagcaggcgcaggttcttcttggcggcgaagacggcgcgggcctcctcgtcggcgcccggcgcgatgaccacttcggtgaagatgccggtgatggcgcgagcgtcgtcgccgttcagcgggcggttgaccgcgatcacgccgccgaaggccgagacggcgtcgcattccagcgcgcgggcgtaggcttccgacaggtcctcgccgaccgcgacgccgcaagggttggcgtgcttgacgatgacgcaggccggggcctcgaactcggccaccagctcataggcggcgtcggcgtcggcgatgttgttgtagccgagctccttgccctgcacctgttcggcatgggccacgcccggccgacgctcgccggtgcggtaaaaggcgccggtctgatgggggttctcgccatagcgcagggtctgggccagtgcgcccgcgatcgacttccggaccggcgcgtcgtcttccagctgcccggcgaaccagccggagacggcggcgtcataggcggcggtgcgggcgaaggcgcgggcggccaggcgcttcctcagggcaagcgaggtcgatccgtccgccttcagcgcttccaggatcatgccgatggactcgccgtccacggcgaccgcgacatagccgtggttcttggagcctgagcggatcatggccgggccgccgatgtcgatgttctcgatggccgcctcgaagccgccgcccgcctccaccgtcttctcaaacgggtagaggtcgatccagacgatgtcgatcgggccgataccgtgcgcgcgcatggcctcggcgtgatcagcggcgtcgcgcacgcccagcaggcccccgtgcaccaccggatgcagcgtcttgacccgtccgtccatcatctcgggaaagccggtcaggtcggccacatccttgaccggcagcccgatcgccgcgatggccgcacgggtgccgccggtggagaccagctcgacccctgcgtcgtgcagggcgcgcgcagccgcctccagtcccgtcttgtccgatagcgagatcaacgcgcgcgcaggcttgaccgcatcaggcgcgggcggaaagtcgggagcggcgggcatggcggcgtccgtgaatggcttggaggaggatggcgcggcctctagcatcggggcggcgacgcgtcacccttgcgccttcaggcctggaccggatcgtcgctcgcgccggcggggctcagcttccagcggaccttggtttcggcgtcggtgcgggccgagccgcgcaccacgatctggagggagcgacgggtcaggccgtcgtcgatgtggacgctgggctcgatcgccacgtcggggccgtcggtgcggaaccaccagccccggccggatgcgccgcgcagcagaatggcccgacggtcgcgggacagggtggcctcgacgccgggctccaggtgaaagcgcgcggcgtagggggcggcgatggcccgcagcacctcggggcggccgggcgtcggataaaggcgctcctcggcccgcagctcgtccaggcgggtgtcgagatacagccggcgctggtgcgtcaggccgaacggctcgacccagccgtcgtggtccatctccagccacacggcgccctcgccgtcgcgctggctgacgtgaacggcgtaggggcggccggcaagcctcggtcccagcagttcccctttccagccgcccagcggttcgttcagcgagcgctcgcccagcgtcagggtggaatgggccggagtcaggcgcagcgcctggcggtcggtggacttgggcgtccagcccgagccggtgatcagccgatcccgcccgcaggtgatctccagcgccagcggctgggcgcaggcggtggagccccaggcgccgtgcgcggccggcgccgcatccgccaccacagccagaagcggactggacaggcggtgaaggccgccgaccacgccggacgttcggggggcctccgcgtcgtcgtgcgcgagagccgccgagatgcgcgccgtggtcgaggggccgccgccctggaagctggcgaggcgcgcgtccggcagggtcaggaggcgaacggcctccgtcaggcgggcgacggcgcggctgatcggttccggcgtgggttccgacagctgggccagggcgtcgtccagcgacagcaggtccagcagcagctccagcgccgcctcgggcgagcggctggcgtgcgatccgtcggtcaggatcgtcgcgtgcagggcggcgggcagaccggccagggcgcgcttgcgcaggccggctccggccactccggacaggacgcagccggcgatggcggcggcgaccgagcgctcggcccggctggccaggccgccgggcgggcgcagcagctgccgcgcctggcgcgccagggtgtcggagaggcgaagacgttcggcctccgtcgccaccgctcccatgcgacgcgcagcgcacgacaggttgatgacgcgccggggcagggtctcggggccccaggcgaacggcgaccagcgcgcgaactggtcggtccaggacagggtcaggcgcacggcctcccgcgcgccgcgctcgccctggctcatcagcgccggcagccagttgaaggcgtgaagctcgaccgcgaaggggcgcgacgggctggggcggccccacggatcggccggcgcctccgcctccagagtcgcaccggccagcgtgaagcgccccttcaacaggcccttgccgggagttggatcgtgcgggcggaagtcgcgcggcgtggctgcgaagctggtggacttggccccgcccagagtcagggtgtagccgggcaggccatagagctcgatccacagctggcgggtcagcatccgtccgacgatggccggccacaggctgagatcggtcggcgcctcgccgtcgcgcacaggcgttcgcaccggcgcgcccggaagtcccgggatggcgcccgcgcccacgtccggacccgcgggcgggcgcggagcgaaggggccgagcgggctcacgcgggggcctgcgccttcaaggcggcgatgttcgaggcgtaggcctccgccccgcccttgaacacgaaggagccggcgaccagggcgtctgcgcccgccgacacgcaggcggcggcgttggcggaggtgacgccgccgtcgacctgcagatgcgcggacgatccggcgcggtccaggacggcgcgcgcgcgctcgatcttgtgcagggcgctgtccacaaaggcctgaccgccgaagccgggattgaccgacatgatcagcaccagatcgaccagatcgacgacctcttccaggatcgagaggggcgtgccggggttgaacacgatcccggccttggcgccgagctggcggatgcggcccagcgtccggtgcaggtgcggcccgctttccggatgcacgctgagaatgtccgcgcccgccgcgcgataggcctccagccatggatcgaccggcgcgaccatcaggtggacgtcgaacggcagggtcgaatgcggccggatcgccttcacgatgtccgggcccatcgtcaggttcggcacgaagtgcccgtccatgacatcgacgtggatccagtcggcgccggccgcctccagcgcccgcacctcctcgcccaggcgggcgaagtcgctggcgagaatggacgggcagatcaggggcgcggtcatgctttcccggatacggcggccgctcgccgggggcaagaaggcgcggctaggcgatgcgctccagccgggcggcgaagaagccgtcaagggcgccgcgctcgggccagaaggacggaaggatgcgcagccagccttcgggggtcagggcctccggcgggcagccgagggccgccggatcggccggaactgtgcggaagtccgggttgcggcgcagaaaggcgatgatctgggtctcgccctcttcgcgctccagcgagcaggtgcagtagaccagacggccgccgggcttcacccgctgggccgcggcgtccagcagccggtgctggacatctgccagcttggccacgtcggcggggcggggggcgcgcagcacttccgggttgcggcgaaaggtgccggtggcggtgcagggggcgtccagcagcacggcgtcgaaccgacgggcgtcttcccagtcctccgccggaaccgccacgacctcggccgacaggccggtgcgctccaggttctgcgccagccgcttcagccgcacggccgaacggtcgagggcgaccacggcggcgccggcggcggcgagctgcagcgtctttccgccgggtgcggcgcacatgtccagcgcggtttcgccggactgaacagccagcagccggccgggcacggcggcggcggcgtcctggacccaccagtcgccggtctcgaagcccggccaggacgccacgtcgccgcggcggccggtgcgcaccgagccgccgggcaggacctcgccctccagcgcctcggccacggcggcgggatcggcggagggtttaaggctgaggtcggtcggcggctcctctcgggcggccagcgccaagccctccagcgcggcttcgccccaggtcgcgcgccagcgggcggcgatccagtcgggcaagttggacgcggcggtggtcaggccgggcccgtcgcggtcgatcccgcgcagcacggcgttgaccaggttcttgtaggggcgggtctttggatcgcgctcggccagcttcacggcggtggagacggcggcgaaggcgggggtgcgcagcaccagggtctgggccagcgcgacccgcagcagggtgcgcacagcgtccggcggcgacttctgcaatcgacggtcgaggatctgatcgatctcgcccagacgccgcagggcggccatggcgacggcgcgggcgaaggcgcggtcagccggcggcagggcgcgggcgggcgcctgcgtcagcgcctcgtccagcccgttgcgcttctccagcgccgcgttcagcaagagccccgccaccgcccgcgcctcgacgccgatgtcgtcctgcggcgccgcctcggcgggcgtcgaggccggacgcggcctgcccttggtggcgatccggcggccgcgcgcctccgaactcttgcccggccgggcgcccggccctctcatacggcgacctgcgcgcccagctcgaccacgcggccgggcggaatgtggaagaagtcggtcggattggcggcgttgcgcatcaggaagatgaacagccggtcctgccacagcggcatgccctggcgcgccgaggggatcagcgaacggcggcccagaaagaagctggtcgacatgatgtcgaacttcagaccctgcttgcggcacaggccgagtgcgcggggcacattgggcgtctccatgaatccgtaggtgacggtcagccgcttgaagtcgtcgttgatcggctccatccgcacccggtcgctttccttgacgcgcgggcgctcggaggtgcgaaccgtcagcacgatgttcttctcgtgcagcaccttgttgtgcttgaggttgtgcatcagggcgaccggggcgacgtccgggtcggaggtcaggaagatggcggtgcccggcgcgcgatgcggcgggcgcgcctgcaacatttcgatcaggtcactcagcggcaggctgtccttgcgggtcttggccgtcagaatttgggtgccgcgcacccaggtccacatgatcagcaccagcaccgcgcccagcaccagcggcatccaggcgccgtccgggattttgagcaggtttgaagtcaggaacaccgcgtcgatgaaggcgaatgggatcagcgtccccgccaccgcccacatcggccacttccagcccttggtgatgacgaaataggccatcagggtgttcaccagcatggtgccggtcaccgccacgccgtaggcggcggtcaggttgtgcgagctctggaacaccaccagcagcaccagcaccccgatcatcaggaagctgttgaccgccggcacgaagatctggccggcctgggtctcggaggtgttgcggatgtcgatgcggggcagcaggcccagctgcaccgcctgttgcgtcaccgaaaaggcgccggtgatcacggcctgcgaggcgatcacggtggcggcggtcgccagcgccagcatgggccagtagatggcctgcggcaccatgctccagaacgggttctcggacgctcccggattgtccaggatcatggcgccctggcccaggtagttcagcgtcaggcagggcagcacgaaatacagccagccggcgcggatcggcgcctttccgaaatggcccatgtcggcatagagcgcctccgcccccgtcaccgccaggaacacgctgcccaggatgatgaagcccagaaagccgtcggcgatcagcagctggatcccatagtgcggcgacagggcgcgcaggatcgagatgtcgtcgaagatgtggatcaggcccaacacgcccaggctcaggaaccacacggcggtgatgggcccgaacagcttggccaggccggcggtgccgcgcgactgcaccatgaacagggcgatcaggatgccggccgcgatcggcacgatgaaggggtccatcgccgtgccgaccccgggcgcgtcctgtacgccctcgatggccgaaagcaccgaaatggccggggtgatgatgccgtcgccgtagaagagggccgcaccgcacacgcccagcatgaatatccaggcgctgcgccggccgacggcgtgctgggccaaggccatcagcgacagggtcccgccctcgcccttgttgtccgcgcgcatgagaaagaagacgtatttgaacgtcaccaccaccatcagcgcccagaacgccagcgacaccacgcccacgaccgccaggtcgccgccgacgccgccccgcgcgtgatcaatggcctctcgcagagcgtagagcggactggtgccgatatcgccgaacacgaccccgatggcgcccagcgtcagcccccagaagccgccgtgcgccacggcctggccgcccggaacgtgcgcctcgggcgtgacggtcgctgtcgggccggaagcgggtgggggcgtgacggcggcgccgtccgacccgaggggagcatcccctgtcatgcctgatctccgggcgtcgcctttggagcgggccttcaaagcggcgagccctttaggcgcattcccgccgtcgttcaatcgcgcgcacgccattgggttgcgggcgtctggcgccggccgtttgtgattcgagccgcgcgcgcctattttgattgccgatcatgtccgacagccagcgctttcccgtcgccgcccacgccctggcctatatggcccacaagggggcgttcggccctgcgcaggcggcgcccagcggtctgctggccgcctccatcccgaccaatccggtggtggtccgccggattacggccctgctggccaaggccgggctgatcgccacgcgtcccggcgcgaccggcggctcctggctgctgcgccggccggaggacatccggctggacgaggtgctgaaggcggtcaacggctgcgcgcacctgggctccaccccggccggagccaagggttgcccggtgggcgagcacatcccgcgccaggtggccaaggcgctgacggcggccgacgaagcggccagcgcggccctgtccaagatcaccatcgccgacctgctggccaacgatcccgcttcgctgcggggctttgcgccgcattcgtcctgtccgctggcggcgggagagccggtcgatgcggacgccgtcgcggcctgatccgacgtcgcgcacggttctgatcaccggcgcatcggccgggatcggccgggcgctggccagggtctatgcggccgagggctgggacctgatcctgacggcgcgccggatcgagccgctggaggcgctggcccaggagctgcgccggatcgggcggaccgttcatgtgacgactgaagacctcgccgatccggccgcgcccgagcggctgtggacggcgatgcaggcgcaaggacttgccatcgacggcctggtcaacaatgccggcttcagccgggtcacgggtttcctcaagaccgatctgcaggcgcaccgcgacatgctgcgggtcatgctgaccgcgccggtcgagctgtcgcggctgttcctgccgggcatggtcgagcgcggcttcggccgggttctgaacgtcgcctccctggccgggcagatgccggcgacgggtggagacaccctgtatgggccgatcaagagctttctgatcaaggcctcgcaggggctgcatctggagacgcagggcacgggcgtgcatgtcacggtgctgaaccccggctacaccctgaccgagttccacgacgtcaacggctcgcgcgatcaggtgtcgcgcgcctatccccgctggatgtggatggacgcagagcgggtggcgcggatcggctatcaggcctgcgaggcggaccggcccagcgtcacgcccggcgtaatgaacaacgtcatggccgggctggcgcgctttctgcccgaccggatggcgctgaggatgacggccaatcacgcgcgtcggctggagcgcctctgacggttcaatggccgccggtcggatagggcgcggtgaccgagcccgagatcatgccgggaatggcctccgacagtcccagcagcaggaactggatggccagggcgcacaggatcaggcccagcacccgcaccacgatggccatgccgacgtcgcccagcacgcggctgatcggtccggtggcggcgaagcagatgaagatggcgatggcggcggcgacgatcgcgaccaccccggccgcctgaccggccgggccgatgcgcgcggcctcgccggcctggatgatgatggtcgagatggcgcccggcccgatcagcagcggcatggcgaagggcaccaccaggcgctggaaccgccgacgggcgtagccgcgcacgtccttggcgtcggccacggcgtcggcgtccttgaacatggtcaggaagtcgccgcgcgtcatgtccagccccagcagcagcagcagaatgccgcccgcgatgcggaacgccgccagcgagatgccgaagaactgcagcagcgccaggccggtgaagaagaagaaccccaggaagcccacgatgaacaggcacatcagggccgagacggaggtgcgctgtctcagattggcgccggcggtggcggcggcgaagatcggcacgttgccgatggggtccagcagggcgaacagggccacgaacaggttgacacccagatcgaccgcgtccatcgcctgccctcgccctgacaccccacacgccggacaatccgacgcaggccaagcgtcggcatagccggtccgcgcgagcccgtcgatgaccccagcccccgatccccgcctgatctgcgccctggatacgcccactaccgacgaggcgcgggccctggtcgaccggctgggcgacgctgtcggcttctacaagattgggctgcagctgttcgcggcgggcggcatggagttggcccgcgacctcaaggccgaggggcggcgggtcttcctggactggaagctgcacgacatcggcgcgacggtggagaaggcggcggcgaacctggcggggtcgggctgcgacctgctgacggtgcacgcccggccgcaggtgatggcggcggcggcgcgcggggtgaagggctcgggtctcaaggtgctgggcgtcaccgtcctgaccagcctgacggcagatgacgtgcgcgccgacgatcacagcctgtcgccggccgatctggtcgcgctccgggtgcgccaggcgctggacgccgggatcgacggggtggtctcaagcccgcaggaggcggcgcgggcgcgcgagatcgcgcgggcggcgggtcggaacgacttcctcatcgtgacgcccggcgtgcggccggacggcgcatccctcgacgaccaagcgcgggcggcgacgccctcggcggcgctggccgccggggcgagccacctggtgatcggccggccgatcacggcggcggccgatccacaagcggcggcccgagcgatcgccgagagcatcgcccagctgtagcgtcagccccgctcgcccggctcctgccgatagttgtgcggcggagggggaggcggcggcggcggcggaggcggcgcggcctcttccagtccgtagtactggttcggcgtgggcggcggcgcgtcataggggaagggctcgggcgcgggcgcatagaccggcggcggcgcgatcacctgcggcggcggcgcatagacctgggccggggcgacgtgaacctcggcgggcgcgacatgcacctcggccggggcgacgttgacgcgcgacggctccacgtagacgggggtcggctccacatagacctgcgacggcgcgacgttcacgtccggcggcgtcacatagacgggcgaaggccgcacatgaaccggtggggcctgcacgtgcacgggcggcgactgcacatagaccggcggagcgtccacatagaccggcggctgctggatgtagacgggcggcgcgggatggtggccgccgcgctgttcgtagcgttcctcgtagcggtagccgccgccccgcgcgggatagcagcggcagtcctcgcggtagccgccgcgatggccggcggagtagccatagggacgccagccgatgtagtcccggccgaaaccgtgcaccggatagccgacaggcgcgctgaccggcggacgaccatgcagaggcagcgccggcgacaccacatagccggcgtagccgccgcccgcatagccgccctcgacgtagcctgcgctgttgtagaaggtcccgccgccgaccgcgccggagccgtagccatacccgtagccgtaggcgctggacgaggcgctggaatagctgctcgaacgcgctatgctgtaggacgaggcgcgggcgcgggcgtcgatgttcacattgacgttgttgtggccgctccagccccctccgttgcagcgcgagccgcagcctcctccgccatgacctccgccatgggcgaagtcgcctgcgacggcgggcgccgcgcccagcgtcagggccgccgcggcggcgagcagaaccgaatgtgtcgtcacgggacagcctcctctaagtcgaaggagccatggcaagcccggcgccagatgcttgacgacaggttaacgcggccgacggcgatttgcatgggcgtctggcccgcgtctcctcacgcctcggtgtcgtcgacgcggccgggctgcggacgacgctcgttcgagccggagtactccgcgccgagataggcggatcgcgccgcgtccagcacgggcggcccgccgcgcaggccgcgcttctgcccagcctgccccagttgctgagccgcaaagacggcggcggcgtccacgccgctgggcgagggcgggacgggggcttgcgcccgtccgtcagacaagacgtcatctgcgtccggcgtggacgagggcgttacggcagagcgggacgcatcaggcgcgcggcgctgtccgtctcggcgctcgaccttgcgtcggtcgaccgacgcaagcgggcccacaggatcgacgggtcgggtcatcgcggcctcgcttcgggcgccgccagacgatccagtcgggcgcgcatttcgtccatctgccgtcggatctcggcgagggacccctgcaccccgtccgggtccggcgtcgtcggtcgtgagtggaaggcgccgagcgacgcttccagatcatccggggccgcggcgccccggctgtggagttcgatcagccggcgcagaaaggcggcgggcaggacggcttcgccccggttttcctgctcgtacagaacatgcatcagcacctgtcgggtcaggtcgtcgccggtgcgggcgtcctcgaccacgaagcggatttccgcgcacaccattcgcgccagatcgtccagcgtcacataggcgctgtttcgcgtgtcgtagagacggcgattcgcatatttgcggatcaccacgacatcgatgccgtcggtgcgttcgcccgggttcgtcttcctcgccacgcttgttctcgcgcttgctgcgcggccactatcccgcaagccggcgggaagcgccagtgaggtcggggtggtgggaggtcaggtcgttgcggtcaggccagggccgccggcgccagcaccacgcccaccagcaccgccgcccagtggacgcccgcgcccgcgaccacgaagccgtgccagatcgcgcggcggtacttcaccttggggctgatgaagacaaagacgccggcggtgtagatcagcccgcccagcaccagaaggcccagcgccaccggatgcaccgtctccagcatcggcttcagcgccagcaccgccagccagccgaacaacacatagaccccgctccagaaggcgtcggagatgcgcggcgccaaaagcttggttccgacgcctgcgaacgccagggtccacaccagcagggtgaagccgacggcccaggccccttcgaaccgttgggtggtgaaaggggtgtagctgccagcgatcatcagaaagatcgccgcctcgtccatgcgacgcaggaccggccgcgccgcgcacggcctggccaggttgtagatcgtggaggcgctcagcatcgccacaaggcagacggcgtagatggcggtggcgatggccgggccgacgccgacataatgcatcgccaggaccgccaggatcacgccgcccagagccgcgaagcccaggccgacggcgtgcacccacaggtcggccagacgctcggatcgggtgctgtaatgctcgatcatgtcgagctcgtccggcgtgcagacgtgaaccaccagctttttcagcgcgcgcttcatgctggataaatcgagagcgggccgtgtttgttcctgctccgctcgcgtgccgctcagccccaggggccgcgcgtcgagggcgtggccggaacgccggtggtgaccgatgtgcgacgcggcgtcggctgatgggtcgctggccggacgcgcggcgtcatgcgcgccgcctgttctgtcagggctcgaacgcggttgaccgtggcggggtgggtcgagaacagattgtccgcgccgcgccccgccaggggattgatgatgaacaactggccggacgccggattgcgctcggctgtgggattgtggatccgccgcgcccagccgtcgattttctgcagcgccgaggcgagcgcctggggatccccggcgatctcggccccgatccggtcggcctcgtattcgcgcgcgcggctgatcgccagctgcaccagaccggccgccatgggcgccaggatcatcagcgccagggtcccgatcaggccgcccggccgctcgcgatcctcaccgccgccaaagaagagggcgaagttggccagggcggcgatggcgcccgccacagtcgcagtcaccgtcatgatcagggtgtcgcggttcttcacatgcgccagctcgtgcgccatgacgccgcgcacctcgtcccgggtcagcatgtccagcaggcccgtggtcgcgcacaccacggcgttggccgggttgcgaccggtggcgaaggcgttgggctggtcgctggggatgatggcgacgcccggctgcggcagcccggctcgatcagccatctcgcggatgtcggacacatagttgcgcaccacggcattggggtgcgcctcgtccaccggctgggcgcgatacatcttcagcaccagcttgtcggcgttccagtagctgaacaggttcatgccgcccgccagcagcagggcgacggccatgccgccggcgccgccgatgagatagccgagacccgcgaacagcgccgtcagcacgcccagaagaacaaaggtcctggcgtggttcatcatcgtcggtcctcctcttccttatcgggcgtcatggcggcacgagtcccgccccctatctgagaggatcaacgcctgtcctcaagggagccgccctgtgaccgaacatcccaccccggccgccgatccggcagccacggcggaccgtctgaacgccgacgtgccgcacgcgacggccgaacgaccgctcagcgatgcggcccgacgagccctgctcgaggcggccgcgcgtcgagagccgttggagccggcctccggggcgggcgagcacggcgggccgtcagggccggagccgacccgctatggcgactgggagaagaaggggctggcgatcgacttctgatccgcctcagctgcgaaaatccatgtcccggcgcgaggcgacgatggtgacgatgaagccggccagcacgtccagcagcaccatgatcaggatcaggaaaaaggtcgaggtcgcaaacccccgcagcagcaggaattcgatcagacagaccacgaacaggatcatcgacagggcgtgattgacgatggccgcgcggtggctggccgttgatttcaaaagctcgaagaacaggatcaccaaggcgacgaacaggatcaggtcgccgacgcccacgctccattgcgcgccggacgccatggtcaccgtgaacagcggatcgctcaggatcgcatcggcctgcgccatgccgacatctgagccgttgaacagcaccacgatgttgtagagcgccaccgggatcagcagcagcggcagggcggccaacatcgaagggtcctcatcaaggcgcgatcgccgtgcataaaccgcttcgaggctgttcaacaacggcgcgccgggtcaggcgcggggaaaccggcccgcccgactgagggcggatggcgccgggcggccgatcctctcgccgatccagcgggcggcctcgatcagggcgtcgaggtcgtagcctgtgctgaaacccgcccgctccagcatgtagaccaggtcctcggtggcgatgttgccggtggcgccgggcgcgaacgggcagccgccgatgccgccgcagctggcgtccaggatgtccacgccggcctccacccccgcatgggcgttggccaggccggtgttgcgcgtatcgtgaaagtgcaggcgcaaccgggcgtcgggcgctgcgggccgcgcgcgctccaccacccgcgtcaccgaccatggatcgccggccccgatggtgtcggccaaggcgatctcggccacgcccatttcgccgatccggcccacgacgtcgacgacgcgattgatcgccacctcgccttcgaacgggcaaccccagacgcaggacagggtgacactgaggcttggcgatccctcgggcgcgcctctgcgtcgggccaggattgtctccagcatcgcgatctggtcttccaccgccatgccctggttgcggaggccgaagccgtccgtcgccgccatggcgaggttgatctcgttcacgccgctcgccagcgctcggtcgtagccgcgggcgttgagggcgaggccgatgcggctgcgtccctcctggcgcggcaggtcatccatgacggcctcggcgcccgccatctgcggcacgatccttggattgacaaaggaggccgcttcaatccggcgggcgcccgccgcctccagcctccgcacgaagtcggcccgttccgacggcgtcaagacggcggtttcgttctgcagcccgtcgcgcggcgcgacctcgacaatctggatcggacggttcaagacgatctcccggcgcgtgaatcaggacctggcggcctccacacgctgtagcacaggcgccacggtgttgcgcgacggcgacgtcgcgtccgcgcagcctcgactctgggaagctccgctgttatgcacggccgaggcgaaacgatcgccgaagactttatcagaaagcgagggacctcccctatgcgtatgaagacactcgttctggcctccagcgcagcagcggccctggccctgtccgcgggcgcggcctcggcggagccggacggctggtacggcgcgattgacgcgggttatcagtggatcgagccgatcaacatcgagtcgcaagcgaacggcgccaacttcaacatcgacgtgaacgacggctgggccgcgtttgcgcgcctcggctaccggttcaacccgaactggcgcgtcgagctcgaaggcggctaccgctcgggcgacatcggcacggttcgcgccgtgtcgggcacgcagggcgtgtgcaacttcgctccggcgaccggcccctgctactcgccggaaggcgacctcgagtccgccaccctgatggccaacgtcatctatgacttcggcttcgagtactggggtctgcgtccgttcgtgggtctgggcgccggcgccaactacgtcaacaccgacttcgcgggccgcatgcgcgccacgccggcggtcagcttcgtggccgacgacagctcgaccaagttcgccgcccaggcgatcgcgggcgtggccttcgccgtcggcgagcgcgccaacatcgacctgacctaccgctacctgaccagcgacctggagttcgacacggtcaccgccggaacgggcgctgcggcgttcggcaccttcgacggcgactatgacgagagccacacggtgacgctgggcctgcgctgcgtctcttgtacacctctgacg

SEQ ID NO: 3 - DNA, 818508 bp, brevundimonas massiliensis
  source 1..818508: mol_type = genomic DNA
ttggcgacgcggtcaacggcctcgcgcttgaaagaatccggaaagttccggcgttgaacactcatcagacactcctctccagctccgaaaagctagcatgggtgtccaccaaaccgagggaggatcaggtttggccaatgtcagatgcttgcactccccgctctccctccaccctcgcgcagcgcattcgaacgcgacaggtgaagctcgccatggcccacacctgggcaatgactgagcgccggcttacgtcccgcaaggggcatggctaaggtcggcgttcctttcactatccggtgcgatcccgtggattccagtttcgtagacctcgacatcctgctgaccaaggtccgcaacccgcaatcccgcacctacttcctggacgccgtgcgggcctacaaggccggggcgctgcgcgcctcgctcacggccgcctgggtcgctatcgcctatgatctgatcgccaaatatcgcgagctcagcgccatgggcgatgccgcggcgacggccttcctacagtcgtgggacaatgcgacggccatccgcgacatccggcaactgcttcagctagagggccgcattctcgaagacgccgcagacaacacccaggcgatcagccagatcgcgggccggcagctcgaacgcctgcgcgaggatcgtcacctctgcgcccatccggccttctccgccgaagccctcctattcgaaccgacccccgaactggttcggatgcatctcgtcaacgccgtcgacctggttctcggtcaggaagccctccagggccgcgccatcttcgaggtcttcgacgccgacgtccaatcgtccggcttcccgaccgatcccgcgcggatcctcgactatgtcgagcagcgctacctcgcgcgggtccggccgcaggcgatccgcaacttcggcaccgtgctggcgaagtctctgctgaagggcgttcctgcccatctcgacgtcgtccgccccaaggtcgaagccgcgctggtcgcggttcgcgaccgggcggctgcagcctggcctgacgtggtggccagcatcgtgcgtctgctcgacgcgctcgacccggccgaccgcgcgcgcgccatcgccttcgtcgcagccttccccgacttctggcacctcgtgcaggagccgacccggacctccctgcaggagacggtcaacaacgccgacggcgccactctgacggactacctcctcctaaagggcgtcgccttcgcgccattcagggcgccgatcctcgcccttatcgccgggttagaccgcgagcctctggctcaggcgatcgccgccgcgcccctgcgggagctttggccccatgcggttgagctctacgcccagtccggaagcttccgcggctccgaagccaatttcgacgcgtacatcacgccctacacgggccggctcgacacggcggccctcgatcaactgctcgacgccgtcgccgccaccggccagaactacgcggcgtccggcaccagcgcgctgctcctgagcctggttcggaacgcgggcggcggacgcctgccctcgccggacgcccgcaatcgcttctatcagatgctcctacggtcacatcggcgcgaggctttcggcgaagtggtcgccctgttcgaagccgacggctggacgccgcctccgcgggaacgcgaggacgaagacgactgacgtcttggcgacgccggggactgagcagggaccagcgcgaatgcggcctacgcggcgactttcggtttcgacatgaaggcgaacttgaccttgccgcacatgcactggaggtactcacgtcggccacgtcccggacttacctcgatcaggacgccgcactggtcacagttgaagagcacgaacagcgcctgaaacgcgtcgatgaccgcgatcatctccgccttctgcaggtcagcccatgcattgtagtggacggccggattgatctgccattgttcgaccttggcgtcggtcacggcctgggcgaaggccgtttcgctcgccttcaccgccgccaaccgctccgtatccgaccagctttccgccgccagacgcgcgtctttgagaagagacttcatctgtccgatggccggatccagcaggtcgcccaggtcatgatgtccatcgacgctgaactcgaccttggcgcgcagcgcctggcaggcttccgcggataggtgctccaaagatcgacgcagagcgccagccgcgcctgcgacatcgtcatttcgcgccttctcgcgcatttcgtcccacacgtcgcccttgctccaggtcgtgggaccttcctccaccgtccatttgcggaactggaccgtgtcctttggggccacgaggcccgtggtgctcatgaacttcagccaggcgcggtcgtgggtggtgagaacgaactgcgtgtccgggaactccgccttcagcagcttcgacacctcgcgccgatgaccggcgtccactgacatcagcacgtcgtcaaggaccgcgaaggtgaagcccgttcccaggagataccgcatcagggcgaggtagagacacaggcccatgctgtcctggtgtccctcgctatggtaggcgcccggcggaaagaagccccgtccgtagaagtccaccccgaagccgagctttcccagggagggtttcagtttggcctcgaagttcccctcgtcatcggcgttgatgcggcggtagagctcggcgaaatggccttgaacatcttcgtagaccttctccagcgccgcggtggagggcgcagagtacaggtcgaagaccttcttcgccctgtcggcgcgggcgttcgccgtccgggcggccgcgctggctgtccgcaacgcctcaaggcgcaactgacccgtgatgaggtaatcgcgcgcggcgtcctggtccgaaggctccggcagtccgccgatggctcccgaaagccgggtcaacacatcgaccaaacctgcggagggcgtcagctcgtcaagccgggccagcgtcttgtcgagcggcagaagcgccgcaagcgcagcgccggcatcgaccagagccttgccatggtcggcgatctgatcgagttcatgggcttcgagaagcgacttgcctgtgaggtagaccggccgggtcaaagccgcttccgcttcgagcgcgtctcgaacccccatcagcttgtcttcggccgccgcgcgcaggaccttgaccgcctccagtttcgcccgcttggcctgaatgatcgcggtgagctcgtccagggtcttgggcgtgtcgcagacgggacagacttcaccctcatagagatcgagagccgtcttgagaaaatcgtcgcgcacgacgtccttcagcaaagattcgtcagcgattagccgctcgaccgccgtcctcgccgccgcgacctgggcgcggacgtcttcccccgatcgccgatcgactgagtcccgcagcgcggcgagatcagcggcggcgaccgccttgttgaccgcggcgaccgggccgcccgcttgtgagctcaacccatcgcgtagcgacccctcgggccccagcgtcgaaagaccctccagtccaagcaccctccggcgccggttggcggcttcgaggatttccggtgcggtcgcgtcagcgatatccatggcgcgtacaaactcagccttcgccgcatcacgggtcgcggccgcggccttcgcagcggcctgactggcgttagagatgcgctgcagccgcgttctcaggacttcgaggtcgtccagtttgaggagagcctggacgtccttggcgcgttgacccggctcggtcaggacaaagcgaatgatctcccggcgagacagggcgatctccggatgggcctccagctggcggaacaccgcctgcacctccgggctgtcaggatgggcctgaagcacggcgggcgccttcaccgatcgccgaacctggacggatcgcctgagcgacgggatccacactgtcgcttcgacgaacgccttctccggttccgtcttcctatcgacgtgagggccatgatccttgatggacaggtcgccgcggcctttcccggtcaggcgcgagattgtgcccgtcagaacgaactccaaggcgtccacgacgccgctcttgccggtgccgttggagccgcagacggcgaagttccgccgctgaagattaagcgacaggctgcggatgccgcggaactccgcgatcgtgaggctctcgacctggatcatgccggatcgcctccgaagagcgcctgactgatcgcggcctcgctgagatccttcttcgtgatgagcgtatcgaccaaccgctgtgcggtgtcagccagcccctcttcggattcaacagcggtcgtgaacgccgtcaatacacggtcgagcacggacaggtccgtggccggttcgttcgattgagcgtcttggtctgtcatggtcgcctccccggtcaggagcctagagcaactgcgcggcacaaccaacacgattgaccgagacgactttcccgcttgctggcgggtaagccaagcccgccggcccaatccgtgataaagccgatcagcgccctgtcgcgctcgccatccgcgcgcctgccaggctatcggactcgcgactatttcatttcgacgctggagcgtcggcgccgctcgagcagacggctagagccgcaggtgaggacagtcgatgacgctccaacatcccgaatggcatccacagcgccatcccgagttcgacgaccgaatggccgtcgaaagcgcgacgcttctccaaaagctgcgaacggaccccgtctatcggagggcctgcctggacgatccgcgcggtcttcatcgagacctctactccgccttcgtcccgccagcccatccggaatacgccggcggctatcgcggcgtccccggcacatccctcgcgctgcgtgtcatgggcggtccgagcgtcatcgtcgagggtcagacgttcaccttcatggacccgccggacgtcccttcggccatgcaaagcctcgtcgggaccgtgcgcttgcggatcgacaccctcgtcgagccgtgggaccagttggtgacgctctcttatctcttcagccagttcggcttcatccatcccttcctggatggaaacgggcatgtgcaacggtcgctcttcgcggccgcggcggtggagatgaacctgccgctctccaaccggttcgcgatccatccacgaccgtacgacttcctgctggcccacacgcttgaaaactacagtcgccgccccgcccagcgaccgcagtggttgagcgccgtggcggagtatctggttcagtggcttgagggaccgttcgacgccccgggcatgggcatggcgcctcttgaccgggagggtggctaacggcggggatgggcgcgccagcccccgcgcggagaccgggcccgacgttcgatcctctggccgtgcgataggccgggatatccagaagatgggcgtcgccgtcggttcgagcgcccgcgacgatcaccacgccgtcgccgaactcgatcccgcagttcgatccctgcggcggatcgtcaatccccgagacacccgcgcccgggtagggatggctcctggagaaacgaaagcgcatgcgccgtctgcgcccgccgcgtcgtgcggttcccgagccctgaacgtcgggatatggacgcgcgctggcggcctgagcccgacgattgaccgatcaggcatccgatcggccaacagccgagccgcacccggttgcacagggttcggtgatgcgcccttcaagccaccgggcggtcagaactcacgcccggctgcgccggtggtcgccgcggcggattgagccaggcttgcaccgggccgtcgaaaccgtatcggaacaccgccgccgccgcaaaggcggaggccagacccagcccccagacgccccagcgaacggtcgccggccaggccgcctggccaagggcgtcgaacgcgccaaaccagacgatccgggtcacttcgtttgtcaggaacatagcgaaggacataagaccaagctgctcgatcagccgtgacggacgcgccacgggcagggctccggcggcccagatcatgacggtgagcaggagaagcgaaatcagggcgagatcggacacggcctgggccgcgatcagacccgcgaaggcggcgagccccatccatgccgcacggaccggcgggacccagacgcgcgcgcctaggatcgcagccgcgacgcccagcaggaacaggggcagcgcccggatgaatccgtgacggagcggaagccggtagagggggtcgcccaaccatgcccggctcgcaccatccgccaccagaagcagcattacgacgcctgcaaccacgagccaagggcgcaggcgccagagcgccctgcagatccagggcagggccaggtagcagcccagcagcgccgatagcgtccaggtcggggcgttccagccctgcccgcccgggacgccgtaggcctggacgaggaagacctgggccggaagctcgggccaggcgaaccattgcgggttgctcggacggattccgacggcggcggcggtcgcgacgagcagcgcgagcgcggcgatgacgacgagatgagagggcgcgacgcgaagaagccgttggcgcacatacagggagagcgagagggtgcgattggcgaagccctccccgtagatgcgcgcgaggacgtaccccgagtcgatgatgaagaagttcgtcaacaggtagccccggtcgaagacgggatgaacctcgccgagcgcgaccggggcggcctcgcggaaatggtaaaggacgatcagggcggccgccacgaaacgcagaatgtcgagccatcccccgcgcgtgatccggacgggaacccgcgcagtggcctctagggccgtcatcggccgggcctgacggaagcggcggcgtctgggacggcgtgcctgtggggcggcgcgagattgatctgatcgcgtccgacgtacaaggcggcggtcccgagaacgcacaccagcgccaggatcgcggccaacagccggccggccgggtccttggccgccatccggaaggtcaaggcggtcaaaagaagcatcagcccgccgaaggcgccgtacaggggaaaccggtaagtcgtcgccatgggcgccgccacgcagaagacgacgaaggcggccaccaggccggccccgaccgcgatcagggtgtctcggaccggccgaaacggcgccggcggacgggggcgccgggacctaccgcgggcgcggtatttgccgggacgccagcggggcgcccggctgtggatcgtggaccgctttgagcccatcggcctagttcgtccgcatgcgggtggccagccacacccgcatgcggacgatctccgcctcctgggtccggatgacctcttgggcgaggccgcgtacctccggatcagagccgtgctcgagcgcgatcctggccatggcgaccgcgccctcgtggtgggcgatcatgccccgcatgaagtcgacgtcggcgtcgccgctgtactcgatctccatggccgaatgcatccgggcgttcgcctccttgtaggaccgcgtcgccgggctgtcggccgccgcgtcgctgtggccggcgtgttgatcgatcggccgggcatcgaccgccggggtcgcggacggtctcgcggcctggcgggacaatacgccgaagccgaacaccgagacgagaaggaagagcgcgatcacgctgacccatccgatgcgtttcataggggttctcctgtgcttggggtttgcgagttcacgcggcctctcgcgggccgcgccaggcgagcagacgcagcgcgttgaagacgaccagcagcgtcgaaccctcgtgcagagccaccgccggaccgatgccaagcccgaagatcgtcgccggaacgaggaaggccaccacgccgaggctgacgaacaggttctgacggatgatgcggcgggtctgccggctgaggccgacggtgaacggcagctttgacaggtcgtcggccatcagggcgacgtcggccgtctccagggcgacgtccgatccggccgcccccatggcgacgcccacggtcgccgtcgccatcgccggggcgtcgttgaccccgtctccgaccatggcgaccttggcctccgcccgcagtttcttgatggcctcgaccttgtcctccggcatcaggtcgccccaggcctcggtcaggccgacctgcccggcgaccgcctgagcggctttctgatgatcgcccgagatcatgatcatccggcggatgccgagcgcgcgcagcgccgtcagtgtctcgcgcgccttcgcccggggcgtgtccagaagtccgatgacgccgaggtccttgttcccctgccgcaccaccataagggtgcggccctcgttgcgcagggcggcgaccgcgatctccgtatcggggcccagcggcgcgatgccgtcggcgccgaacatctccggcttgccgatccagatctccttcccctccaaccgggcggtgacccccttccccgtcaggctgcgcagatccgtcgcggttcgcgcgggcgcggtcgccaggcgctggcttccatcccggacgatcgcctccgcgagcgggtggtcgctgagccgttcgacggcgacggcgatctccagcagttcgtcttcggtcgtctggccgaagggcacgacatcggtgatccgcggcttgccttcggtgagggttccggtcttgtcgaaggcgatggcatccagcgcgccgaggttctccagcggcgccccacccttcaccaggaccccggcccgggccgcccgggccacgccggacagcaccgcgctgggcgtggcgatggccagggcgcaggggctcgccgccaccagcaccgccatcgcgcggtagaagctgtcgcggaagggctcgtcgacgaccacccaggcgaacaggagaacgaaggccagaccgaggaccagggggacgaagacccgttcgaagcggtcggtaaagcgctgcgtcggcgatttctgggtctcggcctcgctgaccatccggacgaccttggccagggtcgtgtcgttggagcgccgcgtcgtctcgatctcgatcgcgccgccgccgttgatcgtgccagcgaagaccaccgacgacgccgcgaccgatgcgggtctggcccgcgcttcctcggcgtccgcgaccggctgcttgtcgaccgggatgctctctccggtgaccggcgcctggttgacgctggacgtgcccttgatcacgaagccgtcggccggcaaccgctcgttcggccggacgacgaccaggtcgccgatctccagctgctccacgggcagttcgacgacctgatcgccgcgccgcacatgggcggtgcgcggcgccagggccgccagcgcctcgatcgccttcttggcgcggcccatggcgtagtgctcgagcgcgtgccccaggctgaacaggaacagcagcagcgccccctccgcccaggcgcccagcgcggccgcgcccgcggccgcgaccagcatcagggtgtcgatctcgaaccgcttgcgccgcaggtttccgatagcttcgccgaccgtgaaccagccgcccaaggcgtaggcgatcaggaagagcgcgaacggcagcgccgccgggagggccggaacgaatttctcgatcagccagccgaccgtcagggcgacgccgctccccacggcgaagatcagctccgtgttcggccccagcaccccgccatggctatggtcatgaccgtcgccttcggaatggccgtggtcgtgtccatcgccctcggcgtgtccgtgatcgtggccgtcgtccggaccatgacccgacgccgcgttccgggccgcttgcggcgccggacccacagccgccgatgggccggcgacgtccgacgtctccgtcaatttgagaccaagagacgccaggcgctcgaccaatctctcgcggctcgtggcctgacggtcgaactccagacgcaaggcgcccgccggatccagcgcggcttcgatgacgccggcttcctcgcccagctcggccgcgagcgtgcgggcgtggcgcgcatgccggacgccgtgcacccgtcccgtcaggtggccgaaccgctcgctgacctcggcgccggcctgccgcgcccgccgtctgacctgggccagcgacagcaggtccggatcatagtggatgcagagctccgcgccgtccgcgccctcgaccagatgcgcctcggacacgcccgcctcggcccgcatgagggcgatcagacgtcccacgcagccgtcctcggcgtcaggcgcgtggggaagaaggacgggaatattgagccggagggtcttgggcatggtcgggcctcaggggaagtcgcgggtagggttggagcgttcggggatgagaagaccggcgccgtgcatggctgcgcccgcagcgaaggcggcgagggccaggatcgcgctgagcagggtgacgagacgtttgcggttcacctcgcacctcctcagggcaatgcgacgacggcgtcgagccagccgatcgcctggaggcgctccagcccctcgaacacgggcagcgccaggagaaagaccaagccgtcgcggacggtcttgagaaagaacgacgggcggaccgacagctccgcctcatctcgccagaggcgaggatcgggcaggaagcgcggggtccgctcgaaatacgtccggtaggtctcgccgaaggcggtcccccggtaactctcctcgcgtctcgcgacgatcaggaagaccccccagcaggccagggcgaacgcgaggccgacgctgaggctgccggtctgggcgccgaccccgaaggccccgatgacgctgaagacgtagagcggattgcggcacagcgaatagggtccgctggtgacgatctcctgcttcttgcgcccgccgatatagagggagcaccaggcgcgtccgagcacgcagaccatgatcgccaccatgccaagatgctcgaccgggtgttcgagcccgggcagcgctcgcaccagagcggtccaggccagcagggcgaacaggcccgcgccgatgaagagtttccgccaacgctggaccgaggcgatgtcgatcaggggcgggctcatgcgtccggctccggtccgtcgcgtcgcgcggcccgggcgtcgccgaggatgtcgagcccccccttggccgcgatggccgcgaccaggacgccgaccaccaggtcgggccaggcctggtccagccacatcaccagaccgccggcgacgaggataccgccgttggacgcgaaatcgttgaggctgaaggtctcggcggccttcatgttgacgtcgctgctctgctgccggcggatgagcatgaggcagatcaggttgatgaccgcggcgatgacggcgaggaccatcatggtcgggccgaccggttccgtcccggtcagcgtcctgcgcagggcgtcgagcaggacgaggaccgcgaagatcagcagcatcacgccggagacctgcgccgcgcgggtcttccagatcagggcccggccgaccgcgaggaagctgatcagatagacggccgcgtcggatccgttgtccacggcgttggccagcagggcgctggagtcggcggcgaggccgccgactcccaggcccacgaacagcagagcgtttagggccagaaccgccagcaggatacggcgctggacctgctccgtgtcgtgggccccgctcattcctccagtccttccgcggcgcggtgcttcacagccttggccgcgaaggtgggcaggaccaggagggtgagggccgtggcggtcagaagaccgccgatgaccacggtcgccagaggcttctgcacctcagcgcccgccccgtgcgcgatcgccatcggaatgaagccgacgatcgccaccagcgctgtggtcaggaccgcgcgaagacggcttgaagccccctcaatggcggcgatcatgggttccgccccggcctggagccgttcgcggatcgcctgcatcaggaccagcccgttcaacgtcgcaacgccggagacggcgatgaagccgactgctgcggacaccgagaagggcatgcccctcaacagcagggccagcgccccgccgaccagggctaggggcacgcaggcgaagaccagaccggcctccgcgaaggagcccagagccatgaacagcaggatgccgatcaggatgaagacgacggggatgaccagacccagccgctgctcggcccgcttcaggttctcgaactggccgccccaggtcagggagtagcccgccggaagttgaacctgttcctgcacgcgcgcctgggcgtccgtgacgaagccgcccagatcgcgcccgcgcacattggcctggaccaccatgcgccggctgccgtcgttgcggctgatctggttctggccttcggcgatctggatgcgggcgaccgaggacaggggcaccgtgacgccggtcgtcgtcgtgatcggaagcgcggcgagcgccgccggatcgttgcgggcctcatccgccagacggaccaccacgtcgaagcgccggtccccctcgaagatctgccccgcttcggcgccgccgatggccgcagagacggcgttggacacctcagccgccgacagcccgtagttggccgcagcgaaacgatcgacgctgaccgtcagggtcggcaggccggaggcctgttccacccgcacgtcggccgagccctgggtattgcgcaggacattggccacctggtcggccgtggcctgcagttgggtgaagtcatcgccatagaccatgaccgccagatcggttcgtacgcccgagatcagttcgttgaaccggagctcgatgggctgactgaactcgaagctgttgccgagctgggccgaggccaattcctcgaaccgcgcgatcaactcctccttctccagccgcggattcggccattccttgcggtccttcaggatgatgaccgcgtcggagatgttgggcggcatggggtctacggccgcctcggcggtgccggtccgggcgaagatggtcttcacctccggctgggccgcgatggcgcgctcgatcgccatctgcatggcgagggattgttcgagcgaggccgacggaacgcgcagcgcctgcatggcgatgtcgccttcgtccagcgtcgggatgaactcccggcccagggtggtgaaggcgacgccgcccaccgccagcgcgcccagcgccgcgatcaggacgatcttgggacggctgacggccgcccggatcgccggttcggcccagcggcggacccagcggatgatgaaggtctcgtgctcgtgcgcgtgaccgtgctcgtccacgtcgaccttcttgggctcacgcaccagcagcgccgtcatcgccggcacgaaggtgaaggagaagatgaaagccccgacgagggccagcatgacggtggcgcccatcggaatgaaggtcttgccctccaccccctcgagcatcagcaggggtgtgaagacgagcaggatgatcagttggccgaaggcggccggcttgaccatcttcatcgccgcggccccggcgacgctcaggcgctctttgcgcgtcagcgcccgaccgacctcgatccgcttctgcgatagcatcagaagcgtactttcgactacgatgaccgcgccatcgaccagaaggccgaagtccagcgcgcccaggctcattaggttaccgctgatcccgaaccggttcatgccgatgatggcgaacaggaagctgaccgggatcatcagcgcggtgatgctcgcggcgcggatgtttccaagcagcaggaacagcaccacgatcacgagcagcgcgccctcggtcaggttccgagccacggtcgcgatggtcttgttgaccagcgcgctgcggttcaggaccggctcggcgacgatgctcggcggcaggctggcgccgacttcctcaagacgttcggccgcagcttgggcgacggtgcggctgttgccgcccgccagcatcagggccgtgccgatgacggcttcgtggccgtcgcggcttgcgccgccgagacgcggcgcctgccccacctcgacggtggcgacatcggcgacgcggacgaccagaccgttacggttgacgacaggggcctgggccagatccggaatggtctgtgccagggcgtcggtgcggacggtcagggcttcacccgagcgctggacatagccggcgcccgcctgggtgttggcgttctccagcgccaggattagatcgctgagccccagaccatagctggccagcttcgccgcgtcgggacggaccgcgaactccttcacatagccgccgttgacgtccacgccggccagaccagccgccgtgcgcatgcgcggggcgatgatccagtcctgaacggtgcgcagataggtcgcccgcgcctgcggcgtagtcagcagctcgccttcgggcgtcagataggcgccgccggcctgccagccgggctggcccggtttggcgaggttctgggagttgaacggcttgtagtcgaccgtccacatcagcacctcgccgagacccgtggtgatcggagccagacccggctcgaccccttcggggaggttctccctggcttgggccatccgctcggccacctgctggcgggcgaaatagatgtctgtctgttcggtgaagatgaccgggacctggctgaagccgttgcggctcagggaccgggtgctctgcaggccggggatgccggccatggcggtttcaatgggataggtgacctgccgctccatctgctcgggcgcgagcgccggggcgatggtgttgatctggacctgccgattggtgatgtctggcacggcgtcgatgggcagcttggtcagctggaacagaccccaggccgagacgagggccgtggcgaggaccacgaaccatcggaatttgaccgaggcttcgatgatgaatttgaacatgcgatcgcccccttagtgaccgtgctcggcctcgcccttggccagttcggccttgagcaggaaggcgttggcggaagcgatgcgttcggagccggtcaggccgcgcaggatttcggtgcgcccggcggcctggcggccagcgagcacctggacagcctggaagccgccctggacctgcacgaagaccacagtgttgccgtcgacggtctggaccgcttcggacggcacggtcatgccgcccgaggtcgcctgtccggtgaccaccgagccggacacggcggacccggcgggcggcagggttccggaagacggacgggcgcggatgacggtcgctccgctctcgttcagaccggcgtccgcggccaccccggtgacgaccgcgtcgaactcgccggacggcccggtgacccgcatcgccgcgcccgggcgaacattcgccgccagggcgggaggcgcgttgaacaccatctcgacgcgggccgggttggacacttcggcgaccacgccgccctgggcgacgaagccgcccggtccgacctgcacattgctcaccacgcccgagatcgggctggtcacgctgagccgtcctgacgcattgggcgatcctgcggccgcagagcgcgcccgcgccgcgcgggtcgccgcctctgcgctgagaagctgcgcccgggaggcctcgacctcctggcgggcgaccaccccctgttcggacaggttgcgattccgctgataggcctgacgcgcggcctcggcggaggctgcagcggcatcggcgtcggcgcggaaggtggcggcttcaccgctgaccaggctgacgagcggctgaccggcgcggaccgactgaccgggcgccacaagcagccgctcgacccggccgccaaccgcagcggcgaccgcagcgcgggaatcgaccatcggctcgacccgccccgccagacgcgtttccgccccgccgccggcgcttacgccgacgacggagatgccggccgcctggatctgcgcggcggtcagttcgacgcggccctcttcggcctcgccctcctcggcatgaccggcctcgccttccgcatgcccgccttcctcttcgccatggccggcttcgccctccgcggccgccggagcaggcggcgcgtcggcgcctcgcgtggcgagatagagcccgccgccgccaaggacgacgagggcggcgacgccgccgatcaacagggtcttgttggatgtgcgcttgcgcatcactgggctccttggaagggggcgcggccgtccaggcgcgcgagatcgatttcggcgcggacgcgcgcgaggcgggcgtcgacggcggcggaccgcgcgttgacgagggcggttcgggtgacgcgcagctcgacctgggagatgcgaccggcctcgaagccgatgcgcgacagccggtaggcctcctcggccgcggtgacgccggcgtcggcggcggacacgcggctcaccgaggcggccaggcgcgccaccgcggcggcccggtcggcttgggcctcctgccgcgccgacatcaggcgggcgtcggccgccctgaactcggcctgcgccgcctcgatgtttccccggttccggtcgaacagcggcagcggcatgctgatcccgaaggtaagcgcggtggcgtcctccgcctcgaagcggcgaatgcccacgctggcgttgatgtccgggcgggcctggacacgttgcacgtcgatccggcgttcggcggccgtgcgctcggcctcggccacgcgcacggtgggcgcgtcgttgatcgcggagcccaccccggacggcgcctcgtccagcagactgacgtcgatgcgcgtcacgggcgacgggatcatcgccacggcggtgaggcgggcgtaggcggcgtcccgttcggcgacggcttcgtcgagggtcgcccgggccgacgcggcttcggcctcgccctggatgccgcgcaggagcggctcgcgcccctcctccaccagcgccagggcggcgcgggcgtcggccagggtcagggtcaggacctcatccgccagggccgcgcggcgctgcgccgcctcggcttcggaatagaccagggccaggcgaccggcggcgtcgatcaccgcaagatcgcgctgcaggccgacggcgccggcctcggcgcgcgcggcggcgatgcggctcgcgcgacgtccccacaattcgaggtccgtgctcaacgcgagggtcgtatcggcgttgtccatccccgagaaggggccggagccgtacgcgttctcgacatcgagcccgagcacggggttgggacgcacacgggcctgacgcacgcgggcttctgcggcgtcgaggttcgcgcccgcctccagggtggcgggcgtctggccgagctgcgcgagcagttgggcgtaggtcggggcggggtcagcccaggcgggactgaccagagtcgctgcgatcgcagcaaccgcgcagccgaccgcgagacgcggtcgccggcgagatgtgggagacatattccatttccagatttctgatcacgaagaggcgcccgcaagggcgcaggccttcggtcagactctggggggtcgcttcaggccgtcgggcgtgaccgaggccaggacgtcatcgtggcggccgctttgcagcagcagttcgccgaacgcgggtgcgatggcgtcgacgccgtgagtgcgcgctgtggaggtatggtggcagtgtccgtgcgcgcagatgccatggcttccggacgggtcgccgtggtcgccgtcgtcgggattgtgatcgacgaacgcgtgcgctgctgggggctccggcatgcaggtcacggcgtcgacggcgggcgcaaagaagaaggcggcgaagacaagtgtcatcaccgcgatcagcttggcccatgtcgtcatcgacgaggtcatcgcgcgttcgttacttccgttctgcggaggtggcaatctgttacaaagtccacgggcctgccaaccaccctgccagcggcgacgtgtcgcgtgcgcggagccggcgtgctgctaggatcaggtccatccgcaggagccgtcatgtcctctcttcgcctcacccgccgcgccgcgctcgtcaccggcttggcgaccgccgccctcccgccgctcgcccaggctcagacccccggtcgggtcgcgcggcagatcacggtctacaagacgccttggtgcgggtgctgcggcggttgggtcgcgcacatgcgcggcgccggctggacggcgctcgtggtcgatcttgatgacctcgccccgatccgggcccgtcacgggataccggaccgcctcgcgtcgtgccacaccggcgtggtcggccgctacgcgatcgaaggccatgtgcccgcgtcggatgtcgaacggcttgtgcgtgaagcgcctatcgcgcgcgccctgaccgcacccggcatgccggccggatcgcccggcatggaggccgccggccgagagccctatgtcactctcctgatcctcgcggatggctcgacgcgccccttcggacgacacaacggcgcttaaggcggccgcgccacccgatcccatccgaccaggcgggatcagcttcacggggcggacagggagacccggctcgagccgtcacttggaggcgctctcagggcgtcgaggacgcagcaggcttcgaccgtcgtccgcccacactggtcgagcaccgagacaagggtcttttccaaccgccgaagatccgagatcttgacccgcaccgcgtccagatgcgccgccgccacgtgatcgaccgcctggcacggaccggcggcaggcccggtggacagcgtcaacaggctgcggatgtcgtcatgcgagaagccgagatcgcgggcgcgccggatgaagaacagccggtccagatgcgcccgttcatagacccggtggccgccctccccgcgttccggcgcgtccagcagaccgatctgctcgtagtagcggatggtgaccaccttgcagccggtgcgccgccccaactcgccgatagaaaatctctctgtcaaaggccttgaacctatagggactatagatcgtatatcggcggccgacacgtttccggcaaggctcgctccgatgaaagactgctgctcctctccgacgtccgacgaggtcggaccgacctgttcaagccggagcgtcctggagccggcgtccgcgccggcggaggcggggtgctgcgccggaccgagcccctgcgcctccaagccgcccttcgtcacgaccgcgcccatcgtcccggcccatacccacttcgcgggcgatgactgctgttccgccaagggcgacgagatcgccgcgctgggtgagcacgccgacgtccggcgcgtgctggtcatcgtactgacgatcaatctgctgatgttcttcgccgagttcggggcgggtctgtttgcgcggtccaccgctctgatggccgattccatcgacatgctcggcgacgccctcgtctacgggctgagcctttacgccctgaagcgcagcctgcgctggcgcgccggagcggcgctcgtgaaggccgccgtcatcgccgccttcggcgtctgggtcttcctggaagtggtccgcaagctgatgggcgacatcaccccgaccgccgagaccatgggcgtgttcggcgcgatcgccctggtcgcgaacctcgcctgcctcgccatgctctaccggttccggaaccgcgacgtgaacctgtcgagcaccttcgagtgctcccgcaacgacgtcatcgccaacaccggcgtgctcatcgcggcgggcggggtggcctggttcaacgccggctggcccgacatactcgtcggcggcgtcatcgcccttctgttcttccgctcggcgatcaaggtgctcggcgaagcttggccccagttccgcgctgcgcggccacaggccgttgcgctcgactagagcggatcgcgcgccgcagccgaggcggcgcgacggaaacgacgaccccgctgtctgaaagcgccagccggaggtcaggaccccggcgaggtctcggggtcgtcgccggcctcccggccgaagcttgtctgcaaggcccgaagccgactggcgatctcctcgtcggaaacctccaccttcagatggtcctggatatactggagccgggcgtcgcattcgcggaggatttcgccccagcaccgcacccacaccgtatagttgggctgtcgcacggcgatgccgatctcgcgtccttcctgggtgatcgcctgtccgacgatgtcgtcgtattcccccacgaccaggaagaagttccaccgcgtgtcggtgtgccggaagtcgggcgcgccggccaaggccagggcgtagtcggaaatctggttgagcatcttgcgatcggccttggccgacggccgcttgagctccacgatcagatactcccgcttctcttgatggggtccgggaatgctgcggccgagcaactggtcgacccggccggttcggccgtcaggcttggtgacccgcccgccggcgcgcttcccgcccaggtcctccgagacccgttgcatcaccttggtcaggcccgcttcgggcaccgcgaggtgaaactgctcgccgaagatccaggtgttgtcccgcaccagcaggtccaggccgccgcgttcgcgaatgaccttcttgccgtcggtgtcgaacacagcctggcgcagcgtctggaggaaggcgatccggtccgcgatcaggctggacgccgcgatgatgttggacagttcggtcttcttgagcagggccgagaactggttctgccgctccttggggagtcccaccacggcgtgaaggatctgggtgagcgagtccggattgtgccgcagagcctcgcgcagcagggtcagggtcatccgcttcaggccggtgtcggccttgcggaactccttggagtagttggacacggcgtaggtcgccatgtcgaacacgtcccgctcccgctgctgaagcgtatcggtcgggtccccctcgtagggataggcccctgcggccttgagctcctcgatcaggcgtccggcccgctcgtggccgcgtcgacggaagtgcgcctgcgactgatcgcggaccgcctcgacgaccttggcgaaatcgccgtcggtcagctccagttcgagcaggttgtcggcggcgagttcgacgaagaagctggaggtcgcgtagatcgagaaggcgaagtcgggcgcattgatccgcgccggctgcgagccgagcacaatgccgttgtcgccgcagaagtggatcttgcggctgtcgatcggcgtcgaccattcgacgatgtcgagcttcaagtcgcggatcgtccggtccttgccgacgatgggcggcaggacgagagagacggcgtcggcgatcgccgtcgacggatcgatccgggcgccgtcgtaccagagctccagctgcgggtagagcttcagatactgggcgaaggtggcggtgaactgccggcgctgctcgtcggtgacgagagcgtcgaggttctgtttcaggggatgcagcgacaccgaaacgcccggagcgccgaccgccggctccgggtcgccaatctcggcggtctcgatggcttcggcgcggatgtcgatcgacagctgtttgagaccgtcctcgctcgcgtatcgcgaggtccagcgggcgcggtcggccagggagaagaaccgcagccgaccccgtccctccttgccgtgataggcgcggccgctcggcgcggcggagcgtttccaggattcgccgagttgtccgaagtcccggtccgcgcggtccgcgctgatcccctcgccgtcgtcgttgacgatgatctcgtcgacgccgcccagcgccgtgcgccggaattcgacatggacgcgcgtggcgcccgcgtcgaagccgttccacaccagttcggcgatcgcgcgcagcggctccgtcgtacggacgacggtctcgatgtggtcctgcttggcctgaagctgaacgcgatgggtcgccatcaggcggccagcggccgcgacgccaaccagcccttgtcctgcaggacgtcataggccagccgcagctgctcgggcgagaactggcgcttgcgctcgccccaggcgtaggtctcggacaccgccgcgtccgcgcttccggcgtccagacgggtcgcgacccagtgcaccgtcgccagaagctccaggccgaacggcgactcgaagccctcgaccaggtcggtcacgcgctcgaagcgcgcctgcgtctcgggggcgtccttgagcttggcctgggcgtcgacgaccgcgccgggcaccagctcgagccgcttggtcggcgcgtcgccgccatcggcgtagccggacagatagtggccttcgacctcgcgcagcacgtgccggaggttctcggcgtagggcccgtaaaaggccttggcgtagcgcagcttcagcggttcgccggcctcctgcatgaaatacatcagcttgtggacctctagcagactgacgaacgggtccagaaggccgttgagatatcggtcgaccagcccgaccagcgccgcgcgccccggcgacatcgcgggcgccgcgcgcgacctcgacatcgcgtcggccgcgggcgcgccgcccggctcatagacgatgacctcgacatccgggactgcctgcagggcttgctcgatgcgcggccgcacctgacgccaatcgagaccgcccaggccgctgccgagcggcggaatggcgatcgaccggatcttccgctcacggatcacgcgaaccagatcgatcaggccggcgtcgatgtcctccatccggctcttgccgcgccagtggcgtttggtcggaaaattgatgatgaagcgcggcgtatccaggcgatgacgctcatagacgaacatccggcccggctggacctcctgcgcttcgcacgcccgcgcataggcctcgtaattgtcctggaacgcgttcttgaattgcagcgcgacgccccggcccatgacgccgacgcagttgacggtgttgacgagcgcctcggcgcccgacttcaggatgtcgccgctggtgaatgtgatcatcgctcccccctagtaataccacgtcggctgcaggtcgacgcgcgccgcgtgggcggcgccgcgcaatcgggcctccaccgccagcttgacgggctggttcaataccccgatgcgttccaccagatcccacgggacgctgtcgtgcaggagaaactcggcctgcttgccttcccgaacctcgggggcggaccaggcgttggacatcaccgcgtcccgacggatttcgtcgagcgcctcgaggctgtcgcgaaattccgcatagtaggcccctgcattcgacaaggtgaacgcccagcgccgcccatgagcctgcgcccagtccaccaccgtgcgcaggtcggcctccaagtggacgatcggttcctggccgccgcggtagttgacctcggggtgattgccccggtgtagcagatagagcattaccgatctagaacaaaaatagaacgggacatactggccgaccgtatcgccaggatggcagcgcaccggaaggtccaggcgccgcgccttgatcgaggccatgccgatggcggtgaccgggccgccggcggcgatcatccgggcgtcgctgaacagcccgccctggccgatgatcgtcggcaggttgtccatgtgggtgatgtgatagattttcgggcgtgccggcgcaggcatggcgtgcgtggttccccccgagaaatgcggcaagtcctttgtctgcctgattcggacgattgtcgtgcagaagccgccagggagcaatgcgcgaccccttgcaaaacgccggcaagcctgccgacctgtctgatcggtcgccccatcgaccggacgggcaggcgctgccggtcaagcgcgtctcagaatccgaagtcgatctgggccccggggtcagccggccgacgccgtggcttcctgggcgcaagcgcaggggccgcgaccgggaggctcggcgtgggctccggtccggaactcggacgcggcatggagcgcggcatgcccggcaacctcggcgcgcgggcgcccttgcgcggcggggggggcgggacctcgcctgaccggctccgcttccattgggtcagttcgctctcccaccaaccgacgcggcccggcgacacgcggacgcggcgcgggaacgcgccatcgcgctccatgcgccaggcggtcgaccggctgatgctggcgatccgttccacctgatcccaggacaaaagacggtcgtccctgccgccgacgtccggcgcgccctcatccacggtcatcacagatccccacaagcctctggtccgcctcgtcttccaagaggtcccgcagcaaccgggcgtcgttcgccgcgtcgatcgggtcccgccgtcgccaggccatcaggacggctttcagggcgaaactcgccgcagggtcggcgagaacctgcgccgctgtgacctcggccctagccacgacgccgcccccgagcggccgtcggcgccccggttcgaacgtcggtgatctggctgcacgcccagtcgcgcagcagcccgcggggataaaacggcttggaacggatgtggcggcatggcggtccgttcgaccccgtcgaccagagccgcgcgaggctcgccggcttcagctggatgccgagctgcgacaggaaggcggaggcttcagcgcgcgtcaaaaggtcgtccgcgtcaccggcggcgcccgcctcctgcccgaccccgagcccgatcatgggtgtacacgcgggcggcaatggcggctgttgcgcggggcctgccccgccgtcagcgccaggtaacaatcgatgaccgcgatcacatacgcctgggtctcggcgatgtccggaacccggccgagccgcgcgacgcggccgggcccggcgttgtaggcgccgagcgcgaggcgcagatcgccgaagcgcaacagttgtcgggcgaggtagtccgcgcccccgcgaaggttctggaccgggtcgaagcgatcgtccaccccgagctcgcgcgccgtatcgggcataagctgggtcagtccgcccgcgcccgccggggacagggccgcaggttggtaggcggactcggtcaggaccagggcgtgcagcagcttctcgtccagtccgtgcgccgccgccgctcgggcgatctcggcctggaagggctggctgagcgcggccaggcggggcacatccccttccccggcgtcggccggcgccgatccggcctccgccgtcgctcggccgaacagatcgccgcccgccgcgcgccaatcgacggtttgggcggaagccggcgcacccagggcgaggagcgccgccgcccaaaggatcgatctcaccatctcagcacctcctgatatacgccgagcacctcggagcgggtcacgggcccgaaataccggctgtcgaaactcccggccgtgtcgccgagcaaaaagagttcgtccggcgcgagccgtcggcatccggaccagcgcggcaggattgcgccgcgccgatcacgggagcggaccgtccagacgccgtctggcgtcagcagttgcgccccttccacgcagacgcggtcgccgcccgccgcggcgacccgtttgatcagcgccgcgtcccccggcatgcccagatccccgagataggcacgcgcggcggccggttgggggatggccacgacgacgccgcgctcgatctcggcgccgaaccgccgggcgtacagcccctcgggcaggctcgggctttcgttgacgagggccagcgccgggacgtgttgagcgaccagcgccaggcagccgagggcgaagacggcgacgcctgttacgcaccagcggtttccattatcgagcgggctcatggctggtacggctcaaggatgaggtcacgggtgatcatcacccgcacgggcgcgcccgcccgcagccggatggacgggcggacctccagttcccggtcgatcagccggccgccgacgcgggcgccctcgatggcggccgcatcgccggcgtcgccgagaaggccgccgccgccctcgtcgtcgcgggcgatctgcccgagcgtggtgatggccccggcgaacagcgtcccgaccagcaggggaaacagacgacgatcgaccgaaccccgaacgccgacggcgccctgggggtcgacgccgggctcgccggtcaggaccaggctcttgccgttgggcaggatgagccggtcccacgtcaggaaggcgcgccggtctccgtaggcgctctcgccctcatgccgcccgatcagccgcgtcccctgcgggagcaccaggtggcggccgctgaccgtgtcgtagacgttctgggtgaccgtggcgatcaccgggcccgcgcgggcggtgtcgaccgccgtcagcaaggcggcggggatgatcgcgccagccttcagttcatacggcgacaggggtgcggtcaggacgtggccgttgtagggggcgccgtagtccgcgctggccggagggacgccggtcggagcccggcgctcggcgcccgccgggaccgcggaggccgccgcaccgtcgcgaacctcggcgaagaacaggccggaccggcgcgccagatctccgggcgcgggtccccgcggttcagacacggggcgatagacgggcggggccgcccgaggcggcggttcggaaagctcggccggcgcgtcgtcgatctcgctcggctccgccgatgaacgcggctccggcaggcggtcgtaggtggccggttgctcggtgacgacctcggccggacggaccacgccgcgggcctcgtcctcgcgtgcggcctcggcgcgggcgcgagcgccctgccgcaattccggctgtacgacgaacgcccatgccagagacccggagatcaggaccacgccgccgatgacgatgatctggacgacggatttgcgcagacgcaccgcgctcggacgaggcgcccggctggcgagctccggggccggagacttgggcgcgcggggcccggcgccgtcgcccggcgtcagaccgggggcgggttgcgggggcgtctcgatcatgggcggactccttgaagacgacgaatgcggaccacctgcggcctgcgatcgcccagtcgcagttcggcgcgatcgagcacgcgatcgacgatgaacaggccgccggcctgccggtagttgacgagctgcgcctcgccgtcgggcgcgatggcgaacagtgcgggcgcctcgtcgacctggaggtcggcggggaaggcgatgaaggtgcgccggccgtcgtggaacacggccgagggggtccatctcggacgccgtccctggggttcgagacggtatcgggcgtcgagcggcccttccggcattacgaccgggtcaggcacccgcacggccggttgcaaggcgacagcggctggccctgcgtcgacgcccccggtcggcgcgctgtcccaggcgacggcggcgttgaaggcgtcggcggctccgctgcgcagatcgaccaggtagacgcgctggttggtggtcaggaccaggttggtctccaggccgcgttcgagcggcttgatcaggacatggacgcgacggtccggcccctcccccgacgcgacctcgccgatctgccagcggacggtgtctcccgccgccttggcgatcaggctttcccccgcgccgagcgtcagggtcgtcacccggagcggcgcggtccacacctcgaacacccggccgggctcccaggcgaagatctggacgccgccctggaagcggtcggaccgggacggcgcgctcgccgcgctgttggcttcggcgatcgccctgcggccggtcagcgccgggagcgccggcgcggcatccgcggccggtcgcggcgccgtttccatgagatagggccgcgccgcgttcgcctccggcgccaacgccgccggctccggctccggctcgtccgccgtggtcggcgccggcccgtccagagcgatcggagcctgcggcagggcggacgcctggctcaggcttgcggtggacgccgcattgggcgcgaccgcgtctcgcaggatcgcgcagccggacagcagggcgctcgaaagcgccaggatcaggacgcgtcgggggtccatgacacatcctcgatcttcaatcccaggggattgcgcaggagttcggcctccgtgcgcggcggttgcagggtggtggtgatcagcgcgcgccagcgctccgagccggcggcctggccgttgacgaaacgggtttcgcgccattgcagatcgaaggtgcggccggagcggcggaccacattgaggatctcgacgttgacggcctcgcgccccgcctcggcgaaggggtcatgggtctgcgcccaggcgttcaggaagcccgccgccttcggcgtcagaagatcgtaggcccgcagccagttctgccggatgacgatcggatcgatcgacttggagcggacgtcccggacccagccggcgagggcgtgggcgatctgcgcctcgttgggctcgtagcggccgccgatggcggtgatccgctgggtctcgccgtagtccgacacctccaccacgaagggtttcaccacggcccgctcggcctggacccaccatcccgcgccgaggaagccggccaggaccaggttggcaatggcgatccgacgccagttccgcgcatgggccagcgacaggcccatgcggtcgtcccacatctgaccggcgcgaagccatggggtcgcttccggcgcggcggccagggtccgcttcgggcggaagaacggatgcatctcaggtctcctctgtgcggaggttgggggacaggacgccgctggtctcgcccgcgggcatcagggttcgtccggcgttggcgacgaagaaggcctggagggcggccgccctgcccggcgggcggggacgcccgggcgtcgatcccgacgcggcgacggcgcggtgaaagcccgagcgggcggcccgggcctccgcatcgcggacggaggcgggccggctggccccggcgcccacggctccatcgcccggctccgccttgtcggagccggtctcggtctcggcggcgccaggatgatgggaccacgcccgggccggctccgcgacccccggaccggacgatgacgccgaacccgccggacggaccgcgccggcgctggggcgcatcgacccgttgtcgttcgaggccggcggcgtcgacgggccgccgccgcccggattcggcccgaacggtggcgacgacggcggcgcccgtccgccggtcgccccggcggcggcgcgcgccggccccgcaagccgcgccgcgcctccgccgatcagggcgccggcgcccgcgatcccggccgcgcccagggctccggcgccgcccacggcgagcgcgccggtcagagcgccgcccgcccctagggccggcccgccggtgacgagcgcggacgcgaggttcgggatgaacatcgccagcatcgccaggagcattgaggcgacgaggatggtgagggcctcgtagatgtccgggttggccgagggctggagttgatcgaacaccgtccgcgcccccgacactacgatggcgagcgccaggaccttgaggccggaggagacgacgtagccgagcggcctctcggccaggaaggcggacttcgaccagatgccgaacggcaggaggatgaagccgcccagggtgacgatcttgaattccagcagggagacgatgatctgcagcgcgagaagggcgaaggccagcaggatgccgatcatggccaggcccaggatgagggcgtccgccatgttgccgaccacgtccaggggattgtccaccggcgccggggtctcgcccagggccttgacgatctcccacccctgctggagcacggcacccgggttgaggaactcggcccgcgaaagcgagccgcctccggcgacgagccccagctccaggaagccggcgtagatagtctccgacaaggcctgccagtcgttgatcagccaggcgaagacgccgatgagcagcaccttgccgaagccggcggccagcacctcccggttggaggagagcgcccactggattccggtgagggccacgaccagcacgatcaacaggccgaacacgccgttgacggcgccggacagggcgtcgaagcccgccgagacggtgttcgagaacaccaccatcaggtcgttgggcgtgtccatgctgaccggggccatgacgatcagtcccgggcgcgggcgaacggatcgaaggacggcgcgacggggacttcgcccgagccggcccagcgctggcggcgggccgcgtcgccggaggcgcggtcggccgcctcccgcgccgtggcctccgccatcagccgcgactgggccagcaccagggtccgcagggccgccaggtcctcggccagaaccgcgagcagctgattggtcgactgcacggccgcggtctgtcccgcagccgactggctggcgccgagcgcaccggccacccgggcgtcgcgggtcccgcccagccgttccagttccgccgccgtccgcgccagatcctcggcggtgcgccgggcgttcgcggtgcgcgccccgctctgctccagcaggcgcagggcgtccgcgccggccagatcgtcgggatagtaggtctcgaactggcgctccagaccgctgaccgaggtcgccagcccgcgcgccgtgcgcgccagctcggccatatcccgcagcgactggctgctgcccgccagatggctgtagggcgaggcggcgaggctgcgggcctcgttggcgaggctctccagctggcgggcggcctgcagcgcgttctccaggtgattgcgggggtcgaacaccacctgctgggcgccggccgaaaccggcgccgccagggcgaggagaccagcgacggccaggccggtcgccctattccgccgcgagcggcgggtcgaaggcgtcgaaaacggaatccacattctgcactcccttggctttgaggaattcgcgggcgaaggcggcctcgccggatcgggccaggacgtcgtcgatgagggtctggtcctcgggcgtcccggcgccgcacagagccagggccacgcccgtcaggcgcaggtcgaacagccgacggccccgaggctgccgccagtagtaggaccgcttgggcggggcgaaggcgatcagctccagctggcgccggttcaatccgaagccccggtagagcgcggccgaagacggctccatcgcgcgcgggttcggcaggaacacctgggtcgggcagctctcgatcaggctggcggcgatggcggaggcggccacgtcgtcgaggctctgggtggcgaacatcaccgccacccgcttcttgcgcagggtcttcagccactcccggatcttcgccgcgaaggccgtctcgcccaggaacagccaggcttcgtccaggatcagcagggtcggccggccgtcgaacccctgctccagctcgcggaacagggccgagagcaccggggccaccgctgacggcgtggccatcagcgtctcgagctcgaaggtgtcgaaccggctggttcccagcgccgccccctccccgtccagcaaggcgccgtgcggtcccttcagggtgaggggttcgagggcggcggcgacggcgcgatcctgcaccagggcgcagaacaccgtcagggtccgttgagacaccggcgcctcggccagggccgcgagggccgcccagatttcctcgcgcacccgcggggtgggctccagcccggccagccgcaccgtctcggcgagccattccgaggcccaggcgcgcgcatcatcgcgatcgatccccgccagcggctgcagcgagagccccgcgcccggctccatcgcgcgccagcgcccgccggccgctagcgtggccgcccgcgcggagcggcccttgtcgaaaaagaccacgcgcgcgtccggataccggaaccattgcagggcgaggaaggccaacagcgcggactttcccgagccggtcggtcccacgaccatcgcatgaccgacgtcgccgacatgaagcgcgaggcggaacggcgtcgatccggttgtgcgcgccgtggccaagggtgggccgtcgaggcaggcgtcttccgacggccccgcccacaccgccgagatcggcagcaggtcggccaggttgagggtggacaccagcggccggcggatgtccgcatagggttcgcccggcatcgatccgagccaggcctccacggcgttgaggtcttcgatgcgcgccatcagaccctgcgcgttgagcgcggcctcgatcgcgcgggccttggccgtcgcgccctcctcggtcgcatcgaggacggagaccgtcagcgtcagatagccaaaggcgcagctttccgcgcccagcgcggcgagcgcgccgtcgcactcttcggtcttggacgcggcgtcggtgtcgaggagcggcacctcctccttggtgatggcctcgcgcagcagcacgccgacgcccttgcgcttggcgaaccagcgcttgcgcagtttgacgatctcgcgctcggcctcgggcttgtcgagcccgatccagcgcgcggtccagcggtagtcgaacgggagggcgcccagggcgtcgagcagacccggccgggtcacggacggcagcccgcgcaccgagaccaccttgagccaccgatcgccgagcctgggcgcaattcccccggtcaggtccgcgtccgccagccagccgtccaggaacatcggcgtctccggcgggcggacctcgaaggaccggggggacacgcagtcatggagccaggagagaagaccggcgtcgtcgagctggcggatctccgttaggccgtccgacagcaggtcgaacaccgcgtgtgcctcccgggtgaaggcgtcgagcgccacccgccagtcggcgccgctcctggccagaccgtcgaacagccagcgctcaaggcgtcgggtctcatcggcgggcggcagccaggtcagcgccagccggtggtcggtctcgaaggccggatcggcggtttcgaaccggctgcggcgttcctcgtcgagcagccaggcgacgccgaggtcgaagtcgctttgcggatagggcgctgcggcccggcggtgcgcctcgacgtgaaggcaccagccggtccccagccggcgcagggcgttgttcaggcgcgcgcggaccgccatcaactcctcctcggtggaggattccaggtccggcccgcggaagcggaagcccgccaggaaggagccgtccttgttcaggacgacgccgggggcgacgagggccgcccagggcaggtggtccgcgagggctgcgggccggcgccggtattcgtcgagaaaccgcatcgcccctcacccgtccagatggcccggcagggccagatggcgccgcagaacgtcgaagaagcgccgatccgaccgcgcggcccagaggccgatggcgtgggcgaccgcccaccacagaagaccgagccaccagatgcgcagcgccagacccagcacgacggcgatggtgcccatggcgatggcgtagtcccgcggcatgccggccatcaggaccggctccgccagcgcctgggccacgggcaggtcccaaccctcgggccggtcttcggaccgcgacgccatcaggcgaactccacccctccggcgaagccgaagaagtccaggaagaaggtggaggcggcgaacgcgatcgagaggccgaacatgatccccagcccccggcgcatcgaggagccgttctcgctcatggcgataccggcgccgaagatcaccacggcgacgacggccgccgcctggaccacgggtccggtgatcgactggaccacctgctggagcgggccttcccaaggcatgcccgacccgccggccagcgccggtccggcgaccgccaggccaagcatcatcgtcgcgccgaacaggcggcgcccaagtctccgtcgcatgatttgctttccttgtgttcagcgcgtttcaccgcgcttcgactcattgcaagcaaaactatcccgctactgtcaacagtaaaatacgcaaataattcacgacttgaagacgactacactgtaactcagatcgacttgaatagtaacttggatcgacttacagtgttgatgccgcgacgacttggtttgacttgagacaagtcgtcacacaatgccttgaattatcctcgcttttctggagtcggcatttgcgacgccattcgcggcgtcgtcaggccaggccttcgaccgcgtagcccgcgtccgacgcgccgttcaccgcgatcacggattcaagccgccgccccgccgtcgagcgacggatatgagcgataacgtccaccgcctggccgatggtgcgacgcggcggcgccgcggcgatctcgagggccagatcctcgatccggcgcagcgcctcctcggcggagttggcgtgaagggtcgagaggccgcccggatgacccgtgttccagctcttcagcgtttcgagggcggccgcgccgtcgcgcatctcccccacgacgatccggtccggacgcatccgcaaggcgtcgcggaccagatcggcgacgccgatggctacgggggcccggcgcgtcaggaccgacaccgtgtcccaggccgagcattgcagctcggcggtgtcttcgatgagaaacacccggtcgtcggcgaaggccggctcggccaggatggcgttggccaaggtggtcttccccgaccccgtgccgccggagatgaggatgttgcgccgctcgcgggcggcctgggcgaggacatcggcctgccgggccgtcatgacgccgtcacgcacataatccccgagggtccagatcaccgacgggcgcttgcggatggagaaggccggcgccggcgacaccgccggaagcaagccctggaaccgttcgccggtggcgggcagcacccccgacaggcgcggatcgtcccgggtgaccacttcaccgacatagtcggcgatcagacgaatggcgcgttcgcgcccttccaccgacagacgcgccccggtgtcggcgcggcctcggccggcgcgatccaggacgatccggccgtcggggttggcgaggatttccaccacctccgggtcgatcagcgccgctagcaccacctcgcccagggcgtgacgcagcgcctccagcttgcgttccgcgatcaggggatgagccgtcatgtcagttcgccgccccgaacgatcgctcctcagcctcccggccgtgtgggtcgtgctcggcccggcccgagacgatccgcgccgcggtgtcgtcgagcatccgctcgatgcggcggtcgacggcggcctgcaccgtgggatcctggtcgccgacgccatccgggagccggacgaacagcgcccgagcgacctccaccaccaactcctgaatgatctgcatgtcctgtcgagtggaccgcatatggcccttgagggattgctcgagcgccaggagcctgtcgtcggggtcggcccgcgggttcccctgaaggccccgcgcgatggcgtgtccggcggcctgactgatcgagacccggccggaccgcgcttcgcggctgataccggcgatgattttgggatcgctgagatagacctgaacgcggcaggtctgcaccggcgcgcgcctaaccatcgccctgccctttcagatgatcgaggacggcgtcctgcgccgccatctcctgggctacgcggccatagatgtccgcggcgcgcgcggcgaccttcttgtcgtccatcgccgccacgatctccttgaacaggggaagggcggcttcggcgtccacgccgaggctgcggcggccggcccacggatggggcgcgggcgtcggcgcgtcaacgcccgcggcctggtcgggcggcggcagagcggctctctcccggaaggggcggcggcgatcatattggagcttgcgggtgcgcagagggcgttggcccgccgcgaagatcagctgaacgtcttcgggcagagcgcgcacctcgccgggttcgagcaacggacggtcgatctgggaccgggacacggtgctgcgtcccgccgccaggccggcgggcgcgctgcggctttcacgcatctcgccgatcgtgccggtgagtttggagaccttgtcctgggtcagcggatccagcgccgaaaaggctgtgtagatggcgcagttatcgaggatcgtgttgttggcgccgtacgtctcgatgatgtcgttcagcgactgggcgacgaacatcaccttcaccccatagccgctcagtagccgcagggatttctcgaagaagctgacgcgccccagcaggggaaactcgtccatcagcatcaagagccggcgctgcttcggccgtcccgccgcatcccgggcctcgtccacggtgagggcctgggcagcggcgtagaacaggagccgcaccagcggccgaagcgccgccgcgtccgccggcgcgacttgaatgtagagcgagaccggtgcctcagcgcacatcaggtcgcccaggttgaagtccgaggccgagagcgcgcgctcgacgtcgtcgcccgcgagccacttcagataggatcgggccgtgccctggaccgatgtccggaatcgatcgtgcatggcggcatagccccgcaccgccgttcggatgaagggatgggtttcaggctcgcggttcggacccgaccggtgcagcgccttgaccatcacctcggccgtgtcgtcgaggtcggcgagcagttcgcgcaccttcagcagcgtcttgtcggcatcctcggccgtgtagaggacatgcaggattaccgcctccaggatttcggaggccgccttgtcccagatggcctcgtcatcccggacccctccgggatcggcgaggatcgaaaccagccgctggacctgggccagttctcccgggccgggttggatttccgcgaggggattccagcgcgcggatgcaggatcgcgcgggtcgaaatagagcgcgtgggagaagcccgaccgccagccggccgtctcgcgccagagctcccgcttgggatcgtggaccagcacgctctcgctccacagcagcagcgtcggcgtgacatggcccctgccttttcccgaccgcgtgccgcccgtcaccagggtcggccgcatatcgacggtggcgaggagccgccccttcagctctccgagggcgcaccccgcgccggcgagcagcccggcggcgcgggcctcggccaagccgccccatccgcggatacgtcggcgcggtccatcgccctgcgtgagcatgccggcacctagcccgcccatcacccccaacaggatcaagaaggcgctggacgagaaggcctccggttcggccccgccgaactgcctgcgccagctgaggatgcgccacggcggatagatgcgaacctcttccgacaccgtccagccgtcgcccagcacgggatcgtggcgataggtccaggcgaaggtctgcgtggccagctgcaggccggccgccaaccccgccccgagcaggatcagccgaaggatcatggcccctcgtcctccccgccctccccccccggatgacccgcgacgtccatcgacaggagcgccgcggagcggccgcgacgataatgatacgcccgcaggccttcgcggagttcgccattggcccgcgtcgccgccagctcaagaagatcgtccgcttcggcgtcgaggtctgcgaaaatccggcgctccgcgctccggaacggggtcagctggccatcgacgcggtgataggcgtcaagcagggcgccgttcccagtccggcgcaccaggctctcgaacaagtcctgcaggtcggtcacggcggcgccgtcgcgcgcgggcgatcgcccgtagccgggcaaccccgcggtcaggtcgagcgcagccgacagataggccaggcgcagatcgtagcgatcccgcaccgcgccggcgtccagacgggccgccagaaacccgcccgccggtccccgctcgatcaagccctccccgcagagccaggccagcgcttcccgaaccggcgtggtcgacaggtcgagacgacgcgcctcctcgacgatgacgatcgactgacccggcgcatagccgccggcccgcgctcgctcccgaatgttgtcgagggccttgaagaaggggtcgcgacttttcgccatgacagtctccggctcccgcgcgcccgacgcacgcggcatgtaaccgctcgccaacaagttgcgtggtgtccggatgcagactcgccgcatatcggcgttggggccgccgctatgtggcgggaatcgatttgaaacggagaggtgatcgccgataagtcggcgaaccgaaaatcatcagctaacggagggagcaagctttgacgtccagacgaatgcagccgcagcgcgatagcgatgttctctcccaggcgctgaaattggtgcgccgtcaccgccgcatgacgcgcgcggtcgtggcccaaggcatgcagatggcgctgcgaacctacgatcgttttgaggcgggcggtcgcagcctgaacctcgactacattcaccgtttcgcggcggccacgcgaagcgaccctcacgccatcgtcatggcggtcgcggtcggttcgcctgagttggcgctgcgatgcgcagacaataagctggtcaccgccctgaccatcgggggccagcgcttcaacgccttgctcggcgacgacatcgccgggctcgaggcgcggcccatcatcctcgcggtctgcgccatgtacgacgccttgctggccgagagcgaccggcagcaggccgccacacgctggctcgagaacggcgtcaccgacctcgcgcaagtccgccccgctcccggccgatagaaatatatttcgaatatagttttgagacttcgccatccgggcgctgactgtgttcgccacactcgtggcgaacacttgatggagagactgagatgaagaagaccactctgcgcctcgtcaccttcggcaatgcgaagacgctcacgcgtgacgggctcggcaccatgttcgaagaggccggcgtgaagatcggccgctcccctcccgagggctgagcgagggggggcggctggtgacagccgcccgccgttcgtttcggcgacgtctatgacccaactcctgtggtgtgcgcctggcgtcttcatgagccgtgtggatgacgacgtggtcattcttgatgtcgagagcgacgcctaccagtgtcttatagggggtggagcagaagttcacttcgctcctcaaggcgcgcttcgaattaccgaccccgatctcgccactgagcttcaactcgctggcctgatcaaaccagatagaccgccgcgacttccttcctctccaattgcagcaacgagagaactgccacttccagcacgaatgtcggcatctgaagttctttcgaccggcttcagttgggctatcgctgccgtgagatttcaacggaagtcgttaaggcaactgcttgcgtttgagcaggccgatgggcttcagcggtatagcgaagagaagctttcccggctggtgggtgcgacacggatctcgcgcacatgggttccgggcgaaggcgaatgtctccagcgttcgtttcagctccggcacgtgctcgccgcgcgaggcgtccgtgcagattgggtattcggcgtacggacctggcccttcaatgcgcattgctggcttcagatcggcgatctcgtcgtcggcgacaggctagcccgcgtgcgccgctacacaccaatcatgcggtcttgaggatgggcgattatctgctgatctgccgcgcgcccaacgacccccgagcctcaaggctcttcaccgatctgcgggccagagcatcggcagagggatatgttgtcactccgatcaatgcccacgcttggctaggtgtccgcggcccctgtccgccaaagcgtgtggacattggaggttgggtgctcattggggatgtatttgatcgccggtcaccccgtctcccctacgttgacccacaagatcagtgggctttcgagcgaaagctcgtcgcccgcgtgtggggacggtatgcaggagttctctttggccccaaggaccaaccggcagcctttatcagagacccgtccggcgccctggaatgcgtcgcttggacccactgcggattgaccgtggcgtgctcggcggccgacgactggctcgtccgttgtcttcgtccccgctggcgcatcgactatgcccgcgtcgccgaggcgttgcatagtctggttgcgggaaccggcgcgttgctccttgacggcccgcacgcccttgagcccggcacggtgcagccgacgccgctgacggtccccccgatagctgtgtggaccccgcgccagatcgcgatgcagagccttgacccgccccccgcagcccaggcggaagtcagcattcgctcggcggtggacgaggccgtgtcccgcctttcaaacctcgccgggccgctcgcggccgaggtgtcgggcggtctggattccagcatcgtcgccgccgctctcgcgaaggtcgcgttggaacctgtcagcttgtggatcaatgcttacggcgccacgccagagtccgatgagcggtcctatgttgaaatccttggcgatgctctcggcttcaagccttactgcaccccccatgccgtcggtccgctgacatcggattggctcaccgcgctcgcgggtgggttccgcccggggttgaacgccctcgatcatcctcaaaacctgcgctgggccagccttctacacgaccacggagctaaggcggtgatgacgggaaaagggggtgacagcatcctgtttcaagccgccacgacggacgtcttcacggatcaatggctggcgcatggatggcgagcactggcttggcccgatctcaccgagctcgccgccgccaatgagctctcggtctggtcaatggttcggacggcccgccgatatgaaccggggaaacccgatcccctcctccgcgatcaccccattctcgcgccgcttgatcgacagcctccgccacatccttggctcagagaccttgagggcttcggacccgccaaatgctttcatatcgcaggggtcgcggacagcatttcccatcacaacccctcgtcgctcacgcaggcggtcgacgttcgccatcccctgtgcgcgcagcccgtcgtcgaggcctgcctcgcccttcccaccgctcagctctcggtcggcggcagagaccgggggctggcgcgaagggcgtttcgcaaccgattgccgaccgcgatcgtcgatcgccggacgaagggcgagatgacccggatttacggacgaatggtgtcggaaaatctggacaccctccgaccgtggctggccgacggccggttggcgtcatgcgggattatcgatcgggagagggtgttgaccgaactgtctccggaagtcttgatctggcgcgggcagcacgcggctgtcctcacggcggcggcgtttgaaggatgggttcgcctttgggagcgtcggctgacgtagtctcagaaccagcatcatcgagtgtgagcgccaaccaatcgaaaatctgctggtagcgatcgcggatgttggccgggctccatgtcagatgcttctcgccccaataggtcacgatgcgggcgtgtccgtggttgcgaagaatggcgctaaacattctctcggcttgtgtggccggcgtgaagtcgagatcagccgtcaggaacaggatcggcctcgttatgtgatcggcccgaagaaatggactggaggcggcgtaatcttccggcgcacgccacggcggatcttggagcgccccctgaccggtctcggtccaaccctggttgaacctgaagaacatgccgttttccggctgtatgcgccctaaggcgtcgaactctccccagacaccaagcatgtcactgtaggcggacgaagcgatgtaggatctgaaccggcccgagcgcgtcgcgatctcgagggctgaatagccgccaaagctgtgtccccaaaggaccatcctgtctgaaggaagctccggaaaggcggccaacgccgcatcgacggcgagatcgacgctgcgggcataagcatcgccacgctccctgacgggtagatccccagggacagatgggctcaggacggcatagccggccccaacgaagacctccggccgaaaactgtacgtcatagtgagcgggtccagccgcgccagattgtcagcccagcccgggtaggggttcacgatgacgcctcggggttcgccgttcggcagaaacagccagctttccgtttcgcgaccgtcgaaacccaagtggcggatcggcctgggctcggtgacgaacatgttcgcaagggtcgagttaacctcggctatcgcttcagtcgatcccggtctatgatgcaaaagggcatctgcgagcccgcgcggacggagtgtcagcacggcctccggagaaacggcaagtgtcttgtcgaggtcagcgccgccgccccccaacgtcggcgctgcgccgtccctcaccaacctcacctggccttcgccatcaatcgcgatcgaccaatctctgcgcggcgcctcgttgcttttcgggcgacgccccatggtgaggtcgaagatcatggcctcccggaggttaaggttgggtggcgagagcgcatgggctccgtgcgctgtgatttcccagtagcggccgtccgcgaaggcgagcaggccctccggcccggatgcagcgatgcgcgtcggagccacaaccaaatcgcccgtcagggattctgggacaccgtcctgagacagcagataccagtccccgcgctcaccctccgtcggtcgtgcgtacatgaccggggtgagacccagccagtcggcttgcacgccagcgacaacaacgctggctgacgcgccggcacgcaacccgccgcggttgaatgggtcggtcgactcaaaactggcgctcatcagcgttccctcgtcccaccgagcgccgtctgggcgggcccaaacgaggacggccgtcgagtcgggtgaccatcgaagaaggtggggcgcgatgtccagcccatcgactcgcagtggcacgcgccctgtcctgagatcgatcagaacaagccggcgccttcgatcatcctccatgtggagaagctgcggatctcccaatgggatcggctcctccctcatgaccacggcgacgcttccgccgtcaggcgagacggtgaagtcggcaagccatccctcttgcaaggtcgtgatctgcagcgtgtcccgttccagccgaaccaaggcctggcggggctcggggcgctccggaacgaccacgcccccccgcgcgtcgatgacggtcctggagggttcgcgcccttcggcggtccgctcccacgcctcggcgcgacgtctcgtgcttgtacgatcatacccgagagccagcggaagactgtggtcggggcgcactggcagcagcagcgtgtttgcagacgcccatgtcgcagtcgccccgcccaggggaagatcgggcgtcaggccggtccatcggacggatcggtcgactagggacacgatcccgtattcgaatccgtcgccttgaagcctcgtgataaggagatgatccgaggacggcgaccaagcggcgaactgcagccccaagccttcgtggggaagcaacctttcctctggagaggttggatcgctgagatcaacaatccagagctccatgatttgccaggtggaacggccattcgcttcgatgcggggcatggtgtcgtaaggaccgcgcctctcgtaaatcgcccatcggccgtccggagagatggccgctcttccgaacgcctccaaccccagcaaatcatcaaccgtaagcgatcgatccgcctcgataccttggccgtgcgcggcccccgccaagcaagccgctgcgatcgccgttccgacgacgcgacagatgagcgtccacatttcggatactcaccagcgtcgcgtcagttgcagggagatcacgcgtcccaagatgctggcttgaccgggatcgaaccccaaaccagtcggggcgtcgtagaacggcggcgcttcgttgagcagattttggacggcaagctgaacctggacgccgggcgcgccggccaggtccgaagtccacccggccgttgcgtcaatcgtattccaggccgagaggcggttgccggcccgatctttgctgccggccacatggttccaatgaagcccgaccgcgacgccgtcacgcgaccaagtcgcaccggtccgcgctctcaggtccgtcgggtaacctacgaggccggcgacctcctcaatgggcgctgtcggcgtcgtctggctttcgtagtccaaaatccaggacgctgtcaggtcgagcgcgagacgaccgttgctgatctcccaaccgtgacctgcctgtacgtccagaccgctgacacgcaccgcgccagtgttgacccagcgtgtatccaccacagcgccgtacgctgtgaccgggaagaggctggaaaatccgggagcgtccgagaagctctcgatgagtgcgcggtcggcggagctgttgaccggatcgacgaaggtcacgaagggacggagcgtggggtcgatgagcgccccgtcgaagttggcgttcacgggctgcgcgatgcggtcatcgaaactggtcgtgaaaaagttgaccccgagcctcggccctctggtcgggcgatagtcgaagccgagtgtaaaggtttctgaggtctcaggctgcagatcggggttgccaccgtacagcatgaggatcaacgcctccgacccatcggcccgatccaaaaaggccggggacacgccgaactggtcgaacagctgcgtgagcgctgcggcgcggaaggacgtcccccaagatgtccgcatggtgatctgctcgtccggcgaccagatcaagccaagcttcggattggttgtcgaaccgaaatcatcgtagtcctcgaaccgggtcgcgacagaaagctccaggcgccggatcccggctctttcattgtccggtcccacaatcggaatgcgcgcctcggcgaacactgcggagatggctcgagatcggtcggggctggagataaaacggggcgcggctgccgtcaggaaggtctcgccctcggtctcaaaggcctctcgtctcgcctggcctccgacagccaacgagatatcacctcccggaagacgccaaagaggtccctgcacaagcaggttcgccgaacttgcgcggctacgattccggacaacaccgtagccgctgccgatgaagtccgacacagcctgggcgttggcgctgccgtctccgaagaggttgaagtaaccatctactgcagcacggaagggcgttgccgggtcgtctgggatgttccccaaggcttccgacaggaaccgagtgttgacgcggttgcttacgccgaagtccgccagttcccaagcgtcggccacgtaggcctcgaccgaccaagtcggcgaaacgtcgtaacgcgcaccgatagtcaagcccaagctctcggattcggtcgagctccgcgctggccctatatcccgaaggaaagaatacgccacggtatgcgatgaagcgccgttcggcgacacgaaccacggattggcttgtgtgacattgaagatccccgcggcggccgccgttgccgactccgtcgttcgaaggctgtaacggatgtccccggtcaactcgagccgttcgcctatcgattgccggatgcgcgcatacgcgctgtggcgttcgagtgcaggcagaagatcgataccggcgagcggggattgaagattgctctggcctgccgcgaagtcgccgggggtctgcgccgttccaccggtcggtgggcggatcgcgaactggacttcgaacgcagatgtcgcggggttgagcgcgagaatattgccgggcgcgctgtagaaaccacggcggtcactcccaccgaagggtcgcagatctccatccgccgtgacgcttcggtccgaaccgctcaacgcgttggcggattgatattcataggccaggtaggctgcgcccgatccccagttacgacctatgaggtgcgagacttggacgtcctctgcaccgccttccgcggcggagacgcgtgctcgcgtctcctgtccgtccacggatcgccgcatgatcacgttcacaacgcccgcgaccgcatcggacccgtaaagcgcagatgcgccgtccagaagtacatcgaccctgtcgacggccgccgacggaagggccgagacgtcggcgaactccgcacgagacccggttcctgcgagccgacgaccattcacgagaaccagcgtggacgccgccccgagaccgcgaaggttcaccccggtggcgtagacatcgttcgaggtgccggcatcagcgagcgtggcttggctcaccggcgtggacgtgccggcgtaattctgaggtaaggaaacgagaatgtcggcgacagtgccacgaccggttccatccagcgcatctcggtccagttgaaccacgggcgatgccaaatctcccgacgaccgcagcagcgttcccgttacgatgacttcatcgatctcgaccgcctcgtcgacactcgccatgccggcccgctgcaccgcgaagaccccaggccggctctgcgaccaggtcaggccggaaccggacagaagccggtccaaggccgcccccggctccagccgaccgctgacgccgggcgaccgcaggcccgccacggtgtcggaggtaaagaagatctggtgaccggactgccgcccgaaggccgtcaacgcctcgctcatcggtccgtgcggaatccgaaactcccgcacggactgagcgcacgcgggcgagctggcggcgacgatgcaggcgaccgcggcggcgcctgacagcagataggaacggctcatagactggtttcccctcgacgcccccagtggcgctgaagagagagaccatcgagaccggggctaaccctctcggcgtcccgaattaatttctgcgccgggagagcccgaccgatccgtccgccttcggaacagcccgcaatcccatgacatccgaagacgcggccacgaaggcgtcgcggtcgccggtgcggaagacgccattgaccgccaccgaccggatggcggggtcgtcgatctcgatcttctcggtcaggtaacggttcatctccgccaccgcctgcgccagcgggatatcggtgaagacgagttggcccgtggcccagctggtctccgcctcgacgtcgaccgcgcgcgtatcgatcctcgcgccagagactcgcacctgttggccggcggcgatgcgacggggcggcgacggcgcctggtcggactggacgtcgatagcgccagacacgagcgtgacgcgaaccccctcccctgccctgcgcacgtcgaaaaccgttcccacggccgtgacccgggtctcgccggcgtagaccacgaagggacgcccagcgtcatgcgctacattgaagagcgcctgaccttccacgaggtcgatccgccgctggcggtccgtaaatctgacgcgcactcgtgaatccgtatcgaggctcagactcgatccgtcggcgagcgggatcacccgctgctcgccgacccgtgtggcgaacgcgttcctatcgctccagaaccaggacccgcccaccatcaaggccaccgccgtggccacggccagaccgccaaacagaacggaccgccgaccggacgccgggctcacccggcttcggcgacgggctccctccagggcgtcggcgagcgcggggtcgggtccaagaccctggctctcgcgccagacgcggtcgacccggctgtacgcctcggcgttgccgggcctggcccgccactcgaagaattcctcgatggtgcgagtctcgatcgaagtcgtgccgaggcggacgtgccacgccgccgcctccctctccgccgcttcaacccgcatcgtcgggttggccatgtcgcgccccatcctagcgccggagctgggcggcgcagtgggccaaggcccgggtcatgcgcccttccacagtcttgggggagatccccagtctgtcggcgatctgggcgttcgtcagaccgtcgatccgggacaataaaaagacatctctcacggattctggcaagctcaggacggtctccagcaacatcaatcgttcggtttggtcagcatcgacccgatcatgaaccgaccggatggcttccgcccggcaagccagttcacgtcggcgccttgcgttgcaggccaggttcacggcgatccgtaacaggaatgctttcgggtatcggagaccgtcaacagatttgcttgaggccacgcgaagccaggtttcttgggacaggtcgtcgcattcgtcctgcccaaaccgtctccgaagggcacgccgcaaccatgcgccgtaacgacgttccagagccgtgagccgatcctcgaaccggccttcaacactatcgactcggtcatccacgcgtcgctccgaggacttcgccctccaaatcaagggatgtcagagcgtaaaccaccatcggaatggtcactatagtgactggcccaaaatgtacgttgggcgccgcctgcgtctatggcgcttacgagaatctttgggcggaacgtacgtcgtgcaagacagaaaaaaggcatgacaatcgagggcttggcagacgccgtgggcctgtcctacagctacatgggagagcttgaacgggggaagagaaatccaacgctgcgcgtcgtggaaaatctcgccgtcgtccttgaaacgccgccaacggcccttttggccgaatctcactcctgattccctgacaacgcggcatgcaccagcggctcaactcacagagccacaagtcgcaatggttactatgatgactggctgctcgacgcgctttgcgtgtgcctgtatgaatgagtttgacggagacttttgggcgcaacgtccgccggattcggcttgagaagaagctcacgatcgaggggctcgcgaccgacgtaggactctcatatagctatatgggccaactccagcgcggcgagcgaaatcccaccttggatgtcgtggagcggattgccaaagcgttgggcgttaaagccattgagctcttccgcgaacgttgaccgctaaatgccgacagacgcggttaccctgctagcgagaaacctccaaaccctccgacgcgccgccgggctgtcgcaggaagagttagcattccgtgcggggacaaagcggagctacctcagcgacttggaacgcggcgtccgtaatccatccgtccgtctgttgggccgtttggccgagggtctagacgtgccgccagcgcggctcctcgagtgagatcgcgcgggacgcggctcagctggtcagtcagcctcctcgtcccggatctgcgatgaagaagtcggcagcaggcaacgcaacaagtcccggatcagccgctgctgatccggacccaagcgcgcggccgagcgttcgatcgttagggtaagcctcgtgggcggaggccccatcgtctccgctgtcgctccaccggtctgcgccaggccttttcaaagaagtagctgacggacacgccgaggaaacccgccgctttccagagcctggacgcggagacgcgattggcgccgcgctcgtatttctggatctgctggaacgtgagcccgagcgcctgaccgaggtcgctctggctgagtcccagactgcgccggcgatgagcgatccggccgccgacgtgaacatccacgggattggcccggcgatcgccgtcgcccttctccactggttcccggtcgaacatcagactccccggcgttcgcgctcgacactgaaagctgcagccgctccggatcgaccgacgaagccgccagagccgcagcgttcgggatcatcatgtcagcgttcgagggctgcgcaagccattggccccaggcagggcatcgcagtcatagccgtccgaaccgaaagggccgccaaccgcagcgctcaggcgaccttgtccagcaacgccgtcaccttgcgcgcggtcgccttggccgatcccggattctgacccgtgaccagcaagccgtccgcgacgacgtaaggtccgaagggcagcagtcccttgaggtagaccgcgccgcgccgtctcatctccgcttcagcattgtagggcatccggcccgcgacgccggccaacacctcctccgcccacgagaagccggtgagcatgcgatccatgaccagcagtctgccggtcgtcaggcgcgtgttgagcagcgcgcaatagccatgacagacggcggcgacgataccgccgcgttcccacacggcgcgcgtcagggtctgcaggcccggactgtccggaaagtcccacatcaccccgtgaccgccggtgaagaaaagcacgtcgcagtccagcggatcgatgtcttcgggccgctgcgtcgtctccagtcgcgccatctgtcgaggatcgcgcagccaggccttcgccgaaccgtccaacagaggccatttgagcgcgcgcggttccagcggcgaccggcccccgacgggactgatgatgcgctgttcgaagccgcgctttgcgaaatgatcccaggcatgggtcagttcggacagccacagtcaggtgggcctgccgtcctcatagcgatcgacattggtgacgacgtgaacaacgcgcttgtccatggtcggagcccttcggtcgtcagttggctgcgctcggcaatacaactcactatgctggataatacaaccggaacggtcaccgttccaacccgctcccgcgccctctcaggacctgcgccaagccggcgccggtcggggcgagcgccacggtcttgccgatctcaagcctgggctcacccgcgcgcagccgcgcgtagtgttcggcgccgtcgccgtcccgcacgatcacgaacggatgcgcgcctagctcgtcgtgaaacccggtcttgaccacgcgtcccttcagcggcgacgcccccatgggtctcacgtcccgcccgacctcaagccgccgctggttcagggtgcggatgatgtcgcggcgcgcctggagcgtccgaagcttcgtctccatctcgggatcgagccgataacgccggccggcgcggaccgcgagacccaagccttccagatgacggaggcggcctcgactcagggcgttccaggcgtcgctccgtcccacgccgtcttcaaccatcccgcccggctccgccgccgccaggagccggcgatcaagtccggtgaagcgatccgccgacgtctcgcgccaaacacgcttctcggcgtcgacccgggccaggtcgccgagcctctcctgtgcgacctcctgggcgcgggcgcggaaaccgtaggcgatatagtcgcgcgggatcacaaggtcccgcccgtcaccacggcgaccgcgcacgagcacatgcgcgtgcggctggtccgtgtcgtaatgacaggtcgcgatccaggtcagctgcggctcgcccagatccgccgagacccgcgccataacctcgcggacatagccgcgcaggtcgtcgatccggtcgccgtgctcgggcgagatgatgaagcggaaatggtgccggtcgtcggtccagcctctcgtctcgacggccgcttgaacgccgtcctgatgccgatcgaagaactcgggccgggcgccttccacgccagcgccggagcgaccgaggtaggcgacgtgcgccgccaacgccgcgccacgctctgcgcccttgccggcgtggcgagacaccagagccttgacgatgacgcgctgtcgcacgtccaggcggaaggcccgtcccgaccggttctgcgccgcccggagaacgcccgaccgattgccgagagcaaacattcgggaactggcgaggcgcttcatcatgccaagacgaaccggatcgcggtcggtcttcagtcgcgtcggaagcctcacgccgcccggggcgtcctcgacgccgccgcgtatcgacagcctggtttgaatagcctggtgaacagacatgatccgcgctccggccccggaagatccgccgaagaacgacaactcaaagcaagtcgtcgatccgggtcgacctctcctccaagatgctgaaagcataaagaaagccggccaggcccaacactcccttttatcttgccctcagccgaaattcgaagatttccggacagcagcatcatacttgatccaacccgatcaacagtcgccacagatcggcaggccggccggacgacagaaaaaatcccgcccggccgaagccgagcgggtccagtgttcaggcgggtctcaggcggcgcgggcgcggatggcgacgtgccggacgccgtgctccatcgccttctggccgaggttcatcgccgggccgaacggacgatcgcccgagcccctgccctcgcccagggagtgcgccagggtcaggcagcaggtcggctcgagcgcgatcaggtcatcgttcgcccggaagggagccgccttgccatgtgtgtcgaagtccgcccgcgccaggatcagcttcacgcccttctgctgggaccatttgatcgccagcttctcggagcccttcgccccggttgtggcgagcgccatgtccggccattccgccagcgcccagttcagggcgtcgaaaatccgcccggcgtcttcggccgtatcagccgagggcgccccccggaaggcgatcaccggtccgcccggatccgcctcgccggacgtcctagcgcggagactgcggatcgcctgcttcgcctccaactgggccgccgtcaggaagttgccccggcggctgccgcgccaggctgtccagacctcgccggtcgagaccgtccagcagtgggccgccgcgtcgcgcaccagctccgtcgccagggcggcggcgtctcccgcgcgggccttggccgtggcctcctgcagctcgacgtcggccgcctcggagccgtcgaagtcgcggtccagggcgcgcatcgtgtcccgggcccgatcagcatcgcgttcaatccgccccgccgccgaatgaaaggcgccgatgagcgcctcgcccaggatggtctgatagtcttccagagcggtgtcggcgatcacgtcgagcagctcggtcatcagggcgtgccccagctggagcagcgcctcttccgtcgggtgcgggcgaacctcgccgagggcggccgtttggtcgtcgaaggcggaggcggacttgatgaaggaagaagaagtgaagggttgcatcgggaacatccttgaagatgtcgaagcgccccatgcgcaacgaccccggtcttggccacgtcggggtcccgggcagtcaccggagcggaggaccgcttgtcctgcgcggaggggaacggcgaagccgttgacttccggggtgacgtgacaagatcggagggcgttgtgtgggggcatgtcctcgcccccttcgggcgaggactccgttcggcgccgtcgcgccgagaccgcccgaggagacggtcgccgcccgtcccgtcgtcgccggcgccgccggcgacgttcccgttgcggtcgtatccagccggccgtcaggccaatcctgcgagctgcatcagcgcctcggtcgattgtggcctccgctggtaggcgatctccgcgtgcgcggcgcagaagacgccgcgcgcgaccggacggccgcagaggcggaacgtcgatgcgccgggttcgccataggggaagcggcagtcgcaccggcggacgttcaggatggtggcgagcccgaacgacggcgcctctgacgcggcgcggggccgggcggcgatccgcacgggcgccggacggccggaacgccccggcgcgcggcgcggtcctttcggcgcggtaacaggcgaaatcaccggcggggcctgcgaacggccgagggacagtttcattcgatgcaccttgccgagcacggcgctgcgggtgacgtcctcgccgagagtgtcggcgatccgctgggcgctccacccctgagaccagagcgtctcgagtctcgcgatacggtctttggtccagacagacatgatcaggctccctcgcctttcgagccccatcggctcgcccgtccttccccgcctcttcctccccgccctcagcacaagaagggcccggcgcgcgaagcgtccgggccctccccctgtcgcgacctccccaatcagaacgggatgtcgtcgttcagatcgtagccgccgtcgccttccggcgaccggtccgccacgccgccggcggacgcctccgtcgcggcgcggcggttcttcaaccggatgtcgctgacgatcaggcgcagatcgtaatgctcgacgccgtccttgcccgtccaggtgtcgttctcgacatggccctggatcacgacgcggctgccgttgcgcgcgtagggctgcaggtagttctcggtcgtggcctcgttgaagcagatgcagttgaagccggtcgtccgttcgccgggcgtgccgtcggcgcgccggaagcgcgtggtctccagcacgcggaagctcgcgcgcttcttgccgctgccctgggccgacaggatcgagggatcggcggccagatagccttcgagagtcagggtctgcatggttcaatctcctaggaatgaggggttgatggatgtgcggatcaggccgcgacgcggtcttcggtgacctggtcctgccggtcttccgcccagtcgagaacggtcagccggttcaccaccagctccttggcggtacgctccaggccgtcccgtgtggcgtaggcggtgtcgatgaaggcgccgacgaccacggcctcgcagccctgcgccaggccgcgggcgatgaccttctcgttcaggcccttcgaccagctgacgcagttgacgccgaccagccgcggcttgccggcgttgtcggtcccgcgttgctcgagcagccggaaaacggccttgccgaaatcgtcgctgatctggggatcggccgcgaggcggcccgtgaacaccatggtctgcatgtcagtctcctgttgatccgaagcggtccggggagacgatctccccgatcccgcttcatccgggacctccctccctcccgacctcctcccggtcgggcctccgcccgaccgggacccggatcacgcggccgcgccgtcgaggacggactgcacggggtgacgccgcagcaccgcctccaccacatcgggccgatccaccggcacgaagagcctcggggtgtaggcgatgatctcgacgaagcagccgagcgccacgagcgcgtcccggtccatccgtccgcccaccacctccagccgccagcgatccatcacccgggcgcgcttcagccacagtcccccggtcagcgcgagctgcacgttgcggtccaggagcgcggccgccgatcgcgcgccatcggcccaggcgtcgcctagggacgtgaggccgagcgcggccttcagcgacgacgcctggacctcgtccagcacccggccgagccagcgccgaccgtccggcgcgcggacacggcgcacggcgcagcccttggccggcagccgtccccagatcggcaggagaagtccggtcgccagcgtcagccgacgcgtgcgccaaggatccgccgcggccacctcggcgtcccagatcgtgcgccatgtcgcggcgtccgcctcggcccaggcggattcttcgaacgtcttttccggcatgactccccgttggtcgggccgcaccagtcgcacggcgggcacgagacgatcgtcgtcggtcgtcgtggtcaggccgagttccgccaccgccgctcggcccgagcgcgcattgacgacgaaccggcaggcttccgccgtcgcctgagcggacgccgtgtcggctgggagcaggtcgcgcgcgaccttgagctcgaaggtgacgagcgccgtctcggcgccggtggcgacatcggtgcggatggtctcggcgtcgatcacctccagcgcctccgcctctatgtcttccagtccgcgatcgagctcccccgaggccgcagcgcgctccagaatgccggagaggactgcatcgaggtccgcgaacagggcgttctggtcggcgatccgcagggccagaagccggttcaggaaggtgtggatcggcggcaggtcgtccgacggcttcaggccgccgtcggcgtcgcgcaacttcagcccggtcttgccttcgaaggtctccaggtccatcgccgccagctccccgaagccgagcgcgccgtagaacaccagcagcgcccgacgcgcccacggactttccagattgtcctcggcccggaaaaggccggcgccggccgtgcggcgttcaccgcgcgtcagggcgcccagggagtcgagccgtcgggcgatggtggaggtgaagcgtttctcgccatggatgtcggtgaccacgggccggaacaggggcgccgaggcctggtgcgtccggtggctccgccccagcccttggatggcggcgtcggcgcgccagcccggctcgacgagatagtgaacgcgacgctgccggttcggggccgagaggtcggcgtggtagctgcgccccgtgccgccggcctcggagaagacgagcacccgtttgcggcccgacatgaaagcgtccgtctcggcgcgcgcggccgacgcaccgcggcgctcaacgacgcgacggccctcccgtcgcaccacgcggcgcgaccgtccggtgatctccgccacatggtcggtcccgaacgcgtccagcaacgcatccagcacgccggggaccgcgggcaggccggccaatcgggcgatcaggagggcgcggcgctggagcgcctcttggctgacggcaggccgcccatcgaccaggacgggaacaagcgtcacgccgccgtccgcgtcctcgatcgcttccatcagatgaacgggaaaggcctcgcgcagatagtctaggacgtattcgcgcggcgtcaggtcgatcgagaggttgttccactcctccggcggaacggaggccaggcggcgttccatcaccgcctcgttggtcgacacgatctggacgacggcggagcgtccttcggcgaggtccgcccggatggcggcgatcagggtgggcgccttcagcccggccagcagatggccgaagaagcgcagcttcgccccctcgaacgccgaatgaaccgcggaggcggccatcgggcttttgggtttgccgtccgcgtccgccaggccggtcgccttcagggcttcggcgagatgggcgtggatcatctggaacgcgtcggcccaggcgtcccagatggcgacgtcgtcctcggtcagggcatgggcgagcggcgcatattcgacgccctcgaacgacaggctgcgcgccacatagaggccgagcgccttgagctcgcgcgcgaccaactccatggccgcgacgccgcccttgtccatggcgtcgaggaagtcctcgcgggtcgtgaacggcgcctccggtccgccccacaggcctagccgcgaggcgtaggcgaggttctcggccgtcgtcgcgcccgtcgccgaaacgtagaggatgcgggcgttcggaaggcggttctgcagggccaggcccgccatgccttgcaacgacgccttcttcgcgccccgggcgcccttgccgcccccggcggcgttggccatggcgtgagcctcgtcgaaggcgatcaccccgtcgaaatcctcgcccagccaggcgacgatctggtcgaggcgggacatcttggggccgcgcgcgggctgccgcagcgtcgcataggtggtgaagaccacgccccgatcgagccgtacggtctcgccgagcttccagctgttcagcggggtaaggtccgacgcgcccccgccgatggccgcccagtcccgccgggcgtcctccagcagggcgtcgctgcgggacagccagagcgcgcgcgtgcggccctgggccatgttgtcggcgatgacggcggcgatctgacggcccttgccgcagcccgtgccgtcgccgaggaagaagccccggcggagctggacggcgccgggcgcgtcgtcacgggacaggaccagccgatgggccgcctcgcccggcgtccaccaggccggcaacaggccggagtgggcctcgccggcgtagatgacggtttcggtttgggcgtcggagatccgcccttcgtcgcgcagcgcccgcggcaacaccggccggtaggtcggcgcgggcggggccacggaggccatcggcccggactccaccagcggcgacgggtgcggccgagggtccggcaggacgatgcgcgccagcccgtgggcctgatagaggccgatgtcgcgtccctcgcccgtccaggcgcgcgtctcgtagtccacggcggacgcgcccgctaggaaggcgaggcgcgcggacgcgcgcgcgccggcgcggcctccgggtgccagaagcgaagcgggagacgcttcgagccgggcgcgcggccgggcgcccgcgcgccccggcacggcggcggccaggatcgcggcggtcgccaggtcgtccgccacggcgagcggtgcgacctccgcaccggtctcgtcccgctccagcaccagcagaccggtctccaccgacgtgccgtgccgggcgaaagcgcgcggcggaaagagtatccgggcgacgatgcggcccccatccgacagccggcgcaggccgccctcgtccgacagggccgaagccggcgcgaccgccgcgagacgtccgccgtcggcgagcgcgcccagcgccgccttcagatggcggtcaaggtccgtgaacggaggattgcaaaccgcgacgtcgaaccggcccgcggcgtccagcaggtcgtggatgtggcggccgtcgaggcgcgagcgccgcgccgccggaaacaggccgtcgagcagggcggcgcggccgtccgccggctcgttgagccacaggacgccgccgcaggcctccgccacagccgcgatcagacccgtgccggccgagggttccagcacccggtcgccggggcgcacctgggccgcgagcaccgcgatcgccgccagctccggtggtgtggagaactgatccagggcgacctggtcctcgctgcgccggctgtgcgtcaggccgagcgcggagaccgcagccagcagggcggcgatctccgctggcgcgtcctcgaggcgggcgacctggggggctaggcgccggatctgaagcaccgtggcggcctcgatcgcctcgtaggcgtcgcgccagagccatttgctttctgtgtcggcgccgccgaagagggtcgtcatcacctccgagaccagacggcgatccagcgggcgcgatcgcgcgagatggcctgccagcgcccgggcggccgccagcacattggcggcgtggggcgtgtcggtcgcgggaggaaagagggacagggtcgaggtcgaggacatggtcgcggctccgctcgccgggagcggagggcgcatcccccacggtcctccaggctcgccgcgcctagccctcttcttccctttcaacaggaacggcgcgcacaaaacccgccccgccggacggcggagcgggttcttgggcggcaggggtctcaggcggtctgctggagggccgcctcccccgcctcggtgacgacgaaggcgccggcgccgtccgcctcgggcgaggcggccccttcggccgcggcgtccgacgggtcgggcccgtccatcaccgccgcctccggatcgccgtccggcatgtcggtcgtccacgacagactggccggcgcccaggtgcgttcggccgcccgttccgccacccagtcgaccaggtccgtcttcttaagcacgccgacgcggggatcgctcggctctcccatcgcctccagcatgccgagcaggagcgccttggaatgcggcttgaggaagtcggcgtccggcgtccagtgcaaggtgatgtccgcgccgcagagagcagccagttccgccgcctcggcgcgcgcggcccgccggatcaggctggtccgctcttcgcgcagatcgagcgtcagggccgtcagctcggcgagcaggctcatcttgtcgccatgcgcgagcgcgtgaacccaggcgatcaccgtctggtccgacccctcccaagccgcgcgccgttcatcgagccgttggcgaacgtcgccgtccagaggctcgatgatccgtccgccggcgggattgaaggccgtcgcggtcagggcgaaggcggattcggatcgtgcgccggacccgcggaccgcgacctggacgaacaggcgcgcgatcagcgccgtgagcgccgcgcccggatcgtcggccagcgcccggatcaggccgcgtgttgcgacatcggtgcgcaccgcgtgcagggcgtgattgatcccctcagtctcgggctccggcgcctcgacctccggcgcccgatagaatcgcccgttcgccggcgacagatcgccgtcgtcgtcgacctcatcgcgagcgtcgctgagctcctcgttgtcctggatctccggctcgaccggggtgaagcagcggatgtcgaggcccgcccggacggacgggaagaagaccagtgtcgtggcgacgcgaccgccccagctgatctggtccatcgcgaggcgcgccttcgccatcgcgatcagcaggggatcgacgacggccgggtccgtggtttcggcaagccgttccccgaccgcctcggcggcggcgttgaagacctcgcgcgcctcgcgataggcgtccagctcggcggcgggcagcatgccgccataggcgtagcgtgccggttccagatcgtcgggcagctcgagagcgtcgcccgccgacacatggacggcaaggccttccgcctcgaagaccagggcgatctctcgcgcgcgccgcgtccagacgtcggtcaggatcgccgggtcgagaagcaccggcgcgcgctctccgaacagatcgacgacggtgcggccgccggccgccgcatagcgctccgcgccgaccagggcgcagcgcgcgtcgccctctgtgacctggtcttcgtccagcttctcggtgatgcgccagtcctggaagccgtgcccgtcgagcgtcatttgcgcatattcggcctgctcggccttgtccggcagccgggcgagcagccgggcctgccgcagattgagccgaccgcgccgcaaggcttcgagggccacgggtggcagggccgacagggcggcgagccgcttcacgtcgatctcggcgtaccccaaggccttcgcgatcccgggcacggcgagtttgcccttgagcatccggccgatcgcggcgatgacgtcggcgacgtgaaccggggcggcggtgttggtgagcaggacagcggccgcctggcgcgcgggatccgtctccaccaccacgtccacgaggaagccgtcgtcgatgcggccgccttccagcagatagcgcaaggcgaggaggcgacgacggccgtccagggccatgttcgcccgctcctttcgccgtcccgggcgcacggtcagcggctccagctggcccgccgcgaacagggtttccgccagcagcggaatgtcgtcgtccggcggttcgccgaagcgcaggttctcaggggcgatatccacatcgcggaggggaacccgcagccgggcacgggctgcggcgatgtcgaacggcgtctcgacgaccgtgagggcggcggaggcggatctgggcatggcggaactcctgccggcgacggggcctatccccgcctttccggcgccccaccgcgcccttccttttccctttcggcggtcgtgcggatggcgtcgttccaatcgccacagccgggcggcggcagacgcatctccaccgcaaggccgagcgccgcaaggcgatgcttcaaacggcgggcggcggcctcgccggcgagaccgcggtcagcggcgatcacaacgctgcggacatcgggcggcggcgtccaggccgccagattgccggcggagagcagcgcccagccgggcaggtcgaacccgcgcacggccgaaagggtcgtgacgaccccttcggccaccagcatcctgcggccgacgacggacaaacggacggcggcgccgggcggaacacagcccacggtcttgcgtgacaccgccaatcggaccgcctgacgcgccgcagcgtccagataggtcagttccaccccggtcgtgcgcccgtcgggatcgctgatgcgggccatcagagcccgcagggtcggcccgccggtccgatagaccgagaccggcgcggcgggatgttcgagaaggtcgcgaacgccaatggaccaaggaacggcgcgacgctgcagatgacgggcggccaggccggacgggccgatcctcacgccctgcgaccagagccgctcggccgtctgccgacgaacgcgcgtatccggacgtgcgaccgatgcggcgccggacagcggcgcgcccgtcggccggcccgccgcgtccacgaggccgcgacggcgcagatccgccatcacggcgcgccagtccgaccctccgaacgaatgggccacgacgcgcccctccgtcagccacagggacacagagcggtcttcgccggaatggccgggcccaggcacgttggcgcgcgcgccgttgtgatagagatcgccgccgagggcggcgacaatgccgcgcaggctcatgggagcaaccccatctgccgaaagctcgccgtgccctcccgacccaccacgagatggtcgtgcaccgggatgtcgaacacccgcgccgcctcgaccaccttgcgcgtcatggcgatgtcggcctgcgacggctggggatcgccggacgggtggttgtggatgaggataagggcggatgcgccagcctcgagcgcccgccgcaccacttcgcgcggataaaccggagcatgatccaccgtgccatccgccgccgcttcgtcgcagagcaggcggttcttcttgtcgagatacaggacgcggaactgttcccttggccgatgaccgacggacacacgggcgtaggcgacgaggctcgaccatgaggtgatcacaggccggcggctggcggtttcgcgggcgagatgttcggtcagtcccgccaagcgtttgacgcggtctaccgtcttctggtcgagaccgtggcgcttcaactccgcagtgtcggcgtgaacgaaggcgccgactgtgtcgaaccggcgctggagcgcgccgaccagggctccgtcggccgcgaggtcgagatcgatgaggagacggtgaagccaggcgcagccgccgtcggcggtggtgacagcgcgaccggaagtggacagccgccccgggtcgggcggcgcaatgagggcgagagacatgatgagctccgtaccgctccgaagcggagcgcccctccccgcccttcccttccctccggtcctggcccgggggacggtcttgagacctgttcagcggccgcaggagttccgcgacgacttggccgctcccctcagacgcgcgttggcctcgcggcgcatgacccggcgccacattcgttcagacgccttctcggattcaggctcaggccgcgaccggaaagaccttctcggcatcgaggctcccggcgggcaatgcccgcaacaggtcgtcgtgcggtgtctgcagattgagccaggccgcaccgtcttgggggcgcaagactacgatctggcggtcgtgatagggggcgatgtccacccccggctcggtggtcaacatggcgaaggcgccgtccttgatcagacccgccacccagaagagccgctggccggcgagggtgaaacgccacttcgtcttccgcttctggcccggttccgcgtcggtgaactcgaaaaagccatccgccggaatgaggcaccggtgcgatccctggaacgaccggccatcggagcggaagttgaacaccggccgtccccccggccccttccaggcccatggcgtcatgagcacctcgggccccgacgctcccatgtgaatgacaggcgcgcgttccccgatgcggatcgacgccatcggtccgaaattcggcatgcctcctggaaagaccagccggtcgcccgtctggttgaacgccgcgatgatgtcatcaaacggcaggatgagctgatattcgttgcacataggaccttccgggggccgtccggcgcaggatttcacggctccggcctcgccgcaaatcggcggggataagcgcaccaccggattgactcccccccggcgccaaaccagaacgtttcgagaacatttatcgtgacgaagaggagttcgtcgatgccggccgcccgctcggccaaacttgaagatctgcgtgctcaggtccttgccctggagcaggccgaccgaagaccggtcggtgtgttgccattcggcgtggagccggtggatgccgccctgccgggcggggggctgacgctgggcgcgctccacgaggtggccgggggtggtgacgacgccgtcggcggcgcggcggccgcgctgttcgctgccggggtggtcgcccgcctccccggtcccgtgctctggtgcatcacgcgaccggacctgttcgcccccgcgctcagccaggccggactggagccggatcgggtcatctatgtcgaggccggagacgagaaggcgttgatggcctgtttcgaggaaggcttgcgtcatcgcggtctcgccggtgtcgtgtgcgagacgtcccgcctcagcatgaccgcctcgcgccggcttcaactcgccgccgaagcctcgggtgtgatcggtctggcggtccgccgatggcgtcgcgcggccgaggctgcagacttcggtcaaccgaccgcggccgcgacccgctggcgcgtcagcgccgagccgtcggcgcccttgccggttccaggcatcgggcgagcgcgatggcggatcgaactcatgcgctgccgcggcgccgacgcggcggacttcattctggacgcttgcgatgagacgggtcgtctcgctcttcctgccgaactggcccgtcgatcggcttcgccgacggctcggcgcggacgcgccgccgcctgatcggcctctcgtgctcaccggccgggtgggccgcaggcgcgtcgtgaccgcctgcagcgccgccgccgccgccggcggcgcgcgcgtgggcatggcgacgacccaggcgcaggtcctgatccctgatctggacgtgagagacgccgatccgcgcggagacgccgacgcgctggatcgtctcgccgtatgggcgatgcgccgctacgcgcccgtctgccaggctgatccgcctgacgggctggccatcgacatcaccggggccgcgcatctcaagggcggcgaaacggcgcttctgggcgatctgacggcgcgcctcgagcgggtcggcgtccgcgcccgcgcagccgtggctccgacctatggagccgcccatgcggtcgcccgcttccgccgcgacctggacgtcgtcggcgagttcgcgatcgacgcggccctggccccgctcccgctcgaggccttgcgcctcgcggcggaactgcccgccgccctgcgccgaatgggcttcgagcggatcggcgacctcgcccaccggccccgcgcgccgctgcagctacggttcggcgcggaactggggcgacggttggatcaggcctacgggcgggcggccgagcctctgatccctgtcgaggcgccggagacaccacgcgtcgaacaggtcttcgccgaaccgatcggcgcccccgagacgctggcccgctatgcgggcgttcttgccgccgccctgtgcggccttctggaagcgcgcggtcttggcgtccgccgcctcgactggctctgccaccgcgtcgacaaccggatcgaagcggtccgcgtcgggctggccgggccggtacgggatacgcgtcgcctgacgcgcctgttgaccgaccggatcgagaccatcgagcccgggttcggcatcgagcgcatgacgctcgcggccagcgcggccgaaccgctggattggcgtccggccgcaggccgcctcggcgagccggcgatgcccgatgtctccgggctgatcgatacgctctcgaaccggatcggcgccgagcggctctatcgcctggcgcccgtcgagagcgatgttcccgagcggtcgatgcgcaagctcgcgccgttggccgcgcccaccggtaaggcctggtcgccggactggccccgccctgccaggctgttccgccgaccggagccgatcgaaaccctcgcgctcctccccgacaacccgccgacccacttcacctggcgcggggtccggcgccgtattcgccgggccgacggcccggaacggatcttcggcgaatggggccgccgcgatgccgagatgtgggcggtcagggactatttccaggtcgaggacgaggcgggcgagcggttctggctgttccgggccggcgacggcgaagacgccgcaacaggatcccaggcctggttcatccacggccagttcggctaggaccgtcagggttgggcgtcgccgcgcccctccccgcccacggcgccctcgcgctcgacgtcgtgttcgacatcgtcctgggatctctggtcgctctcaccgggtccgacggcgtcaggactctcgacgccgggggaccggtcggcgtccgaattgcgctccacgtcgtcggggcgggaggcaggacgggaacgcgggtctggagcggggctcatgaggattctcctttgtcccgtgaacctcagcgctccgcgcgaggttcctttcgtaaaggatcatcgcgctgcagttcaggatccgacaggacggcgatgacctcgaggtcgaacgcgtcgagcgcctggcgctcctcggcgatccgctgcgcctgaacgaaccgccggctggacagctcgaagccgctgaggtgcgcggcaccgcgcgcgctcaggcgctcgatccgttcgagcgttacgccggcttccgaccgcaccaaggtcttgcgcgtccccataggcctattctgccatgaagcggcgcggcgttgaagatcggcggtcagccacgtcgtcgcgacgagccggcccattcgctgttggccaagcccggtggcgactcggacgcggaccgcgtcgctgcgtggcctgattagctgattatcgtgcgaggaccgcgatcgcggaagcggcggaatgagccgcgcttcgatcgaaggcacgaccgtccgcacagccccggccaccgttcgcggcgcccacgcgttaacgccggatgacgtctcagaccgatctgttcggcgcgccggcgcaggagccggcaggcctccggctcgatccggccctgatcgacgccgacgagcagtctgcactggtcgccgtcttcgccgaactgccgttcgcaccctttgaatttcatggctggcagggcgcccgtcgcgtcgtctcctacggctccctctatgacttcacgcgcgggcgtctcgaggccgccgagcccatcccgccgtttctccatccgctggcggaccgcgccgccggcttcgccggcctcaagcgggacgccctcgcccaggcgctggtcaccgaatatcagccgggcgccggcatcggctggcatcgggaccgaccgcagtacggccagatcatcgggatctccttcggcgcaccggcgcggatacggttccgccgccggaccgcgtcgggttgggagcggcgggcgctcgacctgccatcggggtccgcctatctgctggacgggtcggcgcgttgggactgggagcacagtatcgcccccatggccgcgctgcgatattcggtgaccttccgcaccttgcgcgagacctgagttgacgaacgccgccagaaaaaacaaagcgcgaacatgtctgcgcgatatgtcgagctggaatgcgcttcccatttctccttcctgaggggggcgagctcctgcgaggaactcttcagccaggcggcggtctgcggcgtcgaggccttggcggtcaccgatcgcaacagcgtggcggggatcgtccgccctcacgaggcggccaagggcacgggcgggaggctcatcgtcggctgtcgcttggtcctgaccgacggcgccgagcttctcgtctatccaaccgatcgggcggcctatgcccggctctgccgtgtgctgacgctcggcaagagccgcgccggcaagggcggctgcgatctgtcctgggacgacctcgccctctggagcgaaggcctgatcgccgtcctggcccccgatcgggccgatgctgcgtgcgcgcgtcgtctggatcggctggcccaactctttggccgcgacgccttcgtcgcgctgaccctgcgtcggcggccgcgcgatcagctgcggctgcacgttctctgcgagatggctgcggccgccggcgtccgccccgtggtcaccaacgacgtcctcttccatcatccggatcggcgtatcctgcaggacgtcgtcacctgcatccgcaacggatgcagcatcgacgatgtcggcttccgccgcgagcggtccgccgaccggcatctgaagcgggtcgaagagatgcaccgcctcttcgcccgtcaccccgaagcgctggcgcggactctggagatcgccgaccgctgccgattcaatctggacgaactggcctatcagtatcccgaggaggccacgccgggcgcgaccccgcagcaggagttgacgcggctgacctgggccggcgccgccgagcgctacccggaaggccttccggacgcggtgcgcgcgacgctcgatcacgaactcggactgatcgagagcctcggctatgccccctattttctgacggtcaacgccatcgtccgcttcgctcgcagccggagcatcctctgtcagggccggggctcggccgccaactcggcggtctgttacgtcctcggcatcacctcgatcgaccccggccgtaacgaccttctgttcgagcgcttcgtcagccaggagcgcaaggagccaccggacatcgatgtcgatttcgagcacgaacggcgcgaggaggtcatccagtgggtctatgacacctacggccgcagccgcgccgccctgtgcgcgaccgtcatccgctaccgctcgcgcggggccctgcgggatgtcggtaaggccctgggtttgtccgaggacctgctcaagtccctgtcgtcccaggtctggagctactccagcgagggcgtcgaggaccgacacgtcgaggaactgaacctcaaccttcaggaccgccgtctgcggctcgccctagacctgtcgcgccagctgatcggcttcccgcgccatctcagccagcaccccggcggcttcgtcctgacccaggaccggctcgacgatctcgtccccatcgagcctgcggcgatgaaggatcgccaggtgatcgaatgggacaaggacgacatcgacgccctgaagttcatgaaggtcgatgtcctggcgctcggcatgctcagttgcatgcggcgcggtctggacctgctgtccgaacacaaggggatcgatctggacctggcctccatcccggcggaggatcccaagacctacgccatgatccgcaaggcggacactttgggggtgttccagatcgaaagccgggcgcagatggccatgctgccccgcatcaagccgcgcaccttctacgatctggtcatcgaggtcgccatcgtccggcccggcccgatccagggcgacatggtgcacccctatctgcgccggcgggaaggccgggagccgatcgtctatcccaagcccgaactggaaaaggtgctcggcaaaaccttgggggtgccgctgttccaggaacaggccatgcgcgtcgccatcgaatgcgccgggttcacggcctccgaagccgaccagctccgccgcgccatggccaccttcaagttcaccggcggcgtcagccatttcaagaacaagctcgtctccggcatggtcgagcgcggctacaccgcggagttcgccgaaaagaccttcagccaactggagggcttcgggtcctacggctttcccgagagccacgcggcctccttcgccctgatcgcctacgcctcctcctggctcaaatgccaccatcccgatgtcttctgcgcagcgcttctgaatgcccagccgatgggcttctacgccccggcccagatcgtgcgggacgcatgtgagcacggaatcgatatccggccggtctgcgtcaacgccagccgatgggactgcaccctggagccgaccgaccgggaggaccggttcgccgtccgtctcggcctgcgcatggtgcgcggactggcgaacgccgatgccggtcgtcttctcggtcaccggcagaccggggcgttcacctgtatggaggacgtatggcgacggtcttcgacgccggtcggagccctgacccgcctcgccgaggcggatgcgttcctgccgggtctcggcctgcaacgacgcgaggcgctgtgggccatcaaagcgcttcgcgacgaccctctgccgctcttcgcggtcacccaggaagacggcgcgaccacgtcggaggtctccgaaccgcagtcgatgctccccgccatgccggccggccaggaggtggtcgaggactacagccatgtcgggctcaccctgcgggaccatccgatgaccttcctgcgggacacccttcggtcccgccacgtcatgacgtgcgccgacgcctccgcgatgcgcgatcgacgcctgacgcgcgtcgccggtctggtgctcgtccggcagaagcccggatcggccaagggggtgatgttcatcaccatcgaggacgaaaccggcgtcgccaacctcgtgatctggccgagtctctacgagcagcagcgccagatcgtgctcagcgcaagcctgctgatcgtcgacggcaaggtccagcgcgagggcgaggtggtccatgtcgtggcgaccaggctccatgacggctcggatctgctggcctcggtcggcgatcgcgaggcctttcccctaccccacggccgcggtgacgaggtctatcacggcagcctgccggatccgcgcggatcgcaccgacgccacaaggcccgcgacatttacatccccgatctgtcgctcgacgccatccgggtcaggacatgggatttccgataaagctcaacgaactcgagcacaccgtgatcgagatccgctaaggtctcgcgtttctccctgcgctaccgcccggctgcgtcagcgtgtccgtgtcaacagagccgccagcccgcaatggatcgcaaagccttcgcccgcgccgtcgatcgcctctcgcccacggctgccatcgccgccctagggccggcggatgaggcgctcgacgtcgaggagatggcgggacttctccaacgcgccggtcgcttggtgttccggatggccaatgcggagcgcgaaggggcacggaacgccttcatcgataccctgacggcggcggtcgccgcccgcctcgggacggcggccggggatcggatcgccgccgtcggcgatttgatgcgggagctggaagcgggctaccgagacgtcgcgcacggtctcgcgaccgccgccgtctcggctctgcccctcgaccgccaaatcctcgcggtccttcaccggacggcgctggaggtcgacgacatccggcggcacgtcgacgtcgcgctggcgaaggcggagtcgatcgtccccggtcagccgctgcacgtcatgaccgaggacggcgtcgtctacgaggccaacgccggcctgcagttccacgtctcgaacctcggctcgtgcctgaagctcctcgtcgggcgtctggacgaggatcgcgctcgcggtcccgtcgtccttcccccgctcggggaaacaacggaagacgagcggttcaaggcggggaccagcggcttgctggcgacggccattcgccgctggcgccgcctcgaggaacggcgccggttctggggtggcgaactcatcgtccaccgtccgccagatctccctgctgacgtcgccccgacgttcgaggtcatccgcgagcatcgtcggccggtcgatgacctttgggacatcatcgccaacgaacgccagaaggatgtctttcaacggcagaccgacgacgtggcgctcaaactcgccgactacgattatggcggtctggatcggccgacaggactgggggccgacgagctgttctccctgggagaggccgccgccttgcaggcgctctcggggctgctgttcgccccggctttcgaagcggaccagcagtttcagggcctgacgctgcgggaatgggtccgcggctatgcggttctgcaagcgctcggcgagcgcgcgatcgagagggagacgaccgcctatggtcgcagcctcgcgcctttcccgcccggccagctggacgcgacgctcgtcgccgcagggctgaagacgtcgacggcggcccggttcatcgccttcgcgacgttgtccgatcattcggacgacatcttcgactgcccgctgttgcgcatggccgacggcggcaacctgttgttcacgccggctgtcaccacggccgtcatcgcgcgtgtggtcctctccaacctggcggccctcggagagcgcttcgagaacaagggcgattggttcgaagccgaggtgctggccttcttcaagagccacggcttttccgccttcacgatcaagacgaccctgatcgccggcgagccctatcaactcgacgtcttggtcccttggggcgatcacctcttcgtcttggagtgcaagaacgaagccttgtcaggcggcgatccggtcgcggcttataatttcgagcggggtcggcaagaccatgtcgtccagatccagcggcaggttaacggcctcagggcccacccggagctcgccctgaaggcgggcggccccgacccccgcacatcgacgattattcccgtcgttctctacgccttcccctacgcccgcccgtccgaagaccacgaagttgcgatcgccgactggtccggcgtcacgcgctttttccgcggtccaacgctcggcttcaccacccgccacagggtcggagagggcgaggcgctcctccgccgccacgaaaccacgaggctttggcggggcgataccccgacggtcgatgacttcatcgctcaccttcgggcgcccagccaggtcacgttgaaggctgaggcgctggagatcacgcccggcgatttctacctctgcgaccaccggggcgcacgaaccaccgaggttgtggcgggaaacccgcgatcagcggcgacgccacggtttgaacgagcgctccaggcaagcatcgcgcgggccgagcgggatgcgcgagcgatcacccggcgaaagcttgagcgcgagctgcgtcagaccgcccggcggtcccgcaagctgcgacagggcggcattccgccgtcggcttgataccggacgccgttggctcacacagctgccggtgacgttctgcttagcttagacgccctgatggtaggcgtcggcggggccgcggcggacgcagccgggggggaagcttctgtcgtgtcgacgagcgtccagtgcaatcagatggtcttcgcaatccgaaagtccgaatcccgaaaaccctcgctcatgcggtctcgggcgaagtcgcgaagacccagttgtgacccgtccttgtcttcaagcgggccatcagcttttccaatcgggtgaccacggcttcgtcgaggtaatcgacaagctcgtgccaaggctttgcaccgccaacgtagaatcccagctgtagcgcgaaccgtacggagaagcgggcctgatcgaagtcgatgtgcatggcgttctcgatcgacgggtggtcgtcgttatgagcgaaccgcttgtttcgcagatcgagaatttcgtcgtgagcggatcgaagtttggctggcaagtctgaacgtgagaagccgctggctctgccgccgttgaaaagccgggcgtaggtcacggcgaaggccgtcgtcatcatctcaagttccaggaccgactctaggtcgggcgagaactgatacgcagccagccgatcccggatatgcttcagagtcaccaaggtggcgaacgagttcgatagccgactgagccgggaaagctcggggtctaccgacttgaggacggcccggccgttcgcggcggtggattgaaaatgctctcgccattcctcaggcagaaactgaaacgcctcttccggtacgacgcaaaactcctcgccctcgataatgacttcctcaagctccttcatcgcacgccgctcctgccgattcgcccaatctcggggcagttcgtacctttcgcatagaatcgcacaggggttggggacccgcccagcccggtgatgctcgcgccgcagcccgcccgctctctttcgtgtgcgacggtggctagatcctcatccgcgggaatgaggccttatcagcagttcggtctcgaatggaaaacacgctgcgcagccacgcacagcgatgaagccccgaatcaggcctgtgccccatatgtgccccaaatcggaattgcgaaggggccgccacaaggcagccccctcaaaaccattccaaatcaatgatttagatggtcggagcgacaggattcgaacctgcgaccccttgacccccagtcaagtgcgctaccaggctgcgccacgctccgaaggcgctccctatagaggcgactcagccgggccgcaaacgtaaaaaggcgttgtttcctgctatcgccccagcacggcgcccagccgcgcttttgcagcatcaatgtccgccagcagcgcgtgaagatcatcggcagacgccggcgcgccggtgcgcgctcgggtgacgccgtcggcgtcctccgctgccaggattcgcttcaagccgccggcctgatagagcctttccacgccccggatggtcatgccttcgtcgtgcagcagccgacggatcgccttcaaggtttggatgtcggcaggacgatagaagcgccgcccgcccgcacgtttgacaggcgcgacgaaggcgaacttcgtttcccagaaccgcagcacatgctgaggcgcgccgaccgcctccgccgcttccgagatggtccgaaaggcggcggcgctctttaccgacggcgcagccgccatcaatcgcaggcgccggcgtcgtgcacacgagccttcatgatctgcgaggcgcggaagctaatgacgcggcgggggttgatcgccgccggttcgcccgtcttcgggttgcggcccatgcgggcgcgcttttcgcgcacctggaacacgccaaagccggacagcttgaccagttcgccgcgttccagcgactccacgatcatctcaagggtgcgctcgaccaggctggagcactcgtgccgcgacaggccgacctccatgtggacggcttcgcacaagtcggcccgcgtcagggtcttctgttcggacatccgcttctccaggtcgcggtccccataaggacgccgcagcgattcgaaatcaagaaggccttatagacggattgcgcaagcgccccaggtcaggccgccgcccatggcttccagcagcaccagatcgccccgcttgatccggccgtcgcgaatcgcggcgttcagcgccagggggatggacgcggcagaggtgttggcgtgctcggcgactgtggagatcaccttgtcctcgtccaggcccagccgatcgcccacgcccttgatgatgcgctggttggcctggtggggcacgaaccagtcgacctcaggcacggttacacccgcgacctcgcaggcggcggtgatgccctcggcgatgttcactacagcatggcgaaacacctgattgccggccatgcgcagatggccgactgtcccggtagaggccggcccgccgtccacgtacagcagatcggtcttggagccgtcgcagcgcaaggcgaagccgagcaatccctggtcctgcgccgtgccccgcccctctcgcggctccaccaccacgcagccggcgccgtcgccgaacagcacgcaggtggtgcggtcggtccaatccatcagccgcgtcatctcctcggcgccgatgaccagggcgcatttggacatgccgcgcgccacaaagccgtccgcgacgctcagcgcatagacgaagcccgagcacaccgcctgcacgtcgaaggcgatgccgacccccgtacccagcttgcgctgcacgatggaggcgacggcaggaaaggtcatgtcgggcgtggtggtcgcgacgatgatcaggtcgacatcggcggccgtgcgtcccgcatcctccagcgccttcttcgcggcctcgacggctaagtcgctggtcggctgatcttcgcgcgccttgtgccgctggcggatgccggtgcgttcgacgatccattcgtcggaggtgtccacgatctcggccaggtcggcgttggtgacgatctgctcgggcaagtaggaaccgacgcccgtgatcgcgctgcgaacgacgctcattgaaccgcctcgctggattggggctgcgcccgcgtctgctccaccacgctgccgagccgctgcaggccggctccgaccttggtcatgtagtcgctgcgggcgagatcgacggcgatgcggatcgcattgccgaagcccgccgcgtccgccccgccgtggctcttcaccacaatgccgttgaggcccagaaggggtccaccgttgacgccgctgggatccatgcgacggcgcatcttgcgcagggcgggataggcgatcagcgcgccgatcttggactgcagacccgaagtcagcgcctccttcaacagagccccgacgaagcgcgcggtgccctccgccgtcttcagcgcgatgttgccggtgaagccgtcggtgaccaccacgtccaccgtgcccttggcgatgtcgtcgccctcgacgaagccatgataggcgatcccaaaggcgccttcgcgcaggatccggtgcgcctcgcgcacctcttcatgccccttcatgtcttcggagccgacgttcaacaggccgacggtgggacgttccacgccatgaacagcgctctggaaggcctcgcccatgatggcgaactcgaccagctgctcggcgtcgctgtcgatgttggcgcctacgtccagcacggcggtgaccccgcgaaacgtcggccagctggcgacgatcgccggccgctccagtcccggcgccgacatgcgcaggatcagcttggagatggccatcagggcgccggtgttgccggcggaaacaaccgcgcccgcctcgcccgtcttgacctgctcgatcgcgttccagaggctggagcccttgccgcgacgcatggcctgggctggcttctcgtccatggcgaccaccttgtcggtgtgccgcccctcgcagacctcgcccgaaagccggcagcgcgtcagctcgcgcgcgatcgcctgttcgtcaccgtgcaggacaaagcggacgccctctccgccgtagcgccggatgtagtcgcggacaccggccaccacgacggacggaccgtgatcgccgcccatggcgtcgagcgagattgtgactggcgacggcaaggatacctcaggcaatcgcgccgtttgtcgcagcgcttggaagaaggggcgtgtggaacgaggcggccgtcgcgtcaaccttgaccaggatcgccgcggtcgcggacggtcttcagcaccgcaaatggggacagctcgcccggctcctcaggctgcacgaactcggcgtcgggcttgcgcggaaacgggtccagcgacagcgccagttgctccaccgcatactggcccaggtcgatgcggccgtcctcgatcacgtccggcgcgtcctcgtccatcagcacctcgatctcggaggtttcgtccggcgcggtctccgccaagccgacgctgaagcgttcgttcacgtccacgggcagcggctcaagcgtcagcccacagctttgcaccgcatgcgccgagatgacgccggacagccgccagccgccggtggagggctcgaccgtcacctcggcggtgaaccgatccagcgcctgcaggtccagcgcccgcgcgatccgcgtccgcgccgcctcgtccggctccagccggcgcgtcacgccgacgccgacctgattcatgcgcaggggttcgctgtagggaaggttctgggtcatggatgaatgtccggccacttcggcccgctcttgatcgctttcaagccctgcgtcgacagaccggcgcgcgcatccagcgcgtattgggccaagaaccgggccgcgtccgcgttttcggtctcgtagacgtttcgcgccagcgcgccggccaagaccgtggcgtccccggcgcggagcggcccctcataggccttcatgcgcccgtagagagcctcgccgagcttgcgcatcttcttgccgacggagacgtcgccgaccccgagctctctcagcgcgtgatcgagagccgagacataggcgtcgaacagggcctgcgccgcctcctcgccctcgcccgccccttcgtcacgcagccgcagcaccagcagcagcacatgcagggtgtacaactcgaagcgcgaatcaatccggtcagcgacgcccagagcgatgtagaagcctggttggcgcgcctgcgtcaccgcaagcgcatacagcgcgtcgcccgtgcggtccctggctttggagcgcagaagtctggtcagcatggcacgcgccccttttccgccgcgccgttgaactaggacgcgggtccgtctaggtcaaagaccttatcctgttgcaggcgttcgatcatgtcccgtctcaaagcccttgccgtcgcctccgccttggctggcctgtccgccgcctgcgctccgaccatcggcagcaacggctttcaggccatcgacaagaagccggcggatattgtggcgggcacggacaccaaggagacggtgctggcccaactcggctcgccctccacgacctcgacctttgagccggatcaggtctggtactacatcagccagacgaccgagcgttacacctacaaccgtccgaccatctcccgccgcacggtgaccgagatcaccttcaacgaggcggacggcaaggtcgcggcggtgcgcacccttggtctggaagacggccaggagatcgcgatgaacggtcgcgagacgcccacgcgcggacgctccctgtcggtgctcgaacagctgttgggcaacgtcggtcgcggccagctgccgcgcacggacgaggatgtgccgggccagcgccggcgcgactaacggcgatctaggccgtcggcatgcccgtgcgacggcgcgggttctgggcgagcacttccacacgcgtgaccgagcctcgccccgcgatggcggcggaggcggcgatcaggctggcggacagcgcccgttcgttcaggcgcgtccagtcgccgggcacgctgaacggcgcgcggtgcgccgccttgaccagggcgtcccgcaggaaaggctccttgctcttcatctgctcaggcgtcttgccggcccccagatgcacgcgcagcgacacgaagacatagttcctcagccgcccgtcctcgatcaccggcagacccaggcccgcgatgctcatcgccgcatccggcgcgccgcctgacgaagaggcctggctggttgaagcgacgccggttgcaagagccgcagttccggcggcgatcaggtgtctgcggtccatggcgggaccgtagggccgcgctgttgagattccgtttctagcggtggcgccatccgggcgacgcgatcgcgacgggggcgtgcttgtgccgaacctcgacgccggaccccgcctcgacgcgtccgatccgcgtcaagcgaacgagctgcgcctcggcgagccgcctcagcgtttcctcgtgccgtgcgggtgcggtgaacacgatctcgtagtcgtcacctcccgtcgccaggtcgctcagggcggccacctcgtctacgcgctctcccagccaagcctgcgccgcagccgatgtcggcaggacctccagatcgagtcgtattccgacctcgctggccttggcgatatgcgtcacgtccgcgatcaatccatccgacacgtctgccgaggcgctggcgaagtcccgcacgacgccggacgcgtcaagccgagggaccggcatgcgatagtggctgatcagcgcgtcgatccgcgccggatccagcttcaactggttgcgcgccgccttcagacccagccagccgtcgccgatggcgcccgtgacgaacacgaggtcgcccggctgcgcgccggatcgggatacggttcgcccgctcggcgtccagcccagcgccgtcagagacagggacagcggcccgggcgtgccgacagtgtcgccgcccagcagatgcatgccgaaccgcgcctgatcctcggcgaggccgcgcacgaacagctcccgctccggccagccgcagcgcgggctccagtggcaggccagcagatagccgaacggctccgcacccttggcggccaggtccgacaggttcacccgcagcagcttcttggccacggtgtccagcggatcgtccggcaggaagtggacgccctcgaccatggcgtccttcgtcaggacgaggtcatgcccgagccgcgacggcagcaccgccacgtcgtccttcagcccccttccccactccggatgggccagcggcgccagcagcgtctcgatggtctcgaactcgccggcgacgtccagcgcgggcatcaggcgcgggtgtcgcttgccgcccgatcccgggcgaccccgtccagcgccgcattgacgaaccgcgcctccgcgtcgtcgaagaaggccttggccagttcgacatattcgtcgatcaccacctcgcgcggggtgtccggatgcttcaacagctcccaggcgccgcagcgcagcagcgcgcgcaaggtcgcatccacacgctccagccgccagttggacgccagccgcgtggtgatggccgcgtcgatctcgcgctggctttcgatcacgccgcgcaccacctcggcgaaataggcctcgtcggcctcggccagaggcgcgccctcgatgtcggcgtcgaaacggaaattggagaactcggtgatcaccgtctccacgccctcgcccgcgagctccatctgatagagcgcctgcacggccgcgaggcgcgacaccgtgcgcgcacgccgctggcggctgctcagctgcggctcggcgcgctgcttttcggcctcggcgagttgttgaaggacggactggatgctgttgggttcgctcatgcgccgacgcctaggcgaagtcgcttacgcaatgcaatcagatcaagacaggcgcgggccgcgccgccccccttgtcgccctcggacgggcgcgcgcgagcccaggcctggtcctcgtcctcggtggtcaggatgccgttgcctatcgccagtcccttgaccccgaggttgcgcaagcccgccgccgactgatccgacacgatctcgaaatggtaggtctctcctcggatcacgcagcccaaggcgacaaagccatcatagcgcggcgcggtcggatagcgtccggcctcgtccgccatggcgatggcggtgggaacttccagcgcgcccggcacggtcacgacgtcgaagtcggccccgccctcggtcaacgcgtccttggcgccgctcagcagcgcatcagccagctcgtcatagtagcgcgcctcgacaatcagcacgcggggtcgggtggtcacgtcttggtctctccgtccatgccgcgccagccgacgatgcgcaggccatagccttccagcgcggtcggctcgggacgcgtcgagctcatcacgatcatgtcgcgcacgccgagatccagcaggatctgcgcgcctacgccatagttcctcaaggttcggtcatcggccccgaccggcttgtcgccgcctgcaaggcgctcggccaggccttgaagggccggatcgcgcaggaacaccaccacgcccgccccgtcgtgatcggtgatctggcgtagggccttgggcacatagtcctgccggcgttcgaagtgacccagcaggtctgcggcgaggtcgatctggtgcatccgcaccagcgtgggtctggatggatcgatcttgccgtgcaccagggccacgtgctcggcgccctcgatggtgttccgatacagcatcagccggaacgggccgccgtggacgctctcgaatggcgtgtccatcacccgttcgacgaagcgctcggtgcggcggcgataggcgatcaggtcggcgatggtgccgatcttgatgccatgaagctgcgagaaggcgacgaggtccggcaggcgcgccatggtcccgtcgtcgttcatgacttcgcagatgacgcccgccggcgtcaggccggccatgcggctgatgtccaccgccgcctcggtgtggccggtgcggaccagcaccccgccgtcgcgggccaccagcggaaagacatggccgggcgagacgatgtcgtccgcgcccttgttgggatcgacggccgcctggaccgtgcgggcgcgatcggcggcgctgatgccggtggtcacgccttcacgcgcctcgatggagacggtgaaggcggtgcccatgctggtgcggttctcggccgccatgggcggaaggcgcagctggcgcgcccgctccgtcgtgatggccaggcagatcaggccgcgggcgtgccgcgccatgaagttgatctggtccggcgtcgcgaactgggccggaataatgacgtcgccttcgttctcgcgatcctcggcgtccaccaggatgtagggacggccgttgcgggcgtcctccaagatgtcctcgatcgggctgatcgggctgtcgttcatgttcgcggccgccgtttgcatcatgcggtctcctgccaccgcgcgagatatcgcgccagcatgtcgatctccaggttcaccgcatccccgggctgaagccgccccagggtcgtgacctcccaggtgtgcggaatgatgttcagcgagaagacgcgcccctccaccgcgttcaccgtcagcgacacgccatccacggtgatcgatcccttgggggcgatgaaacggtgcagcggctccggcgcctcgacctcgatccggtgcgagccgccctccggcgtgatcgacaagacgcgacccaggccgtcgacgtggcccgaaacgacgtgaccgcccatctcgtcgcccaggcgcgccgcgcgctccaggttcacgccgtcgccggccttccaggcccccagcgtcgtcttggacagggtctcgcccgacacctcgaccgcgaaccagccctcgccggtttgcaccaccgtcaggcagcagcccgcatggctgatcgatgcgcccaggtcgatgcccgaagcatcccaggcggtttcgatctcatagcgccggtcgcgctcggtctcgtggacgctgcgaacgcgtccgatgtcggtgacgatgccggtgaacatgcctactgccgtttctcgtagcgttcccacaggtcgtcaccgagaggctcgaccgcaagacgccgaaaggccggggcgtccgaaagcttcgtgagcgacaatccggccacgcagggccgtccctccgcccccagcaggacgggtgcgcggaaccactcgatccgatcgaccgcgcccgcccgcaggaatgacgccgccacctgtccgccgccctcgatcagcagggactgaacaccgcacccggtcagcacgtccagcacggcggcgacagtggggcgtccgccctccgcccccacccggtgcacttcggcggcgcccaccgcaaccggttcggccgcggtcaggatcagcgtgttcgcgcccgcgaccttgctgtccgcaggcgtgcgcagccggctgtccagcaccacacgcagcggctggtccaccgtgcgccccggcagacgcgccgtcagctccggatcatcggccagcaccgtctccaccccgacaaggatggcgtcatgcgacgcgcgcagccggtggccttgcagacgtgcctcttcgcccgtgatccagcggctctcgcccgacgccgtggcgatgcgcccgtccagagacgtcgcaagcttcagggtgacggcggggcgcatcagccgcggccgtggcccggctcgtccagcccctcgtcgcccaggaacttggcgaaatcgcccgtgtggcggaagtccttgtagacggaggcgtagcggacgtaggccacctcatcgacggacttcagcgccttcatgatgaagtcgccgacggtagatgacgggatttccgtttcgcccaggctctccagctggcgcacgatgcggctgaccagctgctcgacctgctcgggctgcaccggccgcttgcgcaaggcgataccgagcgagcgctccagcttgtcgcggtcgaacggcgtgcggcggccgttccgtttcaggatcaccagctcgcgcagctgcacccgctcaaaggtggtgaagcgcccgctgcattgcgggcaggaccgcctgcgccggatggccgagccgtcgtcagacggccggctgtccttcacctgggtgtcctgattgccgcagaaggggcacttcatcggcgggtcaggcgtagatggggaagcgctgcgtcagctcgcgcacctgcgccgccacgcccgccaccacggccggatcggcctcgtcgccgccgttcatgctggtgaccacatcggcgatccagcccccgatctgctggaactcggccacgccgaaaccgcgcgtggtgccggccggcgtccccagccgcacgcccgaggtgacggtgaagggcgcggtgtcgaacggcacgccgttcttgttgcaggtcatcagcgccttttcgagctggtgttcggtcgccttgccggtcacgcccttgggccgcaggtcgaccagcatcaggtggctgtcggtgccgcccgagacgatcttcaggccccgttcctccagcaccgccgccagggcgcgggcgttgtccaccacctggcgcgcataggccttgaactcgggcttcagcgcctcgccgaacgccacggccttgccggcgatgacatgctccagcggaccgccctgaaggcccgggaacaccgccgagttgatcttcttgcccagttccagatcgttggacaggatcatgccgccgcgcggaccgcgcagcgtcttgtgcgtcgtcgtcgtcaccacatgggcgtgcggcagcgggtcgggatagacgccgccggccaccagtcccgcatagtgcgccatgtccacgaacaggtatgcgcctacgctatcggcgatctcgcggaagcgcttgaagtcgatggcgcgactataggcggacgcgccggccaggatcagcttgggctgttccttctgcgccatctcggccacgtgatcatagtcgatcaggttggtgtcttccgtcaccttgtaggtgacgggccggaaccacttgccggattggtttgcgggcgagccgtgggtcaggtgcccgccgcaggccaggtccatgccaaggaaagtgtcgccgggctgcagcagcgagaagaacaccgcctgattggcctgggcgcccgagtgcggctggacgttggcgaaggcgcagccgaacagctgcttggccctctcgcgcgccaggtcctccaccacatcggcgaactcgcacccgccgtagtagcgccgacccggatagccttcggcgtatttgttggtcaggacggacccttgcgcctccagcaccgccttcgagacgatgttctccgacgcgatcagctcgatctgctcctgctgacgcccgagctcgccctggatgcccttgaagatgtccggatcggcgtcggcgagcggcttcgaaaagaaggcgtcgtgggtgaaggcggtcacgctggcgtcgtccttgcttgggcgaataggtatggcggcttctctacgcctcggcctgcatcaccacaacatctggtggtcagctcgcgcccagcgcccgcttcagcttggcgatcgccacccgctccaccgccttgggttcgttcaccggccccatggcgctgacttcccggcctgacgccacatggacggccgagcatttcacataggcgccgttgcgggtgaactcgacgatcacctcgccgagcgccggatcgctcacgccgcgacggggcggcgcgcgacgttgcagtgcgcgaacagccggtccatcgcggtcaccagacgatccatcatctcgtcggtgtggttcggcgagggcgtgaagcgcagacgctccgtccccttggggacggtcggatagttgatcggctgaacatagacgccatagtcgtccagcagcatgtccgagatcatcttgcagtgcacgggatcgcccacgtgcacgggaacgatgtggctttcgctgtccatcaccggaatgccggcggcggcgaagcgcgacttcagcgtggccgcgcgctcctgatgcgcctgccgcagttcagggtgggtcttcaggtgacgcaccgacgccagcgccccggccgtcaaggccggcggcagactggtggtgaagatgaagcccgaggcccagctgcgcaccgcgtccacgatcatcgcatcggccgcaatgtatccgcccatcacgccgatggccttgcccagggtgcattcgatgatgtcgatctggtccagcacgccgtcacgctcggccacgcccgcgccagtctcgccgtacaggccgaccgcatggacctcgtccagataggtcagggcgccgtacttgcgggccagagcgatggtgcccttcaggtccgcgatgtcgccgtccatggaatagacgctctcaaacgcgatcagcttgggagcgtccgccggcgcatccgccagcagggcctccagatgctgaagatcgttgtgcttgaagatgtgccgctcgccgccgccatgacgaatgccggcgatcatggaggcgtgattcagcgaatcggaaaaagtgatcagccccggcaggatgcgctgaagcgtcgatagcgtcgcctcgttgccgacatagcccgaggtgaacagaagcgcggcttccttgccgtgccaggacgccagctccgcttccaggtccacggccgaacgagtcgtgcccgaaatattgcgcgtgccgccggcgccggcgcctacctcatcgaccgcttcgtgcatggcggcgagcacgtccggatgctggcccatgccgagatagtcgttggagcaccagatcacgacctcctgctcggacccgtcctcccggcggcgcagcgcaagggggaattggccccgaacgcgcttcagatcggcgaagacacgatagcggccttccttgcggacctgctccaccgaagtctgaaaggcggccttatagtcaaacaagacagaagttctttcgcttatgcggctttggcgcatatctgcgccgacgcaggaaagatgtctattgatccggacggacaaaacgccccaacctcttaattgataacggttctcagcagctgagccgtcgttgcgatgctgcccttgctctagccgcagccggccctccggtccttgatctggatcagaaggcttccctgctccagcgccggcgatgttcgttgcgccggagagatttgcacgaagccgttcggcggcgtagggcgctcgcctctgatcggagtgcgtcatggttccctatcaacccgcccccttccccctggcccggccgcgccgcctgcggacgtcgccctgggtccgccggctggtggcggagaccgtactcaccccgtccgacctgatctggccgatcatcgttcacgacggcccggaggaccgcgtcgccgtaccgtcgatgccgggcgtcttccgcctgtcgcccaaggccgcggcgcaggccgcggtggaggcgcgtgatctgggcattccgatgctggcgctgttcccgaacgtggacgcctcgatcaaggacggggttggaagcggcgcgaccgatcccgacggcctgatccccgactgcatcaaggccatcaaggatgcggcgcccgagatcggcgtcatgtgcgacgtcgcgctcgactgctacaccgaccatgggcacgacggcgtgctggaggggcagcgcgtggccaacgacgcgacgttggagcgcctggccgagcaggccttcatccaggcccacgccggcgcggaagtggtcgcgccttccgacatgatggacggccgcgttcaggcgatccgcgaggcgctggaggccaatggtttccaggacacgctgatcctgtcctacgccgccaagttcgcctcggccttctacggcccctatcgggatgcggtcggctccgcgcggatgctgaccggcgacaagaagacctatcagatggactacgccaactccgacgaggcgctgaaggaggtggccatggacctgtcggagggcgccgacgcggtgatggtcaagcccggaatgccttatctcgatatcgttcggcgcgtgtccgagaccttcaaggttccgaccttcgcctatcaggtctcgggcgagtacgcgatgatgcaggcgtcgatcgccaacggctggctgaacgaggatcgggcgatcctggagacactgcacgccttcaagcgcgcgggagcggcgggcgtgctcagctatttcgcgccgcaggctgcgcgactgctgggcgcctgatggcgcccctgaagatccggccgctgaacgacgccgattggcgcgacctgtggccgatcatcgaagctgtgacgcgagagggcgagacctacacctatccgcttgatctgaccgaggcagcggcccgtgctctgtggacgccgccgcctcccggcgggacgctggtggcgcttgctgacgggcgcgtcgtcggggccgccaagatcataccgaaccaacagggtcgcggctcgcacgtggcgaacggcagcttcatggtcgaggcgcaggcgcgaggacgcggcgtggcgcgcgcgctgggcgaggcggccctggacttcgcccgcgccgcaggcttccggtccatgcagttcaacgccgttgttgaaagcaacgccaatgccgtcgccctgtggcgcaagcttgggttcgagatcatcggcacggttccggaggccttcgatcatccgttgcacggccttgtcggcctgcacgtcatgtaccggccgctttagcgagctcgtctggcgttcgcagtcgcaccgcaaggcttgacgtgtcccagcggtttccgcccagagcctgcacctcggcgtagaactgatccaccagcgcggtctgcgccagtcgcgcaccgttcgcgcgcgcctcgtccagcaccaggccgaggtccttgcgcatccagtcgacggcgaagccgaagtcgaactcgcccttggcggccgtcttccagcggttgtccatctgccaactttgcgccgcacccttggagacggcctcataaaccgcgtcggtgtccagacccgcgacctgggcgaagtgaaccgcttcggccagaccctgcaccacgccggcgatggcgatctggttgaccatcttggtgagttggcccgagcccgaggggcccatgtgctggatcgccttggaataggcccgcagcgccggctcggcgcgcgcaagcgcgtctgcgtcgccgccgaccatgacgctgagctgaccgttttcggcgcccgcctgaccgccagagaccggcgcgtccagaaaggtccgacctaccgccgtcgcggcctcgcttatctcgcgtgcgaccttggccgaggtggtggtgtgatccacgatcaccgcgcccggcgccagccgctccagcgcctgccctgtcacctggcggacgtcgtcgtcgttcccgacgcacaggatgaacagctccgcgccgtccgccgcctcggccacggtctcggccgcccgtccgccggtcgcctgcgcccaggcctgggccttggcgcggctgcggttgaagcccgtgacctcatggccggccccggccagatgccgcgccatcggcgcacccatgactcccaggcccgcgaaaccgatcttcatcgtcgaaactccgttcttcaggcctcggcgacgcggccgtagcgcccccggaagtaggtcagggcctcgccgtccgagccgctgaagcgctcgacccgaccgacaaggatcatgtggtcgcccatctggatgcgatcgtgagccgcgcaatcgaagcgggccaaggcctcaggcagaccgggcggcccctctcccacccgcgtgaactcgccctcggacagggtgcagacgcccttggcgaatcgcgaagcgagctctcggtcgctggccggcagcacgtgaatggcgaaccgttccgcggcggcgaaaaccggccagcggtcggacctttcgtcgatgcaccagagcaccaggcgtgggttcagcgacacggaggtgaaggagttgaccgtgattcccatcggcccgtccgccgtgtcggcggtgaccacgcacaccccggttgcaaaggcccccagcgcgcggcgataggccgacgcctcctccacctcggcgtgcgacaggtcttcggggatcggctcgatgctcacggctccgacctatgcggcgcgggcgcacagggcaaggcgagcctttcggaaacgcgcccttaaccctgatccggcatccaggaggcgagaatcctcgggggcgaacgtccatggctgtcagcgatcgtccgatcctgatcaagaaggtcaagaaggtcggtggtcacggccaccacggcggcgcctggaaggtcgcctacgccgacttcgtgaccgccatgatggccttcttcctattgatgtggctgatcaacaccacggacccagagcagaagcgcggcattgccgaatatttcgcaccggccagcgtgtcggaaacgacctccgggtcgggcggcatcctgggcggcacggcgctgggcgaagacggtgtcaagagcgcgggctccatgtcggtgctggagcaactggcgccggaagcgccgccggacgcccaggcgccgggcgccagcgatctcagctcggcgagcgacgctgcgctgcaaaaggaagtcgaaaagcgcgaggcggccgagttcgcctccgccgccgaatcgctgcgccaggccatgcagtcgatgcctgagctcgccgagttgtcgaagcagctgatcgtcgatcagacgccggagggccttcggatacagctggtcgatcaggaaggccgctcgatgttcgacaccaactcggcccggccgaacgcgcgcgcccaggtgctgctgcgcgccgtgtccaaggtcgtcaaccagctgccgaaccgcatctccatcaccggccacaccagcgccgtcgccggctctggccgcgccagcgccccggccgactggagcctgtcgtccgagcgcgccaacgcctcgcgtctggtgcttcaaggcgccggcgtcgatcccgaccgcgtctattcggtcgcgggcaaggcgggatcggatccgctctatcccgacgatccttcgctggccggcaaccggcgcatcgccattgtgctgttgcgagaggcgccggtcctgcccatggacaccagcctgtaggatgccccgcccgcgagaacaggcttgcgggcgaaagggtgatggagcgacagtgcggtcgtgacgcagcacgttcccacacggcagcttcggttcttcatgaccgcgacggcgccctgcccctatctgccgggcaagaccgagcggaaggtattcgccaacctgccgttctccgacggggcgcacgtcaacgacgagctgacggcctccggttttcgtcgcagtcagaacatcgcctatcgccccgcgtgcgaagcctgcgacgcctgcgtttcggtgcgtctgccggtggagcggttcgccttttcgcggtctcagcgcaagatcctgaaccgcaacgacgacctgtcccgctgcctggtcgaggccgaggcgaccgtggagcagttccagctgctgcgccgctatctgaccacgcgccatccgaccggcggtatgagcgagatgggctggctcgactacgtcgccatggtcgaggacacggccgtgcgcacccacctgatcgaatatcgcgcgccgtccgaggacagcggcccaggccggttgctggccgtcgccctgaccgaccacctgcgcgacggcctgtccatggtctacagcttctacgacccgaccgagacgcgacgcagcctcggccggttcgccatcctggatcacgtccgtcaggccgggatcgtcggcctcccgttcgtctatctcggctattgggtcaggggctcgcgcaagatggactacaaggccgagttccgccctgcggaggtcctccgcttcaacggctgggagccgctggagtagctgaccgaacggctaccggaactttctcaagcctctcggaccctgccggcctgcgcctgcgcgtttgcccagccagtccttccagtccggccattgacggcgacgcccgccgccatcgacccattccggaccctgttcggcgctgaacatcgtcacgtcggccagaccgccctgcttgaagccctgcagcttcacgcccttgccgcgccccatctccggcagttcggccagagggaagatcagcgtcttgatgttgtcgccgatggtggcgacgtggtcgcccgtgacacgcagcatggccagcagctcgccgttcagcacctgcttgccgccgcgcttttgcgccagcagatcgtcctcgggcgcgatgaagccgtagccggccttggacgccatcagcagcttgcctcccgtttggtgcgccaacacgttgatgatctccgccttctcctccagctcgatcatcagccgcaacggctcgccgtgcccgcggcccgacgccagccggtcggcgcccacggtgaacacccggccgtccgaggcggcgatcagcagcttgtcggtggtgaagccgggcaccaaaaaggccagcttgtccccctccttgaacttcagctccgacggatcctccacccgccccttggccgcacggatccagccacggtccgacaggatcaccgtgatcgcctcgcgcgggatgaaggcctcgggtgccacaaaggcggaggtgtccacagcttcggcgatggtggtgcggcgcggcgagatcagcgccttgcgcaccgtctccagctccttggagatggccttccactgcttgccctcggaagaagtcagggcctgcaggcgcgccagctcctccgacagctcggagaactccttttcgatcgtcatctcctccagccgcgccagttggcgcaggcgggtgtcgaggatgaagtcggcctggacctccgtcaggccgaagcgggcgatcagcaccgccttgggctgctcctcctcgcgaacgatgcggatcacctcgtccaggttcaggaagacgatgcgcaggccttccagcaggtgcaggcgcttctcgacccgctcgatgcgccagcggctgcggcggttcagcacctcgcgccggtgatcgaggaaggccctgaggcagtccttcagccccatcacgcgcggcgtgccggtggcgtccagcacgttcatgttgatggggaagcggatctccaggtccgacagcttgaacaggctctccatcagcacctcgggcgtgatggtgcggctcttgggctccaggatcaggcggatgtcctcggccgactcgtcgcgcacgtcggccagcaaaggggccttcttctgctcgatcaggtcggccagagcttcgatcagcttggacttctgcacctggtagggcatctcggtgacgacgatgcgccacaccccgcggcccaggtcctccgtctcccagcgcgcgcgcagacgccccccgccgcggccggtctcataagcgtccaggatcgcggtgtgcccttcgaccgcgacgccgccggtcgggaagtccggacccggcacgatctcggccagctcggccgtggtggcggacgggttggtcagcagcaactggcacgcctcgatcaactcgccggcgttgtgcggcgggatggacgtcgccatccccaccgcgatgcccgacgagccgttggccaggaggttggggaagccggctggcaggacgaccggctcctcgtcctggtcgtcataggtcgctttgaagtcgacggcgtcctgatcgatcccttcgagcagcagttgcgcggccggcgtcagcttgcattcggtgtagcgcatggccgcggccgaatcgccgtcgatgttgccgaagttcccctgcccgtcgaccagcggatagcgctgggcgaaatcctgggccaggcgcaccagggcctcatagatcgaggcgtcgccatgcggatggtatccgcccatcacctcgccgaccaccttggcgcatttacgggcggccgactgcggattcagccgcatctggtgcatggcgtagaggatgcggcggtgcaccggcttgaagccgtcgcgcacgtccggcagcgcccggttggtgatggtcgacagcgcataggccagatagcggcggctcagcgcctgctccatcggctcgtcgatgatgcggccgccttccggcggcggggtgtggatcgtcataggcctgcgaatcgcggattgaacccgcgaagtctagtccgatcccgcgcccttctccgcctcgaacagggcgcgcagcaccggcggcaacaggcccggcagatcctctgcgatcaggccgggtccaaaggcgttcgccgcctccgaatgcatccagacggcggcggaggccgcctcgaagctgtccatccgctgagcgaccaggccgccgatcatgcccgacagcacgtcgcccgtgccggccgtcgccagccaggcggagccgttgcggttgacgcgcgctcgcccgtcgggtgcggcgacgatggtctccggccctttcagcaccaccacggcctgcgcgcgccgggccgccgccagcgccgccgcctctcgcccctgagccagcagtccgggaaacagccgctcgaactcgccctcgtgcggcgtcagcacgtcgtcgcgatccaggccggcgaacagttcgtcggcgcgtcccctgaaagcggacaggccgtcggcgtcgacgatcagcgcggccccgctctggctcagcgcgtggatggcggcgatcgtgtcttcgcccgcgcccgcgcccggcccgactacaatggcgtccagtcccgccgcctcccggcccagcgtctcgggcgagccgaacggggtcagcagcgcgccctccagcaccggcgccagcaccgccgccgcctcggacgggcacagcacctgaacccagcccgcgccgatccgcatgccggcgcgtgtcgccagccgcgccgcgcccgtctgatgcgcccggccggagacgacgcccagccgtccgcgcgaatgcttgtgcgtccggggcccgggccagggaagaagccctcgccagaggtcgggggtgttcggctggatcatccgcgttccaattaagcgcggccgtgcgcgaaaagcgcttgccatgacgcccgcagccatgtcccattcgcccccgagcgtcgagccgttttgcgcgccgctgccgggatcgccatgaaaaagatcgaagccatcatcaagccgttcaagctggatgacgtgaaggaagcgctccaggacgtgggcgtgcagggtatgaccgtgctggaggccaagggatatggccgccagaagggccattccgaactctatcgcggggccgaatacgtcatcgacttcctgcccaagatcaagatcgaggtcgtcgtggccgacgatctggcgcccgccgtagtcgaggccatccaaacctcggcccggaccggcaagatcggcgacggcaagatcttcgtctcggacgtggccgaggtgatccgcatccgtacaggcgaaaccggcgcccaggccgtctaggccagccccataggccggcgggtcttcgggtccggcggtcgtcctcctccccaaacgaccaagaaacaggatttccgagaatgagcgccgcagacaagatcttgaaggagatcaaggacaaggacgtgaagtacgtcgacgtccgtttcactgacacgcgcggcaagctgcagcacgtcaccttcgacatcgacctggtggacgacgacttcctgaacgaaggcacgatgttcgacggctcttccatcgccggctggaaggcgatcaacgagtccgacatgctgctgaagccggacctgaccacggcctacatcgaccccttctatcagcagaccaccctgttcctgttctgcgacgtgatgaacccggacacgggcgagccctacaaccgcgacagccgctcgatggccaagaaggcgctggcctatgtgcagtcttcgggcgtaggcgatgcggtctatttcggccctgaagccgagttcttcatcttcgacgacgtgcgctggtccacgcagccgcacaacacctcctacagctacgactcgaccgagctgccggcgaacacgggcgccgagtacaccgagggcaacatgggccaccgccccggagccaagggcggctatttcccggtcaatcctgtcgattcgggtcaagacctgcgcggcgagatgctgggcgtgatgaaggacctcggcctcgatccggaaaagcaccaccacgaggtggcgccggcgcagcacgagttgggtctgaagttctcggacctgctgaccatggccgaccggctgcagctctataagtacgtgatccacaacgtggccgccgcctacggcaagaccgccaccttcatggccaagccgatgttcgcagacaacggctcgggcatgcacgtgcaccagtcgatctggcgcgacggcaagccgctgttcgcgggcgaccagtacgcgggcctgtctcaggaatgcctgtggtacatcggcggcatcatcaagcacgctaaggccatcaacgccttcgccaactcgaccaccaacagctacaagcgcctggtgccaggctatgaggcgccggtgaagctggcctattcggcccgcaaccggtcggcctcgatccgcatcccgcacgtgtcgagccccaaggccaagcgcctggaggcccgcttccccgatccgatgggcaacccctatctgacgttcgtggccctgctgatggcgggcctggacggcatcgagaaccgcatcgatccgggcgcgccggccgacaagaacctctacgacctgccgccggaagagcgcggctcgatccccgaggtctgcggcagcctgcgcgaggcgctggagaacctcgacaaggaccgcgccttcctcaagaagggcggcgtcatggatgacgacttcatcgacagctacatcgagctgaagatggaagaggtgatgcgcctacaactgcatccgcacccggtcgagttcgacatgtactacagctgctgatcccgcgatcggcagggtgatcaaggcgccgggcggaaacgttcggcgcctttttctatgcggcggcgcctgtctcggcggccgggatgaagccgcgatccagcaggccgtgcagggcgtcgacatggccgtcgcgcgtttcctgcggttcgggatccgaggtcatgaccaccgtcaatcgaaggtccggcaccacgaacaccatctgcccgccgtagccccaggcgaagcgcacgtcgtgtcggcccgaccgcttcagccaccagccgtagccgtaaggattgccgctccacctggacgtgccccgcccgttccaggaagcctcgacccagttctcgggcagcacgcgccggccctcatgcaccccgtcgttgcgataaagctctccaaacttcagcaacgcgcgcggcgacaggcgcatgtcgttgccgccgaagtagacgccctgtgggtcggccggccaactcgggaccgatatgtccagcggctcgcccagccactcgcgcatgttggccagcgtggatcggccgctcgcccgcgtcagggccgccgacagcaggtgcgacgtgcccgtggaatagatcatccgcccgcccggctcggcttcgaacggccgcgccagggcgtatctcacccaatcccggctggacacccaggcgccgtaattcgcgccggacgtcgcgcccagtcccgcctgcatcgacagcagatgccctatcgtgatttggttcatccgcggatcgggatcggcgggaaaacggtcgcccaggaaggcggagatcggctggtccacacctgtgaacacgcccttgccgatggcgatccctcccagcgcggccaacaccgacttggaggcggacttgatgttgacggccgtgtcgagacccggcccccgcagcacccgctccaccagcgcctgcccatcgcgtgcgacgatcacgctgtgcaccttgggcaggctttccgccgccgccagggtctgggcgatcagcgcagcgtccagtccgttcgtctgggtgagcggcaggtccagggtctcggccgcgcgtccgcaggcgctggtggccgggatcagcgacagggcggaagcgacaaaggttcggcgatgcatcggccttttagcgcgtcgcccacctcgcggttgccgtcagcgacccgaggccgcagggtcacggctcagggctcagggcgcagccgcagcgctcaggcggcttcgaccatcgcgtcggcgtcatcggccttgcgccgccgcatctcgatcaggcgcacgcaccagatcgacacctcatagaggatcaccagcgggatcgcgagcatcagctggctgatcggatcgggcggggtcaccacggcggccaccacgacgacagccacgatggcgtagcggcgcccctgcgccatcacctggctgctgatcagtccggcgaggcccagcaatgtcatgaccacgggcagttggaagcacagaccgaaggccagcagcagcgccgtcaccaggttcagatagtccgacaccttgggcagcagcgccgcctgcacgccgtcgccgacgatctgctggctcagcgagaaccacatcacgaacggcagcatgacaaagtagaccagcgccgctcccagcaggaacagcagcggcgcagccagcaggaacggcagaaaggcgccccgctcgttgcggtacaggcccggcgccacgaaccggtacagctgccaggccagcacgggaaaggccagcaccacggcgccgaaggccgccagcttcatcttggtgaacaatatctccagcggcgccgtgtagatcaggttcaccatctgcccgtcgatgtgcggcagcggcgtcaatccggccgtgccgaggatcaggtccagcggcgacacatggccgtgcggcccgaccgaggcgtgaaacgccgccgccgccgcgaacggcttgaccaggaacaggtacagcggtcccgaaaaggcgaagcacaggataaaaccggccgcgaacgccaccacgcagatcagcagccggttccgcagctcgaccaggtggtccatcagcggcgcgcgcgaggcctcgatttcggcctcgtctcgatcaagggctgtcacgacgccgtctttcgcgggctgcgcttgcggaccggggtctcgcccggctcaggcggctgggccttggcgcgggtcttgcggacggtgggcgccagctcgccctccgccgtcttggcgcgccggggcttgcgggcggactcgaccggggcggccggcgcgctgaccggctccagcaccggctcggcctgcgccagggtggcgggctccgccgagggatcgggaaactcgggcatcggcggcggcgaggcgtccgccggcttgttcaggtcgtcgcgaatgtccttgaaggccgcctcggcgtcggcgcccagattgtacatcccctgccccgatctcagcgcctcgacctccttgcgcaggtcgtctagctcggactgccgcgccatttcgtcaaagctggagcggaattcgttggccatggcgcgggccttcgacaccatctgcccgacgcggcgcatcagcacaggcaggtccttgggccccaccaccagcagggccaccagaccgatcacgaggatttcgaagcccccgacgccgggacccaggccgcccattatacgctgctcatcaagaccgaggcgactagcgtttcagctcttccttttcggcctcggtgcgcggcagggaggacacgccctcgtgcggcccgtccttcttgtcgtcgtcgcgcaggccttccttgaaggccttgatgcccttggccgcgtcgcccatcaggcccgacagcttgccgcgtccgccgaacagcagggcgatgacgacgatgacgatggcccagtgccagatgctcatcgagcccatgacgaatctcctgcgattggaccgcgccggtccgcctcgtttcttgatcccgcatataggccgagtgatggccatgcgccaagggaggctgtaggcgtgcgcgaccatgagtccctccgatcacgtcatcatccacaccgacggcgcctgcaagggcaatccgggaccgggcggctggggcgcggtgctgcaggccggcggcggccatgaaaaggagctgtggggcggcgagcgcaacaccaccaacaaccgcatggagctgatggcggccatccaggcgctggaggcgctgaaacgcccctgcaaggtcgagctgcacaccgacagcaaatatgtgatgcagggcatcaccgaatggatgcggggctggaaggcccgcggctggatgacggccgacaagaagccggtcaagaacgccgagctctggcagaggctggacgccgccaggcttcgtcacgacgtgaagtggcgctgggtcaagggacacgccggccacgagttgaacgaacgcgccgacgggctggcgaatcgcggcgtcgaggaggtgctgggccggcgctgaggctcagtcggcgcgcaccgtcaggcaggagccgctgacccgctccaccagcacgtcctggcccggtccgggcggggagccgaccagctcggccgaccattccgcgccggtgacgaacacccggccgcggccgttcacaaagggctccaccacccgggcgcgctggccgatcaggcgaatttcccggtcgttgacgtccggcccgatcggattgacccgcccagccaggcgacgcgacagcagggtcgcgatcaccgtgagcaccgcgaagatcgcgacctcccacgccgcacccggctgaaagcccgcggcggtcatgacggccacgatcccggccgcgaccgccggccagagcagccactcggtcgagaacatcgcctccaccgccagcagcatcaccccgatcgccagccacacccagaacggctgggcggcgtacagttccacaagccaggtcatgctccctctccctaggccgtcggcggaaccgcggggccgctcgcgctgcgggacgccggcctggacggcgaccggttcgccccctcgcgctgctgctcgcgcgccaggccgaccagttcgcccagccctgcgatcgtgccgaccagcgagcccatatcggcgggcacgatcaccgtgcgctgctgcgggctgcgggccagttcggcgaaggcgtcgacgtagcgttgggccacgaaatagttgatggcgttgacgtcgcctcgcgcaatggcttcggacaccatggcggtggcgcgcgcctcggcctccgcctcgcgttcgcgcgcctcggcgtcgcggaaggcggcttccttgcgcccctcggcctccagaatggcggcctgtttggcgccctcggcgcgggcgatggcggcggctttctcaccatccgcctcggtgatcacggcgcgacgctcgcgctcggccttcatctggcgcgccatggcgttggtgatgtcggcgggcggggtcaggtccttgatttcgatgcggttcaccttgacgccccacggctcggtcgcggcgtcgatcacgtgcagcaggcgggtgttgatgctgtcgcgctggctcagcacttcgtccagctccatcgagccgaccacggtgcgcagattggtcatgcacagttgggcgatggcgtagggcagattgtcgacgcgataggcggcgcgggcggcgtccatgacctggatgaagacgatgccgtccaccttcaccatggcgttgtccttggtgatcacctcctgggtggggacgtccagcacctgctccatcatgttcatgcgcttgccgacgcgttcgatgaagggcgtcaggaatccgatgccggggctcagcgtcttggtgtattttccgaagcgttccaccgtgaattcacggccttgcggcacgatcttgatcacgctgaacaacagcgcgccagccagcaccagcacgacggcggcgaatattgttgtggcgtccattccgatccctccccgatccgaaggcagcctatcgctcaagcggagccgacgccagcgtcaggcgaaccgttggcgagcgagcgtcaggatgcgccgggtctccagccactcgacccgccgtaaggcctcctcgaacggaaaaaatgcggcttccgccgcatcgtctccggcccgcggctcgcctgacagccagcgggcggcgtagtcgatcagcacatagtggcggccatgttcgggaaagaggccatcgaccacatcgacgagcccgagcatctcggcctcgactccagtctcctcgcgcagttcgcgcagggcggcctggaccgcgcgttcgccgggctcgatgcggccgccgggcaggctccattcgccaaggcggggcgacgtcccgcgtcggatcagcagcaccgcgtcgccccgcatgcagacgacgccgaccgccgggatcggcgtcatcacgcgagattccatggctggatgctagctgcgcccttccccatcggccagggctttgacacaaggcgggacatgaaagccgccgtctcgcccgccttcgacgaactgaaagccgcgctgggtccgggcggctggacgcaggatccggctgagatcgcgccgtggctgacggagtggcgcaatcgctggaccggccggacgccgcttctgctgacgccgcgctccaccaaagaggtcgcacgcgccgtgacgatctgcgccgcgcacggcgtcgccatcatcccccagggcggcaacaccgggctggtgggcggccagatcccgcatggggaggtgctgctgtcccttcggaagatgcgggcggtgcgtgacgtgacgccgctggacgacgctatgacggtggaggccggcctgacgctgctggaggcccaacaagcggcaagcgcggccgggcgcgtgtttcccctcagcctggcggcggagggatcggcgaccatcggcggcgtgatctcgaccaatgcgggcggcacccaggtgttgcgctacggcatgatgcgcgacctggtgctgggccttgaggccgtgatgccgaacggtgaggtgtttcatgggctgaagcgcctgcgcaaggacaacaccggctatgacctcaagcaactgctgatcggggcggagggaacgctcggcgtggtgacggccgcgacgctgaagctgtttccggtcatgcggtcgcgcgccgtcgccattgtcgggttggaaacggcggcggcttccgtggaactgctggcgcgcgccaaggccgagaccggcggcggcgtcgaggctttcgagctgatgaagcggctagggacggacctggtgctgaagcatatcccggacacgcgcgagccgctggagagccggcccgaatggtcggtgctgatcgagatcgcgtccggtacggccggcggcgcggatacccagatggagcggctgctggaggtcgccttcgaggaaggcctgatcaccgacgccgccatcgcccagaacgacgctcagcgcgccgccttctggcgcctgcgggaagaacactccgccgcgttgaagcccgagggcggcggctggaagcacgacgtctcggtgccgatctcccagatcgccgacttcatcgacgaggccacggcggccgtggagcggtttcatcccggcgcgcgggtgtccgtcttcggccatgtcggagacggcaacctgcactacgacatcctgccgggcgtcggagaggacgtgccggccttcatcgggcgttggaaggacggctcgcgcatcgtccacgacgtggtcgcgcgctacgacggctccatctcggccgagcatggcctgggccggctgaagagcgaggaggttcttcgctacaagaccccgctggagatcgagaccatggccgccatccgccgcgctatcgacccgcagcggatcatgaaccctgcggtgctgttctagtcctcccggttcaaatcgggcgcggaaagccttatgtcgcgcacgcctgaaagagccggagccgccacgccttgctgatcgtcctgtctccggccaagcggctggacttcacccccgccgatcccgcgatcccggcgactgaccgccgcttccttgaagacaccgctcaactgtcgaagaccgccaagcgtcagacgcgcgccgacctgcgccggctgatgggcatctccgaggcgctggcggagctcaatcaggcgcggttcaaggcctttgaggcagattccaccgaaggtgttcaggcggccttcgccttcgcgggcgatgtgtacgaaggcctgtgcgcccgcgaactggacgcgggcgccttggactgggcgcaggcgcacctgcgcatcctgtccggcctctacggcctgctgcggccgctggatcgcattcagccctatcgtctggagatgggcgtcagactggccacgcgacgggggtcgagcctttacgacttctggggcgatcggctgtcacagcagctcaacgccgacgccgagggtcaggccgaacccgtcctggtgaacctcgccagccaggaatacttcggcgcgatcgacgtcaaggcgctgcgtctgccggtgatcacgccgcacttccgcgaagaaaaggacggccacagccgcatcgtctcgttccacgccaagaaggcgcggggtctgatggcgcggtacgccgccgaccgaggactggagcgcgcagaggagctgaagggcttcgacgtcgcgggctaccggttcaacgccgcggcctcgtcggacgccgactgggtgttcacccggccggatgcacgttgagcttcagccgacaaaccccgcggcgcgccgcagccggtcgttgatggcctcgccgagaccgtgatcggggatgggcgccacggcgatgccggccgggcgttcgcgatcggcctcccgcaggcggcggaacaggttggccgccgcctccgcaagatcgccggagggactgaggctccaccggaactctccgacctccggaccgaagcccagccaaatctcgcccggcttcgcctcggccgcctcgatcctgaccggcgcatcgggggcgtagtgcagggccaaccgccccggcgaacggtgtccctccccgtcctgacgcaccgggccgaccaccgcctcgatctcggcgcgggtcaccgcgcccggacgcagcaggcgggcttcgccgtccagcaccgacaccaccgtgctctccagacccaccgcacaggggccgccgtccagtaaagccgccgccgaggcgcccgtctcctccactgcatcggcgtgggtggtggggctgggccggcccgagcggttggcggagggcgcgaccactggcccgccgaacgccttcagcacctcgcgcgccaacgggtggccgggcacccggacggcgacgctgtcgaggcccgcccgcgccagatcgctgatccggtcgttatccagcaccggcagcaccagcgtcagcggaccgggccagaaggcgtcagccagggcgttcgcctgagcatcgaactgcgccagcgcccgcgccgcctgagcatccgccacatgggaaatcaacgggttgaagcgcggtcttcccttggcttcgaagatggctgcgacagcggcggcgtctccggcgtctgcggccagcccgtagacggtttcggtcggcaggatcaccagccgcccgccccgcagcgcctcgaccgccgcctggacggtgtcgctcatggtcggcgcgggatcagcgggatcatgcgatgcaggacgttgtcgcgattgatgaagtggtgcttcagcgcgcccaggacgtgcagcgcgatcaggatgtagaggctcttcaccaccgcccgatggatgtccatgaaggcgccggccgcctctcggccgccgcccacgggcaggagcggccactggaacaggccgaaccattcgatcgcacgcccgcccgccgaagacgccagccagccggtcatgggcagggccaacagcacgacatagaacagcacatgcgttgtgcgcgccgccatcttctgccagcgcggcgtctccgcgggcagaggaatggcgggattggccagccgccacgccagtcgggccagcgtcagcaccaggatggtcagccccaccgacttgtgcaggccgatgaacgacccagcagccgggccctcggcgttgtcggcggccgagatcagcaccacctgagtcaccacaagggcggccgtcagccagtgcagggtcagggacactgtggagtagcggttgcgcggttcggccatgcggcttcccttccgtggcggcagggcgccagcttggcggatcagggcggtttcgccaagcgcttgcatcgtcgcccgccggcgcggcacagacggcgcaaagaccaaaggatggatcatgacctatcgcgcccccgttcgcgaccttgccttcaccctggacgtcgtgggcgcggatcagctctccgccaccggcgccttccccgactatgattcggatgttcgcgacgccgtgctgcaggccgccggtcagttctccgaagaggtgctggctccgctgaaccgcatcggggaccagaagggttcgacctacgccgatggcgcggtcacggccgcgccgggtttcgccgacgcctatcgccagttcgccgccggcggctggaccggactgtccgcctccgtgtccgccggaggacaggctttgccaaaggctttggagctcgcggcctatgagaccgtgcacgccgccaacatggcgttcggcctgtgccccatgctgtcgctggccgccatcgaggcgctggagcaggtcgggaccgagcagcagaaagagacctatctgacccggctggtgtcgggcgaatggaccggcgccatggtgctgaccgaaccgggcgcgggctcggacctcggtgcgctgaccgccaccgccacgccgaacggcgatgagacctacagcctgaccggccagaagatcttcatcacctggggcgaccacgacgccacggacaacatcgtccatctggtgctggcccgcctgccggacgcgccgaaggggccgaaaggcatcagcctgttcctggcctccaagttcgaggtgacgccggacgggacgctgggcgagcgcaacagcttccggccggtcgggatcgaacacaagctcggcatccacgcctcgcccacctgcgtcatggcctatgagggcgcccgcgccgaactggtggggcggccgaacgaaggtttggcccatatgttcgtgatgatgaacgccgcgcggctggcggtgggcgtcgaaggcgtcgggatcgccgaacgcgcctatcagggcgcactggcctatgcgttggatcgacgccaagggcgatccgtgtggacgggagaggcgtcctccccgatcttcgatcatccggacgtccgccgaagcctggcggtgatgaaggccaagatttcggcggctcgggccatctgcctgctgactggcgtcgccgccgacatggctgagcatgcggcggacgagaccgatcggcggcgctggaaggcgcgcgaggacctgttcactcccatcgccaaggcctggtccaccgacgtcggcgtcgaggtcgcctcggccggccttcaggcgcacggcggaatgggcttcatcgaggagaccggcgccgcccagcattatcgcgacgcccgcatcgccccgatctacgaaggcaccaacggcatccaggccatggatctggtcggtcgcaagctgtcgatggacggcggccaggccgcgcacgacctgatcaaggacatgaagacgacggcggcggagttgtcgcggctttattccggcaagccggtcgaacgcttcgccaccgcgatcgaggcggtcgaggacgcgaccctgtggctgctggaccgcaaggccgacacggccgccgccgccgacgtgctggccggcgccgacgcctatctgaagcttctgggggacgtggccggcggctggctgctggccaagggcgcgctcctggccaaggcgcgactggacgccggggacggtgatcccgcatggctggaaggcaagatggacctctacgaggtctacgccgccaacgtccttggtcacgtctccagccggctggcggcggtcggccagggcggcgaactgctgaagcgcatgacggtggaagctctcgccggctagaacccgggcggcgcgtccagcagggcgatggccgcgcggacgtcttcggcatgggcgaccacgccgatgctaagccgctcgtcgttcaccctcacctcctgtgtcagcatgccggcgacgtaggggtgattgggcgcccggtcgctggcggtcttcctcgccgccggcgtccagaacaccggcccgcccgagttgccgggaaagaccgcgaagtcgagcagaaaggtcggaaaggccgtgatcggcgtcagcggccaagaggcgatccttcctgtccgcaggatcggaaagcccgcgcgattagccgacagtccatggggaaagccgagcgtcagcatctcgtcccccggcccgacctgcgcctcatcgaacatatccggtcccgccagccacgccagcggaatggccgcacgggcgaaggcgggcggcgcttcgatcgccatcaccgcgatgtcgcgatcgggatggcgggtccacagcggctggtcgctttggtcgcggattgcgaggggttccggatcgaaccgccaggcgccgccggtcgtctccacccgccagcccaaccgcgccccccgcccctgcatgcggtccaggacatggcccgccgtgaccagcaccgtgcgaggcgcgccgtccagctcgggcgcgttcaccagaaaggccgttcccaccgtgcgtgtcccctgcccgttcggctggtcgatctgcacagtggcgtcgatcaggctccgcgtcagcgtccaggtcggctgcgcggcctcgacggggggttcgacctgtatcggcgtgctgtcgaacatcgcggctcctgatccttgggcgcctttcatttgacgagcgccccttgcccgcacaaggtcccgcccgcatgagcttttcgggggaaacgccgccatgaaccgccgccagatgatcgcttccagcgccgccgccgccctgtcggccgccgccgcgccttccttcgccagccccaccggagcccagatgcccgccaatcgcccgacgccgcccgtcgccaagaaaatccccgtcatgatcgaacagctggggcgcacccgcaccgacgactatcagtggatgaaggacgacaactggcaggccgtgctgcgcgacccctcgctgatcaaggccgaggtcaaggagcatctggacgccgagaacgcctatcgcgaggcgatgatggtctccaccctgccgctgcaggagacgatgttccgcgagatgcgcggccgcatcaaggaggacgacgcctccgttccggcgcccgacggcccatgggaatattacgtccgctacaacaccggcgatcagcacccgctgtactgcaggaagccacggaacggcgggcctgagcaggtgctgctggatgcgaacgccctggccgaaggcaaggcctattccgaggtgtcgaacgcctcgcacagccccgaccacgcccttttcgcctatgccgaggacgcgcaggggtccgaggtgcacaagatctacgtcaaggacctggcgacgaaccaggtactgcccgaggtgatcgacagcgcgacgggcgacttcgccttttcacccgacagccagtggatcttctggactaaccgcaacgacaacggtcgccccgacaagatcttccgccgtcccgccaccggcggcgagacgaccctggtctatgaggaagaagacgagggcatgttcatcggggtgggctgcacctccgacgatcgcttcatcgtcatcggcgttcagaaccaggagacgtccgagacccgctacatccctggcgatgcgccgacggccgcgcctgtcgtgctggagccgcgcgaggtcgcgcatcgctatgacgccgatcactggggcgaccgctgggtgatccgcacgaacggcggcgacgccgtggacttcaagatcgtgacggcggcgacggacgcgccggcccgcagcggctggaccgacctcgtgccccatacgccgggacgcttcatcgagagcttcgacctgacaagggaccatctggcgcgccaggagcggtcggacgccaacacccgcatcatcatccgcgaccgcgccggcgccgagcacgagatcgcggcggacgagcccgccttcgccctctctctggccggggcgtccgaatacgacacgggtgtcacccgctacgcctacaactcgccgtccacgccgacgcagacctatgactatgacatgggctcgcgcgagcggaccctgcgcaagacgcaggagatcccgtccggccacgacgtcgcgaactatgtggtcgagcggctgaacgcgccggcctccgacggcgaactggtgcccgtgaccgtgctgcgccgcaaggacacgccggtcgacggctcggcgccgctgctgctttacggctacggctcctacggcatcccgatggcggccagcttctccaccaaccggctctcgctggtggatcgcggctggatctacgccatcgcccacatccgggggggatcggacaagggctggggctggttccaggcggcgcgccgcatgaccaagaagaacaccttcaccgacttcatcgccgccgccgagcacctgatcgacaggaagtacgccacggccggccgcatcgtcgcgcagggcggctcggccggcggcatgctgatgggcgccgtcaccaacatgcggcccgacctgtgggccggggtcatcggtcaggtgccgttcgtggacgtgatcaacaccatgagcgacacctcgcttccgctcacgccgccggagtggcccgagtggggcaacccgatcgaggatgccgccgcctacgactacatgatgagctacagcccctacgatcaggtggaggccaaggcctatccggccgtgctggcgaccggcggcctgtccgacccgcgcgtcacctattgggagcccgagaagtgggttgccaagcttcggcccgccaccacctcgggcaagccggtgctgctgaagatcaacatggaggccgggcacggcggcgcggccggacgcttcgactacctgaaggaagtggcgcacgactacgccttcgccgtctgggccattgacgagggctggaacaaggcctgaccgtgcttgccgccgccgcgttgccccacgcggcggccgcccctatgctggagcgtgaagatcgtgcgcttccttctgatgctgatgggcgtggcctccgtgctttcgctgggcgccgtctcggcttcggcggcccctgcgtccgagccgccgtgtcaccagacggaaggcgcggcgccgcatcaccccggcggcccggcttccgacgcgccgcggtcgatgaaggtcatggcctgctgcgtcgcctgcatcgccgcgtcgcccctgcccgccgccgcgccggaagaggcgacaaggggcgccgcttcgaccggtttcgccctctccgccctgccgcgcggccggtctccggcgccgcctatcggcccgcctcgcctcctgatcgtctgacccgccgcgcccgccccggcgcgatttcacgtcacgatctgaaaggaggaagccgccatggctgtccgatccctcgccggcctcgccgccggcgcatccctgcttgttctcgctgcagaggcgaaggcgcaggatcacagtcaccatcctgcgccgacgaccgccggctcgctaccggttgccccgccgcagcagccggcgccgcacgaccattcctcgatggctcatgatcacgaggccatggaccatcacgccgccgccggccacgccggcatgaccagcccgctcgggccctggtccatgtcccgcgacgcctccggcaccgcctggcagccggacctcggcgagcacggcggcgtgcacgcgcgggtcggcgactggacgttgatgagccatgccctgctgaacctcgtctacgacaaccagaacggtctgcggggcgacacaaagacctttgcggcgggcatggtgatgggcgccgcgcgccgcgacttcgccgatggatccaagctgaacctgcgcgccatgctcagccccgatcccttgatgggcaggtcgggctatccgctgctgctggcggcgggcgagacggcggatgggatcgacccgttggtcgatcgccagcatccgcacgacctcttcatggagctgtcggccagctactcgcgccagctgtcgccgaccgacagcgtctacgcctacatcggcctgccgggcgagccggcgttcggaccgcccgccttcatgcaccgcatgagcgccatggacagcccggaggcgccgatcactcaccactggctggattcgacccatatcgtcttcggcgtgacgacgctgggctggacgcacgatcgcttcaagatcgaagcgtcggccttcaaggggcgcgaaccggacgaagaccgctgggacatcgaagaaccgcggctggacagctggtcggtgcgcggctcgttcaatcccacgccggaatgggcctttcaggtctcctacgccgacgtgtcagcgcctgaacagctcgagccggacgaggatcagcggaagtggtcagccagcgccatccacacccgccgcttcgggtcggacggctggtggtcctcgaccctggcgtggggtcgcaagaccaacgatcacgacgagagcaacgacgcctgggcgctcgagaccgccctgcatcccgacgagcgctggacggtcttcggacgcgccgaacggatcgagacggacgaactggttcccggcgtcggcggcggacacgggccgctccacaccgtctccaaggcgtccatcggcgtcgtgcgtgactggcgtctgaaccgaaacgtgcggttcggcctcggcgggctctatgccgtcaaccgcgtgccggccgcgcttgagccgctgtatggcggcgatccggacggcgccatgctgttcgtgcgactgaagatcggctgacgccgaagcgggagccggcgcgcatccgcgcgtcggctctcagacgtgtccgtgacccagcagggccgagccgaaacggaccagaaggccggccgcgcccacgcccgccattacggtcagcagccgaaagtgccgatggatgaagtaaaggatctcgcccgccatgcccgcctcgccgctcgccttccagcagcatctaggcacgataacagcggtcgctcaccttcacacgtccatcacgcgaatttaaccaaaccgccggctcagaccagccggctctgcaccagcgccgcctcgatgaagccggcgaacagcgggtgcggcgcgaacggtcggctcttcagctccggatggtactggacgccgatgaaccaggggtgatccggccgctccacggtctcgggcagcacgccgtcgggcgacaggccggcgaagatcagcccgcccttctgctcgatggcctcgcggtagttgatgttaacctcgtagcggtggcgatgccgctcgctgatgtgggtcgagccatacatctcggcgatcttcgatcccggcgtcagggtggagtcgtaggcgcccagccgcatggtgccgcccaggtcgccgccctgctggcgcagcacccgctggttgccttgggtccactccgtcattaggccgaccaccggctcgtccgccgggccgaactcggtcgagctggccttggggaagcccgccaggttccgcgccgcctcgatcactgccatctgcatgccgaagcagatgccgaaatacgggatcttacgctcgcgggcgaaccgcgccgcctcgatcttgccctccgatccgcgctcgccgaagccgccgggcaccagaatggcgtgggcgccctgaagccgcgcgttgcaggcctccgtgtcgccttcgaaagtctcggcctcgacccagtctatgttgaccttgacccggttgtgcacgccgccgtggtgcagcgcctcgatcagcgacttgtaggcgtcctttagcaccgtgtacttgccgacgcccgccacggtgacctcgccgtccggattcaggcggcgatcgacgatgtcggtccagcgcgacaggtcgggctccggcgcgtcctgcacgccgaagtgcgccagcacctgccggtccagcccctcccggtgatagtctagcggcacggcgtagatgtcggccgagtccatggcctggatcacgccggattcccgcacgttgcagaacaggccgatcttgcgcttctcctcggccgggatcggctgttcgcagcggcacagcaggatgtccggctggatgccgatggagcgcagctccttgaccgagtgctgggtcggcttggtcttcatttcgccggcggtcttgatgaagggcaagagcgtcaggtgcacaaagcagctctggccgcgcggcaggtcctggcccagctggcggatggcttcaaagaacggcaggccttcgatgtcgccgacggtgccgccgatctcgaccaggatgaagtcgacctcctcgcccgcgtcggtcagcgcttcccgcaggcagaaggccttgatctggtcggtgacgtgcggaatgacctgaacggtcgcgcccagatagtctccgcgccgctccttctccagaatggtctggtagatgcggccggtggtgatgttgtcagacttggcggccgacacgccggtgaagcgctcatagtggccgaggtcgaggtccgtctcggcgccgtcgtcggtgacgaagacctcgccgtgctgatacgggctcatcgtgcccggatcgacgttcagataggggtccagcttgcgcaggcggaccttgtagccgcgcgcctgcaacagggcgccgagagcggcggaggcgaggccttttccgagcgaggaaaccacgccgccggtgatgaacacatagcgagccatgtcagaccaccttcaggctgagcgtgaagtcgggcgtaacgcccgaaacgggcgctacaaacgcccaactttgtccaacagtgttcaacgctgacctgtcccaagagctcgaaataaaaggaaatccctgatttcctgcattttctggtcgtgcaacgacgcaacgagccatgggcggacaccttactccaagcttcgccggccggaccagccgctcgcgcgaagaaactgttgatcacaagaagaaagcgcgccgggcggcgcgctttcaggtcgtctggtctgcgtggagccttacggctgaggcgcggggttcggacggctggcctcggtcggcgtgccgccctgcgaaggggtgctgggcgaggcggtgaggctgctctccagatcgtccagtgagggcgcggccggctgcgcgggcgcttgcgccggagcggtctgggcgggcgcgctctgggtcggctggctgtccagcgcgatggagcccaccgcatcggcgtcgatgaccgagttgtcgcgcgccatgttgctgacgatcgtcaggatgatggtcagggcgaagagcgccgcagcaagaccccaagtcacgctggtcagcagattgccggttcctcttgcactcatgaagcccgacggtccgccgcccatgccgagcgcgccgccttccgaccgctgcagcagcacgacggccgtgagcgagatggcgaccaggatgatggcgacgagcaggatggtctggagcatggcgtcaatcatgtgggcgcggagctgcgccgatcaagcggcggcctctatcaccgaagcccccggcgggcaaatgagcgctcagcccgccgcgcggatgatgcggaggaaatccgcggccttgagcgaagccccgccaaccagggcgccgccgacctccggtgtctgcagaatggccgcggcgttcgccgggttgaccgagccgccatagaggatcggagcagcgcgtccgccctccccgaaccgctcgaccagcgtccggcgaatcgccgcatgcacctcggcgatctcgtcgcgggtcggcgtgcggccggtgccgatcgcccagatgggctcataggcgacggcgaaccccttgcccgccaagccgtccggcagcgatccagagacctgcgccgtcacgacatcgaccgccctgccggcgtcccgatcctccagccgctcgcccacgcagacgatcggttccagcccgtgggcgagcgccgcctcgaccttggccgcgacctcggcatcgctttcgcggaaggcgtcgcggcgttccgagtgccccaggatcaccagcgtcgccccggcgtcctccagcatctccgccgaggccgagccggtgaaggcgccgcagctttcggagtggcagtcctgcccccccacctcgatggagccgcctcgcaccgccgtctccagccgatggatcagtgtcgccggcggacagatcaccacccggcagggcgcgggctggcggcgcaggtcggcgtcgacggcgcgcgcctcgtcgatctgggcgcccagcccgttcatcttccagttgccggcgatcatcttcacggattgtttcatgcctccctgtctaggcagggtggcatgccaagccaagacccttcgccgcaatgcggccccgaagctgttcttgcggcggcggggcgcccccgcctatacgccatgcatatcgccctgtgacgctcgcgtccgccatcgcccggtttcttcgatgatctccagcttccgcgacttctcccggtccaagtgggccatcggcctgttcgtgctgatcatgatcagcttcgtgatcgtgggcgcccgcatggacgtcttctcgaacctggggcccaagcacgtcatcgatgcgggcgagcgcaccatggacgaggcgaccttccgctcctccatggacagggtgcgcgccaatctgcaggaacaggccggccgtcccgtgaccatcgaggacatggtggccgagaacatccacacccgctttcttgaaagccagacccagcagctgggcttcctgaactgggcgtggaaggcgggcgtccgtcccggtcagcagctgatcatcaagcagatccgccagatcccggccttcttcaactcggtcaccggccagttcgatcaggagcagtaccagcaggcgctggcccagcagaacgtcaccgccgcccagctggagcaggacctgcgcgatcagtatgtgatcgagcatttcggcgcggccgtcttcgccggcgcgcgcgtgccccgcgtttacggggcgcttctcgccggacaggcctttgaaacccgcgacggccgctggttcgaggtcacccaggccatggcgggcgcagcccccaatccgaccgacgcgcaactgaccgccttcatcaacgagaacgccgcacgcctgcgcagccccgagctgcggatcgcctcggtggtcctgttcacgccggacgaggcggcgcgcaccgcgcccatctccgagcagcgcattcaggagcggttcgagttcaagaaggccacgctgggacagccggaacgccggacctttgtcaccctgaccgcgccgaaccgcgagatcgccacccgcatcgcggcggctctgcgtgcaggccagacgcccgagaacgtcggacgcgccaacagcctgcagcccgcgaccttcaccgaccagccgcgcgccgccgtcggcgaccaggccgtggccgccgccgtgttcggcctgcaaaacggccaagtgtccgatcctgtccaggccggcgtgggcttcgccgtcgccaaggtcaccggcatccagcccggccaggaggccagcctggagaacgcgcgcgagggcctgatccaggagttgcgcgaggaagacgccaagggcgcgacctacgccaaggttgaggcctatgagaaggcccggtcggaaggccgcaacctggccgacgccgcccgccaggtcggcgcccgcatcgttcagctgccgcccttcacccaggacggaaagctgccgaacggccaggcgctgaacgctccgccgcagatcttcgaaaccgcatggggcctgagcaagggcggcgaaagcgacgtggtcgacgcgggccagggccagtacttcgccgttcgcgtcgatgatgtgcgccccgccgccctgccttctctgaacgaagttcgcgcccccctgacgaccgaatggctgcgtcgcgagaacctcaagcgcatcaccgccaaggccaatgagctggccggtcgcgttcgcgccggtgaggacatcgccgccgttgcgcgctcggccaatgcgccgctgacgacccgaacgggcgtggtgcgcaatcccgaaaccacccaggcgctcggccagggcctgctgcaggggctgttcggtcagggcaagggccaggtgttcgtccagcccgcttcggaaaccgccgtcgccgtcggccgcgtggacgacgtgcgcgccgcctcgcccgccatcgccgggccgttggccgaacaggtgcgtccgcgcctcacctccgagctggtgcagtcgatggtcgaaagctcgctgacggccggcgcggctcgctccaaggccaagaacgatcccgcggccgcgcgtcgcgcgctgggtctgtcggatcaagcgacgcccgccgcgcccacgcccgccgcccaatgatcaaggccgagggcgcggatctcgcccgcttcatcgaagggctgaaggccggacggccgcaggtagtggtccggcggctgatcgacgatctggagacgccggtctcggcgtttctgaagctcggccgcgatcggccctacgcctgcctgctggaatcggtcgagggcggcgcggtcaagggccgctattcgatcctgacgctcgacccggacgtggtctggcgctgccggggggaacaggccgagttagcgcgcggcccgggcgtgacgaccggacaattcacggccgagagcctgccgacgcttcagtcgcttcgcaccctgatcgccgcctcgcgctttgacctgcccgacgacttgccgcccatggccgcgggtctgttcggcgtcttcggctatgacatggtgcggctgctggagccgctgggcgcggccaacccggacccgctcgatctgccggacgcagtgctgacccgtccctcgctggtcgccatcttcgattcggtccgccacgagatcgtgctggtcgccgccgcctatcccgacaacacgaccgatgccgaggttgcgtggtccgaggcgaacgcccggctggaggccttcgaggccgcgttgcaccagcccctgcccgcccgcacgacgcctgccccggcgcccccgcccgccttccgttcgcccatcgacgaagccgccttcaccggcatggtggccgccgccaaggactacatcgccgccggcgacatcttccaggtggtgctgagccatcgcttctcggctgactggagcggcgatccgttcgccttttaccggtcgctgcgccgccagaacccctcgccctatctgttctatctgaacttcgaaggctttcagctggcgggctccagcccggaaatcctggtgcggctgaaggacggcgaggtcaccatccgcccgctggccggcacccgcgcccgcggcgcgacgcccgaggccgatcgcgcgctggaggtcgaactgctggccgatcccaaggagcgggccgaacatctgatgctgctggacctcggccgcaacgatgtcgggcgcgtcgccgcccctggcactgtcgaggtgaccgagagcttcgtggtcgagcgttacagccaggtcatgcacatcgtatccaacgtgcgtggcaaggccgatcccaggttggatgcggtcgacaccctgctggccgccctgcccgccggcaccctgtcgggcgctcccaaggtgcgcgcgatggagatcatcgacgaactggagagcgaaaagcgcggcgtcggctacggcggcggcgtcggctacatctcggcgggcggcgaggcggacatctgcatcaccctgcgcaccgccctgttcgccgacaaccgcatcttcgtccaggcgggcgcgggcgtggtcgcggacagtgatcccgcggccgaatacgccgagacccggcataaggcgcgcgccccaatgaaggcggccgaggacgcctggcgcttcgaaggctgacgccttagtcgacctgaaccgtctcgtcgatctgtacgcccggccccagcaccaccacgcccgccatcagcacggcggcgatcgcggcgaagctcgcggcgcccaaggccgccaacccgctggccggacgcgccgcttcggtcagcatcgtccgggcgctggcgatctttgcggctgcggtcatggggcggtcctcgatcaacatggcgactgtcgagcgatagggttaaggccgcctttaccgggctaacggcttggcggatcggcggcgggggcctagaagccgtgccatgatcctggtcgtcgataactacgacagctttacctacaatctcgtccactatctcgcagagctgggcgcgccgacgcatgtggtgcgcaacgacgacctgacgccggacgaagcctgggcgctgaagccggacgcggttctgctgtcgcccggcccctgcgccccggatcaggcgggtatctgcctgccgctgatcgagaccgcgcccgccgacatgccgattctgggcgtgtgcctcggccaccaggccatcggccaggcgttcggcggcgaggtggtgcgcgccaagacgctgatgcacggcaagacctcgccgatcgaacatggcggcgacagcgtcttcgccggcctgcccgcgccgttcacagcgacgcgctatcattcgctggccgtgcggcgcgacaccttgccggacgcgcttgctgtcaccgcctggacggccgacggcgagatcatgggcctgcgccaccgctcgcggccgatccacggcgtccagttccacccggagtcgatcgccaccgaacacggccacgacatgctggccaacttcctgacactggcgggcgtcaagcgcctcgccgccgcctgatcgcgcgacgctcgccgtggccgacgggttcaagccgatcctcgcgcgcctggtcgacggccaggcgctgacgccggaacaggcgcacgacttcttcgccgcctgcctgcgcggcgaacccacgccgccccaggtggccgccgccgtcaccgccctgcgcatgcgcggcgagacggtggaggagatcaccgccttcgcccgggcgatgcgcgaggccgccctgacgctggaccactcctatgaggtgatagacacctgcggcaccggcggcgacggccagcacacctacaacatctccaccgccgcagccctggtcttggccggcgcggggctgaaggtcgccaagcacggcaaccgcgccatgtcttcgaaatccggctcctccgacgtgctgtcgatgctcggcgtggacctgagggcgggaccggaccagcagcgccgcgccctggacgaggccggcatctgcttcctgttcgcgcctgcctatcacggcgccatgcgccacgtggggccggtgcgggccgaggtcggctttcgcaccgtgttcaacctgctggggcccctgtccaatccagcgggcgcgcggcgtcaggtcatgggcgtctatgacccgcgcctgctggagccgctggtcgaggctttgggccgtctgggcgccgtgcgcgcctggaccgtgcacggccagggtctggacgaactcaccaccacgggtgcgtcggaggtggcggagtggagagacggccaggtgcggcgtttccaggtgtggccggaggacgccggcctgccgcgcgcctcgcttgacgaccttcgaggcggtgacgccgaggagaacgccgccgcgctccgcgccctgctggacggcgcgcgcagtccctatcgcgacatcgtgctgctgaacgccgccgccgcccttgtggtttcggaccgcgcggagaccctgatggacggcgccgcgctggccgccgcatccatcgacgggggtcatgccgcagcggcgctggagacgctggcgcggatcacctccaccccgcccgaacccgcgcctgaggcctgacgccatgaccgacatccttgatcggatcgccgcctacaagcgcgaggacgtgcgcgcccgaaaggctgcatgctcccaggacgagatcgagcgcctcgcctctgcggcttcggcgccgcgcggcttccgatcggcgctggaagccgcccacgaacgcaccggccggccggcgctgatcgccgagatcaagaaggccagtccgtccaagggcctgatccgcgccgacttcgagcccgcatcgctggcccgcgcctatgaggcgggcggcgccgcatgcctgtccgtcctgaccgacggcccgagctttcagggcgacgacgcctttctggcgcaggcgcggaacgccacggccctgccctgcctgcgcaaggacttcctcctcgatccgtggcaggtggcggaaagccgggcgctcggcgcagactgcatcctgatcatcctggcgatggtcgatgacgccttggccgccgacctcctggcggaagcggagcgattcggcatggacgccttgatcgagacgcacgacgaggcggagatggcgcgagcctgcgacctcggcggcgatctggtcggcgtcaacaaccggtctttgcggaccttcgaggtcgatctggagaccacggccatgctgtcgatcctcagcccggttcgcgcgctgctggtctccgaaagcggcgtcttcactcccgacgacgtgtcgcgcgtgcaggacgcgcacgcccaggccatcctggtcggcgagagcctgatgcgccagccggacgtggaggccgcgacccgcgccctgcttgcctaagagcctcttcctccgcttaggttgacattaaccgggaacacttacagaacatcgtcaatgttcacggcccgttccgattctcctcgcggcgggcagatcaagggtccggcgatgctcacgcgcaagcagcatgaactgctgatgttcatccacgagcggatcaaggagaccggcgtctccccttcgttcgacgagatgaaggaagcgctgaatctggcctccaagtcgggcatccaccgtctgatcaccgccctggaggagcgtggcttcatccgccgcctggcgcaccgggcgcgcgcgcttgaggtcaccaagcttccggagcaggccagcgcctcgtccggccggtcgcgccagccgttccgaccggacgtgatcgacggcggcgcgcgcagccccgcgcccgaggccgccaacgacacgcgcgaactgccgctgctgggcaagatcgccgccggtacgccgatcgccgccatccagcacgagcgcgaacgcatgcccgtgcccgaatcgatgctgggctcgggcgaccactatgttctcgaaatcgagggcgattcgatgatcgaggccggcattctcgatggcgacctggtggtgatccggcgcggcgacaccgccaacaacggcgagatcgtcgtggcccttgtcgagggcgaggaggcgacgctgaagcgcctgcgtcggcgcggcggctcggtggcgctggagcccgccaatcgcaactacgagacccggatcttcggcccggaccaggtggccgtccagggcaagctggtcggcctcatgcgccgctatcactgaaatcggggtcagagcgacggctccacggccggtcgcctcgaacatcgccgctccagcgcgcggtccagcggcctccgtcatgacgtcgcaactcgaccgcgcctttttcgaaatcaaccgcgtccagcaccagccgcccctcgcagcccgccggcagggaagcgacggcggcgcgcacgcttacgaccggggccgaccggcacaaggcgtcgagcgccgccgcatccggcgcctttccgccccaccacagggcgaccggagcctgtgcggacggtcggggaaagcaggagaagcgggtgcagacccactggtccgcggtcctgtccgccagagccaggccccgtcgtctcgaccatagttcggaggcgaacgcgcccacgccagggcgcagcgcgacggcctcgggtccgcgactgtaggcggcgaccgccccgccgtcggcgatccacaggtccggtgcgctcggcttgggccagagcaggacggccgcggcgagcggcaggccgagccaccgacccgaccctcgccacaggcacatgaagaggacgccgagaaaggagatcgccagcaccggatccggcgcgctcgcgatggtccgcaccgcgccgggcaggtttgcggtccaggcgccgatcgccagcatggcgtcgacgccccaacctgtcaccgtcaggaagggcgcgccaaggccgatcggctccagcaaggcgccgagcgcgaggaacggcatcatcacgaaatccgaaatgggcgccgtgacgaggttggcgacaaggccgtaggtggcggtgcggttgaagtgctggacggcgaagggcgtggtggccagacccgccaccagactggcggcgacggcggcccccagccacgcgccgccgcgctggacgatcaggatcggcaaaggcgcggagatctcccgcaggcggctcggccaggcctccaccagcgccaccagggcggcggtcgcggcgaacgacatctggaaccccggcgtgacgatcgcctgcggatgaagcagcaggaccaccatggccgcgaccgcaagggcatgcatggtgatcgcctgccggtccagcaggatggcgacaaaggcgatggaggcggtgatcgccgcccgctcggccggcggcggcgcgcccgacaccaccagataggcggacacggcggcaagccccgccacggccgcgaccttcttgcccgatacgcgcagcgccagccagggccacgccgcgaccagcagccggacggagaagaaggcgaagccgccgaccaccgccatgtgcaggccggagatcgacaggatgtgcgccaggcccgaggcccgcatcatctcctggtcctcgcgcgcgatccaggtctcgtgtcccgtggtcatggcggcggcgacgcccccggtgcgctcgcccagccgcgccacgatgcgctgcgcgagatcgaagcgcgcgccgttgaccgccatctccagccgcaaccgccaccccggcgacgggagatcggcgaatcgcgtctcgcccaaggcgaaggccaccccgcccatgccttcgaaaaaggcgttgcgaccgaagtcgtatgcgcccggcgccgcgggcggcggcggcgggttcagaatggcgaacagccggacgggccggcccggctccggcggggcgcctctcaccgtggcgcgaaggcggacaggcgtatcctccggagcaagcccgcggatgcgcacgggggctacgatgacgcgatgcccgcgttcgccgggtgagtcgacatccacgacccaggcctcgaccgtcgtcggttcggcgatggccggcgcgatcggcgcctcgaccgtcatggtcttcagccgcgcattagccatgcccatcgccgtcaccgccagcatcagcaggggccatgtccaggcgcggccggcgcctgctcgcttgagcatgcgccaggcgcccagcagcaccagcgccgtcgccgccagcggccacagcggcggctcgaagcgaagggcgaagtagaggccgcatcccccgccgaacgccaccggcgtccacatcgcccaccgcgcgtcctgcagcgcgacggcctccctcaggcttgcgcgcaggcgcgtccagggggtgggctttggcgaagcggggcgtataagggcctcgcctacggaccctcctccccccatgaccgcttcttcctcgaccgtcgtcacccgcttcgcgccctcgcccaccggctaccttcacattggaggggcgcggacggcgcttttcaactggctttacgccaagggtcgcggcggccgcttcctggttcgcatcgaggacaccgatcgcgaacgctcgaccgaaggcgccgtgcaggccatcttcgacgggctcagctggctggagctgttcgccgacgaggcgccggtgttccagttcagccgcgcggatcgccaccgcgaagtggtggaccaactgctggagagcggccgcgcctatcgcgacttcacctcgccggaagagaccgcgcggctgcgtgacgaggccaaggctgacaagcgcgccttcgaatcaccctggcgcgaccgcgaacccagcgtggacgatcttctcctgccgcacgtggtgcgctttcgccgtccgcagggcgcgaccgtgaccgtgcctgacgaggttcagggcgccgtcagctggtcgacgaacgatctcgacgatctggtgctgctgcgctcggacggcgcgccgacctacaacctcgccgtggtcgtcgacgaccacgacatgggcgtgacccacgtgatccggggcgacgaccacctgaacaacgccgcccgccagagcctgatctatgacgcgctggactggccgcgcccgaccttcgcccacattccgctgatccacggtccggacggcgccaagctgtccaagcgccatggggcccaggcggtgcacgaatacgccgacatgggctatctgcccgaggcgatgcgcaactatctggctcggctcggctggtcgcacggcgacgacgagctgttctccgacgcccaggcgctggaatggttcgatctgtcaggcatcggcaaggcgccggcgcggctggacttcgacaagctggcgcacgtcaacggccactggcttcgtctcggcgacgacgagcggctggccaagctggcgctggacgtccacctcgctcgcggccgcgctctggccgaagacgacgaggcgcggctgcaaatggccatgccgttcgtcaaggatcgcgccaagacggtgctggagctcgccgaccagaccgcctttgtgctgctggcccgcccgctgatcctggacgacaaagcccgcaagccgctgaccgaagaggcgctggaacgtctggcgcggctgcgttcgcggcttcagctgttccagtcctgggacgtgttcgccctcgacgccgacctcaaggcgttcgccgaggaagagggcgtgggctttggcaagatcggcccggccctgcgcgcggtgctgacggccggccatccctcgcccgacatcgcgcgcatcctgtcggcgctcggacgcgacgaaagtctggggcgcttggatgatgcgctgcaagggcttaagtgatcacccataaccacaaggcgaccggcgctcccccgcgactggccgtagatgcaaaggggcattcatgactgaacaagccaaacccgccggctcggcgacctttacgctcggtgatgcgtccgtcgagcttccggtcctcgccggttcgacgggtccggacgtcgtcgacatccgcaagctctacggcgcgacgggcgccttcaccttcgatccgggcttcacctcgaccgcatcgtgcgaatcggccctgacctacatcgacggcgacgcgggcgtgctgctgcaccgcggctatccgatcgatcagctggcgtcgcagtcgaactttctggaagtctgccacctgctgctgcacggcgaactgccgacggcatcgcagttcgagacgttcgagcagaacgtcacccgccacaccatgctgcacgcccagttcgaccgcttcttcgaaggcttccgccgcgacgctcacccgatggcgatcatggtcggcacggtcggcgccctgtcggccttctaccacgacagcctggacatccacgatcccgtgcagcgcgacatctcggcgatccgcctgatcgccaagatgccgaccatcgcggcgcgcgcctacaagtaccacatcggccagccctttgtgtcgccgcgcaacgacctgagctacgccgagaacttcctgcgcatgtgcttcgccgtgccggccgaggaatatcaggtcgatccggcgctggtgcgcgccatggaccgcatcttcatcctgcacgccgaccatgagcagaacgcctcgacctcgacggtgcgtctggccggctcgtcgggcgccaatccgttcgcctgcatcgcggcgggcatcgcctgcctgtggggcccgtcgcacggcggcgccaacgaagaagcgctgaacatgctgcgcgagatcggcacgcccgaccgcatccccgagttcatcgagggcgtaaaggcccgcaagtacaagctgatgggcttcggtcaccgcgtgtacaagaactacgatccgcgcgccaaggtgatgcagcagtcggcctatgaggtgctggcggcgaccgggcgcgagaacgacccgctcttccaggtcgccaaggagctggaggccgtcgccctgaacgacgagttcttcacctcgcgcaagctgttcccgaacgtcgacttctattccggcattaccctgtcggcgatgggcttcccgaccaccatgttcaccgttctgttcgccctggcccgcaccgtcggctggatcgcgcagtggcaggaaatgatggccgatccgtcgcagaagatcggccgcccgcgccagctgtacaccggcccgaccgagcgcgattacgtcgcgatcgatcagcgcggctgagaccggacgggtcgcatccggtccgccggacgcgacccctcttcggctatcggcgttccgcgatgaccctgagcaccgcctcagcagcgcgctcggatgggtcgtggtcgccgcgtcccatcgcctgcaacgcctctgtctgcgccaccgactgactccgggcggcgtcggggtcggtcagcagccgatgcagggcgctcgccagccgttcgggcgtggcggcgtcctggatgaactcgggcgcgacctcacggcctgcggcgatgttgaacagggtgatgaagggggcggtgacgatccgcctggcgatggcgtagctgatcgcgccgatgcgataggcgatgaccatcggcgcgcccgccacggcgacttccagcgtcaccgttccgctggtggcgagggccgcgtcggcggccttcatggcgtcgtacttctccaactcctcgaccaagtgggcgcggaacggccaggcggcgacgcggccgcgcacctccgcatcgaccatggcggaggcgacgaccgcgatctgcagctccggcagctcggccttcagccgcaccgccgtctgctcgtacacgggggtcatccgggcgatctcccccggccggcttccgggcaggatcagcagcaggggcgccgctgggtcgaccgcatgccgccggcgaaacgccgcgccgtccgccgcgctcagatccaggttcagcgcctgcgatcccacgaccgtggtggccaggccttcccgctcgaaccacggcgcatcgaagctgtagagggcgagcaggtgatccgccgtcttcgccagcgctcgggcccgcttcggccgcgacgcccagacctgcggccccacgtatttaatcaggggcgtgtccggcgacgccttgcggatcgccttgccgacgcgggaggtgaagccccagctgtcgatcagcaccacggcgtccggccgctccctcgccgccagatcggccgtctcccgcacccgccgccgcacgcggccataggcggacagcgcttccgtgacgccgacgatggcgagttcggcgatatcgaacgggctcgccacgccctcggccgccatccgggaccctccgattcccacaaaggcgacgccgtcgccgagccgcgccttcagcgctctcgcaagccccgcgcccagggcgtcgcccgacgcctcgccggcgaccagcatgatcttcaccgcgcctggccccagacgaacaggcccaggcgatcggcggcggcgatgatggcgggccggtcgatcaggatcagccgtccttcgacgccggcgacgcccgaaaggcccgcctccgccgccagttcgatagtgcgcgcgccgatcaccggcatgtcgacccgcagatcctggatcggcttgggcgctttcgccagcactcccttgcggtgctcggccgagccgcgcagatcggccgccaatccggcgacccgccgcagcatggcgtccgtgccctcctgcgcctccaccgccagcaccaggccgtcgcagacgaccgccccctggccgatgtcgaggtcgccggagcgctccgccacatgcagcgccttgatcagatcggccgtctgttccggcgtgggtcggacccgccccagcgcacccgccgacagtgtgtctccacccaggatgtcgtcggcgccctcaaccgagaagccttcgccctcgaacacggacagtatcttccgcagcagggcgtcgtcgccctgcccggccgccttgatgatgccgggcagcagcgtcgcgcccttgaagtccggcttcaacgtcttgaaatccggccggctgacattgccggccaggcagaccgcctcgcagcccgcccgcttcatcgccttcagtatgccgccgatctcggccatgccgaagtccgcgccgggccagcgcgccagcgccggatcggcgaagcccgccaggcggatgacgaacagttcccgcccctcggcctcgcagcgatgcgccaccgccagcggcaggtcgcctccgcccgcgatcagccccagccgcctcattcgcccggcaggcacagcggccgcttgccgccctcgcggatgaaggcgacgatttctgcgatctccggcagatcggcgtaggcgtccgccaccctctcaatccgacctgcgaactcgcccgatccttcgaacaggtcgcgataggccgccagcagccgccgcagctggtccttgccgtagcccttgcgcttcagcccgatcaggttcagcccgtgcagccgcgcgtggttgccccaggcagagccataggggatcacgtcgcgcgtcaccgccgccagcccgccgacgatggcgccctgccccacgcggccgttctggtgcacggcgcacagcccgcccaggaagacgcggtcgccgacatgagcatgcccgcccagcgtcgcattgttggccatcaccacatcgtcgccgaccacgcagtcgtgcccgacgtgcgcgcccgtcatgaataggttgttcgaacccacgaccgtaacgcccgtcccctgcggcgtgccccgattgaaggtgcagtgctcgcggatcaggttgttcggcccgatctccagccggaccggctcgcccttgtagccgttgtgctgcggatcgccgccgatgacggcgaacgggtggatggcggtgccgaccccgacatcggtgtcctgctgcaccaccacatggctgatcagccgcacgccctgcgccagcacgacgttggggcccaccgtgcaccaagggccgatctcgacgtcgtcggcgatccgggcggaggcgtctacgatggtggtggggtggatgctcatgcggacgccggttggtccaccttgaccaccatggccatgaactccgcctcggccgccagcttgccgtcgatgaaggtctcgccgcggaacttgtaagcgtcgccgcgcgccttgatcaccttgacctccatccgcagctggtcgcccggccgcgcgggctttctgaagcggacgccgtcgatggacatgaacatgatgaccttgtccgccaccgccacgtccagcgtcttggacatcagcagcgcgcccgtctgcgccatcgcctccacgatcagcacgcccggcatgacggggtcgatcggaaagtggccgggaaagaagggctcgttgtgggacacgttcttgacgccggtgatcgaggtcgccgggacaaaatcctccgccttgtcgaccaggaggaacggatagcggtgcggcagccgccgcatgacctcggcgtagtcgatcttgccgtccgcttcgctcatgattccctgcgtcccttgcgtgaagagacctgtttggcgagccagaccgcctcgcgcaaggactggcggatcggcttggcgggatagcccgaccaggtctcgcccggcggaatgtcggccagcacgcccgctccggccgccactcgcgcgccctcgccgatggtgatgtgatcgccgacgccggcccgtccgccaaacatgacgttgtcgcccgtcgtcacggagcccgagatgccggtgtgcgccgccatcaggttgttgcggccgatgacgcagttgtggccgaccatcaccagattatcgatcttggtgttctcgccgatgacggtgtcgtcataggcgccgcggtcgatgcagctgttcgcgccgacggtgacgccgtcctgcaagatcacgcgccccagttgtgggatgtcgacgggaccgcttcgcgacgcggcggcgccgaaaccggcctcgccgatccgggcgcccgacaggatcttcacccggtctccgatcagcgcaaagccgatggagacgttcgagccgatcaggccgtcgcggccgatctgcacgccggggccgatcacggtgttggcgccgatccgcgtcccgcgcccaacgcggacgccctcgcccagcactacgccgggaccgatccggacgctgtcgtcttcggcggcatcttccgcagggaaggcgacgtccagcatcaccggcaggtgcagcagcgccgaggcgcgcgcccagctggcctgcggctcggtcgagacgatcaccgccgctttggtcggcgcggcctccgccgcagatggatgcacgatcacgcagccggcccgcggctcggccagttgagccgcgaacttgcggtcgcccagaaacgcgatcgcgccctcgtcggcggaggacaagggcgcgatcgatcggatgatccgctccccgccccttccgacctcgcctccgatccgcgctgcgatatcggcgacggagagcggctggagcgtctggaagaaacggggatcgggcatgaagcgcttagttggcggccgcggcggcgggctgctgcgccggcacctgcaggcggttgaagctcagcgtcggcagagcggtgttcaggcgctggatcgccaggtcggtgatgtcgtgcgccgggttcatgatgaaaacgctttcccggtcgatcagcatgccgcagccgcgctcctggtaaacggcgaccaggatcggcgacagggccgtggtgatggcctgacgctgggtggccagggtgtagcgcagctcgttctcacgggtggcttccagctgctgcgcctcctgggcgcgctgctgcagggcctggcggcgctgttgcaactggtcggccggcaggctggcgcccgaggtctgcagcgactgagcttccgtctggagttgctgcgcatagggcgcgagctcgccctgaacttcctgcgctagctgctgcatgcgcgcatcgaccgcctggccgacgctggactgggccaggaggcgggcgttgtggaacacgcacaggccggggatctgcgggcccgggttctgcggttgggcgggagcggcggcctgctgcgccgaggcggtcgaagcgatgagcgaggcggcggccgtcgcggcgatgatcagagacttcatgacgtttccttgggtgcgagcggttctggcttgcggtttagaactgggtggaggtcgagaagcggaagctctcggtcttgtcgtagtcttccttggcgaggaccttggacaggtcgaagcggatcggccccatcggcgaacgccagtggatgctgacaccggctgaggcgcgcagcgacgcctcgtcggcgatggtggtgtcgcgcacgccctgttcggtcagcttgtagcgatcatcgaggctgctgagcgtgccgacgtccgcgaacagcgaagttctgatgccatactgctccggcaggaagttcggcagggtcagctccaccgtgccgatggcgtagaagttgccgccgagagcatcggtggtggtcagatcgcgcggccccatgccggcggtctcgaagcctcggaagctgttgccgcccttgaagaagcggtcgctgattcgaatggagtcgccgttccagcccgagatatagccggcctgcccgcgcacgctgaccacccaggacggtgtgatgccgtagtaccaggtcgcgtcgccttcggtcttcagatagttcacgtcgccgccgagacccgccagatcctggatcagcgagccggaccagccgcgcgtcggccgaatcggatcgttcagatagctgacctgcagggtgtagccgaccgacgagttcaggaacgagccgatctggtcgcacagcgccgacgagccaagcccgcccgtgcttgaacagaagttgttcggcacgatgatctcgtcatccttcaggaagtagcgcgcgctgaacagggcgttctggttcagcggataggacaggcgcaccccggcgccggtcgagcgatagtcgtaggacgaatattcgctgagatcgtagcgcgagtggaacaggtcaaagcctgcgcgcaggtcgcgacccaggaacttcggctcggtgaagcggaagtcgacctgctggcgcagggagccccactccaggcgcgccaccacgttctggccgcgaccgcggaagttgcgctcgctgatgccgaggttgacggtgaagctgtcgaccgagctgaagcccgcgccgacggacagttcgccggtgggctgctcctgcacggtgacgttgacgacggaccggtcgggcgccgatccctgcgtctccgcaaccgtcacgtccttgaagaagcccagcgcccgcagattgttgcgggaccgctccagcagcgcgcggttgaaggcgtcgccttcggtcagcacgatctcgcggcgaacgacgggatcgatggtgcgcgtgttgccgaccacattgatgcgctcgatgtagacgcgctggccttcggacacgttgaaggtcacgtccaccgtgtcggtgtccggattggcgcgataggtcgggttgatgtcgacaaaggcgtagccggccgaacccgcggcgaaggtcagggcgtcgaccgcctgctcgatcttgtcgctctggtagaggtcgccgctacggatcggcaccagcgccttcaggaagtcggcgttcaagcgctcgttctcggtgacgacgctgatctcgccgaagttgtagcgatcgccttcgtccagcgtcagcgtcagggcgaacgccttgtcgtccggctgtagctcggctaccgacgagatgatgcggaagtcgtagaagccgcgattggtgtagaacttgcgcagctgctcctgatcgtactcgagccggttcggatcgtagttgtcgttgttggtgaagaacttccaccagcgcgagcgctcggtgaccatgacgtcgcgcacgtcattgtccgaaaaggcgcggttgcccagcacattgatcgcgctgatgccggtctgcggcccttcatcgatctcgaatacgacgtcgacgcggttctgctccagctgcaccagctttggcgtcaccgtggctgagatgcggccctgcaggcggtacagctcaacgatggagcccacgtcctcctgcaccttggcgcgcgtgtagatgccgcgcggcttcagcgtgacctcttcgttcagcttgtcctcgcggaccgcgctgttcccctcgaacaccacctggttgatgatggggttctcgacgatctggacgatcaggtcgccgttctgcacgcccagctgcacgtcggcgaacaggccggtgcggttgagcgtgcgcaccgcaacgtccagcaccgccgcatcgaccgtgtcgcctggctggatgggcaggtaggacaggaccgtggtctgatcgatccgctgtgtgccctgaaccaggatccggttgacgcgcacctgctcgggcgcggcggcggtcgccacgccctgggtcgcgccttgggcggccgcacccggggctgcaggcgcttgcggcgcaggcggggtggtcgccggagcggcttgcggctgaggcgtcgtcacccgaggcgcggccgtctccgccgtcgtgccggaggacggcgtggggcccgacggcgtggggttcaccaccggcgcaggcgcggccgatccggagttcgacggaatggcgaccggcgcggtctgggccagcaccgggctggacaggccggcggcgatcacaagcgcgaccatgctggaacgagcgccgaggcgggcggaggcgctggggatcatctgggtcattcgggaaaccatcgggggctggcgtcggctcaactgacgagcccgccgaggaatttgaacaggttaagcttctgcaggtcgttccaagtcgcgaacaacatcaatcccgccagcaacgcaagaccaacccggtagcccgcctcctgataccgtgcggcgaccggctgccgcgccacggcttcatagccgtagaacaacaggtggccgccatccaggatcgggatgggcaggaggtttagaaagccgattccgatcgaaagtatggcggcgaagcttgtcagcgtcagcagcagattggccgcgatcgcccagggatggggattggcgtccaccgccgcgttggtcagggcgcccgaggccttggcgatgccgagcgggccgctgagctggtcgcccgactcacgcccggtcacgatgcgtccgagataggtcagggaggtgctgagtaccgccccggtctcctgcacgcccttggctgcggcctccatcggattgtagcggacgtggcgcacgtcggcgcgcgaggcgccgagccccagcccgatgcggccgatgctgacgcggccggcgatggggtcctcttcgacccgccgctcgggcgtggcgaccagttgcaccacggcgccgccgcgctccaccgtgaagcgcaccgggtcgccgctggacagcgacaccacgcgcgtgacctccgacccgtcctcgatggcgcgcccgttcacgccggtgatcaggtcgccgtccagaaaaccggcggcggcggccggcgagttgggctgcacctggatgacgcgcgcgggcgtcatgctgacgccgaccacgctgaacagcacggtgaagatggcgatcgccagaatgaagttcgccgccggccccgccgcgaccaccagcgcgcgctgccacaccggcttgaagtgaaagtagtcgcgctcggcgcccgcgccctcgcgcgcgatgatgtcggccttcagcgcatccagcccccgccgatccggcacgctggaggcgtcgaggtcgcccgaaaacttgacgtagccgcccagcggaagccagccgacccgccactccacgcccttgcgatcgacgcggcgaaagacggtgcgtccgaagccgatggcgaaccggtcgatcttcacgccaaaggcgcgcgccaccgagaagtgacccagctcatggatggtgacgatcgccgtcagcaccagcaggaatggcacgacataggtgatcacctgcgtcagggcgcccagcatgctcttgtccgtctcccctgtggccgatcaggccgcgatcgcgagcgtcgacacgacgccctcggcgatccgccgcgcctgcgcatccaccgacagggccgaggcgcaggcgtcgccggcgccgaaggcaaggccctcgcgcgtcgaacgatcaagggtttcggcgacgactgcggcaatattgagaaagcccagccggccgtcgagaaaggcccaggccgcgacctcgttggcggcgttgaagatggccggcgccgctccgccttcggtcagcgcctgccgcgccagggacagcgccgggaagcgggtctcgtccggcgcctcgaacgtcagcttgcccagcgcggcgagatcgagcttgggcgccggccaggcgatccgctcgggccaggccagggcgcaggcgatcggcgtgcgcatgtccggcggccccatctgcgccagggtcgagccgtccacgtattcgaccaagctgtggatgatcgactctgggtgcaccaccacgtcgatccgctcgggcggcataccgaataggtaggccgcctcgatcatctccaggcccttgttcgccatggtggcgctgtcgaccgagatcttggcgcccatggaccagttcggatgcgccaccgcctcgcgcggcgtcaccgcccgcatccgctcgagcgatgtctgtcggaagggccctccggacgcggtgagggtcagcttctcgacctggtgcggcgcatcggcgggaaacacctggaagatggcggaatgctccgaatcgaccgggatcagccggccgcccgcgtcgcgcacccgctgcatcagcgcgggtccgcagcagacaaggctttccttgttggccagcgccagcacgcccccgttctccgccgccgcccaggccgaccgcagaccggccgagccgacgatggaggccatgatccagtcggatggccgcgcggccgcctcgacgatcgcctcgtcgcccgccgccgcctcggtatccgtgccggccaaggcgtcgcgcaactcgcccaggcgcgagggatcggccgtcaccgcgatcccgggtttccagcgccgcgcctgttcggccaggcgcgcgatgttggcgccgccggtcagcgcctcgacctcgaatgcgcccgtgcccgtctcctcagcccgcgccatcaggtccagcgtcgaggatccgacggagccggtggatcccagcacggtgacacgcctgcggatcacgccgtacgctccagcatcagaacgatcaggcgccccgcggacaccaccaccacggcgaacatcatgccgtccacacggtccagcagcccgccgtgaccggggatcagcgagcccgcgtccttgacgccgaagcgccgcttcagcgccgactcccacagatccccgcccatggtggcgagcgccgcagccaggcccagaaccgcgccccagaacacatttagccgccccatctccagccaagcggccatgccggcgccggccagcgtcccggccagcagacccccgatgaaaccggaccaggtcttgttgggagaaaagcgcggccaaagcttgggcccgcccaacagcgagccgaccagataggccatgatgtcggaagcccaggccacggcgaagaccagcaccgtccagtgcaggccgatcgggttgtcgacgtcgcgcagccagatcagcagcaccgccggccagccgaggtaaagcaccccataggcggcgttgaccgcctcctggccccggctgcgggcgtaaagtcccgccgccgccgcgccgaacaccagcatgacgaaggccacggacatgacgccgaaatgggcgctgaccaccccggcgatcagacccagcgccaccgcgacggagaccgtgcgccaggcggcgggcgcgctcatcatcgcccattccgcggccagcagcacgcaggccaggatcatcagcgccaggaaccagacgcccccggcccaggtcgccagaaccgcggccggcgccagcaccacggccgacgcggtcctgagacctatgtcgccgaccttgatcgccatcagcccgccacacgcgcgggcgtcgcctgcaggccgccgtagcgccgctcgcgcccgccgaactgcgccaccgcctcggccagcgccttgggcccgtagtccggccacaggatgtcctgaaacaccagctcggcataggcggcctcccacaggaggaagttcgacagccgctgctcgcccgaggtgcgcacgatcaggtccagcgggggcgccgacgccgtggcgaggttgtcctgcagcgcctcttcggtgatcggccccaccggctcgccggccatcagccggtcgatatgcttctgcgccgcgtccaccagatcggcccgcgcgccatagttgaaggcgacctgaagcaggaaacggtcgttgtccgccgtctgggcctcggcccgctcgatgatcgcggcgatgtccgcgggcagtccgcggcggcggcccaggatgcgcaggcgcacgccctcgcggtccagccggttcaggtcgctggccacataggaccgcaccagacccatcaggtccgacacttcctcttccggccgcgcccagttctccgtcgagaagccgaacaccgtcaggcactggatgccgaggtccggcgccgcctggagggtgcgcttcagggcttggaccccctcgcggtggcccatggcgcgcggcaggccgcgctgcttggcccagcgtccgttgccgtccatgatcaaggcgacatggcgcggtcctgcaggacgcgagccggcaagaggcgcggcggtcgtggccgtcatcgtgttacgcgtcccttgtccggcctcatccgcctcagacctgcatgatctcttgttccttggccttcaaggtctcgtcgatgcgcttgatggcggcgtcggtgtccttctggacgtcggcctccatcttcttttgctcgtcctggctgatctccgacgccttttcggccttcttcaggtcgtcgttggcgtcgcgtcgcacattgcggacggcgatcttctgctgctcggcgtatttgccggccagcttgaccaggtccttgcggcgctcctccgtcagcggcggaatggggatgcgcagggtctggccgtccacgatcggattcaggcccaggcccgccgcgcggatcgccttttcgaccgacaccaccatgcccttgtcccagacgctgaccgagatcatgcgcggctcgggcacgctgatggcggccaccgcgttcagcggcgaggtcgagccataggcctcgacctgcaccgggtccagcaggccggcgttggcgcgtccggtgcgcaggccggcgaagtcgtccttcaacgcggcgaccgacttgtccatgcgatcgcggtaggatttcaggtcaggcttggccatgggatcagcgtcctcttttttgcagtcttgcggccggtcaggccggcgtgtcggtgatgaccgtgaacgtgccttcgcccgtcagggtccggcggatggccttgtcctcgcggatggagaagaccacgatcggtatgcccgtgtcgcgcatcatggcgatcgccgatgcatccatcacgcgcaggtccttggccagcacgtcctgataggtcagggtttcgtagcgggtggctgacgggtccttcttgggatcggccgtgtagacgccgtccacgctggtgcccttcagcagcgcatcgcaccccatctccgccgcacgcagggccgcgcccgagtcggtcgtgaagaagggcgcgccgacgccggcggcgaagatcaccacccgtcccttctccaggtgccgcaatgcgcgcctgcggatatagggctcggcgatggcggccatcgggatcgcgctctgcacccgcgtcgagacgccaatcttctccagcgccgactgcatggccagcgcgttcatgatggtggccagcatgcccatgtagtcggcctgggcgcgctccatgcccgccgccgccttggacaggccgcggaagatgttgccgccgccgatcaccaggcagatctcgacgccctcgcggacgacctcggcgaccgccgccgccaccacgtccaccgtcttcatgtccacgccaaaggactgatcgcccatcagcacctcgccggacaccttcagcagcacgcgcttgtagcggaactcggcgggggcgtcgggcatgcaggataatccgtgaactgcggcgccgcgcgggaatcgggcggctccatataaacgaagggcgcgccggccttcaaagccgaacgcgcccgaatgcgtatttctcctccctgttcgcgcagcgcacggggaggtggatcggcgcgcagcgccgagacggaggggcttgtccggcgttggaccgtcacccctccaccgcttcgcgcggccccctccccatcggcgatggggaggatctggaccttactggccgcccatcatggaggcgacttccgaggcgaagtccggtccttcgaccttttccacgccctcgcccagcgccagacggacaaagccggccagcttcaggttcgccgaacccagctccttgcccgagttggcgaccagctgctcgatggtcacgtccgggtccatcacgaacggctgcttggtcagcaccacgtccttctggaacttggcgatctggccggacacgatcttgtcgatcatgttttccggacggccttcttccttggccttttcggtcaggacctgacgttccttttcgatggcggccggatcgaggtcgtcggtgttcagcgacagcggcgaggtggcggccacgtgcatggcgatcttgcggcccagctcgcgaagcgccgccttgtcgcccgcgccttccagcgcgaccagcacgccgatgcggccgacgcccggcgacacggcgttgtggacataggtggcgacgacgccttcttcgaccgacaggcgggcggcgcgacgcagctgcatgttctcgccaatggtggcgatcatgttggtcacttcgtcctggacggtcttgcccgtctccagctcggcgccgtggagcgcttcgatcgagtgatgctccaggcccagttcggcgaaacgcttggcggcgttctggaacaggtcgttgcgcgcgacaaagtccgtctcggcgttgaactcgatggcggccccgacttcgcccttgccgtcttcacgcgaggcgacggccaccaggccctcggcggcgacgcggtcggccttcttggcggccttggacaggcccttggcgcgcagccagtcgatggcggcttcgatgttgccgtcgttttcctgcaaggccttcttgcagtccatcatgcccacgcccgaacgctcgcgaagctccttcacgagggcggcggtgatctcggccatgttcttctcctatgggattcgtatgcgggaacggccggactgacttagcccggccgtgtaacagttcaacaggcggcgctcacagggcgcgcgccgcctgaaaagcgcgatcagcccgtggcctgctcggtctcgacggcgtccagcgcctcggtgttggccgaggtgtccgcgctggccagcagttcgtcggcggcgccttcggttccggccggcgcggcttccgcctcgaccggagccgaagcttccgccagcatcggctcgaccgggttctccgacgcgcccaggtccacgcccgacgccgaagcgcccgcggccaggccgtccagcacggcgtcggcgatcaggtcgcagtaggtctggatggcgcgcgcggcgtcatcgttgcccggcaccggataggtgatgccgtccggatcggagttggtgtccaggatggcgatgatcgggatgttcagcttgcgggcttcctggatcgcgatcgcttccttgttggtgtcgatcacgaacatgatgtccgggatcgaacccatgtccttgatgccgcccagcgacagctccagcttgtccttttcgcgctgcaggttcagcagctccttcttgacccgaccctcgccgccgttctcaagaatgccttccagctcgcgcaggcgggcgatcgagcccgacacggtgcgccagttggtcagggtgccgccgagccagcggttgttcatgtagtactgggcgcagcgcttggccgcttccgccaccgggtccgacgcctggcgcttggtgccgacgaacagcacgcggccgcccttggccgccacgtcgcgcacggcgaccagcgcctggtggaacagcggcatcgtctgcgacaggtcgatgatgtggatgttcgagcgcgagccgaagatgtagcggtccatcttcgggttccagcggtgcgtctggtggccgaagtgagcgcccgcttccagcagggtgcgcatcgagaattcaggcagagccatgatcgttcagtcctttttccgatcaacgtggcgcgggcgataaaaggaccggctggtccctcggaatggagcggatcgggatgtctccccgaggcgcgccacgcccgcgttgcgaaatgcggggccgatgtagtcgggatcggcccgcaaggcaagctggataggaaaagggcggcccttgcgagccgcccttcccttggctgatcggaagatcagttcatggcgttgcgcagttcctgcgcgcgctgcaggtgcatctcgatcttggggaccacttcgcgggccagagcggccagttgcggcgtctccgtgtggtccgagaagccgcggtgcagcgtcagggcctcgttgtgcgcggcgatctgctggtcgagatagacgcggtcgaagtccgccgcagaagccgcacgcagattgtccagcatgcccatgcgccgctggtcgagcgcggtcggaatggcgacgttcggcgcctcggccggcgcacgctgcttcagcatggcggtggaggcggtgtgatcggtggtgatcatctcggccagcgccttgacgtcggcgttggtcgacttctccatcgcgatcttggaggattcgatctcaaacatgtcgcccatggcggccgacggcacataggagtccacggtgttggcgcccagggtggctgcggacgtctggcccacggcggcggatgtcgcgtcctgcaccgcgttgaccggctcggtctggcccggcgactcggcgttctggttgcaggcggcgagcagcgccaccgaggcgacgctgatgatggcgatctgtttcattgaaaaggtctccctatggttcaggcagaacccttcacgcgcccgtgaagttccgaaatcattcgcccgaaaggcgatactccagatcatacagatgccggccgtctccgatcttcaggtgaaagacgccgctgatcccggccagatcaccgtctcccgagcctggaacgatcgtgatcgacaggtcctgcgcgccttggtccatgatcccgcgatgcaccagcatgaagccgcccgaccgaccatccagcgttccgttcacccgctccatcgccacataggcgccggactgctccgcgttcagaaccgcaagcatctcgccggcccccgtcccttccagtccgccccgaaaggtcttggccaggatcatgcggccgggcccgcccacaggggagtccgcgccgggctccaccggcgtcatcttgacgtcgaactcacccgtcgcatgccgcgccgcctcagccgattgcgtcatctccgccgtcttcccagttccgccgcccgccacgatcagcgacagcgccatgacccatcccaacatcaggcgtcctccagcatgaccacgcccggcgcggacttcagcgccccccgcagcgccccgtccagcttgtagcggcccggcagcttcatctcgacctcgcgccccttctccagcgaggcgatcagcgagatctccccgcccttgccgatcgcgcccgatcgcgcccttcccagccgggcgcgcagggccgccgcatccgccgatcgcgccgacacatggatgcgcaggccgatgcccgcgtcgtccagcagtccctccatgcggctggcgtcgtcgccgaagaagcgcacctcgccgtccgacgccttggcccgcaccttgaccatcaccgatgcgcccggttccagcacctcgcgacaccgacgcagctgctccggcggaaagaggcattcgaactcgccggtggggtccgagaaggtgacaaaggcgaacttctcgccggtgcgcgcgctggcgcgctcctgccttctgcgcaccacgccggccatctggaaggcctcgtgcccggcctcggcgcgctgcacggcctcggccacaaaggtcacgcgcttgcgacgcagcgccggctccatgtcttccagcggatggccggacagatagaagccgaccgccgccaattcctggtccagccgctcgggaccgacccagggctccacgcttttcagccggggccgtgcggcatgggcctggtcgccgccgaacaggctgacctgggcggaggcgcgttcggccgccacgctctggcagtaggccatcagcacgtccgcctgctcgaccagctggcggcggttcgggtggatgctgtcaaacgcgccggccttggccagcccttccagcgcccgcttgttgacgcagcgcggatcgacccgctccaggaagtcgaagatgtcggcgaagcggccgccctgttcgcgcacctccaccacatggcgcatcgcctccagccccacgttgcggatggcgcccagcgcatacagcaccgccccttgcccgttctcccatgacacgtcgaagtcggcgctggagcggtttacgtccggcgctcgcaccggcacctcgaaccggcgcgcgtcctgatagaagaccgccagcttgtcggtgttggacaggtccagactcatggaggcggcgaagaactccaccggatggttggccttcagccagccggtctggaacgaaattagcgcataggccgccgcgtgcgacttgttgaagccgtagcccgcgaacttggccaccaggtcgaagatgccgccggactggctctcggacacggacttctcggatgcgcccttgatgaagcgcgcccgctggaaatccatctcctccttcttcttcttgcccatcgcccggcgcagcaggtccgcctcgcccagcgaatagccggccaggatctgggcgatcttcatcacctgttcctggtagatgatgacgccgtaggtctcggtcagcacctccgtcaggctggggtgcagatagtcgacctcggcccggccgaacttgcggtcgatataggtgtcgatcatctccatcggcccgggccgatacagagagatcagcgcggtgatctcttcgatggagccgcaccgcatcttgcgcagggtgtcgcgcatgccctgcgattccagctggaacaccccgaccgtctggccggacgccatcagctcataggtgcgctcgtcgtccaacggcagctggttccatgacggctcagccccccgccgcgccagatagccgtgcgcccggtccagcaccgtcagggtcttcaggcccagaaagtcgaacttgaccagccccgccggctcgacccacttcatgttgaactggctggccgggatggtcgagcgcgggtcctggtacagcggcaccagttcggtcagcggccggtcgccgatgacgatgccggcggcgtgggtcgaggcgttgcgataaagcccctccagctccagcgccgtctccagcagcgccttgacggaggcttccgcgtccctcgcctccttcaggcgcggctccaggtcgatggcctgggccagggtcaccgggttggcggggttcgccggcaccatcttggccagccggtccacctgccccagcggcatctgaagcacccggccgacgtcgcgcagcaccgcccgcgcctgcagcgtgccgaaggtgatgatctgggccacccggtccttgccgtagcggtcctggacgtagtcgatcacctcctcgcgccgctcctggcagaagtcgatgtcgaagtcgggcatggacacccgttcgggattcaggaaccgctcgaacagcaggccgaaccgcaggggatccaggtcggtgatggtcagggcccatgcgaccagcgagcccgcgcccgagccccgccccggcccgaccggaatgccgtgctgcttggcccacttgatgaagtccgacacgatcaggaagtagccgggaaagcccatctgctggatgatgccgacttcccactccaggcgggtccagtattcctcctcgggcgcggcgggcgtgacctcggtcaggcgaaccttgaggccctcgcgcgcctggtgcgccagctcgtcgggctcggagcgcccggcgccggtgtcgaaacgcggcaggatcggcttgtgcgtcttgaccagaaaggcgcagcgacgcgcgacatccagcgtgttgtcgcaggcttccggcaggtcggcgaacagcgcgcgcatcgcctcggccgacttgaaccagtgctcgcccgtgacccggcgtcgttcctcctggccggtgaaggccccgtcggcgatgcacagcagggcgtcgtgtgatttcgcctgggcggccttggcgtagtagacgtcgttggtggcgaccaggggcacgtcgttgtcataggcccaggcgaccagcccccgctcggcgcggcgttcgtcgtccagaccgtgacgctgcagctccacatagaagcggtcgccgaacgcctcgcgcaatgcagccagcgccgcatgcgcctcttccgtcttgccctggacgaacagcggatcgatgggtccgcacggaccgcccgacagcaggatcagcccatcggagcgcgccgcgacctggctccagtgcacgcccggctccgccatctcgccggcgtcgaggtaggcggcggacgacagggcgcacaggttcagccaccctgtctcgttctgcgccagcagcaccacggtcggcgtcttggcccagcgtgcgttcacctgcccgccgatccccagcaccggcagggcgcaggccacgatcggctggacccccgcctccttggcggtctggctgaactcaagcgcgccgaacagattggcgcggtcggccaccgccacggccggcatgcccgcatccgccgccatgcggccgatcttgccggccttgatcgcgccttccagcagcgaataggccgagcgcacccgcaggtggacaaagccggattgggcgggatcggacacggctcacctcatgcgcagatgcgactcagaccgtcagcagagccgcctgccagaccatccagacaaagccgccgcacgatgcaagcgacagcatatccctcatcagacgcggcatggccttatccccagatcaacctgtgtgttccgggaatgttctatgttccgcttccgttctcgtcaagcaggcttgttctagtaggcgtggctctcggccgcgcgctgttccagatgcccgtccttcaacgcgaacacgcggtccatgtggcccgccagctccatgttgtgggtggcgatcagggcggcgacgcccgtggtcttggcaagggtgcgcagcgcctcgaacaccgcctggctggtggcgggatcgaggttgccggtcggctcgtcggcgagcagcaggcgcggcttgttggccagcgcgcggacgatggcgacgcgctgctgctcgccgcccgacagttgcgccggctggtgcgtcagccgctcgccaaggcccagcgccgtcagcgtctgctccgctcgcctgcgcgcctcggcctggggcaggccggcgatccgcatcggcagggcgacgttatcgcgcgcgtcgaactcgggcagcaggtggtggaactggtagacgaagccgatgcgcgacaggcgcagccgcgtgcgcgtgcgctcgtccagcgcgccgacattctcgccgtcgatcatcaccgtgccgctcgtgggccgctccagcaggccggcggcgtgcagcagcgacgacttgcccgagcccgaagggccgatcagcccgaccagctcgcccggatgcacgtcgaggtcgacgcccttcaggaccgtcaaaccgccctgggccgtcggataggtgcgggtcaggtcccgcacggacaggaccggcgacttactcatagcgcagggcctccaccggatcgatgcgcgaggcccgccaggagggcggcaggctggctatgcagctcatcagcagcgcccagaacgcggtccaggtcacatccagcggatcgaccagggccggtatgctgtcgagcatatagacgtccgagttgaacagttgcacgcccagcaggccttccaggaagtgctggatcgaggcgatgttcaggcagaacaccagacccagcaccaggcccgccaccgggcccgccacgccgatcgccgcgccggccatgaagaagacgcgcaggatcgacgacggactggcgccgatggtgcgcaggatggcgatgtcgcgccccttgttcttcaccagcatgacgataccggaaatgatgttcatggccgcgatagcgacgacgaggcccaggatgatgctcatcgccacccgctcgacccgaagcgcgccgtagaaggcggccaggcggtcgcgccagtcggtgatggcggcgccggggcctgcggcctcgcggatcggctggatcagctgaccgacctcgtcgggcttcgccaccttaacctcaagcgcgtcccacacgccctccttgccgaagaacagctgatgctgctccagcggcatgaagataaaggcctggtcgaactcggaggtgccggagctgaagattccgccaacgatgtaggtcttctccagcccgccgagattgccgaaggcgctgtccgcgcccgtcggggaatagagggtgatcggatcgccgacccgcacgccgttggcctcggccatggccttgccgatcagcacgcggtcaccgccgtaggcgccttggccgaagctgcgacgcgcctcttccgacaggctgcgatagacgtaggtgttcgccggcaggtcctgaggccgcacgcccttgacgatggccccggtcgtgaagccgccgacgcgcaccagactttgcgcctcgttcagcacggacacgctgaccacgccggggacctcggagatgcggcgcaggcgcgcctcccggtcttcggagaccagcacggacccttgcacatacatgtggccgttgaagctcagcatcctgtccagcagggtggagcggaagccggccatgatgctcatcacgctgatcagcaccgcgacggccagcatgatgccgatgaagctgatcaccgcgatggtggcgacgccgccttccttgcgctttgcgcgcaggtagcggagcgccagcccgacctcccaggccgaaaaggcgcccgcgggtttgccggacggggacgcggggccgctcaagccgaaagcctcagcagggcgtcttccagcgacaccgagaccttttcgccggtggcgcggcgcttcagctcgaccacgccgtccgccagtcccttggggccgatggtcagttgccagggcacgccgatcaggtcggcggtggcgaacttgccgcccggccgctcgtcggtgtcgtcgtacagcacgtccttgcccagcgcctccagccgagccacggcgtcctcgcacgcgcccgacaccgccgcatcgttggcgcgcaggttgatgaccaccacgtcgaagggcgcgaccgagtccggccagacgattccgccctcgtcatgactggcctcgatgatggcgccgagcaggcgagacacgccgacgccgtagctgcccatgtgcaccggccggtccacgccgtcgggacccgccacgatggccttcatcggcgcggaatatttggtcccgaagtagaagatgtgcccgacttcgatgccgcgcgccgacagccggtcgtcctcggcggtctcgccttcgaaacgggcggcgtcgtgcatctcctcggtcgcggcgtagagcgcggtgcgctcgtccacgatcgactgcaggtcgttccagtcgacgtccgcgcccggcgccggcatctccaccagcttgcggtcgcagaagacggcgctttcgcccgtttcggccagcacgatgaactcgtgagacaggtcgccgccgatcggaccggtgtcggcgcgcatgggcacagccttcagccccagccgcgcgaaggtgttcagataggctgtaaacatgcggttgtaggcccggcgcgccgccgcctcgtcgatgtcgaacgaataggcgtccttcatcaggaactcgcgcccgcgcatcacgccgaagcgcggccggcgctcgtcgcggaacttccactggatgtgaaacaggttcagcggcagcgacttgtagctcttcacataggcgcggaagatgtcggttatcatctcctcgttggtggggccgtacagcagctcccgctcatgccggtcggtgatgcgcagcatctcggggccgtaggcgtcgtagcggccgctctcgcgccacaggtcggccagttgcaaggtcggcatcagcagctcgaccgcgcccgcccgctcctgctcctcgcgcaccacgcgctcgatcttgcgcagcacccgcaggcccagcggcagccaggcgtagatgccggcggcctcctgcttgatcatgccggcgcgcagcatcagctggtgcgagacgatctgcgcgtccgaaggcgcttccttcagcgtgggcaggaaatagcgcgacaggcgcatgggcggggaatcctggaaaggcgagacgaacaccggctttagccggtggacgggggcgaaagctaggccgggcccctacaggttcggcgcgacgcgcgaaaagtccggcaggggcagccagccggtgtagatcaccagcatcaccacgatccaggcgatggccgagacccaggtggtggtgatgaacttgcgcttcaggttcggcgtcgccggcgccccccactgggctccgtccgtcggcggctcgtgcgtctcgcgcgaggtccccagcggcagcaccgcgaacagcacggtccaccacagcaccagatagacgccgatcatggtgacggggccgatgggcatggggcaactccgctgaccggctttgaccacgccggttttcggcggtctaacggatagcgaccgactcgacgagacctccgatgccgcagatcaccctggaattttcaagccgcctggacggagccgactggcgggccgtggcgctggacgtgcacgccgcctgcgtcgacatcgcgcaggccaagctgacgatgtgcaagacgcggctggtccggctcgagcacgtcgtgatcgccgacggcgcggccgaccaggccatggcgcattgcgagatccgcctgctgcccgggtgctccgccgatcaaaaggcgcgcctcagcgaccggacgcttgagcggttgcagagcgcgctggcgcacctgccaagcccggtgtccatctcctgcgaggtgctggagctcgacggcgagacctaccgcaaggtcgtgcgcccggcctagccgcagtccgcgccgaagccgggcgcccgcagcgccagcaggatcgacgatcgctgcgcctgggtgactgcgccggatgattgcagcacgcagccaaccgccgtgttcgaagttggcgccaacaggccgtatcgccgccgctccacctccatccgcgcgcgagagccctgcagcgtggcgacggcgccggcgatccgctcggggtcgtcagtgatacgcgtcatctcatgcagcgcctcgcccgagcttgggaaatcataggcgtcgggatcgtacggcgcgacctcggccgccagcaggtcgggatcgagatcaacgccgaacttggcgttctggctggcggagaaggcgatggccggcccgctctgcggcaccaccaggaaataggcgtgcctgggaaacagcagatagtgcgccaaatacttggtgacgtgcaaccacggcgcgccgtcgggacccagcgcgtgcgcgccgatgtagacgccgggcggaatggcgcgcccgtcgatccgcccgttcatcgaaaggatgcggtcggtcatgacgtggctgagcagaaacacgccgtcgtcggcctcgcgctcgaaatagtcgcggatggcgtcggcgctcggctcgggtcccgggtcccggccatagacgacgggaaaggccgtctccggcatgggacggccttccggcgggctgaaccacagcactcgcagctcgtgcaccgtccgcgccagggggtcctcgccgcgaaaggtcgtcaggctgagggccaggttgaccacggcgaacagcgcgaccagcccggccagcgcctgcccggcgatgaccagccagcgcctccatccttgaaggggatggcgggcctgacgcacccgattcagcaggcgttgaccgcgtccgccgcgtgccgtgttcatcccgcctccctcgcttccacgccgccaaatgcgacgcggcggcgaaggttgcggtcagacgcgcaggaccacggtctccacgatcggccggcgatcccagatctgctggctggccttcttcagggtgcgggcgaccgcctgctcgatgacgtattcgtcctccagcgcctcgcccttcaggccgcgcaccacttgctcgacccgctccgccaggtcatccagcgcatcgcccagcggcgtggccggatcacccggaagaccgacgctgcgcacgtcgatgtcgctgacgatgcgcccgcgcttgtccagggcgaagctgacgatcagcacgccgttggtggaggcgtggcgacgctccttcagcgcctcgccctgctcggtcaccagcatgccgccgtcgacatacagccgtccgttcggcacctcgtcgatgatggcggcggggccaggcgccagacgcaccaggtcgccgttgcgcggcgtcaccgtctcgggcacgcccaggtcggtggcgaggttggcgtgctccagcaggaagcgccggacgccgtgcgtcggcaccgcgatccgcggccgcgcccaagcgtacatctgcttcagctcgtcacggcacgggtggccggacacgtggatgccgggatggtccttttccgtgtagaggcgcacgccgcggtcagccagcttgtcctgcagccgcccgatctgcagctcgttgcccgggatctggcgcgacgagaagatgcaatggtcgcccaggcccagcttgacggtcgggtgcgtgccctcggccacccgtgaaagggccgcccgcggctcgccctggctgccggtgcacagatacaggatctcgtcggccggccagacgcgggcctcctcgtccgacaggaagggcttcacgtcctgcaacaggccgatgtgcttggccgccgccgtgatccggtgcatcgaccggccggccagcgccacgcggcgccccgccgcctcggccgcgcggatcacgctgtccatgcgcgcgacgttggaggcgaagcagcccacggccaccctgcccttcagcccgccgatcagctttgtcagcgcctcgcgcaccccgccttccgatcccgccacgccgtccacgaagacgttggtggagtcgcacaccatcgccagcacgccctcgtcgccgagcgcggtgatcgcgtcctgatcggtgggcgaaccgatcaccggctcgtcgtcgatcttccagtcgccggtgtggaacacggtgcccaggggcgtgcggatggccaggccgttcggctcggcgatcgagtgcgtcaccgtcaccatgctgacctggaacggccccaggtcgatggtcccgccgaccggaacctcgtggatcaccgcctggtccagcaccccggcttcgcgcagcttgtccttgatcagataggcggtgaagggcgtcgcatagatcggcgccttgatgcgcggccacagccagcccagggcgccgatgtgatcctcatgcgcgtgggtcagcacgatggcgcggatgttctcgccctgaagaaaggtcggatcgggcacgatcacgtccacgcccggcgtcgacaggtcgccaaaggtgacgcccacgtcgacgatcagccattctcggttcgcctcgggcccatagccgtaggcgttcaggttcattcccacctcgtccgagccgcccagcggcaggaagacgagttcgtcgttggtttgctttgtcattcagccgttagatgggtgttccgccgccagatttcgagcaggccgcggatggtgagatcagggtcgaaatggtcgatgctgtcggtcgcgccctcgaacagggacgccacgccgccggtgccgatcacggtcatgggcgcggcccattccgccttgatgcgggccaccagcccttcaatcagcgcgatatagccccagaacacgcccgactgcatgttggatacggtgtccttgccgatgatggtctggggcttctggatggcgatgcgcggcagcatggccgccgcctcgtgcagcgcctgcaggctcaggttgatgccgggcgcgatgatcccgccctcgaacgcgccatcggccgccactacgtcaaaggtcgtcgccgtgccgctgtcgatcacgatcaggtcgccgggatagcgcatgtgcgccccaaccgcattgaccagcctatccgcgcccgcctcgctgggtttcaggatgcgcggggccggtccgatgctgacgttctcgccgatcaccagcggctcgacccgaagatagcgccgcgacaggttgcgcaggttgaagatcgactgcggcacgacgctggagatgatgcagccggtcagggcgtcgaagcgcatgcccttcaggtccaccagctggctcagccacacggcgtattcgtcggcggtgcggcgcgagtcggtcgccgcgcgccactgggcgatccactcggccccgtcgtggatggcgaacagcgtgttggtgttgccctgctcgatcgccaacagcatcacgccgcctcgccgaagaagacgtcgccagcggaaatccggcgcagcgtgccgtccgccagcctcaaccgcagcgcgccgtcggcctcgacgccgtccgccaccccttccaagatctcggcgcccagccgcgcgacgcaggggccgttcaacccacgggtgcggtctgtccaggcgtccagcaccggctggaagccgatctggtcccagcgcgcccgccaggccgacacgctgtccacaagacgccccagcgccgcctcaaaggttggcgcttcggttcccgctccgccgattgcggtcgccggccgctcggtttcctccggcgcatgggcaaggttgatcccgatgccgaccgccagccacaggccgccgtccgcatgggcgccgctttcgaccaggatgcccgcgaccttgacgccgtccagcatcacgtcgttgggccatttgatgcctactcgctcgcgggcgacatagccgtccagcacctcggccgcagccagcgccgccacgaacgtcacctgcgccgcctccgcaggcgcacggtgcgtgcgcatcagcagcgtggccgccagattgccgctgtcgctttcccagcgacgcccgcgccggcctcggccttcggtctggcggcgcgcggcgatccacagcggacccgcctcgcccgcttcggcccgccgccgcgcctcggcgttggtcgagtcgacggtctccaggatcaggacgggcggcaggtcgcccaagtcagcgcaggccgaaaccgaccgccgccgtccgcgcagccggctcgatccagggcaaggcgatcagcacgaccggaaacgagaacgccgccgcggcccatgcgatcgacttggcctcgaccggcgacttgtcgaacggaacatcgtccacgggcgcgtcgaaccacatcagcttgatcaggcgcagatagtagaaggcggccacgaccgaggcgaccaggccggccacggccacgcccaccatcaccgggctggcgtccgccgccgcgccgaagacgtagaacttgctccagaagcccgagaacggcggcatgcccagcaccgacagcgacagcaccgtcagcgcaaccgccgtcagcggacgatcccgcttcagccccgccaggtcggcgatccgacgcaccggccgcccgctcttggagagcgacagcagcacgccgaagaagccgaactggtccaccacatacagggccatgaagatcagcatggcctgcaggccgaccgccgtccccgccgccacgcccagcagcgcatagccgatgttgatgatggacgaataggcgagcaggcgctgcaggtccttctgccccaggcccccgaaagcgcccacggcgaacgacagcaccgagatgatcagcagcacctgcgaccactggtcgtgcgactgcgcaaagctgccgtccagcgcgcgcgccatcagcaccatggccgcgaccttgggggcggtggcgaacagggccacggccggcgtcggcgcgccctcatagacgtccggcgtccacatgtggaacggcgccgccgataccttgaacgccagtccgcagatcaggaacaccaggccgaacaccagccccggcgaaggattgtcggcggcgaaggcggcgatctcatcgaagcgcatggtgccggcgaaaccgtagatcaggctggcgccatacagcagcaggcccgaggacaacgcgcccagcacgaaatacttcaggccggcttccgacgccttcaggtcgttgcggtggtaggcggccagcacatacagcgccagcgaatgcagctcgatgccgacgtacatcgagatcaggtcgcccgacgaggccatcatgcccatgccgaccgaggccagcacgatcagcaccggatattcgaacttggcgatgcccgcgcggtgcatccagccgtcgcccaggacgatggcgaccgcggcggccagatagatcaccaccttgccgtagacggccaggctgtcggccacataggcgccgttgaaggcggtccccagcgggccggtcgccgccaggatcgcggccacgaccaacagggcgatcgacagcagcgacacggcgcgcgcgctcttttcgccgccgaatgcgccgatcatcagcagcaccaggccgccgatggcgagcgtcagctccgacgaggcgatgtgaaaggcggaggacagatcaggcattcttcagtctcacccgccgatcgcgacgcgataggcgttggtcagggcctcgacggcgggcccggtgtagtcgaggacggcggcgggatagacgcccagccagatcgtgccgacgatcagcgggacgaacagcagcagttcgcgcttgtcgatgtcggtgatggtctggagcttaggattggtgatctcgccgaacatcacgctgcggtacagcgtcagggcgtagaccgccgagaagatcacgcccgaggccgccaccagcgccgcccaggtcgaggcctgataggcgcccgtcatggtcagcacctcgccgataaagccggaggtgcccggcagaccgacgttggccatggtgaacatcaggaaaatggccgcgaaccacggcatcttgctggtcaggccgccgtagaaggcgatctcgcgggtgtgcatccggtcgtagacgacgccgacgcagaggaacagcgcgcccgagatcagcccgtggctgatcatctggaacaccgcgccctgcatgccctgctcgttgcccgagaagatgcccagggtgacgaagcccatgtgcgccaccgacgaataggcgatcagcttcttgatgtccgtctgacgccacgcgaccagcgacgtatagacgatggcgattaccgacagggtgaacaccagcggccggaacgtctcggacgcatcggggaacatcggcacgttgaacaggatgaagccgtagccgcccagcttcagcaggatgccggccaggatcaccgaacccgccgtcggcgcctgaacgtgggcgtccggcaaccaggtgtgcaccggccacatcggcatcttcaccgcgaacgaggcgaagaaggccagccacaagagcggctgcaccgccggcgagaaggcgtaggttttcagttccggaatgctggtggtgccggcttcaaacgacatccacagcatggccagcagcatgagcacgctacccagcagcgtgtacaggaagaacttgtacgccgcatagatgcgattctggccgccccagatgccgatgatcaggaacatcggcaccagggtgccttcaaagaagatgtagaacaggaacaggtccaacgccgtgaacacgccgatgaccagcgtctccaggatcaggaaggcgatcatgtattcgacgacgcgcgtctcgatcgaacgccagctggccaggatgcagatcggcatcaaaaaggcggtcagcagcacgaacaggatcgataccccgtccacgcccaggtggtagctggcccccgcgaaccaggggaccatctccacgaactggtatccagggttcgacggattgaaaccggcgaccagcacgacggacaccgccagcacgaccagcgtcgtgatcagggcgatccaacgcgcggccggcgcggcgccctcctgcgtcttggatcccaggcgcgcggcgaagatcgcggcggcgcccagcagcggcaggaatgtaacgaggctcaggatgtagggcacgatactcaggctccccacgcgaggatggcgaaggtgagcaggccagccaccccgagcagcatcacgaaggcatagtagtagacgaaaccggactggaacttcgacagccagccggcggacttcagcgaggcccaggcggcgccgttcggccccaggccgtcgatgaccttcacgtcgccgaccttgtagaagacctcgccgaccgcacgcgcgccgcgcacgaagatgaagtcgtaggcctcgtcgaaccaccacttgttgtagaggaagcgatagaacaggccgttgcgggccgccatgcgccgcgccatgccttcacgcagcacgtagatccacacggcgaaggcggcgccgatcagcgtcaggatcagcggcgaccacttcacccaggtggggacctcgtggctctcgtgcaggacatggttgccctcgccgatgaacagggccccgcgccagaactcgccctcgtggtggccgatgaagtgcggcgcgaacacgaagccggcggcgaccgcgccgatcgacagcaggacaagcggcagcagcatcacccacgggctctcgtgcggatgcaggggtccgtggtggccatgatcgtcatgcgcatgaccgtcgtgcgccgcgtctgcgaccgcctgaccgtgatcgtccgcatccggcagcggctcggagtgggtctccagctgcgcatgcgtggcgtgatcgtcggcgtggtgcgcgccctcttccttccacaccggcttgttgtggaaggtcatgaacaccagacgccaggaatagtaggacgtcaggccggcggcgaagatgccgataaagaaggcgaacaggccgaccgccgaatgtccggtcgtcgcggccgcgaaggcgctctcgatgatcgaatccttggagtagaagccggcgaaaccgcccacgccggggatgcccaggccggtgatggcgatggtgccgatggtcatgacggcataggtcacgggcagcagcttccacagaccgcccatcttccgcatgtcctgctcgtggtgcatgccgtggatcaccgatccggcgcccaggaacagcagggccttgaagaaggcgtgggtgaacaggtggaacatggccgcctgataggcgccgacgcccgccgcaaagaacatgtagcccagctgcgaacaggtcgaataggcgatgacccgcttgatgtcgttctgggtcaggccgacggtcgcggcgaacagggccgtgatcgcgccgatgatggcgatgatctggctggcgcccggcgcatattcatagatcgggctcaagaggcagaccatgtagacgccggccgtcaccatggtggccgcgtggatcagggcggacaccggcgtcgggccttccatcgcgtccggcagccaggtgtgcaggaagaactgcgccgacttgcccatggcgccgatgaacagcaggaagccggccaggtcgagcgccgaccactggacgcccaagaactcccacgtcgtgccggcgcgctcgccgacctgcgggaacagctcggcgaactcgatcgtgccgtacatccagaagatcgtcatgatccccagaatgaagccgaagtcgcccacccggttgaccacgaacgccttgatggcggcggcgctggccgtgggcttcttgtaccagaagccgatcagcagataggacgccaggcccacgccttcccagccgaagaagatctgcatgaagtcggcggccgtcaccagcgccagcatcatgaaggtgaacaggctcagataggcgaagaaccgaggccggctgtcgtcctcggccatgtagccccaggaatacaggtgaaccagcgacgagacgctggtcaccacgatcagcatggtggccgacagggcgtcgatgcggattgaccaggccgactggaagtcgccgacgttgataaagggcagaaggcggatcgtgaaggcctccatgtggccccacgtccaggcgctgaacaccgtccaggcgacaatgcaggagaagaacagcaggccggtcgtgaccgcctgcgacgggatgttcccgatgcggcggccgaagaagccggcgatggcggcgcccagcagaggagcgaagacgccgagaatgacgagggtctgaataggcacttgcaggtcagcccttcatcacggaggcgtcgtcgaccgcgatgtcgccgcggtttcggaagaaggtcacaaggatcgctagcccgacagcggcttcagccgccgcgacggtcagcacgaacatggccatgatctgcccggagatgtcgttcagataggtcgagaaggcgacgaagttgatgttcacggccagcaggatcagctcgatcgacatcaggatgatgatgacattctttcggttcacgaagatgccgaacacgccgatggtgaacaggatggcggcgaccgccagatagtgggtcaggccgatcatcagagaagctcctcggccgagaggcccttaccggtcgcggcaggcttgatctcgacggacttgcggcggtcgcgattgacctggtcgcccgggttctggcgcttgatgtgcggcttgtggcgcagcgtcagggtgatggcgccgatcatggcgatcagcagcaccacgcccgccgcctggaagaagtagatgtagtcggtgtagagcacccggccgatcgcctcgacattggtgacgtccgggccgagagcgccgggggccgaagcgccgttcgccgccccgccctgcaccacggcgaccgacaccatgatcatctcggccagcagcaccgcggcgacgatgccgcccagcggcagatagcgggcatagccctcgcgcagcttcacgaagtccacgtccagcatcatgaccacgaacaggaacagcaccgcgaccgcgccgacgtagaccacgaccagcagcatggccaggaactcggcgcccagcagcacgaacagcccggccgacgagaagaacgacaggatcagccacagcacgctgtgaaccgggttgcgggcgctgacgaccagcagggccgaaaccacggccaccgtcgccagcagatagaaggctacgccttgcatgtcgggacagagcccctttccgtcttcatgccggcgatccgtgaatcgccgcctgttccaagcgagaagcgccttagcggtaaggcgcgtccagttccagattcttcgcgatgacccgctcccagcggtcgccgttattcagcagccgctccttgttgtagagcagctcctcgcgtgtctcgaccgtgaactcctggttcggcccctccacgatggcgtccaccgggcaggcttcctggcacaggccgcaatagatgcatttcaccatgtcgatgtcgtagcgcgtggtgcggcggctgccgtcggcgcgcggctcggactcgatggtgatggcctgcgccgggcagatggcctcgcacagcttgcacgcgatacagcgctcttcgccgttcggatagcggcgcagcgcgtgctcgccccggaagcgaggcgactgcggattgcgctcgaacggatagttcacggtggccttgggccgcgccatgtacttcagcgacaggccgagggcgccgatgacgtccagcatcatcgcgcccttggtcgcctggacgatacgggtgaacatcagaaacggtccttgggagcggcggccgctccggtcgatggggtttgttccggcttgggctgggcgtcccgccactggcgctcgatggcgtcctggcggcgttgccactggtagccggacgtcggcatggcttcgtagggctgggcgcaggcggcggccaacggcgccagcaggctcgcgatcagcagcgcgcgcatcacgcccccaccacgaacacgcgccaggccgagacgatgatcaccgcgaccagagaggccggcaggaaaaccttccagcccagccgcatcagctggtcatagcgatagcgcggcacgaaggccttcaccatcgagatcatggcgaaccagaacacggtcttggccacgaaagtcaggaagtagatggtgtattccagccagccgggcagcgcatccagccagccctgcggcacgccggggttccagccgccgaagaacagaaggctgatcatggccgacatgaagacgatgttgacgtactcgcccatcatgaacagcaggtacggcgtcgagctgtattccacctgatagccggccacgagttcggattcggcttccggcagatcgaacggcggccggttggtctcggccagcgccgagatgaagaagatgatcgacatcgggaacaggaccaccaccagcggccaggtccccgccccgccgccgaaaccgtaccagttccagaacatgccctgctggttcagcacgatctgcgacaggttcatggtgccggccaggatgatcacattgacgatgatcaaacccatcgagacttcataggacaccatttgcgccgccgaacgcagcgagcccaggaacggatacttcgagttggacgcccagccgcccatgatgatgccgtagacgcccagcgacgacaccgcgagaatatagaggatgccgacgttcaggtcggacaccacccagccgggggcgaagggaatgaccgcccaggccatgaaggccaagatgacggtgatgatcggcgcgatgatgaagaccgccttgtcggcgcccgccgggatcacgacctccttcagcacgaacttgatcatgtccgcgaacgactgaagcaggccgaacggcccgacgacgttggggcccttgcgcatctgcacgccggcccagatcttgcggtcggccagcaacaggaaggccacggccaccagcacgccgacagtgatcagcaggacctggcccaccgtcatcagcgtccagccgatcggcgtggcccagaaggaaacgggatccatgtgttcttactccgccgcgatcgcgaccggcgccgaccgctgggcggacagctcggccatggtcgcgctggcgcgcgctatcgggttggacaggtaggggtcgacgacgatcgaggcgaaggcgcggtcgcccagctcgcccgcacggcccagcgcgccgaggtcgaaggcctgcggcgccggcagatagtcgatccgtccgaacgtcggatgatcgcccatcagcttgccgcgcagctgttccagcgtgtcgtagggcaacgtccggccgacgcgggccgacagcgcccggatgatcgcccagtcttccttggcctcgcccttggggaagaccacgcgctcggccatctgcacccggccctcggtgttgacgtagaggcccgacttctcggtataggccgcacccggcaggatcacgtcggcgccgtgcgccccccggtcgccgtggctgcccagatagacgcggaaggcgtccgaacccgtcggatcgacctcgtcggcgccgagcaggaacagcacgtccagcgcgcccggcttcagcatctgcgaaacggtcaggccgccttcgcccggcacgaagcccatgtcgaggcccgccacgcgcgccgcggcatgatgcagcacgttgaagccgttccaaccgtcggcgatcacgccgatctcgccggccagcttgcccagctgcgccagcacggcctcgccgccctcgcccgtcagcgccgaggcgccgacgatgatcgccggacgctgggcattggtcaggaagtcgcgcgcgcccttcggcagatcggccagggtccgcgcgcccgcgcccagatagtgatggtcataggtcaggtcggcggcctcgccgatcaggccgatctccatctcgcccttcagccaggccttgcgcaggcgcgcgttcagcagcggcgcctcgacgcgcggattgacgccgaccagcagcaccgcgtccgcgttttcaatgccttgcaggccggagttgaacagccagccctcgcgggggccgtagcccagcgccgcgccgtcctggcggcagtcggtgttggccgaacccagcgcacggaacaggtccagcgtcgccttcatcgactcggcgtcctgcaggtcgccggcgaccaccccgatccgctcaggcgacgccgccttcagcttctcggccacgacgttcagcgcctcgtcccagttggccggctgcagcttgccgttcgtgcgcacccacggccgatccagccggcgcgtctgcaggccgtcgaccacgtagcggctcttgtcggacagccactcctcgttgatgccttcgtgcacgcgcggcagcacccgcatcacctcggccccgcgcgcctgggccgagatgttggagccgagcgcgtccatgacgtcgatggtctcggtcttcttcagctcccacggacgatagtggtactgccacggccggtgcgtcagggcgccgacggggcacaggtcgttgacgttgcccgacagctcggaccccaccgacttctcgagataggtggtgatctccgcgtcctcgccgcgcgagatcatgccgatgtccggcacgcccgcgacctcggtgatgaagcggacgcagcgcgtgcactggatgcagcgcgtcatataggtcttgatcgtcggacccatgttcttgttttcgaccgcgcgcttgttctcggcgtagcgcgacccgtcgcggccatagcccatggcctggtcctgcaggtcgcactcgccgccctggtcgcagatcggacagtccagcgggtggttgatgagcaggaactccatcaccccttcgcgggcctttttcaccatcggcgtgtcggtgaatatctcctggccgtcggcggccgggagcgcgcacgacgcctgcggcttcggcggccccggcttcacctcgaccaggcacatgcggcagttgccggcgatcgacagccgctcatgatagcagaagcgcgggatctcgtgcccggcgcgctcggcgacctgcagcacggacatcccgggctcgaactcggtttcgacgccgttgaccttggcgactggcatcagcgggcctcttcttcagcgggaacggtcaactccgaccggtccgtcgtcccatcggggagagtctgtgtgatggcgatgcgctgcccgtccaggacatagcggatcaccggatcgccggactggttcatccagcggaccagggcggcgtcaggaaggtcgagcggcttccacacgatcaggtcgccgtcgacgcggcagtcggcgcgcatgcggccgccgtcgaccggtgcgcgccaggaggcgtggaccacctccccttcgacgccgtcgaccgccaccgcgccgggctgctgtccgtggatggccgccagtcccgcgcggcacacgcgccgcaggtcggccgccgacagcacggccggcgcggcgggcgccgcatccgaagtcggtagcgcggccgacacctgttccgccggcgtcggcgcagcctcgcgctcgccgcaggcggcgagcgacagaacagtcagcatccccacagccgtcatcctcgggctcgacccgaggatcggacggtccgccgcacgagcgcgcgacgcttcggacgcagagcccgaggcgcgctcgatcctcgagtcaagcccgaggatgacgcagactgtggaaacgacgcccatccctactccgccgcgatcgcgtggccggcgaagttggcgcggcggctacggtagctggcgatgcggtcttcgatctcgtggcggaagtggcggatcaggccctgcaccggccaggcggcggcgtcgcccagcgcgcagatggtgtggccctcgacctgtccggcgacatccagcagcaggtcgatctcggacgggtccgcctcgccgatcgccatccgctccagcacgcgccacatccagccggtgccctcgcggcacggcgtgcactggccgcagctctcgtgcttgtagaagtagctgatgcgcgcgatggccttcaccaggtcggtggagttgtccatcacgatcaccgcggcggtgcccagacccgagcgcatctcgcgcagcgagtcgaagtccatcagcgccgtttccgacatctcgcgcgtgatcagcggcaccgacgatccgcccgggatcacggccttgaggttgtcccagccgccgcgcacgccgccgcagtgctcttccagcaactgcttcagcgggatcgacatggcctcctcgaccacgcacggctggttcacatggcccgagatggccatcagcttggtgccggtgttgttcggccggccgaagcccgcgaaccactggtgtccgcgccgcaggatggtccccacgaccgcgatcgactcgacgttgttcaccgtggtcgggcagccgtacaggccggcgcccgccgggaacggcggcttcaggcgcggctggcccttcttgccctccaggctctccagcagcgcggtttcctcgccgcagatgtaggcgcccgcgccgtggtggatgtagacatcgaagtcccagccgtggacgttgttcttgccgatcagcccggcctcgtaggcctgtttgaccgccgcttccatgcgctcgcgctcgagcacatattcgccgcgcagatagatgtaacaggcgtgcgcctgcatggcgaaggacgcgatcaggcagccttcgatcagcagctggggatcatggcgcatgatctcccggtccttgcaggtgccgggctccgactcgtcggcgttgaccaccagatagtgcggacgatccttcacctccttgggcatgaaggaccacttcaggccggtggagaagccggcgccgccccgtccgcgcaggcccgacgccttgacgttgttgatgatccagtcgcggccaaggtccagcatgtccttggtggcgttccagcagccgcgcgccttcgccccctccagcgtccagtcctggaagccgtagaggttggtgaagatccggtccttgtcttcgaggattccgaccatgggtccttaaagtccttccgccagacggcgcttgtggtggcgggtgcgcatccagacggcggcgatcaccatcacccagcccgcggcgagcatgagatacgacaggttcaccgcccactcgcccagtcgcggcgtctgctgacgcaccatcaggatcagcacggcggccgcgacgaccatggccaggccgccggcgcgcaagggccgtccgaccgaccgcagctccttgcggtaggcggcgcgaccctcatccgtttcgaggttcggcgcgctcatcaggccggctctttggccggttcgggatccgagttcggcagcttggcgatcggctgggcttggcggccgtcatacagcgtctcgtccagcagcgtcttggcgccgccctgcggctcggatgtgcgccgcccggcgtagctgcccggctgaggcgtcttgcccgctttgaaatcgtcgatgatctgcgccatcgactcggctgtcaggtcttcgaaatagtagtcgttgatctgggccatcggcgcgttggagcaggcgcccaggcactcgacttcctgccaggtgaagccgccgtcggccgacaggtgatccttgggcccgatcttctccttgcacacgcgcatcaggtcgcccgcgccgcgcagcatgcagggcgtggtgccgcacacctggatcagcgcggtcttcccgaccggctccagcatgaacatggtgtagaaggtcgcgacctccagcacccggatgaagggcatgcccagcatctcgccgatggcgcggatggcgggctccgacacccagccctcctgcttctggaccagccacaggatcgggatcaccgccgattgacgacgctcggccgggtatttggcgatccaccagttcgccttctccatcgtcgcgtccgcgaaggtgaaggaggccggctgttccttggcgaggcgacggacgctcatcggtccacttctccgaaaacgatgtcgagcgagcccaggatggcggacacgtcggccagctggtggccgcggttcatccagtccatcgcctgcaggtggcgatagcccggagccgagatcttgacccggtacggcttgttggtgccgtccgacaccagatagacgccgaactcgcccttgggcgcctcgaccgaagcgaacacctcgccctccggcgtgcggaagccctcggtgtagagcttgaagtggtggatcagcgattccatcgaacgcttcatctcgccgcgacgcggcggggtgatcttgttgtcctcggccagcacgggctgaccggggcagttgcgcagcttgtggatgcactgctccatgatgcgcaccgactgcttcatctcctcgacgcggacgagatagcggtcccagcagtcgccgttcttgccgaccaccacgtcgaactccatctcggcgtagcattcgtagggctgcgacttgcgcaggtcccaggcgacgttggagccgcgcagcatcacgcctgtgaaggcccagtccagcgcgtctttcttagacaccacgccgatgtcgacgttgcgctgcttgaagatgcggttttcagtgaccagcgcctcgatgtccttcagcgcggccgggaactcggcgcaccagcggccgatgtcgtcgatcaggtcgggcgacaggtcctggtggacgccgcccggacggaagtagttggcgtgcaggcgggcgccggaggcccgctcatagaacaccatcagcttttcgcgttcctcgaagccccagagcggcggcgtcagcgcccccacgtccatggcctggggcgtcacgttcagcatgtgcgacaggatgcggccgatctcggaatacagcacccggatcagctgcgcgcggtacggaacctccagccccagcagcttctcgatcgccaggcagaaggcgtgctcctggttcatcggcgagacataatccagccgatccagatagggcacgttctgcagataggtgcgcgactccatcagcttttcggtgccgcggtgcagcaggccgatgtgcggatcgacccgctccacgatctcgccgtccagctccagcaccaggcgcagcacgccgtgcgccgccgggtgctgagggccgaagttgatggtgaacttgcggtcgtccatcgcccgggcgtggtcggtcaggccgtcgtcgaacacttgggtgtccgttccagccaaaggacgctcctgggggcggttcacgggatgaagatcgtcggccatcagcgggcagccttttcgtcgccgggcagcacgggcgccggatactccgcgccctcccagggcgacaggaagtcgaactggcggaactcctgcgtcagcttgacgggctcgtagacgacccgcttctgctcttcgtcgtagcggacctcgacatagccggtcatggggaagtccttgcgcagcggatgcccctcgaagccgtagtcggtcagcagccggcgcatgtccggattgccctcgaacagcatgccgtacatgtcgaacgcctcgcgctcgaaccagccggcggccgggtagacctcaaccgccgtcggcacgggcttcacctcgtcggtggagaccttgacccgcacgcgcgcgttccgcgtcatcgacagcaggtggtagaccacctcgaaccgctcgcggcgatccggatagtccacgccgcacaggtccagcagctgctgaaagccgaagcggtcgcgcaggcccagcagcacctcggcgatccgctcgcgcggcgcgaccagcgtcagttcgccgaacgccacctgcgcctccacgcccagcgcccccaccagctcggcgcccagcggcgtcagcagcgtctcctgttcggcctgaacggcgagagaggtcatcgctcgatcgtccccgtccgccgaatcttcttctgcagctgcagcagcccgtacagcagcccctccgccgtcggcgggcaccccggcacgtacacgtccaccggcaccacgcgatcgcagccgcggaccacgctgtagctgtagtggtagtacccgccgccgttggcgcagctgcccatggagacgacgtagcgcgggtccggcatctggtcgtagaccttgcgcagcggcgcggccatcttgttggtcagggtgccggcgacgatcatcaggtccgactggcgcgggcttgcccgcggcgccatgccgaaacgctccacgtcgtagcgcggcatcgacatctggatcatctcgacggcgcagcacgccaagccgaacgtcatccacatcaacgagcccgtgcgcgaccagttgatcacatcgtccaggctggagacgagaaagccccgttcgccaagctcggtgttcacctgctcgaagaacttgtcatggatggcggggtcatagccctcaacggtggagcgggcgcccgagccatagctctggacggagccctggcctgcggggaccagcgggctggaaggcgcgatcactcccattccagggctcccttcttccattcatagatgaagccgatggtgagcacccccaggaagaccatcatcgaccagaaggcgaagatcatctcgccgcgtgccaggtcgaacatcgacaccgcccacgggaagaggaaggccacttcaaggtcgaagatgatgaacaggatcgacaccaggtagaagcgcacgtcgaacttcatgcgcgcatcgtcaaaggcgttgaagccgcactcataagccgacagcttctcggtgtcggggttcttcggcgccagcaccagcggcagcacgacgaacagcacgccgatcagcagcgccacgcccgcgaaaatgatggtcgcgagatattcgaggagaaattcgttcattccggaagcctcgcccgccagggggagaggcgggattcggcgcttcttagacccatcgtccgcgcggttcaaacccaagcgaactaaaggtttttgttgagaacggctcgcagcatagcgcgcctttgtcgcagggccggcgcttgcccgcgccctgctgcttgcggcctatgaccatggggttctgcaaggattactgctcatggggctggcggctcgcgcgctgaatggcattgaacggttcggcaaccgcctgcccgaccctgtcttcctgttcctctggctgatcctggggctgatcgggctgagcctcgtcggcgcggctctgggctggtcggcggtcaacccggtcacgaacgagctgttgacggcgcagagcctgctctcgcccgagaaccttgaacggctgatcatcggcatgcccaagacgcttgccgagtttccgccgctcggcatcgtcatcaccatcatctacggcgcggcggtggccgagcgcacaggcctgttctccaccgccattcgcggcgccctgctggacgcgccgcgcgccatcctgacgccggtggtggtcatcaccggcatggtgtcgcaccacgcctccgacgcctcctacgtcgtggtgatcccgctggcggcggtgatcttcgcggcggccgggcggcacccgctggcgggattggctgccgggttcgcggccgtgtccggcggctacgccggcaatctgttccccggcgccagtgacgccctgatcctgggcatcaccgagccggccgcgcacctgatcgacccctcctattcggtcaacatcgccggcaactggttcttcatcgtgggggtggtgatcgtcttcacgcccattgtctggttcatcaccgatcgtgtcatcgagccgcgcctggggccatggtcgccagcggcgagcacgcccgccacgccgtcggaaaggcagccgctcaccgctgcggagaagcggggtctgctgtgggcgagcctgacgatcctaggcatgatggcgctgtgggcgctgatcaccgccctgcctgcatcgccctttgtcgatccggaggccgagccggcgcagcggttcaaccccctgtaccggtcgctggtcgccttcttcgcggtcaccttcttcgccagcggcgcggcttacggggcaggctccggctccatccgctcgcaccgcgatctggtgcggatgatgggtgaaggcatctcgcaactggcgccctacatcgtgctcgccttcttcgccgcgcacttcgtggccatgttcaactggtcgggactgggtccgatccttgcggtgaacgccgccgccgcgctgcagcaggtcgccctgcccacgccgctgctgctgatcagcgtcgtgctggtctcctgtgtcttcgacctgttcatcggctcggcctcggccaaatggtcggcgctcgcgcccatcgtggtgccgatgttcatgctgctgggcatctcgccggagatgaccacggcggcctaccgaatgggtgattcggtgaccaacatcgccacgcccctgatgagctacttcccgctgatcctgaccttcgcgcagcgttgggatccgcgattcggcctgggctcgctgatggcgaccatgctgccctatgcgggcgcctttctggtcgcgggcctgatgatggtggcggcctgggtggcgctcgacctgcccctgggaccgggggtgggcgtgcattacgagccgccgccgccggctgtggccggtcaggcgccggccgacggcggccttctggggcccgacacgccgccgcagccggcagcgacggcccccgcacgatgacccgcgccgtttccgcagaaaccctgcttgacgcgccccaccagccgacctaaacgacgcccctcgccgcggcgcaccagcgcaacggtcgggaatgcgggtgtagctcagttggttagagtgccggcctgtcacgccggaggtcgcgggttcgagccccgtcactcgcgccacttcttctagaaatagaagggtggcgctgccgccttcccagaacagctttcgaaacagctcacaagtttcgaccgggtacgcgggtgtagctcagttggttagagtgccggcctgtcacgccggaggtcgcgggttcgagccccgtcactcgcgccacttctcctgacaccaggaagaagtggcgcgccccccccctcgcccttgtgatctcagtgcacggcccactcgccgtccggctgcacgaacgccgcttcgcccgtcaggtcgccatagaccatgcacaggtcttcaaagacgcggctccaggcgaattgctcgaccgtgtggattcgcgccgcctgacctacggcctcgatgtcgcgctggaacaaggcttccaccgcttcggcgtactgcgcaggatcggccgacgccgccagctgcccgacctcggccgtgacggtctccgccacgccccctgcattgacgcccaccacggggcgcccgcacgccatggcttccagcacgatcaggccgaacggctccttgtcgttggcgtgcacgaatgcgtcgcagctcgcgatgatgcgagccaccgccttgggatccttctcatatggcaaggcgatcacccgatcctcgggcggcatgccggtgccggcgccgaccagcaccaggtgatagggcgcgcccagcttctgcaccgcctcgatcagcacatcgatgttcttttccttggccggccgcccggcgaagcaaagcaggcgggcgtccgcgctcagacccagcttcttcagcagccagtcgcggtcgcggcggctgggatgaaaggtgtcgatctcgacgcccagcggacgaatcacgatgttctcgacgcccgcctcctccagacgctgggcgatgaagcggctgggcgacaccacgcggtcgaactgcgagaacagccgcgcccagcgcttctccaccggcttcttggcccactcgccgaagtgcagcgccgccagccccgccggatcggagtggcaaaagccgaccacgggacaacccgcacgctggccagcctcgatcgccgcctgtcccggcgtgtaggggtcgcccgcctcgatgatcgacggacgggtggaggccagccacgcgccccaccgcttgaccgaactcggccagcggtaaccgtcgccaaacggcagcttggtcgcccgcagcttgatgattccgtccgcgcccgggtcgtgccgagcgcccggcaccaccagcgaatgggtcacgcccggccggtgggcggccagccacgccttcttggacatcaggtagcgcttcaccccgcccgagcggggcgcatacagcatggtggtgtccacaagacgcggccggggatcggcggccgaagccttgacgcgtctcagggtctccgagacctcctcgtcgaggccggggatcagtcgaagttcgctttcctgaacgtcggtgtcgatcatgctcacggtcaggccctcgtctgtcgcgggctcagcaacgtcctgagggggattttggatgcgtcgggatgtgcgtcgagccgtcatccgcacgccgataggctcagccaaggccaagctcaagaggcgagcccacgccttgtattcgcctcaaattcgagaaacttggggcatggcggaccggaccctgttagagggtcgcccacgtccgtgcgcgtcaccaggggttctgttcgaatgcgtatattgcttgcgaccgcggccgcgatcgctcctctgacggtcgccgccggcgctcacgcccagcaggtgatctccaccgcacggaccacgccgatcgcgaccgctacggcgacaggcacggctccggattcagtgcgcatcgccagcggcggctcggtcgcggtgaccagcggcgcggcggtgacgctgaactcaagccatacggtcgacatcgacaacggcggctcggtcaccatgaccaatgcggccgacggcgcgacaggcgtgctcgccaatggcggcaactccggctcggtgcttatcggcggcgcgatcaacatcaccgattcgatcaaccaggccgactacaaggacgccgacggcgacggcgacctggacgggcctttcgccgccggcacggatcgttatggcgttcgggtcgtgggcgcggcgcctttgaccggcgatgtccggatcgagagcggcgccaccatctcggtcgaaggcaaccagagcggcggcgtctacatcggcgcgccgctgacgggatcgctgcagaacctcggcaccatcacgaccatcggagatgcaaactacggcgtccgcaccgtgggcgacgtcagcggcaacgtcgagatcctgggtgcggtcaccgcgaccggtgccggcgcgaccggcgtgtcgctggaacgcgacaccggcggtcaggtcaagatccagggcgcggtcagcgcgaccggctaccgctacaccaccccgccccagcctaagccgaccacgggcaccgttccgaatgaggccctgttcctcgaggacctcgacgccgatgatctgctgcagggcggcccggcggtcgcgatcgcgggcaatgcgacacgcggcgtggtgctggaccgggcgcccgcctatggctcgggcggcgtcgaaggcgatgacgacggcgacaacgtcaagaacggcgacgaagacgacgacggcgacggcaccatcaaccgcaacgacaccgaccgcgacggcgacggcatcctggacgccagcgagagcacggcggcgctgacgtcgctgggcggagcgccggcgctccagatcggctcggccagccagacggtgaacctcggtgccgcgggctcgggcgacagcgcctacggcctgatcaatcgcggcacgatcaccgccagcggcctgtacgcggatgttgacgcccgcgcggtccagctcggcgtgacgggcggccaagccgtatccatcgccggcggcttccgcaacgaaggcacgatcgccgcggcggcgctgaaggcggatgcgacggcggtcgccgcgctctccaacccttccgcccccgccctggtgaacaccgggtcgatccagtcggcggtgaccagcgacggacgcgacgtcgcgaccggcgtcctgatcggcgcgggcgccaatgtgggcggcctgaccaactccagcaccatcaccgcggtggtcgcgggcaaccacggcgattccgtcgccgttcgcgatctgtcgggaagcctgacgtccgtcaccaactcaggggcgatcggcgccggccgcacggtcaacacagccgacacgacggcggtggacggccagcagatcgcgctcgacctcgccgccaacaccagcggcgtcaccgttcgccagttcggggtgcgggccgcgacaggcagcaccgcgaccgacagcgacagcgacggcgtgccggacgccgccgagcccaccatcgtcggtcaggtccgcctcggctcgggcgcagacaccttcaacgtcgagaacggcacggtggtcggcgacatcagcttcggcgcgggcgccgatgcgctgaacatcaccggcggcgcggccgtgaccggggcgatccgcgatgcggacggcaccctcgccgtcaacgtcgccaacggcacgctgcaggccagccagacgacggcgaccaacatctccagcctgaacgtgggggcggacggcgcgctgatcctgacggtggatccgacccagtccacgccgagcggcttcaacgtcagcggaaacgcgactctggcggacggcgcggcgctgggcgtgcgcttctcctcgctgttgcaggagccggagcggttcaccgtggtgcaggcgggctcgctgaacgtcggcgcgctggatcagtccgccctgtctggaaattcgccctatctctatgtcgtgtccgccacggccgacacggcggccggccggctctatgtcgatgcacgccgccgcaccgccgacgaggccgaactgaccgcggtcgaggcctccgcctatgacgccgtctacggcgctctcggacagaaccagacgcttcaggacctcttcgtgcgccagaccacgcgcgagggcttcatcaacgcctacgagcagctgctgcccgaccactcgggcggtccgctgatgtcgctggccagcggcgtggacgcggtcacgcgcgccctgaccggccgcaacacctcggctgcggcgggcgagaccagcgcctgggtgcaggagatcaacttctacgccgacaaggaccgcaccgactcctacggcttcacctccgaaggctttggcgtggccggcggcgtggagcgcggcacgcgcctgggcgccttcggcgtctcggccgccttcacctcttccgatatcgaggaccccgaggcgcaggccgaagaggtcctgtccgccaatctgctcgagctcggcctctactggcgcgcgcaaggccagtactggacgacctgggcccgcgcggctggcggctacgccagcttcagcgccgatcggtctctggtcgcggacggcgtctacctgaacaatgagtccgaatggcacggctggtcggtggccgcagcgggcggcgcctcctacgagcgtcgcttcggccgctggaacatccgtcctgaggcctatgtcgaatatttcggcttgacggaggacggccgcaccgagagcggcggcggcgacggtttcgatctgcatatcgaagagcgcgacggccacatgttctccgccgtggcggccatgaacgtgggctacggcttcggccgcgacggctgggtgcgcccggagctgcgcgtcggctaccgccagaacatctcctatgacgccggcgaaaccatcgcccgcttcgccagcggcggccccagcttcaccctggatccgggaggcatcgagggcggcggcctgatcctcggcttccgcctgaacgtcggcaacgaactgggcatgctgtcgctgacgggcgacgccgaaatgctggaggactacgtccgctattcgctgctgctccgagccagcttccgcttctgatcgaatcaacagccagaagaaaaaggccgccggagcgatccggcggcctttttcttgttcgatggtaggcggcgacgggttcgaaccgccgaccctctcggtgtaaacgagatgctctgaccagctgagctagccgcccgcacgcatcgcagacgggcttaatgcctgcgtccggctatccgttcaaggcgcttttcaagccttcgcccgcacgaaagcgcgcggtgcgggaggcctgacgggcgatggtctcgcccgtctgcggattgcgcgccagacccgcctttcgctcggccatgacgaaactgccgaagccggtcaggcgaacgtcgcggccggcgctgagcgactcggtcacgccgtcggtgaaggcttcaagcgccagcttcgcctgctcgcggctgatgcccgccgccgccgccattcgcccgatcagctccagcttggtcatgtcagatgtggatcacgcgcccataggcgtccagcgcggcctcgtgcatggcctccgacatggtggggtgcggatagaccgtgccgtgcaggtcctcctccgtcgcctccatcgtgatggcggtgacatagccctggatcatctcggtgacctcggcgccgatcatgtgcgccccgacgagggcgccggtctgggcgtcgaagatggtcttcacgaagccgtccgtatcgcccgaagcgatcgccttgccgttcacgcggaaggggaagcggccgaccttgacctcgcggcccgccgccttggccgcctgctccgtcaggccgacggacgcgacctgcggctgggcgtaggtgcagccggcgatcggcgacaccacctgcggcgtcttgaagcccgcgatgtgctcggcgcagtggatgccctcgtgcgaggccttgtgcgccagccacggtgcgccggcgcagtcgccgatggcgtagagacctttcacattggtctcgcagtgcggcccggtcttgatgtgaccgcggtccagctccacgcccagcgcctccaggccgatgccgttggtgttggcggtgatgcccacggcggagatgcacacttctgccgtcagtgtctcgggcttgccgccgacttccacatcgactttcacgccgttggcgtccttggacaccttcgtgacctttgcgccgatgcggaacttcatgccgcgcttctcgaacgatttctgcgccgccttggagacctcttcgtcctcgaccggcatgacgcggtccaaagcctcgacgacggtcacctcgcagccgagggcgcgatagaagctgccgaactcgatgccgatagcgcccgagccgatcaccacgatggacttcggcatgaacttgggcgccatggcctcgcgataggcccagatgcgttcgccgtcggcctcaagtccgatctgcggcaaggcgcgcgcgcgcgcgccgacggccagcataaccgacttggcttccaccgtgcgagagccgcctgccttgagcgcaatcaccaccttgggggcagccgagcccttctccagcttggccgtgccttcgatcacctcgatcttgttcttcttcatcaggaagccgacgccctggttcagctgcttggccaccccacgcgagcgctggatgatggcgtcgaagtcgaagccgaccttttccgccgacaggccgtagtccttcagatggctcaggctctcatacttctcgcccgacttcagcagcgccttggtcgggatgcagccccagttcaggcaaatgccgcccaggttctcgcgctcgacgatggccgtcttcagaccgagctgcgaggcgcggatagccgcgacatagccgccggggcccgagccgatgacgatgaggtcgaaggtgtcagccatgattcagagcagtttctcgatgtcggcctcgatggccttcggttcggtctggggcgcgtagcgggcgacgacctgcccctcgcggtcgatcaggaacttggtgaagttccacttgatggctcgggagccgaggaagccccgcttctgctcggtcagccaggcatacagcggatggcggttcggcccgttcacctcgaccttgtcgaacagcggaaaatccacgtcataggtcaggctgcagaaggccgcgatctcggacgcgcggcccggctcctgcccgccgaactggttgcagggaaaacccagcacctcgaaagggcggtcggcgaaggcgcgatgaagcgcctccagcccttcgtactgaggcgtgaacccgcatttggacgccgtgttgacgatcagcagcgcctgtccgcgccaccgctccagcggcacatcggtcccgtcgatggcgcgggcggagaagtcatagaccgaggtcatgaccgccctcgccttaagccagcatggtgacggggtcttcgatcagcggcttgaacgcctgcaggaagcgggcaccggtcgcgccatcgaccacgcggtggtcgcaggtgacggtaacggtcatcaccgtagccacggcaagttgaccgttcttgaccacaggccgttgttcgcccgcgcccacgctcatgatcgcgccctgcggttcatttatgatcgagctgaactgcttgatgccgaacatgcccaggttcgagatggagaaggtgccgccctggaactcctccggcttgagcttgcgctcgcgcgctcgcttggcgaggtccttcgactccgtggcgatctgcgacagcgtcttggtttcggcctttcggatgatcggcgtgatcagcccaccctcgatggcgacagccatggccacatcggcgttgtgatgcagggcgatgccttcgggcgaataggaggcgttggcttccggcacagccttcagcgccattgcggcggccttgatgacgaagtcgttgaccgagaccttgacgccggacttctccagcatggcgttgacgcgagcgcgcgcggccagaagcgcgtcgatttcgacgtcgatcgtcagcggaaagtgcggaacggcgttgacgctctcgaccatgcggcgagcgatggccttgcgcatgccgtccagcgggatcaggtcgtagctgccatcggggatgcccatctgagccagcgtctgcaccttgcgcggctcggccgaggacgacgcgggctgcgccgcagccggcgcgccagcgccctgccccgcaccttccacgtcgcgcttgacgatgcggccatgcggccccgtgcccttgatggacttcaggtccacgcccgcctgagcagccatgcgacgggccagtggcgaggcgaagacccgctcgccctgcgtcttggacgatgccgcagacgatccgccctgcggcgtgagcgcctgctcggccgacttcacgccttcgggcgtggcgacggcgtcgccgctctcgtgtccggccggcgcgggcttggcgtcagatgacgtcgacgagggcgatggctcaggcttcgcgtcttcagccttcggagccggcttcggccccgcgccgctttcgtccttcagcctggcgatgggcgtgttgaccttcacgttctcggcgccctcggcgaccaggatctccaggacctcgccctcgtcgacggcctcgacctccatggtcgccttgtccgtctcgatctcggcgatgacgtcgccggcggagaccacgtccccgaccttgacgtgccatttggccagaacaccctcttccatggtgggcgacagggcgggcatcaggatgtcggtcatcaggcttttccctcagcttgggaggccggctcggcgacggtgcggacgttgtccgccttcaccacttcgctgatcccctcgaggatacggttgtaggcggccgtttcatcatggccgtgacgaacgccgtagccatgcgccatgtggcgcgcggcgtaggccagcagccggccgaactggattgggtcgttgaaggccggcttgacggacatcaccggctcgtccctcgaccaccacatccgcagcacttcgatggcctgcggatcggccgcgacgctgtccggcggcgtcatcacaaaggccgaagcatccccggcccgctgatcgaagtcgctgggtgcgctcaagcgaccacctgcttgaccgccttgatgatcttgtcgacgcccggcagcgacagggcctcgaggttggcggcgtagggcagcggcacgtcttcctggtgcacgcgcagcggcggggcgtccaggtagtcgaaggcgtgctcgatcacccgggccacgacctcggcgccgacgcccatcggaccccagccttcctcggccgagaccaggcggttggtcttcttgacgctttcaacgatcgtttcgtgatccagcgggcgcagggtgcgcagatccacgacctcggcctcgatgccctcctccgccagcttctcggcggcggcgagtgcgaaaccgaccatgcggctgtgggcggtgatggtgacgtccttgccttcacgacggaccttggccttgccgatcggcagaacgtagtcctcgacctcgggcacgtcgaactcgagcccatacatcatctcgtgctcaaggaagacgaccgggttcggatcgcggatggcggccttcagcaggcccttggcgtcggcggcgtcgtagggggcgatgaccttgaggcccggaacctgcgcgtaccaggcggagtagtcctggctgtgctgggcgccaacgcgcgaggccgcgccgttgggtccgcggaacacgatgggcgcgcggatctgaccgcccgacatgtacagggtcttggcggccgagttgatgatgtggtcgatcgcctgcatggcgaagttgaaggtcatgaactcgacgatgggcttcagcccgctcatcgccgctccgacgcccagacccgcaaagccgtgctcggtgatcggggtgtccaccacgcggcggtcgccgaactcctgcagcagctcgcggctgaccttgtaggcgccctggtactgggcgacttcctcgccgatcaggaagacggcttcgtcgcggcgcatctcctcagccatggcgtcgcgcagggcgtcgcgaatggtggtcttgaccagcttggcgtcggccgggatctccgggtccttcagcgtctgcttgggcgtgacgggcgcggggccttcgccttccggctgcggcttggcggcttccggcggcgacttctccggatcaccggccttctgctcgtcggcgccctccttggccacggcggacgaggcggaggccgcgttggtcgcaggcgaagcgcccgcgtcgtcacccgacaggcgagcgatcggcgtgttgaccttcacgttctcggcgccctcggccacgaggatctccaggacctcgccctcgtcgacggcctcgacctccatggtcgccttgtcggtttcgatttcggcgatcacctggccggcggacacggtgtcgcccgccttgatgtgccacttggtcagcgtgccctcctccatcgtgggggacagcgccggcatcagaatgtcggtcacggatcaggcctccacgtagacgtcggtgtagagctcggacgggtccggctccgggctctcttgagcgaactgcacggcttcggcgacgatcgccttgatctcggcgtcaatggccttgagctcctcttcggtcgcgttggcggcctgaagcagggtcttgatgtggtcgatcgggtcgcgggtcttcttgacctcgtcgacctcttccttggtccggtacttggcggggtccgacatggagtggccgcgatagcggtaggtcttcacttcgaggatgtagggcccctcgcccgcacgggcgcgctccaccgccttcttcaccgcgtcgcgcacggcgatcacgtccatgccgtcgacctgctcacccgggatgccgaagctggcgccgcgctggctcagctgggtcgtggccgacgagcgctcgatgctcgtgcccatggcgtactggttgttctcgatgatgtagatggccggcagcttccacagctgcgccatgttgaagctctcgtagacctggccctggttggcggcaccgtcgccgaaatagataaaggccaccgagtcgtcgccccggtacttgcccgcgaacgccaggccggtgcccagcgccacctgcgcgccgacgatgccgtgcccgccatagaagccggtcggcacgtcgaacatgtgcatggagccgcccttgcccttggacgagccgccgatgcggccggtcagctcggccatgacttccttggggtccatgccggcggccagcatatggccgtggtcgcgatagccggtgatgatcttgtcgtgaccctgcttgacgctttcctggacgccgaccgccacggcctcctggccgatgtagaggtggcagaagccgccgatcaggcccatgccgtacagctgaccggcgcgctcctcgaagcggcggatcagcaccatctcgcgatagaagcggagcaggtcttccttggacgcgggcggcggcgtgttggggatagagtcaggggtcttctgggcggctttcgccatcgggcgtctcccggcaacggccccgaagcgggaggccttcttgtcgttacggaagggggctttagcagccttcctttgcgggatgcaaagggaagacggcccggctgtaacaatagttcaagaggcggagacggcgggggaaaccggcttctgcgccgagacccggatgacgtagtcgcgcgggtcagagaagcccagcacggcgcgcgcgcgctcttccagcaggtcgcgcgacaggctgtcggtgcgcagaaagcggacgcggacctccaagtcccggcgctgctcagtcagttgggccaactgctgctcgcgctggcgcagcaaggcgtcgcgctctccgccgctcagcaggccgcgctcgcctgtcagagcctgcacgcccaggtagccgatcaacagagcaaggacgatggacaggcggtacggcttcatcttgtcgagcactacggacgctccttctgagcgtggaacacagtcaatggaccgtggtcgaaaatgcctaacaaaccgtagcttggccgttgagaacggctcccgcagccggtcgcggcgggagccgaatcatcctcagcgcgacagcagcatgccgtcgccgtagtagacgccctggtcgcccagcatctcttccagccgcagcagctggttgtacttggccacccggtccgagcgcgcccgcgagcccgtcttgatctgtccgcagttagtggcgacggccaggtccgcgatcgtcgaatcctcggtctcgccggaacggtggctcatcactgcggtgtagccggcgcggtgcgccatatcgaccgcgtccagcgtctccgacagggtgccgatctggttgaccttgatcaggatggagttggccaggccctcgccgatgccggcggcgaggcgcgccgggttggtcacgaacaggtcgtcgccgaccagctggatgcggtcgcccagacgctcggtcagcagcttccagccctcaaaatcgtcctcggccatgccgtcctcgatcgagacgatcgggaagcgttcgcacaggtcgaccaggtaggcggccatgccgtcggcgtccagcgacttgccctcgccggtcagggcgtacttgccgtccttgaagaactcggtggaggcgacgtccaggcccaggtggaagtcctcgccggccagatagccggccgcctgtcccgccttggtgatgaagctgagcgcctcttcggccgaggccaggttgggggcgaagccgccctcgtcaccgacgttggtgttgtggccggcgtccttcagctgcttcttcagcgcgtgaaagatctccgcgcccatgcgcaggccttccgagaagctctccgcgccggtcggcaggatcatgaattcttggatgtcgatcggattgtcggcgtgggctccgccgttgatgatgttcatcatcggtgtcggaaggacgcgggccgacacaccgcccaggtagcggtgcagcggcaggtccgaggagatggcgctggccttggccaccgccagcgacacgccgaggatggcgttggcgcccagccgtcccttgttctcggtgccgtccagcgcgatcagcgcctcgtcgatacggcgctggtcctcggcgtccatgccggacagggcgtcgaagatttcgccgttcaccgcgtccacggccttctgcacacccttgccgccccacaggtccttgtcgccgtcccgcagctctaccgcctcgtgcgcgccggtggaggcgcccgagggcacggcggcccggccgaacgagccgtcgtccaggatcacgtccacttcgaccgtcggattgcctcggctgtcgagaatctggcgggcgacgatgtcggcgatgtcggtcatggctgggctctgtcagcgaagaaggatgcgaagaggctttagccgccgcagcccgaatcgccaacctaggcgcagccctcgacgtactggatggcggggccgccagcgtggatggccatgaccttgccgtccgagccgatctcatagcggatgccgcgcgcagccggggtggtgacgtaggcggtcgatgcgccctcgcgccaggcgaacagatcctcggcgggcgccgactgatacttgtgcggctgggcgatgaccgcgccgccgtaggacgccttgatcgccgaggccgcgtcgcccaagccgaaaccgcgatcggtcttcagcgtcgccgcgcgcgccagggtgatccgcgccagtcggtcgtccaccatcatgacacgcaggccttcgggcgcccgcgcggggtgaaactcgtcgcaggatgcgggatccgcgccacccacggcgttcggctgcgaatcagccccgaccgccgccgtgacctcggccaccgtcatgccgacccgcaggggaccccacccgtcggccgacaccagattacggtcggtcacggcgggcgtggcggccgccgggggtgaagcaactgccggcgccgcgtcattattcgcactcgtggcggacgcggcggacgacggctcggccggagtttccgggcgatcgcaggcggcgacggcgaacagggccagcaggctgacagcggcgggacgaatcatggagggcgcgcctctttccgttgatctcgaccaacagaacgcacgaaaacggcgcgtggttgacccacgcgccgtcgacaagctcagcttacaggtggaaggggcttagtcttccttaggcgtcagcacctggcggccgcgataggtgccggtcttcaggtcgatgtggtgcgagcggcgcagctcgccggtgtccttgtcctcgacgtaggggttggcgcccagggcgtcgtgggcgcggcgcatgttgcgacgcgagggcgatactttgcgcttcggaacggccatgtccgtctcatctcgtggtcaggcgccgtggccggatgggcgtaagcgcagaaaacagaagcggcggccctggaacagagccgccacgtgagcgcgggcttatgcctcaagccgccggtgatttcaagcggggccgatccgcttgatgacccgcgctggattgcccgcgaccaccacgtccgaaggcacgtcccgggtcaccacggcgccggcgccgatcaccgcgcgatcgccgaccgtcacgcccgccagcacgatggcgccgccgccgatccagacgtcatcaccgatgcggatggtccgcgccgtctccagaccgcgccgctgtacggcgtccagcggatgctcgggcgtcagcaactgcacgcccggaccgcactggaaatgatcgccgatgatgatctcggcgcagtccaggaacacgcagttcccattgacgaagccgctgcggcctatgcggatgttgaagccgtagtcgcagaagaagccgggcatcaccacggcctcgccgtccgcagaccggatcaggtcgttgaccagcgcgcggcgggcgtcgcggtccggctcctgattgatgcggatgatcaggccgacagccctcgcccgtccatcgcgcagttccgtatcgccaggatcatacggcaggccggcgatcatcttctcgcgctcggtcatgcgtgctcctgcaacatcgccgccacagcctctccaatggcgagcgaactggtcaggcccgggctttcgatgccgaacagggcgaccaggccggggatgccgtgccgctcggcgccgtgcagctggaagtccggctgcggctcacccgggccgtgcagcttgggccgaacgccggcgtagtcgggcgtcagcgcgttatcgggcaggcccggccagaagcggcgcacataggcggcgaactcgcccgccttggccggatcgacggaatagtcctcgccgtccacataggtcaggtccggcccgaacaccgcctgcccgcccaggtccttgcgatagtgggtgccgagcgcgcccgggatcggcggcggatagatcagccggtcgaacggcgcccgtcccgtcaggcggaaatagacgcccttgccatagtgcgccttcgggatcccgcctgccggatagccgtcgatgcgcccggcggcgtcctgggcctgaagccccgcagccgtgaccagaaggcgtgtggtcagaacggcgccgcccgctccgcccgccgtgatgcggaagccgccgctgggcagcggctcggcccgctcgaacggcgtcccgaccacgaccgaccctcccgcgtcctcgatcccgccctgcagcgccagcatatagccgtggctgtcgaacacaccgctctcggaggacaacagcgccgcctggaccctcaactcgggctccatcgccagggcctgagtcgccgtgagccgctgcacgccttccacgtcgttggcgaccgcctgatcaaggatggcgtccagccgctcgacctcgtccggctcggtcgcgacgatcagcttgccgcacttccagtgctcgaccttgtggctttccagaaaggcatagagggcgcaccgcccctcgacgcagaaccgcgccttcagcgagccagtcggataatagaggccgccgtgaatgacctcggagttgcgcgacgacaccccctgaccgatcgcgccttccttttccaagaccagcaccgacaatccccgcgccgcgagcgcacgaccgcaggccaggccgaccgcgccggcgcccaccaccgtcgcgtcgaagtcgaagctcaagcgatccggctttgtggcgccgagccgtagcgccgccgcgcctcgccctcgaaacagccaatcagcttgccgaccgcccgttgaaagttggcgtgcagcatggcgtccagcatccgcgacttgaaggcgaagtcgatggtgaactccagccgcgtccccgccggatcgggataaaattcccagcggttgcgcagatgccgaaacggcccgttcagcaggccgacctcgaccacaggtccgctgcggtcatgacgcacccaggtcgagaagcgctcgcgcaagaatgagaagccgacctgcgcctcggcgtcgatgacgcttacgccctcgccctcctcacgcgcgttccaggtgcgcatggccgtgacccacggcacgaagcgcggataggcctgcacgtccgccaccagatcggcgagttgctcaggggtgtagggcaggtatcgggtgacgcggtgaacggccatgctgggcttaacgcgcgcgtccggtctgcgcctcgcgcgcggccttcagccgggcgaagtcctcgcccgcatggtgcgacgaacgcgtcagcggcgaggccgacaccatcaggaaccccttggcccgcgcaatcgcctcataggccttgaactcttcgggcgtgacgaagcggtcgatggcggcgtgcttgcgggtcggctgcaggtactggccgatggtgatgaagtccacgccggccgagcgcatgtcgtccatcacctgcatgacctcctccttggtctcgcccaggccgaccatgatgccggacttggtgaactggttggggtcgcgctccttgaccatctgcagcaggcgcagggagtggaagtagcgcgcgcccggccggatcttcagatacaggcgcggcacggtctccaggttgtggttgaagacgtccggccgcgcatcgatcataacctcggccgcaccgtccttgcgcaggaagtcgggcgtcaggatctcgatggtggtccggggcgcctggatgcggatctggcgcaccacctcggcgaagtgggccgcgccgccgtcggacacgtcgtcgcggtcgaccgaggtgatgaccacgtggttcaggcccatctggctgaccgccagcccgaccttgcccggctcttccgggtccagcggttgcggcaggccggtcttgacgttgcagaaggcgcaggcccgcgtgcaggtgtcgcccatgatcatcagggtggcgtgcttctggctccagcactcgccgatgttggggcaggccgcctcttcgcagacggtgtgcaggcccttgtcgcgcacgatcgccttggtggcgttgtactggcccgaacccggcgccttgacgcgaagccagtcgggcttcttcaggaccacgctttcgggccggttctgcttttccgggtgacgcagttccgagggcttgcgcgtcagggtgtcgatcagggtgaccatggccggtatttcggactttgcgggccccaaggcaaggcacagagggtaacggcggaaccctcacgcggcgttacgcatcttttcaagatgacgcggcgtcattatggatcgccagctcaacggagcgagggcgcatcaagccctccgaaggagtggacgcttgcggcagcctcttgatccccagacctacgacgaacccatcttcgatgcgctgatcaccgcgcgcgagcggttcggcgacaaggaaatcctggaggatcaggatcggcatccgctgacctacaccggcctgatccgcgccgccttcgtgctgggccgcaagatcgccggcatgaccgaggctgaggaacgggtggcggtgctgctgccgtcctcgtccggcgtggtggtgacgttctttgctctgcacgccttcgcccgcgtcccggtgatgctgaacttcaccgccggcgaggccaacctgaaggcggcgatcaagacggcgggggtcaagaagatcctgtccgccaagcgcttcatccagcaggccaagctggacgagctggtggatcagctgaagaccgtggccgagatcgtctggctggacgacgtgcgcgcctccatcaagctgccggacaagctgtatggcctgaccgccggcgcggcgccccgccgtttccgcaagaagaccgacccggatgcgccgggcgtcgtcctgttcacctccggcagcttcggcgcgcccaagggcgtggtgctgagccagaggaacctggtcgccaacgcgcgccagatctccacccacatccacctgaagccggagtgggtgatgttcaacccgctgccgacattccactgcttcgggctgactggcggagtgatcctgccgctgctcagcggcctgaaggcgttccagtacccctcgcccctgcacgccaagaccatcacggacctgctgccgcaggtgaaggcctcggtgctgttcgccaccgacaccttcctgaaccagtacgcccgcgtggccgagccgacggatttctcgacgctggagttcatcgtcggcggcgccgaaaaagtgcgcgaggagacccgcgccctgttcaacagcaagttcggcgggcctgtgatcctggaaggctatggcgcaaccgaggccgcgcccgtggtggccgtcaaccatccagaccgcaaccgccccggcacggtgggtcagatcctgcccggcatggactaccggcttgagcccgtacccggcatcgatgcgggcggtcggctgctgctgcagggccccaacgtcatgagcggctacatcacggcggacgacccgcgcgcagtggaaccgatcgagggcggctggctcgacaccggcgacatcgtcgatgtggacggcgagggctatgtcaccatccgcggccgggccaagcgcttcgccaagatcgctggcgagatggtgtccctgacggctgtggaaggcatcgccgtcgccgtctggccggaccagcgccacgccgtcgtctccgtgcccgacagccgcaagggcgagcgcctggtgctggtcaccgacaatgcggccgccgagatcgcgcccatgaccgaatgggcccgcaccaacggcgtgcccgagctggccgtgccccgcaagatcatgaaggtgggcgaggtgccggtgctgggcaccggcaagaccgactatgtcgccatccagaagatggtcgaggccgacaaggcggcttgattaaggccgcttacatcctggaatgatcggctgctcaggtagcgccctgtaaaggccatccgcttcagggcttacacgtaaggcttgctctgtgttgtaggagccgccgttcatcgctcgatcatggaagcaaacgacagagccttgcgcatcctggctgacgacccggagcgaaatgaaccagctgcgatcctcctgccaaagttcgacgccgtcctttgtggcttcaacgtgggtgaagccgtaatccgccggcgttcgcagatgcgcttgtcggcgtggtccggtggagttgcggaacgacctcagatcaagccggtcggccacatgcagggcggcgtccgggcttgggtcggcggtgagtaaggccaggatggcaagaagcatgctggagcgtacgccgttaaactgaacgatgaaacatcagggcaccagccgttgaggtgatcaacagccggcgcctgaacctcagccgaccagcttcttggcgatgtcggcgatgaagcggccctggaagcgggcgccgcccagttcgttctcgctggggaagcgcgagccgtcgcccttggtcagggtcgaggcgccgtatggggtgccgccggtgatctcgtccatgttcatctggccgggataggcatagggcaagcccgccacgatcatgccgtggtgcagaaagaagtggtgcatgccgaccagcgtcgtctcctggccgccgtgctgggtcgcggtggaggtgaaggcgccgcccaccttgccggtcagcgcgccgcgcgcccacagaccgccggtctggtcgaggaagttgcgcatctgcgaggccgccgtgccatagcgcgtgcccgcaccgatgatgatggcgtcataggcgtccaactcgttcggattggcgatcggggccgcctgatccagcttgtagcccgactgcctggccaactcttcgggaacgagttccggcacgcgcttgatgtcgaccgtcgcgccctcgacctctcgcgcgccttcagcgacggcctgggccatggcttcgacgtgaccataggtcgaatggtagaggacgaggatcttgggcatggaggcgctcctgtttcgataaccggacatctgcaacagtgtccggcacggtatgtgagagatcaagcctcccggcgcaacccctcaggcgaacagctgaagggacaaatggccctgtagaaggcggcgtcgcccggcgcggcgcggccgtgcatcagccgaaaccggtgctcgaccaccatcgcctgctgctcgatgttcaaagcctcccagcgcaagccgggttccaccgcataggcgtaggcgcggggaccatcgccggcgcggagcttttccagcagcaggttcacgccctgttgcgcctgccagacatgggtcagctcgtgcatcagcacgccctgcagatggactgacgcgtggatgaagttcgcgggcaggctgctcgccggccacaggatccagtcgcgtccgaaccaccgccccggcacgaaggcccggttgaacagccatggcagcgccaggatgcgcacatgcgccagacgcaccaccccgccgaaggtctcccgcgccagctcagcctcttccgccgtcagcgcccggacgccgaacgccgtcatccgcccacatactcccaatgccacggctcatacacatagggcacaaagccgaaccggcgggcgttcgccgcgagccagcggtacgtctggccccgtgacatctccagccggctctccggtctggtggagtccacgccatggccgtccagccgcccgacatagagatcgacggccgtgccggtccgatgcggcgagcagacagcgcggcgcagaccgtcgcagttgccctgctgggcgcatcgcgcggcgtccgcctccggatcgcgaaagccggaaaagatctgcagcagctcgggatcgtccgcgatcaccttgacctcggcgcgagcagcggcggccatgcggcgataggcctccagcacgtcgcggcgcagcagccgcgtcagtcggtccgcatgctcctccgcctccaccagataggcgaggtcggcgatcggcggcggctcgggacaggccccgccgacccgcgccatcacgaatggccgtcgctcctgccacaggccccgcagcacctgaaatgtcgcctggtcgaacacccccgtaccgggcaggccgcgcgcgttctggaacgccgccaggcgctctgcgaagaaggacgtgcccgcgccgcagacggtctccagctccctttgcaccagcggcagataggtctcccatccccactccggccggtcgaagggggtccactccagggtgtgaagagacaccgcgttcgatcccgcctgggcggcccagacctctgcccccgcgtgacagtcttcggtttgagcgcgtgcggcgccggcgaacgcgaaacacagcaggccgagcgcggcgaagaggacgcgaagcatcatgacctcatgcaagcccgacctccatgaccatagcaaggctccgcacgccctgcgatgatgcccggccgactcgcgcggggtcgactcgaggggatcgtccatgccgaccaccgccatccagccccggcgcagcaatgcggtgctggccgccttctccggaccctgcctgccgctggcggcgttcggcgtcgccctgcccgtcaccctgcccgagtactacgccacccacgtggggctctccatcggcgtggtgggcgtggtctttatggcggtgcggctgatcgacatcgccttcgatcccctggtcggctggggcatggatcgcacgcgcacgcgtttcggacgctatcgcccatggatggcggcctcgacgccgatcctgatgctggcggccctgatggtgttcgtcctcgtgcggccgggcgcgggaccggtttacctgttcgcctggctgctggtgctctatgtcggcttttccatcggcaccctggcgcagctgggatgggcgtcggtgctggcgccggagtacgatcagcgcagccgcgtctacgcctggtggcaggtgttcaacatcatcggggtgatcgccattctggtgctgccggcggcggtgatccagctgggcttggggaactacatcgccggcgtccacatcatgggctgggcgatcatagcggccctgcccctgaccatcggcctggccctgatgcgcgcacccgagccggtcaacgccggcgatgccccgcacggcggcttcggcgcctacctcgcgcttctgaagcgcaagacggtggtcaagctgctgacatgcgacctgctgctgggcgtcgcgcccggcatcacgggatcgctgctgttcttcttcttcgaccaggtgaagggctatggccgggccgaggcgtcgctcttcatgctgctgtatttcgtgggcggccttgtcggcgcgccgatctgggcgcggctggcgaaccgggtcggcaaggacaaggcgctggcggtcgccagcctgatcttcgccggcctgtatttcgccgccaccctgctgccgggcgggaacttcgctttgacggcgggcgccatgttcatcgccggcctgccctacgcggccggcctgttcctgctgcgcgccatgatggcggatgcgggcgacgaggtgaggttggaaactggagtggatcgaaccggcttgatgttctccatcctgtccgcaaccaccaagatcggccacgtgctggcgctgaccccctatctgatcctgcaggcggtgggctttcaggccgtggcgccggcgggcggcaccggcggcgtgtcgctggtggtcctccaggtcctgttcggggcggcgcccgccgtgctgatcgcgctggcggcctgggtgctgaagggctatccgctgacgcccgcacggcacgagcagatccgcctcgccctcgccgcgcgggacggagccgccgcatgacgcccatcgaccagctgaaagccgtcatggcgcgcctgcgcgacccggacggcggctgtccgtgggacgtcgagcagaccttcgccaccatcgccccctacacggtcgaggaagcctatgaagtcgccgacgccatcgagcgcggcgacatggacgacttgaagtccgaactgggcgacctgctgttccaggtgatcttccacgcccgcatggccgaggaagccggcgacttcggcttcgacgacgtggtccaggccatcatcgacaagctggtccgccgccatccgcacgtcttcgccgaagaggccgcgcgcggaaccgccgaggcgcagaaggcccgctgggaggacatcaaggcggccgagcgcaaggcgcgcgcccagggcggcgttctggacgacgtgccggtcggcctgcccgccctcacccgcgccgccaagctgaccaaacgcgccggacgggtcggtttcgactggccctccaccgacgaggtgttcgacaagctggcggaggaggtcgaggagttgcgcgccgagatcgccgccggcgacatggccaaggcgcgcgtggagatgggggacctgctgttcgtcgtcgccaatctggcgcgcaagctggaggtcgaaccggaagacgccctgcgcgccgccaacgccaagttcgtgcgccgcttcggcttcatcgaagccgaactgcaaaagggcggccgcacacccgagcagtccacgcttgaagagatggatcgcctctgggacgccgcaaaggcggccgaaaagcccgccgcgtgaactacgacctcatcatcttcgactacgacggcgtggtggcggattcggaggttctgagcagcaccatcctggcggaacaactgacggcgctgggcatgccgaccacgctggaggaggtgctggcccgctatgtcgggcggcgttggcgcgacaaccgcgccgatgtggaggcgcgccacggcaaggcatgccccgacgacttccacgtcggcttcggccaggcctgtcgtgcggaagccgagcgttcgctgctgccggtcgcggggctgcgcgacttcctcgccgcgcggcccgaacgtcgatgcatcgcgtcgtccagcaatctggaatggctgcggctcggcctggatcgcttcgggttgagcgacgccttcgagccgcacctctacagcgcggcgcaccacgtccagcgcggcaagccgcatccggacgtctttctgttttcggccggggacatgggtgtcgatccctcgcgggtgctggtgatcgaggacagcgaggcgggcgtgcaggccggcgtcgccgccggcatgacggtgatcggccttctggccggcgggcacgtgcgggccggtcacggcgagcgcctgcgggcgcagggcgcgcgccatgtcgccgcggactacgcctcggtctccgccttcatcgaagccgtctagacgtagcgaagttcctgcaggtccacctcgcggatcaggcgccgagccgtgacctcgtcgatgtgacgcgagcgcgccagtcgcatcagttcctcccgctcggcggccaggcccgtcaggcgcaggcggcgctcgatctcgtcgatccgacgcgccatggcggcgtcgtcctcggccgcgtgcgatcggctggcgatgcgctggcgatagatctccatcaggcgcgcggccgtatcggcatagaggtcggggttcggccggccctcggccatggcgtgctgggcgtcttcgatggcgcgcagggcggcctcggccgcggcgacgcgggaccggtcctcctctcgctggtgcgagggctcggggggaagctcgatggacttcaacagcggcggcagggcgacggtggccagcaccagcgacaccacgatcacccccgccgccagaaagatcgccaggttccgcgccggcatcggcgaaccgtcgcccagcacgaagggcagcgtcaggatgcccgccagggtgatggctccgcgcacccccgccagcgacatcacagccaccagccgcaagcccacgcggggctgcgcccctcgccggcgtttacggaacagcgtcagcttcagcgacgtccacacccaagcgaagcgcagggccgcaagcgccgcgacgatggccagcacatagacgcccagccaccacacctcgtcgcgcggcgtcgagtcgatcacctccgcggcgcgggataggatcgacggcatctgctcgcccaggatcacgaagatcaggccgttggcggtgaactgcaccgcatcccacaccgccgtgcgccggatgcgggtcgaggccagcgcctgattgctgcgctcggtgaagctcatggtcacaccggccgccaccgccgctaggatgcctgacgcatgcagctcctccgccgccagataggcggcgaacgggatcagcaggctgatcaggatctgcgccccgacatcctccccccagcggcggcttacccacagcttggcgtagctgatggcgaaggtcacggccacgcccgcggcgatcccgcccaccgccagccaggcgaaggtggtcacggcggacgtcagggagaaggcgccggtgggggcggcgatcaccgcgatgcgcatgcaggtcaggccggtggcgtcgttcagcagcgcctcgccttccagtatgtgcataagccgctttgggatcggcgcgcgcgccgccaccgcctgcaccgcgatcggatcggtcggcgacaggatggccgccagcgcaaaggccacagccagcggcatgcccgggatcatccagtggatcaggaaacccacgccaagaacggtgaacaccaccaagcccagcgccagttccagcaccaccgcgcggtcgcggaacaccgcctccttgggaatgcgccagccgtccagaaacagcagcggcggcaaaaacagcagaaagaatatgtccggctcgagatcgacggactctccgctgatcaggacgatcacggcgcccagcgcgatctgcaccagcggcagggcgaccccgctcatgcgcgcgatcgagcccgacaccaccaccgccagcagcaggaacaggatcgtctcgatcaacgccacggcggatcagcccgccagatggggatactgccgctcgaaccggcccagcgccgccgggtgaagccggaccacaaggcgtgtgcggccgtcctcgtcggtttcgcgagacgttacgcggccgtgctcgtacagccaggccagcgcctcgccttgcgcgggctcaaggatgatctccgtctccggatcatcgtcgatcagtccggcgatggcctcacgcaaggcctccagcccctcgccggtccaggccgagacggccgccgccttgccttcgtcgccgaggcgatcggcatgaccgagcacggtctcgcgcgcctccggctccagaaggtcgatcttgttccagacttccagcacccggcggatgcggccttccggcgtcggaatctgcttcagcaccgcctcgacatcggccgcctgcgccgcggtgtcgggcgaggcgatgtcgcgcacgtgcaggatcaggtccgcttcgcccacctcttccagcgtggcgcggaagctctccaccagttcgtgcggcaggtccgagacgaagcccacggtgtcggcgatgatcgccggccggccctgcggcaggcgaatggtgcgctgggtggtgtccagcgtggcgaacagcaggtccttggccagcacctccgagcccgtcagccggttgaacagcgtcgacttgcccgcattggtgtagcccaccaaggcgacggtcgggaacggcacgcgcttgcgcgccgtacgatgcaggccgcgcgtgcggcgcacctcctccagctccgccttcagcttgacgatgcggtcggcgatcaggcggcggtcgagctcgatctgggtttcgccggggccgccggtcgagccggtgccgccgcgctggcgctccaggtgggtccaggtgcggaccagccgcgaccgctcgtagtccagccgcgccagttcgacctgcagccgcccttccttggtgcgcgcgcgccgcccgaagatctccaggatcagtccggtgcggtcgacgaccttcacctcccaggccttttcgagattgcgctgctggaccggcgacagctggtcgtcgatgacggcgacgtccgcctctgccgcgcggatcagggcggcgagttcgtccaccttgcccgagccgaacagggtcgccggcgccaccttgcgcatccggacgatctcttcggcgcggatgtcgagatcaagcgcgcgggcgaggcccgaggcttcgtccagacgctcctgcgcgaggcgcggcgactcggagcgcccgtcgggatgaatgacgaccgcccgctgaacgggggcggcatgatcgatgagtttggaggtcaatcagtcttcttcggtctccggctcgtacagctggacgggcgcggacggcatgatggtggagatggcgtgcttgtagaccagctgcgactgtccatcgcggcgcagaagcacgcagaagttgtcgaaccaggtcacgatcccctgcagcttgacgccgttgaccaggaagatggtcaggggcgtcttggtcttgcggaccgagttgaggaaggtgtcctgaaggctctgtttcttgtcttgcgacatggcaggttggtcctgttcttgattgtttgtcgccggagtttggcgaggggaagcagcggcgaaccttaaccgccggcgccgcaaacccgcaacgcctagatggcctcgcggcgggcttgttcaagatagagttcgcgcagccgcgtcgcgaccggccctggacgaccgtcgccgatccgcacgccgtccagcgacaccagcggcatcacgaacgagctggcggcggtgacgaacacctcgcgcgcgcgtttggcctcctccacagtgaaggcgcgctcctccagctcgatcccttccacttcggccagcttcatcagggctgtccgtgtgatgcccttcaggatgttggcctgcgcgtctcgggtgcgcagcttgccgtgctcgtccacgatccaggcgttggtggacgacccttccgtgaccagccccatctcgtcgaacatcaggcattcataggcgcccttttcgcgcgccgcctgcttggccagcacgttcggcaacagccccaccgtcttgatgtcgcagcggccccagcgaatgtcgggctgggtcacgcccgccgcgccgtttttcgcgagcgcctcgcccttgttcggatcgatcgtcttggccgtcaccacgacgctgggcgccgcatcgcgcggaaaagcgtgatcgcgcgacgccgtgccgcgtgtgacctgcagatagacgatgccgttcctgacccggtttcggcggatggtctcgcccagcacgcgcgacagggcgccgtcgctcatcgggatgtcgatcttcagctcggtcaggctgcgcttgaggcgcgtcaggtgcccttcgaagtcggcgagccggccgtcgaacaccgaccacacctcatagacgccgtccgcgaactggaagccgcgatcctccacatggatcaccgcctggctgtgcggttgatagaccccgttgacgtaggcgacgcgcgacatcaggcggcttcctcctcttcggacccgcgagcgggggagacgcccagggacttgagcttgcggtgcagagccgagcgctccatgccgataaaggcggcggttcgagagatgttgccgccgaagcgcatgatctgggcggccagatactcgcgttcgaacacctcgcgcgcctcgcgcagcggcagcgcgatggtgcgctccgcccccaacgacgacgggctgttggaggtcgccacctcctgcggcagcatgtcggctgttataggctgggccggatccccggtcgccaggatcagcagccgctcgatgttgttcctcagctgccggatgttgccgggccagggatgaacctgcagcacggccacggcgtcgtcgccgatggtgcgtcgcggcaggccctgcgatcccgcgatggtgtcgacgaagaactcgaccagttcggcgatgtcctcgcgccgttccgacagggcgggcacccggatcggcaccacgttcagccggtggaacaggtcctcgcggaaccgcccctcggcgatctcggccttgaggtcgcgggaggtcgaggtgaccacgcgcacgtccacctgcacgtcctgctcgccgccgacgcggcggaacctctggtccaccagcacccgcaggatgcggctctggctttcgcggggcatatcgctgatctcgtcgagatagagggtgccgttgtgagcgcgttcgaagacgccgatcttgcggggtcgaccgtcctggccttcctcgccgaacaattcgacgtcgagccgttcgggcgtcatgccggcggccgatatggcgacgaactcggcgcgggcgcgcggactgttctcgtgtatctggcgcgccaccaactccttgcccgagccggcggggcccgagatcagcacgcggctgttggcctgggccaccttgccgatggtggagcgcagcgcctgcgccgccgccgaacgcccgatcaggccggtggggaccatggtctgggcgcgcagccgccggttctcgcgcctcagggtcgccgcctcgatggcgcgctcgaccaccaccaccagccggtccgacttgaacggcttttcgatgaagtcgtaggcgccccgtttcagcgcgctgacggccgtctcgatgttgccgtggcccgagatcatcaccaccggcaggtcggagtccagccccttgatgacgtccagcagctccagcccgtccagcccgccgccttgcatccagatgtccagaatggccagcgacggccgccgcgcccggatcgccgccaaggcctcgtcggagttggaagcgacgcgcaccgcgtgcccctcgtcctccagaagcccggagaccagctcgcggatgtcggcttcgtcgtcgacgaccagaatgtcggaacctgtggatcgcatcaggtctcgctcctattcagccgcgaccagggcgcgggcgggcgccgggtcgccggcgacgccggtgggttgcagggggaagatcaggcacacgcgcgcgccgccgaaggtctcggcatcggccagcttcagctcgccgccgtggtcctcgcagatgcgcttgacgatggccaggccgaggcccgtgcccttctcgcgcgtggtgacatagggttcggtcaggcggtcgcgatcgcgcgacggcaggccgacgccgtcgtcctcgatcacgaacacggccgcaccgctttcgacgaccagtgaggcgacgacgccgccgtctgcgtggttgtcgacagcacgtcgcgccatcaccgcttcgccagcgttcttcaggatgttgaccagcgcctgtcccaccatgcggccgtcgcagtgcagaaccgcgatcggcagcggctcgacgagctgcagcgccacatcggggctcgccacgcgttgcgcgaacaccgcctgacgcaaaagctcggccggatcctcacgcgcaaagcgcggggcgggcatccgcgcaaaggacgaaaactcgtccaccatccgcccgatgtcccccacctggcggatgatggtgtcggtgcagcggtcgaagacctccacgtcgtcgccgacctggggccgatagcgccgtttcaaccgctcggccgacagctggatcggcgtcagcgggttcttgatctcgtgggcgatgcggcgggccacgtcacgccaggcggcgttgcgctgtgccgtgaccaggcgggtgatgtcgtcgaacgtcagcaccatttcgccgccgaagccgccttcgatgcgcacacgcaggcgccgggtctcgccgtcgcggctgacgtcgatatcctcttcgatgtgcgcctcggcccgccccaccagatcgctcagttcgggcgaaagggtcgccagaggctggccgtgcacctccccttcggggatggccagcagttggcgggcgctgtcgttgatggccgagatgcggccatggcggtccagcccgatcacgcccgctgagacccccgacagcacggtctcgatgaagcggctgcgatccttggcctcgtcgcctgcggccttgagcgcgctttgctgggcctgcaggtcttcggtcatgcggttgaaggcgcgcgacaggtcggcgatctcggcgggcgcgccgccgtcctccacccgcacggtcaggtcgccgccggccgcctggtcggccgcccgcaccagccgtcctatcggcgccgaaatcgcgctcgcggccgacatccccagccacaccgccccgaccagaaccagcagcgccgtctccagatagctgagcgcaaacacggtctggatcagggcgcggctgtcctgcgcctcgcgataggcctgaatggaccggctggagtcgttcatccgcgcgatcagcccgtcgcgcagcggccgcaccagatagagataggcgtcgccataagcgggcaaggcgatgatcgaacggacggtgtccgggttctgcgtcacctgctgcggcggcttgcctccctcggccgcggcctccagctcagaacgcggcggggacaggtaaggcggcgctccgggctgctcgccccgcgccagcacctcgccttccccgttcaggatgtagatcgccggatagccgaagatctgcccgacctgggccagcgcatccgaaaactggatgcgttgttcgaacagcggacgggcactgtccagctggtccgcgatggtcaggaggtcggcatccatggcggcggacacgtcgccgatataggcccgcccgatctcggctccgttctcgaccgaggcctggacgttctggctgaaccactggtcgacaccacggttgaccagcatgccgaagatcagggcgatcaggatggccggcgcgacagccacggcggagaacaaggccacaaagcgcaggtgcagccgcgctcccgcctcctgccggctcctcgccagggccagcacgcgccgtccaagcagggccgccagcacgccgatcaagacaagattggcgaacagcacgtacagcacgatgtcgccggcggccgcccgcgcgccgcccgaggcgctgggcgcgacggcgaacagccagatgctggcggcggtcaccagggccgccaccgcataggcggcggcgaaggcgttgcgggctcgcccgtgctgcaatcgaccccagaacgacccgtgcgccagatcggcgtcggcctcagggatcaggactgcgggcgtgtccgtcatgccatggcagtttccgacacctgttgcccgctttcaacagcagagttgcgcgtttgcgccatttcttgccgccagagtgcggaaagcgcggcttccacctcgcccggcgtctccaggcggcagagtgaggccttggccgcacgccgatcggcggcctctgcgggccaaggcgcctgctcgatgtaccagcccaggtgcttgcggaacatcttcagacccagcggcaggccgtagaaggcgacggaggcgcgcagatgctcgatcacgatagccagtcgctcctcccggccgggttcgcgcagccgttcgccgtcctccagcgcccgatcgaggtgcgacgccagccatgggcggccgtagacgccgcgacccagcatcagggcgtcggcgcccgagcggctcagcgcctcgcgcgcgtcctcggcggtcaggatgtcgccgttgacgatcacggggatggacaccgcgaccttgacctcgcccaccgcgtcccaatccgccagaccagtgtagaactgcttgcgggtgcggccgtgcacggtcaccgccttcacgccgatcgtctcggccgcgcgcgcgagctcgggcgcgttgcggctgtcgtcatcccagccgagccgcatcttgaccgtcacgggccgcgcagtcgcgccgaccaccgcctccatgatccgccgtgcgaggtcgggcgtgcgcatcagcgccgagccggaggcgacgccggtgacctccttggcggggcagccgaaattcaggtcgacgatgtcggcgccggcggcctcggctatccgcgcgccctcggccatcgcggcgggatctcgcccgaccagctggatcaccgtcagcggcagcccctcgcccaccgctgcgcgccgcaccacgtccggccgtccccgcgccagctcggcagaggccaccatctcggtcgccacataggcggcgcccagccgcgaggcgacctgacggaagggcaggtcggtcacgccggtcatcggcgccatcagcacgcggccggggatcgtcacgtcgccgatctgaagggatgaggtcatgcgcgcctcttcgccctccttcgcgccccctcgtcaagctcgaccgcgccgcctagaaggccgacatgaccttttcagccattgtggtcgcggcgggctcgggctcgcgcgcgggcggcgacaagcagtatcggctgctggccggcaagcccgttgtgcgctggtcggtggaggctcttcagggcgcgggcgccggcgaaatcgtggtcgttgtcgcgcccggcgacgaggcgcgcatggcgcaggcgctgcacggcctggcggggtggagagctgtcgcaggcgggatcgagcgcgccgattccgtccgttctggcctggcggcgctgacctgcgcgcccgatgcagccgtgctgatccacgatgcggcgcgcccgcttctgtcccgggacatcatcgagggcttgatcagggcgctggaccacgccgacggcgccctgcccgccctggccgtcgccgacagcttgcgtcgaggggatgcggacggcgtgatggcgggcgccgtggatcgcgcaagcctgtggcgcgcccaaacgccccaagcctttcgccgcggcgtcatcgagcgcgcctacgccgcctggccccgctccgagccgcctaccgatgaggcgtcggtggttcaggccgccggcggaaccgtccgactgatcgagggcgatacccgcctgctcaaactcacctaccctgaagatttcgccgtggccgaagccctgatcccccgccagacccgcatcggctcgggctatgacgtgcatcgctggggaccgggcggatctgtgtggctgtgcgggatcgaggtgccgcacgaccagacgctgatcggtcattcggatgcggacgcgggtctccacgccctgaccgacgccatcctgggcgccttggccgagggcgacatcggcgatcacttcccgcccagcgatccgaagtggaagggcgcctcgtctgatcaattcctgttgcatgcggcaggcatggtcgaggcgcgcggcggccgcatcgtcaatgtcgatgtgaccctgatctgcgagcagcccaaggttaagccgcaccggctggccatgcgcgagcgcatcgcccacctgcttcagctgccgctggacgccgtcagcgtgaaggccactacgtccgaagggctgggctttaccgggcggggggaaggcctggcggcccaggcggtctgcgcgatcgaactgcccgcgcctcagcccgccgcatagcgcatctggcgcaccagcgagccgaacaggttgacgtagtcgtcggtccagggccgcacctcggtcggcgcgagcgttcgccagcgcggatcggcgcggaaggcggcgagcccggcttccgtcggcgcgatcaccagcgcctccgtcgaggcttcggacatgtccggctgggccggatcctcgatgaacacctggtgcaggctgggcgcattcagcgtctgcgccgccgccgacgccggcagggtgatctccagattgcggttagacaggtgtagcaccacggccccatccggccgcagcagcctgagatagccggcgatcgcctcggtggtcagaaggtgcgtcggcaccgcatccgaggagaaggcgtcgatgaccagcaggtcgtacgaccccgccgactccttgttcagcgtcagacgggcatcgcccaacaccgtacgcaccggcccgtccgcgcagtcggagatgaaggtgaaccagcgcggatcgcgcgacagccgatccatcatcgggtcgatctcgaaaaaggtcagccgatcctcggcccgcttgtaggcggccatggcgcccgagccctgcccgaccacgccgatgttcgcaccgttgggacgccgctcctggatcttcagcgccgcctgccccagcggcgtgcccgtggcgtagtagagggtgggcgagcagcgcgacacaggcgaggtcggctgcgcgccgtgcagcgtggtgccgtgcatcagcacatgaacgtcgccgcccagtctggcgtcataggtcgtcgccacgcgcatcacgccgaagaagctgcgctccgacaggttccactcatagccgcgcgggatgtggtgcgccgaagccgtcagcatggccagcatcagggtgaagaccggcgcgcggtcccgcaccagaaaggcgcaaatggcgcccaggccgaacaccagctgcgaaatgtggatcagcgcctggttgctcagcaccgcccggatgtccggctgatagcggatgatctcaagcgcgatcggcggagtcaggatgatgacggcgcccagcgcgatcgccgcgatctcgacccggctgagcggccccttgtcccagggccgcgccaggccgacgaggaccagcaccagcggatactcccacaccgtgttgaacagcaccggcgccagcagggcgttgaaggcgccgcctacgacacctcctaacgacagcagcagaaaaaactcggtcagccggtcgggcgccggacgccgctgcgccaatcgctggtggcacagaagcgcgatgaagaagaaggccagcaggtgcatgccgaacagcaccacccactcgccggtcttgaacgccgccatgctgaccaccgccgcgcccaacgccgccgaaagcaccagggtcgtctcgaacggaacgatcggccgggccgaaaaggcgatcacgaaggtcagcagatacagcgccagtggcgcgacccacaggaagggcgccgacgccacatccaccgacaagtgggccgtgacgcccagcatcaggctagagggcgcggcggccagcagcaccagcacgcccttctcgcgccaggggatcggcgggctggccgccagccccgccggcgcgctcgccgcgatctcccgccgtctccagatcgccacgcccagcaccgcgaccatgacaacaaacaccccgaaaccgccgctccatccccaccgctggcccgacaaggcggtcagcggctcgatcaggatcggataggcgagcagggccagaaagctgccgaggttggaggcggcgtaaagaacgtacgggttggcgccgtccgcatgccccgcccgcagccgcgcgaaccacgcctgcatcaggggcgccgtcgccgacagcaccgcgaacggcgcgcccaccgaaagcgccagcgtcgccaacagccagacgatcggcgcgttcggatcggggtcgcccagcaggccgctgatcctcagcggcagaaacagcgccgcgaccagtagaagcgccaggtgcacgccggcctgcgccttcagcgaacccatccgctgcaggccgtgggcgtaggcgtagccgaccagtagcgccgcctgaaagaacaccatggaggtgttccacaccgaaggcgacccgcccagcatcggcagcaccagcttggtcaccatgggctggacggtgaagaccagcgccgccgaggtgaagatcgcggcggcgaacagcacgcgcgtctgcgatccccgtcgtcttgccggtgctggagaaagggccgcgtcggtcatgaggctggttagaccggatcgccccggataagaaaggccatgacgccgcacgacattgaagctttggcccaccgcgtgatcgagacggctgcggccaaggggctgatgctggccacggccgaaagctgcaccggcggcctggtcgcgggggcgctgaccggtgtggcgggctcgtccgcggtggtcgatcgcggcttcgtcacatacagcaacgaagccaaggcgcagatgctggaggttccggccgcgctgatcggagtccatggcgcggtgtccgaacccgtcgcccgcgctatggcggaaggcgcgcttcaacgatcccaggcgcaggttgcggtcgcggtgacggggatcgcggggccgggcggcggctcggcggacaagcccgtcggcttggtccatttcgcggcggccggccccgacggagtcgttcaccacgccgcgcggttcggcgacatcggccgtgagggtgtgcgtctcgccagcgtggagcaggcgttgcatatgctggccgcccggatcgccgccgcgtgagttcgcccgtcgtcgtcgacgcgcggggccacgcctgtccggtgccgaccctgaagctgatgaaagcgatgcgcgcggcccaggccggcgatcgtttgatccttttagcgacagacccgatggcgcggatcgatgcgccgcacctcctcgctcagcgcggcggccgcctgctgtcggtcaccgaggacgcgggtgtgctgacgctcacggtcgagtgcggggatcccggccctgcgccagacgcccgcgcgatggaaagctgaccaccgaatcttcgggatcgcgcgccttctccgccgcccgagccttcgcgatctccatctcggtggcgaaggccccgccatagaagacggcgttgacgttccaagacagccagatcagcagcaccaccaccgcgccgaccgagccgtaggtcgcccccagcggcgcgatctgctccacatagatggcgcacaaccacgacgacaccaccgacatcagggtggcgaccgagccgcccaccaccgccggaagccaggccaccggcgtccggtgactcatggcatagcggtagagcagcgtcagcccgaccaccagtccggccgagggcgccacggcgtcgaacaggacgcccagccccatcaacgacccctcgcccgaggcatgccccaagattcgaagggtgaccaccgaccccgacaccacggtgaacagcacaaaggcgaacaccgcgacgaaaaaggccaggaggttgaacttgaagaagccgtgcggctcggtctcgtcatggatcaggttcagcccggccagcagcgccttgaaccctcggtgcgcggcataggcgccgaccaggacggcgaaggcgctctgggcagaaaccgtgcgcgccgaggcgttggcgagccgtccgatctcttcgcggaagattccctgcgccgcgtgcggcatcagctcggctagggcgaaggcctgctcgctgacctgcccgatcgacagcaccgccttgtagaagccgatcaggatcgcaatcgccggaaatacggcgagcagcgcaaagaacgacaccccgcccgtgtagagcatgacatcgcggccccagctgcgggcgaaggccctgccggcgagccgcgcgacgttccctggtccgaaaagcaagctggtccccgcaatatgcgcgaaaaccggactaactagcgcaattcgctcagccgcaaacccttggggacattttggtcggccggccgcctcggcattgcttcgtaaaggaagcgctcgttatgctcgcgctcacatgcgggcggccagttcacggatgaccaccagattgatcgaggcttccgacatcgagagcccgcccgcgagcgcgcgcgtgctggtcctgacggccgacgaccggctggcggacctggctcacggactggacggcttcggctggcgcacgctgatctcggacagtgtcgaaggcgccgctgtcgccctggcggacctgccgctggaagccgccatcgtcgatgcggcgatgctgtcgtcgggcgtgatcgccacctttcgcgccgccgccgagccgcgccgcctgcccgtcgtggtgatcggaaccccgcaagaagcaagcgcggacgccgatctggtcatgtctacgacgccgcacccggcgcaggccgccttgcggcttcagcagctcggacgcgccgccatcgccgaggaggagttccatctgcgtcggctgaccttcgccgaacgcggcgaacctctgggccgtatcgaggacgaggcggtcggtcccttgcgcatcctggcggcgggcgcggccgatcggcgctttctcgccctcgccaacgcgctttccgccggcggcgcggaggtggtggcggcccccacgccttacaccgccttcgactatttgcacgaaagcgcctttgacgcggcggtcctgtggggcgccgatgatcatgcgccagcgctgtcgatcgcctcgggcatgaagcgcaacacccgcctctatcatatcccattggtgctctatttgcgcggtcgggccgaaatcgatctgggcgagctttatcagcggggcttcgccgacgtggccgcctccgatacgcccgaggacgagaccgccggccgcatcctgggcctcgcccgcacgcatcgtcgccagcaggtgacgcgtcgggcgctggacggcgtacgcggatcggggctgaccgacgcctcgaccggcctgttcacgccgcagcttttcgccgcccacctgactcgcgtcgcccaggccgcgcgccttcgccagcgcccgctctcggtctgcgtgctgcgcgtgcggcagagcgacagcgtggtggcgtcccgcaccgggggctggcttgatcgggccctgccgcagatcggggccatggtgtcgcgcctggtgcgtgtcgaggacaccgccgcccgcctagcgcccgaggtcttcgccctgacgctgcccgccacgcgcgcgggcgaagcgcggctggcggccgagcggatcgccgcggtgatcggctgcaccgcctttgacgctggaccggaccgatcgccgttcgtggtcgacttcgacgtcggctgcgcccagctcggcgtaggcgagaaccccgccgctctgctggagcgcgcctcggccgacctctacgcgcgctcgccgcgctaggcgacgctcatcaagcggacgccacccgcgccaggtccgaggtgatccgttcggccaccttcagccgctcttcgggcttgggccaatcgccggtcacgacgatcttctggtccggccggatcttccagaaggcgtgatttttctggatcaggccgacaagaccgccgggattggggaagctgttttcgcgcagcgtcagcaccgcccccttgggcccgatgtcgatcttctcgatgcaggcgcggcggcagttggccttgatgccgacgatccgcagcagttgctgcgcctcgtcggggagcggtccgaaccggtcgatcagctcggcggccaaggcctcgcgatcctcggcctgttcggcgtcggacaggcggcgataaaggctgaggcgcacgttcaggtccggcacatagtcctcggggatcaggaccgacgccccgacgttgatcgacggcgaccagccgcgatccaccgcgccctcgcccttctccttcagctctgcgaccgcatcctccagcatctgctggtacagctcgacgcccacctcgcggatgtggcccgactgctcgtcgcccaagaggttgccgccgccgcgctggtccaggtcgtgactggccagctggaaaccggcgccgaggttgtccagcgactgcagcacctgcagccgacgctcggccgacagcgtcatcggcttcttgggatcggtggtcagataggcgaaggcccgtgctttggaccgccccacccgtccgcggatctggtacagctgagcgagaccgaacatatcggcgcggtgcacgatcagggtgttggcggtcgggatgtccaggccgctttccacgatggtggtcgagaccaggacgtcgtactcgccgtcgtagaaggcgctcatcacgccttccaactgggtcgcgctcatctggccgtggccgacgacgaacttcacctccggcacctgctcgcgcaggaagcgctcgatgtccggcaggtccttaaggcgcggcgcgacatagtaggcttggccgccgcgatacttttcgcgcagcagcgcctcgcgcaccagcaccgggtcccatggcgtgacataggtccgcaccgccagacgatcgactggcggcgtggcgatgatcgacatctcccggatgcccgtcagcgccatctgcagggtgcgcgggatcggcgtcgcggtcagggtcagcaggtgcacgtcggcgcgcagcgtcttcagcttctccttgtgcttgacgccgaagtgctgctcctcgtccacgatcactaggcccaggtcgcggaagccgacctgttcggccagcactgcatgggtgccgaccacgatctcgaccgagccgtccttcagccccgcgcgcgtctcattggcctccttgccggtcaccatgcgcgacagctggcggaccttgaccggccagccggcgaaccgctcggtgaaggtcttgaagtgctggcgcgccaagagagtggtgggcgcgacgatcgccacctgctggccggtcatggcgacgacgaacgcggcgcgcagcgccacctccgtcttgccgaagcccacgtcgccgcagatcagccgatccatcggcacgcccttgccgaggtcctccagcacgtcgccgatggcgttcagctggtcgtcggtctcttcgtaggggaagcgggcgcagaactcggcgaacaggcccggcggcggcgtgacggcgtcggtctggcgcaacgcgcgcttggcggccagggcgatcagcccctcggccatagcgcgcagccgctccttggccttggccttgcgcgcctgccagcccgcgccgccgagccggtccagctgaacgccgtcggcatccgtgccgtagcgggtcagcaggtcgatgttctcgaccggcaggtacagcttgctttcgccggcgtagagcagctccaggcagtcgtgcggcgcctgctggatatctagcgtcttcagcccctcatagcgcccgatgccgtggtcgaggtgcaccaccagatcgccggtggtcagggccgacgcctcggccaggaagttggacgcccgacgcttcttgcgcggccgggccagccggtcccccaggatgtcggtttcggagatgacggcgacctcgtcggtgacgaagccgtgttcgaccggcaggaccccgcgcagatagacgccctccggcgccgcctgtacatcggcccagtcgcgcaccgccactacatgctgcaggccgtgatccgacagcatggcctgcagccggtcggacgagccctcggtccaggaggcgaacagcacccgccggccttcggtcttcagggactcggcgtgccgggccacggcctcgaacaggttgacgctgtcctgcgaccgctcggcggcgaaggtgcggcccagccgcccgcccgcgtcctcggcgccgcccgcgaaaggcgtcagccgccgcacgttgcggcccgccagggcgccgttccagtcgccttcgctcagatacaactcagccgggggcagcgcccggttcgcggccgccgcgcccttggtcttcgccgcctcgctacgcgcgtcataggcgtccgccgccaggtcccatcgctcggcgcgcgccgccacgacctgatggtccagaaacaccgccgcgtcgtctggaagatagtcgaacagcgtgtccagccggtcgtagaacagcggcagccactgctccatgccctggcgtcgcgcgccctcgctgatggtggcgtacagcggatcgtcgcccggcgcgccaaacagcttcagatagccggtgcggaagcgcgagatggcgtcccggtccagcagcacttccgagactggggccagcgacaccgccgtcatctggcccgtcgagcgttgcgtctccggatcaaaggtgcggatcgactccagctccgagccgaacatatccagccgcaccggctcgtcaaagccgggagggaagacgtcgatcaccccgcctcgcaccgcgaactcgccgcgctccgacacggtggaggcccgcacatagccgttggcggcgaaataccgctccaacgcctgcgtatcgagatcccgcccgaccttggtctcgaagcccgcggccgtcgtcacccgcttcggcggggtgcgctgggtcgcggcgttcaccgtcgtgaccaccagcagaggcttgtccgaaaccgtccgctgcgcgagccgcgtcagcgtcgccatccgttgcgccgagacgcccgccgtcgggctcagccggtcgtagggaaggcagtcccaggcgggatactccagcacttcaatatcttgcgaaaagaagcggaaggcctggatgaaagcggcggatcgtccgtaatcccgggcgacgaacaggccgacgccaccggccttcagccgctcggcgacgaccagcgcatccaaaccctcaggcgcgccgccgaggtcctgatccgtgcgatgttgaacctgcgcgtccatcagccggctcccttggccacttccgacgccacgtgcgcgcgcatgaaggtgcggatcttgcccatcagggcgtggtcgtgctcgggcggcgtcggctcccgctcgatgatccagccgtagaggaactggtcgtcttcgttcagcagcccttcaaaggcgtccagctcatcgtcgctgaggctcggccccacctgatcggcgaacggccccagcaccaggtcggcctcacgaaagccgcgtcgccaagcgcgaaagctgatccgccccagcctctggctcttcaggtctttgatgtcgggacgcgcgtcggtgtcggccacaagaatccttgcccgctcgggtctgaaatcggaagcggtcagatagcggctcaggacccgcttcgccagcgcctccggtctcgctatgttccgcccgacatgcggccgccgattctctttcccctgttcgccgaggtgaccagcctgaaaggcgtgggcccgcgcatggcgccgctggtgcagaaggtcgccgggccgctggtgcgcgatctgctgttccttgccccgaccggcgtggtggtgcgccgtcccatgaccgccgccgacgcggtggagagcgagtacgggattttccaggtcacggccgatcgcctgttcacgcccggccgccccggtgcgccgctgaaggtgcgcacctccgacgccaccggctttgtgcatctggtctggttcggcggctcgccccagcagatcgaccgcctcctgccgcgcggcgagccgaggatcgtctccggcaaggtcgagcgctttaacggcgaggtgcagatcccgcatcccgatgtcgccacgctcgacaaggctggcgagattcccgcggccgagccgacctatccgggcacacaggggctgacctcgcgacaggtccgccgcctgatcggcgccgcgctctccagcgcccccgagatgccggagtggcaggactccgcctggatgcaggcgcgccgatggcccggctggcgcgcggcgctggaggcggtgcatgcgccgatggcggaggccgatctgtcccccgacgctccgtcccgccagcggatcgcctttgacgaattgttcgcgcaccagttggcgctggcccgacgccgccgcgcccgcctcatccacccggctccggtcatcgcgcccggcgaggcgtcgcggcgcatggaagccggcctgcccttcaccctcactggcgcacaggcgcaagccgtggccgagatccgccgcgacttgtcgtcgggccagcagatggggcgcctgctgcagggcgacgtgggatcgggcaagaccgccgtcgccgccctcgccctggctgatgtcgccgccagcgattttcagggagcactgatggcgccgacagaaatcctggcgcgtcaacattatcagcggcttgcaccgatgttctcagacgcaggcgtcacggccgttctgctgaccggccgcgacacggcgagcgagcggcgcgagcggctggcggcgctcgccagcggcgaggcgcagatcgcgatcggcacccacgccctgttccaggacgccgtccgctttgaccgactggcgttggcggtgatcgacgagcagcatcgcttcggcgtgaacgaacgccagcgcctgcaggccaagggcgatccgcggctgggcgccgtgcacctgctgaccatgtccgccacgccgatcccgcgcacattggagctgacccagtacggcgagctcgaggtcagccgcctgaaggagaagccgcccggccgcaccccggtgaccaccgccgtcctgccgctggcgcgcatcggggaggtagcgaaacggctgaaggcagccattgacgccggcgcccaggcctattggatctgcccgcttgtcgcggagtcggaggcgacggatcttgcggcggccgaggcgcgcgccgccgacctgcgccgaatcctgaatgttgaggtcggtctcgctcacggccagatgcccggcgcgcagcgcgaggcggtgatggccgacttcgccgacggccgcatcccgctgctggtcgcaaccacggtggtggaggtcggagtggacgtccccaacgcctccatcatggtgatcgaacacgccgaccgtttcggcctggctcagctgcatcagctgcgcggacgcgtggggcgcggcgccaaggccagttcctgcatcctgctgtacggcggtcaggacggggcgctcggagaaacggccaaggagcggctggagacgctgcgtcgctcggaggacgggttcgaaatcgcggaggaagacttcagactgcgcggcgggggcgatccgctgggcctgcgccagagcggctttcccgcctatcgcttcgccgacccggtgcggcaccgctcgctgatgatggccgccgctgacgacgcccggctggtgctggcccgcgacccggatctgacttccgaacgcggccaggcgatccaggtgctggaggagctgttcgactggaaaggccacaaggctggcgccgactgatcagccgatattcgtgctccaaccgtcataggcgacttcgacattggctggaactatcgccgacaaggccttgtaatccatatcgatgtgaaggtttgtcaacagcgccctctcgacgcctgatcgcgcgatccagtccagcgcccggtcgagatgggcgtgcgttggatgcggcgtgtagcgcagcgcgtccacgatccacagccgacacccccgcaccgcctccagcgccgcttcgtccaggtccgacacgtcgctggaataggcgacgtcgcccagccgatagccgacagatcggatcggcccatgcccctgatcaaaggtcacgaccttgatcgacccgccctcgccctccacgctccaggactccccgtgcggcgggatcatgcgggcgtccagcagcggcggataaccgaactggctctcgaagatgtagtggaaacgctgcgtcagggccgcgtgggtggccgcatccatccacgccgggatgcggctgcgcgcccgcgtggcgaaggtgcgcagatcatcgatgccgtgggtctggtcggcgtggtcgtgggtgtagagcaccccgtcgatgtggcgaacgccggcgctcagcatctgctcgcgcaggtcgggcgaggtgtcgatcagcacgttggtgacgccgcccccgcctgtccggcgagccagcatggagcaacgtctgcgccggttcttcggctcggccggatcgcagtcgccccaatcgccgtcgccgcgcggcaccccgccggaggaaccgcatcccaggatcacgatctccagcgcactcaaactcttcaggcctccgggcgggggatgcggtcgaacagggcgaagaaggcgtcggtggtgcgccggtccgcctcctccgcactccagcccctgatctccgccagcttctgcagcacaaggccgatgtaggcgggttcgttccggcggccccgatatggaacgggggccagataggggcagtccgtctccacgatgatccggtcggccggcatgtctcggaccagcgcgcgcacctcctccgccgccttgaaggtggcgatgccggagacggagaaccaggcgcccatttccgccgcctgccgggccagctccgcaccgctggtgtagcagtgcatcagcatccggaacggccctcgcgcgtgctcctcgcgcaggatctcggccatggccgcatccgcctcgcgcgtatggatcaccagcggcaggccggtctcccgcgcggcgtggatgtgctgacggaacacctgcgcctgcccctcgcgcgggctgaggtcgtagtggaagtcgaggccgcactcgccgatccccaccactttcggccgagccgcaaggtcgatcagcgtctcggcagttaggtccgcatgatccttggcctcatgcggatgaacgccgaccgtgcaccagatgtcctcgtgcgcgacggccagcccgtgggtcgcttcaaaggtcgacagacggtccgaaatctcgaccatcagccggacgcccgcctctcgcgcacgggcgatcacggcatcgcggtcctcgtcgaactgcggcgcgtgcaggttgacgtggctgtcgatcagcatcagccgagcgcctttgtcttgcgaagatcatgcagggctccggccagcacatcggcccggtccaggttcagcccggcggcccgctccggcaggacgctgagccgctcccatagttcggcccagcgggcgccgacacccggcggactgctgagggcgcgcatgcggaccgccgcaatcagccggtccatcagggtctcgaaccgctcggccccgtccgcaccgcgaaacttgtcggcgatcgccagggcctcggcccgatccgcgtccgcgcccttgacccagccgcgcgccagctgatccatctcgaacgtcgcgccggacgccagcgccagcgccgcgcccggcgatccacccgccatggcggcggcgtgttccgcgtcctcgcggtctgcgccggtcctgtcgcgcacaaggcgctccaaccgatcctgcggccacgagggcagggtcacgcgccgacagcgcgagcggatggtggccagaagccgcccaggcgcatgggtgaccaggaacagcacgccgcgctccggcggctcctcaagaaccttcagcaaggcgttggcggcgttcatgttcaggtcgtcggccgcgtcgatgatggccacgcgataggcggcctgagacgggctcttggagaagaactccggcagttcgcgcgcctgatcgaccgagatcgacttcttctgcttgccgccctcgacggctcgctccagcaccagcagatccggatgcgcctgggccgagatcaggcggctgaccggatcgtgcggactggcgcccagcgggccgcgcaccggatcggcctgtgcgcccaacagacgccgcgccgcgcgataggcgaaggtcgccttgcccgcgccctcgaccccgcacaccagccaggcgtggtgcagccggccccgcgccagggcatccagaaaggcctcctccgccgccgtgtcgggcagcaggtcatagcgatcgcgcggatgctcgctcacagcagccggtcctcgactgcgctccagacccgcgcctccacctcctccagcgtcccgaccgcatcgatgcgaacgcagcgttgggggttggcttcgaagatgcgcaggaagccctcgcgcagccgctggtgaaactccaagcccttggactcgaaccgggtttcgaacagcccccgcccgaacgcgcgctccaagcctacatcgactggcagatcgaacaccagcgtcaggtccggctggtcatcgcccactacgccccggtccatctgctcaatgaactcgggcgcgaccccgccgccggcgccctggtaggcccggctggagtcggcgaagcggtcgcacacgacccagtcaccggccgccagcgccggtcggatggtgttctccagatgatccgagcgcgaggcgtacatcaacagcgtctcggtgatggccgaccagttctcggcgtcggaagccaccaccaggttgcggatgatttcggcgcccctggagccgccgggctcgcgggtgcggatcacgccctgaccgcgctcagccagaaccggagccagccgcgccatcagccggccgacctgggtcgacttgccggcgccctcgccgccttcgaacgtgatgaacctgccccgagtcacgccgggcacaatggcgcgtgcggtcagaagggcaagcccgccttccgcttatcgcgtagatatcagcgccgcatcggcatagccgcgcgcaaccaccgactgccgggcggcctcggcggcgttggcgtcaggccagggcccgaccagcacgcggtacagttcgcgcccgccgacgctggcggcgctgacggacgccggcgctccgatcccctcggccatcagccgcgccggcaggggatcgccgaacgaacccgcctgcacccagaaggtcgagggcggctcggccaccgcctgacgcggagcgggtgtcgcagctgcaggtgcggcagcctgcagcagcagacctccgcccagcctcggggcgcggccaagatagcgcacccgcacttcgcccacacccttgccgatcaggtccaactgctcggcggcgccgcgcgacaggtcgatgatgcggctgtccacgaacgggccccggtcgttgacgcgcagcaccacacgccggccattggcgaggttcgtcacctcgaccaggcccggcaggggcagggtcttgtgggcggcggtcagcgcatgcatgtcgaaccgctcgccggtggccgtcggccggccgttgaactgatctccgtaccaggaggccaggccgacctcgtcgtagccgggctgctcctccggccggtaccagcggcccttgatctggtagggccgcatggtgcccgtgacgatgggtgcgggatcgctgaccggcggcggcgcgacggccagcggcgcaggcccgccgtcgcttggcccgcctccgccgatgctggcgcaggcggccaggagggagaacaagcccaggatcagaagtccccgcaaccctcggccaaagcctgggttcatcgtcggggcgggaagatcgatcgcgtgcgccatgccgaccagcttggtccgccaacgcttccattctggttaaccggagcttgccgacggtcagatccggtagatgcggtccagcacgtcggcgacctcgatcaggccggcgatagaaggatcgaagcgctccccggccgccattcggcgggcccagtcggcggcggcgcgtccgccccaatcttcgggcggagacgccagaatctctcggcttgtgccgcggaaccgctcggtcgtgaagtcgtagaaggagccgccgacgttgcgcatctccgcgccgcctccgctaccgtagaagccggcggagatgaccgcgtcctgaccggcgggcagcttccacgagcaggccaggcgaaccaccgtgccgccctccagcaccagcgtggcgaccgcataatcctccgccttgtcgcggctcttgagcggccggccctcgctgaacaggtgcgagctcacctcgaccacctttggcgaacccagcagccacagcgccaggtccaccaggtgcacccccaggtccatgacgcagccgccgccggacagcgcgggatcgtagaaccagggcttgtccgggccgtaggcgttgtggaacgtcaggtcgatcgcgtggacatggcctagttcacccgcctgcagcagctcgcggatgcgccgcacgccctcggtgaagcgataggacagatcgacgcccagcagccggtcggccgcgcgcgcggcgtcgatggcggcttccgtctcggcccgattgcggcccagtggcttctgacagaagaccgcgacgcccgcctccagcgccctgatcgtctgctcggcgtgcaccgcgctgggggtggcgatcaccagaccgtcgaggtcctgcgccaacagcgcatcgagatcggctacgcgcgccgcagcgggcgccaacgcctgcgcgtccgcgaccgcgccgtcgaacgggtcggacacggcgacggcctccaccgcgcccgtcttgagcatgtgctccatccggtgccggccgatccagcccacgcccaggaaaccgatacgctgccgccggtgagcggcgcctgcgggacgttcgatcgcgaggtcggtcaaagcgtcaccagcgccttcaggaagccgtccggccggtcgcgcgtggcgtccagcgcctcgcccagacgatccagcgggtaggtgtggctgagcaggggctcgatgtccaaacggcctgacgccactgcttcgaccgcctcgcgcaccccttgcgcatagacggccggatcgcgttcgtgcgcgctggcgatgtcgaagccgcgccagttccacagttgcatgttcacctgacgcgggccgtcctggtgatagccggcgatgaccagccgcccccgctcgcgcgtcagttcggccgccaaatccagcggccactgcttgccgatcgcctcgatggtcacgtcgcagaacacgccgccggtgagttcaccgacccggttgatgatgccgtagtgatcctccagcggaatggtctcggcggcgcccatgcgccgggcgaggtccaacgagaacggccggcgtgaaatggcgatgacacgcgcgcccgcatcggtcgccagtcgcgtcagacccgcgcccaggaaaccgatgccgacgatcgccaccgtctgtcccgccttgatctcggccctgcggaagatgttcatggcgcagcccagcggctcgccagggaacggcttgccggcgagtgctggcggcagtttcaccaccgccgcctcgtccgcgacgtcgtattcggcgaaactcttgtgcgacagggccgccacgcggtcgccaacggcgaccccggtcacgccttcgcccaaggcatcgacgacgccccagccctcgtggcccaggccgcctggctcggtcggaaacgtcatccactccggccccgcccatggcgtcaggttggaggcgcagacgccgcagccttccagacgcacccgaacctgcccggagcccggctgcggtcgagcgacctcgcgcacctccatctcgccaggccccgtcacgacggcggcgcgcatggtggcggtccgatcaagaacgtcggtcatagtctacgctttccagtctcttgaggacgacagtgccgcccttggtctttggctcaggcgccgaccgcttcgggcaagggatcgttgcgcagatgcccggcctcggcgtcgaaccagcgggcggtgcggcgcagcccctcctccagcggcgtggcggggcgccagtccagcacctcggccgccttgtcgatgtccggccggcggcggcgcggatcgtcgatgggcaggggccgacgaacgacctgagagcgcgagcccgtcagcgtcagcaccgtctccacaagttcattgacggtcagctcgaccggattgccgagattgatcggacccggctgcgcgccctcataggccatcagcgccatcaagccgccgaccatgtcgtcgacatagcagaaggagcgggtctggctgccgtcgccgaagacggtgatgtcgcgctcgctcagcgcctggctgaccacgttggacacgacccggccgtcggcggccgacaggcgcggaccataggtgttgaatatccggcagacccgcaccaccgccttgcccatgcggtcatagtcgaacgacagggtctcggcggcgcgcttgccctcgtcgtagcacgcgcgcggcccggtcggattgacgttgccgcggtaggtctcaggctgcggatgcacctcgggatcgccgtagatctcgctggtggaggtcagcaggaagcgcgcgttcgtccgctccgccagtcgcagcaggtgcagcgtgcccattacgctggtcagcatggtgtgctcgggatcggcctggtacagcggcggcgaagcggcgcaggccaggttgtagatctcgtcgaattcgcggctcgtcaggctggccggaagcggctcgacgatgtcgtgatgtacgaactcgaagttcggatgcttccgcgcctgctccagattggccatgtcgccggtcagcagattgtcgaggcagaccaccgtatggccctcatccagcaggcgatcgcacaggtgcgatcccaggaaccccgcgcccccggcgacgagaatggtcctggcggcttttgggacggcgaacggggtctgcatcgggtgttcctgacggatcatgtctttgcgtcgaacggcggcggccagttcgcgctccagggtctcggcccggtgaacgggcgtgtgggcctcaaggatgcggcgacgtgcggccgcacccatggcgcgggcctcctcatctgaggccaagagcgccgcctccacatcttcaaatgattgggccagcacgatctcttcgcccggcgtgaacagctgctccaggccgtcccatgcgtccgagatcacgggcgtcgcgcaggcggccgcctcgaataagcggatagacgggctgtgccccgcttcgatcatgtcggcgcgcgtgacgttcagggtgaagcggctggcgccataaaaggcggggtggtcggcgggcggcaggtgctcgatgcgttcgacattggccggccagtcgatgtccgaggggtacaaaggtcccgccacgacgaaccgcagatgcggcagacggcgggccggctcgatcagcaggcgctgcagcgtgggctggcgatcgtcgctgtaggtgccgagatatgacaggtcccagcgcttgggcgcatcgatcgggcggtagacctctgggtcggccgaacagaacagggccctcgcggcgggtgatccgaactcactctccagccgcttcagcgtcgggccgccggtgaaggagaagtagacgtcgtagtcggcgatctgttcagagccgagatattcccggtcgccttgcgccagccgcgccagcgtcacgggcgtgtcgatgtcgtagaaggccacaacaccccgcgccgtcgctttgacccagcgcccgacctccaccccgtccggcacgtaggagccgacgatcaccgcttccgcatggatcacctcgcccgcgaaccgcttcaggtcctcgagatcgtcatagaagcgcagggtgcagaaatccggctccggcagatcgcgatgatcgcccgcgtaccagggaacctcccgctccaggaacaggatgtcgtgcccgcgcgccgccatggccttcagcagggcgcgataggtcacggcatgcccattgccccaggacgaggccaggctgagccccaggacgacgatcctcatgccgccggtctctcgcgccgctcggccagaagcgtgcggaacagggcgtccgcctcttcggcgcgctgggcataggtgtggtcgcgcagcacgcgccggcgcgccgcctcgccgatggcgcgggcgcgctcgggcgtcagacgcttcagatgctcagccacctcagcgccgtcgcgggcgaccagcacctccacgtcgggctccaggaactgctcgatgccttcccaccagtcggtgatcaggcaagccccggcgcccgtcgcctcgaacacgcgggtagcgggcgaaaagcccacctcggccatgctgtcgcgcgccacgttcaacaccgccaacggcgagccgttgaacgcgttgtgatcgcccgtgccgacgtggccaagcgtgcgcacattgggcggcatcggcttgtcatgccagccattgcctcccagcaggaaggtgcgatccggcagcatggccgccggctcaagaaagaagcgctcgatccgcgcctcgcggtccggcagacggttcgccagcagggccagatcgacggagaagcgctcgttccgctcgacaggatggtgggtggaaggatcaagcgcattgtagatcggccggcacgcgcgggctcccatggccagatacgcctcgatcaccggaggcccgccgccataggtcagcacctggtcgacgcgtggcagcggcctcttcagcgcgtgctccggcgcggcgcgcatctccgccagcgtcgccggcgcgtccacgtcccagaagatcgtcagagcatcgggccgcgcgtggtcgaacacccccagcagctcgtcatcgaacacgccgacgcccgaggccttgacgaccacgtcggcttcggacgcgcgccgcatcacctcgcggcaggcctccaacgtattctcccacaccaccacctccgcccactccggcggatcgatgtcgcggtgctgctgccggtcaaaggcgtccggttcgaagaacacgacctcccaaccgcgcttggccagttcgcccagcatgccgcgatagtaggtggccgctccgttccagtaggcgctgagcaggcttgagccgtaaaaggcgatcttcatcaggcggtccccagcgctggccgcgccggagcgacgacgccgttcagccgatcgtagacggccagcagttcatcaacccggtgcgcacaggtgtggcgatcgcggatggtcgccaaccccttcgccgtcagcgcctcacgcagatctgggtcgttcttcaggtcggtcagcgcctgcgtcatcgcctcgccagagcgcaccatcaggaagtcctcgcccaccgtgaacagccgctcgctgtcgctccagggcgcgctgaccagcggaatgccgcaggccagcgcctcgaacacacggatggttgggatgccgggcaactgctcgacatagaagcggcgcggcacatgcaccgtcgccaggtggcgggcgaaggcggccggcgccgccgcattggccatccagccgtggtagcgcacgccgtagcgttcaagcgtcgccagcgcgtcggcgggatagcgaacgccgtggatgtccaggccgagccccgcatcctgagccggcttgaacagataggtctccagctcgcgcgtacgctcgccgtcgccccagttgccgatccagatcagcccttcgcgcggaccttcctcggccggcggatggaacaggcggacatccgccgcctcgtgccagacgaagacgcggccgtcccagccccagcggcgatagacctccgccagcgtttccccgaaggccagcacgccgtcgtagccggacagatcgaaggccttgatgccttccggctcgctgaccgcacggtggtgggtgtcgtggaacaacagggtgaagcgtccgccctgcgctctcgcctcgccgacggccgccaccaaggctgggtcgttccactcgtgcaccagcaccagatcggccctgtcgagcgcccggtccaggttggccggcgggtcgaacctttcgctcgtcagctcagaataggcggcgcggtaaggctcaagcccttgctcgccatggtcgcgcaccaggttctcgcggctccaggcgtcgcgaggctcccacacagcaacctcgtgcccgcgagcgatcaggtcgcgcaggacgccccgaaggaaatgcgcattgccgtggttccagcaggactccagcgagtgggtgaaatagaccaccttcatgccgcgacctccctcaccgggacgcgcgccgccatggcctcggcatagacggccagcgtacccgcggccgacgcttcaagcgagtacagacgggcgcgcgccttcgccttccggctgaggcgggatcgttcggccgggtccgacgccaccccatccagcacccgggccgcctcgtcttcgtcatgcggtgacacgaacaccgccgcgccgtcccacagctcgcggaacgtggggatgtccgacaggaccagggcgcatccggcctgcgccgcctccagcacgcccagcccgaacggctcgtacagcgccaggggggcgaacaccgccgctcggttcaggcggtcggcgacgccggccgcatccagatgaccgaggctgtcgatgttggacaaggcgatcgtctcgccgtgagggccggcgcccgcgcccgccgccgccacgggcgtacgcatttgcccggccgcgcggtcgagcaccgccacgttcttgcccgcgtcccagagccggccggacgtcagaacgcccgatcgtcgttcgaccgtcagatcacgcgcagagcgacggccgttgagaacggtcttcggctcgagcccatagcagagggcggtcgcatcccggaagctgcggctgggcgcgatcagggcgtcacaggcctgatatccgcgcgagagcaattcggcgcgccaccggaagtcggacggcatgtcgccgcccctgaccgcgctccaccaggtggcggggcacgaagggcacgagccgaccacggggacgccgaagtccgcgtcggcggccagcgacggcgcgtgcagatgcacgacgtccacgcccgcctcttcagcgaaacgggcgatcgcctggccggaacgcaggatctcggcctcgcccacgccccaccagtcgagcgggaaacccgtctggatcatggtaaggccgatctggctgacttcggcgcgttgggccggccccggctcgggcccgatgacggccaacgtcgtgcgaacgccatgctccgccagcccccgtgcaagatcgagagagtatgtccacactccgccgaccgcgtcggtggtcagcagaacgctgccgggcggacgcctcatgccgccgccgtctgctgcgaggggaacgagcgttccgcccgcagccaacccgccagttcggccaccccgtcacgccaggcgacgggcgcgttcaagcccagcgtctcgcgcgcggccgaggcgtccgccacgaagtagcgctgatcgcctgcacgccagtcctcgtacgcgacggggatttcccgcccgatcagaccctccatgtggctcagcaactggcgcagcgacaccgcgttggtcggcccgccgcccaggttgaaggcgcgtccgctgacctgctcgatccgttcccaggccgagacataggcctgaacggcgtccgcgacatgcatgatgtcacgcacctgccgcccgtcaccgtagagggtgatcgtctgatcctcgagcgcgcggatcaggaagtgagcgacccagccctgatcctccgtgcccatctgacgaggtccatagatgcagctcatgcgaagcacgcaggccggcacgtcgaaggagcgggcgtagtccagcacatactgatcggccgcccccttggagcagccatagggcgtgtggaagtccagcggccgcgcttcgtctacgccgcgctcgcggaatgtcggatccacaggcgtccaggccccgttgctgagctcgagcgcgatgtcggccaggtcgccgtacaccttattggtgctggcgtagatcaccggaaccccgcgaccgcgcgcggcctccagcaggttcaacgtgccccgaagattgatctcgaagtcctcgcgcggatcaaccaggctggtggtcaccgccacctgggcggccaggtggaagacgacgtccgcctcggccacagcgcgagcggcctcggcctcgtcgcggatgtcggcgtgcagatgccgcacccgatccccatgccgcgacagcaaccagttcagattccgttcgacgcccggccgcgccagggtgtccatcacggtgacccggcagccgtcgctcgccacccggtcggcgaggttcgagccgatgaagccggccccgccggtgatcagtacgcgccccccacgagccatcaggcgaccagtcccctcgcttccagctcgcgccgcgcctcttccaccttgtcctgcgattcctggcgagccacccactccgccaactcctcaagccccgcggagaaatcctgcgtggcttcgtagccgagcagatcacgcgccttggacagatccgggatgttgtggcggatgtcgcccgccctcgccttctgcgtgatcagaggctggatgtccgaacggcccatggattcagcctgaagcctggcgacatcctcgaccgtgcggtcgacgcccgaaccgatgttgaacacctcgccgtcggcttccggcttgtccatcgccagcagaaaggccttggacacgtccgacacgtgcacgaagtcgcggcgctgctgcccgtcctcgaacaccatcggctgctgcccgtgcgagatacgcgaggcgaagatcgccagcacgccggtgtagggattcgaaagcgcctggcccggcccatagatgttccacaaacgcaaggcgcagctttccatgccgtactgcgccgtcagcgtcagggtcaggcgctcctgcacgtacttgttgatcgcatagacgctcttcagcgccggctgcttggtctccggcgtgatcacggggatcagcgggcgcccctgagcgtctttgggatcccaggtgccgtcggcgttgcgggggccgcgcaccacatcctgcatcagttcgccgtcctgcgtctcatacaggccctcgccgtagatgctcatcgaggaggcgaccacgacccgcttcaccggattgtcgatcagctgctggaacagcaccgccgtgccgtaatcgttgaccgaggtgtagcggtcgatctggtacatgctctgaccgacgccgacctcggccgccaggtgcagcaccttgtcgacgcccttgagcgactggcgcaccttgtcctcgtcgcggatgtcgccgacgatcagctccacttccggatcaagatcgtccgggcgtccgctgccggagtgaacctgctcgataaggctgtcgagggcgcgcaccttgtggccctgctccagcatggcccgggcgacatgccggccgacgaaccccgcgccgccggtgatgagaactgtgtccgccaatgggacctccgcagttagaaccgtcgccgccagccgccccgcaggccctcagccttgcgcacgccccgaaaatctggtgacttcaccctcttaacggcacagcttcatcttagttccagaagaagatgaagctgttggcctagacgcgatcagcgtaacgcatcgtttgtatgcggatcgatggaaccaatctggccagcatctacttacctcgtcaagctgcgccgtgagccttgagccgtgcggtcgcatgaagggggcgtgatgagcagaaacaaggtgcgcgtaggcgtggtcggcgtgggcaactgcgcctcgtcgctcgtgcaggggatcagccactattcggcggcgaccagcaacgaaccgccgcccggcctgatgcacgtcgagctcggcggctaccatgtcggcgatctggagatcgcatcggccttcgacattcatgccggcaaggtcggccgcgacgtgtcggaggccatcttcgccgagccgaacaacaccatccgcttcgccaagcccgacggcgcgggcgtccgcgtctcgcgtggtcccacgctggacggtgtcggcctctacatggccggcgacatccctgagtctgacgaagcgcctgtcgacgtggccgaggtgctgcgcgaaagccgcacggacgttctcgtctcgtacctccccgtcggttcgcagcaggcgacggaatactacgccgaacaggcgctcaaggccggctgcgcctatgtgaactgcattcccgtcttcatcgcctcggacaaggactgggcgcgacggttcgaagagcgcggcctgccgatcgtcggcgacgacatcaagagccaggtcggcgccaccatcgtccaccgtgtgctcgccaacctgatgcgcgagcgcggcgtgcgcctggaccgcacctaccagctgaacttcggcggcaacgccgacttcaagaacatgctggaacgcgagcgcctgcactcaaagaagatatccaagacccaggcggtgaccagccagttggacttccccctgcccgcggacgacgttcacgtcgggcccagcgaccatgtgccgtggctgaccgaccgcaagtgggcccacatccgactggaaggcaccaccttcggcgacgtgccgctgaacatcgagctgaagctggaggtctgggacagtcccaacagcgccggcgtggtcatagacgcgatccgctgcgccaagctggcgatggaccgcaaggtctcgggcccgctgatcggtccttccgcctggttcatgaagtcgccgcctgagcaattcaccgatgaggaggcgcggctgcgcaccgagcgcttcatcgaaggcggcgatgcgccgcgtccgccccgcctggtctcgtgacgacgatctatctcgtgcggcacggcgttcacgatcaactgggcggccgattgtcgggtcgcacgcccggcgtgctgatgggccaggcgggcctggcgcaggccgaggccgccgccgagcgcctgtcgggccgcaatgtggagacggtctacaccagccccatggaacgcacccgccagaccgcagagccgatcgcccgggcctgcgccgcgccgctggtcgaggaaccggccctgaacgagatcgacttcggcgactggaacggcgccgctttcgccgacctggatcggcagccggagtggcggcgttggaacacggaccgcgatcacgcccgcgccccctccggcgagacgatgctgaaggtgcagcttcgcctttcgcgctggcttgaagacgtgacgcaaggcggcgcggaggcgatcgtggcggtcagccatgctgacgtgatcaagagcgtcgtggccttgaccctggggctgtccatgcgcgcgcacgatcggttcgaggtgtctcccggttcgatcacgacgctgaccgccgacgcctggggcttgcgtctgcatgcaatcaacgaggcgccttgatgaagctgacgaccgaagacatccgcgcgcgggtcgaggccctatcgccctggttccatgacatggatctgaatggcgtgcgcaccgcgccggaccacttcctgcccggctatccggccagcaagttccgacgtttcgcccacgccctgcccgccgacatgacgggcaagagcgtgctggatatcggctgcaacgccggcttctactcgctggagatgaagcggcgcggcgccgatcgcgtcctgggcgtcgacttcgacgaccgctacctggatcaggcgcggctggccgccgaggtcgagggcgccgacatcgaattccgcaagctgtcggtctacgacctcgcagcgctcggggaacgcttcgatctggtgatcttcatgggggtgctttatcacctccgtcacccgcttttggcgctcgacttgatttatgagcatgtggcggacgatctgttgctgtttcagtcgatgcagcgaggttcaaaggccgactttccggttcgcgccgactacgacttcaatgagacgcagcatttcgacgagcctggctaccccaagatgcacttcatcgagcaccagtacgctcacgactggaccaactggtgggcgccgaatacggcgtgcagcgtggccatgctgagaagttcagggttcgaaatcctcgaccaccccgagagcgaggtgtttctctgccgccgcgcgacgcggccgaccgaagccggggccgtctatcccgcgcagggcgccctgaccaagactggagacctcgccggatgatcgaagccgtcaagatctggaacgagccgaacaacaagtcgcactgggacccgaacctcgatcccgaatgggacctgttcgccaacatgacctgcctggccggtcaggcgatccgggaggccaatcccgacgtcacgcgcgtgctgggcggcatgtctccgatcgatccgggctttatccgccggctcgaggcgcgcggcgtgatggaggcggtggacgtcgtcgccgtgcacggctttccgctggactggaacctgtggtccatcgacgaatggccggccaaggtcggcgagatccaggccgtgaccgacaagcccgtgtgggtcaccgaggtcggcgtctccgccttcggctcggaagaggtgcaggcctggggcgtcaagaagaccgccgacctgctgatcggccgggccccgcgcatcttctggtacagcctctacgacctgccccaggcgtgggaggccacgacgcgacacaaggaggccgagggctcctcctattaccggcacttccacatggggctgctacgcgaggacggctcacccaaggccgcgctggaggcctatcggccctacgccgccgacatgggactgtgccaatggttccactaccatgatcaccgcctggacgaggccgtacggatcatgcgcgacttgggcgtccgtcacgtccgcaccggcatctcatgggccgacagcttccgcgaaggcgctctggaatggttcgaccgccagatggaagccttggcgccgttcgacacgacggtcaccttctgcttcacgcccgagcatcgcggtgtcgagccccaccacaccagccctccgcaggtcgcggaggagtacgcccagttctgcgccgacatggtcagccgctatgcgccacgtcgcgccgccccgaccctgccggtcgaagtctcggaggaagccgcatgaagatcgggatcatcggaacgggctatgtcggcctggtcaccggcgcctgcctggcggaggtcggccatgaggtggtctgcatcgaccgggacgccggcaagatcgccctgctggagaacggcggctgccccatctacgagccaggtctgccagaactgatcgcccgcaaccgcaccgccggccgcctgaccttctccacccgcatcactgacggcgtgcgcggtgtcgaggccgtgttcatcgccgtcggcacgcctccgggcgccaacggcgacgcggatttgcgcttcgttcatgcggtcgccgaggagatcgccgaccatctgagcggcttcaccgtcgtggtgaccaagtccaccgttcccgtcggcaccggcgaccaggtggagggcctgatccggcgccgtcgcacggccgcggatttcgccgtggtgtccaatccggagttcctgcgcgaaggctgcgcgatcggcgacttcctgaagccggatcgcatcgtcgtcggcgccgacgagccccgcgcccgcgaggtgatggaggccgtctatcaaccgctgacccgccagggcgcgccgctgctgctgaccgagcgccgcacgtccgagttgatcaaatacgcctccaacgccttcctggcggtcaagatcagctacatcaatgagatggccgacctgtgcgaggaagtgggcgccgacgcgctcaaggtcgcggagggcatgggtctggacccccgcatcggcggacgtttcctgcagcccggccccggctatggcgggtcgtgcttccccaaggacacaaaggcgctgctcagcaccggtgctcagtccggcgtgcgcctgcgcgtggtgcaggcggcggaagaggccaacgcggaccgcaagcgctgcctggccgcgcgcgtgaccgccgtcgccggcgaccttcagggcaagacggtcgcggtcctgggcctggccttcaaggcgggaaccgacgacatgcgcgaggccgcgtcgctggagctgatccctgagctgcaggcgcgcggcgcgaccgtgcgcgccttcgatccggaagcgatggaagcggccgctcccatgctgccgggggcgatcttttgccgcgacgcctatcatgcgctggacggcgccgacgtcgcgatcgtgctgacggagtgggacgacttcgcggacctggatctcggccgtgcggccgaacgtatgcgcaggcgcctgatggtggacttccgcaacctctatcggcccggcgacgttaccgccgccggcatcgactatgtgtccctgggacgtccggccgcgtccgccgaacgacatcggagagccgtctcatccgtcgatgcggacgaggcgcagcctctgcaaagggctgtggccgagtaaaacgattgaagggcggagcctgcggctccgcccttcttcgttcagcccgccagtcgccacccgacagcgcgccccccggtgatctccgcgaccgatcgtccggccacgcgggtgtcgccccaccaggcggcgcccggcgcggcatcagccgcctcaacgcaagcctgggacgccctggtggcgcagaccaccagcagttgcgcgccgtcgtgctcccgagcaaaggccagggcctcgcccgcgcgcgccccttccagttcgagcggctggtagtctcccgaggcgaacagatcaggccgacgctttcgttcgtccagcagccgtgagatcagcgacaccttggcggcgccttggcgccagtcctcgacgtcgcccgcttgctctagccaggcctgtcgaaccgcataatccacaggtcggcgattgtccgggtcgaccaggctgaagtcccagccttcggtcccctggtagatatccggcacgccgggcgtggtgagcttcagcagcgtctgcgccaggctcttggccacgccggcgggagcgatgcgctcgatgaacggcacggccgcggtcaggaagtcgctgttcggcgccaggatccgctccagataggtgcggcacgcctcttcataggcctcgttcggcatggcccaggatgaacgcagcttggcttcccgcaacgccttccgccaccatcccaccagccgctcgcgcagctccgccagtccgtctcggtaggacgccgacagatcaagcggccatgcgccgacgatggcctgatgtagctgataggcgtcggcgggcgccacgccttccagaggaacaatgtccagccagcgccgcgcggcctccacccacagctccggaagttcgctcaggaccgccagacgcgcccgcgaatcctcgccccgcttgtgatcgtgcgtcgccgtggccagcatggcgtgcgaatgatcggcggttcgcgcctgcacagcggcatggaagtcgccagccgaggcgcccagcctcgccgggtcgaaccccacatcggtccgcgagagcagccggccgtatcgatagaaggcggtgtcctcgaccgacttggccgagaccggcgcgctcagctgttgaaagcgccggaaggcgtccgccttgaggtccaggtcgccgccgccctcgccggccagccacctggcgacctgccggatcatctcggcgtcggaaggcgcgacaagcttgacggcggcctcgacgacgcggtcgcggacggccgcgtcggacgccggcgccgcgtcgcccacgccgtaggtgcgatagaccgggaacaccgtcatcatggcgcgcaaggctcgccggaagccggcgagggtcaggtcgcgcgtcgccagatcgcttcgggccagccgttcgaacgcggcggcgcaggcgtccagctgaccggcgaagctccggtccagcgtctcggcgcgggccagccgttcctcggtatggaagtccgccgtgcgtgcgctgatgtccgtccagagggcatcaaggccggacgcgccggctggatcgtgcagcacggccgagacgtcgttcatgaagtcatagccggtcgtgccgtccgtcaaccagtcggcggccagcggctcgcccgccgccaggatcttctcgatcaccagataggcgggcccctcggacgcggcctgcgggcgccgaggctccagctcggtcaggcacccccgcagctgtcgacagtagccggcgggatcggccaagccgtcgacgtggtcgatgcgcaggccgtcgatcagcccctcggcatagaggcgcagcggcatcgcgtgcaccgcatcgaacaccgtctggtcctcgatccgcagcccggccagttcggagatgtcgaagaaccggcgccagttgatctggtcgcccgcggtgcgccaatgagcgagccgatagtgctgccgctcaagcagatcatgcagggccgccctgcccgccttggtccggccatcgaatgcccgcgccagcgcttccggcgtcgcgtttgcaaggctgtccgcgcccgccgcgtgcagcacggcggcgtggtcctcgcgccggatcggaaaacggtgggcgccgtaggccacgaccgaaatgcggtctcgttcgggctccgcctccacgacgagatcgcctgactccagcacctcggcgtaggggccgcccaggaaaggcgccagcagcttgcctgtcagcgccggatcgtcgctgttccagtcgatgtcgaagaagcgggcatgggcgctggcccgccccttctccagcacgtccagccaccaggcgttgtcgtcgccgcccacggccacgtggttcggcacgatgtcgaggatgacgccgagatcgtggcgccgcagcgtctcgaccagcgtgcgaaagccctcttcgccgcccagcgccggattgatcgtcgtcggatcgaccacgtcatagccgtggatcgaccccttgcgcgcggtggcgatcggcgaggcgtagacgtggctgacgccaagcttggcccagtagggcgccaggcgttgggcgtcggcgaaggtgaaatcggcgtggaactggacgcggtaggtggcgcgtggcgtcatcgaggtctttcagcgttcaggcgttcgacccgcgcggcgacgcgcggttcttcgagcaggttctcggtcgcggccggcaggcggcggcgccagttgggatgcacctcgacgacgccaggcaggttcggctgctcatccagaccgagcagatcctcgaccgggatcagcgccagttcgcaggcgctggtcgccgcataggcgaccgatgcgtcgacggcggcgtccggcgcgtcggcgggcggcggatcgcccgaggcgaccccggcctcgaccgccgcgctccagaaggcctcgcgatagtcggcccgctcctggcgctccgcctcgcggtcgccgtcggcgcccagccgcccccgccactcgatgtcgcggcccttccaccatccggcgacgggcgccaggtcgtgggtcgaggtcatggcggcggccagagggtcccagctgtcgggggacctgagcgcgccgtccttttcgcgttcgaacggcagaacgcgcatgccgagcaggccgtgcgtctccagagtgtcgcgcagaccgtccggcaccacgcccaggtcctcgccgatgatgatggcgcgggcgcgatggctttcgagcgcacacaggcgcagcagatccttcagcgggttgaccagataggcgccctcgagcggcgaggcgccgtccggcaggacccacaggcggttcaatcccagcgcatggtcgatccgcaatccgcccgcgtgccgcagcgccgcccgcaccgtgcggatgaacggcgcatagcccttgcgtttcagcgccgtgggcgaaaagctggtgatcccccactcctgccccgccgcctgaaaggcgtctggcggcgcgcccagcgtcaggccgtccagcagttcgtcgcgccgcgcccaggcgtggctcccgccgggatcgagcccgaccgccaagtccgcgaccagccccacgcccatgccggcggccttcgcctgcgcctgcgccgtctcgagccccaggtcggccagccattggcagaacagctgaaagcgcacatcctcggcatgctcgcgggcgaaagcctgcacggccgcgctgtcggggttctgatactcggccggccagccccgccatccgcccgcgccgttcagcgcgaagaaatgaccgtgcagcacctcgaacagggcgtgctggcgcagcggctcgccgccgtcccgaacaaaggcgtcgaaccgcgcatcgcctttgaaaccggtgaaaacctcgcgcagcgcggtgacgcggctgtcgctggtcgcgggccaatcgatcaggtcgccgccggctccgctcgcgccccgtccgccgatcaccgccgaatcggcgaacagggggttcagccagtcgcggctggacggcgaataggggctgtaacgctgcgggtcggccagaaacagggcgtgcaccggactgatggccacggcgtccgcgcccgcccggcccagccgcgcggcgaaatccgcgagcgcgccgaagtcgcccgagggcgtctctcgaccatcgcgcaggctgtagagctgcaccgtcgcaccccacgccttgcgaccgagaacgtcgcgggcggtcaggcatcgcggcgggcagaccgccagggtcacctcccgcccgccaagctccagccggtgatagccgatggcgtccggcgccgtgaaccggccggtcacgtccagagcctttccgtcttcaaggatcagccgcccggaggaggcgccccccggcagctccagcgcctgccccgccacggcggtgatcagggccggctcggccttttcggccaacatcgccaggctgtcgcggcggtcggcggcgctgtcgcaggcgaggcccatgctggtcagaatggcgcttagcgaggcgtcggacacgcgctggtctcggccctgcgcatcctcccagtcgatcaccaacccggcggcgctcgccagcgcatgcaggtccgcctggctcacgccaccggctccagccacgccagcaggcaggcgggggcgatccggccgtccgtggccgtgtctccgacggcgaacaccggctccgccgccggggcatcggcgtaggcgacggcctccgaacccaggttcaaggcgaggctcagcctgaagccgtgccccagcgtccacgcggccgcgaccgccttgtcgcccagcacctgcgagccggccgacttcgcctccgccaggcccggcgtgatcatctcgcgacgcaagcgcagcaggcggcgatagaggtcgcgccattcgtcggcgtcctcacccggccggaccctggacatctcgaatgtcgagggcgcgttcggatcgggaatgcgctcgcgcgcctccggatcggcgaaggcctcgaacttggcgaactccctgcgccgtccctcgcgcaccgcatcggccagttcgtcgtggaagtcggtgaagaacagaaaggggctggtcgagcccgtctcctcgcccatgaagatcagcgggatctgcgggcacagcagctgcatcgccacggccgccttcagccggtcgtgatccaccaggctggtcagccgctcgcccatggcgcgattgccgacctggtcgtggttctgcaggaacgacacaaaggcggccggccgcagttgggcgctgggcttgccgcgcggcgccccttcgtggttcggcgagccctcgccctgatagatgaagccctcggccagacagcgggccagccgctcctccgggtcgtcggcgaagtcttgatagtaggcgctggtctcgccggtcagcagcacatgcatgacgttgtggaagtcgtcgttccactgagcgtcataggcctgctccagtcgctcagcgtcgttggcctcgttctccaggatcaggtgcacttggcgggggccggctgcgtcccgcacctcgcgcgccatgcgatccaggaaagcctcgtcgccgatggcgtggaccgcgtcaaaccgcagcccgtcgaaacggaactcctcgacccagtagcgggcgttgtcgataaagaagcgcgccaccggctcgcgatcaaaggcgatggcggcgccccacggagtctgcttttccgggtggaagaagcggctcgcataggcgttcagatagttcccgtccggcccaaagtggttgtagaccacgtccaggaagatcatcatcccgagctcgtgagcccggtctacgagcgccttcaactcgtccggcgtcccgtaggccgcatccggcgcatacggcagcacgccgtcgtagccccagttcctctggcccgagaagtcgttgaccggcatcagctgcacagccgtgacaccgaggtcggccagctgcggcaggtagtcggccacccctgcaaaaccgcccaagacgccgcagtgtacttcacagatgacggcctcttcccaaggcctgcccgaccaatcgatccgccagcgatagctctcgggatcgaccaccaggctggcgtcgttcacgtcgccgtcctgcgcccgagacgccgggtccggcacgacgaggtccggacccacgcggtagcgataggccgcgcccacgcccacgtcagattcgacctcgaaccagccgtcgtcgcagggattcatcggcagcgatggacggccctccacctccagcgccgcctcggataggtccggcgcccagagccgaaaacgggtgcggccgggtgcgatcaggcatgctcccgcgcggtcggccgcctcggtcacgcttggcgctccagcgaggtgatgatcacggccgcgccgctcatcacgcgatagacgtcgggctcaagatcgaggtcgcgcacatcggcgtctgcgctgtcgatccgcaccacatgcgcgaggttctgctccggaagccggaagtcgagatcttcatgcgaactgttcagcagcaggctgacgctgcggagccggccgtcctcgtcgatctgcgatcgccgcatgaccagggcgcgcccctcggcgttgcgccagtcgtcctcggacaactgcatcccgcgctcgtcccaccactcgatgtccagcaccccctcccgaaccggctcgccgtacaggaagcgcccagaccggatcggcgggatgtcacgacggatctcggccagacggccaacaaaggccgtcagcgcctgtccgtcctccgagtcggcctggttccagtcaaaccagctcagctcgtcgtcatggcaataggcgttgttgttgccaccctggctgcggccgaactcgtcgcctcccagcagcatcggcgtgcccatggatccgaacagcgtcgccagcatcgatcgctgcagtcgctggcgataggcgttgatgtccggattgtccgtcgggccctcgacgccccagttatgcgacaggttctcgctgtggccgtcgcgattgtcttccttgttggcctcgttgtgcttctcgtcatagctgacgacgtcggccagggtcatgccgtcgtgggccgacaggaagttgacgctggcccaagggcggcgcgcacggcggtcgaacaggtcgcccgagccggacaagcgcgcggcaaggtccggtcgctggctggagtcccgcttccagtatttacgggtggtgtcgcgatacttgtcgttccattcggcgaaggacggcgggtggttgcccaactgatatccgcccggcccgatgtcccacggctcggagatcagcttcagcttctgcaggacgggatcctggcgcagcacgtcgaagaaggcggcgcccggatcaaagcccttgttgccgtcccgccccagggtcacgcccagatcgaagcggaagccgtcgacgcggaagctctcggcccaatagcgcaggctgtcggacaccatctgcaccacacgcgccttggacatgttcaggctgttgcccgtgcccgtgtcgttgacgcagtagcgcggattgtcgtcgtgcagcctgtagtaggtggcgttgtccagtccgcgcagcgacagggtctggcccatctcgctgccctcggcggtgtggttgtagaccacgtccaggatgacctcgatgcccgcggcgtgcagccggcggaccgcgagccggaactcgtcggcgctgcccgtcgccatgtagcgggcctcgggcgcgaaaaaggccagggtgttgtagccccagtagttggccagtcccctttcctgcaggaatcggtcctgaacaaaggcgtggatgggcagcagctcaagcgccgtcacgcccagcttttgcagatgatcaatgacgcgcgggtgcgaaagcgccgcaaaggtgccgcgctcgggcgggctgacgtcctccagcagcttggtcagcccctttacatgggcctcgtagatgacggtcttgtcccagggcgtgttcggcctctggtcgcccgtccagtcaaaggcgtcgatcttgaccaccgacttggggaccgccggcgcgctgtcgcgcttgtcgaagctgagatcgcccttctgcgagccgacgcggtagccgtgcagggcgtcggtccagcgcaccgcgccgtgcagcttcttggcgtaggggtcgatcagcagcttgttcggattgaaccggtgtccattctccggctcgtatcgcccgtgcgcgcgaaagccgtacagcagccccggcttcacctccggcagatagccgtgccacacctcgtccgtgcattccggcagcacatagcgcgcgatctcgcgcttgcccgacgggtcaaagatgcacaggtcgatctggtcggcgttggcggagaaaacggcgaagttgacgcccaggccgtcaaaggttgcgccgagcggaaaggcggagcccggcagaagccggtcaggcagcaggttcaagcggcggtccttcgtacttaaggaagaccccggccagtggcggcagcgtcaattcgagcgactgcgcgcggccgtgacagggatgaggcgccgtccgaacggctccagcgttgccgatgttcccgccgccgtagatttccgcatcggtgttcaaaatctcgcgccattcgccggcctccggcgcaccgatgcgatagccgcgtcgaacctcgggcgtcatgttcagggccacgatgaccggcgctccgccgtggaaggatcgacgcaggaacacgaacacgctgctcgccggatcatgctccacgatccattcgaagccgcgtggatcggcgtcggtgtggtgcagagcgccttcgcgggcgtagagtcggttcaggtctcccaccagccgctggactccggcgtgctcggcctgctgcaacaggccccagtccagttcccgatcgtggttccactcgcgcggctgcgccagctcaccgcccatgaacaacagcttcttgcccggatgcccccacatgaaggcgaaataggcgcgcaggttgccaagcttttgccagcggtcgcccggcatcttctcgatcagcgcgcccttgccgtgcaccacctcgtcgtggctcagcggcaggacgaacttctcgctgaaggcgtagaccaggccgaagccgatgtccccgccgtgccagcgccggtacagcggatcgcgctccatgtagcgcagggtgtcgttcatccaccccatgttccacttgtaggaaaagcccagcccgccattttcgaccggcgcggtgactcccggccaggcggtggactcctcggcgacggtcatggcgccggggcatcgctccgccacgatggtgttcaggcgctgaaggaaggccacggactccaggttctcgcgcccgccgtagacgttgggcgtccactggccttccttgcggctgtagtcgcggtacagcatcgacgcgaccgcatcgacccgcagcgcatcgacgtgaaaggtctccagccaatatagggctgaggagatcagatagccctgaacctcgctgcgccccaggttgaagatcagggtgttccagtcggggtgatagccttccttggggtcggcatgctcgtacagcgccgtgccgtcgaagaaggccaggccgtgcgcgtcgctggggaagtgcgccggcacccagtccagaatgaccccgatccccgcctggtggcagcggtccacgaagcgggcgaagccctccaccggtccgaaccgggccgagggcgcgaattgcgacagcggttggtagccccacgatccgccgaacggatgctcggcgatcggcatcagctcgacatgggtgaagcccaagtccttcacgtaggggatcagctgttcggaaagctcgtcccagctgtgcgcctcgggaaagtcccgccacggcttgcgccaggaggcggcgtgcacctcgtagatcgagatgggcgcgcccgggtggtggcgctcggcccggctcttcatccatcccttgtcgccccagcgatgcgctgggggcgcggccaccaccgaggcggtagccggcggagtctcggtggcgcgggccaacgggtcggccttctcgcgcaccacgccgtccgcgccggtgatcgcgaacttgtatcgctcaccgggctgcagccggggcacgaacagctcccacacgccggaagctccgcgcgagcgcatgggatgccttcggcggtcccaggcgttgaactcaccgatcaccgacacctgccgcgcattgggcgcccacaccgaaaaggccacgcccttgcagccctcatgcgtcatcggcgccgcgcccatgcggcgggccaactcgaaatgcgagccttcgccgaacaggtgcaggtccagctcgcccaggacgggaccgaaggcgtatgcgtcttcggtatcctgcacgccgcccggccagatcacccgcaggcgataggcgatcggcttcttcatccgaccgacgaacaggccaggcgacacctcttcaagccggctgacgacgcggccgttagcgcgggcgatgacctccaccgccgccgcgcccggctggtaggttcgaaccgatccgtcatgaaggccgagaaacgcaaaggggtcggagagccagtcctccacggctgatcgctgcaacttgaccccttccccgaaatcccgcgcgaaaacaggaaagccgcgcgacgcctagggaaccttagccgctggcatcggttccgtcccgcacagggagaaacaacagaatgccacccagtgcgaccctccggggcctgatcagccgtcaggccatggcctttgttctggccggaggtagaggcagccgattgctcgagctgacggaccgccgcgccaagccggccgtcttcttcggcggcaaaacccggatcatcgacttcgccctgtccaacgccctgaactcgggcgtgcgccgcatctgcgtggcgacccagtacaaggcgcacagcctgatcaagcacctgcagtacggctggaccttcttccgccccgagcggaacgaaagcttcgatatcctgccggccagccagcgggtgtccgaggccaactggtacctcggcacggccgacgccgtgtaccagaacatcgacatcatccgcagctatgcgcccaagtacatcatcgtcttggccggcgaccacatctacaagcaggactacggcgtgatgctcgaggagcattgcaacaacaacgccgaggtcacggtcggctgcgtcgaggcccctcgctccgaagcgtccgccttcggcgtgatgcacatcgacgagaacgaccgcatcatcgacttcctggaaaagcccaaggatccgccatcgatgcccggcaagccggacacggctctggtcagcatgggcatctacatcttcgacaccgagttcctgttccagcgtctgatcgaggatgcggcggaccccacgtccgagcacgacttcggcaagaacatcatccccgacctggtcaagaacggccgcgccttcgcccatcagctgggccgctcggccatccgctcgggtccgcgcgccgaggcctattggcgcgacgtgggtacgctggacgcctatttcgacgccaatctcgacctgaccaacaccacgccggacctcgatctctacgaccgcgagtggccgatctggacctacagcgagatgacggcgccggcgaagttcgtgcacaacgacgagggccgacgcggcatggcggtgtcctccgtggtgtccggcgactgcatcgtctcgggggcctcgctggagcgctccctgctgttcaccggggtgcgcgtgaacagctactcccatgtcgagaacgccgtgatcatgcctcgggtcgagatcggtcggtcgtgccgcctgaccaatgtcatcatcgacaaggaagtggtcattcccgaaggcctggtggtcggcgaggacccgatcatggacgctcagcgattccgacgcaccgacaagggcgtgtgcctgatcacccagccgatgatcgacgcccttgccggctgaggcctccgttcgcgccgccgaagcgacgcgcccgctgcacgtcctgtcggtcacgtccgagatcttcccgttgatcaagaccgggggtctggccgacgtggccggcgcgctacccgcggccctgcgtccgcatggcgtcgagatgcggacgctgattcccggttacccggcggtgctggaccgacttggggaggcggaggtggtgaccaccttcgacgacctgatgggcgatcgcgcgcgggtgctgcaggggtcggccgcagggctggacctctttgtattggacgcccctcacctgttcgcacgaacgggcaatccatatctgacgccggacggcgaagactggcccgacaacgggctgcgcttcggagccctggccagggtcgccgccgagatcgcgcgcgggcgcataggcggttatcgcccggacgtcgtgcacggtcacgattggcaggcctccatggttcccgcctatctgcggtatggctcggagggtgcgccgccgttcgtgctgacgatccacaacctcgcattccagggccgcttcccacgcgcgctgctgccggcgttgggcctgccagacaaggcgttcgcgctggacggcgtcgaatactacggcgacatagggttcctgaaggccggtgtcctgatggccgaccgcgtgaccaccgtgtcgccgacctacaccgccgaaatcgccagcgagggcggcggcatgggcctgggcgggctgcttcaagggcgtggcgaggacctgatcggcattctgaacgggctggacgtcgaggtctggaacccggccaaggacgccctgatcgcccggacctacgacgcccccgaccctgcgccccgcgccgcgaacaaggcggccttgcaggcccgcttcggccttgatcctcgtgcggacgcgccgcttttcggcgtagtcagccgcctgaccagccaaaagggtctcgacctgctgctgactgctctgcctaccgtgctggagatgggggcccagctcgccctgctcggcgcgggcgagccggggctcgaggccggctttcgcgccgcggccgaggtggcgcccggccgcatcgggtgcgtcatcggctatgacgaggcgctggcgcaccagatccaagccgggtgcgacgtgctgctggtcccgtcacgcttcgagccctgcggcctgacccagctcagcgccctacgctacggcgccgtgccgctggtggcgcgcacgggcggactggccgacacggtggtggacgcgaatccgatggcgctgtcggcgggcgtcgccaccggcgtccagttctcgccggtcgaacaggcgccgttcgagcgcgccctgcatcaggccgccgccctttaccgcgacaagccgacctgggcccgcatccaggccaacgccatggccaccgacgtgtcgtggaacgcttcggccgcgcgctacgccgccctttatcgagagcttgcgacggctcagtagcgggcgatcgacaggtcggcggcttcgatctcgggctcgcggccggtgatgatgtcgctgaccacccgggccgatccgcaggccatcgtccagcccaaagtgccgtgcccggtgttcagataaaggttcgggacgcgcgtcgcgccgagaaccggtgtaccgtccggcgtcatcggccgcagcccggtccagaacttcgcctcttccaaagcgcccgcccccggaaacaggctgttcagggaatacttcagcgtggcctgtctgcgcggcggcaggtcgtggctgaagcccgacaactccgccatgccgcccacgcggatgcgcgagccaagccgcgtcatggcgatcttgaacgtctcgtccatgacggtggagacgggcgccgtctcctctctcgcgatcggcacggtgatcgagtagcccttcacgggataaaccggcagaccgatccgcgtgggtttcagcaacgccggcgtatagctgcccatggccgcaacatagacatccgccgtccgctcgccgcgactggtcgagacggatacgacgcgtccctggtccaccctcaggccgcgcacctcggtcccgaacaggaagcggacgcccagcgccttggccatctcggccagccgctgggtgaacagggccgcgtcccccgtctcgtcgttgggcaggcgcaagccccccgcgatctccgcctgggaggccttcaggccgggctccgccgccagacagccctcgcggtccagcacctcgcatggcacgccctcgtgacgcagcacctttacgtccttggccacgtcctccagctgcctttccgtgcggaacagctgcagcgtgccctgctgacgcccatcgtactggatgcctgtgtcggcccgcagcagcttcagctggtcgcgactgtattccgccagtcggaccatccgctccttgttcagggcatagcgttcggccgtgcagttgcgcagcatctgcagcccccagcggatcatggcggggtcgaaagtcggccgcaggatcagcggcgcatgcttcatcatcagccagcgcggggcctttttggggatcgacggcgccgcccagggcgaggaatagccgggcgaaatctggccggcgttggcgaagctggtctccagccccgggcccgcctggcgttcgatcaccgtgacctcgcagccggccttggccaggtagtaggcggtggtcacgccgatgacgcccgcccccagaacgatgcacttcacgctcgacctcccgcgcgcttttggccgcaggataacgaagatcgtatcgccgatcctgcgccgctgtggcaggatcgttcagtaacaacatcaaacgcgcacgatctgcgacatcttcagcaaggatcagcatgcccggcctcgacgatgtggatcgcaggatcgtccgtcagctgagagcaaacgcacgcattcccaatgcggcgctagccaagagcgtgggcctgtcgccgtccgcctgcctgcgtcgcgtaaagctgctggaggatcggggcgtgatccggggctaccaggccgtggtggccgagggcgatgaggacagcgtcgtcgctattgtcctgatcactttggagaagcagaccggcgactacatgcgccgcttcgagaccgcggtccgcgagcaccccgagattcaggaatgctacctgatggcgggagaggccgactatgtgctgcgcgcggcggcgcccagcatcgcggcctatgaggtgattcacaaggacgtcctgtcctgtctgcccggcgtgtcgcgtatccactccagcctggcgatccgcaacgtgctggcgggtcgaggccggcgttgaagccgaccccgccctcgacctaggcgctcagtcccgcagccgagaccgccgcgacgcccgtgctcgcgaccggacgcagcttgcggaaggtcgttagggcctgcccgacgacttgatccatgttgtagtagcgataggtcgccaggcgtccgacaaaggctacgtccggacgcgccagcgccagcgcttcgtacttcttgaacagcgcctggttttcggcgcgagggatcggatagtacgggtcgccttccgccgcaggatattcgtaggtgacggtcgtgcgcggatgcgactggcctgtcaggtgcttgtattcggtgatgcgcgtgtacggcgtcgcctcgtccggatagttgaccgtggcgacgggctggaagttcggctggtccagcgtctcgtggcggaagcgcagcgaacgatagggcagcttgccgtagcgatgatcgaagaactcgtcgatcgggccggtgaacaccagccgatcgtggaccacttcgtccaccacatcgcggtattcgacgcccgtctccacctggatgttcgggtgatccagcatattttcgaacatcttggtgtagccgtgcagcggcatggcttggaaagtgtcggtgaaatagcgatcgtcgatattggtgcgtgtgggcacgcgcgccgtcaccgacttgtccagctcggacgggtcgagcccccactgcttgcgcgtgtagccacggaagaaggtctcgtagagttcgcgacccacagccgaaatcaccacgtcctcggaggtgcggatcttctcgacgggctcggcgcgcgaggcgagaaacgcctcggcctgctcgtccgattgcaggtccacgccgtacagggcggtcagcgtagtccggttgatcggcatcgggaccagcttgtcgccgacccgcgccagcacgcggtgttcgtacggccgccactcggtgaagcgcgacagatagtcgaacacctcggccgagttggtgtggaagatatggggcccatactgatgcatcagcacgccggcctcatccagccggtcatagggcgttgcccgctatgtgcgggcgccgatccaccaccagcaccttctgcccgctggacgccagccgctcggccagcaccgaacccgcgaacccggcgcccacgaccagagcgtcatagtgcgaggcgcgtcccgccgcctggatcgccggagcggcgacagggccggacagcttcatgaaaccccttccgaggcgcttgcgcaccgcgccgtcgatcaaggccgacatgcgcagttgcgtctgctcccatgacaggctggccagcgcctcatcgacctgttccagccaggccggcgtctccttgagcgcgagctgcgcctcgcaggcggcgatgaaggcctcggccgtttcggcgatcttcacgccctccagctcgccgtagtggcgcaccacgtcacggatcggcgtggacacgacgggtcggccggccgccaggtattccggcgtcttggtcgggctgatgaaacgcgtcgaatcgttgatcgcgaacggcatcaacgccacgtcccagccgctcaggaaggctggaaggtcgtcatagctctgctgacccatgtagtggatgttgggacggcgcggcaggtcctgctcggcgatcttgaccaccgggccgaccagcaccagcgaccagtcaggacgcgcgtcggccaccgccgccagcagttccaggtccatccgctcgtcgatgacgccgtagaagcccagcctcggccccgccaccgccgactgagccgagggctggttcaatccgctgcgcgcctgcgcgaagtgctcgcgctccacgctggaggggaaaggatggatgttgtcgtgccggttctgcttggcctcatagaggctgtagccgccggtgaacacaacgtccgcccggctcatcaactcggcttccaactgcgtcagctcaggcggcgcgaacctgaaggccgatagttcgtccatgcagtcatagaccacggccgacgcctcgatgtgccgcgacaaggacagcatcatcggcgtgtagtaccagagcacggggtgctcgatgctctggccggccagcacctcgtccagcaactggcgcagcaccgcggtgcgacaggcgccctccagcccctcgggcaggcgcggcgtcgccacgaccacgccgcttgcggcgcatcggcgaagatcgacgcccatggccatccccgcctgcgccggcattggctcctcgaagaccaccaccgttcgtgtccgggcgaaccgcgtcatcaggtgctgcgggcgctggaacacaaagtcccatcgcaggtgagagaagcagacgatcggatcgccgcgatcttgcggcttggccagttcgacgacgtcggcgcggatgctggtgtctgtggtgttcaaggctggcctttccggagatctaggctgaggccgctgttcggacggagccggttcgcgggatgggttgtttttgggggggcggctgcgtcaccagaccagggctgatccagcagcaggtcgacggcgcgagacagggtcgaaccgctgtcgaacgtcttgacctccagccacggagcatcgtggccgagctcgcccggacggacggcgtgcagcccccgctgctcgcactcaatcgagagttcgcgccaccggtcgccgtcgtcggtgctgttcagcaagataggtcggctgaacggtcggcgtggcggcggcgcgccctcttccgccacaggatgaggcggatagaccagacggccgggcctgcgccaccagccgggctcatgcgcataagggcaatcggtgtgactgtcgcgggccaggtctctcagaacctgggccagcgcggtgggcctcagcgttccgtccgaaaggtcgaagacgccgctttcgtatacgccgtccggacgagtcagcaggctgttccagtcaaagccgccaagcagattccacacggtcaccgcttcaacgtccacgccctcttcacgcgcctgcacggcggcgtcccagcattcggacagccagcggacctgttcttcacgcgtacagccgagatgacattcggtgacggcgatcgtccggccatagcggagccacagcgtgcgcaggtgttccgcccagccgacgggcgcaggatcgatgaccctcacagcctcgacatcggcgtaggcgagccggccgtttccaccatgaaggtgctcggggtagcgctccagtcggtgatccaggaagcggtcgctggtggcgtaatgattgagcccgacgacgaagtcggtcggctcgtccgcgatcgccgccagacgatcccccagacccagccgggcgatatgctggtggagcgggcgcccaggcgacacacgtcccgccagcaggtcccaggtcgcgaaccgacgcacattgtcgtgcttggcctgagctgcgcacgcagccgtggcgtaggtgcgcccgaaatcctcggtctggatcaggcgcgcgtcgggattgaccgcccggatctcggccatcgccaggcgtatgccgtcgatctggttcagcaccgccgtccagaaggccgtctcgtccctgaaatggggataccagtgaccatagagagcgctaaaccgggccgtggtcagcggctcgttgatcggcgtccagtcccgcacccacggatatcgcgccgccgcccgaccggcgaaggcggccaacgcttcaggaaactccggatcaagcaggttggtccagccggggcccgatccatggtgaagcaggccgacgatgggccggacttgaagctcgcgcagacggttcaggcgggcgtccgaccaggaccactcaaacttcccgggcgcgacttccgtgcgctcccacagcacgggatagcgcagaaccttgacgccaagctcggcgaagcggtccagatcttcgatacgatcatgatgtccggaaaggcgcgtctgatctcgccaatcatcgcccacccggttcacggtgcactcgtgccctccccaaagggcaaggcggccagccgaccggcgcggagcgccagccgtgggcgtcaaccccggatcaatcatcggtggtcccttccgacgaccagaatgccgcagggagacgaaaggttccacaaggcattgaggcgcaagggcgtttcaccgccactgtcgatcaatagctgcgggtcaaaagctcatcgagacccaccgctcgcacgtactgaaacgccggcgcggaggaaccgcgccggcgctcagaccgtgtgccgaccaccgcccgcgcaaacgggcggacttcaggtgatcaggcgaccagttgccagtcgacgtgaaccttggcgatcgcatccggccggcccagatcgccggcgtcccaggacgccgagccgaaggtcggcgtcgccacgtcattgaaccaggcgccccgcagatcgcgagcgcccacgccttccagcaggatcgacgatccatcctcgaacgagatcagggtgtctcgcccgctttgctggacggtgtgatcaatgccagccgccgtcatcgccgaccagtcgatgacgtccccgctgcggaagtccgtgatccggtcccctaggttcggaacctaagacaaaggtgtcggtgcctgatccttccgtcaggatgtcgttccctgccttggaccgaaagccagaaggcgcgattgcagctggcgcgcaaagccctagctggagcccgtggtcgagttgggccgcggtaatcgttctgcgcggccgttagcgatttggtaatcatcctcattattgaggagacgaggttcgtcgagcagcgggattcacaacgctcgccggcgttagccctgtaaaacctatggctcgtcagggttttcgcgtcatgagagaaaacgcgggaaggctggctttttttcggattaagctcgaagcttaaccttatcctgcgctgattggcaactttcgccaggtgtcgatcagcgagcctgatcgcgaaagcacggcgacgcacccgtcgagaggaaaatcccggaagtgggacagacatacacaagatcggagccgccgacgccggcgccggctatgccccggctgcaggagccggcgtacgccgcggaggtgcttgaggctttggggctcgccgcgttcgtctgcggtgcggatggcaaagtgctcgccgcaacatccggcggtctgcgcttgtttgatcaaggcctctatgtgcggctgaaggacgagcagttggagatgcgagcgtcaggatcacagacgcttcgcgcagccatcagcgagacggcgtcagctcaggctgcaggcgctcggctgctgccgctgcacgcgcctgacgggggcgaaacggccttggccgagatcgtgcggctcggcgatggcgaggggagtgggacgggcgtcgtggtgatcgtgcgctggcccggctccgactcagcggaccgcgcctcggctgcggcccgggtgctgtatggcttcacggccgccgaggccgccgtggccgcccatctgctaaagggactgagcccccaggcggtcgccgaccgcatggaggtgtcgatcagcacggtgcgcagccacatccgatcgacctttctgaaggccggcgtgaacagccagatcgagatgctggcggcgatccgctgccgcatctgaacggcgggacctagagcggcgcgcaggcccttttgagccacgccccgacgtcctcgtcgagcagcggcctgatcttggccagggtctccgcgtgataggcgtccacgtaggcccgctcggccgagctcagcagatcgacgtcgatcagcctgcgatcgagcggcgcaaacgtcagctgctcgaagccgtgcatcggccgctcgccaccttcgacggcggttgcaggcgtcaccacctgcagcgtttcgatccggatgccccagtgcccctcacggtaatagccgggctcgttcgacaggatcatgccctcgagcaatggctggtccgtgccccacttggcgatccgctggggcccttcgtggacccccagatagctgccgacgccgtggccggtgccatggtcatagtcgaggcccgccgcccacatcggcgcgcgcgccaccgcatccagctgtcgccccgacgtgccttcgggaaagcgcaccacggccatggcgatatggctcttcagcaccagggtgaacatgcggcgctggtcggccgtcggctctccgaccgacacggtgcgcgtgacgtcggtggtgccgtcgaggtactgccctcccccgtcgaccagcagcagcgagcctcgctcgatgcgccggatggagcttccgacgggcttgtagtgcggcaaggcgccgttcggcccggcgcccgcgatggtgtcgaacgacaggtccttcagcgcgccggtctcttcgcggaaccgctccagcgcctcgaccacctcccgttcgtccggcagggtctcctgggccaccgtatccacccagtgcaggaagcgcgacagtgcggcgccgtcgcggatgtgcgcctggcggctgccttcgatctcgaccgcgttcttggccgcccggggaacggcgcacggatcctgtccgcgcacgacctgggcgcccgccgcctgcagccgctcgaagaaccaggcggaagacacggccggatcgaccagcacccggcggccggacagcgcatccagcgccataggcaggccgtcggggtcctcaatcgacacggtgtcgccgagccaccccggcagttcattggtcaccttgcgcgggtccagaaacaggcgcgcgcgcccatccgcctccaggatcgcctgcgccagcggcaacggcgtgcggatcacatctccgccccggatgttgaacagccaggcgatggatgcgggcgcggtcagcaggaccacgtcggcgcccgcctccgccaccgcgcgtccgatgcgggtgcgcttgtctgcatggctctcaccggcgtagcggtcttcgtggggcgcgacaggcgccgacggctgcgccggccgatcgtcgccccaggccaagtccatcggattggcttccacagccttcagttcgcctcccgccttgaggaccgcgcgccgcagcacgctcagcgcatcgggactgtgcagccgcggatcgtagccgatgaccgatcccgcaggcgcgccctcgagccaatccggcaaggccgctagatcgacgcgctcgaacaggtccccgtccgtctgggcacgcacctgcacggtgtagcgcccgtcggtgaagatcgccgcgcgatcgctcagcaccaccgccgcgccggctgagccggtgaagccgctgatccaggccagccgctcattggcctccgggaggtattcgttctggtgctcgtcttcgtgaggcacgaggaagccgtcgagcccctgctcggccatgcgcgcgcgcagcagcggcaggtggcgggctccgaacgcaggatcggtggattcgtcgaatgtctggcgcattctccagccctaggccggtctcccgccgggctcaagtcgtggcccgcgcgatcaaggattgctgatggaacgggcgagggtgcgtcttgttacccctttcacaccctaaccgcagaaggactttgcgatgaaccgcttcgcaggcaagaccgtgatcgtgaccggcgccggctccggcataggccaggcgaccgcccgccgcttcgctcaggagggcgccaacgtcatggccgccgacgtcgacgaagacggcctggcggaaacgctgaagggagtggacgcctcgcgcgtcgtgacgcgcatcgtcgacgtgtccgaccaggcgcaggtcgaagccatggtgaaggcggcgaccgatcgcttcggccgtctggacgtgctggtcaacaacgccggcgtcggctgcgacggcacggtcaccgaaatggccatggacgactaccgcaaggtgatggcgatcaacgtggacggcgtcctgttcggcagccgcgccgcttatcccgagctgaagaagaccaaggggtgcatcgtcaacacctcgtcgatttcgggccttggcggggacggcgccatgatcggctacgacatggccaagggcgctgtgtcccaactgacgcgggccatggcgcgcgacagcggccgcgacggcgtgcgcgtgaacgccgtcgcccccacgctggtgcacaccggactgaccgccgacatggaggacgacaaggcgctgatggacgccttcgcgaaggccatcccgctggggcgtggcgcccagccggaggagatcgcctccgtcatcgccttcctggccagcgacgacgccagcttcgtgcacggactggtgatgtcggtggacggcgggctgttcgcctcgaccggccagccggacttcaaggacttcagctgatcagccgacgcggcgcagaaccagggcgctccaggcgtcgtggcgtatgcgccgctccagccggaaaccgcgggacagataagcggcggtgacgcgccgctcctgcgtccgtagcaaccccgacaggatcgccacaccgtccagcttcagcgccatgcggatgtcctgtgacagggccaccaacggcggcgccaggatgttggcgaacaccaggtcataggggccgtgccggcgcacccgctggtcgttcagccccgaagcatgaacaaacgtcgccttggcccggttcagggcggcgttttcgttggcgatgcgcaccgacggcgcgtcgatgtcggtgccgaccgccacgcggctgccggtccgcgctgcggcgatggccagcacgcccgtgccgcagcccacatccagcacccgctcgaagctttcgcgcttcagcagttcgtcaaaggcctcaagacagccgacggtggtgccgtgatgcccggtgccgaaggcggcgcccgcgtcaatcttcagattgatcgagttcggcggcacacggccttcgtcgtgggcgccatagacgaagaagcgaccggccgtgaccggcggcaggcccgacagcgacatggccagccagtcggcgtcggccagcttctcgactgacacagtcacgggatgatccgccatcgccgcttgcaagccctcgacctcgtcagccgtggtcggaaaggcgtcgatgcgccagaggcctcgatcctcgtcctcctccaggatcgaataggtggcgccctccagcatggggtcggcgtcgatggcggcggcggcggcctcgcaggcggcgcgttcgccccgcgcgatcacctgaacggcggtttcggacatgtctcaaacccggttaggatggggaatcggcgatggcgcgacagacgcgcccgcgcacgtgctgtcaatcggagggtggcaaatccatggccaagacgccgtcaaacatcgaaaccggaccctctgaagaggccgccgcgaagccgaaggcggcgcccaggccccgggcgcctcgcacgaaagccgcgtcctccgtctcggacgccgaagccacgccagcccccaagaaggccgcgacccgctccagaacgacggcctccggcgtcgccggcgcgaccacgactcgcgccgccaggccgaaggcttcggcggttggggaaggcgccgcgaagtccccgcgcccgcgcacgaccaaaccccggatccagccggctcccgaaggcatggtcgccgcccccatcgtcgatccggttcatgaggaagcgccggcgacggtcgatcccgcgcccgccgcggccgcctcgaccatcgcgccggaagccgcgatccccgccgccgcagccagcgcggaggccgagactggctcttcgccccagcccgaggctgcgtcgccgatgacccaggcgacggccgaggtgacgccgcaggcgcataggcccggcttcttcgccaccctggcgaagattatcttcggcaagcgctgaacgcttccctgaacagcagaaaaggccggacggtcacgcgtccggcctttgccctcgccatgtcgcgtgcggctcagtcctgcaggtcttccgccaggatcgccatttcgaacatgaaggagccggcttcgtcctcgtcttcgaacaccacgccgatgaactcgtcgccgacatagacctcagctgagtcgttctgcttgggccgcgcctttacgatgatgccgccggtgttgaaggtgcgcttgagatggctctcgatgcgcttcaggtcggtgtctttcatcggtccagcctttgttcggggattggcgcgggaccctagagaaggccgtccgcgatgaaaacccgtcagatgacgaagtcgtagaccacgtccgcaagcgtatgagccatggtgcgtgcgggctcggcgttggtcgggcagttgaccagccgcgccggcacgcccgcgaccgtgcagcccgacggcaccgccttcagcaccaccgagcccgaggccaccttggcgtagtcgccgatcacgatgttgcccagcacctttgccccggcccccagcagcacgccccggccgatcttggggtgacggtcgccgcgctcggcgccggtgccgcccagggtcacgccatgcagcatggacacctcgtcgtccaccaccgccgtctcgccgatgacgatgccggtgccgtgatccagaaacagccccttgcccatgcgcgcgcccggatggatgtcgagctggaacagctcggagatgcggctctggaagtgaaaggccagggtctcccgcccctgctcccacagccagtgcgcgatgcgccagccctgcagcgcctgaaaacccttgaaatagaggaacggctgcagcagcgatcggatggccggatcccgctcggcgaccgcctgcaaatcggcctcggcggcctctacgatgcctggatcggcggcgtaggcggacaggcagatttcgcgcgccgacatggcgccgagttcgtcgtcccccagcttgcgcgcgacctggtagctgagcgcgcccgccatgtcgtcgtgcgacaggatcaccgagttcatctgcgaggccagttgcggctcctcgcgcgtggccgcctcggccgaggcgcgcagctggcgccagggtccggccgtctccgggaccacttcaagcttgggcatcgccgtctcctcgtggcgggccatcatacgccctcgagcatggcgcgcgccagcgcgggcggaagcagaccctctcgcgccatatggtaggcccgatagacggcggcgatggtcatcacgtcccagaccgcgcctcggccgatggcgtccagcacctgtcggaacggcgcgcggaccaccgccagcacttcggtcgcatccgccgccgtccgcgcagacgggcgcaggtcccaggcgatccaggtgtgcgccacctcgtcggtgatggagttagacagctccaccaccatgggcgccgaccagctgtcggccgcgaggcccgcctcctccgccaactcgcgtcgcacaccctgcgcggggtcttcgccgggctctgcgccgccctcgggcatctcccaggaatagttcatgcgcgcgaaccgctgctggcccaccagcaccaccgcgccgtcgtcgtggatcggcaggacgccggtcgccacgttcttgggacgcatcactgtgtattcggtgtcggcgccgctcggcgccacggcctgatagcggatcagccgcatccacgggttttcgaacaccggcgtctcgcgggtggagcgccatgccggcggcttcggcagatcggcggcccaggggggttcgggaacggcggcggcggtcatctccgacctatgcggcgccgcgccgagcggaaccagccctctagaaaagcccctcgcccttgggcagttcagcgtagcggtgcacccgcgtcgccatgaccagggcgaagccgaacatcaccgtcatcatcgacgatccgccgtaggacagcagcggcatcggtacgcccaccacgggggccaagcccatgaccatggcgccgttgatcatcacgaacagggcgaaataggcggtcatgccggccgccgcgatgcggccgaagtggctgtgcgacagggaggctatccgcagcgcgatcaggatcaccgcgatgtagcagcccagcatggtgaaggagcccaggaagccgaactcctccgacacggtggagaagatgaagtcggtgtggcgttcgggcaggaactccaactggctctggctgcccaggccgtagcccttgcccagcaagccgccggcgcccagcgcgatcttggactggatgatgttgtagcccgtgcccgacggatccgaggctggatccagaaaggtcagcacccggtttcgctgatagtcgtgcatcacgaacatgacgaacggcggcacgatggcgaccacggccgcggcgcaggccgcgatgatccgccagctcagccccgccaggaacatcaccaccgcacccgtcaggccgatgatcatggccgaccccaggtccggctgcttggcgaccagcagaaagggcacgccgatcatggcggcggggaacaccagcttccaagaccaccgcgcttcttgcgcgctatgcttgtggtaccagcgggccagcgccagaacgaggccgatcttcatgaactcggccggctggatgcgggtgaagcccaggttcagccagttgcgcgcgcccccggccgtatagcccagcggcgtgaactcgatcatcagcaccagcagcagcagcacgccgtagatcggataggcggcgcggaaccaccacttcaggtgcaccagcgacagcacaagcatcaccgtcagcaagccgccgaaccggatcaggtggttggccgcccaaggctgccagtggccgccagcgatggagtacaacatcgctgttccagtgccggcgatgacgcacagaagcgcgaccaggcgccagtcgatctcggacagtttggtcgaaacgcgttcgcgctcgcccggacgggtcagggccgaggcggtcaacgcggcggctccgcgggcgcgggcgcggctgcggcgtccggctgaaccgcctcgggcgcggcgccctgcgcagcggcgccggcgtcttcggtctcggcgaagcccgactgctcgatgcgggcgcggatttcggggtccttcagcagggcgaccttcatcacctcgcgggcgcgcggcgccccggcggtgcccccgcccatgccgccgtgctgcacgatcaccgacacggcgtagcggggattgtcggtcggggcataggcgatgaacaggttgtggtccttctgcgcccagggccgtcccgcgcccttgcgggagcccgcgccatagttctgcgcctgagcggtgccggtcttgcccgccatccgcaccgggcccagtcccagctggctgttccggaagcccgtcccgccgatgtcggtcacggcttccatgccgtcacgcagcaccttcagcgcctccggatcatacgggaggtccgcgaagtccgcgcccggcgcctgctccaccccgccgaccgacttgatcaggcgcggcgtcaccgccttgcgaccattggccaggcgcgccgtgtacaccgccagttgcagcgcattgacgttcaaggcgccctgcccgatgccgtagctgggcgtctcgccgggataccacttgccgtcgccgcgcacaggattgtcgcgccgccactggcgatccggcaccagcccccgcttctgccccggaatgccgatgtcgaagatctggcccagccccatctcgcgcgctgtctcggcgatggcgtccggccccatctccacggccagcgtcatgaagtagacgttgcaggagttcttgatcgcgccgcgcatgtccaaggcgccgtgccgtcccaggcaggcgaagcgccgacccagataataggcgccgttgcagacgatgcggcggtccgggttggccccgcgcttcatcgccgccagccccacgaccggcttgaaggtcgaacccggcgcgaaggtgcccgtcaacgccttgtccagcagcggacgccgctcatagtccgccagcgcccgatagatgtgggacggaaccccgcccacgaacagattgggatcgaacgacggcgccgacaccatggccaggatgtcgccgttgcgcacgtccatcaccacgcacgatcccgcctcttcgccgaacacctccagcgcacggttctgcacgtcggcgtccagcgtcagcaccacttccttgccgggcactgcggggcgcgagccgccgacgtcctcggccaccacgcggccgcgcgcgtccacctcgacccggttgccgccggcctcgccgcgcagttcggtgtccagcgccttttccacccccagcttgccgatccggaacgccgggttgaacaggatggcgggcggctcctcgcccttctcgcgcatggtcttcacgtcacggtccgtgaccttggccacatagccgatgacgtgggcgaacgacccgccgaacgggtagtagcgggcgtcgttcatgtcagccatgacgcccggcagctcgttggcgtacaggttgaccttggcgaactcttcccaggtcaggtcgctcttgaccggcacgggcgaaaagcgtggcgcggcgttgacgtcgcggatgatcgcccggcggcgatccaccgtgtccggcaagagctgacccagcagatccagcgtctggtccagatccttggtttcgtcccgcaccaccagcacgcggaagctcggccggttgccggcgatcaccaccccgttgcggtccttgatcaccccgcgcggcggcggcgccaggcggaagttgaactggttgttagacgccagcgtcgcatattcctgcgcctgcaccacctgcagctggcccaaccgtccgacgagggccgtgacgcccagcgccgacaggccgccgaagaccagtgttcgcctgaggaacgatccctggcgctcgttgggatcggcgaaaaagatcgacggttcgctgctcatcggaacctcacgtcgccgtcgtcgaaccggtccagcatccaggcggcgatgggaaacaggatcagggtcgggatcacctgaccggcgaaggacaggagacttggcgcatttgcggctcgcatcgtgacgatcaaatacgccacgccgaaggcggcgagcacgcagccgacatagccggcgaacagaaacagcatctgctgtcccgccagcaggttccgcgacaacagcaccacggcgtagacgcccatcaggcacagcggccacagccccagcacatcgccccagaacagatccaggaacagacccagcccgaacagcacggcgggcgccagcatggacggccggatcagcggccaggcgaaggccagcacgaacgggaccaccggctccggcaggcccatgccgaacagccgcagcggcgttcccagcaccaccgtggcggcggccgccagcagcgccggatagacgatccactgcatcggcccgatcactcgaaccgcgacaggccgtctcacagcgcgcctcccggagaggggggcgtctcggcgggcgcaggcgacgccggggtcggagcgggctgggtcgagggcgtctgcgtcgtctgcgccggcggcgacggccgcacgggggcggacgcgaacggcgcgcgctgcgttgtcggggttggagccgccgccgctgtcggtcggccggtcgcgggggtgttcggcgccgcggcgggcgcctgggcttgagcctcggcctgcacctgggcggccacggcggcgcgggcgcgctcggcgtcggcttgcgccagcgcctgaaggcggcccaccgcatcggcgatgatggcggcctgctcgggcgtaggcggcgcggccgaccgcaggcccgacagggtcggcgcgttcagcgccgccgggttcaccagctgggcgaaatcacggaacagcagcacgcgcacatagtcgaccgcgcctcgatcgctgaacagcttgacccgccaggatccgtccagccccttggccgcgaccccgatcggcacgccgcgcgggatgccgccgccgtcgccggacgacaggatgcggtcgccggccttgaccgcgtccgcgccgcgcacgaacgccaggcggggattgccgctgccgtcgccggtcaggatggcgcgcgcatcggtgcggtcgatcagcaccggggtgcgcgaagccacgtcggtcagcagcaccatgcggctgaccccgccggtcacgccggagatgcgcccgaccagcccgtgctcgttgacgaccggattgccgacctgcacgccctcgttggagccgatatccagcaggcgcgcgttcttgaagggtcctcgtgcatcggagatcgtccgcgccgtcgccatcggcacctcgggctcgacgcgcaggcccagcatggtttcgtagcggcgattgacgttcttcagcgcgatggcgtcgtcgcgccagccgcgcaggtccgccacctcgcggcgcagacgccggttctcgccgagcgcgaagaagtagctgccgacatagtcgatggcgccgcccacccagcgcacgggcgcggaaagcgcgctgccggccggcgcggccgccgcctcaaagccgccgcgcgcggcgccgtagctggtgtttgtctgcggctcgttggtgtcgctgatcagcagcaggacggcgacgaccaagccgaccacgacgacgacggccgccgtccagaccagcggcaccttgatggtatcgaacgggccgtcgcgaaacgccacggtcagccttcctgtaagaagagtgcggtgacggcagtccccctgccgttcttcccgcctatcgcaaaatcacggcggggatggaaccattcgcgacatcgctgcccaagattatttgggcgagctcaagctttaccgcgaggccttgcgcatcagagcgccgagtcgaggacccccttcatccagcgcggatgctccagcacgcgcccgcagccgatggccacgcacgacaggggatcttcggccaccgagaccggcagaccggtgtggtcgcggatctccacgtccaggccgcgcagcagggccccgccgccggtcagcatgatgcccttgtcggcgatgtcggcggccagttccggcggcgtggcttccagcgccaccttcaccgcctcgatgatctgcgtcaccggctcagccagggcttccgccgcctggcgctcggagatgcgcacctcgcgcggtacgccctgcatcaggtcgcggcccttgacgtcgatggtcaggccttcgccgtccagcgggatgcgcgccgtgccgatatccttcttgatccgctcggccgtggtctcgccgatcagcaggttatggttgcgacgcatgtaggagatgatgctgtcgtccatcttgtcgccgccgacgcggaccgagcgcgaatagacgatgccggacagcgacagcacggccacttccgtcgtgccgccgccgatgtcgacgaccatggagccggtcggctcatggatcggcaggccggcgccgattgcggcggccatcggctcgtcgatcaggccgacgcggcgcgccgaggcgttcaggcagctgtcgttgatcgcgcgccgctccaccgccgtggcgcccgagggcacgcacacgatgatcttggggttcacgaagcccttgcgattgtgaaccttgcggatgaagtgcttgatcatctcctcggcgacttcgaagtcggcgatgaccccgtcgcgcatcgggcggatcgcctccatgtggccgggggtgcggcccagcatctgcttggcctcgatgcccaccgcgtggaccaccttgcgcccgccgacgttgcgaagcgccaccaccgacggctcgttcaggacgatgcccttgcccttcatgtagatcagggtgttggccgtacccaggtccatggcgatgtcattggagatcacgccgaacagggatgaaatcatgggatgcgcttaccgtttctcgggcctgaggacgacttgattgcagtctgcctgacgacgcccagccgtcccgcgcatccccagcgcgagaaggctcctgacagctcgcgccacgcctacctgcggcccgtttgcccgtcccaaggtgtgatggcaagccccttcgcatcgctgtggagccgataagcgcggctgttcgcggccgccgcgccaaggcgcattcacgatgccgtcatgagctgcgacagcggccagccgcagcccgtcagacagcctcgattccctcagcggtcagggcgcgttgaaccgccgggcgggcctgcacctgctccagatgggcgttcagcttgggataacgtgcggggttcagcagaccagcctgccgcgcccagcgcgtgaacacgtaaagatagccgtccgccaccgtataggcttcgcccatggcccacggcccctgcagcagactgtcctccaccagcgcgtacttggccatggcggcctccaccgccgcatccttcgcctcgccttccagcggcggccggctgaacagcgcccgaccgatcagcgggtgcagcgacgacgccagaaagccgttgaacgcctgcatccgtccgaactcgaagcttgagtcgaggttcgccagcttcgcctccgggtgggtctcggcgatgtagcccatgatcaccaggttctgggtcagcacgccctcgtcggtccgcagcgccggcgtgacgcccgccggattgaccgccagatactccggcgtcttctgctggccctgcttcaggtcgatcttatccagctcgaactcggcgcccgcctcctccagcgcgatgtgcgaggccagcgcgcacgcgcccggcgaatagtagagtttcagcatcattttctctcctgcgggccgcatcgcgttgccgcccttgcggcgcttgcgtaaacagacccgcctccccggcgcaatcgttcaatcgacgggtcctcgccatgtccagcctgcagtcgtccgccctcgcccgcgtcaagccgtcggccaccatcgccgtaagcgcacgcgcccgcgagctgaagcgcgagggtcgcgacgtgatcggcctgggcgcgggcgagccggacttcgacaccccggacaacgtcaagcaggcggccatcgacgccatcaaccgcggcgagaccaaatacaccgacgccgacggcatgccggagctgaagcaggcgatctgccgcaagttcgcgcgagagaatggcctgacgtacgagcccgcgcagatccacgtcgcgcccggtggcaagccggtgatcttcaacgccctggtcgccaccctgtcgccgggcgacgaagtgatcgtgcctgcgccctattgggtgtcctatcccgacatggtgctgctggcgggcggagagcccgcagtcgcgggcggcgaggagaaggaaggcttcaagctgcggcccgagacgctggaggcggccatcacgccccccacccggtggctgatcctgaactcgccccccaacccgaccggcgccgcctacagccgcacggaactggaggcgctggccgccgtgctgcgtcggcatccgcaggtctgggtgctgacggacgacatgtacgagcatctggtctacggcgacttcgaatacaccaccatcgcccaggtcgcgcccgatctctacgatcgcaccctgacggtgaacggcgtgtccaaggcctacgccatgaccggctggcgcatcggctatgcgggcgggcccaagccgctgatcgacctgatgcgcaaggtcgccagccagaccacctccaacccctcctccatcagccagtgggcggcggtcgaggcgctggacgggccgcaggaattcatcatcgagcgcaaggcggcgtttgagcgccggcgcgacctggtcgtttccatgctgaaccaggcatcgggcatcacctgcgccacgcccgagggcgccttttacgtctatccctcgatcgccggactgatcggcaagaccactgagagcggcgtggtgatcgacggcgattccaccttcaccaccgaactgctgaacgccgagggcgtggccgtggtgcagggcgaggcgttcggcctgtcgccctacttccgcatcagctacgcgacatcggaagcggtgctggaaaaagcctgcggccgcatccagcgcttctgcgcctcactgcgctaagccgcttgctcgtctacggagatcacgccgacgtcgtcgacgggccggcggttctgaaacgcttcatcgaagacggcgcggacttcggcggcttgcaaggcttgtcgctgcgcgcggcggtgtttcaggtctttttgcgcctttcgtccctgcttcagggctgggccgacgccgaaagcgaggcggccggcgacatcgacgatgtctcggacgcacaggaccggctgatggaggttctggtcgatcttgcgcgcgcctttgacagggcctgggcgcaccccgaccaaccggcgcctgctgtcgatctggagcgattgcgcccgctagtccgccaggccccgccccgcctgacgctgaagcatccggaaggtttcgcctactacgccctctatcccgagctttacctgcaggctgcgcggggcttgccgaacggttgcgtggtcatcggcctgcgcagcatcggcgtagggctcgcggcgttggtggcggccgtggcgaacgcccgcgcctgcgtttccgttcgcccacgcggcgagccgttcgcgcgcaggctggacatcagccccgccctgcgcgcccgcatcctgaccgacccacaagccaccttcgtccttgtcgatgaaggcccgggcctgtcgggctcctcgctgggcggcgcggccgactggctggaagaccagggtgttccggccgagcggatcgtcttcatgcccagccactcgggcgatcttggtccgcatgcccagccgcatcatcgtgcgcgctggatcacggccgagcgccgggtcgcctcgttcgagtcggtcattctcgacgcccccggagccccgctggcggcctggttcgaagacgtggcaggcaagccgacgcggccgttgaaggacttgtcaggcggtgcttggcgcaggctctcgccttggcccgatgcgcccgccgatccgtcgcgcgaggcgcgcaaataccggctgaccacggaacggggcctgtatcttctgagcttcgtcggtctggacgcgaccgccgaagagaagctggagcgagcgcgcgccctcagccgcgccgccttcgcacccgagccgctcgcccttcggcacggttttctgctggagccatggatcgacggaggcgcgcccgaccggcgacagatcgtcgaagcgctgggtccctatctcgcctttcgcgcaagcgcctttcccgccgcgcaccagggtgcgagcctgagcgagcttgccgccatggcgcgccagaacctccgcgaagccatgggccaggcggcgccggacctcggcgcatggaccgagcggcggctcgagcggcttcaagccgccagccgacccgtgcacatcgacggacgtctccatcgctgggagtggctgcacggaccgcgcggcgtgctgaagaccgacgctgttgatcactcccagtctcacgacttgatcggtccacaggacatcgcctgggatgtggccggcgcggtcgtcgaattcgacctttcggcagcggagcgatccgcgctgttaacggaaacccaggcagatccggacctgtgcgacttcatgacagccgcctacctcggctttcaggtcggctggtggtcaatggcgcaggaccccagcgccgcgagcgaagtctcccgctacgtccaggcggtccgtcgcttgtcctgaaacgacaaaggccgccgagccgttcgcccggcggccttgagttcggcttgcgcgcccgatcagggtcggctggccatgcccagcttgaccggtttggcgtcctcgacgagcgcgccgcgcttgacgccccacagcaggatgatcggcgcgccgacgtagatcgacgaataggtgccgatgacgatgccgaacatcagggcgatcgagaagccgaacaacgcctcgcccccaaacaccgccagcgccgccagcaccatgacggcggtcacgccggtgatgatggtccgcgacagggtctcgttcagcgacaggtcgatcacgtcgcgcagaggcagggtcttgtacttgcgcaggttctcgcgaaggcggtcgaacacgaccaccgtgtcgttcatcgaatagccgatcaccgtcaggatggcggccaccatgttcaggctgaactccagtcgcatcaccacgatcaggccgaacgtcaggatcacgtcgtgcaacaggccgatgacggccccgaagccgaactgcggctcgaaccggaaccagatgtagaggaacatcaggccgatcgcgacacccagcgccaaaaggcccgaggtgaacagttcgcccgagaccttggagcccacgacgctgacgccggaataggtgacctggccgacagcgccgctgatcgcgccttcgacctgctggaccacctgggtctggttgcggccttccggcacctggaagcggacaatggcggtggagccgtcgttggcgttgctgtcgcgccgggcgatgccctgcacctgcacgtcgccgagctccagggtgttcaccgcctcgcgcacgcggtccagttcgatcacctgcccggcgggttttgcgacctccatcgaggcgccgccgcgaaagtcgatgcccatgttcaggccgggatagaagcagccgatgatggcggcgacgcacagaatgaccgacaggacgccggccgcccgcgcatacttcacgaactggaagttggtcttctgcggcagcagcttgataaggggccatccacgcatcgccatcactccgcgatcggcagtttcttgggtttggccgttttcagccagtaggccagcagcacctgcgccaccagcaccgacgagaacaccgaggtgaacacgccgatggtcagggtccaggcgaagccgcgcaccggtccggccccgaatatgaacatgatcgcggcggcgacgagcgtggtcaggttggcgtcgacgatggtgcccatggccttgttgaagccggcgtccatggaggcgatgacgctgcgtcccgcccgcgcctcgtcgcgcatccgctcatagatcagcacattggcgtccaccgccaccgcaaaggtcaggatcagaccggcgatgcccggcagggtcagggtggcctgcgtcagcgacatggccgccacgatcaggatgccgttcaggatcagccccagcaccgacaccccgccgaacaggaagccgtaggccaggatcatgaacaccacgatgatggcgaagccgatggcggtcgacagggcgccggccgcgaccgcgtccgcgcccagttcggccgtcaccacgcgccgttcctcgacgttcagcggcgccggcagggcgccgccgttcagcaggttcaccagcgtggaggcctcctcgatggagaactggcccgtgatctggcccgagccgccggtgatggcgctctggatcgtcggagccgagatgaccttgccgtccaggatgatggcgaagggccggccgatgttctgggccgtcgcctcgccgaagcggcgcgcgcccgtaccgtcgaagcggaaatcgatggcgggccggccgctctggtccgcgccgacacccgcgcgcgtcaggttctcgcccgacaccaggatgcggcgcttcaccagatagggcgtgccgcgttcgtcggtcagcagctgcgaatcgggcggcacccgcccggcgacggcatcgttcaccgagttttcgacatccaccatctggaaggtcaactgcgcggtctggccgataacgcgctccagctgggtgggatcgctctcgccgggcgcctgcaccacgatgcggtccgcgccctggcgggtgatggagggctcgcgcgtgcccaggctgtcgatgcggcggcgcaccacctcgatcgactggtccacggcggtggagcccatgccctgcatcgccgcgtcggtgtagccgaagcggatgcggttgtcggacaggcgcgtcgccgcgcgttcgacctggccgctcggacctgtcgctccgcccagggtgcgcagcgcctggaaggcggcgtcgtactggccggcgttggcgacggtgacgaccaccccgccttcttcacgttgaagctggttcacgccgatcccggcctctcgaagagtgacccgcacgtcctcgaccagattggcgacccgcgcctggcgcatggccggcacgtccacctcgagcagaagataggaaccgccctgaaggtccagccccaggttcagcgcgttcttgggcagccagcccggcaggctcgcccgctgctgcggcgacaggaggttcggaaaggccagcagcacacccatgatcagggacagcaccaccagagtgactttccagcgcgacagctgaatcatggacgagggtctcggttaccggccgccgggcggcgcggagggacgcggatcaggacttggcgagcggctttgtgtcattggcggcgatggcggtgcggttgcgcacctcggccaccatggccttgaccacccgcacattgacgctgggggcgatctcgacgttgacctcggcgtcctcgacgcgggtcaccttgccgatcatgccgctggacagcaccaccgtgtcgccgcgcttgatggcgccgatcgcggtcgcgtgctccttggcgcgcttctgctgcgggcggatcagcaggaagtagaacaggatgaagatggcgaggatcggcaggaactgcacgatcacggccatcacgccgccgtcggctgctggggacattggtgaactccgggcaggggcgggccctcgtcggcgccccggtcaaaacgaggcgcggaacctagggccgaggcttgacgattgcaacgcggcgaaagcgctaccttggcaacaccgtcagcggatcgaccgcgacgggatcgtcgccctgcatccggcgggtctcatagtgaatggagggccggccgtcgccggcggtcaggcccaccgtgccgatctgctggccctggcgcacgtcctcgccgtcgcgcacggtcgccgagccgaggtggccgtaaacggtgcgccagccgtcggcgtggacgatcagcaccgtcagcccctgccccaccaggtcgtcgccgacgtaggccacgcgaccggcggccgatgcgaccacctcagcgcccgccgaggcgccgatgttgatcccgttgttgcgctcgcccatgccgaccgggccgaagcggcgcaggatgtcgcccctcaccggccagatcagcgccacctgcgccgccccttgggtcggtacgctggccaagggcgcgctgggccgcgactgcaccggcagggcggcgttgcccgaagggggcggcggaggcggcggaaccgcgcccccgctggggaccaacacgcccaccggcgaaggcccggtggcgtaggggtcgcgccccgtgtccaccgccgagtcgggcagcacgatctgctggcccggcgtgatcgccccgcgcggccccaggttgttcaggtcgatcagcgtctgcaccggcgtctggaaccgccgcccgacgcccgacagggtgtcgcccggctggatctgataacctgcgcccgccacgaccggcgcgactgggcggggcggataggccgatgcggggctgggagccgcctcatacggccgggccgatgtcggcggcagaacgccgccctccacgggagcgaccggcgcggcggacggcggcggcgcttcataggacggcgtcggctggacaggtgcggtcggctgggagccatagggattgtacggctggcccgcgggcgttccgggcggcggatagccggcggcgcccgtgtccggcgcggcgcgcgtcgaatagcgcggctccgacggatagctgacgcaggcggcgaggctcgccgccgcgcccatgatcgccgccatcctgatcacgcccgaccccttggccattcgtcgcctcgcctgctgcctgaagaattcgcccgcccggtgtgcccgcaagagccccacaagccaaccccgcaaacggcgcggaagttgggcgataaggttaaggacgcgccttacccctccttggccgtcccctcgaccagcggcacgaagcggacctccgtcagggtctcgcggcggaaggagccgtcgccttggccgacatagcggttcagcatctgcacggaggtgcggccgacaggcgcgaccagcacgccggtcggcttcagctgcttcagcagctcggtcggctccgtcgccgaagccgcggtcaccatgatgcggtcgaacggcgcctgttcgggccagcccaagccgccgtctccgtggcgggtgatgacgttgtcgaggcccagcgcgcgcagccgctcctccgcctcgttcagcaggctgcgatagcgctcgaccgagtagacgtagcgcgccaggcggcccagcaccgcgcactggtatccgctgccggtgccgacctccagcacgcggtggcgcggctgcacgtccagcgcctgggtcatcaggccgacgatgaagggctggctgatcgtctgggcgcagtcgatcggcagggcctgatcctcccacgcctgatccaggaacttctcgtgcacgaacagggcgcggtccacgccttccatggcgcccagcacccgcgcgtccgtcaccccctggcgacgcagggccaggatcagccgcccggcccgttcgtcgtccagcttcacgcccgctcgaccttgcgcggcggagcgccgcccagcaccttcctcaggtcatggacgctgggcatgtgggtcaggtcgacgtgcagcggcgtgaccgaaatccgcccctcgtcgatggccctcaggtcggtgccctcggcgtgctcctgcttcttgccgcgaaagctcatccaatagtagtcgcgcccgcgcaggtcggtgcggcgcaccgcgtgcatctcgccgatgtcgcgaaatccttgcgtggtcacctcgacctcgctcaccgcctccggcgggcggttgggaaagttcaggttcatgatcacgttgggctgccaggtctgctccagcaggcgcgagacaatcgccggtgcgaacgcctcggccgtttcccagcgcgcgatcacctcgtcgtggaaccgctcaaggctctggctgagcgcgatggagcggatgccgaaggccatgccctgcaacgcgcccgccaccgtgcccgaatagctgacgtcctctccgatgttgtgcccccgattgactccggacagcaccaggtccggcttctccggcatcaggtcgttgaccgccaggataacgcagtcggtcggcgtgccgctgaccgcgaaacgcttgtcgcccagctggttgacccgcagcggctcggtcagggtgatcccccgccccttggccgactgctcggtctgcggagccacgatccagacgtcgtccgagagcgtccgcgcgatccgctccagacaggcgaggccttccgcctcgatcccgtcgtcgttggttagcaggattctcagcgcagcacccgcacgctgtcggcctgaattacaaaggcgccgcggcacaggttgcggatgcgcgatccctgccaaaccagtgtctgaccggggttgggctggtgccaggccgccgcacgaccggtgaaggtcgcctgcgttccgttgaggtccgcggccgcgcgctggacgttccggggcagggccccggacacgcagggccgcgagaatggctccctcagctgccgctgctcgcgaaagagctggaactcgccttcggaaactcgaacccagcccgtgaactcgttcgccacagcgtcaaaggacggatcggcaacgatctccccgtcccggccggtcgcgcagccagccagcagggcgcccgccgccacgatcatcgccgttgtcttcatcactcagcctccaatgtgggtcacgccgcccatatagggctgaagaacgcccggcacggcgatccgcccgttctcatcctgatagttctccatgatcgccaccagggtgcggccgaccgccagccccgagccgttcagcgtgtggacgaactcggtcttcttctcgcccgcacgcttgaaccgggcgtccatgcgccgcgcctggaagtccccgcagttggagcaggagctgatctcgcgataggtgtcctggctgggcagccagacctccaggtcaaaggtcttcctggccgaaaagcccatgtcgcccttgcacagcagcatgcggcggaacggcagctccagcatcttcaggatggtctcggcgcaggcggtcatgcgctcgtgctcggcgtccgagtcctccggccgcgtgatcgacaccatctcgactttggagaactggtgctgacggatcagcccgcgcgtgtcccgtcccgccgacccggcctccgcccggaagcacggcgtcagcgcggtcaaccgcatcggctcggccaactcctcctccgccaggatgctctcgcgcaccaggttggtcagggagacttcggcggtggggatgaggttaagcgcaagcgtattcagcgatcttaattcttcgacaatgttctgacgcaggtgccgatcgtactcttcgagctttgataacacgaaatcacgtagatcgtacccgcccctcacggctctgtagctgtcaccgagatgctcatgcggatcaagcacgtccggtatgccggaattgaaggctggttcgtgcacatacatgaaaggatcgactaagagcgtatcctcatcatcgaagtcgaaggaggggactacgcggaataggtcttcctcgaacttcggcaactgcccggtgccgaacatggcttggttgcgcaccagcaaaggcgggttcacctccagatagccgtgctgctcggtctgaaagtccagcatgaattgaccgatggcgcgctcaagccgcgccaactgccccttcagcacggcgaaccgcgcgcctgacatcttcgccgccgcctcgaagtccagcaggcccagagcttcgccgaggtccgcatgattctttgccgggccggtgcggcgcggctcgccgtggcgatgggtctcgacgttgcccgcctcgtcctcgccgtccggcacgtcgtcggccgctaagttgggaagcgccgagagaaacctatctctggcttgctccgccacctttttctgttgttctaagcgcgcgaccagcgccttaccttcacctccggccaagccgattgctcgcttgagttcagcctcgtagaaagccaggtcatcatcgtcctcctcacggcgcgctttctgcacatgcccttggagcacgccaatctgcttggcagccgctttctgaaccgactgaccttcttcgaaggcggtggtggcctctctaaaggcgcgatcaagcgcggcgaactcgtgcatcttgagttccgcctcgtccacgccgcgcgacagccagccggccacaaaggcgtccgggttctcgcgaatggctttgatgtcgtgcatggcggcgtcttcgtggctcgtcaggaagcgcaacgccttaacgggccgaacgggcctgagcaacgccgccgccctcgcgcggcgtcgccaatccgcctatcctgcagggactcatgccgatccgccgccttccgcccgaaaccgtcaaccgcatcgccgccggcgaggtggtcgagcgcccggccagcgccatcaaggagctggtggagaacagcctggacgccggcgcccgccagatcgagatccaagccgacggcggcggcctgtcgcgcatcctgatcgccgacgacggccgaggcatcccacgggacgagctgccgctcgccgtcgaacgccacgccacctccaagctggagcccgacgacgcgggcgacgtggacctgttgcgtatccacaccctgggctttcgcggcgaggccctgccctcgatcggttcggtcgcccgcctgacgatcaccagccggtcgcgcgatgcggacgacgcctggtccatcgccgtcgagggcggcgatcagcacccgcctgcgccctcgggcttcccgggtccgcacggcgcccgcgtcgaggtgcgcgacctgttctacgccacgcccgcccggctgaagttcatgaagtccgagcgcgccgaggccatggccatttcggaagagatcaagcgccaggccatggcgcacgaggcgacggccttcaccctgtcgctggacggcaagaccaccctgcgcctgccggccgagcaccccggcgacgagggacggctgaagcggctggccgccctgctcggccgcgacttcgaggccaacgccctgttgatcgaccaggagcgggacggcgtgcgcctgtccggctatgcgggcctgccgacctattcgcggggcaatgcggcgcaccagtatctgttcgtcaacgggcgccccgtgcgcgatcgcctgctgcagggggcgttgcgcggcgcctacgccgacttcctggcgcgcgaccgccatccggcggcggccctgttcctgcagatcgatccgctgctggtggacgtcaacgtccatcccgccaaggccgaggtccggttccgcgaccccgcgctggtgcgcggcctgatcgtcggcgcgctgcgccacgccctgcacgccgctggtcaccgcgcctccaccaccgtcgcggccgacgcactaagcggatttcgcgcccacgccggcgcgccggcctacagcccgtccgcgccttccgccgtcggcttcagcggctggacgggctggagccagccgacggcggcggcgcaggtcctgcccggcctcaacgaacgctccgcccgcgtcgaagccgactggccgcagccgggggccgcgcccgactccgccgccccacaaccttcgtccgtcgtcgatccgctggactatccgctgggcgcggcgcgggcgcagcttcacgccaactacatcgtggcccagacccgcgccggcctggtcatcgtcgaccagcacgccgcccacgagcgcctcgtctatgagcgaatgaaggctcagatggcgcgggggtccgtcccccgccaggctttgctgacgcccgaggtggtcgaactcgatcccgccgaggccgagcgcgtgtccgtccgcgccgacgaactggccgagctgggcctccttctggagccgttcggcgccggcgccgtgctggtccgcgaaaccccggcgctgctgggcgacaccgacgtgcagggcttggtgcgcgacatcgccgacgacctttccgaacacggcgccgccctgtcgctgaaggagcgtctcgccgccgtctgcgggaccatggcctgccacggctcggtgcgctccggccgtgtgctgtccgcgcccgagatgaacgccctgctgcgccagatggaggccacgccccactccggacagtgcaatcacggtcgcccgacctatgtggagctgaagcttcacgacatggaaaagctgttcggccggcgctgaccggcgaaatacttgactaattctcaggggcttctatatcagcgccagcctcgggacaggtctgcgatccgcgccgcccgctcgcccaagcatcagggcggttccgtcgcttaaagacgcacgcagacgcttttttcgtccccaaggatacatgacagaattcaccaccctgggcctttcgcccacgaccctgcaggcggtcgccgagaccggctacaccaccgccaccccgatccaggcctcggccattcccgtggcgctcgccggccgcgacgtgctgggcatcgcccagaccggcacgggcaagaccgccgccttcaccctgcccctggtcgatcgcctgtccaccggccgcgcccgggcccgcatgccgcgcgccatcgtattggccccgacacgcgaactggccgaccaggtggccgaaagcttcgccaaatacgccaagggcacaaagctctcctgggtgctgctgatcggcggcgtgtccatgggcgaccaggtcgcggccctgaacaagggcgtggacgtgctgatcgctacgcctggccgtctgctcgacctcttcgagcgcggcaagatgctgctgaccggcgtcgagatcatggtggtcgacgaagccgaccgcatgctcgacatgggcttcatccccgacatcgaacgcatcttcaagctgacgccgccgcgccgtcagaccctgtttttctcggccaccatgccgccggagatcacccgcctgaccaccgccttcctcaaggatccgacccggatcgaggcgtcgcgtccggccatgaccgccgacaccatcacccagtatctggtgcgcatccccaccagcgaccccaaggccaagcgcaccgccctgcgtgcgctggtcggccgcgaggacgtcaggaacggcatcgtcttctgcaaccgcaagtcggaagtggacatcgtcgccaagtcgctcaaggtccacggcttcgacgccgcgccgatccacggcgacctggatcaggcccagcgcatgaagacgctggccgacttccgcgccggcgatctgaagattctggtcgcctcggacgttgccgcccggggcctcgacattcctgacgtcagccacgtcttcaactacgacgtgtcgcaccacgccgacgactacgtccaccgcatcggccgcaccggtcgcgcgggccggctgggtcaggccttcatgatcgtcactccggccgacgacaagtcgctcgacaaggtcctgaagctgatcaagaaggagccggaggagctgtcgctcgacatcgacttcgccgccatcaccgacgcgccgcgccgtgacgagagccgcggccgcagccgtggcgaccgccccgagcgcggtcgcacgcgccgcgaagagacgcccgaggccgtcgctgcgccgtccgccgaagtggaagcctcctccacccgctcgcgcgcccgccgaggccgcaagccggaggcggaggttgagacgcaggtcgcgcccgcgcccgcgcccgaacccgttttggtagaggcgcccgcagagccgcgcactgaagcccgcacgccccagcgctcggaacctcagcttcgccagtcggatcgtcgcggcgagcgccgggcgtctgaacctgaacgtggcggcgttcgcggcttcggcgacgatatccccgcttttctgcgtcgtcccgtctccatcccagcctaggggcggcgcggacttaactcggcgttacggatagtggcgctactgtctccataggaacggcgaatcgcaatcgccgcagtgggggatgagaatggcggctcaggttgatctcgcgataaggggcccggcggcctatggcctggcccaacgcgtcatcaccgagatggaagccgccggcgtctggccgacgccgctgaacttcgaaatctggctcaacgccgttcacgagccggaaggcgcgctggccaccgagatccagcgtgtgctggcggtcgagggctccatctctgaggccgactcggaacgcctggccgccaagttcctgccgcgcaacaagctgagcgagcagatgcgcgacgccggcgcggtgctggatcgcgaactgtccagcgtcgccgacgtgatcgccgaggcgcaccgctcccagcatgcctatggccaaaccctggcgggcgcgtcggagaccatcagccacaccaacgacgggcaggccctgaagacgctggtggccagcctgacctcggccaccgctaaggcgcaggcccagacctccaagctggagcagcgtctggagtcgtccacggaggaaatcgcccgcctgcgcgagaacctggatcaggtccggcgcgaggccatgaccgacgccctgacggacctcgccaatcgcaaggcctttgacgaacagctggcgcgcgcctgcgcccatgccgacgccaccggctcgccgctgacgctggccttgctcgacatcgaccacttcaagcggttcaacgacacctggggccatcagacgggcgaccaggtgctgcgctatgtcgccagcgtgttgtcgcgggtgtgcggcgagacccgcttcgccgcccggttcggcggcgaggagttcgccctgatctttccaggcgaggcgtccggcgcggtctcctgcgcgcttgaggtcatccgcaaggagatcgcctcccgctcgctgcgcaggcgctccaccaatgacgatctcggcgccgtcaccatctccggcggctttgccgagcgccaggcgggcgaaagcctgctggccctgatggagcgggccgacgccgccctgtatcgctccaagcgcacgggccggaacctgatcagcgccgccgagacccgggttcgcgcggcctgagaccacggcggtgcgaagcttcgccttcaacgccgcctactggatactgtcgatcggctacggcctggccgccgccttcgccgcgcttgcacccggtcgcgggccgaccggctgggtcatccggcggtatgtgaagcgcatggtgcaggccatgcgcctattcgccggcatccgcctgcacgtgctgggcaaggagcgtctgccgacgggcgccttcatcattgcttcaaagcatcagagctggggcgacggcttcgtcacctatgaccagttcgacgacctggcgttcgtcaccggcgaccacctggagaagtttccgctgctgggcggggtgctgaagaagctgggcgccatcgtggtcgcctcctgcggcgggcacgaggcccgcaaagcgctggcgacccgagccgcagagacgcgcgccgagaaccgcaggatcctgatctacccagagggccatctggcgcccgtcggcaagaaatatcgctaccgctcgggcgtctggcacatgtaccgcgacttcgacatgccggtcgtgccgctcgccaccaacctcggcctgtgctggccggaggagcggtacgaaaagcacccgggcacggccaccctcgacttcctcgagccgatcccgaccggactgcccagggacgagttcctgacccggctcgaaaccgccatcgagacccgcaccgccgaactggtggccgaggcgacgggccggcccgtcacgcccgccgagctcattcccacaccgggggaagcgccgaaggtctaggcgtccagcgccgccgccggcacgatggtgacgctctcgccgcagccgcaggcgtctgtctggttcggattgtttaacacgaacttggatgacaggcgcgaggtctcgtagtcgatctcggtgccgatcaggaacagcaccgcctttgggtcgatcaggacggtgacgcccttgtcctcgaccacctcgtccagcggcccggcggcctcggcgtaggcgaaggtgtattcctgccccgcgcagccgccgtttttcaccccgacccgcaggccgatgtagggcttgtcggcattgtccatgatctcgcgcacgcgctcggcggcggcgtccgtcagggtgacgaccttgggccgggggcgacgcgggcgggtggtggtctgaagctcggtcatggtcagaacatgttcagcgcgagcttggcttcgtcgctcattttcgaagggtcccacggcggatcgaacaccagattggcgtgggcggagcgcacgccctccaccttcatcaccgcatcctgcacccagcccggcatctcgccggccaccggacagccgggggcggtcagggtcatgtccaccaccacgtcgcgatcgtccgacacgtccacgcggtagatcagccccagctcatagatgtccaccgggatctccggatcgaacaccgtcttcagcgcctcgatcagatcgtcagtcagcttgtccaactcagcctgcgacagggcgcttttctgcggctcgttccacgcctcggcgaaggcgtcgctgtcggaaacgggggtttcggtcatggcttacacaaagaagttgcgcgccttgatcagcgcatcggcgaaggcgtctgcgtcctccagggtgttatatagggcgaaggacgcccgcgtgctcgacgtcacgccaaagcgctgcgccagcggctcgcagcagtgcagtccggcgcggaccgccacgccataccgatccatgatctgggccacgtcgtgcgagtgtgcgccctcgaccgcaaaggccaggatcgcgcccttgtccggcgcctcgcccagcgccctcagccaatcggcgtcggccagccgcgcacgggcgtgttcatacagcgcatcctcatgcgcccgcaccgccgcacggtcgaagcccatgaaccactcaagcgcagcccccaggccgatcgcctccaggatcggcggcgtgccggcctcgaagcgatgcggcggccgggcgtaggtgacgcggtcgcggctcaccgtctcgatcatctcgcccccgccttgatacggcggcagcgcctccagcgcctccgctgtcccgtacagcaccccgatcccagtcggcccatagagcttgtgcccggtcagcacatagtagtcgcagccgatcgcccgaacgtccggctgagcatgcaccccgccctggcagccgtcgatcagcacccgcgccccggccgcgtgcgccatctctgtgatccgctgcaccggattgatcgtgcccagcacattggacatgtgcgtgaccgacacgatccgcgtgcgctcgctcagcaggcccgcataggcctccatgtccagcgagccgtcgcccagaatcggtatccacttcagcaccgcgccccgccgctcgcgcagcaggtgccagggcacgatgttggagtggtgctccatctccgagatgaggatctcgtcgcccggctggatcgactgtccgacccccgacgccaccaggttgaccgcctctgtcccgcccttggtccagacgatgttggaggcggcctccgcgttcaggaaccgcgccgccgtctcccgcgccgcctcgaacgcctcggtggtctcattggccagagtgtgcaggccacggtgcacgttggcgtatgacccctccatcgcgcccaccatggcgtcgatcaccgcccgcggcttctgcgccgaggcggcgttgtccagataaaccagcggcctgccgttcaccgtccgcgacaggatcggaaactgcgcgcgcgcggcgtaggggtcgaagcgggtcagagtcgcgccgtcagccattcccgcaccacttcccgagcgccctcgtgcttgatccggtccaccacctcgatcaggaaggcctgcgtcagcagcgcctgggcctcgtccgccggaatgccgcgctgctgcatgtagaacagcgcgcgttcgtccagattgcccacagtgttgccgtgcgcgcactgcacgtcgtcggcgtagatgatcagctcgggcttggcgtcgatctcggcgcgttcggaggcgatcagcgcatggtggcccatccgcgagtccgtgtcgtcggctccgcgccgcaccacgatcttgccctggaacacgccgcgcccggtatcgcgcgccacgcccttggtcagctggctggtggctccgttcggcgcgacgtggtcggccaccgtggtcatgtccacgtgccgcgccccgttcagcagatagagcccgtccatccgcacctcggcgccctcgccgccatgcgtcagctgcgtctccagccgctggagacgggcgccggtcgccacgatcgtctggcgatagacgccgccggcctcgacccgcacccgggcctcggtgacggacatggcgtcctccggctcttcgaccaggacgatgcgcgtgacatcggcgccggacgcgacgtccagctccagccggttgtgcgccagataggccgagccctggccctcatggctctccagcagcagcagcttcgctccgggccgcgccgacacccgcgccgaggcggcatgcgccgttccggtcgcatccgagatgaagcgcaggcgcagcgtctgctcgccgcccgcgatgaaatccgtcaccccgaccggccgcccgttggcgaagacgatggcctctccgcccaggtcgtagaaaggtcccggtgcgcccacctgcgccgtgcccgacggcgccggcgcctcgcgcagcagccgcctcaggtcgctgtagcgccaagcctccacccgccgcgacggaaaggtcgaagcgtcgcggatgtcgagggccgccgtcatgcggccgccggcaggtacttgtcgtagccctccgcctccagttgcagcgccagctccggcccgcccgaagcgacgatgcggcccgccgccagcacatgcacccggtccggtttgatgtagtccagcagccgctgatagtgggtgatcaccaacatggctcgctccggcgagcgcagtgcgttcaccccctccgacacgatccgcagggcgtcgatgtcgaggccggaatcggtctcgtcgaggatcagcagcgacggctccaagagcgccatctgcaggatctccatccgcttcttctcgccgcccgaaaagccgacgttcagcggccgcttcagcatgtcgaaatccatgcgcaggcgcttggacgcttcgcgcaccagcttcaggaacgccggcgccgaaacctcgtcctcaccgcgcgcgcgcttctgcgcattcagcgccgtgcgcacgaacgtcagggccggcacgccggggatctcgatcggatactggaacgacaggaacacgcccttggcggcgcgctcggcaggctcaagctccagcaagtcctcgccgttccaggcgaccgatccgtccgtcgcctcatagcccggccgccccgacagggcgtagcccagcgtcgacttccccgccccgttcggccccatgaccgcgtgtacctctcccgccggcacttcgagcgtcagccccttcaagatcggcttgtcgccgacggagacgtggaggttgttgatgttcagcattgtttttcttgttctttaaccgacggagccttcgaggctgatcgccaccaacttctgcgcttcgaccgcaaattccatcggcagttcctgcagcacgtcgcgcacgaagccgttgaccagcagcgccaccgcctcttcctggctcaggccgcgctgctgggcgtagaacagctggtcgtcggacaggcgggtggtggtcgcctcgtgctccagctgggccgagccgttgcgcgcctcgacatagggcacggtgtgcgagccgcattccttgccgatcagcaggctgtcacactgggtgaagttgcgcacgttctcggccttggggtgcaccgacaccaggccgcgataggtcgaatccgaccggcccgccgacaccgccttggcgatgatgcgcgacttcgagttgcggcccaggtggatcatcttggtgccggtgtcggcctgctggcggccgttggtgatggcgatggagtagaactcgcccgagctctcctcgccgcgcagcacgcaggatggatacttccacgtcaccgccgagcccgtctccacctgcgtccaggacacctttgaccggtcgccccggcagtcggcgcgcttggtgacgaagttatagatgccgccgcggccttccgcatcgcccggataccagttctggacggtggagtatttcacctcggcgtcgtccagcgccacgatctcgaccaccgccgcatgcagctggttctcgtctcgcatcggcgcggtgcagccctcgaggtaggagacgtaggagcccttgtcggcgatgatcagcgtccgctcgaactggcccgtttgcgaggcgttgatgcggaaataggtcgacagctccatcggacagcgcacgcccggcgggatgtagacaaacgagccgtccgaaaacaccgcgctgttcagcgccgcgaagtagttgtccgacaccggcacgaccgatcccagatactggcgcaccagctcgggatgctcccgcagcgcctccgagatgggcatgaagatcacgccggccctggacagctcttccttgaaggtggtgaccacgctgacgctgtcgaacacggcgtccacggccacgcgcggcgcgccctccacacccgccagcaccgcctgctccttcagcgggatgcccagcttctcgtagacggccagcagttcgggatcgacctcgtcgaggctcttgggtccgtccttcttcttcggcgcggcgtagtaatacaggtcctgataatcgaccggcgcatagttcaccgccgcccaggtcggctcctccatcgccagccagcgctcataggcggccaggcgccattccagcatccattccggctcgcccttcttctcggagatgaagcgcacgatgtcggcgctcagccccttgggcgcgaactcctgctcgatgtccgaggtgaagccgtgcttgtagcgctccagctcggcgacggcgtcgatggtttcctgaacggcggccatgatttacgcgacttccttcacgcgctctgcctggcgcgtcctgtgcttgatataggcgcccgaccacgcatccgcgaaccggatccagtcgccctcgacggtgctccagccgccggagacgcgcaccgcgccgcgcgccaaggcgtccagccccatggctgcgatcgtcttggacggcgtcaccttgcccgacgaacaggccgaaccggccgagaccatgacgccggccagatccagggtgatcagctgctgcgggctgtcccagccctcgaccgccaggaacagggtgttgggcaggcgcggcgcgtcctcgccgatcaccaccgcgcccgccgccttgaccgcccgcgccgccgcatcgcgccaggcggcgtgcgccgacgcctgcgaaaggtcgcgcatcgcgcactcggccgccgcgccgaaaccggcgatcccggcgacgttctccgtccccgagcgcaggcctcgctcctgccccgcgccgtgaaggatgcgcacacccgcgcggccttgcttcagcaccaaagcgccgacgccctgcggcccgcccagcttgtgcgcggacagcgtcaggctgtctgcttccagttcgagcatgtccacggcgatcttgccggccgactggatcgcatcgacgtgcagccagccgcccgccgcccggaccagcgcggcggcctcggcgatcggctggatcacgccgctttcattgttcgcatggtggatggccaccgccgcacggcccggacgcgccagcgccgcctccagccacggcagatcgaccacgccgtccgcattcaccggcagcacctcgacggcgacgcccgcgttggcggccgtttcggccacgcaaggatgctcggtcgccgacacgatcagccgctcgcatccggcggcaagcgctgaggccacgccttgggcgttcgcctccgtcccgcccgagttgaacaccaccgcggtcggatcggcgccgaccaattcggccacctgcgcccgcgccgtctcgatccgcgcccgcgcgcgccgcccggccgcgtgcaccgccgacggattgccgttgtcggccagcgccctggccacggccgcctgcacctccggccgcgtcagggccgaggcgttgtaatccaggtaaaccccgctcacgccgccaccccgaccgcttcaggctccaggttcgcctcgcgtctccgcccagtgcggttcatcaccacatcctccagcgacacgccggccaggtagcgatggatctcctcgcccaagtcttcccacaggttgtgcgtgatgcagcgttcgcccgccagcatgcagcccttgggcgatccgtgggccacgcaccgggtcgcccggatcggctcgtccaccgccagcacgatctcggccaccaccgtctggtccgcgtccttggccagccgatagccgccgcccggcccgcgcacgctccgtaccaggccgctcttcctcagccgcgcgaacagctgctccagatagctcagcgaaatctcctgccgcgcggcgatctcggccagggacacggcgcgcgtctgcccgtcggcggcgcggccgttcttggccaggtcggccatcgccatcacggcgtatcgtcccttggtcgacagacgcatcgcgcacccatgaaaatccgcgcgctttccggggctcttgtgctagaacccgcgccctcgccagggtgtcggcgcgcaggggggacttagaaagtcccaccagcgtggtcaagtattccccgcaggcgaaacgacacttgaacggattccggaggcccgaatgcccgaagtcatcctgcccggcgcctccggccgcatcgaaggccgctattcgcccggcaagcggccgaacgcgcccatcgccctgatcctgcacccgcaccccaaggcgggcgggcacatgaacaatccggtcgcggtgaccctgcaccagctgttcgtgcagcgcggcttcgccaccctgcgctacaactcgcgcggcgtgggcaagtcgcagggcgagttcgattccggcatcggcgagctggcggacgccgccacggcgcttgactggctccaggccaacaatccgggcgccagccagacctgggtcgccggctaccagttcggcgcctacatcggcatgcagctgctgatgcgccggcccgagaccgacggcttcatctccgtctcgccgccttccaacatgtacgacttcagcttcctggcgccctgcccggcgtccggcctgttcctgcacggcacggccgacaccatcgtgccgccgatcgaggtcgaacgcgtggtcaacaagctgcgcagccagaagggcatcgtcatcgactacgagctggaggaaggcgccagccacttctggcaggaccacgtccccgccgtcgaccgtcgcgtcggcgcctacctcgacaagcgcctcgccgaaaagccggcctagcgagagccgcggccgagtggtatgtcctgaccaactaacaggtcaggaagccatggaccgcatcagcctgtcggacgctaaggcgaacctcagcgcgatcatcgatcgtgtggagaggggcgaacagatcgagatcatgcggcgcggaaagccggtcgccagactggctccgaccctggttgagccgaagtcgaagaagccgttcgactgggatgaacttgatcgtgtcgtcggccggatgactccgcagacggaaagcgccggcgacttcatgcgtcgtgtccgcgacagcggctactagtgttctacctcgatgcgtcggtcatcgtcgcggccgtgaccgacgaaccgcaccgtacggcggttctccagtggctgcgcgcgaaccaggacaagctcgtggtcagcagctggacgctgactgaagtcgcctcggcgctttccatcaaggtgcgggatctccgactgacggaaagcgacaaggatgcgggctggaggcaggtcgaggccatgcgaaacaccgtcctcatgcaaacggtcatcgaggaaccgcacttctacgccgccctgcgcttcgtcagccagcatcagaccggcctgcgcggcggcgacgctctgcacatcgccgtgacggcagactacgattgcgccttggtgacccttgatcgacgcatggcgaagggcgctcgcttgatcggcctggccgtagtggagctgccgaacccgcatcagtagatcagaaacggccggcgcgcctcttcccacgcccgctcgtcgggctgcgtcagcgcgtccagatcgcctggcgccgcctccccatcgtccacccactcccgcagcagcggcgagccgttgatgacgtcgacggccagcttgccgaaggcgtattcatagggaaagtcgcgccacaggtcgtagtccggatacagcccccggatcgccttgaacgccagcgcctgcaccctccacggccggaacgccgcagggtcataggccggtccctccacatgaatctgcacgcccgagcacagctgtcccacatgcttgtggaaggtcggctcgaaccagcaatcgcgcagcacgcagccgttcagccactccggggccagcgcgtgcatctgggcgatcaccgcccgcgcgtcgatgtccggcgcgccgaacagctccagcgggcgggtcgtgccgcgcccctccgacagggtggtcccctccagcatcaccgtgccggcgtatgcgcgcgccatcgacagattgggggcgttcggactgggattgacccacgtccgctccagcaacggccagccgaagccgggcccctcttcgggccgccagccgtccatggcgattacgcggtagtcgacgtccagcttgaagcggtcgatgaaccacaggcccagctcgcccagggtcaggccgtgacgcatcggcatgggtccggcgccgacgaagctctcccagcccggccgcagcgtcagcccctcgacgtgccggccagcgggattgggccgatccagcacccacaccgtcttgccatgctcggccgccgcctccagcacatatagaagcgtggtcacaaaggtgtagatgcggcaccccaggtcctgcaggtcgaccagcagcacgtcgaacgtgcccatccattgcccgcgcggccgccgcacctcgccatacaggctgaacaccgggatgccgtgcaccggatcggtgtagtccgggctctccatcatgttgtcctgcaggtcgcccttcatcccatgctgggggccgaagagcgccgtcagggtgatctccgggcagtccgccagcgcatccaccgcatgcgtcaggtccttggtcaccgacgccggatgcgccagcagggcgacgcgccgccccttcaactcggcccgaagcgcgggatcggacagcaggcgatcgaggccgaagttcataggaggtccagcacaaaggaatccggatgatggaagtccggcttatccgagggatgcctcagcgcccaataggaaatgcgcccgtccttccgcttgaccacggtcgacagcgccagcgcctccgcaccgggcgggagttcgatcagcccctccaacgcccataacgcctcgcccccatccatcccgaagacttccacgcgctcgcccgcctcggccatgccgctgcgatagccgtcgaagcggtaagacgcccactggccggacggcgacaggttaaactcgacgtagccgccgccggcggtgcgcacgaagacctcgaagcaggtgcgccgccacagatcgtctgtccggcccggcgcggccgcctcgggccacgccaccgcgtctacatcgccctccaggatgaaccgcagccagagccggtcgccacgccgctccacctcgaccgccagcgacagcccgtccgcgtcgccgaaagacttcagttcgtgcgtcaccccggcctccgccgccaagcctcccccttgaggcgacagccgtgctacacgccccttccccatcacgccaagcgcctcaagccgaccatgaccgaacacgccttcaagtcccccttcctccagaccatgcaggcgcgcggctatatccaccagatcacccatccggccgaattggacgcggcggcgtcggcgggcgtggtcaccggctacatcggcttcgacgccaccgcgccgtcgctgcacgtgggccacctgatccagatcatgctgctgcgccggcttcagcaggcggggcacaagccgatcgtcctgatgggcggcggcaccaccaaggtcggcgacccgtcattcaaggacacccagcgccccctgctgaccgaagaccgcatcgccgagaacatcgccggcatccggggcgtgttcgagaagttcctgcggttcggcgacggtccgagcgatgcgatcatgctcgacaacgacgaatggctgtcgaagctcggctatctagagttcctgcgcgattacggcacccatttcaccgtgaaccgcatgctgagcttcgactcggtcaagctgcggctcgagcgcgagcagccgctgacctttctcgaattcaactacatgctgatgcaggccaccgacttcctggagctgaaccgccgctacgggtgccagctgcagatgggcggctcggaccagtggggcaacatcgtcaacggtgtcgagctgacccgccgcgtcgatggcaaggccgccttcggcctcaccaccccgctgctgtccaccgcctcgggtcagaagatgggcaagaccgtcggcggcgccgtctggctcaacgccgacgccctgtcgccctatgactactggcagtactggaggaacaccgaggacggcgacgtcggccgcttcatgcgcctgttcaccgacctgtcggacgccgagatcgctcgcttcgagacgctggagggcgtcgcgatcaacgacgccaagaaggcgctggccgacgccgccaccaccatgctgcacggcgcggacgcggccgcccaggcgcgggcgacttcagaaaaggcattcgaacgcggagtagcgacgactgatctgcccactagggatctgctctgggcgggcacgccggaggaacagcaacgtaacagcgaccagccgttcgaactcagaacagccgaggcgcttcttagagcgtcagagctttcaccctcgctcggccaagcccgcaagaagattcagaacgagggtgtctggatcaacgatgaactcgttcgcgatccttcccaaaccttcgcgcgctcggacgctgatccggaactctcagcgttcaaggttcgcttgggcaagcgtggtcagatcgtgctggttaaacccatctaatccgctcatccccgcgaaggcggggaaccagaaaaggcgcacggacgatggccttcttcacctacatgctggccagccagcggaacggcacgctctacatcggatcaaccgaagacctgatccgccgcgtcgcccagcaccgcgccgggacctttggcgggttcaccgcccgtcacggcgtgcagttgctcgtctggtacgaagcccacgagacccgtgaatccgccttcctgcgcgagcggcgcataaagaagtggaaccgcccgtggaagctgcggctgatcgaggccgacaacccgacgtggcgtgatctgtacgacgagtttcgatttggcggcctcagtgatgcggcgtcctggatccccgccttcgcggggatgagcggaaaggaagcatgatgaaagcccccaccctcgatctgcccgccgacggcggcggccgcgtgtcgctgcaggcgctgaacggaccggccgtcgtctacttctatcccaaggacgacacggccggatgcacccgcgaggcgcaggatttcacagcccttgcgcctgagttcgccgcgctgggcgtcaccgtgatcggcgtgtcgaaggatacggtggccaagcacgagcggttcaaggccaagcatggtctggatgtcgtgcttgcgtcggatgaggacggtgcggcttgcgaggcttggggcgtctgggtcgaaaagacgctctacggccgcaaatacatggggatcgagcgcgccacctttctggtggacgccgacgggctgatccgccgcgcctggcgcaaggtgtcggtgaagggccatgcgcaggaggtgctggaggccgctcgcgcgctttgatccactgtcccggacgcccggccgcgttcgccgcttgcgcgaatcgtcgcctcaggggcgaagtcggtaaggttacgtcggctttcgtgtgaagctgccgtggcttgaacacccgtcgtgcggaggtcgccatgttcaacaagcccaaggccaagacgcccgtcgcttcgccggagaccacggccttgacggacgcgccccgccgtcagccgtcgcggatcggagtcgaccttcaggtgcgcggctcggtggtgggcgacggctggctgcagctcgaggggcagatcaagggcgacgtgcacgtcggccgcctgttcgtcgaggagacgggcgccgtcgagggcgccgtgtcggccgaggcggtcgaggtcggcggccgcatccaggggccgatcaccgcgcgcgaggtgcgggtggccgccaccggttacgtccagggcgacatcaccaccgagaagctgtcgatcgacagcggcgcctatttccagggtcgctgcacgcagatccagccgcaggtgaagccgatcctgccggaagcgcgcccggagccggcgcaggccgccgaaacgaattcgaagacgtccccgtcctcgtcgcccgtcgggagcttctcgaccgcgccggcggtctccgaaagccgccattagaagaatagggccggcgtcgccgccggccctcttgtttcactcgacggtggagccgcgcgtctcgccgacccgcgccgccagcgccgcgcccatgaactgatccaggtcgccgtccagcaccccttgcgtgtcggaggtctcgacctcggtccgcagatccttcaccatctgatacggctgcagcacataggaccggatctggtggccccagccgatgtcggtcttggcgtcggccaaagcctgggccgccgcctcgcgcttctgcagctccagctcgtacagccgcgcccgcagcatcttccaggcctgttcgcggttctggtgctgcgagcggccggcctggcaggccaccaccgtgttggtcgggacgtgcgtcagacgcacggccgaatcggtcttgttgatgtgctggccgcccgcgccggacgcacgataggtgtcggtgcgcacgtcggacggattgatgtcgatctcgatggcgtcgtccaccaccggcgacacgccgatcgaggcgaacgaggtgtgccgcttggccgccgcgtcataggggctgatgcgcaccagccggtgcacgcccgattcagacttcagccagccataggcgttcggccccgagatctggatcgtggccgacttgatgccggcctgttcgcccgattcttccgcctcgaccgtaacctcatagccgtgagcgcgggcccagcggctgtacatgcgcaacagcatgccggcccagtcattggactcggtgccgccagcgcccgagttcacttcgagataggcgtcgttgccgtccgcctcgcctgacagcagcgcctccagctcggcgcgcgccgcgcgttccttgatggctttcagctgggcgcgcgcgtcttccagagccgcctcgtcgccctcctcgtcggccatctcggccagcatgacgccgtcttcgacgccctgctccatctcccggacagtgttgatctgggcctcgagccgcgagcggtcgcggctgaccgcctgcgcctcgtccggcctgtcccacagggtcgggtcctcgacccgtgcgttcagctcatcgagctttcgaagcgcgacatcccagtcaaagacgcctcctgagcagagcgacgctctgctcgatgtcggccttcatggcctcgacatccggtctcatcgcaatctccatgcgacagcaaaaaaggaaaggcgcgccggtcggccggcgcgccttggtctgttctatctagagcctcagtagagcccgctcaagtcctcggccggctcgcgtttgggtggcggaggcgcgctcggcggcggcgcggacgtcgcggcttccgtctctcgccggatgacgtcgttgtagttctgaggtccctgcggttggaccggcgcccgcaccggggcgcggaccggcggcgcgcgccgctcggtgcccggccggaacgcctcctcgatgccgttcacaggccggaagatcgcgttcttgggccggacgaacggccgcgccggccgctccttcagcgcggtctgcatgaagtcgatgaacaccggcaccgccgccgtcgtgcccgtctcgccgttgcccagcggccggttgtcatcgaagccgatgaagacgccgacgacgatgtcagtggtgaagcccacgaaccaggccgagcggtattcgttggtcgtgcccgtcttgccgccgacccagcgaccgaggccgcgtgcgctcgccgccgtgccccgctgcaccacgccctccagcatggagctcatctgataggcggtgattgggtcgatcacctgggcgccgcgcggctcgagcttgggcgattcctgaccggagaagccgcgcccgcaatcgccgcaacgccgggcgtcggcgcggaagatggtctcgccgtcgcggtcctggacatagtcgatgaggtaaggcgtgatccgccgcccgccgttcacgaacgccgcataggctgccgtcagctgatacggcgtcacctcgcccgcgcccagcgacaccgacaggttcggcgtgaggccaggtatgcccatccgcgcggactggtcgacgatcttcttcatgccgacagcctgagccaggcggactgtcatgacgttgcgtgacagctccagcccccgccgcagcgtctgcggcccatagtattcgcggctgtagttctcgggcgtccagcgctggccgttcggtccgccggcaaagctgatcggcgcatccagcacgatcgaggccggcgtatagtcgccctccagggccgtcgcatagacgaacggcttgaacgccgaacccggctggcgctccgcctgggtcgcccggttgaagctggacagggcgtaggaatagccccccaccatcgccagcacgcgtcccgactgcggctcgatcgccaccatcgctccgttcacgcgcgggatctgcttcagcgcgtactgcccgcccgagcgctccacatggatcaggtcgccccgcttcagcggccggttggcgttggcccaggcggcgtccgcggccaggaggctgcccgaacgatccccacgcgcggttcggacgcgcacattgtttccgctgacgctctccacagccgccacttcccaagcccggcgctccggcggcgtcttctgctcgccgagcgcccttgcctgccaaccgtccccgaaatcggtcgtgccccaggcgccgcgccagccatggcgacggtcatagttctccagccccagcatcagagcggatcgcgccgccgtctgcagcgtcgggtccagcgtcgtgcgcatgtagaagccgccggccctcagctggtcgccgaagtcggggttggccgccgcctgccgccgcgcctcctccacaaagaagtccgcatcgcgataggccgcccgctgcggcgcgtcgcgcgtgttcagcggccgggcgcgcgcctgctgcagctccgcgcccgtgatccagccgctctgctccatctcgcccagcacccagtcgcgccgccccttggccgcgccgggatgccgcttgggatgatagttgttgggccccttgggcagggccgccaggaacgccgcctcgtccggcgtcagctgcgccagcgacttgccgaaatagttgtaggccgccgaggcgatgccgaacgagcgatatcccaggaaaatttcgttcagatacagctccaggatctgctccttggagagcgtcgcctccaggcggctggccagtatggcttccttcagcttgcggttcaggctgctttcgttggtcagcagcacgttcttggcgacctgctgggtgatggtggagccgccctccagccgccgcccgcgcgccaggttcgccacattcttcagcgaggcgcgcccgatgccgcccacgtcgatgccgccatgctggaagaagttgcggtcttcggcggccagaaaggcgtgccgcaccgtgtcggggatctggtcgtaggagacgtagatgcgccgctcgtccgagaactcgccgatcagggtgccgtcgccggcatagacccgcgtcgccgtgggcggccgatagtcggccagctccgatgcatccggcagatcgtagaacagccacgcggcgtagacggccaccaccagccccgccagcgcgaccgcgcccagcagagccatgcccgcccagacgaaccagcgttcggcaaccttcaccgccaactccgaaagacgcgccccgatcgcatgctttagcccgcgtcccccgccggacgccagagcgcgcgtgcaacgaccaccggggaatgtcgtttcgccctcacttcacccgggacgaaagcatcaaggatccgcacatggacgttctctacaccgctcgcgccaccgcatccggcggcggtcgcgaagacggccgcgccacgaccgacgacggcaagatcgacgtcaagctgtccaccccgaccgagatgggcggcaagggcggcgacgggaccaaccccgagcagctgttcgcctccggctatgcggcctgctacctcggcgcgcttcgcctcgtgtccggcaaggcgggatcgcccgtgggccccgacaccaaggtcacggccggcgtcggcttcggcaagaacacccggggcgaaggcttcaacctcgacgtcacgctcaccgtcaccgaccacgggctggaaaaggctgtaatcgacgacctgatcgagaaggcgcaccaggtctgcccctactccaacgccacccgcaacaacgtcgatgtgaagctcagcgccgaataagcgcctccagccccgcgcgcgtgttgagccgcgcgcgcggggtctctagatggatcgcatgacctcgacgctcgacgccctccccgatccgctgctgacgcttgaacccgctcgccgcgtcaccctgcgcgaagcctttggcgtcgacagcgacatgcaggttccggccttcgccgaacgcgacccgcatgtgcctgagatcgacgacagctatcggttcgatccgcagaccacgatcgccatctgctccggcttcgccttcgaccgtcgcgtcatggtgcagggctatcacggcaccggcaagtcgacccatatcgagcaggtcgccgcccgcctgaactggccgctggtccgcatcaatctcgacagccacgtcagccgcatcgacctggtcggcaaggacgccattgcgctacgcgaaggcaagcagatcacggagttccgcgaaggcatcctgccctggtcgctgcagcgccccatcgccttggtgttcgacgaatacgacgccggccgaccggacgtgatgttcgtgatccagcgcgtgctggagacgcaaggccggctgaccctgctggaccagaaccgcgtgatccggccgaaccgctggttccggctgttcgcgacgaccaacaccatcggcctgggcgacaccacgggcctgtaccacggcgcccagcagatcaaccaggcccagttggaccgctggagcgtggtcaccacgctgaactacctcgaccacgacgtagaggccgaaatcgtcgcggccaaggtcccggagatgaccgacgccgagggccgcagagccatcgccgccatggtccgcgtcgccgacatgacccgcaacgccttcatgaacggcgacatctccacggtcatgagcccccgcacggtgatcacctgggcccagaacgtccagatcttcggcgagatcggccaggccttccgcctgaccttcctgaacaagtgcgatgaactggaacgtcccaccatcgccgaattctaccagcgcgcctttggcgaagacctgcccgaagccgccacacgcgtgaaggtgggctgaccgcctgcgaaggcgaggatcaggctttttccgaaagccgcatgatcgccgccccccacaaggtccaggaccggccgagccctgtcagaaccaggcgtcctgcatcataagcggcgtgtcgtcccttgcatcgagcagatcaagcatgggaccggtcttgggcagttcccagcggaagaagtaacgggcggcctggcgcttgccgtcgtagaagtcgccggtctcgccctgggccgccagcgcctgttccagccagatccaggcgatcacggcatggccgaccgcttccagatagagcgaagcgttggccaaggcgcgttcggcgtcgccgtcgcgccagacgcttgccgtgacctggccgatgcgggcgacggtggccgccagtgcgtccgcgtagccggacagatcaggcgtcacgcgcgcgcggtccgtggtggcgaggatcgtttcagccagcagcctcagccccgctcctccatccatgatcgccttgcggccaagcaggtccatgccctgtacgccgtgcgtgccttcgtggatcgggttcaggcggttgtcgcgatagaactgctccaccggatagtcgcgcgtatagccgtatccgccgagcacctggatcgccaggctgttggcctccaggcaccattgcgacggccagctcttggcgatgggggtcagcatgtccagcaggcgcgtggcgcgcgttcggtcggcctcgttctcggccgtctgctgctcgtcggtcaggcgggcgcagtaaaggttcagcgccagcgcgcctcctgcataggccttctgcgccagcagcatgcgtcgcacgtcggcgtgctcgatgatcggcacgggcgggctggccgcgtccttggctccgagcctgcggccctgtggccgggagcgagcatagtcgagcgcatgcagatagccggtgtagcccagagccgccgcgcccgcaccgacgccgatccgggcctcgttcatcatgtggaacatggcggtcaggccctggtgggcctcgcccaccagccaggccttggcgcccgcctcgccttcggggcgatgcctgccctcgccgaagttcagcagggtgttggtcgcgccgcgatagcccatcttgtggttcaggcccgcgagcacgacgtcgttgcgctcggcgggcgcgcccccgtggtccagcaggtgcttgggtgcgacgaacagggagatgcccttcacccccgccggcgcgccgtcgatccgcgccagcaccatatggacgatcgtttcggacaactcgtgatcgcccgccgaaatccacatcttggagccgaacagccgataggagccgtcggcctggggcgcggcgcgcgtgcggatgtctcccagcgacgatccggcctggggctcggacaggcacatggtgccgaagaagcggccctccagcatcggccgcacataggcttcgatctgttgaggcgagccgtgagcccgcaacaggttggccgcgccgatcgtcagaaaagggtaggcggaaaacgcgatgttggccgcctggaaccaggcgaacgccgcgcgctccaccacgttcggcagttgcaggccgccgagctcgtagtcctgcgaggccgagaacagtcccgcatcgcgaaacgcggccatcgcctgggcgacctccgggatcaaccggacgcgctcgccgtcaaagatcggctcgttcagatcagccttgcggttgactggcgcgaaatgttcagccgcgatgcgcgcacaggtgtccagcacgccgtcgaaggcggcgcggtcgtggtcggcgaagcgatcgcgcgtcgtcaaccgctccacgtccagccattcatagagcaggaaatgcaggtcacgccgggacaggatcagggatgcgtcggagccactcatagccaaaggcgtatcaccccacgcctgtctgtatagatcaccttgcggaaggcttgcgcgtccgcggcgcaagggggctgtgaatccttttcggatactggaaccttggcctcagcttcgcgcttgccgatcatgagcaagtggatagacgccgtctcgcttcacctgtgccggcgatggaccgcacacgtccggggcggcttcaagcgccgcatcggctgaagctttgtccgtctcctagcggatcacgcccgcaacgacggcgatgacgatcatcatcacgatgatgatggcgaacaggccgatcatgatgcgggcggagcccttgctggctctatccttgggatcgcctgagttggggtcggttggcgccatgctgttgaaatgcgacccgaggcggttcgttgcggacgcgtgacgattcgggatcggcgtcgttcgcacggacgatccggaacggcccgaaagaatcgacggcgtcgatgttgcgttccatcacaatggaacgcatctagcgtgcatgaccgccgcctcgcccgatctcgccgtcgtctatgaacacccgcagtggttcgagccgctgttcgccgccctggcgcggcgcggcgtcgactttgctcggacgccgctcgccggccacagcttcgaccccgccggatccccgccgccggcgccggtgacgctaagccgcgtagccatgtcgtcctttctgcgtgagccggaacatccgatcttctacgcccagagcctgttcgcgcactgggaggctcagggcggacgcgtcgtcaacgcctccgccctgccggtcgacacctcgaaggcccggcagttgtcgctgatcagcagcctgggcctggccattcccgcgacgcgcgtggtgcaccgccgcgccgatctcgtccgggcggcggaaggcctgcgctatcccgtgctggtcaaggccgatatcggcggttccggcgcgggcatcgtccgctacgacacctcggaagagttggccgaggctgcgcgcgccggctcaacgccggtcggcgtcaacggcgtgtccctgatccaggaatacaccccccggcgcggcgacaggatcacgcgtgtcgaggtcatgaacggccgcatcctctacgccatggaggtggagagccccggcgacaccttcgacctgtgcccggcggacgcctgtcttgtgcggcccggcgcggcggccttgaccatgacgcggatcgagccggacgtcgatctggcgcgcgccgtcctggcgatcgcacgagaggcgaagatggagatcggctcggtcgagtgtctgatcgacgaccgcgatggaacccgccgcttcttcgacatcaacgccctgtccaacttcgtggccaagccgatggaggtgctgggcttcgacccgcacgacgatgtggtcgattggctgctgcaactggtttccgagagaaaggcggcggcatgaggtacggttactgggcgcccgttttcggcggctggctgcgcaatgtcgccgacgagcgggaggcgagctgggagaacctgtcgcggctggtccggcgctcggaggagacgggctgggacctgacgctgatcgccgagctgaacctcaacgacatcaaggggatcgaagcgccggcgctggacgcctggtcgtcggccgcggcgttggtggcggtcacctcgcgcatcgagctgatgacggcggttcggccgaacttccaccagccggccctgttcgctaaacaggccgccaacatcgaccgcatcagcggcgggcgtctggcgctgaacgttgtctcctcctggtggggcaaggaggccgaaagctatggcctgcagttcgaccagcacgacgaccgctacgcgcgcaccaccgaatggctgcaggtgctgaacagcctgtggagccggtcgcgcaccgacttccaggggcgctactatacgctggcggacgccatcgtggagccgaagcccgtgtccaccccggttcgcccgcgcccggtgatctacgccggcggagagtcggaggcggccaagaccatgatcgcccgccactgcgacgcctatgtcatgcatggcgacgagcccgagcacatcgcgcccaagatcaccgacatgaaggcgcggcgcgaggcgttcggcctgccgccgatgaagttcggcatggccggcttcgccatcgtgcgcgacagccaggcagaggcagagcgcgagttggaacggatcaccaccattccggggctggctgagggcaagccgccgtcgggcttcgccaacttcgaccaatggctggccggcaccgaactggagcgcgagctgaagatccgggagtattccgtctccaaccgcggcctgcgccccggcttcgtcgggacgccggagacggtgcgcgcgcgcatcgaggcgttcgaagccgtcggcctcgatctcgtcctgctgcagatgtcgccacaggaagaagaaatggaccggttcgcggcccaggtgatccagccgacgcgccccgccggctgacgcagcgcggtctagctgggctggaccttggtcttggccgacggcggcgacccgatgtggggccggccgcgcttgcgcgccaactccatctgccgctgtcgctcggcatagccggcgcgccgatcctcgtcgcgggttccatgacaacgatcacagcagacgccctccaagtagttgggcgatgcgcgccccgcctcgctgacgggcatgcggcagccgcggcacagcgtgtgggttcccggagtcaggttgtgaccgaccgcgacccgctcgtcgaaaacaaagcattcgccttcccacaggctgtccgcctgcggaaccgtctcgaggtatcgcagcacgccgccatgcaggtgatggacgtcggtgacgccttccgccttcagaaaggcggtggacttctcgcagcggatgccgccggtgcagtacatggcgaccttgaccggaccgcgtcgatccatcagcgccctgccctcgttgcgccaccagtcgggaaagtcgcgaaagccgcgcgtgttcggctgcaccgcgccccggaaggcgcccaccgcgccttcgtagtcgttgcgcgtgtcgatcacgagggtgtccgggtccgcgatcagggcgttccagtcctcgggcgcgacataggtccccgcgttttgtgcgggatcaaggtccggctgtcccatggtgacgatctcgggcttgatcttgaccttgagccgatgaaacggcggctcgtccgcccaggcgaacttcacttcaagatcgtcaaagcccggcaaggcgcggatcagcgcgatcaggctcgagacggcttcaggcgcacccgcaatcgtgccgttcaggccctcgcgtgcgaccagcagcgtgcctcgaacacccccctcgtcgcacgcctgaaacaggcgcgcgcgcagggcctcgcagtcttcaacccgggcgaagcgataaagggcggcgatgcggatagggccgcgtggcgggatcggctcagacgacatgccgagcggtatagggggcgctcgcggccttcaccacttcgggaggtgacgccgcgcaaaagaagagcccgacgcgggacgccgggccttgatcagttcggtgatggtgggtgtcctcgaaccgaagacgatccatccatgaagacgcttggttagcggacggttaacgcagggaatctggaagccaggtcgtctgacgaccgccatgcggcgcgctccagcccacgcgccagccgtcgccggccctctcgaccctgaacggttcggtcgcgttcgcatcgcccggatagccgtaggactgattcccgaccgtgatccggcgcggcccggaccccctcggcgcgtcgatccgccagatggggcctgctcggcccggatcgggcagcgcctcgccgtcaagagacagcgagggtgcgcgtccgtccgaaagcggccccgacaggatcatgaccgcgccatccgtatcgacggctcccaggggtccggagcgatccaggcggatgctggcctcgcccgccaacagaacggcgatggggccgcgaccgccgtccaggaccagaaggcgctcgggcgccgccgccgtctcctccccggtctgcacggccaggctgaacagcgccgcggccgcaggcgtcggcgtcgtcagttcaaatcgcccgccggcgtccgccgacaccgcctgggcgttcccgagggcgtcacgcagaaccacccgggcttcggctccggcctgtcctcggatcaacaggcccgacgaagtcgcctcgaccgattggatgcgcggcggctgagaccagccggcgggtgcgtcctgcgccttgcccttgatctcctgtggggcgggggaacaccccgcaagcgccgccgcgagaaccgcaagggagacagcaatccgccgtttcatcctgtccttcatcgatatatggctgtgcgcccggcgaggcgccgacggcgcggcttctggttagctggcgccctgcgacttgaccaacgatttagcgccgcatcaccgacctcgaggccccatgaccctgccccccgtcaccatcgcgccttttgagggccgttccgtctgcctgttctgcggcgcgtccgacggaaacgaccccgcctttgtccaggcggcggcgttggtgggccgggcgtcggccgaacagggctggcggctggtctatggcggggcggcgtggggctgatgggggctgcggcgcgcgcggcgcatgaggccggcgggcgcgttctcgggatcatgcccgcctttctgcgcagccgcgagcggctgttcgacgaggtggagacggtggtcgtcacctccatgcacgaacgcaagcagctgatgtacgaccagtcggacgcctttatcgtggcgcccgggggcgtcggcacgctggaggaggtggtcgagttgctgtcgtggaagcggctggacctgcaccacaagccggtggtgttcctgaacctcggcggcttctggaacggcttcttcgacctgatccgccacagcgtggcgcagggcctgactccggccgcgtttctggacgcctggacggtcgccgacaccgtccaggaggcgatcgatcaggcgagcgccgaggccgatctgaccacctacgacccgcgctgaggcgtcaggcggcttcgccctgaagccgccgcgccatggtctcgcgaccgatcagcggcgccatcgccgccatgtccgggccgtgaggctgtccggtcagggcgaggcgcagcggcatgaacagcgccttgcccttggcgccggtctccgccttgatcgcggccgtccaggtggaccagacgttctggtcgacggtgtcgggcagcagccgcagggccgtggcgatgaagtcggcgtcctcgatgacgggtgcgaccggcccgcgcacgatccgggccatctcggcgacgtcgtccatcttggcgaggtttggccgcacggcgtcccagaccgcctccccaagatctgcgcccgcagcggccaggcgcggttgcgcctgttcataggacagggcgtgcagcgcctgggcgttcagacgatccagatcggcggtgtcgtagcgggcgggcgaccgccccatcttggagaaggcgaaggtctgtcccagcgcctcgaccgacggcgcgatctccagcgggtccgaggtcccgatgcggcccagatggctggtgatggctatgggctcgtagccctggtcgcgcatgtcgctgatggacagggagcccagccgcttggacagggtctgaccgtcggcgcccaccagcagcggcatgtgggcgaagcccggcagcgtcccgccccagccggcggcgatcagggcctcgaaaatctcgatctgggcccccgtgttggtgacgtggtcctcgccgcggatcacatgggtgatcgccatgtccagatcgtcgaccaccgacggcagggtgtagagaaacaggccgtcctcgcggatcagcacgggatcggacatggaggcggtgtccacctcggcatggccgcgcgacaggtcctcccaggcgacgcgacggccatccagcttgaaacgccagtgcgggcgccggccttcggcctcataggcggccttctgctcggccgtcagttccactgcggcgcggtcatagatgggcggcaggccgcgcgacagctgcaccttgcggcggcgatccagttcctccgctgtctcataggccgggtagaggcgtccggccgccttcagcgcttcggcggcggcctcgtagcggtcaaagcgcctggactgattgtgccgctcgtcccagacgaggcccagccagcacaggtcgtcctcgatcccctgctcgaactcgggcgtcgagcgcgccagatcggtgtcgtcgatccgcagcacgaactgcccgccctgccccttggcgaacagccagttgaccaacgccgtgcggacattgccgacgtgcagcctacccgtcggcgacggggcgaaacggaccttgacggacatgggagagagacctcgaaagcgaggcggctaggtcgcgcccccgccagccggagtcaaggcgcgcggttggccgcacagaggatcatgataggctggcagacatcatgaacgctcctgtgcagatcagaaagccggatgtcgccgagcggcttcgcaacatggccctgcgcgagggattgtccattaccgagctcgtcgatcagatggcgcgcgaacgcgaagcccggccggacgaggcgcggcgggccgaaatcgagaggaagatcgccgccgtgaacgagatcgtgagagagttcaacgccctgccggttctgggccctctgctcaccgacgacgacatctatgatgaggacggactccccaaatgaccgtggcggtagatgcctccgccttggtcgccattcttctggacgagccggaaaaatcccctttcgtgaggcggatgctggctggcgactgcgaaatgtcgctcgttggatactgggagaccgctatcagggcgcggcagttgcatggcgaggatggcgtggcccggctggaccggctgattgcggagttgggcatccgcattgcgccggcttccgcaacgaccgctcgcctcgcgagcgatgcggaacggcaatacggcaagcgtacccccgccaagctgaatctcggcgactgcttcgcctatgcgctcgcgcgcgaacaaggcgcgcccctgctcttcgtgggcgacgacttcgcccggaccgatatagagccggcgctgaagacttgatcagtcgtcgcggtgcacgcgttcgcggcgttcgtgccgttcctgcgcctcgaccgagagggtcgccgtcggccgcgcctcgagacgccccaggctgatcggctcgcccgtatcctcgcagtagccgtaggagccgtcctcgatccggcgcagcgcgtcgtcgatcttggagatcagcttgcgctggcggtcgcgggtccgcagctcgagcgcccgatcgctctcggacgaggcgcgatccaccaggtccgggtggttctcggtctcggccttcagattgatgacggtgccccggctttcgcgaaggatctcgtccttccacgacagcagctttcccttgaagtaggccaactgccgctcgctcatgaacggttcgtcgtcggacggcctgtatgcggccggctccgccgtaatcctggacgccaatgcgttcatcgcactcacgctctcaatgcacgccccccatggcgtaagcgccgtataggagcgtgcgcgaggctcggcaacgacttcgcgtttccgtgatcgacgatcaggaaagaggcgtccgcctgcgtgacatttcgccctcactcgaaagggttgttgcttgaaaaagcgtcactttggcgctcaggcggcggcccgccgcatctcggccttcgccagctcgaccgacgcgcgcagatcgatctgatccaggagttcgctgagacccgcctcgcgctcttccggccggtcctctctcaacccacgcgccagccgctccagtgtcccctggccttcgtcgcctgagagcagcgcgagcttcagctcgtccagcctgtccagcagccccccgccccgccggatcgcgcgccgccgtcgctccgtgaccgtttcgacgccctgaagcgccatcagcgccgacacatcggccacgtttgtcgcagccgaggtggcggacgccgcagcagtcgatgtcgcctgagacgccccgccggagccggcgacgctgaaaccgccggcatgcgggcgcgccgccgccgggccgtgggcgctacggggtccggtcgatcctgtgatcttcatcgcggcatgctcccgaccatggagcgactaagccgcgcacccgtcaccttttggttaatggatcggcaaaacttgccgcctgatcgctgagcgaaatagcctccgccttgaacccgtttagcttttcccccggcacgatcctcgcaagagccccggcgctagtttcgacggagccgacccatgcagaaattgctggccagactgatcgtccctttcgccgcagggctggccctgtttggcgcaggccaggcggcgcaggcgcagtcgcgcatcaaggacatcgccgccgtcgagggcgtgcgcaccaaccagctggtgggctacggtctggtcgtcggcctgaacggcacgggcgactccttgcgcaactctcccttcacacgccaatcgctggaagggatgatggagcggctgggcgtcaacatccgcgacgccaacgccaacaccaagaacctggcggcggtgatggtgacggcggagctgccggccttcgccacgccgggatcgcgccttgacgtgtcggtctcgaccatgggcgacgccaagagcctcctgggcggcacgctgctggtcacgggactgcagggcgctgacggccagatctatgcggtggcgcaaggctcggtgcagacgggtgcggtgtccgcctccggcgcctccggctcgtccatcacccggggcgtgcccacggccggccgcatcgcctcgggcggcgtggtcgagcgggagacgggctttgagctcgccaacatgaacgaggttcggctgaacctgcgcaatcccgacttcaccaccgcccagcgcgtcgcggccgccatcaacgccgcctatccgaacaccgccctggctgaaaacggcacggtcgtggcgctgcgggcgcccggcgacatgggtctggccggcttcatctcgcgggtcgagaacctgccggtgcgggtcgacacgccggccaaggtggtgatcgacgaggtcaacggcgtcatagtcatgggcgaggcggtgcgggtgtccactgtggcgatcgcccaaggcaacctgaccgtctcggtccaggaaaccccgcaggtgatccagcccgcccccttcagccagggccagaccgccgtcgttcccgatacgcaggtcgcggtggaggaagagctcggacgcgagatgcgaatcgtgcggggcggcgagagcctctccacggtcgtcaacggcctgaatgccctgggcgtcagcccgcgcgacatgatctccatcctgcaggccatcaaggccgccggcgcccttcaggccgacatcgaggtgatgtgagaatgagcgacctgtcgatgtccgccgaatggctccgcacggcgcccccgcagccgtccggcgccgccgccaaggtgcgcgagaccgccgaggcgttcgaagcgagcttcctcgcccagatgctgaagccgatgttcgaggggctgaagaccgacggccctttcggtgggggtcaggcggaggcgacgtggcgcggcttcatgctggacgagatggcgaagaagaccgtggccgccggcggagtcggcctggccgacacggtcatggccgagatgctgaagatgcaggagcagcgtgcatgacgtccgacatcgaactcgccgcccaacgcattcgccagctggtcgacctcacgaaagctctgaccgcgcgcctcgccgaagaaactcgcgccttcgaagcccagcgcccgcaggacgccgccgccagcctgccgaagacgcaggagctggccaacctttatcggcgcgacagcgcccatgtgaaggcgaatccggcgttgatcgcctccgcgcccgccgccgacaaggctgccctgctgaaggcgacggaggcgttcgagaccgtgctggctcggcacagtcgcgcggtcgatgcggcgcgcaggatttcggaaggcctgatgcaggcgatcgcgcaggaagtggcggcggcgcgtactcccgcctcggcttacggggccggcggccaagccaacgctggtgacggacgcgccttcgctctgaaccgcacggcatagccgacgcgcccgcctcggatatgcgtcaaccacgcaagcgtcgctgtttcttaaggataaccgggcaaggtgagcctcatgaacctcaccgtccgccttctgggtctggctttcgcgtcgtctgacggcctcgcggaggtcgacaaggacggcgtggtccgcttcgcgatgggcgccgggccgatggcccgtcaggacgcggccgccgtgtggcagaaccgccccttcgccgaactgcttcatgacccggccgcctactatcgcctgatcgcgggcctgacgcccggcctgcgatccaagccggtcgaagttctggtcaactgctcggaacagcgggttcggcgcgcaacggtgcgcgctttcatgctgccgcagctggcgccggccgtgtcgctgtccatcagctatgaaggttcggccttcgccgccgccgatcttgaggcgccgcccatgttggacgctgaaggcttcctagcgtccgccggccgcatgctggtgaacggtcgagagcatggcgacacgcctgtgtcgctggtgtttctggacgttcacggcctcgcggccgccgacgccggcgccgccgaacggatcgcacgtcgaattcaggccaccttgcagtccgggtcgatcgacggttcggccgcagcgcagctgacccacgaacgcttcgccctgatccgatcgtccggcgacacacgcgatctggccgccgaggtgcgcgaggccggcaaggccgaaggcgtggtcctggacaccgccgcgacggacgccgccattcccgtgggcgccgagcctctttgcgcgctacgggcgatgcgtttcgcgatcgagggctgcctgaaggaaggcgggctcgccaaccctgaactggccttttccgagtcgctgaaacgcacgctgagggacgccgagaccttccggaccgtggtcaagcagcgggatttcgccgttcactaccagcccatcgtcgatctgaactcgcgcgccgttcaccacttcgaggccctcgcacgtttcaacagcgacgtgggccccgccagcgccatccgcatggccgaggaactggccctgatcgagcagttcgacctggtcgtcgcggaaaaggtcgtgcagcgcctgcgccagcccggagccggcctgctgaagatcgcggtcaacgtctcggcggcgtccctggcgaacgacgcctatgtggcctcgctgctgcggatgaccaacggctttcccgaagatcgccgtcgcctgatgatcgaggtcaccgagaccgccgccatggcggacgtcgaggccgccaaccggcgtctggccgtgctgcgcgaggccggcgtgcgcgtctgcatcgacgacttcggcgcgggctctgcgacctttgactacctgcgccggctgtcggtcgacgcggtcaagatcgacggctcgctggtccgcgacatccaaaaggacgatcgcgcgcgcacgctgatccgctcgctggtcgagctgtgcggctcgatgaagctcagtacgatcgccgagatgatcgaaacggagggaggcgcaaccgagctgaaggcggtcggcgtcaacatgggtcagggatggttgttcggccgggccgaggccgagccccgcacgaccctgtcatctcccggctccatccgccggcggggcaccgtggaggcatggggctgaccggtcagccgcgcggacgacgatgcgcccgggcgcggaccggcgcgcgcttcggctgaacccctcgtgcggcgaggagcagggcggagagagccaaaccggccgccattgcgctgatcatgatgctcgatcctccaagccgtgttggtcgagaacagaggatgggcgtcgcaagttcccgacgcaagggccggcttccgcccgcgatgtgacccggctggctgacgagacgccaggcgcagcgttgacgcgcgccgcaatgttcgcacattgttcttgctgaatgcggcggattagtccccatataccgctgtcgctccggagccgccggggtctcctccgcgttctcgacaggcatgaccgaaaagcacaacttcatccgcgttcgcggcgcccgcgagcacaacctcaaaggcgtggacgtcgacattccgcgcgagcagctggtggtgatgacgggcctgtcggggtcgggcaagtcatcgctggcgttcgacaccatctacgccgaagggcagcgccgctacgtcgagagcctgtcggcctatgcgcgccagttcctggagctgatgggcaagccggacgtggacctgatcgagggcctgtcgccggctatctcgatcgagcagaagacgacatccaagaacccgcgttcgaccgtcggcaccgtcacggagatccatgactacatgcgcctgctctgggcgcgcgtgggcgtgccctactcgcctgtcaccggcctgccgatcgaaagccagacgatcagccagatggtggacaagctgacggcgctgccggacggggagcgcatcctgctgctggcgcccgtggtgcgaggccgcaagggcgagtaccgcaaggagctggccgagtggcagcgcgcgggcttccagcgggtcaagatcgacggcgagttctatgcggtcgaggacgcgcccacgctggacaagaagttcaagcacgacatcgacatcgtggtggaccgcatcgtcaccaagacggggcttgagggtcgctacgccgacagcctgcagaccgcgctgggcctggcggacggaatcgccaccgccgaatgggcgagcgccgcagaaggcgaagagccgcgccgcatcgtcttctccgagaagttcgcctgcccggtgtccggcttcaccatcagcgagatcgagccgcggctgttctcgttcaacaatcccttcggggcctgcccggtttgcgacgggctgggggtcaagctggcgttcgacgccgacctggtgatccccgaccgcgacaagcccctgcacaagggcgcggtgtcgccctgggccaagggtccgtcgccactttacccccagacgctgcaggcgctgagccgccactacggcttctcgatggacaagccctggcgcgacctgccggaacaggcgcgcagcgtgatcctgcacggcaccaagtcggagaaggtcacgttctcctatgacgacaatgcgcggaagtatgaggtctccaagccgttcgagggcgttttgcccaacttggagcgacgctggcgcgagaccgacagcgcctgggtgcgcgaggagctgggccgctatcagtccgagacgccgtgcgaggcctgtcacggcaagcggctgaagcccgaggcgctggcggtcaaggtggccggagaagacatcgccgacatctccaacctgtcgatccccaaggcctatctgtggttcccgacggtcgaggagcagctgacggacaagcagcgcgacatcgcccgccgcatcctgaaggaaatcaccgaccgcctgcggttcctgaacaacgtcgggctggactatttgaatctgtcccggtcgtccggcaccctgtcagggggcgaaagccggcgcatccggttggcgtcgcagatcggctcagggctgaccggggtgctgtatgtgctggacgagccctcgatcggcctgcaccagcgcgacaacacccgcctgctggaaagcctgaaaggcctgcgcgacctcggcaactcggtgctggtggtcgaacatgacgaggaggcgatcctgaccgccgactacgtcatcgacatgggcccggccgccggcgtccacggcggcgagatccgggcccagggcacgcccgatcaggtcatggccaatccggacagcctgacggggcagtacctgaccggcgcgcgggagatcgccctgccccaggacggccgccgcccgatcaaccgcaagaagatgctgaagatctcaggcgcgaccggcaacaatctgaagagcgtcaccggcgagatcccggtcggcgtcttcacctgcgtgaccggcgtgtccggcggcggcaagtcgactttcacaatcgagacgctctacaaggcggccgcccgtcgcctgaacaatgcgtccgaagcgcccgcgccgttcgaccggatcgagggcctggagcatttcgacaaggtcatcgacatcgaccagtcgccgatcgggcgcacgccgcgctcgaacccggcgacctatacgggcgccttcgggccgatccgcgactggttcgccggcctgccggagtccaaggcgcgcggctatggccccggccgcttctccttcaacgtcaagggcgggcgctgcgaggcgtgccagggcgacggcgtcatcaagatcgagatgcacttcctgccggacgtctacgtcacctgcgacgtctgcaagggcaagcgctacaaccgcgagacgctggagatcgtgttcaagggcaagtcgatctcggacgtgctggacatgacggtcgaggaggcggccaacttcttcaaggccgtgccgccgatccgcgacaagatgctgacgctggagcgcgtgggcctgggctacgtcaaggtcggccagccggcgacgacgctgtcgggcggcgaggcgcagcgggtcaagctgtccaaggagctgtcgaagcgcgcaaccgggcgcaccctctacatcctggacgaacccaccaccggcctgcacttcgaggacacgcgcaagctgctggaggtgctgcaggagttggtcgaggccggcaacaccatcgtggtgatcgagcacaacctcgatgtcatcaaggtcgccgaccacctgctggacttcggaccggaaggcggcgacggcggcggcgagatcgtcgcggtcggcacgcccgagcaggtcgccgacaaccccgccagctggaccggccgctacctcaaggaggtgctggaccggcacgagcagcggcgcgtggcccgcgtgtccgagctttcggccgccgccccagtgaagtcgccgcgcacccgagccaggaagacggccgcggcctgacggtcaggtggaggcgaccacctgacccgacgcctgatgagccgccctgacccttcgctaggcgggtcgcatatcgcgccacgccgcagcgaagggcgcatagatggcgaccatctgcagcgtggacaggatgctgttgaccacgatccacgtcgcgatggcgggccctgcagtcgagagcatctcaccgaaagacgcgccttccatcgacgtgagcgtctgcatcccgcccgtcgccagcgtcagcggcagggcgacgatgccgccaagcagccccaccactatgctcatgatgacggcgatcaccgccatcccgagcagcggccagaacacgcccttggtcgcccgccacgactccttgaaggccatgcgcttttcggtgaacgtcgccggaaccaccaggctgaaccggatcgccagaaagaccaccagcgccagaacggctgcgcccgccagcaagccgacaagccaggcgacagcctgtcctgcaagcgaggccaccccgaccagcagacccgcggcgaacgccgccagcagcgtgatcgccgcgcccgccagcgtcagcagcagcgttgcaccgagcacccggaactcatccgcgctcaggcgcagataacccaggcgcccctcctccgggcggagcacggcgcgcacgatcgcggtgttcagcacggcgccgaacagaaggcccgccggcaacagccacgccagtcccgcgtacgccgccccgagcctctgcatgtccgcaggcgaaggattgaccgcattcatggtatcggcgatcgtcatcacctcgatcaggcttggcccggccagggcgaatgcgacggcgaacagcacgaggtaggccagcgcccaccaggccacgaccgtcggcttgcgccgcacgactctgaacccctcgaacgcggcttcggtggcggacaggctcatgcccaggctcccctgcattggactcgccagaacgatagccgcagtcgccggttcaaagccatagcgtcgccgcgcaagaaggctgacggcgcgggccgggctcgctagaaggccgcgatgaccgatatcgcttcctcgacccgccccgttcacgtcataggcggcggcctggccggctccgaagccgcctggcagatcgcctcggccggcgtgccggtgcggctgcacgagatgcggcgggacggcgtcaccaccgacgcccaccagacggacggcctggcggagctggtgtgctccaactcgttccgttcggatgactggcagttcaatgcggtcgggctgctgcacgccgagatgcgggcgctggattcggtgatcatgtcggcggccgacgccaaccaggtgccggcgggcggcgccctagccgtggaccgcgagggcttttcgcaggcggtgacggagcggctggaggcgcatccgctgatcacgatcgtgcgcgaggagatcgcgggcctgccgcccgaggactgggagaacgtggtggtggcgacgggcccgctgacctcgcccgccctggcccaggcgatcctgaatgcgacgggcgaggagtccttgagcttcttcgacgccatcgcgccgatcgtccatgccgacagcatcgacttcgacatcgcctggcgtcagtcgcgctatgacaaggaggggccgggcggagacgccgccgcctatgtcaactgcccgatggaccggaatcagtacgaggcctttatcgacgccctgctccatggccccaaggccgagttcaaggcgtgggagcacgtcccctatttcgacggctgcttgcctatcgaggtgatggccgagcgcggacgcgagactctgcgccacgggccgatgaagccggtcggcctgaccaatccgcgcaaccctaccgtcaaggcgcacgccatcgtgcaactgcgccaggacaatgcgctgggcaccctgttcaacatggtcggcttccagaccaagctgaagcacggcgcgcaggcggacgtgttccgcatgatcccaggcttgcagaacgcgcagttcgcgcggctgggcgggctgcaccgcaacaccttcctgaactcgcccaggctgctggaccggcagctgaggctgaagagccatccgcgcctgcgcttcgccggacaggtgacgggggtcgagggctatgtggagagcgccgcgaccgggctgctggccggaaggctggccgccgcgcaggcgctgggccgctcgttggaagcgccgccgtcgtataccgccatcggggccttggtcgagcacatcacgggcgggcatctggaaggcgcaaagttccagccgatgaacatcaactatggcctcttgccgccgctggaggcgcccaaggtggatgagaacggccagaaaattccgatgaaggagcgcggccgggccaagaagcggctgatgagcctccgggcgctggacgggctgaaagcctggcgcgacgtcggctgacggagcggcgtcggcctctcgcgcgttgaggcgtcatggcctatccggacgccctctcctcttcgtcgctgaccgatccggtgaggcgcgcgatcgcccagcgggtggtgcgcatcttcaacgatccggacaagggcgagagcccggtcgtgcgccggcccgatggtctgtacgggccgaactcggtggcctggcgggtgcacggcgacgtgacctccatgatggtgggcggcgtatctgggctgttgctgcagatgctccacccggcggtgctggccggggtgtgggaccattcgaacttccgcgccgacatgcacgggcggctgaggcgcacggcgcgcttcatcgccctgacgacctatggcgggcgggaggaggccgagggcgtgatcgggcgggtgcggcgcatccacgatcaggtggcgggcgtgctgccgagcggacggccctacggcgccaatgatccggccctgctggcctgggtgcacgtgacggaggcgtggagcttcctcaacgcctggatccgctatggcgagcccggcatgtcgatggcggatcaggatcgctacttcgaggagatgacggtcgtgggcgccatgctgggcgccgatccgatgccgcgcagccgggacgaagcgcggcgcatgctgcattcgggccgcccggccctgctggtggacgagcggacgcgggaagtggcgcatctggtgctgaaccagtcggcgcggtcccgggcggcggagccggtgcagcggctgatcatgcaggcgggcgtcgccctgctgcccgaatgggcgcggcggatgcacggcttctcctcgccggtgctgcgccagccgctgctgcgggcccagacgcggggcgtggcgcggacgctgcgctgggcgttcgagggtcagccgaaccggcgcgtcacacccgcccccgcagcaccgcccaggtcagacgcagccgcttgacgggctcgggcgtatcggtccggatcagggcggcgtgggcgacggcgggaaaggcctgcgccggcagcgccttcagcgcgcggttggcggcggggcgcagcgccctcgcctcctctccccggccggtctgggccaggccgcgcatccggcccgcatcgatcaccgcgtcggcgtggccggggccggcgaggacctgcaccgccgcctgcatcgggccgacatagaaggcgtcgaggtcgtgcggctcgctgcggacgcggccgatgtgcgcctcgatcaggccgtcgaagggggcgcggtccagggcgtggcggccgacggcggcggtcagcgcctcaagcaccggatggcccaggcgaggctcgcccgagaagacgccgtccatctgatcggcccaccaggtgtagcgcatctcggccagcagcggctgggtgacgcgggtcgggatggccagcagctcggcctcgaaggcgtaaagcgcgatcaggtcggcgcgcagcgcctcgtcggcgacgaagcggctggagagccagcggtcgggatcggcctcgcggacctggtcgtccagggcggccaagcgcgatcaggccgggcgcgagacggcgaagtcggccagcgcctccagcgccgcgcgccagtcggaggccggcaggatcgacagcgccgccttggccgcatccgcatattcgccggccagatccagcgtcgcctgcaccgcgcccgagcccaggatgatctcgcgggcgcggcggaagtcgtcgggcgtgcgctcgcccctggtgatggtccgctcccagaaggcgtcctcgcggccccgggtgcgggcgaccgccaggatcagcggcagggtcgccttgccctcgttgaagtcgtcgccggcgttcttgcccagggcctcggccgaggcgccgtagtccagcgcgtcgtcggccagctggaaggcgatccccagcgccatgccgtagtcgcgcatggccttgatcaccgcatcctcggcgccggcgcccaccgcgccggattcggcggcggcggcgaacagctcggccgtcttcgccgagatgatcttcagataggtttcctgctccaggttgaggtcgtgcgcgcgcgtcagctgcagcacctcgccttcggagatgacgcgcgaggcggcggccaggatgcccagggcgcgcagcgaatcggtctcgaccatcagctcgaaggcgcgggcgaacaggaagtcgccgaccagcacgctggtgggcgcaccccagatgaggtgggccgccaccttgccgcgacgcagctcggacgcgtccacgatgtcgtcgtgcagcagggtcgcggtgtggatgaactcgaccgccgccgccagccgaagcggaccgccgatgtcgcccgccgcgccgctcgcccgcgccgccgccaccgtcagcagcggacgcagacgcttgccgccggccgagatcaggtgctcggccagcatggggatgaccggcacgtcggactgcatccggtccaggatcagggcgtcgaccgccgccatgtcagccttggccagccgcacgaggctgtcgacatcgccctttgatcggggcgcggcggcgagggcagcgtccaaggagaactctttcgatacgcagggcgcgggaggcgcgcccatgacaaacggccgcgtcgggcttgcccggtcgcgatgcggcgcacaatggtgatcggcccggagagggtcaaggcgcttcgacccgcaagcgtggtggagagcatggccaatatgtcccaggttattgaaagcgggctgctgggcgggcgggtgcggctgcgccagccggcgacaggttaccgcgccgggatggatgcggcgctgctggcggcggcggtcgctgcaagtcccggagagcgggtgatcgaggcaggctgcggcgcgggcggcgcgctgatgcaggtggcggcgcgctgtccgggagtcggcctgtccgggctggaacgcgatgcggcgatggtcgatctggcgcgcgggaacgcggcgctgaacggcgcggcggatcgggtcgaggtgcgggcgggcgatgtggccgccggatttcgtgcgctggacctcgaaccgttcgactgggcgatcagcaatccgcccttctttgacgacgcgggcgccatgcgggcgccggggccgggcaagcgcgacgcctggatggccgacgacgggctgggggcctggacgcggttcctgctgaaggcggtgcgagagggcggtcatgtcgtcatgatccaccgcgccgaccggctggccgacctgctggcgctgctgggcgacaaggcggggtcgttcgcgatccggccgatccatccgttcgccgatcagccggccaagcgggtgctggtgcgggcgaccaagaccggcaaggcgccgctgcggctgttgccgccgctggtgatgcatgagcgggactccgaggccaagcacacgccggcggcccaggcggtgctgcgcggcgaggcgacgctggattggtgacgcgcgaaagccccggtctgcgtttgcatccggttggagggcgggcgggacgccgggccttcgcccggagtgtgagtagaggttaccgtttcgacgaaagctgacgccccgcgcggatgattacgctgcaagctcggggcggaggatggtggcggtcttatcgcctaaccccataagcctgcggcgggcggggcgctctgcgacagcgctccccggtgcggccgagtatccccctcgaccctccaacgccggggcgatccccgacgccggcgggtccggtcgacctgaccgaacccctcccgctccatccgctcccgcgcccgcaagtccgcaggccaggcgagccctccagtgcgacgagacggatgcaggatggcacgggcgggaactcaggcgaggacgttgggacgaggttcggccaaggtgttgttcaggcgcgggtttgtcgcggctgatgcgtcggctgagtttcttttctcgtcatcctcgcccctgtggcgaggatccagactcccggtctttgccgttggccaccgggagtctggaccctcgggacaagcccgagggtgacggagagaggtgggaagaggaaagggatgcacgtcggcgccttctccctcccccgttcggggagggtggtcgcgcgagcgaccgggtgggggcggcccggcaaggtcgcacggatcgaagcaggtcagatcgtcgatgggtcgccttgccgcccccacccggcttcgcctgcggctcagccaccctccccaaatggggagggagaaggtcggccttcacctcgccgtttcggaaggctatcccctgccccatgtcgctacgtccgctgttcgtcacccaggtctaccaagccaccctggcggaaggtcgcgggttcgccgagttcaacgcgcagttgatcgacgcctgtcgaatgctggcggaagaagatgaaggcggacgccggtggtgccgggcgaacggctatcggggctacacctcctacggctcgttgaacgacctgccgcagcggctgccggagttcgccgagctgaagcggcatctggaccggcacgcgctggcatacgccaaggcgctgaacttcgatctggcgagaaagccgcgcctggacaatctctgggtcaacatcctgaagcccggcggcgggcacacgggccacatccatccgcacgccttcctgagcggcaccgtctatgtggagacgccgcccggcgcctcggccctgaagctggaggatccgcgcctgccgatgatgatggcccggccctccgtcaacgatgaggcgtcggaggccgagcggccgttcgtctatctgaagccccagcccggcacggtgctgatgtgggagagctggctgcgccacgaggtgccggtgaacgccgccaggtcagaccggatttccgtcagcttcaactacgcctgacgagcctaggcgcgcgcccgccttatttgcccttcggcctcgggatcgctacatccccgaccaatccccaacgcacacgatttccaagggcgcaccgcacctcatggcgcagcaatacatctttcagatgcagggcctgaccaaggcctttcccggcggcaagaagatcttcgagaacatctggctgagcttctacaacgacgccaagatcggcgtggtcggcgtgaacggctcgggcaagtccaccctgctcaagatcatggccgggctggacaaggagttccagggcgaggccaaggccgccgacggcatcaagcgcggctatctggagcaggagccgcaactcgatccggcgctgaacgtgcgcgagaacgtcgaggcctggtgcgaggagaagcagtgggtcaaccgcttcaacgccgtcgccgccgcgctgggcgagaactacaccgacgagctgatggaggagatgaccagcctccaggaaaagatcgacgccggcgacgtctgggacatcgacagccgcatcgagatggcgatgaacgcgctgcgctgtccgcccgacgactggtcggtcgagaacctgtccgggggtgagaagcgccgcgtggcgctggcgcggctgctgctcagcaagcccgacatgctgctgatggacgaaccgaccaaccacctggacgcggaatccgtcgcctggctgcagcaccacctggagaacttccccggctgcgtcatcctggtgacccacgaccgctacttcctggaccaggtgaccaagtggacgctggagctggaccgcggccgcggccatccgcacgagggcaactattcgtcctggctggaggccaagcagaagcgcgtggtgcaggagcagtccgagtccgaagctcgccagcgcgccctgacccgggagctggagtgggtgcgttcgggcgccaaggctcgtcaggccaagtccaaggcgcgtctggccgcctatgagaagatggtggccgagcaggagaacagccgtcaggcccagtccttcgccgtgatccagatcccgcccggcccgcgcctgggcaatgtggtgctggaggtcgagggcctgcagaagtcatatggcgacaaggtgctgttcgacaatctgaccttcaagctgccgcccaacggcatcgtcggcgtgatcggccccaacggcgccggcaagtccaccatgttcaagctgatcaccggccaggagacgccggacggcggctcgatcaaggtcggggagacggtgaagctggcctatgtcgaccagtcgcgcgacgacctgaagccggacgacaccatctggcaggccatctcgggcggcaccgacatcatgatggtgggcaagcgcgagatcaattcgcgcgcctatgtcggctcgttcaacttcaagggcggcgaccagcagaagaaggtcggccagttgtcgggcggcgagcgcaaccgcgtgcacctggccaagaccctggcgtctggcggcaatctgatcctgctcgacgaaccgaccaacgacctggacatcgagacgctgcagaacctggaagaggcgctggaggagttcgcgggatgcgccgtggtcatctcccacgaccgctggttcctggaccgcctggcgacgcacatcctggccttcgagggcgacagccatgtggagtggttcgaaggcaacttcgaagcctatgaagaagacaagaagcgccgcctgggcgccgacagcctgatccccagccggatcaagttccagaagttcgggcgttaagctgaagggcggtcagaggccgagttgcaatctgaccgcccgctccacccctgaaagatcggcggccgaaagcatgccgatgcgccggcccagacgcagcttggacgccgtcgtgatctgatcggccatggccttgccgggctgtcccgcaacggtgatcagcgcttccgccacatagacgcgttcgacgttgctggtgaccggcacgacctggatgcggttcatgcgacgattggcggcgtcattgctgatgatcaccgctggtcgggtcttgcgcacctcgccgccgacggacggatcgaacgaaacccaccagacctcgccccgacgtggggagtccgtcattgtgcggcgtcgccaagcagagcctcgctccacgcgtcggcttcctgctcgcgctcgtcgtccagggccatggccgcataggcgtcatcgagtgcaccgtcgatgaccagaggccgcaccagatcgttgacgaaccggctgatccggcctggcccgatctggctatgaagccctgcgtaaacgtcgtcatcaatggtgagggtcagcttcttcatgactccatcatacgtatagatgcacgtgtcgtcgagccggccaatcggcggcaattcccttggacaaacatataaggatatccttatatgaccgcatgagcctgaccgccgaccagaccgtggaagcgctgcgcgccgccggagagccgacgcggctgcgggttttgtcgttgctggcgggcgaggagctgtcggtgatggagctgtcgcgggtgctggatcagagccagcctcgcgtgtcgcgccacctcaagctgatgaccgacgccgggctgatcgagcggtttccggacggggcgcgggtctattaccgactgtcgcacgacgcccaggcgcggcgattgatcgacacggtgctggacatcctggccgacgatgcgggcgaggccgatcaccggcggctggacgaggttcggcgcgatcgcgaggagcacgccgcccgctacttcgagcaggtggcgccccagtgggacaaactgcgctcgctctacgtcagcgaaagcgcggtggaggcggcgctggagcgggcgatcggctcgggcccgttcgagcgggtggtggacctggggaccggctccggtcggatgctgacgctgttcggacgacgggccaagatgtcggtcggcctggatctcagccagaacatgctgaacatcgcccgcgccaacgcatccaaggccgggctggacaaggtcgagctgcgtcacggcgacatcttcgccacccgactgccggccgagagcgcggacctggtgatcgtgcaccaggtgttgcactacctggccgatccggcggcggcggcggcggaggccgcgcggctggtcatgcccggcgggcggctggtcatcgtggatttcgcgccccacgcattcgagcacatgcgcgaggcgcatcagcatcgccgcctcgggttcgccgacagcgagatcgccggctggctgaccgaggcggggttgaagacatcggcccccatcgccctgccccctgagtccgagggcctgaccgtgaccatctggatcgccgaacgcgagcgcctagcccaaaggagcgtcgcctgatggccgcatcatccaccagcctggccgaggcgcgggcgctgctgttgtcgccgctggggcccgtggcgcgcgcaggctcgaaccgcgacgcggtgaaggtgtcgtttgagttctttccgcccaagaccgacgaggccgaggccaatctgtggaaggcgatccgccggctggagccgctgcgccctgatttcgtttcggtcacctatggcgcgggcggctcgacgcgcgagcgtacgcaccggacggtgcagcgcatcatcgccgagacttcgctgcgccccgccgcccacctgacctgcgtggacgccagccgcgacgaggtggacgcggtgatcgagggctacaagaccataggcgtcgaccacatcgtcgccctgcgcggcgatccgccgaacggggtcggcatcggcggcgtctatcagccgcgctcggacggctacgcgaacgcgaccgaactggcgcgcgccatcagtcgcgtcggcggcttcgacatcaccgtcggcgtctatccggagcagcacccggaaagcccgtcggtcgatcacgacatagacgtgctgaaggccaaggtggacgccggcgccacgcgggcgctgacgcagttcttcttcgacatcgatgctttcctgcggttccgcgaccgggtgcgggcggcgggcgtgtcgatcccgctgatccccggcgtcatgccggtctccaacttcgcggggctgaagcggatgagcgcctcatgcggggcggcgatcccgtcgtggctggaggcgcatttcggcgggctggacgacgatccggagacccgcaagctgctggccgcctccatcgccgccgagacctgcgcgcgtcttcaggaggaaggcttttcggacttccacttctacacgctgaaccgggccgatctggtctacgccatctgcagggtgctgggcgtgcgcgaggccgcgcaatgagccgccccatgacgcgagccgatcgcatcgccgccctgcatgcggcggccaaagaacgcatcctggtgctggacggcagctggggcgtgatgatccagcggcgcggcctgtcggaggccgacttccgcgcggaccgctttgtcgcggccaacggctatgacgagaagcaccagatgaaggggaacaacgacatcctctgcatcacccggccggacatcatctcggacctgcacgaccagtactacgacgcgggcgccgacatcagcgagaccaacaccttttcggcgaccaccatcgcgcaggaagactatgcgctggacgcgcaggcggtgtgggacatcaacctggagggcgccaggctggcccgcgcctcggccgaccgctggacggagaaggaaccgcacaagccgcgcttcgccgccggatcgatcgggccgctgaacaagatgctgtcgatgtcgtcggacgtgaacgatcccggcgcccgcagcgtgaccttcgaccaggtctatgaggcctatcgccagcaggtgcgggcgctgaacgagggcggcgtcgacctgtatctgatcgagaccatcaccgacacgctgaactgcaaggcggcgatcaaggcgatcaaggatctggaggacgaggggctggagcccctgcccatctggatttcgggcaccatcaccgaccgctcgggtcgcaccctgtcgggccagacggccgaagcgttctggaacagcgtgcgtcacgccaagcccttcgctgtcggcttcaactgtgcgctgggcgccgatctgatgcggccgttcatcgccgaactgagccgcgtggccgacaccctgatcgccgcctatcccaacgccggcctgcccaacgccatgggccagtacgacgagcagccgcacgagaccgcccacttcatcgaggaatgggccaaggccgggctggtcaacatcgtcggcggctgttgcggcacgacgcccgaccacatcaagcacgttgccgaggaagtggcgggcgtgacgccgagagccattccggaacggccggtggcgctgcgtctgtcggggctcgaaccgttcgagctcgtcgcatgagcaagcccgccttcaacttcgccgacgccgacttcgtcgccagatacgtcgagaaaggtccgcgcgccttcatgcccggacagcccggcgtgctgcagatggcgggcgtcctgctggccgagcgcatgccggacgacggccatgtgctggtggtgggcgccggcggcggtctcgacacccatgcgctggccaaggccggaccaagctggcgcttcaccggcgtcgacccggccgcgaagatgctggacctcgcccgccacatcctgggcgaggagacgatgcggcgcgtcgagctgatcgagggcggcgtggaagccgcgcctgagggcccgttcgacggcgcgacccttatcctggtgctcggcatcctgcccgacgacggctccaagctgacgacgctaaaggccatccgccgcagcctgaagccaggcgcgcccttcgttctggttgatcgctgcgacagcgccgacaatccgcagtttgaccgcaacatggaccgctacgtcgccttcgcggcggccaacggtgtcgaccctgagacgctgaagaccgcccgcgcgagccatcgcggcaatcccggcctggtcaccgccgcccgggacgaggcccttttggccgaggctggcttcaccgacatcgaagatttctattatgccatgaactggcacggctgggtggcctacgcctgatgcgtcctgtcttcatcaacgtcggcgagcggaccaacgtcaccggctcggccaagttcaggaagctgatcgtcgaggggaactactcggcggcgctggacgtcgcgcgccagcaggtcgaggcgggcgcccaggtcatcgacatcaacatggacgagggcctgctggacggcgccgtcgccatgcggacctttctgaacctgatcgcggccgagccggacattgcccgcgtgccggtgatgatcgactcgtccaagtgggaggtgatcgaggcggggctgaagtgcgtccagggcaagccgatcgtcaattcgatctccataaaggcgggcgaagccgagttccgcgaacaggcggtcaaatgcctgcgctacggcgcggccgtcgtggtcatggcctttgacgaagtgggccaggccgataccgccgcgcgcaagatcgagatctgcacccgcgcctaccgcatcctggtggacgaggtgggctttccgcccgaggacatcatcttcgatcccaacatcttcgccgtggcgacggggatcgaggagcacgacaactacgccgtcgacttcatcgaggcggtcaaggtcatcaaggccaccctgccctacgcccgcatctcgggcggggtgtcgaacgtgtcgttcagcttccgcggcaacgagccggtgcgtcgggcgatccactcggtctttctgtaccacgccatcaacgccggcatggacatgggcatcgtcaacgccggcgacctgcccgtctatgacgacatcgacgcgactctgcgcgaggccgtcgaggacgtgatcctgaaccggccgcagcggaccaacgtgtccaacaccgagcggctggtggacatggcgcccggctacaagggcgagaagggtgcggccaaggtcgtggacctgaaatggcgcgaacagccggtcggaaagcgcatcgagcacgcgctggtgaacggcatcaccgaatacatcgaggcggacaccgaagaagcccgactgttggtcgagcggcctctgcacgtcatcgaaggccccttgatggacggcatgaacgtggtcggcgacctgttcggctcgggcaagatgttcctgccgcaggtggtgaagtcggcgcgggtgatgaagcaggcggtggcctggctggaacccttcatggaggcggagaaagccggcaagccgagggaacaggccggccgcatcctgatggccaccgtcaagggcgacgtccacgacatcggcaagaacatcgtcggcgtcgtgcttcagtgcaacaactatgaggtgatcgacctgggcgtcatggtcccggccgaccgcattctggatgaggccgaggcgcacaaggtcgacatcgtcggcctgtccggcctgatcaccccgtcgctggacgagatggtgttcgtggccgccgagatggagcggcgcggctttgacatccccctgctgatcggcggggcgacgaccagccggacccacacggcggtgaagatcgagccggcgtaccgacgcggctccaccacctatgtcgtcgacgccagccgcgcggtgggcgtggtttccggcctgctgtcccagaccgaccgcgcccggaacgaagcggccacgcgcgacgaatacgtcaaaatccgtgaacagtatgcgcgcggccaggaggtcaaggcgcgcgccacgatcagggaggcgcgcgacaatcgctggcggcccgcacctgaccagacgcccgtcgggaagcccggcttcatcggcgtgcgggcgttcgacgcctgggacctgcaggacctcgccgaccacatcgactggacgcccttcttcgccagctgggagctgatcggccgctatccgctcatcctggaggacgaggtggtgggcgaggccgcgcgcgacctgttcgacgacgcacaagggatgctgaagcggatcatcgaggagaagtggttcaccgcacgcggcgtggttggcttctggccggctcaggcagttggggacgatatcgcagtctacgccgatgaggaccgctcggacgagatcgcccgcttccacaccctgcgccagcagatcaagaaggcgaacggcaagccgaacttggcgctatccgactttgtcgccgaggacggccaggactggatcggcgccttcgccgtcaccgcgggccacggcgagctcgacatcgccaaacggttcaaggatgcgggcgacgactactccgccatcttggctacagccctggccgatcgcctggccgaagctttcgccgagcggctgcacaaggaggtgcgcacgcagctgtggggctatgcggcggacgaggcgaccgatgtcgacgccctgatcgccgaacagtaccaaggcatccgccccgcccccggctatccggcccagcccgatcatacggaaaaggcgacgctgttccgcctgctggacgcgggcgggaacgcgggcatggcgctgaccgaaagtttcgccatgacgccgccggcctcggtttcaggcctgtatttcggccatccgggcagccactatttcggcgtcggcaagatcgaccgtgatcaggtcgaggactatgccgcgcgcaaggggtgggatgtcgccacggccgagcggtggctggcgcccatcctcaactatgacccgtatcaggccgccgcgcgcgatcaggcggcctagccggcatcagcttcaggaggccggcgtctccgccggcgtcgcctcgcgcagacccacgtcggcgggggtcgccggcgcggtggtgatgttgtcgcggatgcggcgcgcggcgtgctcgcaccgccccggcaggccgaagaacaggccaaaggattcgctgcgcacccgctcgtcggtctgggtcagcagcggcgcccacttggccttggccgccgccgcggcggcgcgcgcctcggccttcgccgccgcgctctgacgcggctcggccgccgccagggcgctccggaaatcctgcgcctcaagccgtcccaggcgcaccagttccgaatcctcgggcgtccggttggtcagggtctcgcctagatccgcgtggcccgtcaccagcgcgtcgcaccacgccaccagcggataatccgccgtcggcgcgcccgtcggcagcggattggaataggccagcgcctcgcgcagccgcaccgacgcctgcgcctcgcccctgctggtggcggtggcgatcggcccgtctgtctcctgagctagggcgggcgcgcttagaaggccgacgagaatgagggtggtcgggagcagacgcatagaagcttccatcatggatccagggacgcgctaacgcatagccaagctccccgatccgtgtggctatagttcggcgcaaagaaaaaagcggcggaccgaagcccgccgctctcttccgtcagatctctatcgccgtcttagaagcgatagcgcacaccaaaccgcacttggcgcggcgattgatagcttctcggctgcgcataatagggcgagcgcgccgcaaagttcgtcggcccggcagaagcgcttgcatcgttacgaatgaagccctgctccaccacgcgggtcgccgtgtcggcgtcgaacacattgaagacgtcgatcgaggcggagaggatgcctacattgtcgcgcttcaacagatcgaagttgaagttcaggtcgagttggtagacccaatcggtttcaccttgagatccacgcggcgtttggatcgtcgcgttgttggcgcccaaggggcagtaccatcccgaggggccacccgtctgcggcgcaaactgatcaactgacagaggaacccgcccgatacaaccataggcacggcccgattgcgcggtgaagttcgctccgatgctggaccagtcggttggcgcccacgacccgaacagcttaacagtgtgccgatggtggttcggcaagtagccgtaagaaccgagctggttagccgagtggtcgtagtcttgcgtgagcgaggtgtccgtctggccgatgtcggacttcaccgcgccctcgtagttccccttcgagttcgccagtgtgtacgatccgcccaagctccacattccgtcgaatggacgttcgaaggtgaattccagcgcttcgtacgtgcgttcaactttgtcgaagttgaggtcttcggcggtcagatcgatttcctgcgggttgtacgcgggattggcaacgccgttgattgatctcggatcaccttgaagatcgataaagacccgcgcgccgtcgcctgggttgatcagcacgtacggaaagaccgacgagaacgacggcccatctgccggggtatcaccatctgcagtcacgcaagtggtattgttcgtgcggatgcagtaccgcgcgattgcatcgccgatcgcggtgtcctcgatcgcgctctttaggtcacggttcacgtaccgcacacccgcgcgccaatcggcgaacatcccgtcattgaagcgatgctcgtagccgagaatgaactctcgctcatacatcggctcgatgtccgcctccgtcaccgaccgagggtccggcgcaccaggggggctcaggtagtcaagttggaggcttgccccacggaccggatagccatcggctcccagcaccacgttccctgccgcatcgcgcgtgatctcaaaatactcagcggtgtagatctcgccagatgacgcccgaatcgacgtgttggtggcgatgggaaggtagtaatcccccatcgagccatagacacggctcgatccgtcgcccgtcggatcccaattgaagccgatacgaggcgcccactggtcggccaagtcgatgtagggattgccgtctacgttgtcataacgatagcgatcgttccgcaagccgagctggaggctcagattgtcggtgatgtcccagctatcctggatatagaaggccgactgttccgcagtgaacagtcctgagttcgcaaaggtgacgacctcaagctcgtcttcatatacattgtacagcgctccaccagaataggcgctgacagcagtggactcgagatcctcttggtcatacccaagacgaacatggtggttgccgaagaggctgaagtaaaaatccgcgtctacccgataggtgtcacgaacatccttgccctcgaggttgtaagggccgccctgacgtccggcagtgatgtagccgggagccaaggtcccgcctgcgcggaagtaatcgtagatgcccggcaatccgatcggatctccataatccagataggagttgttgaggcgtccgtaaagcgcggacaaagtgaaccagtcggtgaaaacgcccgtgtactggtaggtttggatgtcgccgccggcttcagtgtagatcgggtcggtgatggcagtcatcaaccccgtcgtagcgttgaacgtcctggtctggctgaccgtagtcgactcatcgttgaagtaggtgacttcaaggcgatggttgggattgagaacgaagtcgagtttcgccccccaacgcggatcgtcgtacgatgaaataccctggctcaggttggcgccgggagtgatggctcccctggcgcggttgtaggagaagccgcgactacgcgccccttcggcctcagagtcccggccgttgtaaacaccgaagaagaagacgtggtccttccaaatcggcccgcccagataagcggtgtattcgctgaaatccgattttgcgtattgattgtagatctcggttccggccgagttgtttccaccctgctggtatgcggtgccacgctccgaacgtaggctgttgggcgtgtggtaggcgctgatgccccccgtccattcgttggtgccggagcgggtcacaatgttgacgacaccgccagtgccgcgaccgaactccgcctgatagccgccggttttggtttcgatcgtctggatgaattcaaacggcagctcagcatagccaaggaaggtgcgctggtcggtgacgttcagaccattgatatagtagacgctttcggcagcggaggtgccggaaagcgaaaccagggactggttgcggcgcgagcttgcgttgatgctcgcgtccggcaggctggctccaggagtgaaaagggtgatcgcattgatgctgcgtcccgcgggaacgcggtcggcgaactcctgaacatcaaccgtcaggcccgtatctgtcgcattgaaggactggacgcggcgagccgtgaccacgatgtcttcgagccctgcggcaccctcgttataaagagtgaattcgtatgcggccccacctggagccaccgaaacctgctgggactgtggctcgaaccctgcttggctgatatcgacccggtaggttccgatgggcagcgccggcagacggaactgaccgttgacgcctgacgtagcagtgcgcaccgcgccttgatttgaagttacggagacagttgctccaccgacaggggagccgctcgaatcgatcacagtcccgctaagagcgccactggtgtaatcctgcgcagctgccgaggtcggagccaccagaaccgaggccaccggcaacgcgaccgccgcggccagcgcggcgccgccgatcatcgtggaagccagcaggcgctcacgaatggtttggatattcaaaactgcatccctcctgagtggtcggcgaacggtcgccgatgcagaaccatgcctctacgcccccaaatgcgcgcagattggacatgaccataggatgacaggcgctggcgtccatgtggattacggcggggtaatgatgtgcgccggggtgtgtcgcagttgcgccacagtggcgacgcgaaacagtcatgccgcagatggggctgacatcggatcggacggcttgcctcagcggtctgatccgctacgttttgccgattattcaatatctggcgacacttttttgcacgtaatgaccgtggctcaagtgtggcgagctttgcatcctggtcggcgatggcggagatcgacgaaagctcagcaccccaagggggcgtcaaggccgcccgacaggagaccgatgtgattccttttgtccgagatttcgacttcgcctacggccgcctcgatcttgtcgcaccgctgatcgcgcgggttgtggccgagaacccgggtccgttcaccttcatgggcaccggaacctacatcgtcggccgttccgagcggggcgcgtcggtggcggtgatcgatccggggccgctgaacgacggacatctgcaggcgctgctcgaggccgtcgacgggcggaccgtcagtcatgtgctggtgacgcatacgcaccgggatcatgcgccgctggcgtggccgttcgccgaggcgacgggagcgaaggtgctggcgatgcggccgccggccgtggagacgcatgcgtcgggcggcggggatgaaggggacgccgaggccttttatccggacgaggtgctggtcgggggcgaggtcatcgagggggatggctggacgatcgaggcgatggcgacgcccgggcatgcgtccaatcacatggcgttcgtgctgagggaggagaacgccctgttctgcggcgaccatgtgatgggttgggcgaccacggtggtggcgccgccggacggcgacatggcggattacatgcagagcctggatgcggtgatcgcgcggagcttctcgacgctgtacccgactcacggcgcgccgatcaccgagccggagccgttcctccaagcctatcgcgagcaccgggtgcggcgcgagtcccaggtgctgaagcggctggcggccggcgacgagacgatcgagcagatgctgccgcgcctctatgtcggggtggacaggcggttgtggccggcggcggcgctgtcggttctggcgcacctgatcaagctgtgccgcgaagggcgggtgacggcggatccgtcgcccgtggcggaggcgcgcttcaggctgacctgatcgtcagggacgcaggttggcggcgatcttggcggccaggcggcaggtcgcgccgccgtcggggcgatcgccgcgcgcggccacgcggatgtcggttcgaccggggcggatgcggatcaccgcgtcaaaggcgcggccgaaccaggcggcctcatgcacgccctccacctgaaaggccgaggcgcgcaccacgggaaaaccggcgtcgacaagggcgccgcccacggtctgggccgccagttggctggggatggcggcggcggtggagcaggaggcggtgtcggcgggtgcggccccagccccgtggaaggcggccagcgcggagaagccgggcgcctcatcggtgttcgtggagacgtccagcggccagtcgcgggcaaagcgggtggcttggaatccgaaggcgcccacggtcgcgcccgcgatgcagagggcggtcgcggcgggcagaacccgcgtgcgtgaggcgagagccgccaccgccgcgatcagcccggccgccaccccgatccaggccaggacccgagcgacgcgccaggtcagaagatcatagccgaccgcaagttcgaccatgcccagccggaccagcagcaccgcaaccaggaccagcagaggcgcggccaccgaaagcgcgaccagagccggcgtcaggcgggcgatgagccgctggcgtgcggacgtgtcggacggcgtggtcgcgggcatcggccctcccctgctttggacgccgtcaggcggattcgggcagacggtagtccttcatccgctcgcgcaacagcttcttgtcgatcttgccggtggcgcccagcgggatgtcctcggcctggaccacgtcgtcgggcatccaccatttggcgatcctgccgcgcaggtgatcgaggtgttcggccttgttcagcgtctcgccgggcttgagcttgacgatcagcacggggcgttcgtcccacttggcgtgtggggcgccgatcacggcagccagttcgaccttgggatggccgaccgcgatattttcgatctcgatggaagatatccattcgccgcccgacttgatcacgtccttggcgcggtcggtgatctgcataaagccttgcggatcgacggtggcgatgtcgccggtgtcgaagaagccctgatcgtccaggatcgacgcgtccgacttgaaatagccggcggcgacaatgggccctcggaccatcagccgaccaaaggtctcgccgtcctgggcgaccggctgaccggcttcgtccttaagcgccagttcgacgccaagcggcggcacgccctgcttggtgcgccacttcatctgctcgtcgtaaggcaaggcggcgatctcgggcggcagatggccgatggtcccgatgggcgaggtctcggtcatgccccaggcgtgggtgacctcgacgccgaaatcctcctggaagccgcggatcaggctttcgggacaggccgagccgccgatcagcacgcgcttcagcgtcgagaagcgcaggtcgttgctcttcatgtgcgcgaacaggccctgccacaccgtcggcacggcggcggagaaggtgacgccctccgcctcgatcagctcgtaaagcgccgccccgtccatgcgcgcgcccggcatgaccagcttggttccggaggccgggccggcgaaggcgatgccccaggcgttggcgtggaacatgggcaccaccggcaggatcacctcgctgggcgtcgcccccatcaccgtcgccgtcatcgccatgaaggtgtgcaggaagttggagcggtgcgagtacagcacgcccttggggttcccggtcgtgccggaggtgtagcagaggccgcaggcggtgttctcgtcgaagccgccccaggcgcagtcggccgactgcccggacaggacgctttcgtagtcgtggacggtcgggattcgggtctgcggcaggtgcgccgcgtccgtcaggacaaccacccgctcgaccgtcgggcagtgcggcagcaccgcctccagcagcggcagaaaggtcaggtcggtgaagacgatccggtcttgggcgtgattgatgatccagcccagctgctcggggaacaggcgcgggttgagggtgtggcacaccgcgcccatgcccatgatgccgtaccaggtctccatgtggttggcggtgttccaggccagggtggcgacgcggtcgccaggttcgatcccccacgccttcagggcgttcgacaggcgcttggcgcgctcgtggatggcggcgtaggtggtgcggacgatcggcccctcgaccgagcgggtcacgacctcgcgctggccgtgccagttgcgggcgtgatcaatgatcttgtcgaccgtcagcggccagtcctgcatcaatcccagcatcgctctttccgtcccaatccgtgagtgcatcgaccttgaccgcgatgcttggcggcgacgctatcccgacttatcggcgtttagcaatcgcagcgcgtgcgacgcagggtccctggtggcgcggggcctacgcaggggctaaaggcgcgccatggccattctgatcgcgatcaccgggggctcgggctcgggcaagagcacgctggcggaggcgttggtggcggccctgccgcccggcgcggcggtgctgatgcgcgaggactcctactaccgggacgcggcgtccctgcccgagttcgaccccgacaccttcgatttcgacgacgtggcggcgcgcgatcacgaactgctgacagaacacctgtccgagctgaaggcgggacgaggcgttgaggcgccgatctattcgttcattcatcatgggcgcgagccaggcggcgaggcggtggcgccggcgcaggtggtggtggtggaggggacgcacgtcctgtgcaccccggcgctgaccgctctgttcgacatccgggtcttcgtggatacgccggcagacatccgcttcatccgccggctgctgcgcgaccagagcgagcggggacgcacggccgattcagtgatccaccagtatctgctgacggtgcggccggggcatgagcggctgaccgagccgtcgcgcacccacgccgacttcatcgtggccgacgccaccgccgcggtccggctggaggacccgcaggcggtggtgcgactcgcggccccggtgctggcgcacccgctgctgaggccgctgctgtccgcctagggccagagccgctcgcgccgccaggcctcgccgtcgcgcacgaagcgcaggcggtcgtgcaggcggaacggacggtcgcgccagaactcgatagccgaggggcggacgcgccagccgttccagcgatcggggcgcggcacgtcctccccctcgaagcgggcggtctgttccgccacggcgtcgatcagggcctgacgatccgagagcgggcgcgactggtccgaggcccaggcgccgatgcggctttcgcgcgcgcggctggcgaaataggcgtcggcctcctccgggctcaccgactcgaccggaccgcgcacgcgaacctggcgacgcaggctcttccagtgaaacaccagcgcggcggaaggactggcgtccaactcgacgcccttggcgctctcgcggttcgagtagaaggtgaagccgcgcgcatccacgtccttcagcagcacgatgcgggcgtcgggcaggccgtcggcgtccacggtcgccagggtcatggcgttggagtcgttgatctcgtgcgcccgcgcttcggccagccagtcgacgaacaggccgaagggctcgtcgcgctcgaacgccgcctcatcgctgttggcggccagggcggcggcgtagtcgcgggcgtagtcttcggccgaggggctgggagggatggcgggcgcggtcatgagcctgtttctagcggctgggatcagggctggaaatgaccgacccgatcacggttaaccggcctttgactctgttcggccaagcatcgacgcatgtccgcctcctccgcccggatcgaccccgcccagcggaccgccgccctggccctgctgggcctgctggagagcaccgacggcgaggcgctgaaggcggcgttccgccaggccgtcaaggccgcccgcccggaccaggccggcggcgacgccgagcgcttccgccaggtgatcgaggcctatcgactgctgcagacgccgcaggtccaaccaggcgtagccgtccggcgccccctgcccgaggccccgccgattctggtgctgacgccgcttcaggccctgaacggcgcgcggatcccgacgcgggtgggcgacaggcggctggcgatacaggcgccggcgggcgtgcgcaccggagaccggctgaggctgcgcgaccgcggcgcggaccatctggtggcggtgctgatccggccggcggacggcctctcggcgatgggcgacgacctgttcatggcctggccgacgccgccgaggatgctggacggcgggcgcatcgagatcaagacgcacgccgggctccgatccgcctgggtgacgccgggcctgagcgcgcctgcgcggctgtgcctgcccggccttggcctgcccgcgcgcggcgcgcggccgcaggggcggctgttcgtgacgctgacgcctgcgtccgacgccccctctcccgccgaggatcgcctgctcaggttcacgaagttctggacgcccgagcggctcgccgcctaagcctcagccatgtcgcacaacaccttcggccatctgtttcgcgtcacgacctggggcgaaagccatgggccggccatcggctgcgtgatcgacgggacgcctccagggattcccctgacgacggccgacatccagccgtggctggaccggcgaaagcccggcggcagccgcttcgtcacccagcggaacgagagcgacaccgcgcaaatcctgtcgggggtgttcgacgacggcgcgggaccggtgaccaccggcacgccgatctccatcctgatcccgaacgaggaccagcgctccaaggattacggcgagatcgcgcgcgcctttcgccccggccacgccgactacgcctatcaggccaaatacggggtgcgggattatcgcggcggcgggcggtcgtccgcgcgcgaaacggccagccgggtcgcggccggagccgtggcgcggaaggtgatcggcgacggcgtgcgcatccgcgcgggcgtggtgcagctggggccgcaccggatcgcggacgaccgcatcgacttcgacgccgccctttccaatccgctgttcgccgcatcgaccgaggtcgtcggtgactgggaagtctatctggatgcggtgcgcaaggccggctcgtccatcggggcggtggtggcgctggaggtcacgggactgcccgccggatggggcgcgccgctgtacggtaagctggacgcggaactggccgcggccctgatgtcgatcaatgcggtgaagggcctggagatcggcgccggtttcggcgccgcgacgctgtccggcgaggataacgccgacgagatgcggctggatgcgcagggtcgaccgctctttctgtcgaaccatgccggcggcgtactgggcggcatttcgacgggccagcccctgaccgcgcgcgtggcgttcaagccgacctcctcgatcctgacgcaccgccgcacggtgacgcgcgacggccaggagacggacctgcgcaccaagggacgccacgacccctgcgtcgctctgcgcggcgtgccggtggtggaggccatggccgcctgtgtcctcgccgacgcacggctgcggcaccgcgcgcaggtgggcggctaggccggagttcgcagtctcggctgcggcctcgacggctgcggcgcggtgggggagcgccgagagagctccgcgccgcgcatcaacgccaccaaactcgccagcccagtggtcatcacgatcatggatgcacctgcgattgagaacaggtcgcaggtttgcgcagagtcgcggatcgtgcaagcctcggcgttcaccacatcgacttgaagggcgtcaccgatgcgtgaagacggcaagctggactatctggaactgccgggcggcgccctgccccagaccaaggccttctacggcgagacgttcggctggaccttcacggactacggcccgacctatgcggcgttcgagcagggtctggacggcggcttcgacgccgatgcgggcgaagcgacgccgcagcccctgcccgttctctacgcccaggacctcgaggccatgcaggccagggtcgaggcggccggcggcgtcatcgtgcggccgatctacgcctttcccggcgggcggcgctttcacttccgcgacccggccgggagcgaactggcggtgtggtccgaaggctgacgccgctcagcgcgcctcgacgctctgaccgatagcctcggcctgggcgcgatcggcgccctcaaggctggcgatccagacgtggatctccttgggcgcggacggacgctggaacaggtgttcgaccgcgatacgctgactgttctcggtcagcacgaccgaaaagcgcccgcccgcctggaccacctggccgtcgtagatcggaaactgcgacgccgggccggcgtagacggtgacaaaggtctggccgccccgctggatggcgtagaccttggcgtccgggcctgacggacgctggatcatctgaaagcccgccggcacggtggcccggaacggcagggcgccgatggcggcggcgctcagcggcgcgacctccggcgcacgcggcgcgggcgtcgtctcgggcgcaggcgcaggcgccgcagccggaggggtcggagcgggcgcagcggactgagcggccggtccgcccttcaggctgcgggtgaggtcgctggacgggcgcggcgccgtctggccggacggcgccgcgacggcgagggcggagaggagagcgatcaacatcatcgcggaagattgtcccgcccttgtgtcgagaacaagccccagcgcatcgcctaggcgcccggcagggtgacccagaaggtcgcgccctcgccgggctccgacaccacgccgatctggccgctctgcggctccaccagccggcgcgccagggccagaccgatgccgtgcccctcgatcgtcgaccgctccaggcccagtctgttgaagggctcaaacagctgcgcctgcttttctgaactgaggcccggtccgaagtcgatcacctcgatgcgcaccgcagcgtcctcgcggacggcgcgcaggacgacgcgtccgccggaaccgccgtacttcatcgcattgacgccgaggttggtcagcacctgcgccatccgctgggaatcggccagagccaccgctgtggacggctcgccctgcacctccacggcgacgtcctgcgcctcgggccgcaggatcagggcgcggcgcacgtcctgcatgacgccgaacatgtcggtcggacgcagatcgacgcggacagctcccgcctcggcccgcgccacgtccagcagatcgtgcgccagatgttcgacctcccgcgcggtgcggaccagcatgtcggccatttccacctgctgaggcgtgacaaggcccagctgtcccttggaccacagttcgccgatgccgatcacgcccgcgaccggactcttgatctcgtgcgccacattggccagcaggcgcgacttggcggccgaggcgatctcggcctggcgctgcgcccgtcgggcggcggcgaccagctccgcccgctcctcgatcaggctggccagaagggtgaagggcatgtagccgaccaccacaagcagctgcgccgtcatcacctgctgcgacaggtcgccggccgcgcggtagggaccatgtccgatcagcgaagcgcccaccgcgatcagggcgatgatgcagatggcggccgccacgccgagaacccgaaagcgcagcgcgataagaaccagcgccggcagcagcagaaatccgagcggcaagccgccggtgaaggcgaacaggcaaagcgcgaccaggccgaccagcaaacccgccgcctccagcgcccgctgcggtctggcgagcacgcgcagactgaccggcgttgcggcgacagccgtggagcagatcaccgccatgcccatggcgtggcccagccaccaggtctgaaggttcggcaatatcggcgcgccggtgaagaggcccaggcccagggaggccaccaggccggcggcgagcggcggcagcacggcggtgctgaccagcaagcgcgcggcgtcttccagggtgttcatcgacagggccggcgcgaaccgccgcgccatcgccactgcgccgacgatctcgatcaggttgacgatggtgaagaagacggaaagcgccggcggattgcccgcgagcagttcgccgaccaggagcgccgtcgccatggccgcgaaaaaggcggcgtccagagagcgtcccccgccgccctggcgaagccacaccgccgtcgccagaccgctcgccccccacaaggccgccaccgttccctcggaccgcgcgagcgacagggccaggccgatcagaacgaccacctccaccccggcgacgatgggcgccagcgtccaacccagcccaccggcccgggttcgctcgacgcgcgtctcgcgcgtgcgcggggctttcgaagcagcgaggtcgagcgcggtgctcggggtcatggcgagggccttgggtaagcggctacgttctccacagaccctatctttgttaaatttcctctgaggccccggccagaaccgccgtgaaacgcgacaccgccgcagcggggccttcggggtatgaccacacgcccgccgaaacggcgacgaagtcggcgcccgcgcgcgccagggcggccgcgttgtcgacggtgatcccgccgatggcgacgcaagggacctccaccgtctcctgccaggtcgtcagcagatccagctccggccgatgggtcgtcgccttggtggcggtcggatggaaggcgccgaaggcgacgtagtccgcgccgccctcggccgcgtcccaggccaggtcgcggtcggcgtggcaggtgacgccgatcatggcgtccggccccagaatgcggcgcgcctcggcgagcggcgcatcctgctgcccgatgtggacgccgtcgcaccccagagcccgcgccagctccggccggtcgttcagcagcaccgccacgcccctcgcccgcgcgatgggcaggaggcgccgcacggcctggccgatctcggcctcatcggccggcttcagccggatctgcagcgccgccacgtcgccggcgtcgagcgcgcccccgagctgcgcggcgaaggcgtccagatcggcgatccggggcggcgtgatcagatacagccggcaaggcggacgagcggaggcgggagattggcgggccatggttccgacctgcgacgccgagccaccgacgtcaacggcgatctgccgccgcgaacgatttgcaatcgcccctgcggctgctatagcgaaccattatcagtcgcctgcgtgagtgttcgcctcgtgtacgtctgcaactgcaacggccttcgtcgacgcgacgtggcccagtccattgaagcgggcgccgagcgtccccgcgacatcttcgcctctcacgggtgccaggcccagtgcgccaagtgcgtgtgcgagatgcgccagatgatccaggccagccgcgaaagcttcgcgctcgcagccgagtagatagccggccgcgcgagcgacaatcgtttgcgttatcaatgcactgataagtattcgcagatgaacacagcccggtttgccgtgctacgaagcctgcgacggcgcggatgcgcgatcaggacaaaaggaccatggccatgaagggcgatcccgcgatcatccgcaccctcaacgcggtgctgaccaacgagctgacggcggtcaaccagtactttctgcacgcccggatgttcgaaagctggggcctgaagcacctgggccaagtcatctacgacgaatcgatcggcgagatgaagcacgccgacatgctgatcaagcgcgtgctgttcctggacggccttcccaacctgcaggacctgcacaagctgcacatcggcgagaacgccatcgagtgcctgggcgcggacctgcagctggagctgggcagccgcgagaccctgctgccggccatcgtccagtgcgaggaggcgcgggatttcgtcagccgcgaaatcctagtgcacatcctgtcggacaccgaggagcacatcgacttcctggagacccagcacctgctgatccgccagttgggcgagcagaactacctgcagtcggccatgaccgagatcggcccggacaagagcgcctcgggcaactgaggtcgatggggcgggcgatgcgcccgccctacccctcgccggcgtccgacaagacggcgggcggttcgaagcggcggatcaggtcagccagatcaggctcatgcaccgcgtcggcggcctcggcgaggggcatccaccgccgctggcgttcgccgtcctcgggccaggcgcccagctggatcagaacctccagcggatacacggcgacgacgcaccgccgctctgcgccgttgcgaagacgcttggcgtagcgaaaggcgccgatcgtctccggatgcatctcgccccggacgcccgcctcctccagagcctcctgcgcggccgcctcgaagtcggttttgccgatcatgcggccgcccttggggatgacccagcgccgcgtctcgcgcgaggtgatcatcaggacctgcagcccttccccggtcttgcgccaaggcagggccgccacctggcgcgtttccgagcgtcctgaacgcttgctcttggtcacacgcctgggcccttcaacgcagtactcgctttcaggggctcgaagacggcattcgagcggcggggtcaagatatccgttcacggatcattccttcttggacttccgcccctcttcgcccggcgccttggcgtcgggatcacccagcacgtcttggcggtacagcatggtcaccagggtgtgcagaaccagcgcgagcggcgtggcgaacaggacgcccagtggcccgaacagcgtgccgatgcccaccaccgcgaaaatgcccagcacgaccggcaggttggcgacgttcttctgcaccatgggggtgatgaagttgctctccagctgggagaccacgacgtagaggcccagcgtcagcagcacggtgtccagcccttgcgtcgtggcgaccagcacggccggcacggtggagacgatcggcccgacgatcggcacgaactgcgccaggcccgtcaggaggccaagcgcaagcgccgacggcacgccgatgacggccagccccacgcccgtcagcgtgcccaccagaaccatcgagaacagctgcgccttcagccagcctttcaacgccatgccgcaagtgttcagcacctggcgaagacggggcctgcgatctagggggaagatcgacagcatgccctcgcgcgacttggccggctcgatcgccagaaacacgccggccaccacgaccaaaaccagggtggtgacgccggacgcgaagcccatggcgaatctctgcgccacctgcagcgcctggcccgcgcggtcgccgagatgctggatctgctccagcaactgcgcgccatacggctgggcctggatgtaagcctggacctgatcccagccctgcggcaggacggccgacagcgaggcgacctgctgcgcgatctgcgtcccgaacaggaacagcacgcccgcgatcagcagaaccacgatcaagagcgaggcgaacaccgccagcgcgtccttgatgcgcgtccagcgctggatgggatcggccagggcgcgcaggatcaccgccaccaccaccgcgccgaagaccagcagccacaaggtctgcagattgatgatcagctgcatggcgtagaaggcgaccaccagcacgatcgcggcgaacgccagcctgcccttccacggatcgccgccgtccagcggatggccaggtgtcttcgccttcaagaatccgaacatgtcgcccccgttcatcgtctggcctcaacgcacagcccggcgcggcgttcggtcacgcgaataataaacggctcagctggaacacggacgggatcggcgccgacgcgacctcagagggacggcagggcggccgccatccccgccttcatctcccgacgctggtcgggcgtgcacttcaggtgcacgcagagacgatcgcccaccctcgtcatgatgcccggcatcgcctccatgacgacggcctcggacgctgcattgatgcggggcagcgcgacaaaggtcttttccagcagggcgcgtccgagatcgctttcgtagaaggcgttcagaccgcgcagttcttcgatggtgaagacgtcggcgtacaccggcgccatggcgtcgaacatccgcggcatcagcgcagagaaggagtccaccataagggtcctgatctcagccgattgcgcttcggacagcccttccacaaccgcaggcaggctggcctcgaccaccgccccaagcgcgtccgtcatctgttgggtctgaactcgcgcgatgatcttggtcgccagggccagcttgatggcgtcctcgtcctgcggctgctgcgcctgtgcggccggcgcggcccaaaggctcagcgccgcgcacagcccggcgatcatcggcttcatcaacacgctcccccaaaacggcggctcatggtggattgaaggggcgcggacgcgcaagaaaaaacggcggggatcgctccccgccgttctcaactcaacatgtttgccgcagttcaggcgccgagcgaggccgggtcgatcttgaagcccgggcccatcgtcgaggacaggctgatgcgcttcacataggtgcccttggcgcccgacggcttggcgcggttcagagcgtccacgaacgccttgacgttggcttccagggcttcctgggtgaaggaggccttgccgacgccggcgtgggcgatgcccgccttttcgacgcggaactcgaccgcgccgcccttggcgtccttgacggcctgggcgacgttcggggtcacggtgccgaccttggggttcggcatcaggccgcgcgggcccagcaccttacccagacggccgaccagggccatcatgtccggcgaggcgatcacgcggtcgaactccatgaagccgccggcgatgcgctcgtacaggtcctcggcgccgacgtgctcggccccggccgcgcgcgcttcatcggcgcgggcgtccttggcgaagacggcgacgcggacgtcgcggccggtgcccgagggcaggttcaccacgccgcggacctgctggtcggcgtgacgtggatcgacgcccaggttgacggcgatctcgatcgactcgtcgaacttggcggtggcgttgtccttgacagccttgatggcgtcggcgaacggcatgatcgcctgggtgtcgccggtgcgggccttgaggcgcttggtttgcttggccatgagcttagccctccaccacttccaggcccatcgcgcgggccgagccttcgatgatcttcgccgcggcgtcgatgtcgttggcgttgagatccttcatcttcttttcggcgatctcgcgcagctgcgtctgcgtgatcttgccggcgacctcacggccgaccagcttggagcccgacttcaggccggtggcctgcttcaggtaccaggtcgccggcggcgtcttggtgatgaaggtgaacgacttgtcctggtagacggtgatcacggtcggaagcggggtgcccttggcttccttttccgtgcgcgcgttgaactccttgcagaagcccatgatattgacgccgcgctgacccagcgcagggccgatcggcggcgaaggcgtggccgaaccagccggcacctgcagcttgatgtagccgagaatcttcttggccattgaactctcctatggatgacctgatcggggatcaggccggtgagccgtggtccggcatggctgcctcccacggatttgtcccgcctgcgcgggaggcgcgcctatagcggaagggtgtggaaaaggaaacccccatgtcgaggctgagcctctcgccaccccccatctcgatggggaggagaaatcttctcctccctgtcgcgcagcgatggggaggtggatcggcggcacagccgacgagacggaggggtctgtctaacgcccggtcagttcggcctgaaggaagtcgatcacggccggcaggtcgtccctgacggctatggcttcgatcctgatgacgcgaacaccttgttgcgccagccagattgttcgtcgcgcgtcatgcgcggcgcgttcggcgccgctgtgcatgagaccgtccacctcgaccgccaccttcgcctgcgggcaatagaagtccaggatgtagggtccgatcggatgctgacgacgaaagcgaactccgagttgccgacccttcaacgccacccaaagtcgcgcttcaggtggcgtcagcgccttccgcatagtgcgggcgcgttcgtagctctcggcgtttgccggcatacccctccgtctcgacggctacgccgccgatccacctccccattcgcttcgcgaacagggaggagaagaggagctacgtcaactctcctccggtcgcgaaggaggaatcgctcgagcaagacaaagccgcgcccgtttccggatgcggcttcaaatctccgaaagtgtgagcctcagcccgccaccttctccacctgcccgtattccaggtcgaccggggtggcgcggccgaagatggagacggcgacgcgcaggcgcgcgttgtcctcgtccacgctttcgaccgagccgtcgaagctggcgaagggtccgtcggtgaccttgaccttctcgccgatgtcgaagcggatggtgggcttgggacgctccacgccctcttccaccgcgccgatgatgttctggacctcgcgctcggagacgggcagcggcttggtgccgccggcggcgcccaggaaaccggtgaccttgggcgtatccttgaccaggtggtaggcctcgtccgtcatctccatcttcaccagaacgtagccggggaagaatttgcgctcggagttcaccttgcggccgcggcggatctcgacgacgtcctcggtcggcaccaggatctcggagaacttgtcctcaagcccgcgctgcttggcctgctcgcgcagctgctctgcgaccttcttttcgaagttcgaataggcgttgatgatgtaccacttgtggcgcggattggcggcgggcgctgcatcggtcatgggcgcgtctttctcaggatccgagagcgatgatgtagcggaaggcgaagcccaggccggtgtccacgatccagaagaagatcgaggcgatcagcaccatgatgaagaccatcaccgaggtgatccaggtctccttgcggctcggccaggtgatcttgcggccctcggcgcggacctggctgaagaactgaccgggcgaggtcttcttcttgggcgcaggcgcgtccacggcgatggtctgggccgccggaaccgtctggggccccgcgcccacctggggacgcctgccgggagttttggccttggccatcagctgctcatcaaaacaattgatcctgtcgccgcagatgggaagtcccatccggcggcgacagggggaatggcaggagttgggggactcgaacccacgacccccggttttggagaccggtgctctaccagctgagctaaactcctagacaagaggcggccgtgaagccgttctcgccagaggggcgcgtatgccccaccccgctccgcttttcaagcgcgatgcgtcagcgcgggccgaacagacgcccgttgtgatgcacgaactcgcgcagggcgcccgtcaggacccagccctgctcgcccttcagataaatccagcctgcggccgcgccgacaagcgcgccgagacaatccacgatcaggtcccacatggtgtccaccaacccggacttctgcgtgttcgtgcctagggtctggtccgccgtgaactcgatgatttcccagaacacgccaatcgtcacagcgaagcagaaggcgaaaaaggcgacggtgatcggggctgcggtaagacgctcgccccgcacgagaatcagcatcagcaccacgccggccagaccaaaggccacggccgatccgatatgcagcacgatgtcccaccaccagaagcgttcatagaagtcccgcatttcgccgaggaacagagtcgccatcaggaacgccgcgatcgcaacgagaaagcccgatgggatatgcacgccggaaacgcgcccgacatacaacgggaccagggtcaggccgaaggtcgtcagggccacggcgcccacgatccattcgccattcagcagggcagcgcaggcttcgcccagcaagaggagccatatcagcttcaggggccagggctgctgcaacaggcgcatgggacatctccaattacgaaggccgctaacgccgtttcgcgtggtcagttctcgacgtgcgccgccactgcttccttttcgtcctcggccctgaccacctcgcggaagatcagcttgtcgatgcggcggtcgtccatgtcgatcacctcgacctcgaaccggcccacctgaagcacctcgccctcgtccggcacccgcgacagctggtgcaggatcaggccggccacagtgtggaagctttcgttctcgccgaagtcctcgccgagtcgatcgcacagctcgtccagatcggtgcggccgtccaccagccagctgccgtcctggcgctgggtgacatgggcgtgctcctcgtcgtggccttcgttgaagtcgcccgcgatcatctccaggatgtcggtcgcggtgaccaccccttcgaacgcgccgtactcatcgacgatgaaggccatgtggacgaaggaccccttcagtatctccagcgccttcagcaccgaggtggactgaggaatgaaggccggggtggcgatatgcgcctcgaccgtcagttctccggtggtcagcaaggcgtccagaaggtccttcttgtgcaccacgcccaccgggtggtcgagatcgccgtccctggccaccacgatgcgcgaataggggcacaggcgaatctcctcgcgcagcgtctcgggttggtcgtccagcgccacccaatacacatccgtgcgcggcgtcatggcgacacgcaccggacggtcgccgagacgcaggatctcctcgatcatctcctgctcttccggctcgatcagaccggccgacgtgccctcggcgatcatggtctcgacctcttcctgggtcacgtccgagccgtcgcgatccttgacgcccagcaccttgagaatgcccgaggtcgaggcggtcagaagcagcacaaagggcttgagcacgatcgccagggtcgagatcggtgccgccatcttggccgcgatcgattcgggaaagatcagcgccaggcgcttgggcaccagttcgccgacgatcagcgacacataggtgatgcagatgaccaccagggcggtggagaacacctccgtataagccgacagcgccggaaagctggtctccagaatccggtccagttcgcccgcgatcgccgcctgcccgtaggcgcccgccagaatgccgataagggtgatgccgacctggacggccgacaggaagtgggtcggttcctccgccagcttcagggccgcccgcgcccccctgtcgccccgctccgcccggctctgcaacctggacttgcgggaagacacgaccgccaactcggtcatggcgaacaggccgttgagcaccacaaggagcagaacgacgacaatggcgatgagtaacatctaggggttttgaaaccgacgcggcgcgacagccggcgtccgcagcgactatcttatgggatcacgcgcgcttgcgccacgatttcgtatcaggcgcctcggcccagatcgatggagccgtatccaccgctcgctccgtccgtccgatcgttcgccgacgcacaggcggacatgccgatcagggtgccgatgaacaggccgatgtggagcgcgcgccgcatgtctggttaccgaaagcttaacgttcagaaacgaacgtaagcggcgccgttcggttgcttgcaagcgctctcgcgccttaagcgaagatcagccgagcgcgtctttcggcgtcggataggacagaacgcagcgcacgccgggtttcgcgtcttccatgtcgaaccggccgccgagttggcccgccagcccctggacgatgcgcaggcccaggcttgcaggtcgtgacgggtcgaaatccggcgccaggccccgcccgtcatcgcggacggtcagccgacgtcgttcgtccgactcgccgaactcgatctcgatccggccttcgcgctcggccactccatgctccagcgcgttgttcacgcattccagcaggatcagcatgatcggggtcgcctcctccgccgtcagcgtcaactctccgccgtccagagccagggcgacatcctctcgtgcagcggcggccagggcgtcggcgcacagatcgcgagccaccgtttcgaatcgcgtggcccgaccttcggcgtcggagaggccgcgctgcaccttggcgatcagggccgtgcggctggccgcctcggtcaggatgcgacgcgcatcgccgtccttggccatgccggcctccagcctcagcaacgagctgaccacctggatgttgttggacacccggtgctggacctcgcggtagagcaggtcccgactctgggccagggcggcgctgcgcgcggcctcctcttccagcttgccgcgcgccgaggtcatgccgacgatgaagaagatgtcgaccgcgaccacgaaggcgaagaacaggagcgccacggccgtggccgcgctccagtcgaaacccggcgcgccgatccagaaccaccaggcgctgaggcccgacagcaccgccgtcaggaccgacggccacagccccgcgaaataggcggccaccaccacggcgggaaagaaggtcagatagggaaagcccggaggaaaccagtcggccagggctgcacgcagcacaaaggcggccagccacactccaagcgcaaagccgtagccgagcaacggccgcgttcgaagcatctccgccctcaagctgatgtaccccctgtatggttcagctttggcccatacggcgggagaatgcaaagacgaggctgatcagggattcgaggcgtccagaatggcgcgcgccagtccctccgcggtgatctcggcccagcaggcgtagccttcgtcgttcaggtgcagttcgtcgggtcccacgcctccgcccgccaggccgctccagtccctcatggcggcgaaccggcgcagcacggcgcgattcgccagcgccgcctgcgcctcgatcaccgaggcggcctgctccagagcgggattgcggcccgcaaaggcggggttacgagcgtcgtcaggcagacgttgcggatcgatcagcagggtgtccaccccggcgcgcgccagcaggtagtcgccccacagcaggtcccgcagaaaggcgcccggatcacggtcacgcagcacatcattggtgccgagttgccacagcaccagatccggctgggtcagttccagttcacggggaaggcgcttgaccgtatcctccgccgtctcgccgccgacgccgcggttgtagaccaccaccccgacctcgggcaggcgacgcttcagcgccgcctcgaggcggggaacaaagcccaggtcgggacggctggcgcccaccccttcgatggaggaggagccgacggccaggatcacgaggcgccggtccgcgatggcggcgcggctccgctgcaggccgccgttgacgatcacatggtccgccgagatcggacaggcggcgggaggcgcccagaccggctgaaccgccctctcatcgctcgcccaggcggcgccggtcaccgctccggtcgctgccgccgccagcagcgacgccaccaccctgctccacctgatcaccatcggtcctccgacatccctgcaacgcaaaacccccgccggatggctccggcgggggtgatgtttagcttaaagatcgatcgcgatcaggcgatgatcttggagaccacgccggcgccgacggtgcggccgccttcgcggatggcgaagcgcagcttctcttccatggcgatcggggtgatcagttcgacgttcagctcggcgttgtcgccgggcatgatcatctccacgccttccttcagctgcacgatgccggtcacgtcggtcgtgcggaagtagaactgcgggcggtagttggtgaagaacggggtgtgacggccgccttcttccttggtcaggatgtaggcttcggccacgaacttggtgtgcggggtgatggagcccggcttgcacagcacctggccgcgctcgacgtcttcacgcttggtgccgcgcagcagcacgcccacgttgtcgcccgcctggccctggtccagcagcttgcggaacatctccacgcccgtgcaggtcgtcttctggacggggcggatgccgacgatctcgacttcctcgccgaccttgacgatgccgcgctcgacgcgaccggtcaccacggtgccgcggcccgagatcgagaacacgtcttccaccggcatcaggaacggcaggtccaccggacgctcaggctgcgggatgtagctgtcgaccgtggccatcagctccagcacgcgctgctcgccgatctccgggttcacgccgtcggtcgcggccttggccgagcccttggtgatcggaatgtcgtcgcccgggaactggtaggacgacagcagctcgcgcacttccatctcgacgagctcaagcagctcctcgtcgtcgaccaggtcgaccttgttcatgaacaccaccagcgccggcacgccgacctgacgggccagcaggatgtgctcgcgggtttgcggcatcgggccgtcggccgccgacaccaccaggatcgcgccgtccatctgcgcggcgcccgtgatcatgttcttcacatagtcggcgtggccggggcagtcgacgtgggcgtagtgacggttttccgtctcatattccacgtgcgcggtgttgatcgtgatgccgcgcgccttttcttccggcgccgcgtcgatgtcctcgtacttcttcgccgtcgcgccgcccgacttcgccagcgtcatcgtgatcgccgccgtcagcgtcgtcttgccgtggtcaacgtgaccaatcgtgccgatgttgcagtgcggcttcgtgcgttcgaacttttccttggccattctctagctcctaggtccccgaaccgggggttcctgcagtttgggggtttaaggacgcccggccttgaaccggccgggggcttgtaggaccgcttctccgaaaggaaaagcttaggcgtacttcttgatcacttcgtcggcgacgtgctgcggcaccggctcatagtggtcgtactgcatggtgaactgggcgcggccctgcgacatgccgcgcagcgtgttcacatagccgaacatgttggccagcggcacaaaggcgttcacgacggtggcgttgccgcgcatgtcctgaccctggatcatgccgcgacggccgttcaggtcgccgatgaccgaacccagatactcttccggggtcacgacctcgacggccatgatcggctcgagcagcttgggcccgcccttttcccgcagttccttgaaggcggcgcgagaagcgatttcaaacgccagcaccgaggagtcgacgtcgtggaaggcgccgtcgaccagggtggccttgacgtcgatgaccgggaagccggcgagcaggccgttgtccttggccgacttcaggcccttttcgacgcccgggatgtattccttgggcaccgcgccgccgacaatggcggattcgaacacgaagtccgtgcccggctcgcccggctcgaacaccagcttgacgcgggcgaactgacccgtgccgccggtctgcttcttgtgggtgtagtcgatctcggccttgcggctgatcgattcacgataggcgacctgcggcgcgccgatggtggcctcgaccttgtaggtgcgcttcaggatgtcgatcttgatgtcgaggtgcagctcgcccatgcccttcaggatggtctggccggactcgtgatcggtcgagacggtgaaggacggatcctcggacgccagcttggccaaggccacgcccagcttctcctggtcggccttggtcttgggctcgacggcgatctcgatcaccggcgccgggaactccatgcgctctaggatgaccggcgacttcagcgggtcgcacagggtgtcgcccgtgcgggtgtccttcaggccggccagcgcgacgatgtcgccggcataggcttccttgatgtcctcgcggttgttggagtgcatcagcagcatgcggccgacgcgctccttcttgtcgcgggtcgagttcagcaggcccatgcccgtttccatcttgcccgagtacaggcggcagaaggtcagcgagccgacgaacggatcgtccatgatcttgaaagccagaaccgacagaggctcttcgtccgaggccttgcggaccacttcttcttcggtcttgtagtcgatgccttgcgtcggcgggatgtccaccggcgagggcagatagtcgaccaccgcgtccagcagcgtctgcacgcccttgttcttgaaggccgagccgcacaggatcggatagaaggcgccggtcagcacggccttgcggatgcacttcttgatggtctcttccgaaggctcgttgccctcgaggtaggcttccatcgcttcgtcatccagctcgacggcgttgtcgatcaggtactggcgcgcctcgttggccttggcctgcaggtcggcggggatctcctcgtcgcggaagttcgcgcccagggcgtcgttgtcccagaccacggccttcatgcggaccaggtcgaccaggcccgacaggttggactcggcgccgatcgggaactggatcggcacggccttggcgcccaggcggtcgcggatcgactccaccgacttgtcgaagtcggcgccgatcttgtccatcttgttgacgaacacgatgcgcggcacgcggtacttgtcagcctgacgccagacggtttcggtctgcggctcgacgccggcgttgccgtccagcacggtcacggcgccgtcgaggacgcgcagcgaacgctcgacctcgatggtgaagtccacgtggccgggggtgtcgatgatgttgaggcgcttctctttccagaaggcggtcgtcgcggcggacgtgatggtgatgccgcgttcctgctcctggtccatccagtccatggtggcggcgccgtcgtgcacttcgccgatcttgtgggacttgccggtgtaatacaggatccgctcggtcgtggtcgtcttgcccgcgtcgatgtgggccatgatgccgaagttgcggtagtcttcgattttatgcgtgcggggcattgtgcgtccctgtggggtgcgtgggcgggacgctcaggcgcccccggatatgtcggataagacagcgcgggcgatttaacggaaatcgcccgcgccggatagtctcaagatagcgacgccctatggcgctttgaagacgcttaccagcgatagtggctgaaggcgcggttggcttcggccatcttgtgggtgtcttcgcgcttcttgaccgcggtgccgcggttgttggaggcgtccagcagctcggccgccagcttctcggtcatggtgttctcgccgcgcttgcgggcggcgttgaccagccagcgaatggccagggcgcggcggcggtccggacggacctcgaccggcacctggtaggtcgcgccgcccacgcggcggctgcggacttcgaccgccggggcgacattgtccagcgcggcgtggaaggtggcgaccggctcctggtccttcttcttgtcggccaggatgtcgaaggcgccgtagacgatgttctcggcgacggccttcttaccttcgtacatgacgtagttcatgaacttggtgacgaccaggtcgccgaacttgggatctggcaggacgtcgcgcttctgggcgcggtgacgacgggacataggtgtatcctcttaaatctgactgggcgcgcgcaggcttacttcggacgcttggcgccgtagtgcgaacggcgctgcttgcggtccttgacgccttgcgtgtccagcacgccgcgcaggatgtggtagcgaacgccgggcaagtccttgacgcggccgccgcggatcaggaccaccgagtgctcctgcaggttgtggccttcgccggggatgtagcacacggcttcgtagccgttcttggccaagcggaccttggcgaccttacgcagggccgagttcggcttcttcggggtcgtggtgtagacgcgggtgcagacgccgcggcgttgcggcgaaccctcgagcgccggcaccttgttgcgggtgggcttgggcttgcgcggcttgcggatcagctggttgatcgtgggcatggagactcgtctcgacttctgatggaggcgtgtgcctttcggccggggcgcctcatggaccttcttttggacggcgcgggccgcccgggctgctgtcgagaccggagcgcggcgcacaaacagaaaaaccggaacgcgcgctttgggcgttccggcgggacacagcccgtccgttcgattgtcacgatcccggaagacggcgaaccgcccatcctcgaaagtgggcggcttctacgtccgatctcgcctcccgtcaagggacgccgctccatgcggccccgcctgaaagtcgccgcacttgccgctcagcttgcctgtgagggagaacgcatggcggctctggcggcggataccggcggcctggatgggcgcaagctgtcgatggcggcgctggccctgtgcctcaacgtcggcatgatcggcctgctgtccgtggcgaacctgggcgaacgggctcagcggtccggcgcatggacaccgcccgtctatctcgacatcgagccgcgtctgctgctgcctgacgagcaaccccgaccggcgacctcgttggttcaggctccgaccacgcggctcgtcacaacgcggggtcgcgcctcttccgccgccgcctcttcgtccacgccaacccagagcgacgctccgccctcccctcccgcgccgcggctggccacgcctgcgccgcagggaacccctgcgccgagcagcccctggaccgtgcagccgaacggcggggcctttgcgcgatcgccgcggcaaggtcccgtgggctgcgcctcgccgcagctgttgaacgacgccgatcgcgccgcctgtcggcgggacttcaacgagcgggcggagcgcgcgccgccgctggacggctcaggcgacgctcgccgcgactcccgcttcgcccgcgagggcgcgcgcaagcttcaggagtacgaggcccggcggcggccgttgtccggcggcatcggcaacgtcggggtgcaggagggcgtcggctccaacttcggcatcggcgtcgcgggcgcgcacctggacccgtctttaaggcccgactccacccggaacatccagacgcgccgcgacggtccgcccgcgtccggggccccgctcgttcccggctcgaccggcccggggcgcgagccgagataggcggtcgacacggaaaaggcggcgctgatctccagcgccgccccttcagttcagacgatcctgagccgatcagctctggtcggccaactccagctgcaggtcggccggcagcggctcgatggagtcttcgcgcgcttgcgtgaggaccgcatcgcgctcgttggcgatcttctgcagcgaccgcagataggcgcccgtgcccgccgggatcaggcggcccacgatgacgttctccttcaggccttccagcatgtccttcttgccgtggaccgaggcgtcggtgaggacgcgggtggtctcctggaaagacgccgccgagatgaagctgcgggtctgcaagctcgccttggtgatgcccagcaggaccggctgcgtggtggccagacggccgccgcgcttctcgaccttggcgttctccagcgcggcctcggcgacctcgaccgtgtcgccacggatcagcgtcgtctcgcccgcgtccagaacctcgaccttttgcagcatctggcggacgatcacctcgatgtgcttgtcgttgatcggcacgccctgcagtcgatagacctcctgcacttcgttcaccaggtattcggccagcgcctcgacgccctggatgcgcagcagatcgtgcggatccgggttgccgtcgatgatgtagtcgcccttctggatcagatcgccgtcgtggacggagatgtgcttgcccttggggatcaggaactcgaccggctcaggctgcacgccgtcggcgttgacctcgggcgtgatcttgatgcggcgcttgttcttgtagtcgcggccgaattcgacgcggccgtccatctcggcgatgaccgcgcagtccttgggacgacgggcttcgaacagctcggccacccgcggcagaccgccggtgatgtcgcgggtcttggcgccttcggtcggaacgcgggcgatgatctcgcccggcttgacctcgtcgccgttcgacacggacagaaccgcgccaaccggcagcaggtagcgggcgtcggagcccgaagccagcttggcgtaggcgtcgccgttggtgacgcccatggccggacgcaggtccgatccgcgcgggctggcgcgccagtcgctgaccacgcgctgggcgatgccggtcgcctcgtcggtttcttccttgaccgacaggccttcgaccaggtcctcgaagcgcaccacgccgccgacttccgtcaggatcggggtggtgtagggatcccattccgccagacgcatgccgcgcgtgacctcggcgccgtccttgacccggatgcgggcgccgtacggggccttgtgcgtttcgcggtccttgccgtccacgaccacggtgaccacgacgttgcggctcatcgccaccaggtcgccgtgggccgcgaccacggtcgggcccgtcaccttggccgtaccggcgttggtcgcctccatgaaggaggtctccgcgacctgcgcggtgccgccgatgtggaaggtccgcatggtcagctgggtgcccggctcgccgatcgactgggccgcgatgacgcccaccgcttcgccgatattgacgttggtgccgcgcgccaggtcacggccgtagcagtgtccgcagatgccggcttccgcctcgcaggtcagggccgaacggaccttcaccgactgcacgcccgccgcctcgatcgcctcgacctcttcttcctgcagataggtgtccgcggggaagacgatggtgtcggtgcccggctccttgatgtcctcggcggcatagcgacccaagacccgctgtccgagcgagaccagcacgtcgccgccttccatgaccgcgcgcagggtgatgccgcgcgtggagccgcagttgtcctcggtcacgatcgagtcctgcgccacatccaccagacggcgggtcaggtaacccgagttggcggtcttcagcgcggtgtcggccagacccttgcgggcgccgtgggtcgagttgaagtactcgagaaccgtcaggccttccttgaagttcgaggtgatcggcgtctcgatgatctcgccggacggcttggccatcagaccgcgcatcccgcccagctgcttcatctgggcctgcgaaccgcgggcgcccgagttggccatcatgaacaccgagttgatgtccgggttctcgccttcgatcaggacgcgcggctgagcgatctcgcccatcatcgcgtcggcgatcttgtccgtggccttggcccaggcgtcgacgaccttgttgtacttctcgccgcgcgtgatcaggccgtcggcgtactgttgctcgtactcctcgacctgggtgcgggtctcctcgaccatgccggccttggccgccgggatcacgatgtcgtccttgccgaacgagatgcccgccttggccgcctcgcggaagcccaggcccatcatctggtcggcgaagatcaccgtcgccttctgaccgcagtggcgatagaccacgtcaatcaggttgccgatctccttcttggtcaggttcttctcaagcaggcggtagccgacgttcgggttgcgcggcagcagggcggccagcttcatacggcccggcgtggtgtcgatgaccttggtcacctccttgccttcggcgtcctgctcggtccagcgcgccttgatgcggctgtgcagggtgacgaccttggcgtccagcgccgcgtcgatctcgccgatattggcgaacagcttgccctcgcccggctcgccgtccttgaccagcgacaagtagtacagacccagcacgatgtcctgcgacggcacgatgatcggcttgccgttggcgggcgacaggatgttgttggtcgacatcatcagcacgcgcgcttccagctgggcttcgaggctcagcgggacgtgcacggccatctggtcgccgtcgaagtccgcgttgaaggccgtgcagaccagcgggtgcaggcggatggccttgccctcgatcagcttgggctcgaacgcctggatgcccagacggtgcagcgtcggcgcgcggttcagcagcaccgggtgctcgcggatgacctcgtccaggatgtcccagacctgcggctgctcgcgctccaccatgcgcttggactgcttcacggtgcccgacaggcccttggcgtccagacgcgcgtagatgaagggcttgaacagctccagcgccatcttcttgggcaggccgcactcgtgcagcttcagttccggacccacggtgatgaccgaacggccggagtagtcgacgcgcttgcccagcaggttctggcggaagcggccctgcttgcccttcagcatgtcggccagcgacttcagaggacgcttgttggcgccggtgatgacgcggccgcgacggccgttgtcgaacagggcgtcgacggactcctgcagcatccgcttttcgttgcggatgatgatgtccggcgcccgcagctccatcaggcgcttcaggcggttgttccggttgatgacccggcgatacaggtcgttcaggtcggacgtggcgaagcgaccgccgtccagcggcaccagcggacgcagctccggcgggatgaccggtacgatggtcaggatcatccactcgggcttgttgcccgattccaggaacgcctcgatcagcttcaggcgcttggacgccttcttggccttcatctccgacggattgtcggccagctcggcgcggtgcttttcggcctccgcgttcaggtcgatgcccatcagcaggttgcgcacggcctcggcgccgatctcggcggtgaagccgtcatcgccgtattcgtcctgatagcggtagaactcgtcttccgtcagcaactggttctgcttcagcggggtcaggcccggctcggtgacgatatagttctcgaaatacaggacgcgctcaacgtccttcagcgccatgtccagcatcagcgagatgcggctcggcagagacttcaggaaccagatgtgggcgaccggcgcggccaggtcgatgtggcccatccgctcgcggcggacgcgggccagggtgacctccacgccgcacttctcgcagatgatgcccttgtacttcatgcgcttgtacttgccgcacaggcattcgtagtccttggtcgggccaaagatacgggcgcagaacaggccgtcacgctcgggcttgaacgtgcggtagttgatggtttccggcttcttgatctcgccgaacgaccacgaccggatcttctccggcgaggcgagcgcgatcttgatctggtcaaaggtcggggtgaccgggaccgggttgaagatgttcaggacgtcctggttcatcttggttccttctgcgggctgttccctagatgggggccgcgaaaactatttcgagtggagagcgcgtgagggaagcgcccttccccgctgtggcgcgaggaagggcccggcttcggtcagctgttctccagctccacgttgaggcccagcgagcgcatttccttgacgagcacgttgaagctctcaggtatgccggcctcgaagctgtcgtcgccgcggacgatggcctcgtagaccttggtccggccggccacgtcgtccgacttcaccgtcagcatctcctgcagggtgtaggcggcgccgtaggcttccagagcccagacctccatttccccgaagcgctgaccgccgaactgcgccttgccgcccagcggctgctgggtgaccagcgagtacgggccgatcgagcgggcgtggatcttgtcgtccaccaagtggtgcagcttcagcatgtagatgtagccgaccgtgaccggacgcttgaactgctcgccggtctggccgtcgtacaggatcgactgtgccgacttgtgcaggccggcttcctcgagcaggcgctcgatgtcgccgatgtgcgcgccgtcgaagaccggggtcgcgaagggcacgcccttggacaggttcttcgccagctcgatcagctcctcctcgtcgtccggaagcggcgtctcggggccgtagatctcgcccaggcgctggaccagggcttccttctggccgccgtgttgccacgcctccagcaggcccgagatctgcttgcccagaccggccgcggcccaccccaggtgggtctcgaagatctggccgatgttcatgcgcgacggcacgccaagcgggttcagcacgatgtcgacgtgggtgccgtcctcaaggtgcggcatgtcctcgatcggcaggatcttggagatgacgcccttgttgccgtgacggccggccatcttgtcgccgggctgaagcttgcgcttcaccgccacgaagaccttgaccatcttcatcacgccggggggcagttcgtcgccgcgctgcagcttctcgaccttgtcctcgaagcgacggtcgagttgtttgcgagcatcctcgaactgacgcttcatggcttcgagctcgcccatggcgcgctcgtcgtccagggcgatctgccaccacaggccgcgcgaaacctcgcccagcttggcttcggtcagctcgccgcggcccagccccttgggacccgacacggcggtcttgccgagcagcagcggcttcaggcggccgtagacgttgcgctcaagaatcttgagctcgtcgtcccggtccttgcccagacgctcgatctcggcgcgttcgatggccatggcgcgctcgtccttgtcgacgccatggcggttgaacacgcgcacgtcgacgatggtgccggcgacgcccggcggcaggcgcagggaggtgtcgcgcacgtccgacgccttttcgccgaagatcgcacgcagcagcttttcttccggcgtcatcgggctttcgcccttgggcgtgaccttgccgaccaggatgtcgcccggctggacctcggcgccgatcgccacgatcccggcctcgtcgaggttgcgcagggcctcctcgccgacgttggggatgtcgcgggtgatctcttccggccccagcttggtgtcgcgggccatgacttcgaactcctccaggtggatggaggtgaagacgtcgtcgcgcacgatgcgctcggagatcaggatcgagtcttcgaagttgtagccgttccagggcatgaaggcgacgagcgcattgcgacccagcgccagctcgcccaggtccgtcgacggaccgtcggcgatgacgtcgccggccttgacctggtcgcccacgcgcacgatcgggcgctggttgatgcaggtggactggttggagcgctggaacttcgacaggcggtaaatatcgacgcccgagcgggcggcgtccacgtcgccggtggcgcgcaccacgatgcgggtgccgtcgatctgctccaccacgccgtcgcggcgggcgacgaccacggcgccggagtcgacggccccgaccgcctccatgccggtgccgaccagcggcgcgtccgactgcaccagcggcacggcctgacgctgcatgttggcgcccatcagcgcgcggttggcgtcgtcgttttcaaggaaggggatcagggccgcggccaccgacaccacctgcttgggcgacacgtccatcatgtccaccgccgacttggtcagcagctgggattcgccgttgatccggccggggaccaggtcctcgacgatctggccgtccttcagctcgatgttggcctgggcgatggtgaagcgcgactcctccatggccgagatgtagaccacctcgtcctgagcctggccgtccttgacccggcgataggggctttcgatgaagccgtacttgttgacccgcgcgtgggtggccagcgagttgatcaggccgatgttcgggccttccggcgtctcgatcgggcagatccggccatagtgggtcgggtgcacgtcgcggacctcaaagcccgcgcgctcgcgcgtcagaccacccgggccaagcgccgacaggcgacgcttgtgggtgatttccgacagcgggttggtctggtccatgaactgcgacagctgcgacgagccgaagaactcgcgcacggccgcggccgccggcttggcgttgatcaggtcgtgcggcatgaccgtgtcgatgtcgaccgaggacatgcgctccttgatggcgcgctccatgcgaagcaggccgacgcggtactggttttccagcagttcgcccaccgaacgcacccggcggttgcccaggttgtcgatgtcgtcgatctcgccgcgaccgtccttcagcccgaccaggatctgcaggaccttgagcacgtcgtccttctgcaggacgcggatctcgtcggagacctccggcgtctccagacgcatgttcatcttgacccggcccacggccgacaggtcgtagcgctcgctgtcgaagaacagcgacttgaacatggcctcggccgcctcgatcgtcggcggctcgcccggacgcatcacgcgatagacgtcgaacagcgcgtcctcgcggttgtcgttcttgtccacccgcagggtgttgcgcatgtaggcgcccaccgtgacgtggtcgatgtccagcgtctcgatggtggtgaagccgttctcttccagcagggtgatggtggcctggtccagctcgtcgccggcctcggcgtagatctcgcccgtctcgaagttcaccgcgtcattggcgaggtagcgcgtcagcagcgcgtcggccgccagcgacagcgactgcaggccgttgtcggccagcttcttggccgcgcgggcgctgatcttctggccggcctgggcgaccacttcgccggtgtcggcgtcgatcaggtcgaactcgggcttcaccccgcgccagcgttccggcttgtagggcgtgacccagccttcgccgcgcttttcatacggcacggtctcgtagaaggtcttcaggatctcctcgccgtccatgcccagacccatcaggaaggtcgaggccggcagcttccggcggcggtcgatgcggacatagacgatgtccttggcgtcgaactcgaagtccagccacgaaccgcgatacgggatcacccgcgcggcgaacaacagcttgcccgagctgtgcgtcttgcccttgtcgtgatcgaagaagacgcccggcgaacggtgcatctgcgagacgatgacccgctcggtgccgttgacgataaaggtgcccttgtccgtcatgagcgggatgtcgcccatgtagacgtcctgctccttgatgtccttgaccgaacgggcgcccgtctcctcgtcggtttcgaacacgatcaggcgcagcttgaccttcagcggcgcggcataggtcatgtcgcgctggatgcactcctcgacgtcgtatttgggctcttcgaactcgtaggagacgtactcaaggattgcgcgctcgttgaagtccttgatcgggaacaccgacttgaacaccgcctcgacgccctcgtcgcgacgctggcccggacggacctcacgctgcaggaactgttcgtaggaggcccgctgaacctcgatcaggttcggcatctgcaccgcttccgggatgcggccgaacgacttgcggatgcgcttcttgccggtgaacgaggtggcggtggcgacctgaccgttgatggcgagaccgtgggcgacgtcagtcattcaatgtttcccaatccgcgaaggcctgggcggaccctcgcgtcaaatgcggcggccacggcccgccttcggcgtccgcagccttgtttcttcggcgtccgccctcggccggatcacggcctggacacctcaaatgaaccggctcccttgggaaggagccgcgccttcgcaccggtcggagggcgacgaaccgggcctcggcgcttgcgcgcagactcgtggctgagtgttgcggaaggcggacttatactcgcttccttgacgaaataaaggcccgcgcggaaccttttacacggtgacgaagcagcgccgttcctctcatcccatggctgcgcgtgaggcaggagaaggcgcggctggacggcggcctggcgtagccgtaagccttgtccatgacccgcatcgccctggccgccctgtccgctctctcgctcgccgcctgcgcgcaccgcgagcccgtgtcctatcccgagacccagttggcggccgcccgcgccgcggacaatgtcgcgacgcccgggacgcaggaaggctgggacgccggcaacgccgcctatctggtctggagcggtgcgcggcgcggctggaccaccaccgagagcgggcttcagtatcgccgcgtcggcaaggcgcatcccgagggcgcgcagccgacggcgaccgacacggtacgggttcactaccgcgggaccttcatcgacgggcgggagttcgacagctcctacgcccgcaacgagccgggcgagttcccgctgaaccgcgtcatcaagggctggacagaaggcgtcgccttgatgcgcgagggcgagacgttcgagttcgtcatccctgcttcgctgggctacggctcgcgctgggtcggcggcgacgaactgcccccgaactcgacgctgctgttcaccgtcgaactgctggacgtgaaaccggcgacctgagagccagggcctctgctcgcagccgcttttccaccagccccatcgaacttgccccagcgttaaccaccctgtggtgtggacaccctgaccgacgccctccatcgtcgggtgttcgcggtgccccctccccctgaagcgcgccgctgcaaggatgccgatgccgcgctacttccttcatctccgccggggcgaagaggcgttcctggacgccgagggttcggagttctccgacctggaggcgctccggcgcgctgcgctccatgacgctcgcgacaccatgtcctgggacatcaaggagggccggctggacctgagctttcgcatcgaggcggtggaccagtccgggcgcacggtgctgtcgctgggcttcgatgaagcggtgacgatcacccagccagaaaggcttcggcgcggaggctgacgcttcgccgcagcacggaaccgcgcccgcctgcccgcgcttcggccgtcatgacacatcgcctctccatcgccgccgccctatccttcgccctgctgtcggcgaccgcggcgtccgcccaagatcgaccgacctacggtcctcgcctggagggctacgcctatcctcatcccgtccagagcttcgccttcacctcccagcgccagccgctggagatgacctacatggacgtggcgcccagcggaccggcgaacggccgcacggtggtgctgctccacggcaagaacttctgcgccgccacctgggcgccgacgatcgaggtgctgtctcaggccggcttccgcgttctggccgtcgatcaggtcggcttctgcaaggcgtccaaaccgcaaggctaccagttcagcctgccgcagctggcgacgaacacccgcgccctgatggcgcatgccggcgtagaacgggccgtgatcgtcgggcattcgatgggcggcatgctgggcgcgcgcttcgccatccagcatcccgaagcggtcgagcggctggtgctggtcaacccgatcgggctggaggactggcaggccgagggcgtgccctacgccccgctcgacgccgcctacgagaccgagcgcaagaccagcttcgacagcatcaaggcgtatcagcgcaagttctactacgacggcgactggaagccggagtacgatgcccccgtcgagatgctggcggggatgtatgcgggcccgggcggcgacgccgtcgcctggaaccaggcccagacctccgacatgatcttcacccagccgatcgtgcacgaactcggcctcatctccgcgccgaccacgctgatcataggccagaccgaccgcacggcgcccggcgcgaaccgcgcatcaccggaggttcaggcgcgcttgggcgattattccgcgctcggccgccgcaccgccgaggccgtgccgaacgccaggctggtggagttcgaagatcttggccacgcgccgcagatcgaggatcccgaccgctttcatcgcgcgctgctggacgcgctcgccgactgacgcttgactgcgggaggcctgcggcggagggtcgcaccttcccccagcccccgcggagcccgccttgtttcctgcccgtctcgcgctgcttggcgcagccagcctgctcgtcctcgcctcgctggggccgccggcggtcgcccagcaggccgctgcgccggcccccgccgtcgccggcccagccctgcccatcgcgctgccgccgctgccacaggtgcaggacgcgccctggcctggggtggtgcggctgcgggtcgacgccaccgacctgaaccgccgcatcttcgacgtcaccgagaccatcccggtggagcgtgcggggccgctggtgctgttcttcccggaatggctgcccggcaaccacgggccggtcggccccatcgcccagctcgcggggctcgagatcaccgccaatggccagagggtggagtgggtgcgcgacaccctgcaccccttcgcgttccacctggaggttccgcagggcgccagcgagatcacggcccgcttccagcacctgtcgcccaccaccggcagccagggtcgcgtcaccatgacggccgagatgctgaacattcagtgggaaaagatgctgctctatcccgccggccgctggtcgcggaacatcacggtccaacccagcgtcaccctgcccgacggctggcgcttcggcacggcgctggagccggaaaccgcgtcgggcgccgtcaccaccttcaggcccgtaaacctcgaggtgctggtcgacagccccatgttcgccggcgtccactatcgccagatcgaccttgatccgggcggccgttcgcccgtgcgcgccaacatcgtcgcagacaagcccgagagtctcgaagccaccgacgagcagatcggcattctgcgcgatctgatcacccaggccgatcgcctctatggcgcgcgccacttcgatcattacgaattcctgatcgccatgaccgacaagctgggcggcattggtctcgagcatcaccgctcgtccgagaactcggtcgatcccgagttcttcaccggatgggccacccacgtcggcgaccgggacctgctggcgcacgagtacaaccactcctgggacggcaagtggcgccgcccggccgatcagctggtccccaacttcaacaccccgctgcagaacagcctgctgtgggtctatgagggccagactcaatacttcggccaggtgctggccgcccgctcgggcctgaccagcaagcagcaggctctggacagcctggccatgacggcggcgacctttgacacacgcgtcggccgccagtggcgggcgctgcaggacaccgccaatgatcccatcatcagccagcgccagcccaagggctggctgtcgtggcagcgggacgaggactactattcggaaggccagctgatctggctcgacgtggacaccctgatccgcgagcgcaccaacggccgcaagtcgctggacgatttcgcccgcgccttcttcggcgtcgaggacggcgactacacgccggcaccctacaccttcgaggatgtggtccgcaccctgaacggcgtggtcccttacgactgggccgacttcctgcgcacccgcctggacggtcacggacccggcgctccgctggacggactcgcgcgcggcggctaccgcctcgtctacgccgagacgcccagcgactggcagaagaccctgtatggcgaatacaagcgcaatgacttcacctactcgctgggcatccagaccggtgagggcaatgtgatccgcagcgtccagtggaacagccccgccttccaggcggggctcgccaccggcatggagatcgtcgccgtgaacggaagggccgcgtcgcccagcgccatctcggaggccatcaccgccgccaaggacccgaacacagccgtggagctgatcctcaaggacgccgaccgctaccgcaccgtgcgcatcgactaccacgacggcctgcgctacccgcggcttgagcggatcgccggcacgcccgaccgtctgggcgacattctgacgccgcgccggcgttagacgattgcatcatcgaccttgacgcaagggaggcgcgcggccgaggttgcgcgcctctctttttgtccggactcatcgatgacgcgcactcgcctgaccgccgcctgcctcgccctgctgatgaccagcgtctgcggccccgcgctggcccagcagcagccgaacacggcggacgtcatcgcgccggcggccctgccgcgcgcggttccgccgatcccggccccgaccagcgccgcctaccccggcgtaatcacgctgaacgtcgacgcctcggatgtcgagcgcggcctgatcaacgtcacccagaccatcccggtctcggccgggtcggtcaccctgctctatccgaaattcctccccggcaatcacgcgccgaccggccccatctccatgttgaccggcctgacggtcgccgccaacggtcagccgctgcaatggctgcgtgatccggtcgatccctgggccttccatgtcgaggttccgcaaggcgcgacccagctcgacgtcgccttcaccaccctcacgcccacgggcgagggccaaggccgccggctgcagacgcccgagatgctgaacctgcagtgggagaaggcgctgctctaccccgccggctacaacgccaagggcgtggccgtcgtccccagcgtcaagctgccggccgggtggcgctacggcgtggcgctggagaccgcgtcgttcgaaggcgacctggcgcgcttcgcccagaccgacctctacaccctggtggacagccccatgttcgccgggatcaacttccgcgagatcgcgctcggcggcggcgaccgggccgtgcgcgcgacggtggtggcggacaagccgaaccagctggagggcggggcgaaccgcgtcgagcagatggaatccctggtggtccaggccgatcgcctgttcggcggccagcgccacttcgaccactacaccttcctggtcggcgtcaccgacacgctgggcgacatcgggctggagcaccatcgcagttcagagaacacggtcgccaccggctacttcaacggcgaaggccgggtgccctacggcgatttggcggtgatcccgcacgagtacgtgcactcctggaacggcaagttccgccgcccggcggaccagatgttccccaactacaacgtccccacgaccaacagcctgttgtgggtctatgaaggccagacccagtactggggcgatgtgctgaccgcgcgctcgggctttgtctccaaggacgaggccttggcggtgctggcgggcgtcgccgcctcctaccagaaccaggcgggtcgtcagtggcgccctctgcaggacaccaccaacaccccggtgatgggctatcgcgcacccaatccctattcgacctgggcgcgcggcacggactactaccgcgagtccggcctgatctggctggacgccgacaccctgatccgctcagagaccaacggccgcaagtcgctggacgacttcgccaagcgcttcttcggcgtcacggccgacagctggtcgccgcaaggctatgcgttcgaggatgtggttgcggcgctcaacgccgtgcatccgcacgactgggcgaccttcctgcgcacgcgactggacgccgtgaacgcccctcccttcctggatgggctggagcgcggcggctaccgcctgacctacaccgatgcgccgtcagacgccgaaaagaagatcaattcgagctgggagaacgacttccagtactcgctgggcttctcgctggcgggaccctccaaccgcatcaccggcgtccgctggggcggcctggcgtttgatcagggcgtgggcgcgggctgggagctggtggccgtcaacgacatggccgcctcgcccaaggcgctgcgcgacgcggtcaccgccgccaagggcggctcggagcccattcgcctgatcctgaagaacggcgagcggttccgcaccgtggcgttcccctatcacgacggcctgcgttacccccggctggagcgcatcgccggatcgcgcgaccacctcggcgacattctggctccgcgtcgtcgctgatgacggccgtcgccttgcgcctgctgcccgcgcttctgctgctcctcctgtggggcccggcggcggcgcgggcggcgtgcgatctcggacagcctgcggtgacgcagcgggtggagatcggccgcaccggccgctccatgctgctgcacctgccacagggtttcgatcgggcgacgcccgcgcccctgatcttagtgctgcacggaagcggcggaagcggcgccgacatcctgcgcgactcccgcatggccgaaacggccgaccgccacggcttcattgtcgcggcgccggacgccggcatcccagtcgagcgcggcttcgtctggaacatccccggcgtgcccactgtcaccggcgaggttcccggccccacagacgccgatgatgtggcccacctcaaggccgcgatcgacgatctggcggcccaagggtgcgtggacccggcgcgcgtctacgtcaccggcctgtccggcggcggacgcatggcgtcctggctcgggtgcgtcgccgccgaccgcttcgccgccatcgcgccggtggtgggcctgcgcgccggcaacccggacgaagaagacccctcgcgccccgatccccgcacctgccgcccctcgcagcccgtgccggtaatggccttcgccggggacatcgacaccaccaatccgatcaacggcggcggcgcgggctactggcgatacaccatgcacgccgccgaacagcgctgggcccagctgaacggctgcacggaagtccgtcccacccgatggatcagccccacgatctatgaggaaggctacaccgcctgccgctccgccgccgacgtcctcgcccgcatcacccacggcggaggccacagctgggtcgccgacaacgacgccatgtgggccttcttcgcccgacgtgtgcgggagtgatggcggctgtgggcggcgaaggagacgctgttgttgatgtctcttaagggtagataccgttgaaaaagtcggcaattgccacgggcggcgagtgctgattcactctggtcattgaggctggaggcagcgcgatgatgggcgagcggcgggtcgatcaggcggccctgttctatactttctcgctggaagaccacgtccctgcgaaccatctgctgaggtcgatcgaccggttcgtggagttggaaggtctgagagggcatctggcgccgttctacagcgccatgggtcgcccctcgatcgaccccgagctgctgatccggatgctgctggtcggctattgcttcggcattcgctcggagcgtcggctgtgcgaagaggttcacctgaacctggcctaccgctggttctgccggctaggcctcgaaggtgccgtgccggatcattcgaccttctccaagaaccgccacggccgctttcgcgacagcgatctgctgcgccagttgttcgacacggtgctgcgccgctgcatggctgaaagcctggtcggcggcgaaggctttgccgtggacgccagcctgatcaaggccgaggcgaaccgggaacgcagcgtgcctggcgatccgggccttccgcccgaggcgtcgagccgggccatcgacgagtatctggcggtgctggacgacgcggcgttcggtgcggctactccggtgacgcccaagttcatctcgccggtggatccggcagcgcgctggaccgccgccaacaaggggccggccttcttcgcctatgccaccaactacctgatcgacctgaagcacgccgtcatcgtcgatgtcgaggcgtccaccgccgtgcggccggctgagctgacggcggcccgcaccatgatcgagcgggttcaggataggcatgatctccaccccgaccgccttgccgctgacaccgcctatggctcggccgagatgctggaatggctggtcaacgaccaggggatcgcaccccacatcccgatcatcgacaagtctggccggacggacgggaccttctctcgagccgacttcacctatgatcccaccgccgacctttatcgctgtccgggcggcaaggcgctgaagcagtatcggcgtgccttccgagccgatcatcccgagacgccgccggatgacacctatcgctatcgcgcctccaagatagactgcgacgcctgcgctctgaagccgcgctgctgtcccaacacgcccgcccggaaggtcacgcgctcaatccacgaaggtgcgcgggacttcgctcgcgacatcgccaggaccgacgcctacgtcgtttcacggcgcgagcggaagaaggtcgaaatgctgttcgcccacctgaagcgcatcctcaggctggaccgactgcgtcttcgtggtccctgcggcgcccgagacgagttcctcctcgccgccaccgcccagaacctgcgcaaaatggctcgactgatcccgcaaccgaccgctcccacgcccgcctgaaggcctgaagcgtcacgatcccatcacagcctgaccacgcagccgtgctgtcccgtcagccatccgactttttcaacggtatcggtaggaagcggacattagccgccgaataggccgtcgacgaagccttgtccaagccttacgagcagaaaggccgataccagatacacggcgacatgagtggctattttcacagaacgaagcgcgacgcggaacccagccattctcaaccctcaagtgagatgctcatgattaacgaagatcgcgttgcgcgcaatggattgaacgcatcctggcaccctcctcgtaagcagccgtcgtcgagggatcgcaacgggtcgaaagcgccttttgatgtgcggaccggaagccgacatcgcgtcaccggcatgggtcaccgaaggtttcgactgccgcccacggcctaaagcagggaagacgtaataggaccaaacaagaaagccccggaggtttccctccggggcttcttgatcttcagcagtgccgaaggtgtcggtcttacttgacctggaccttggcgccggcgtcggtcagcttcttggcgatctcgtcggcttgttgcttggagacgttctcgacgacgttctgcggagcgccttcgaccaggtccttggcttccttcaggcccaggtccgaacggacaccgcggacttccttgatgacgttgatcttcttgtcgccgccgtcgaccaggacgacggtgaattcggtttgctcttcggcggcttcagccggagcgcccgcgccgccgccggccggcatggccatggcgacaggagcagcggcggaaacgccccacttttcttccagcagcttggagagttcagcggcttccagaacggtaagcgcggacaggtcttcgacgatcttagcgaggtcggccattgtcagttttccttcggaggatgaggttcagagagtgcagagatgaaagacgggtccgcttacgcggcgtccttggtggcgtaggcgttgaacacccgggccaattgaccggcgggcgcttgaacgacggcggcgatcttggtcgccggggcgttgagcaggccgatgagctggctgcggatttcgtcgagggtcggcagcttggagagagcctccacgcccttctgatcgacgacggtggcacccatgaagccgccaacgatcttgaagcgatcgttggtcttggcgaaatcggtgacgaccttggcggccgtgccggggttttcggcataggcgatgcccaccggacccttgaacagggggtggtagtcgctgccgtcctcggcctcgagcgccttcagcgccaggcggttcttgaccaccttgaacgcgccgccttctttgcgaagacggccacgcagatcttccatttccgcaacggtcagacccaggttgtgggtcacgaccacggagccggcgtcggcgaagacgcccttcagcgtctcgatcgactcggccttttgagcgcggtccattgcggtctccagttcagtattcgccgccgggcggattcccgacgacgtgtgtggccttccgctcccgcatcgctgcgagggcatcggccggtcgtattgtccgaaggatgcaaaccgactgaggtgtccgtcccggatcacgggccacacatccgccagggtcgcgtccccatctccccacggcgtcagagggctctctgacgattatgaagcgggcggcccccgctccccgaagttctcggacaggaccgtcaccggaatgaaccgacgacgggaagcggcgctcttacagccacacgtccgcacatgcaagtgtgcggaaccgtgacgccagcggctcattctctagggcgacgcttaagagggctggcatgaccactatcgacgacgccgtggacgaggtgcgcgaccgcgccgtggacttcctgaacagcgaaggccgctcgacaacccacgtggccacgggcatcgccatcacggcgggattcgccatcctagccacgctgctggccacccaggcgatcaagccgccgacgaccaagctgaagcacctgcgcaagaacgccaagccgacgaccgaacgaccgaaggggccgctcagcatgatcctgccggcggggttctccgccactaccctgtcggcggtgcgggtctggaacgcgccggatcggccggagcgacgcagcgccatgggcctgtgggcggcggcgcaggcggtgaacgccgtgtggctggcctatcgcccggcgacgttggcggtgcaggtcgcggccgccatgaccagcgcgggcctcgccgctgccttcgcccacgaggcgcgcaagctggacgagttggccggcaagctggccgcgccgcgcggcgccggtgtcgccctggccaacaaggctgacgacgcggccaattgatcgcaggcgagcggctccagcggggccgccttgccctttgacagggcttcctctagggatcgcggccgatttgacgcgccgtcgcgacgacgggcgcgcgcctcttcttttcccgatgtgaccccatgaagatcaacggcaacaccatcaagcccggcatggtcctgcaagtgaacggcggcctgtgggtcgtcaccaaggccagccacgtcaagcccggcaagggcggcgccttcgccaacgtcgaggccaagaacctcgagaccggcaacaagctgaacgagcgcttccgctcggaagacaaggtcgagcgcgtcaccctggagcagaaggactattcctacctgttcgacaacggcgacagcctggtcttcatggacgatgcctcctacgaacagatcgagctgcaaaaggactgggtcggcgatgaccgcatcccctatctgcaggaaggcatgaaggtggtgatcgagagccacgaggatcgcccgatcggcctgtccctgcccgaccaggtcgtgctggaggtcgccgagaccgagcctaccgtgaagggccagacggcgtcctcctcctataagcccgccaccgcctccaacggcgtgcgcatcatgatcccgccctatatgtcggccggcgagcgcatcgtggtggacaccgccaccggcgaatacatccgccgcgcggactaagacgcacccgcctctcgcgaggcctctaccccttcttgaacttctccgcatgtccgggctgagcgccttgcaaggacatgcggaccaggagatttcgccatggctctcgcttccgccctgctgcaagtgatgatcgacgcggtccgcaagaccgcccgcccgatgctgcgcgacttcggcgaagtgtcgcagctgcaggtgtcgcgcaaaggccccggcgatttcgtcaccgccgccgacctgaaggccgagcagaccctgttcgaactgctgaccaaggcccgccccggctacggcttcctgggcgaggagcgcggcatggtcgagggcacggacaagtcgcacacctggatcgtcgacccgatcgacggcaccaccaacttcatgcacgccatgccccacttcgccatcacggtgggactggagcgacgtgcgccagacggctcctccgaaatcgtggccggcgtcacctacaacccggtcatgaacgagatgttctgggccgaaaagggcaagggctgctacctgaacgacgcccgcatccgcgtcgcgggacgcaaggacctgtccgaaagccttatcgccaccggcctgccctttatcggcaagacgggccacgcccaggccatcaaggacatccacgccatcggccagcgcgtcgccggcatccgccgcctgggctcggccgctctggatttcgcctgggtcgccgccggccggtacgacgcctattatgagcgcaacctgaagccgtgggatgtggcggccggcctgctgttcgtcaccgaggccggcggcctggtcaccaccatcgatcaggatggcgaccccaagagcggctcgagcatcctggcctgcaaccccgacctgcacccgcagctccgcaaggtgctgcaggcgagctgaaccgtcacgggcgcgtcgcggtcggcatatacacgagcgacgtgatccgcgccgttcttgccgcgctcctgctgacaggaacgcccgccatgtccgagacccccgccaggacacccctggtcatcgcccatcgtggcgcatccggagagcggcccgagcacacccgcgccgcctatgagctggcgatcgcgcaaggcgcccatgtcatcgaacccgatctggtgatgagccgagacggtgcgctgatcgtgcgtcacgagaatgagatcggcggcacgacggacgttgccgaacggcccgagttcgcaagtcggcgcaccacccgcatgatcgatggcgtcgagaccacgggctggttcaccgaggactttacactgtcggagttgaagacgctgagggcgcgtgagcggctgccacagctcagaccgggcaatgtcgcccatgacgaccttgagcccattctgacgttcgacgaggttgtggcgatcgcgcgggagggcgcggcgcgaaccagccggacgatccttgtggcgccggagttgaagcatccgtctcacttcgccgcaacggggctcgacatggaacaggcgttcctcgccgagctgaagcggctgaacctcacaggcccggatgcgccaatcctgatccagtgcttcgaggcaggcccgctggagcggctcgcagcgcagatcgacgcgcctctgattcagctggtcgctgcatcaggcgcgcctttcgacaggcctgcccaatcctatgcgcagatgatcacgccggatggtttggcgacgatccgtcgctatgccgactggatcgctccggaggcgacgctggtcctgtctcaagacgccgcgggacggtcgaagtcaccaagcgccttggtcgcagacgcccacgccgcaggcctgaaggtggcggtctggaccttgcgcgccgaaaacgtctttctgcctctcgagcaccggcgcggaagcgaaccagccgcctacggcgatctcgccgcctatgccgcagccatcctcgatgcggatgtggacgcggtgttcagcgactttccagccattgtggtcgccgtcactcatccgcccctgaactgaagctcggccagccgggcgtagaggccgccgcgcgccgtcagctcggtgtgcgtcccctcttccaccaccgcgccgtcctccatcaccacgatgcggtcggcgcgcagcaccgtcgccaggcggtgggcgatgaccagggtggtgcgctcctccatcgcctggtccagcgcggcctgcaccagtcgctcgctttcggcgtccagggcgctcgtggcctcgtccagcaacaggatcggcgcatcccgcaccagcgcccgcgcgatcgccagccgctggcgctgtccgcccgaaaggctgcggccgcgctcacccagcggcgtgtcgaacccctgcggcagggcgtcgatgaagcccagcgcctgagccttgtccgcgacgtcgcgcgcctcctccagcgtcgtggcctcacgcccgaagcgaatattctccaaggccgagcctgagaacagcggcgtctcctgcgacacccaggcgaagcggtttcgcacctcgacgggatcggcctcgcgcacgtccaccccgtccaccgtcaccagtccggactgcggatcatagaagcgcagcaacaggcggaacaccgtggacttacccgcgcccgagggacccaccagcgccaccgtctcgcccggccgcaccgtcagcgaaaagcccttcagcgccggcaggtctgagcgcccgggataggcgaagtccacgcctgacatcgacacctcgccgcgcggcggctgaggcagggcgcggggcgcggggggcgcggcgatgccgggctcggagcgcatcagctcctcgatgcgctccatggcgccggcggccttctgcatgtcgccccagctttcgcccagcgcgccgaccgctccagccgcgaacaccgacagcagcacgaactggatcagggcgcccggcgtcatggcgccggagatcacgtcctgcgcccccagccacagcaccagggtcacgccgccgaacatcaccacgatgatcatggccgtcatccaggcgcgcgccttcatccggaccaaggaggcgccgaaggcgtcctccaccgccgccccgaaccggtcgatggcgctgcgctcgcgcccgaaggcctgcaccgtctcgatggcgtccacgctttctccggcgaagccgactgcgttggcgaaccggtcctgcgacgccaccgtcagcttcctgacgcgccggccgaacacgaacagcggcacgatcagcagcggcacgatcagcagcaccaggcccgtcagcttgggactgacgaagaacagcagagccacgccgccgatcagggtcaggaggttcctcagcgcataggagatggaggtggtcatcagcgtctcgacaagggcgatgtccgtggtcagccgcgacagcacctcgcccgtgcgcatgtgggtgtagaagctgggatccagcgtcaggatgcggccgaacaggccctttcgcacatcggcgatcacccgctcgcccgttcgcgtgacgtagaagtagcgcgccgccgtcgccaaccccaggaacagggcgttggcgccgagcaacaagaaccacaggtccaggtcgcgtccgccgttctcgaagccgtggtcgatcgcgccgcgcgccatggcggtcaggcccagcgacgcggcggtcgaggccagcagccacagggccgccagcgccgcatgacccttgtgccgcatggcgtagggaaccagccgcgccaggggcttgatgttgcgggtcttggcgcgcttgccccccgcctcgtccatctgctccatcagcagggcgccggcgccggggcggccataagcttcgggtcgggcgggcgaaggaggcgcggcgtcggtcatggctcgcgcctcttgccccggatcgccccccggtgtaaacgccgccctcttcccgccggggccctcggcgggtttctcattttgcatgcgcagcgacggtcggcatcgtcatcgcgccagagaccggacgacgaccatgaaggcggacacccaccccgactaccacttcatcaccgtgaccctggtggacggttccacctaccagacccgttcgacctacgggaaggaaggcgacacgctgaacctggacatcgacccgtcgacgcaccccgcgtggaccggcggcaaccagcagctgatggaccgcggcggccgcgtttcgcgcttcaacaacaagttcgccggcttcatcaagaagtaagcgcccgctcgccgcaggtgcggcgaataggtcactgcaagcgccggtcgcagggccggcgctttttgtttgtccggaacgtcactattaaacggacgttcgatcctgcgggggcttcccgcacggcggacgccgaatcgttgatccagagcgttgagaatgaacagacgggaattggccttgggcgccgcatcgacggccatggccttcgcctccgccgcgaccgcccagcagcctggatacgcccagcgcgatccgcgcgcgaccgccttcttcaacagcttcaacgaccagatcgcacgtctgccgcaagagcagcaaggcgacgtgcgcgccttctacgaggccaacggctggcgtccggtctggaacgccgagcgcctgcgcgcgctgaacgccgtcgccgcccgcggcgagcggcacggtctggcgcccggcgacttcttcgacttcgtgggtctggccgccgatcccggctcggccgagctgcgcaccaccgccgccgccctgctctacgcgcgcgtgctcgccgaaggccgcgtccgccccgaaacggtggaagagctttgggagatgcggaagaaccgggtggatctgcccggcggcatgaccggggccatggcgagcaaccgcctgctggactggttcgaaggcctggcgcccacggacatcggttatcagaacctgtccgccggctacatccgctatcgccgcctcatggccgacggcggctggcccgcctttgcgcaaggcgcgaccatcgagccgggcatgagcgaccggcgcgtccccgctctgatcgcccgcctcaccgccgaaggcgacctgacgcaggaggccggcgcgcgtctgaaggcgcagggactggtctacggctccgagctgcagaacgcggtgaagggcttccaagcgcgtcacggcctgggcgccgacggtcgcatcggcgcgggcacgcaacggtcgctgtcggcctcggcccaggatcgcgcccgccagatcgctctgaacctcgagcgtcgccgctggctgaagcgcgaggtcgcgcccgagcggatcgaggtcaacaccgccgccgccatcatggtctactggaaggacggcaagcccgttcactccaaccgcgtggtggtcggaacggccgacaaccagacccccagcctggagaagcccttcgcctccgtggtcgccaatccgccgtggtatgtgccggccgggatcgcccgccgcgagatcctgcccaagggtcccggctatctcgccgccaacgacatgttcgtgcgcgacggcacggtgatccagcgcgccggccccaagtcggcgctcggctatgtcaagttcgagctgcaggacagctacgccatcttcctgcacgacacgccgtccaaggcggccttcaacctcgccatgcgccagcgcagccacggctgcgtgcgggtgcagaatgcggtcgagttcgcgcgcctgctgctgtcgcccgatccgaccaagctgggcgagttcgacgccgctcaggacagccgcgagacgacccgcgtcaccaccggccgcgacgtcaccgtgcgcctgctctactggaccgcctttgtcgacggccagggccgcgtcgccttccgcgaagacgtctatggccgcgacgacaagctggcccaggcgctcggcatcgccgtcagcctgcccaagccgatcgacgacggccagcgcgacgtcaacgacgtcggcccgtagctccatgagttctccctcccctgacggggagggaaaaaccggcggcgcccttgttaacgcccgaaggcggcctggagccggtccatctgcgtcagcaccggattggcggcgggcggctcgccttcgcccaggtacatacggcggtccagatacaccgtccgctcgaacagcttgtcggcccgcaccagatattcgaccagggcgatcggcagctcggaatggctgggttcgcgctcgatcttgcgttcgttgaggcgatagcgcggctcgcctgcggcctcgggcgtcatgtcgccttcgcgaaccgcacgctgaaccagcagccaggaggcgatctgcatcaggcgcgtggtcagccgcatgctctcggccgcataggccagcgcggccgcacgcgacagcatcttggactcacgcctaccgtcgccgtccagataggcggcggtctcctcgaccagttccatgccttcgcggaaggtgcggtcgaacagctcggagcgggcgaagtcgcgcacggcggcggcgcggtcctgcgtcgtcccggcggtgagttcaggcatcatcatgggctgtgcgcgcgtccgtaccaacttcggcgtcctgcgacgcccggctccccaagcctgcaaccgtcatgccacggatcacgcccggcgtcatgagcccggttgtggagaaccgccgaagctgaatagggcgtcggccgcgctcttctgcaactgcttgcgggcgatggaggcttgcgcccgctcgatctccgccttcagcgcctcgatccggtgttgcagcgcatcgactgacagcggatccaggtcctcgcggcccagggccgtcagggcctcgcccgcccgcacgcgcggttcggattcgtcgaatatcatggccgcctccgcatcaagctcctatctcaacgcgccagcgtcgacgattgcaagagaagggccggccatgcgcgtgatcgagatcgagggcggctcaggccccgccgaagccctgcgggtcgtcgagcgaccggacccccggcccggcgccggcgagatcctgatccgcgtgcgcgccgccgggatcaaccggcccgatctgctgcagcgcaagggggcctatccgccgccgcccggcgcctccgacatcctgggcctcgaggtcgcgggcgaggtcgaggcggtgggcgacggagtggcgcgctggcgcaccggcgatcgggtctgcgccctgctgggcggcggcggctacgccgacctggcggtggtggacgcccggcacgccttgccgatccctgacggcctcgacttcgcccaggccgcggtgctgcctgagacgatcttcaccgtcttcgccaatgtgttcgaggccggcggcctcaaggccgacgagaccctgctgatccacggcgccaccagcggcatcggcgtgaccgccgtccagatggccaaggcggcgggtgccaaggtcatcgccacctcccgcggggcgaaaaaggccgaagcggcccgcgcgctcggcgcagacgtcagcctggacgccaccgccggcgacctgtccgaagcgatcgcccaggccggcggcgccgacgtggtgctggacatggtgggccgggactacgccgaactgaacctccaggcgctcaggcccggcggccgctggatcgtcatcgccaccctgaccggctgggaggcgccgatcgacctgcgccgcatcatgatgaagcgtctgacgctgaccggttcgaccctgcgcgcccgccctgccgaggagaaggcgcggctggccaaggccgtggagaccaccgtctggccctgggtcgccgcgggcgccgtccgcccgcccatcgagcggaccttcccgctggaggacgcctcggccgcccacgccctgctggaggcgggcggccacgtcggcaagatcgtgctgatcccctagatcagcgctcgccgcgccagggtctcaacgaggcgatgctgtcgtccatgcccagccggaacagggtgcgcagatcgccctccaccacccggcagcggccccggtagttccgctccgaacagacctgccactgaccttcggcgcggatggcgctggcctgacggttcaacggcgaacggcgcaggtcgggcgcctcgccgcggaagcgttcggacggtccgcgatagtccggatcggcgtacagggtcagggtctggcgcccgccgttccaaccgcccggtccgcccgcacggccgtcgtcgccgtcccagccgccgccgggacggcccggacggccgccgccgccttctccgtcctcgtagtcgccgcggatgcggccgcagaccagccggccgttgtcgttgttgatctcctcgccgccgcattggccgacctcaatggaggtgccccgcatgcgcccgcgcaggtcgcggcagtcggcgtagagccgtcctcggttcacaaaggcctccgagcagctctgggtgtaggagccgcgcggcgcgacccgctgaaccgacacgtcccctcgcgcctgccccgcggtcagcatcccggcggccagggtcgcgctcaacaacatcgacatcgtctcacctccctttgcgtcggcgcctttcgtggtccgcgcgatctggagcatcgttcagccaagatgaaccgtagctgtatggactgcgtgatgacgttttcttttggcgcagaatgtgggatatcgatttcaatcagcgcccggtcgaaaggccgggcgccgttgtattcaacgcccggcaagcacacgggcagttcacgggacgaacgcgccatgagcgacattctgatgcccaaggccactgcggtctggctcgtcgacaacacctccctgacctttgaccagatcgccgacttctgcggcctgcacccgctggaggtgcgcggcatcgccgacggcgacgtgtctcgcgacatccgcggcgtcgatccgatcaccggcggccagctgacccgcgaggagttggacaaggccgaggcgaacgaaggctatcgcatgaaggcggtggtcagccgccacgccgaactgctgaagtccaacaagcctgcgccgaagtacacgccggtgtcgcgccgccaggaccgcccggacgccattgcgtggttcgtgcgcaaccacccggaagtcacggacgcccagatcgccaagctcttgggcaccaccaagtccaccatcgagagcgtacgcaaccgcacccattggaacagcgccaacatcaagccggtcgatcccgtgaccctgggcctggtgggccagctggctctggacgacctcgtgcgcaaggcggccgacaagaaggccaaggacgacgccaagaacggcggcgcctcgctgcagccgctgcagccgctggattcggagccgcaggagcccgagttcgtgccggaggcgcgcgagcgtccctcggccgagccgaccgccgagtccgtgttcggccgccgcgactgaggtcttcgggatacgccaaggaaaacggccccgggagcgatcccggggccgtcgtcatgtctggcgttgcgcgaccggtcagggcgttcgctgctcgagactggagatctcctccttcagcctgagcttcctctgcttgagttccctgaggtgcagcgagtccacggacgggctttgacgctcccgctggatggcagcatccagcgtgcggtgacggttacccaattcgcgaatacgagcctcgatggtcatggcttgcgcctccatgtctaagggaccactagagtgagcgcccggttcggcggactgtgtagtcacaaatccgtgacgttccgcctggccggacatccaggaggctgaaccccgaaatgggtcatgatgtgaacggagccgtaggcgcgacgccgcgccgcatggtggtcggcgtctccggcgcttcgggcgttgtctacggcgtgcggacgctggatgccttgaaggcgctgggcgtcgaaagccatctggtggtcacgcgcgcggcattgctgaccctgtcgcaggaaacggatttgacgcccgacgatctcctgggccgggccgatgtggtccaccgcctggccgacgtgggcgccagcatcgcctccggctctttccgcaccctgggcatgatcgtcgcgccttgctcggttcgcaccatgagcgagatcgcgaccggcgtgacctccacccttctgacccgcgccgccgacgtgacgctgaaggagcggcgtcccttggtgctgatggtgcgcgagacgccgcttcatctgggacacctgcgcaccctgaccgccttggccgagatgggcgcggtcatcgccccgcccctgcccgccatgtacgcccgccccgcctcgatcgaagagatggtggaccagtccgtcggccgcgctctggacctgttcggtctggactggggcgaggtgaagcggtgggacggtctaaagggagcgcccgacgcatgagactgtgggactgggccgtcgccgcctatgccgcgcctgatgtcgccgaggcgtgcctcttgctgcaggaccgtcatgagcagaacgtgccgctgctgctctggtcggcctgggtcgccgcgaccgggcgccgccccgacgaggagacgctggaggccgcctgcgacaccgcacgcgcctgggacagcttggcggtcgcgccgctgcgcgcgatccggcgcacgctgaaggcgccgatccccgacatcgacgatgcgccgcgcgaggcgatccgcgaccggatcaaggccgtcgagctggaggccgaacgccggctgctggaggcgctggaggcgctcgctcccgaacccgcagggccgccgcgcgccgccatcgacgccctggtcggcacggcccgcatctgggccccggtcacgccccgcccggcgctgatcgcgctggcggactcccttccggcctgaatcgacctcggctatagaccgcgctcgggggagcggccatgaacgacgacacgcccaaggtcagcgaggaagaagcggcgctgcacgcccgcgtccgcctgctgcgtcaggaacacgccgatctcgacgcctccatcgaggcgctgggccagacgccgacgccggaccagcttctgatcgcacgcctgaagcgcaagaagctggtgctacgggacgagatcgtaaagatcgaagcccgcatcctgcccgacatcatcgcttgatcgatgctcaggctgcggcctttcgccgccgccgcgacgccccaaagcggtcaaataacaaagacataagcgcggcctcggccgagcgccttcgcacaagtgggggccacggccgcttttccgccgcttgaagagctgggagacgccgccgaatgcgacgaccgacaggctacgcccacatgacgcgcctcaaggccttcctggcccactcaggccagacggccgtgctgggcgtggtcgccgtcttggccatggccgccgcaccatcggccacccgcagcagcgtcgccgccgagacatcggtcccctcagcggcgcccgtcgccccgcccatcaaggcgatggtggagacgcccggtcctgtcacccgcaccatcgccttctccactccggtcaagggttatgcgatcaattcgcccttcggtctgcgcaagctggcgatcgaggcgaaggcgcgtgcgcacaagggcgtcgacatcgccgcgcccatgggcacgtcggtcttctcgaccagcgaaggccgcgtgctgcgcaccggctatgacgcaggcggctatggcaagttcatcgaggtgcgccatcccaacggcctaaccagcctctacggccatctcagccgcgttgatgtgaccaacggagcggtcgtcgcgaccgggcagcgtatcggtctggtcggctcgacgggcttctccaccggtccgcacctgcacttcgaggttcgtcgcggcggcgcccaggtcgatcccgccaagatcatgggccgagacttcaaggtcgccgccgagggttgaagcgcctcccctgcatgacaggaaattaatcttccccttccctgatgggcgctaggctcccgcgcagggacaaggggggaagacggcatgacggcggcgttgacgctggagggcgtaagcaagagctacggcgattttcacgccgtgcgcgatctcggtttttccgtgcccaagggatcgatctgcggcttcctgggcccgaacggggcgggcaagacctccaccatccgcatgatcctggggctgcagcccgccagcagcggccgcatcgacatcctgggtgcgcccgatggtcggcaggtgcgcgaccgcatcggctttcttcccgaggaacgcggcctctataagaagatgacgccggtcgaggccatcgcctttttcggctcgctgaagggcctgccgccggccgagggcaaggcgcgcgcccgcgacatgctggagcagcagggcctcggcgcctcccagaaaaagaagatgaaggacctgtccaaggggatggcacagaaggtccagttgatcgcctcggtggtgcatcgccccgagttcgtgatcctggacgaacccttttccggcctcgacccggtgaaccagcagggtctggaggagatgatccgaggcctcgccgccaacggcgcgaccgtcctgttctccacacatgtgatgcagcatgccgagcgcctctgcgacaaggtcgtgctgctggcgcggggcaggaaggcgttcgagggcacggtggatcaggcccgcgccacctcgccgcgctttcttgacctgaccggcgccatctcgcccgatcaggctgcggccctgccgggcgtcgaggcggtggagacgaccggcggccacgacggcgtccacgacctgcgcattcgcctgcgccccgaggcggccggccaggacacgctgaaggccgccttcctcggcggactggatgtgcgcgcctttgcgctgaaagagccgacgttgcacgacgccttcatcaatctgacgggcgaccggcccgatgcgccgaccacatctgctcgcgaattggaggcggcccaatgaagcgcaccctgctgatcgctcagcgcgagttcatggcctacgccaagaccgcgggcttctggctgtcgctgctggcgtttccgttattcgcggtgctgggcgggggcattcccttcctgatccgctcggccgagccggtgcgccaggtcgccatcatcgacgaaacgccccaaggctctttggcgggcgcggtgcgcgctgcgctggaggcggaccagcggcgatccgatatcgacgccctgcgcatggcggccattccagaagcgggcacgacgggcggcgaccgggtccgcgcggcggcggaggccggcggttatgaggccgggctggcggagcttcggcggatcgccccccgcgcgggcgcgggcgcaaaaccagccaagcgccagatcgtgctggtcgcgccgccggcgagcatcgcggacgcgcaacccggcgccgaacgcgacgccgccatccgcgaggcgctggagacagccgaccgtgaggagcggccgctcagcgccgtggtcctgctgaaccagcagggcgccgctccctccgcgcgtgtctggaccgagcgcgcaaccgacacgacggtggaaagcgccatccgcgacgccctgcgcgacgtcaatcgccagagcgtcttcgttcgggccggggttgatcccgaggtggtgcgccaagccgaccgcttccgccccgaggtgtccgtcttctcgccccgcgccaccagcggcggcgaggtgtcgttccgtgaccgcctgccgggtctggtcggcctggtgttcggctttcttctttggtcgctgatcatcaccggcgcctccatcctgctgaacagcgtgatggaggagaagtcgaacaagatcctggaggtgctcttgtcctccgcctcggccaccgagatcctgacgggcaaggtgctgggcgtcgccttcctcaccggcacggtgctgctggtctgggccggcatcggcgcggccggcctgcaggcgggcgtgccggacgtggcgcgcgacgtcatgtccgtgctgatgagggacggcctgctgatctacttcctgctctacacggtcggcggctatctgatgtacgccgtgcttttcgcggccatcggcgccttttgcgagacgccgcgtgatgcccagaccttgatggggccgatcatgatgatcctggtcgtgccgatcctggtcatgcagatggccctgcgcacgccggacgccaccgtggtcaaggtgctgtcttggatccccttcttcacccccttcctgatgagcgcgcgggcgcccagcgatccggcgctgatcgagatcgtgctgaccctgctcggcatgttcggcacggcgctgctgatggtctggatggccggccgggccttccgcgccggcgccctgtcggacgtcaagctgagctggaagagcttcggccgcgcggtcaccggccgaagctgaccctctcctcgccatccgggacgacaaagaaaaaggccgcctccgaatggaggcggcctttgatcttctggcttgcgccttgagccttaacggccgccgggaacccggggcttcggcgcaggcagcaggccttcgcgctgggcgcgcttgcgggccagcttgcgagcgcgacgaacggcttcggccttttggcgcgcgcgcttctccgagggcttctcgtagtgcacgtgacgcttcatctcacggaagctgccttcgcgctgcatcttcttcttcagggctttcagcgcctgatcgacgttgttgtcgcgaacgaaaatctgaaccaggtgaatctctcctttggccgcccgccgcgtcctgatgagggaagacgggcagacaaaacaaaacctctcccggcggacggcggtcctcgggtgaaggcgggctgatacacgagcgacccccggctgtccagatggccgcacgtgtttcgcagggctcgaaagcccgttcacgcgggcgtatggtgcgctcatgaccgagccgcattccgcaccttccgactgggccagccgcaccgagcaggccgtcctggacgccgccgtcgcgcaagcgccggcgcttggctggaacgcccggctggtgcgcgaggcgtgtgaggcctgcgacctgtcgcgcggcgacgaggagcttctgctgcccaacggcgcgcgtgatctcgccgccctgctgtcgcgtcggcacgacgtccgtgccctggaggcgcttgaggcgacggacgccaaggcgctgaagatccgcgaacgcatcttcgccgccgtgtccgcgcgcatggaggccggggccgccgatcttgaggccacgcgccgctgcgccgcctttctcgcccttccgacccacgccgacctcggcctgaagctggcgtgggagagcgccgaccatctttggcgctgggccggcgacacctcgaccgactggaaccactattccaagcgcaccatcctgtccggcatcctgatcccggcgctgacgctgcgctggttcgaaggacgcgagtcggccgagcgctttgtcgcccaccgcatcgaaaacgtcatggcctttgagaagtggaaggccggcaaggacttcgacgcgccgttccgcaaggcgacggacgtgctggcgcggatgcgctacggctccaggacggccgcctagatcggtcccagtacccggttgacgtggcccatcttgcggccggggcgggcttgggccttgccgtagaggtgcaggcgggcgtcgctctcgccgttcaggtccgtccagcgctcgacctcgtcgcccaggaggttggtcatctcgacgcgggcgtgagcctgagtcggaccgagcggccagccggcgatggcgcggacatgctgttcgaactggtcgcagacgcagccgtcctgggtccagtggccggtgttgtggacgcgcggcgcgatctcgttgaccagcagcaccccgtcgcccaggtcgaacagctccactcccatgaccccgacatagtccagcccgtccaggatcgcctcggcgacggcgcgggcgcggaccaggatcttttcgtcggcgatggcgggggcggtggtgacgcgcagaacgccgccctcatggctgttctcgcccaccggatagacggccatgcgcccgtcccagtcccgcgcgcagatcaccgacagctcgcggatgaagggcgccgcggcctccaggatcgcgggccttccgccgatcgcggcgaaggcggtagccgcctcggccgggtcgcggacccagacctggcccttgccgtcgtagccgtcgcgacgcgtcttcagaacggcggggacgcccagccgcgcgagcccctcacgcaggtcgtccagcgttgcgaccggatgaaagtccacggtcggcgcgcccaccgcgttcagaaacgtcttctcctcgacccggtcctgcgacacccgaagcgccgtcggcccgggcgccacgcgggcgcccgcctcggccagccgctccagcgaagcggccggcacgttctcgaactcgaacgtcaccacgccgcacgctcggcccagcgccgtcagcgcctccggatcgtcatagggcgcgacgaactgaccggcggagacgcgcgcggcgggacagtcgtcctccggatccaggatcagcacgtcgaagcccagacgcgccgccgcctggctcagcatccggcccagctgtccgccgccgacgatgcccagcgtggacccagggcgaaggggaagatcggccatgagcgtcagtcctccaccgtctcggccacgccgtcggtctgcgctgcacgaaaggcgctgagccgctcggccagatcgggatcgttcaacgccagtatctgcgcggccaggatgccggcgttggcggcgcccgcctctccgatcgccaaggtcgcgacgggaacgccggccggcatctgcacgatggacagcagcgaatcgagaccttgcagcgccttcgactgcaccggcacgcccagcaccggcaggtcggtcatggcggcggccatgccgggcaggtgcgccgcgccgcccgcaccggcgatgaccaccttgaagccttgcgcccttgcgccgctcgcgaactccaccagccgctgaggcgtccggtgggcgctgacgacctttgcggtccagcccacacccagctggtccagccgctccgccgcccgcttcatcgtcggccaatccgagcggctgcccatgatgatggcgacgggtgcgacggacgattcggatgcggtcacggcgaagcccttctgccggaaaggccgcccgttacagcacacgcgttgcgcccgcaaccaagcgcgctagcattgcaaaacagcgtgacccggttgagtcgcgcttcgcccggagccgccgcacccttgaccccagccccgacagacgcggcggagatcgatcctcaggctgagatcgcgcgtctgcgcgccgagctggacgcctggcgcgcgcgcgccgaagccgccgaggctgcggccgaccacgacgtgctgacgcccgccctgaaccgccggggctttgtcgaggcgctgaaccgaaccatgccctactgccaccgccacagggtgccggcggccctgctctaccttgatctggacgggttcaagggcgtcaacgatcggctggggcatgccgccggcgacgctgcgctggtgcatgttgctcggctgttgatgtccaacgtgcgcgagtcggatgcggtgggccggctcggcggcgacgagttcgctctgctgatgctgaacgccggcgtcgaggaaggccgcgccaaggcgcgccagctgaagtccgccctggaaggcgacggctttgtctgggacggacagccgacggggctgggcggttcgttcggcgtgcgcggctgggacggccactccgacgccgaggcctggctggccgaagccgacgccgccatgtgggtgcgaaaaagggggcgctgaggcccccttcccgctccgtgcaggacgttccggttacagcgccagacgcagctggacgccgcccatgtggctgtcggcgtggtcgccgaaccggccgcgatagccgacggtgatctgcagccgcccgatctcgccctcgacgccggccgtcgccagcacctggccgccgaacggctcctcgacctcacgctccaggatacgggccgggctgttgtacaggccgacgcgcacgccttcggagctgtcgtccagcgcgttgcgatacccgccctcggcgaacaggccgaagccagccatctccgcctccgcccgcaacacgacctcgccggtcagcgcctccaccgtgcggttttcaaaggcgtactgcgccgccaccccctgttcgacgtagccgtccacttccgacgaggtccaggcgagcgccgcccgcggcgacagcgacagcccgcccatctcgatccaggttccggcctgcagacgcgcgcccttgctcaggccgtccgtgtcggcggtgtggacgatcggggcgatggtggtcaggcgttcgatgtcgtcgtagcggtcgcgcgcgacgccgacggccgcgttgacgaaggggccgccctccatgcgccagccgccgtacagatcgagaccgaagctttcgacgtcgaagttcagcgcgccgcccgagacctccgatccgcgataggtccccgccaggccgaagcggaggctctccgaagggccggactccagagcgatgcggccgccccacccctcgctgctggccgagcgcacggggccgcgcgcgtcgatgtccacactgtcgcccacgaccgccgccgagacggaggtgcccgccgtccagggcgcccggccggacagcgcctcgccggccatgtccagggtctcttcgcggtggcggaagccggtctcgccctgcaaggcgctctgtgcgccgatatcgccgtagtagaggtagtcggtcgccagagccgcgatgatgcggtgcccggtcgccgtcgggtgcacgccgtcgaagtagaagtagctggacggattggcgcacaccgcgccggttgcttgattaaagcaggcgtcggtgacgttggtgacgccgaaggcgccgggattggccgccagggtgtcgctgatcttgaacaagtccaccaggatgatgttgctggtcgggcgggccgccgccgtggccgccaggtttgtcgccaaggcgccgttcagcgtcgtgaccgcgtagtcagccaacggcgcggcggccgtgttccggaactggggcgtcaggctgagcttgggcaggttggtgaccaggatggttcccgccccggcgcccgccacgctgttcaccaggctgttgatgttgccggccgcctgcaaagccacaggggtgatggccgcaacaggattggccgatgcgccggccgccggcagtccctgaaagatatcgttggccccgccgagaacgctgaccaggtcgccggcgccgaagcggccgccgcgtgcgacatagccgcccagctgcgccagcatgcccggcggcggcgtggtcgaggcgtcggtgcgcgatccgccgaacgccaagttgatgctccccgtcaccgcgccgttaaagttggcggcattgaagcccagcagctcggtgaacactggtccggtcgagaagcgtccctgatagtagggcggcgacggcggctgggtgcggcctgaggccagatacaggttgccgttgtcgctgaggctgtcgccgaacacgaccagccgatcataggtctgggcctcggccgatgcggccgcgccgcaggcggcggccagggtcagggccgcgacggcggccccgtgaagaaagcgaaacatccagatcctcccgcggccgtcgtgatcgcggccgttcgcgcgcactctgcgcctgtttgcgacagtttcaagatgccgcagcgtaagccttggcggctcagtggagggtgcggaacctcagtgtgcccggcaggtcgcgcagcgccttcagcgcctcaggctgatagtcgcggtcgacatcggtgatgacgtagccagtgcgctcgtccgtcttcaggtgctggccgagaatgttcagccccgccgccgccaaggcctggttcagttcggccagcacgcccggctggttgcggtggatgtgcagaagccggtgtgcgcccgacacctccgccagctgcacgttcggcaggttgacgcagaaggtggtgtcgccccggttgagatagcccagcagccgctcggccgcgaactcgccgatggcctcctgcgcttcttcggtcgagccgccgatatgcggcgtcaggatcatgttcttcaggccgatcagcgggctgtcgaagggatcggcgttggtgcgcggctcttcggggaagacgtccacggccgcccccgccagccgcccgccctgcagggcctgcgccagcgcgccgacatccaccacatggccgcgggacaggttcagcagcagcgccccctccttcatgcgcgcgaactgggccgccccgaagatcttcgtgttctcagtccgcccgtcgacgtgcagcgtcaccacgtcgctttcggccagcagggcgtccagcgaccgcatgcgccgcgcattgccgagcgccagccgctcggacaggtcgtgaaagatcacccgcatgcccagggcctccgccagcaccgacagctgcgagccgatggcgccatagccgacgatgcccagcgtcttgccccgcagctcgcgcgaaccggtggccgacttgttccactcgccccggtgcatggcggcggacttgtcggccacgtcgcgcatcagggcgatcatcagcccgaccgccagctccaccaccgatcgggtgttcgaatagggggcgttgaacaccgccacgccgtggtccgccgccgcttccaagtcgatctggttggtgccgatgcagaaggcggccaccgccataagccggtccgcctgctccagcacccgccggctgaccgtggtcttggagcggatgcccagcacgtggacgcccttgatggcggcgatcagctcgtcctcgtccagcgcgcccttgaccgtctcgaccgcatagcccgcctcggacaggcgctcgaccgccgccggatggatgttctccagcagcagcatcttcatgcggctgcgcggaaaggaccagcgaccgaccagcccctcggcgtgcagcacctcgtccagcgaagccgcctcagcgtccgcgatctcgaccaccgccgcacgacgaacaacttcggtgaaggcgtaaaaggcgtcggccgcgccggccagcttgacctccgcatcgttccagccgtccccgaccatcaccacgcgcccgctcaggccgaggccgtggatcacctgcggcttgccgtccgcatggctgagcggattggcgtcgtccacaccgatcacccggccggcgtcgtcatagatcaggtcgttgcacaacacccgctcggccgagacgcccagctcccgggccaccggggcgatgatctcgcgaaagccgccggacaggatcaccacccgccccctggcctcggcgaagaagcgcagattgcgccgcaccgagggcgtcaacgcgtccaccgcccgggcggccacggcttccacatgctcgcgtcgcaggggcagcagcgccagccgccggcgcagcgcctcgccaaaggggatttcgccggccatggcgcgatcggtcagggccgcgatctcggaccgcacggccaccgcatccggcgccccgtcaagcgcgacatccgccagcgcctccagcgtctcgaacccgaccaaggtcgaatcgaagtcgaagatcagggtcgggcgctgggtcatggcctcctgcataacgaaccgcgccgcccggacaaagccggacggcgcgacaggtcgtgcttgttccgctcagccctagacgcggtcgatcaggcggcgaacgcggctgtcgggctgccggctctcccagacggcggcgccgacggcggcggccagggtggcgaccgccagcagcgcgccgccttccttggcgtgatcgcgggcgtaggcgccggcgtcgtcggcgtagcggcgcgcctgcttgccgtggtggtgcagggcctcgcgcgacttggcgtgcgcggacttgaaccgccctcgcgcctcgtagccgacgccggccgcgcgatcgcccagatcctcggccccgtgcttgaaggcgtccacggcgtccgcaaggcgatcgcgcagcgcctcggtgtcgacccaaccgcgcggatcgatgcggttgcggatgcgctgatagcgggtcgggccgctgcgctgcgtcagatagacggcggcggccgcgcccagcaggatcagggccgcgccgctggcggtgatccccggatgcttgcggacttcggccagggcgtcgaactgtcggaccatgggatagtaaacctcttcgtcgaggccgtcctcggtcgggcggtaaagcccgtcgtcggccggcgggtaggcggaaccccggtcccgcaacagcgaaggagcgaaccgggcgaaaagtggttccgccaagcctggcagtagattgtagaaggacgaaatggcgcggcccgatccgccgaccgtgatctcgcgcaccggatgctgcgcgcagtgcaggatggcgtcggccacgacgcgggtcgcatagaccggctggggattgtgcatgggcttgccggtcaggttgcgcgcatgccgactatagggcgtggcgatcggccccggcttgaccagggtcagcacgaccggcgccttgtcgcgcatcagctcgatccggaaggcgttggtgaagcccttcaccgcgtgcttcgacgccgaatagacgccctggaccgggataggcatgtcgcccagcgtcgagccgatgttgatgatcgcgccgccgcctgggcgatcgcgcagatgctcggcggcgatgatcgagccgttcaccagaccccagtaattggtgtcgaacagccgccgctggtcctccagcgtcgttttgcgaatttcaccgaagatggagatgccggcgttgttgacccaggtgtcgaagccgccgaaccgccggcggcactgctcggccgcatcggccaacgcgtccttgtccgccacatcgactgcggcccaaccgacgcgtgctccttgagcctccagctcggcgcccagctgcttcaggtcgccttctccacgcgcgatcaggaacacggccgcgccgcgctgcgccgctcgccgcgcggtggccaagccgatgccggacgtggcgcctgtcaccacaacgatctgctggtctagcggcttcagggtcggtcgggtcatcgaggctcgcggatttgatctctgtggaccgctaaaacgaggtccagtcccacccgttccgatgcgcggctgcgcccgggccttaccatcgtcggcttcggcgcctatctaggccgccaatccgcacatcgatcctcaaaggacctcgccgtgaccgatcacgcgcacgaccacgccgccacgccgccgacggacgacctcgccgccgcctttcagatcgagggctggccggtgcgtggccgcctggtgcgcttgggccagaccatcgacaccatcctgggctcccacgcctaccccgagccggttgcggccctcctgggcgaggcctgcgcgctcgccgccctggtcggctccagcctgaagttcgagggccggctgatcgtccaggcgcagggagacgggccggtgcgttacgtcgtggccgactatgacaccgccggttcgctgcgcggctactgccgctacgatgaggcggaggtcgaggcggcgtcgcaaggcttcgcccgtcccggcgcgcagagccttctgggcaagggcgtgttcatcatgacgctggaccgcggcccggacttcgagcgcacgcagggcatcacgccgatcgagggcgagagcctgtcgctgtgcgccgagcactatttcgaacagtccgaacaggtgccgaccaaggtgcggctggcggtcggctcggcccagaccgaagccggaacccagtggcgggcgggcggcgccatgatccaggtgatcgcctccgacgccgcgcgcggctcgaccgaggaggtgtgggagcgcacccgcgccttgttcgccacgctgggcgacgacgagctgatcgaccccacggtcgggcccgagacgctgctgttccgcctgttccacgaggacggcgtgcggctggaggatgcgcgcccgctggcggcggtctgccgctgttcacgcgaccggatcgtgtcggtcctggcctcgttcgacccggcggaacggggcgacatggtggaggacgacggcaagatccgcgtgacatgcgaatactgcgcctcggtctacgccatcgagcctgacgaggtgacggcggctcaggtctgagccgccgcgggccttcagccctcgaggtccagcgaatagccggccgagcgcaccgtgcggatcggattggggctgtcgccgaggttcagcgccttgcgcagccgccccacgtgcacgtccacagttcgcgcctcgacatagacgtccgagccccagaccgcgtccagcagctgctcgcggctgaacacccggcccgggtgctgcatgaagtggtccagcagccggaactcggtggggcccagatgcacctcctgccccgcccgcttcacccggtgcgagacgcggtccaccacgatgtcgccgtggttcagccggtcgtcggccaagcccggccggatgcggcgcagcaccgcccggatgcgggccatcagctcgaccatcgaaaagggcttggtcaggtaatcgtcggcgccggtgtccaggccgcgaacccggtcggtctcctcgccgcgtgcggtcagcatgaccaccggcaggttgcgcgtctcgggccggttgcggatgcggcggcagacctcgatgcccgacagcttgggcagcatccagtccagcagcaccagatccgggatgcgctcctcgatctgcagcatgccctcgtcgccatcggaggcgacggcgacgtcgtagccctccttttcgaggttgtactgaagcaaggtcgccagcgcgtcctcgtcttccatcacaaggatatagggctgcacgtcaggctctccggcgaggtggcacgcttagtttgtgggcaggttcggcgtcggcgcgttgtcttcgggcgtcggctgcgcgcgcggccgttcgcccatgatgtcgtcgccggtgatctcgtagtggacggtttcggcgatgttggtcgcgtggtcgccgatccgctccaggttcttggccatgaacagcaggtgggtgcaggcgccgatcgtgcgcgggtcgcccatcatgtaggtcagcagttcgcggaacagggcgttgtaatgctcgtcgacctcgtcgtcggtctgccagaccgccagcgcccggtcgacttccgacgccgtataggcgtcaagcacgtcgcgcagacgcatggacaccagccgccccatccgctcgatggagcgggtcaacggctgcatcggctcgctttcggccagaaccagcgcacgcttggcgatattcttggccaggtcgccggtgcgctccaggtccgacgccatcttgatggcgccgtaggtgcgacgaagatcggaggcgaccggctggcgcagtgcgatcatgcggatcgcctttttctcgatgtcgcggtgcagctggtccagcttgccgtcgcgctcgatcacggcgcgggcgagccccacgtcgcgtcgcgccacggagtcgatggaatccgcgacctgcgcctcggccaggccgcccatgcgcgcgatctcggccgtgagctggttcagctcgtcgccgtaagctttgacggtgtgctggttcatgacccgatcctcagccgaagcgtccggtgatgtagtcaagcgtgcgccgctcgcgcgggttctggaagatggtctcggtgtcgccggtctccaccaggcggccaaggtggaaaaaggccgtgcgctggctgacccgcgcggcctgagccatcgagtgggtgacgatgacgatgcagaagcgctcgcgcagttcgtcgatcagttcctcgatccgcgcggtggcgatggggtccagcgccgagcagggctcgtccatcaggatcacttccgggttcacggcgatcgcgcgggcgatcaccaggcgctgctgctgcccccccgacaggccggtggccgaggcgtgcaggcggtcggcgacctcgtcccacaggccggcccgcttcagcgcgctttcgacgaccccgtccatctccgacttggcgctgaccaagccgtggatcttggggccgtaggccacgttctcgtagatcgacttggggaacgggttcggccgctggaacaccatgccgacgcgtgcacgcagcagcacgggatcgaggccgcggtcgttgatgtcctcgccgtccatctcgatgcgaccggtgacccgcgcgccgtggatggtgtcgttcatgcggttcatggtccgcagaaaggtcgacttgccgcagcccgacgggccgataaaggcggtcaccgtcttgtcgggaatgtccagcgagacgtcgtacagcgcctgcttgccctcatagaagacggacacgtccttggcggcgatcttgatggggccttcgggcgggctgtcgaccaccgtcggcccagtcatcggcgaggcgtcctccatgcgcggctcgaccggcgcctgttcctgcgcgggcgcgacctcgggcagcacctggccgcccatgcgcggcgcctccgtcgggtcggcgcggccgcccgtgcgatcgtcggtggcgcggaaaatattgaacttcatgctcttaccaccgacgctcgaagcgccgcctcaggatgatggccgccaggttcatcacgatcatgaacagcagcagcaccaggatcgccgccgccgtgcgctcatgaaacgcgcgttcggaagcgttctcccagatgtagatcagcgacggcagggctccgaccggctggtcgatggccgccggaacgccgggcacgaagctgaccatgccgatcagcagcagcggcgccgtctcgcccagcgcatgggccatggagatgatggcgccggtcatcacgcccggcatggccagaggaaggacgtggctgaacaccgtctgggtgcggctggcgcccatggccagggccgcctcgcggatcgacggcggcaccgccttcagcgacgagcgtgtggcgatgatcagcgtcggcagcgccatcagcgccagcaccagaccgcccacgatcgggctggcgcgcggcaggtgcatccagttgatgaacagcgccaggcccagcaggccgtagacgatggacggcacggcggccaggttgttgatgttgacctcgatgatgtcggtcagcttgttcttgggcgcgaactcctccagccacacggccgcgcccacgcccaccggaatggcgatcagggcggtgaccagcagcatcagcgccgagcccacgatggcccccaagacccccgccagctccggctgggtcgaatcgccctgggtgaacagggtggtgttgaaatgggcggacaccgcgccgtcggctttcagccgctccagccagtcgatctgctggttggtcaggcgacgctggtcttcgggcgtatcgcgcgagatctcgcccttcagataaaggtcggcgtcgtcggacagcggcgcgtcgatcgcgaccgtctggccgatcacctctggccggcggctgaccgtctcggccgccgcgaacttcagctcggacgagaacagcgcgcgcatggccgtggcctgctcgcccgtcggatcggccacgccccagcgcgccagcagctgctgcgccgtcagctcctcgaagttggcgccttgcggataggtgcgatcgacgcgcgccggatccatgtaaacgggaacggacgcgctgtgggcgtagaaggcggtgtgcccctgctccacgatccggcccaacaggatgaccaggaacagcagcgccgcgccgatggcgatgcggccgtaccacttgaagcgctgctcgcgcgcgtgccggcgccgcagcccgaccttcagccggtccaggcgcttgtcgggcgcggccgccagggcgtcgggggtcgcgtcagtcatactgttcccgataggtctggacgatccgctgggcgatgatgttcaaggtcagcgtcaccaggaacagcgtcaggccgaggccgaaggcggccagcgtcttggggctgttgaactcctgatcgccggtcagcagcgtcacgatctgcaccgtcacggtggtcaccgtgtccagcgggttgaaggtcaggttggcggccaggcccgccgccatggtcacgatcatggtctcgccgatcgcgcgcgacaccgccagcagcagcgcgcccgcgatgcccggcagggcggcgggcagcagcacgcgcttgaccgtctcggacttggtcgcccccatggccgaggagccgtcgcgcagactctgcggcactgcgttcaggatgtcgtccgacagcgaggagacgaacgggatcagcatgatccccatcaccgcgcccgccgtcagcgccatctggttctgaaccagggcgagatactggccgacgccgttcagcggcccgccgatcaggaacaggccgatctcgttgaagaagacgcgcagcagcggccccaccgtcaacgccgcaaagaagccgtagaccaccgtcggcacgccggccaaaatctcgagcatcggcttgaccaccgcgcgcgtatgggatcccgcgtattccgacagataaatggccgacatcagcccgatcggcgcggccacggccatggcgatcatcatgatcaaaagggtgcccgcgaacagcgggaccgccccgaaggcgccggacgagcccacctggtccgcgcggatcgccacctgcgggctccactgcgtcccgaacaggaactcggtcaccggcaccgactggaagaagcggaacgagtcccacaccagcgacgagatgatgccgatggtggtcagcaccgccaccgccgaacagacgaacagcgcgccgtagacccagccctcgacccgattgcggatgcgcctgtcgggccgcagctgggtgaaggcccacagccctcccagtacggccagcagcaccgccgccagcgcgccgccccactgcagggtgcgctcgatgcggatcatgcgttgcccctcggcgggcagttcctgcgccaggggggccggccagatctgcagcgccggccggccctgcccgaccaggcgggcgtcggcgaaaaaggcctgacggcggaaaggctcaagctgagcgacgctttccggtgcgccggcgcggatcaaccggctttcaacgccgcccgagaaagccgcggcgagaaccagcgccagaagcgcgggcgcggcgacccagatcagggcgtaggcgccgtgctggccgggccgcgagtgcgaccgcacgcccacagcgcgacgacgcgccaccgcgcgaccgccgaaccacgccgccgcggacagcgcgatcagaacaagcagggacagccagatcattcagggtccaaccagacgccgcagggagaaaagccgcgagtctccccccgggagcatcacggcgcggaacctgcccgcgaatggtcagcggattacgacgcctggatgacagttgcgtaacagcgaaggttgacggcggcggctagggttcctgcctgggcatggggaaccaggccgtgaaggccgcgccggcccccagggcgctttccaccgtcaagccgccctggtggcggttgacgatgtgcttgacgatggcgaggcccagacctgtgcccagacgctcgccgctcttttgcccctccacccgatagaagcgctcggtcaggcgcggcaggtgctctcgcgccatgcccggaccatagtcgcgcacggtgacggcggcgtagtgcgtgccggccgctcgatccggcgtcagcagcgacagccgcgtcgccccgaccatttggctcgcaagggcctggtcgaacgtcaggccgcgccgcacggtgacgtccaccacgccgccggacggcgagtatttcacgccgttgtccaggaggttctgcaccacctgcacgatctcgtcccgctcgccgaccacgatcgtgcgcccttcggcgttcagccgcacctcgacctgacgatccttgaccagcacgctgaccgcgtcgatgacgtcggaggcggcggcgtccagcgccacgcggccggacggcgggatgtgctcgttcagctcgatgcggctgagcgacaggaggtccgcgacgagccgcgtcatgcgctcggcctgcgccgccatgatgtccagaaagcggtcgcgagcgcgcgtatcgtcgcgcgcatgccccttcagggtttcgataaagccgctcagcgacgccagcggggtgcgcagctcgtggctggcgttggccaggaagtcgacgcgcatcatctcggtccggcgggcatccgtttcgtcgcgcagcaccagaagcgccagggcttcgcctggccgtgtgggcgacagcggccgcgtccaggcccgccatcgccggtcgcgggccccgccggtcgcataatccgtgacctgcgacacgccgccgaaaagcgcctcgtccaccgcctccagcacgccgggatcgcgcatgacctggaccagcagcccgccccggcgttgcaccctcaagaggtcccgcgccgcctgattggccatgacgatgcgacgaccggctatgtcgtccggctcctcgccgctgacgatcagaaccgcgtcctccagcgcctcaagcgcgccgtccagcagttcggacgaaaccagcgcctcgccttcgggcgtttccggcgccagcggctccacgcctggtgaaggttcgcgggagcggctgatcagccaggtcgacgccgcgaccagcacggcccctccgatcaacgaaggcgccagttccggatgcaggaccgccaggccgacaaggatcagcgccgccacgccgccgctggcgccggcggtccacagccgcgagccggaggcgggcgcgacaggcgacgacgagaattcgtaagacatcttacccctggcggcttccggcgttcggactcgaccatcctcgcctgtcgctgaacctctccttgcacggagattgtgacggctgatcgaggatgtttcccgacgcaagcttcgccgcacggaatcttcagaagtgcgtggcagggtcgcgggcgaagagagatccgccttgaaccgtttcctgttttgtctggcccttgaacacgattggcggttgacgctgctggcgggccttgtctgcctgatcggcgtcgccaccgcctttcatctgatggagcgcgcgcgcgtccgccgaggccttgttcgtcgaaacaagatcgtgctggcggcgctggtcggcgcactggcgatctgggcgacgcacttcatcgccatacagggctatgtcgcgggcgcagacatgacgttcgacccctggatgacgctggcgtccctcctcgtggcccttgtcggcatcggcgcagggatcgtcatggccatggccggcgccaattcgctgacgcgttgcgtcgcggcgtccgcgggcgtcgccagcatcgccgccatgcactacatcggcatggcggcgatgaacctgccgtctgaagtgacctgggatcgtggactcgtcgttgcgtcggtgatcgcggccatgatcgtcgggatcggctctgcagcctgttaccgccgggacgaccgcctccggttctggatcaccaccgggggtgcggtgctctcggtgcttgttcttcacttcctaggaatggcggcgctgacgctgggcgcgcctgtgtccgtcgcgcctcgcggcggcctcgacccctcttccatgcagatcatcatggccggcgccgtgctgttcgtgatcggcgtcgtcctgatcagaagctggacgaccttcaccgcacgatccggcgccttgcgccagatccgcgaggcggtcgacgccatgcccgatggcttggcctttttcgactcggaagaccgcctggtgctgtggaacgcgcgctttgtggaggtgaatccggagatcgccgatcacctcagggtcggcatgacgggtcgcgacatcctgcagctcggactggatcagcagatctatccggacgctcgcggtcgggagacggagtgggcggcggaacggatgacccaccgcacccgcctgtcggccgtccttgaacagcaggtcgtggatggccgctggctcagggtgcagcaccgctcgacggcggaaggcggcgtcgtcaccgtctgcaacgacatcacggacctcaagaacaatgcccgcatcctggcggaggcgaaggacgcggccgaggccgccaatcacgccaagagcctgttccttgcgaacatgagtcatgagatccgcacgcccctgaacggggtcgtaggcctggctcaggtgctcgcaagcagcgatctatcggacgagcagcgcgagatggttgacctgatccaggcttccggggccacgctgcagacccttctgggcgacattctcgacctggcgagggtggaatccggccgcatcgaactggacgaacagcctttcagcctgcctgagttggtgcaggaggccgcgcacctgtatgcggcgaacgcgcgagagaagcgtctcggcttccacctcgaaatcgcgccggaggccgccgtctgggtccatggcgatgcggtgcgcatcaaacaggtgctgaccaacctgatctccaacgcggtgaagttcaccgacaacggctttgtcgccgtgcgtgttgaacgcgcggccgaccgggaagacggcgcggcctgcctgcgcttcacgatcgaggacaccggcatcggtttcgacgcggacgcccgcgagcgcctgttcagccgcttcgagcaggccgacagccgcatcacgcgccgctatggaggctccgggctgggcttggcgatctgccggcaactggctgagctgatgggcgggcggctggactgcgaaagtgagcccggcggcggctcggccttcatcttcaccctgggccttcgtcaggccgaggctccgcgcgttcccgaaccggccgtctgctcggaaacgaacgctcccctctcccgcagggttctggtcgccgatgaccaccccacgaaccgccgggtggtggagctgatccttgctcaggcgggtgtggaactgacgtcggtcgagaacggggccgaggcggtcgcggcggtgcgcgcctgcgatttcgacctgatcctcatggacatgcagatgccggtcatggacggcctgaccgcaacccgggaaatccgtctgcatgaggcgacgctgggtctgccgcgcaccccgctggtgatgcttaccgccaacgccatgcccgagcacgtagcggccggccaggcggccggggccgacagccacctgtccaagccgttcaacgccgccgaactgctgtcgctggtggagactccgcaggccttgctggctctgcatcggatcgccgcctgacgcccaagctggcggttgcgtatcgagtgtgatgcgtgtattagcccgcgctcttgaattcgagggtgcatcaccccgtcgcgcatgcctggcgtaggcgcggcgtttccgttgtttgttgaggcgagccacatggccgagatcattctgaacgtggacgtccgcgaaggcgtcggcaccggcggcgcccgcgccgcccgtcgcgccggctcggtgccgggcatcctgtacggcggcgacaaggcccccgtcgccatctcggtgaacgagaaggacttccgcaagtcgctctacaccggcaagctgctgggccacctggtgacgctgaagtacggcgacgagacccagccggtgatcgccaaggatgtccagttcgaccctgtgtcggaccgcccgctgcacttcgacctgatgcgcgtcgacgagcatgcgccggtcaagatctccattccggtccacttcaagaacgccgacgaggcgcccttcacccgtcagggcgggtcgctggaagtcgtccgtcacgaagtcgagatcctggtcaacgccgacagcatcccggaagaactggtcgtggacctgaccggccgcgagatgggcgacaccatccgcttctcggacatcgccctgccgcaaggcgcctcggccaccatcaccgaccgcgatttcgtgatcgccaccatcaaggtttcgtccgccgccctctcggccgccgccgatgaagccgccgaagcgcccgcttcggaagcctgatccccggatcaccgctgaagacacgccccgcccggcttgccgcggcggggcttttctttgcccgtcgcggacggcatgaggacgccatgatcatcatcgccgggctcggcaatccgggcgccaaatacgaaaagaaccgccacaacatcggcttcatggccgccgacgagatcgcccgccgctggcgattcggcccttcgcgcgccaagttccagtcggtggtggccgaaggcgaggtcgagacggcggacggcgccgtccgcgtcctgctgatgaagccgcagaccttcatgaacgagagcggccgtgcggtcggcgaggcggcgcgcttctacaaggtcaagccgcaggacatcatcgtcttccacgacgaaatcgatctggcgcccggccgtttccgcatgaagaccggcggcggcgcggccggccagaacggcatccgctccatcatcagccaggtgggcgccgacttccgccgagcgcgcatgggggtgggccacccgggcgagaagcacctggtcatgccgcacgtcctgggtgacttccacaaggccgagcagccctggctgcaggccctgctgaacgcctgcgccgacgccctgcccttcgcgcttgccggcgacgacgagcgttatcagggcgaggtgctgcgtctcgcgcccgcgcccaagttcagcccccgccaggccgcccgcggcgaactgtagaaccggacgccctagccgcgtccgacaaaacgccgtaagcctttgcggtgaaccgcacccaggtcgagaactggtccgccgcgcgctgcctggccttcctggcggcggtgttcgccatcgtgctcggctcgctggttccgttcgcggccatggcggccgctcagcccggccatcccgttgttctgtgctccagcgagggtccgcagaccatccacgtcggcggcgtggacggccccgccaagaagcaggcgatcgccaagtgcgcggcctgcctgcaaccgctcgccgccgccctgcccgcaccgcccgcgccccagccgcagcctcccgtgccgctggcggtcgagacgatctggcctgtcgcttcggccgcgcctccgccgccggcccgcgcgccgccccggccgccgtccaccgcccctcccctcgcctgaaccgaccgaaccgccgcgcctgaaccaggcgtggtccttctggcctgttcaggacccttcatcatgctttcaggaacaatggcggcgccgtgggcgctgctgctcgccgcacaggcggcgcccgtccagcccccggtcgcccagcccctcgccgcccagtcccccacacagctcgacagcgtcatcgtcaccgcgagacgcaaccccgaggatccgcccgtggtggccgaggcgcgcgcgcgcctctcgcgaacgccgggcgcggtttcggtcgtctcggccgagtcctaccaggatcggtacgcgcccactctcgccgacgtcctgcgcgatgcgcccggcgtttacgcccataagaagtggggcggcgacatacggctgtcgatccgggggtcggggatcggcaactccgtccacaatcgcggcgtgctgctggcccaggacggcgtgccgttcaacgaggcggacggctttggcgactttcagctgatcgatccgctgatcgcccgctacactgaggtctacaaaggcggcaacgccctgcgcttcggcggggccttgctgggcggcgcggtcaatctgctcaccccgaccggccgcaccgccgcgcacgatctttccctccggctcgacggcggcgcctacggcgtggtgcgcggccacgtcgaggcggcgggcgtcagcggcgactgggacggcttcggcgccctgacggtgcagagcgtggacggctggcgcgaccagagcgcaggctccgaacagcatgcgtcgctgaacctcggccgccgctttggcgaagaccgcgagatccggctgatcgccagcgccggcaagatcgaccagcagatccccggcagcctgacgctggatcaggccctgaccgatccacgccaagccgcctcggccaatcgcagcctgaactatagccggaacatggagtccctgcggggcgtgctccagacccgctggcggctggatgcctccaccatcttcgagggcggcctctacgccagctggaaggacctgaaccaccccatcttccaggtggtcgatcagcagagccgcaacatcggcctgttcggccgcatcgactggcggggccaggcgttcggccgccgggcggacgccttctacggcgtgtgggcgcggcaaggcgatctggacgccaaccagtgggtcaaccgcgccggcttcaagggcgcgcacaccgcccgcagcaaccaggacgcccgcgccctggacgtcttcgccgagggtcggctgttcgtcaccgaccggctggccctggtcggcggcggaacatggggccgggccgaacgcgactatcagagcttcgccctccccggcgtcgcctccacattcgacctgacggccgagcgcacctatgactggttcgccccacgcgtcggcgtgctgtgggagactgaaaacggcgctcaggtctacgccaatatcacccgttcggtggagccgccgaacttctcgtccctgtccccgaccgccgccggcttccagccgctggtggcgcaggaggccacgacgtgggaggcgggctttcgcggccggggcggcccgctgttgtgggacgtcgcggtctaccgcgcggaccttgagcacgaactgctgaacttcattcccaatgcggcgctgggcgtgcccgccgcgaccttcaacgccggtccgacgatccattcgggcgtggaggcgggcctcgactggaagattgcgccctcgctgcgcctgcgccagacctacagctggtccgatttccgcttcgacggcgaccgcgtctatggccgcaaccagctcccggtcgtgcccgagcacctctaccgggccgagctgcgctatgaccaccccgccggctggttcgtcgcgcccttggtcgagtggtcgatccgcgacgcctgggtcgatcacgccaacaccctgaagtcccccggctatgcggtcgcgtcgctgaacgccggctgggacgtgacgcgttccgtcagcgtcttcgccgatctccgcaacctgttcgacgagcgctacatctccaacttcggggccgtcaccgacgcgcgcgcggcctccaccgccgtcttctttccgggagacggccgttcggcctttgtcgggctgaggctcagctactgatgtccgcgctcgcctcaaacgccgccgcgtaccgcttcgtctggcggtggcacttctacgccggcgtgatcgtcatgccgtttttgttgctgctggccctaacgggcggcctttacctgttcaaggacgagatcgatcaggcgctctaccgcggcctaatccgcgttccggcttccgctcagaacgcctcgccggacgcctggatcgacgccgccgctcagacgggtggcggtcgcgccgccagcgtcattgtgccttctgccccagaccaggccgtgcgggtgcgcgtggaccgtgcgaacggcgagcagcgcaccgtctttgtcgatccgcacactgcgcgtgtcaccggctccacagcggtgggcggcgtcaacgagacgatcaagcggctacattccatgaccctgttcggtccggtcatgaacgtggtggtggagatcgtcgccggctgggccatcatcctgtgcgcgacaggcttttacctttggctgccacgcgggcggccggtcggcgccgtgaccatcaccgacacggacgtgaggcgacgaccgttctggcgggacctgcacgcgatcacggggctttatgtcggggcggtgattttgttcctggccgtcacggggatgccttggtccgccgtctggggccaacaggtcataggttgggtgcgggaaagcgggctcggtcgaccgcccacacccgtggctggcgcctggcacaaggcgcagggtcatgaccggccgaccggcgcggggtggacgttggaccatgccgccctgaccgtctcggggcacagccgtcacacggccacgtcgagcctggccgtcgtcatacaggcggcggaacgcgccggcttggcgcgaccctatgcggtgacgatcccgtccgacccggccacggcctacacggtcactcaccaggcgcgacgagtcgagaacacccgctcgctctacgtcgacacccgctcgggcgcggtggtcgacgacatccgctacgcccggttcggccccgtgggcaaggccgtcgactggggcgtggccgtccaccagggcctccagtacggccagatcaaccgcctcgtcatgctagccggctgcatcggcgtgtgggtgctggcgatctcgggcctgatgatgtggtggaggcgcaggccgccgtcgctgtcgcgtggccgcctcggcgccccgtctccgctcgcggatgcgcgcgcccgcacggcggccatctgcattgtcgcgcctcttgcgatcctgttccccctgaccggcgccagtgtggtcgcggccctcctgatcgagagagcggcgcggggcctgcgccgattcgccccctcgcgttcaaatccattgcactgaaaggatcgcgccatgatgaagcgtcttcttctcaccgccgttctcgccctcgccgcctgcggcgggccgcaagctccctccgccgtcacggcggccgacgcctggtgccggccgacgccgaacggcgcgcgcacgggcgcctgctacctgtccctcaccgccagcgccgatgaccgcctggtcggcgccgccagttcacgcgcgagcgaggtccagatccacgagatgaccaccgagaacggcgtcatgaggatgggcgaactggccggcggcctgcccctgtcccagggtctggccgcgtcgctccggcccggcggcgttcacctgatgctgatcggcctgaacgtccccctggtcgctggcgagacagcgcccctgacgctgcgcttcgacaacgcacccgagatcaccgtgcaggcccgaattcgccaaccctcggcccacgacatggcgcactgacgcgccgatccaagcgtgagcctgacaaaccggccgcgaccggctaaaggctcgcgctcctcactctccacgcctgaaagcccgccgccccatggccctgaaagtcgcgatcgtcggcctgcccaacgtcggcaagtccaccctgttcaacgccctgaccaagacggcggcggcccaggcggccaactatccgttctgcaccatcgagccgaacaccggcgacgtggccgtgcccgagccgcgcctgaacgccctggccgagatcgcgggctccaaggagatcatccccgcccgcatcaccttcgtggacgtggcgggcctggtgcgcggcgcgtcgaagggcgaaggcctgggcaaccaattcctggccaacatccgggactgcgacgccgtcgctttcgtcgcccgctgcttcgtcgacgacgacatcactcacgtcgagaaccgcatcgacccgatcgccgacctcgagatcatcgagaccgagctgatgctggccgacctcgaaagcctggagcgccgccgcgtccaggtcgagaagcgcgccaagggcggcgacaaggaaagccagctgaacctgaagctgatcgacctggcgctggagcagctgaacgccggcaagcccgcacgcctcgccgaggtgtccaaggaggacaggaaggcctgggacatgctgcagctgctgaccgccctgcccgccctctatgtcgccaatgtcgaggaggcctcggccgaccagggcaacgagctgtcggccaaggtcgcggcgcgcgcggcggccgacggcgccaactcggtcgtcatctccgcccagatcgaatcggagatcgccgtcctcgacgacgaggaacagcgcgagttcctggagacgctgggcctggaagagcccggactgaaccgcctgatccgcgaggcctacaagctcctaggcctgcagacctacttcaccgtcgggcccaaggaggcgcgcgcttggaccattcccgtgggcgccacgggccctcaggcggccggcgtcatccacaccgatttcgagaagggcttcatccgcgccgagaccatcgcctacgccgactatgtcgcgctgaagggcgaggcgggcgcgcgcgacgccggcaagatgcgtgcggaaggcaagagctacgtcgtcaaggacggcgacgtgatgcacttcctgttcaacaactaggcgtcagtcgttcttcagcaggccggcgaaaccagcgggcccttgcgccttgggcgatcccggacagcgatacagctgcacggccgccccctcgcggtcgaggtaggacaggttcaggatgtcctcggtgaccgccagccgcacatgctcgcgcacggcgcgtccttccgcctgacaagccagctcggctacataggcgtcgtccacctcgaccaccgaggcgacctcacagcggttctcatagccgtcgaaacgggtgggcgtgatgacgatgggggcttggtcgcccgccggccgcgcgcaccaggcgacgttcgccgcccatcgtccgacaaagctggccggtccggtggcgggtccggcggaggccggcgcttcgcccacgtatgtgcccgagcccgtcaccggctgggccggctcggtcggtgggttgacggactgacgctcgcagcccgccattcccaacgtcagggcggcggcgatgatggggagcggcgctctcatggcgctgcaacgcatcagttccgcccttgttcaggccgactgtccgcctgtcctaccgccgcgcgtcgtcgctcgcagcccgcaccgcaccgaactccgacgtcggcttccaggtgggccattcctcgctgttggccagctgaaggcccagtcggtacagcagcgtcaggttctgcacagcgccggtcatatcccaatccgccgaccattcgtccgacgccttgtgatagacgcggccgaagcgctcgcgccacgccgcccagccggcctccttgccgccctcgacgaagtccacgccatgccacggcataagcgccgggacgcccgcgcgcgcgaaggggaagtggtcggagcggtagtagaagccctgctccggctggccgtcgtcggagacgtagcgcccctcggcctcggccaaggcgcccaggctgtcctccagcgagttctgccccttgccgaagatcggcacgtcgcgcgtggcggggctgagcggcagcatgtcgatgttgatgtcggcgaccgtggtctccagcggataaaccggatcggcgacataggcgtaggagcccagtagccccatctcctcggccgtcatgtgcgcgaacacgatggtgcgctcaggctgcggcgcggccttcagctcgcgcgccatctccagcacgccgatcgtgccggacgcattgtcccatgcgccgttgaagatgttgtcctcgccgccggcgtgctcgccgccgacgccgatgtggtcccagtgcgccgaatagacgatcgtctcgttcggccgttccgatccggtgatcttggccagcagattgtgcgtggtcagggtgtcgatggtctcggacgccttcaggttcagcgtcacgccgtccagcgcctgcgccttgaactggccgctggtcgccgcctgcgtcaggctcgctggatccagaccgcccgccgtcagcatggcgttcgccacgtcgctgttgaccgagccggtgatctccagatcggccgcgccggggctcagggtgcgcacgcggtccgccccgcgcagctggcgccgccagccgtcactgtcggccgcatccttcagcacggtgatcacgcccacggcgcctcggcgcttggcctcgtcggccttgtaggcggcggactggtagttggtggtgtagggtccgttgaacagctcgccgtccggctcgcccgccagcaccacgaccaccttgcccgcgacgtcgaggtcgccgtaatcgtcccagttccgctcgggcgccgtgatgccatagcccgcgaacaccacgcccgcgtcctgcacgtccgcctggccgtcgttggacacggcgcgcagggtgatgtcctgacccgccgcgagcggggtcgaggtcccatccttgccccaggacgcggcggcggcgcccgcgacgggcgtgtagcgattcagctcgaccgcctgaagccattggccgtccggccctccgggctccatgcccatggcctcgtactgcgcctgcagccacgccagcgtcttctgctcgccctcggtgccgggcttgcggccctggaactcgtcggtgctgatggcgcggatttcttcggacagccgctgggcggagaagtcctgggtggaggccacgccgcagatcaaaagagcggcgaggccgacgccggaagcaagcgaaacgcgcatgaacgatctttcccgttgaggatcaatcgcctgtgtaaggaggcgcaggctcatcgcctccttacattttcgtcatgtttcagcggcggctggcgtcgctgcgctcgcgcaccggcccgaattccgaccccggcttccagcccggccagtcgcggctgttcgccagatcgcggccgatccagaacagcacctgcaggtcctcggccatgccgcgcaggtcccagtcggcggaccattcgtcgtccgcctggtgatagcggctgcggccgtattcggccgccgcgtccttcttcgcctgcaccggctcgtccaggaactccccggccgtaccgggataggccatgggcacgccgcgcttggccagcgggaagtggtccgagcggaagtagccgccgccggcgtccgccccgcccgtatccatggcgcgtccctgccgcgcggccgccgcctccagccgctcgtccagctcggactggccgcgtccgaccgccgagatgcgttccttgcggccatagacgttcatggcgtcgatgttgaagcccgcaacggtggcctccagcggatagatcggattggcggcgtagtattccgaacccagcagaccgctttcctcggcggtgaagctcagcatcacgatcgagcgctcggggcgcggcgcccgcccccacagacgcgccagctccaagaggcccgccgtgcccgacgcattgtccaccgcgccgttgaagatgcggtcgccgctcgcatccggctcgcccacgccgatgtggtcccagtggccggtatagagaatggtctcgtccggatgcgtcgcgcccggtaggcgagccaccacgttgcgggtcgtcacctgctgcgtcgccacgtcgaagcgggcggacagcttcgcgtccggcagggtcgtcggttggaagtcgcggctgcgcgcctgcgtcttcaacgcctcgaagtccagccccgcccggcggaacagctcaaccgcgccgtcacgctggatccacgcctccatcggcacgcgctcggcggaggcgttctgccgcacgatgtcgaactgcggcccggaccagctgttctgcacggtgttccagccataggaggccggcgcctgctcgtgcacgatgatgacgcccgccgcgccctggcgcgccgcctcctcgtacttgtaggtccagcggccgtagtaggtcatggagcggccgttgaaggtgttcagcgccggctcctcgaagtccggatcgttgaccagcacgaccagcaccttgccgcgcatgtcctggcccttgaagtcgtcccactgccgttcgggcgccttgacgccgtagccgacgaacaccagcggcgcgtccgcgaggttgaccgccgtccccggcaggcgggtggagaccacgacgtcgcgcccctgcgccaggtcgcgccgccagtcacccaccgacaccgacgcctggacattggaggccagaaagcggttcagcgtcacatcctgggtccagccgccgttctctccgcccggctgaaagcccgccgccgcatactcccggctcagatactccaccaccttgtcctcggcgggcgtcgcgatgccgcgcccttcgaagctgtcgtccgacagcgcgcggatatcctccgacacgcgcgccagatcaatggcgtcgccgcccgctccgttcggcatggtggcgcaggcggacagaagcccggccgcgacgagcagggcggccgaagaggaagcgaggcgcatgaaggaggtctctggatcgtgactgacccgacgaccttagcagccgcttcgcccgtgtcgatgcggcctagcggccggttcgggcgttgcagatgcgggtcacctcacccgcgatatccttgtggggcgtgttgtccgcctgggcctgggcgtcgccgcacctgccctggccgatcagctggtccagccggtcagccaacgccatgcgatgttcatacacacgctcgttgtgctccgcctgactgaggcgtcggcgcacatcctgaatccacaggttgcgctcgttatcagcgaaccggtccatggtgcgggtcgcggcgttggggttcggcgcgatcacctgatggttggacgggggcgttgcctgtttgggcgcggcctggccctccggtgcgaaaagggcggcgaaggcgaaggcggcgatcagcgacatcccggaggctcccatgttcggagaaccgacttcatcaccatccgccgccccgcgcaaccacgccttgcctttagtgcgccacgcccttccagatgcggcggtagctggcgtaggtcaggccggcgaagatcagaagaaagatcatcacgcccacgcccgcctgcttgcgctcgaccatcttgggctcggacgtccaggcgatgaaggcggccacgtccttggacatctggtcgacgctggcgcgcgtgccgtcgtcataggtgacctgaccgtcgcgcaggggggccggcatggcgataaagccgccggccggcacgtgctcgggatcgccggtccagaacggcgtcaggtcgccgttcatgtaggcgttatagttctgaccctgacggatctgcagccccgccggcggcgcgtgatagccggtcagcagcgaatagatgtagttggcgccgtcgtgacgcgccttggccatcaccgacaggtcgggcggagcggccccgccgttggcggcggcggcggcggtcgcgttgggatagggcgacgggaaccggtcggccgaggtggcgtcacgttgcagcgcctcgcccgtctcgctgtcgatgtcgggcacctggatctcggcggccagcgccttgaccacggggttgtcgttcgggttgggatatttcgggttccagaacggcccgttgcggtcgcccaggttgcggaagtgcaccaggttcatgctgtggcacgaggcgcagacctctcggtacaccttgtagccgcgctgaagctgaccctggtcgaaggtcccgaacggcccctcgaagctgaagccgcccgagcgcgggtggtgcgcgccgccctcggccagggcgggcgccgcagtcagcaggccggcggcgagaacggccgaagccagggtcttgagcatggaggttctcatcgcgctcagccctttgtctcgggcgacgccggggcggcggcggtcagggcgggcgcgccatgaccggacagcaccggttcggagatggtggccgggatcggcaagggcgtctcgcgcaggcccaccaccggcatgatgaccaggaagaaggcgaagtagtaggcggtgaacagacgcgtcagccacaggtaggagttcagctgtccgtcgaacagctggaaggacggcatgccggggatcacctgggcgtccggcagctgcgccccgcaccagcccaggcccaggcccaccaccagcaggatgatgaagaaggtccgcatggtcgggcgatatcgcatcgagcgtaccttggaggtgtccagccacggcaggatgaacagcacgccgatggccgcgaacatcgccaccaccccgccgaacttgtccggaatggcccgcaggatggcgtagaagggcagcatgtaccactcgggcacgatgtgcgccggcgtctgcagcggattggcgggaatgtagttgtccgcatggcccagcgcgttgggcatgaagaagacgaacagggcgaacagcatcaggaacaggatgaccgcaaacccgtccttgaccgtgaaatacgggtggaacggcaccgtgtccttggccagccggttcttggggatcaggatgccgaccgggttgttctggcccgcatggtgcagcgcccacaggtgcagcaccacgcatccggcgatgacgaacggcaggacatagtgcagcgagaagaagcggttcagcgtcgcattgtcgatcgccggtccgccgcgcagccagatcaggatcggctcgcccagcaccggcacggcgccgataagattggtgatcacctccgcgccccagaacgacatctggccccacggcaggacgtagcccaggaaggccgtggcgatcatcagaaagaagatcacgcagccgatgatccagatcatctcgcgcggggccttgtacgatccgtaataaagcccccgcagcatgtgcagatatacggcgataaagaacatcgacgcgccgttggcgtgcacatagcggatcagccagccgccgttcacgtcgcgcatgatgcgctcgaccgaggcgaaggccaggtcgacgttgggcgtatagtgcatagccagcacgatgccggtgacgatctgcgtcatcaggcacagggccaggatgccgccgaacgtccaccagtagttcaggttcttcggcgtcggcagcgaggcgtagttggcggcgaagcggacgatcggaagccggctgtccagccacttctcgacgccggtcttcggcacataggtggattcgtgttcgctcatgtccctccccctggtcctcagccgatctttacgcgggtgtcggacacatagtcgtattcaggcaccaccagattggccggcgccggtcccttccggatgcggcccgaggtgtcgtagtgcgagccgtggcaggggcagaaccagccgccgtagtcgcccgccccgaacgtcggcacgcagccgaggtgcgtgcacgatccgaccaccaccaggaactgctgatgccccgccttgacgcgatcggcgtcggcctgcggatccttgaggtccgacagcggcgtcgccgccgcctcctggatctcgcgggcggtgcgatagcggacgaacaccggtttgccctgccacttgatcaccacctgctggccttcctgaaccttggtcaggtcgaactcgatggaggccagggccagggtgtcggcggccgggttcatctggttgatcagcggccaggcgatcatggcgcccgcgccgaccgccgcggcgcccgccgcgatgtggatgaagtcgcggcgcgtggcgtcgccgccgtccgcatccggggtcacgaccgattcggccaaaatgcacctcccatacgccgaccggctcgcctcgacgacgcgccggcccggcttcgtttcctcagcttctttccggaaattcgaggccgcctcagcccctttcggcccctcgccgaaaaggactgacatcattgcgaaaggctcgcaaaaggccgcgacaaatccccaggctgcgcttagtgtccggcttagaatgcgtctcgccctttttcaaccggacattcctcagaacgtcggcgcctgcatccggctgtcggcctgcttcggggttccgctgcatgtgatcgagccgacgggctttcgcttggacgaccgcgccatgaagcgcgccgctctcgattacggccccctctcgcacatgacgcgccatgccgattgggacgcctttcagcgcgaccggggtccgggacggcttgttctgttccccacccgaggcgccgagccgctccccgacttcgccttccagcccgacgacgtgctgctgttcggcaaggagagcgccggcgcgcccgactacgttcacgccgccgccgacgcccgcgtggtgatcccgctgaggccggatgctcgctcgctgaacctctcggtcaccgccggcatcgccctgtgggaaggcctgcgtcagaccggcgctttcccagcaggcggccagttgcggattaaccgagccgattaaagggccgcaaaccgcccgccgccatgatgcggcggttcggagggcggtttggacaatctgacgacactgatcgcgatagctatcttctgcgccttcttcgcgggcaacgtcttctccagcacgcaacggcgttggcgcggacgcaaggccgcgaagtctaagagcatgccctggcggcctcaatcgtcgcatcggccgcagcgcgagccccttcagacgccgatcaccgacgcagccgaacagctgcgcctcgtcatgcaggcgtcgttcgacaagaagcggctgatgtccaaggacgaagccagggtcttcatgctgatcgagcgcgcggtgaagacgcgcgacctttcatggcgtgtgatggctcaggtcagcttgggcgagatcatccgatcgacaaaccccaaggcccacgctgctatcaacagcaagcgcgtggacattctgctgatctcacgcgacggcgttccgctggcggcggtggagtatcaaggatcagggcactacctcggcacggcggccgcgcgcgacgcggtcaagcgcgaagccctccgtcgcgccggtgtcgccttcatcgaaattgatccgtcccacgagccggcggatatcgatcgggaggtgcagcgcttggccgaccggatagccgcgcccgtcgcctgatccgtggcctactccggagccggggcgtccggcaggcgtgacaggttcgggcggtcggcgcgcttgcttgccgccacggcctcgacggcgcgcatgacccgcagcacgttgccgcccgccagcttgcggatgtcggcctcggtccagccgcgcgccatcagcgccgccaggatgcggggataggcggcgacgctttcaacgccgtccggcaggctcccgacaccgtcgaagtctccgcccaggccgacatggtcgatcccggccacgtcccgcacgtgctggatgtggacgaccacgtcgtccagggtcgcgcgcggctgcacgttcgccgccatccaggtccgaagaccgcccgtcaccgcatcgggatcgccggggttcagcgacttcagccgcgcttcctcggccgcccgcgcggcgccccaggcccgcacctgctcgctgatgaagccgggcacaaaggtcaccatcaccacgccgccgtcctcaggcatcatgcgcagcacggcgtccggcacgttgcgcgggtgattggtcaccgcgcgcgccgaggagtgggaaaagatcaccggcgcttcggacacccgcatggcgtccagcatggtctcttcggacacatggctcaggtccaccatcatgcccagccggttcatctcacgcaccacctcttcgccgaaggggttcagcccgccccatttcggcgcgtccgtcgcgctgtcggcccaggtcgtggtggtcgagtgggtcagggtcatgtagcgcgcgcccgcgtcatggaactcgcgcagcagccccagcgaatcgtcgatggagtagccgccctccatgccgatcaggctggcgatgcgcccgcgccggtgcacgcgctcgatgtcgtcggcggtgtaggccagttcgaacacgtcggggtgggcgccgaccagccgcttgacgctgtcgatctgctcgaacgtcgccttggccgcctccacgggcgggaggcttgcgggcacatagaccgaccagaactgggcgcccacgccgccctgacgcaagcgcgggatgtcggtgtgcagggtcgtgggattggcgctctgatcctgcgtcagatcaaccgcgtgcgggtcattcccgaacccctgcctcaaggcccagggcaggtcgttgtgaccgtcgatcaaagggctgcgctccaggatgcgccgcgccctcgcctctcccgccgtgtcctgcgccagcacgggcgcagccagcaccgtgatcgaggcggcggcgagaagaagggatcggatcatgcgcaaagctcctgaacggtctcctccaacctgacagagaccgatcgcgccagtcaaagctttccccccacgcgcggcaaggtctatggacgcggccatgaccgacctgctctccgacaagaagaccgagacgcgcgcctggttcgaagccctgcgcgatcgcatccactcggcgtgcgaggcgctggaggatcaagcgcccgccgatctgtttcccagggagcccggccgcttcgtccgcacgccctgggaccggccggagggcggcggcggcgtcatgggcatgatgcacggccgcctgttcgaaaaggtcggcgtgcactgctccaccgtgcacgggacctttcccgccgactacgccaaaacagtgccgggcgcggccgaggacccgcgcttcttcgccaccgggatcagcctgatctgccatccgcgcagcccgcgcgtgccggccgtccacatgaacacccgcttcatcgccacaacccaaagctggttcggcggcggcgcggacctgacgccggtgctggacgtggatcgtcacgcggacgcgcccgacaccgtggccttccacgccgcgctgaagtccgcttgcgacgcccatcacggcggctggtacgacacgttcaaggcttcgtgcgacgactacttctttctgccgcaccggaacgagccgcgcggcaccggcggcatcttctacgaccatcacgacagcggcgactacgagcgcgacttcgccttcacccgcgatgtgggcgaggccttcctgacggcctacgtcgatatcgtcgcccgccgcatggccgagccctggacggaagccgagcgcgaggagcagctggtgcggcgcggccgatatgtcgagttcaacttgctctacgatcggggcaccaccttcggcctgaagaccggtggcaatgtggaatcgatcctcagctccatgcccccggtggtgaagtggccgtgaccgcctagatgccgctgccgctctcttccgtcggcggcggggtcagcagcaggaaggcgcgtatccaggcggtcagcaccgcgcggtcgttgggacgcttgaggctttccagcgcctgctcggcgaccgcctccgggatgcggtcgcgccggccctccaccagggcggcggcgtagtccgggccgaactccggatggcactggaacgacacggcgtcgtcccacgccagaccggccaaaggcgtgaatgcgctggaggcgatcacgcgcgatcccggcggctgcaccaccacctgatcctggtgcgacacgggaatggcgatgctgtcggcgcgcgggtgcatccagtcctcgatccccgacacctggtagcggtgcaggccgacgccccagccgcggtcggacttctccacgtcgccgcccagggcctgcgccatcgcctggtgcccgaagcagatgccgaccagccgcgtcttgcctcgcgcatcgcggatccagtccagcagcggccggatccagggcaggtcgtcgtacacccccgccgccgatccggtgacgatggcgcccgcgaagtcggacggatcgtccggcagccgcccggcctgcacgtcgaaacgcaccgtcgccacgccctcgcccagcaacgcccggaaccgggctggatagtcgtcgaacgcgtcgcgcagcgcctcgggcggctggccggtttccaagatggcgatgggcttcatgcgcctgacctaagcacgcgggcctacaggcgccacacctcggccttgccgccgggctcgcccaacgcctcgaccacccagccgcagatctcgcgcgcggcggcgtccgctccctccggcgggttcagcaccatcatggcgcagccgttcatcttcatcggattggtcagcggccgcagccgcgcctccgccaccagcactggtccggacagccggcgcaggaatccgtccagcgtctccatgtccttcagcggcgtccacacagcgaccacggccgctcgcctcgccgccgccatccccgcctcggccgagcggacgtagtcgtccggccgctcgaacggcgggtcgatcagcaccagcgcccccggccgcaccgaccctgtcgccgcatagccgtcgcccgcatgcgccgccgcttccggataggcgtctagcgcctcttccagcagttccagcaccggcgggttcagctcatggcctacataggcgtcacccggccgcagcgcgcgcgccgccagcagcggcgaacccgggtaaaggcgcgtctcgccggccgcattgatcgcccgcacggcctcggccagcgcctgcatgcgcggcggcaggccgtccgccgtcatcagccgctgcaccccggcctccgcctccttcgagcgcgcggcgtcgccgctcaggtcgtacagaccggcgccggcgtgggtgtccagtacctcgacgcggcccctctcccgccgctcatccagcagccacagcagcagcgcgtgcttgaccagatcggcgaagtttccggcgtgaaagctgtggcgatagttcatgccgcctcgtcccctgctccgccccgggggtcaagcggaactcgcgccttcgccgccgcgttcgtcgcaggcttcaacggacccgcgccatggcctccaagacccccttcaccgacaagcagcgcaccccgcccaagggcgtcgccgactgcgcggcaaaggggctggagctgcgcgaacagcatggccggggcggcaccgatgtcggccgacggcgcgccgaacagctgaagggtcagcatgccgtcagcgagcgcgacataaagtcgatgtacagctacttcgcccgccacaacgtggacaagcgcggcaagaactggggcgatccggacaagccgtctgccggctacatcgcctggctgctgtggggcggcgacccaggccgcaagtggatcgacgggctgcacgacaagctggatcagcaagaggacgccgcctgatggccgacggcgccgcgaccttcgaggtcgatcttgaggccccagccggtctggcctggtgcaatgacgacacgcccggcatcacccgccgccgcgcgggcaagggcttcacctatcgggacgccaagggcgcgaccgtcaagaaccccaaggtgctggaccgcatccgcatgctggccattccgccggcctggaccgacgtctggatctgcccgcgcgccaacgggcacatccaggccaccggccgcgatgtgaaggggcgaaagcagtatcgctatcacaacgactggagcacggctcgttccgagcacaagttcgacaagctgcccgccttcgcccgagccctgcccaagttgcgcgagcgggtcgagcatgaccttggcttgaaaggtgtctgccgcgacaaggtgctggccaccgccgtgcgcctgctggagatcaccctgatccgggtcggcaatgcgacctacgccaagcagaaccgctcctatggtctcaccaccctgaacaagcgccacatcgacgtggacggcgcggccatgaccttcgagttcaagggcaagagcggcgtcgagcacaaggtcagcgtccgcgaccgccgtctggcgcgcgtcgtccgcacgctggaggatctgccgggccagcagatgttcaaataccgcacggccgatgggaccctgtgcccgatcacctccgatgacgtgaacgcctacatccgcgaggccatgggcgagggcttttcggccaaggacttccgcacctgggccggcacggtgtccgcagcccgcgccttccgcgacatggacccgccgacctcgcaaacggacgggcgacgcaagatcaccgtgtgcatgaaggccgtggcgggcctgctcggcaacacgcccaccgtgtgccgatcctcctatgtccatcctgtggtcgtcgatctctatgagagcggtcgcatcgccgaggtcctgcccggctccgagaccaagggattcgagcccgcgctgatgaagctcctgaaggcgcagtagccgttcaggccgcggcccagaaggcgcggctgcgcgcgttgatcggcgcctccgccgacagattggcgatcgccgcatgaaagtcgtccgccgccgcgtcgctgaccagcagccgcagcgagcggaggatgcgggtgatccgcagatgattgtggtctaccggcgcgcgccaatgccgggtgtcgcggtagaagaccagcatccgcgccgcaccccgccgcagattgccctgcgcctcggtcgagctccgcagggccgcgacgtcagccgcactcagcaccggcgatccgggcacggcgccgctcggctcggtcagcgggaacagccactggatgtagtcgtgatggcgctccagcgccgcgtcgtcgaaggcgagcacctgctccagcgtccgccccgcccggtccgcgccgtcgccgctcagaaagtcgacgacggcgctcatccgattaagccgcccagtccagcaccaccttgccggacttgcccgaccgcatggcctcaaagccctcgcggtagttctcgtaactcatctggtgggtgatcagcggcgtgaggtcgagccccgccttcagcaggcccagcatctttctccaggtcgtgaacatctcgcggccgtagacgcccttgatcgtcagcgccttcaggatgatcgcgccccagtccgtctccatcggcttggccggaatgcccagcagcgccagcccgccgcccatgatcagggtgtccacgcactgtttgaaggcgatgggcgagccggacatctccagcgccacgtcgaagccgaccttcatgcccagctcgtggatcacatcgtgcaggtcctcgcgcgtggtgttcaccgtacgcacgcccggcgccaccttccccgccagctccagccggtagtcgttgatgtcggtcagaaccacggtgcgcgcgcccgcatgccgcgccaccgccgccgccatgatgccgatcggtcctgcgcccgtgaccagcacgtcctcgcccagcagatcgaactgctgggccgtgtgcacggcgttgccgaaggggtcgaggatcgagccgatctcgtagggtacctcgtccggcagctcgatgacgttgaaggcgggcgccacgacgtactcggcgaaggcgccctggcggttcacgccgatgccgcgcgtcttgggatcgaggtggaagtgcccggcgcgcgccgcctccgagttcaggtcgatcacgtgcccctccgccgagacgcgctggccgaccttcagccgacggtcgacttccgaaccgatggcgacgatctctcccgagaactcatgcccggtgatcatcggcgtcggcacgttcttctgggaccactcgtcccagttccagatgtggatgtcggtgccgcacaccgccgcccggtgcaccttgatcagcacgtcctccggcccggcctcgggcaccggcgcatcaatcagttcgaggccctgcacgggcccggtcttggccagcgccttcatggtctgcgtcattggatcactcccagttccttgccggccgtcgtgaaagccgcgaccgcttgatcaatctgctcgaacgtatgcgccgccgacatctgggtgcggatgcgcgcctgcccgcgcggcacgacggggaaggagaagccgatcacatagacgccgagctccagcatccgcgcggccaaatcctgagccagcttggcgtcgcccagcatcaccgggatgatcgggtgctcgccctgcagcagggtgaagccagcatcggtcatggcggttcggtagcggtgggcgttggccgacaggcgcgtgcgcagccggtcgccctcgccgccctgcgcgatgcggatggcctcaaggctcgatccgcacacggcgggcgccagcgcgttggagaacagatacggccgcgcccgctgcttcaacagttcgaccaccggcttggaggcgcagatgaagccgcccatggctccgcccagcgccttgccgaaggtgccggtgacgaagtcgaccttgaccccgtggtgcgcgaacgagccccgcccctgcggccccaggaaccccgtcgcatggcagtcgtccaccatgatcagggcgtcgtagcggtccgccagcgcccggatctcgtccagcctcgcgatatagccgtccatggagaaggcgccgtcggtggcgatgatgatgtcgcgcgccccgtccgcccgcgcctgcttcagctgggtctccagatcgtccatgtccgagttggcgaagcgatagcgcttggccttgcacagccgcaccccgtcgatgatcgaggcgtggttcaggctgtcggagacaatggcgtcctccgcacccagcagcggctcgaacagcccgccattggcgtcgaaggcggcggcgaacaggatggcgtcctcaaagcccagataggcggcgatcgccgcctccagctccttgtgaatctccagcgtgccgcagatgaagcgcaccgaggcggtgcccgcgccccagcgctcggccgccgcgatcccggcctgtgtcacccgctcgtccccggccaggcccagatagttgttggcgcagaagttcagcacctcgcgcccgttcacctggatcgcggggccctgacgagaggcgatgatccgctcgggcttggtcagcccttgggtcgagatgtcttgaagctcttgcgcgacgcgcgcgtggaatccgctggtcatgggcgcgggttacgccgaaacgcgcgacgtttccagcttgaccgatcgtcagcgatcgggctcggcctccgcacggaaggggctgacctcgatcttgcggccgcacggcgtgaagctcttgtcgaggctcagcggcgtcgcatcgttcggcacggcgacccccacgcgcgcggcgctggggcacgtcgtctcgccctcgccttcgttcggcatgacggtccaggccaggtcgaagaaggccttaccctgcgccgccagcgtcaccgcgacgggcgaccgacccgcccgcagatagccgccgggattctgctgtgcgcgcacctggctcagggctcgcccttgcgcgtcctgcagcgtcaccgtgggatagcccagcaggctgcagggctgcgcgccggtgttctgcacgccgatgatgcggacgcgatggcccatacccgcgtcgcccccgtcgtccgacagcctcagctgggcggcgcggcagggctcgacggctccgttcgctcccggcggggcggcgacgacgggcgtctgtcccggcggggtctggggcgccgagcccgccgtcggccgcgtgcagcgctccagcaccgcaaccgccgtctgtccgtcgggtccgagacggctgagggtcgcgccctcctgcccgttgcggctggcggtccaccattccacgccgtcgccgacatagcgggcgccgctggcggcctggactctgcgcgtcgcataggtgcggccgccataggcgatctgcgcgctgtcggcgttcggataggtcgccgtcaccgcctgtccgctttcgcaggcgtaggtcaccgcccccgtggatgcggcgaccgccgcgcccggcggcggagcggccgagggctcgaccggcgccgggccttccggctcgggcgcgccgcaggccgacagaagcgcgctggcggacaacaggacgacaaggcgacggcgcatggtctggctccacggttcggcgagaacaacgactgcgccggctaaaggctccgcttgccgtcgcgaacgcccgccagcaccgcctcgaccgcttccaggcacagctccaacgaaaaccgcctttgcgccatggctcgggcgcgctccgccattcgccttgcctcccccggatcggccagcagcgtccttatcgccacagccagcgccttcggatcgccgggtggaacgagcaggcccgtctcgccggcctcgaccacctcccccactccgccgccgcgtgtcgcgatcaccggcattcccgccagcatggcctcgacgatgacccgcccgaagggctcgggggcgacggaggcgtgcaccgccacatccgtcgccaccatcaagacctgcacgtccgaccgcgcgcccagcatccgcacgcgcgtctccaggcctttggtcgcaatgatcgatctcagcttggcctcataggcctcctccccgaacagcggcccgccgaccaggaccgcctgaacctcgggcaggcgggtcagcgcctcgagcagcaccgcctgccccttccactcggccagtcggctgaagacgccgaccaccggccggtcggacgcaaggcccgtttcggtcagcaacgccccgcggctccttgtgcgctccagcccttcaaacggcgtcgcatcgatgccgttgtggatcacacgggcgtgcgggccgcccgcccgcctcagcgcctcggccgtagcttgcgagttggcgatgacctcggcggcggccgcccggccgagccacgccacgccccgacgccacccgcttccgaaatgctcgggcgtcagcaggtcacgcagatgccacaccaccggccggcggtgcagaggccgcccaagcgccgcaaccacgaacgccttcaaggtgttggcgtgcaccacgtcgaaccgccgcgccatccgcgccaggcggatcaccgccaccaccagtgcgggcgcggctagcagcgctcccagacccgacttccgcctcacgccatcaacgccccccaggccgaggaccctcaccggcacacccgcgtcccggagccgcacggcgaaagccccgtcaccaaagaggcagacctccgagcggcccttgcgcctccgcacgatgtccagcagcgacagttcggccccgcccatctcgcccgactggtccacgaacagcaccgcgggcggcctcatcgcgccagcaccgcgcgatagacctccgccacccgccccgcgatcacgtcccagtcgtgcgcccgcgcatgggcgcggcaggcggcggcgccgggtcgctccacaccctcgatcatcgcgccgatccgctcggccaaggcgcctgcgccggcgttctcgcacaccagcgtggtcaagggccccaccgcctcaggcaggccgccgaccggcgtcaccaccaccggcgttcccgccgccagacattccagcgccacgaggccgaagccctccagcgcctggctgggcgtgacgccgatatcggccgcgcggtaggccagcggcagcgcctcttccggcagaaagccgatcagccgcacgtgggcggccagccccgccgcctcgatccgcgcgcgcaactccgcctccagcggtcccctcccggcgatcagcagcagcacgtcgggacgacggcgcaccacctccggcatggcctcgatcagaacctccagccccatgcgccgcaccagccgccggaccgtcagcagaaccgggcgatcctccggccagcccagccgttttcgcgcgtcggaccggctctccgctacgtggaagcgcgcagcgtccaccccgccgggcacgacatggatgcggcccgcctcgaccccatagtcctcgcacagcacccgcccgaacgcctccgacagcacgatcagggcgtcggcgcgcgaataaacggcgcgctccaccgcccgcttggccagccgccgcgccccgccctgaccctcggccgctccctccagcgcccacggcccgtggaagtgcaccacgtgcgggatgcgaatccggtccagcgccggcagcaccgacaaggcgaagtggctggcgaccagatcgggcgcgttctctcgcaaaaccgcgctgatcgcccggcgggcccccagcagccgcatcggcggcgaggcggacgccggcgcgaagctccgcacccgcccgccggtcgccctggcgacatccgccgatccgaccaccagtccggtcacctcgaaccgcccgggcgcggcgcccagcaggtcgtggaaatagcgcggcagcccgcccgtgcgctccggcagccactccagcccgacctgcagcgtcttcacccccgcgccccgccctctttgtcggccagagccagcgccagggcggcgagcggaaacaccagcatccccgtcgcaccgcccagcacgttgaagaacagcagctgcgcggtggtcccgaccacaatggcggcggccagctgcgcgcccggcccgctccagctcgcccgcagcgcgccgactccgatcgcgatcaccgccgccagcatcaccgcgctcgcccagccataggtgaacagcaggtccagcaccccgctgtcgaaggcgccgcgcgcgccgagcgccgcctcgtccgtgctcaaccgcgtcgccacccccgtgccgccgagcccgcggcccagcggattggccagcacctccatcgtcatctcggcgtgaaaggccgcgcgccgttgcaggctgacgtcctgatccaaccgcgccaggccgccgatcctggctccgatggtcccgccagatccgaacgccgccagcggcgcggtggccactgccagcccacaggcggccgccagataccccaggcgtcgtttcgccgacgccaggacgatcagcaccccgacgccgatgatcagcccgccccaggccgaccgcaccagcgacagcaccagggccgcaccgctcacgggtacgcccagccatcgcccgcgcgcccctgcgcccgccagcatggccagaagacaggccgacatcatcaccgcgaacggccctggggcgttcatcgtgccgaacacgcgcacctgtcgcgggctcggctgaccgatggaagcgatctcggccgtgcgcatccaagccacgtcccacgggggcggcgacagatactgcaacacgccgtacgcgcccataatcatgccgccccaggccaggatcccgaacacggcgcccgccgcatggtcggcgtcgcgcctcagcaccaggatgtggatcgccagggcgatgggcgccagggcgttcagcaggccgaacagcgccgccgcgcccaggccttgcgccagccccagcgccccgccgtacaggcacaccatcgccgccacgctgaacggcaggaagccgcgcccaagcaactgcggcccggcgcgcacggcgctgaacaggccgagccccgtgaccagcgccggcgccagcatgatcgggctgaggtcgtgccgtccgccctgccagtccgccagccgccgcacgaacggcgcgaccatccacaacaggtaacagaaggcgatgaacccccgcgacggcgcgcgcccgtacagccacagcccagccgccagggccacgggcgtgaacagccaggtcagccagcctcccagcccggccgcgaccatcgccgccgcgacaaccagcggcagcagggcggccatcccttcggtccgcgccgtcaagccgcgcctcgaggcgatccgcgccacgtccgccaacccgccaggcggccctccatcgtcgccttcacccgcgccgccgcttgccgcggcccggcccaccgagcccatctgagcccctgcagaagccccggattggcgcgcgtcccgagcagcagcgcccagaccaggaacaccgcccgccgtccgcgcggcaggaagtccagcagcgccagcgtctcgttgtgcgcctggttcttttgcgccggggccgaaaaaccccctctctgatcgacgtcgtgacgcacgccgggatagtggtccacggccacggccgggtcatagaccagccgccgcccggccttccgcagcgccaggcaaaaggccatgtcgttgcacacctgcgcgccttcgcctttcagccccacgtcgaagcgccggcctccgagatggacgtggcgaaagctcatgttggcgcccttcaggatgtccacctcgcgcggcgcgcctgcacccaggtggtgattgccgatgcaacgaccccaggcctgcactcgaccgacctggcggcgttcgccggtcgccaatcggccgtcgatgtgcagccagtcgcgtccgccgaggccggtcagcgtcggatcacgctcgaaggtctcgacgatgcgcctcagccagtccgctcgcggcgccgcatcgtcgtcggtgatcgcgatgatgcctccccgcgcctcctccagcccccggttcagcgccgccacctgcccggcggcctccacgacgacccggcgcagcgccaggccggtcggcgcctgttcaagcacccgcaaggtttcggcgtcctcggcgcgatggatgaccagaacctcatccgccgcccgcgcctggtcggcgagcgcgtccaggcaccggcgcaggtcggcgggccgtcgccacgtcggcacgatcaccgagacggtcaggctcacgaggcctgctccccgacgcgcgccgaaatccgccgcgcccggccgccgaactcacgaaccgccgcccaccccatcgatgcggcgaccacgacctcggctgcgaccgccgtccaggccgcgcccgtggccccgtaccggctcgccagcggccacaacagcatcagccccgccgctccgcccgccaggattgcgcttgtgaacgcgcgcttcagcccgaacggcagcagcagggtcacgcccagcgcattgttgatcccaaccagaaagatcaaaggcgccatggcccgcaaaaccggcacggccccctccgcctccggccccgccagcaagcgcaccaccagcggagcggcgcccgtcagcagcagggccagcgccgccgccagaccgccctgcgtcagcagcagacgccgcgccaaccgacccgccgccgcgggatcactggcgtgcagggcgctgatgcgcggaaagaacactgtcaggatgggggacagagccccttgcgcggacctgcggatgcgctcggccatggcgaacagacccagctgcccagcgcccgcgatcatgcccaatcccaccgacagggtgttggtgtagagcgagatcgcggcggtggatccgaacacatgcgcgcccgccttcaactgcctccaggccgccgggacatgaaagcatgggcgacgcagcagaccgatcgcccgcgcctgccacagggtcagcatggccgtcgccaaggcgccgaggctgacgcacagcgccgccatcgctgcatcgcctgcgtccctcaccagcaggaacaccaggggcacgggcaccagccgcccggcgacggaggtccaggcgaaccgccccagcgcctccgctcccttcagcgcccagtccaagttcagcaccgccgccggcgccgccaaggccgaggcccacagcaccggccgtagcgcatccggcgaaagcgccgccgccagcgccaacccagccagtcccgccgcgcaaagccacgctttggccagcaccgtggcccagatcaggtcgctggtcgcaacgaggtcgtcccgcatgcgcgccaccgcctgcgctgcgctgagggaaaagccccaatccaccaggatcagcgcatagcctgtgatcgccgccgccatgccgatcaacccgaagccttcgacgcccagcacgcgcgccagatagggaaaggtgatcaggggcagcagatagttggcgccctgccagatcgacgccgccgccagcccgcgccggacgctcacgccgccgtctcgcgggcgggcgaaaggccaagcagttcgtccagccgcgccaacatcagggtctcgctgaaccgctccagaacgtgggcccgcgcgcgcagacgcagccgctcggcgagcggcggatcgtccagcacctgcatcaggcgcctcgccaggtcgtcggcgtcgcccggcgcgcaggtcagggcggtgacgccgtctatggccacatcggccacgccggtcggcagacggctggccaccaccggcgcgcccagcagcatcgcctctagctgcaccacgccgaaggcttcggtggcgtcggtcgacgggaaggccagcacgtccaccgccagcaaaagcctcgccttgtccgcttggctgatctcgccgaggaaatcgacgcggtccgcgacacccaaatcgaccgccagcgcctgcgcttccctgcggcaagggccttcgccggcgacgaccgcgcgcacgcccggcatcgcggcgagggcccggatcagcacatgcaagcccttgtagcgtgcatggcgccccacgaatcccaccagcggcgcctcgccatgccgcgccagccgccacgcgcgcgcctcggcccgttccgcctctccggccgcgtgttgatccagcttcaccgagggagccacgaccccgatccgcacatctcgcggcagatcccgcgacatttcaaagttccgcagcgaggtcacgacgacccgctcggcccgacgcgccagatcccggtacagcgggcgcagcagcaaccgcaccagccatcgtccctgcacgtccgcatggtggatcacgaacagacgcggtaggcgctgctgcggcgtcgtccgcagcttcagccacagcaccgtcgcggcgtaggggttgggcgcatgcagatgcacctcttcatgatccgccggccgcatcatccataacagcgacagcgccagcggttgcgacatcagcacggcgtcggtccgcatgcggcgcacccgcacgccgccgatccgctcctcgcccgcacgctcgcctcgccccgcattcaccagcgcctcgacgctgcagcgccgggccagatgttcggcgtgaacctgggtgacgtgctcgatgccacccggccgtgggtggtagtattttcccaggatcagaatgcggggccgcgccgccgcgcccgtgtcggggcaagcccgcgcaccgtgtttcaggccgcgcccgttggccctcagccgacctgcgatcatcgcgcccccgctcacgatccccaagggtgaagacagcagcttcaccgtaaaggcgcaagtcgttcgtgcgcttacgaggccggccgccgctcgtctcgccccgcctcgcggcaggcgcggatcaggtcccgccggagactcggcgcccgaagcagctcaagctgagccgccgagtatccttcgcctgacagggccgagcgtatgtcgctggcgatggcataggcgccggttcgcgccagttcgaacgcgcgatcgatcgcgtgccgacgtcccattcgcttcccgcgaagctgatcatcgtcgggatcgtctcgccccgaccgccgtcagcctgtggccgtgtcgctgaacaacatcttaaaaacggcgaagcttcatcaggtgaagccgacaacccccgcgacagacgggcgaggcgtcactcggccggttggatctggtctcgtcgcgcctcctcgcccgtgcgcccggagtgctccggctggttgttcagcggcttgcgggccggcgtggcgacctgcggggtcggcttgggcccggtcagggcgccgccgacgttggcgcttgggtcggcgctgcggcgaccgggcgcttcctcgcgcgtctgtccccgatcgcaggcgttcaggcacagggcggagacgccaacgacgagaatgacgaacagacgcttcatcgcgatccctccacgtccggctcctcgcccggccgggcgtccgttccagcctgatgctcgatccggccgctctcgacctcggcgcgagaaaaaacctcctcctgcccgtcgatcagcagttcgtccgagggcgcgaaatccccccggatcttcccgggcgcttcggcggcgtacaagggatcggcgtcgcgggtcttcttggcgggttctgacattccgctcgaacgaggcgcgccgaggtgttgttcctggagccgccgctttcatcttattcggcggccacgctcgaaccgagtgccgccccgtgggttgcctcttctcccctctggctccccgcaggagacgaccatgcgcgactatcccaagcccccgttcaagaccgcccagcagccccgccccggctccagcgacgccatggacccggtccccgactacggcgaagccacctacaagggctcgggccgtctggccgacaaggtcgcggtgatcaccggcgccgattccggcatcggccgcgctgtcgccttggccttcgcgcgcgagggcgcggacgtgctggtcgcctatctggatgaagaggaggacgccgccgagacccgccgcctggtcgaggacgcgggccgccgctgcgagctgttcgccggcgacatctcccatcgcgagacctgccgtgaactggtccgccgggcggtggacgccttcggccgcatcgacatcctggtcaacaacgccgcccgccagatgagctacgacagcatcgacgagattcccgacgaggagtgggaggccaccttcgccaccaacatctcggccatgttctacatcaccaaggatgcggttccgcacatggcgccgggctcctcgatcatcaacacggcctcggtcaacgccgacacgcccagcccgcagctgctggcctacgccaccaccaagggtgcgatccagaacttcaccggcggtctggcgcagctgctggccgaaaagcagatccgcgccaacgccgtcgcacccggcccggtgtggaccccgctgatcccctcgaccatgccggccgagaaggtcgagaacttcggctcgcaggtgccgttcggccgccccgcccagcccgcggagctggcgggcgcctatgtgctgctggcctccgacgacgccagctacatttcgggcgcaaccatcgccgtgaccggcggcaagccgatcatctgacgcctcaaggcggcggcggacggatcagccgttcgccgccagcccgccttcatcgacgtcggcgtcctcttcgctgtcggcttcttcatcgaccagcgcctcgtcttcggccaggcgctgggcgtcggcggcggtgatgccgaaccgcgccgccacgtccggcgcatagcgcagcatgtccgcccgcagccgcagcaggctcaggtccttggacttggactccagcataatgtcgaactccagcccctccgccgtccgcatgaaggtggcgaactcgaacggattggtgaagtcggcgtgccccgtccagatcggcgggcgcagcaccgtgcggatgcgcgcggtcggcttgaccgtcgacttcagcacgtcgccctttctggacttcgtcttgccggccgcggcggcttcgcgttgcttgggcgtgatcttctgcttgatctcgcgcagctccgtgcggggcgaagagaagtggatcttgggccgcacgcccgtcggccaagtccgcatgaaggcctccagcgtctcccgcaggtcggcccgctcggggttcaggcaccagaagtgctgatagtcgaagacgcagcgcacgcccgtccgctcgtggatccacaggacatcggcggccgagaagcggatgtcgtcgttctccagcaccagccggcgctggacgtgctcggggcactggttccagccttcgatccagcgcgcacggctggcttcgtggtcgtcatagacgccgccgacgtgagtgatcatcaccgcctcgtcgttcagctccatccggtccagcatctccgcctggctggccagatcccagatgctcttcttcgtcagctcgggattgggcgcgttcagcaggacgtactgcgacggatggaacgacaggcggatgtcatagtcgcgcgccttttgcccgaacgccttcagctctgcgtcgctgtcggccaccatggagtggaactgcggcatgtcgggatgcgtcgcatagggcgcgatgtcggacgacagccggtacatgttcagccgctcggacttcagatagtccagcaccttgtccagcaactccagcgagcatttcaggtgcgggttcttctgccagcgccgggtgtcctgggtcttcatgtccggctttcccatcaccttgacgggaaagccgagacggaggggtcggtgggggtcggtcatgcgtccacttgctgatcaggcaggccgagatcggccacgaatgcgttccagtcggctatcctcagcgcgccgcccgtcgcctgggcgtggccgttgccgtagcggtcgtcggcgccgggcggccggtgctcggccaggaagtcgatgaggttgcgcccggtcgccgagcgcgcggcgaaatgcacccagccgggacggtagccggtgttggccgccagcacgatcttgtcctgtagccgtccgcgccactgctgggcgatcagcggatgcacctggcagccggaggagaagcggatcatcgccacgtcccctgcaatcttcggcgcgacgcgcttggctgcgtccatcgcctcgcgcacctcctgcttggcttgcaccagagcgcgggcgtcggcgtccccgcccctggtgatggccttggggccgtcggcgctcagcagcagccgcagcgccggccacgggtcggcggcggccgtgcggcgcggcgcgttgatcagcgacaccgcgtccttcagcgccgtcttgccccagcggccttgagcctgcgccagctctggaaagcccgcttcgtcggccatgtcgccgatcaggccgatggcggccaaccacagcagatcgccctggtcgcccagcgcgcccgccgcccaccaggccagcagcgccgtggtcggctcaggctccagcccatggccgctgagggtgacggcgcccttgggctctcccgtcggcgtatggtggtcgatcaccagcgtcggcgcgccctccacgaccggctcggcgcgcgtgcccaagtcggcgacgatcagggcggacggcccgacgtccgacagccgctgctgcactgaagcatcccatgccgtctcgcccttgccgaccggcaggggcgtggccgaccagccggcggcggagagcgcccgcaccatgatcgcgcccgccgacaatccatcggcatcgaaatggcagaggacggcgaccggccgggctcggtccgcccgccgcagcacgcgctccagcgcctccgccgccgcgatccggggcgagccgacgctgtccagaactccgatcatgcagagcctaacggcgacgaccgccgttggctccccgctcggagccgcgggtggacggcggctaggcgacgtcccggatgtcgccttccagccccagcgtgcggaccagatcgtcggccgcctgcggcttgtggaagtgatagccctgcagcaggtgcgcgccggcgatgcgcaggaagctggcctgttccgccgtctccaccccctcgcagacgaccttcatgcccagcgcgcggccgacgctgatcaccgcgtgcaggatggcggcggacgccgtgtcctcgcagcagcgggcgatgaagctggcgtccaccttcagcgtcgcgaacttcaggtcccgcagcgcatgcaggctggtgaagcccgcgccgaagtcgtccaaggccacgccgacgcccagcgcccgcagcgcctcgatcgactgctgcgccgaggcgacgttcagcatggcggtctcggtgacctcgatctccagccgctcgggcgggaagctgaccttgcgcaaggccgcctcgacccgcgcggcgaagtcggccgactggaactcgtcagccgaggcgttcaccgacacccgcacgtcgctcagcggcccgatgtccctcatcgcccgttccagcgcgaaatcggtcagtcggccaatggcgcccgcctgctccagcgcggggatgaagtcggcgggcgagcgtcgtcccttgtccgggcaggtccagcggaccagggcctcgaccttgccgctgaaggcgcccttggggtccatcagcgcctgatagtgcatctccagctcgtcgcgggcgagcccctgctccagctcggccagcggtcccgacggctcggccggcgcgccgcccagcgcgaccaccgtgcggcgcagggcgtcggtgatggcctccacccgctccggcgtggccgcctcgccgttccgggccgacgtctcgagaccggccgccagcgccgacaccgcacgggcgcccaggctcaggctcatggacttcagcgcgtgcgcggcgcgcgccacctcctccagccgcccctcgtccgccgccgccgtcagctcggcgaggcgcaaaggcgcattctcgagatacagccgctcgacccgctcgacgaagtcgggccgcccctgctgcgccattcgctgcagatccgcgcgcgtcgccggatcgaacaggtcgtcggcctcctcgccgattttgtcgtccgcctgtgcgccgaccgcgactgccggagtgggttccggctgcggagccgcagcctccgtcacggcttgcgaccggccggcgcagaccacgttcagcacctccagcaggtcgttggtggtgaagggcttgtgcaccacgccgttcatgcccgcctcgcgccaggcctcggcggccgagccgatcacgtgcgcggtcagggcgtagatcggggtgaccgtccgcccttcagcctgctcctcggcacggatgcagcgcgcggcctcgaagccgtccatcaccggcatggagccgtccatcagcaccagatcgaagcgctcggccgagacgcgcgccaccgcctccagcccgttcacggccgtgtccgcctcgacgcccaggctcgccagcgcttcgcacgccacctcgcggttgacctcagaatcgtcgaccaccagcacccgcacgccggggaaggtcacgctcgccacggcctgcgcggccgcccccgaccattcgggcctgcgcccctgctgcagctcgcgcagcgcgtgctccagcacttcccgccgcagcggcgtggacaggaattcctcttcgtccgcacccttggcgccgatgcgcacgccgaggcccgggatcgcctcgcccgctccgaccagattggccggcgcttcgccgacggccccttctacgacgccgtaagcctcaagatagcgacgcacggcgcggccggtcatcacctccagcgcacccaagcccaccgaccacccgccgggcgccgacatcggctccgccgccggcgaaatctcctgaagcggcacggagaaggcgaaggtcgatccttcgcccaccacgctcgacagctcccagcgcccctccatggcgccgaccagacgatcgcagatggtcaggcccaggcccgtcccgccgtagcggcgtgtcgttgactgatccgcctgggtgaaggcctcgaacagggtcggcaggcggtccgccggaatgcccggcccggtgtcctccacgctgatccgcacacgccccggctcggcggcgcgctcgaccgacagcaggacgccgccgacgtcggtgaacttcagcgcattgttcaagaggttgctgacgacctggcgcagccgcaccgggtcggcggcgaccgtgcccagtgtcggatcgacgtaggtcgcgagatcgagccccttctcctgcgccttgaccgcgaacaggtcggccacatcctcgatcaaggcgccgagatcggtctcgatcgcctccaactccagcttgcccgcctcgaccttcgagaagtccaggatctcgttgatgatgttcagcagcgaccggcccgaggtcgagatgatgtcggcgtatcgcttcggcttaggcggcagggcggtgcgcgccaacaggtcgctgagcgccaggatgccgttcagcggcgtgcggatctcgtggctcatcaccgccaggaagtcggacttggcggcgttggccgcctcggcctcgcccttggcttcggacagttcggcggtgcggctggcgacctcggcctccaggttatcgatctgatctgcgatgcgggcgtcgcgttcgcgtatactgccgagcagatctttgaagccgtccaccaggtcgcgcacctcgccctcggcggcgatgtcgttctgcgcctcgaagcggctggtgcggcgcacttcgccgatctggcctgccaacgcgacgatcggcgcgctgatctttcgcgccatgcgcagcgcgaccacaagcgccgccagcatggccaccagcgcgccaagcagtgtcggcagcacggccgccagaatgcgggtccgcaggtccggcgtgcggccgaacagcgtcaccttgccgacctcggcgccttcccacaacacaggcgctgacgcctcgatcgagccggtcctcagcgtctgcagcaaagaaggcttattcgtgtgactgacgctgacgtccgagatcaggcgtgcgccggcgccggtctccgccagcaggaacccgtcgctcgtttccagccgcgcatagctgaggctaggcatctgggagatcgatctcaccgcccggaaggcgccggtgcgatccttctgcgccactgcttctgaagacaaagaaccgatcacccgggccgtgcccaccagccgctcgctctccagccgcgcctgcgccgtcgcatccatccatgcggccgtcagcgcggtcaccgcaaaggagacgcccagcgccgtcagcaccagcttggccagtctgctggcgatggtttgggtcttgggcaaggcgggcgctcgttcggtgtccgatcctcaaccgatacgacacgttaatgacccacggcttaaggacggccggtggtcgtggtccccccgggccgagtgcgagggcctgagttgagcggctttttctacgttctggacgaagacgtccgcatcctcttcgtggacgacgatccgatcctgagggagttcgcgcaggtcaacctggcctccgtgcacgccgagatcgaggtcgccggcgacgggatggaggcgctggagcggctggatcaaggcgccttcgacctagtggtcaccgaccttgagatgcctcgcatcgacggcttcgacctattgggccggatgcgggccgatccgcgttgggatcgcctgccggtgatcgtcgccaccggccgcgacgatgtggaggccatcgaccgagcgttccaggccggcgctaccgccttcgtcaccaagccgctgaactggcggcttctgacctaccagctcaagttcatgctgcgctcggcgcgcgccgagacggcgctgctccgcgcacgccaggaggccgcaccagccgcctgacgcgcttcgggcgtgcttactcgctgatggaaagcggcggcgtctgctggtgctgcaccacgcgccagacatcgtgctcgatccggcgataggtggaggtgcagaaggcggtgtagtcctcggcgtccggcttcgacgccgtcacctgataggcgatcacgatcaaaccttcctgcgggcgcgagacgtgctgctgttcgaaacgcacctcgctccagcgcggcgtgttgatcaccgcctcgatcgcctcgggcccggccaccacgtgcgggtcggccggcaccaccatcaggcagcagtcgtccaccgcctcgcggtagtgttccgcatccgcggtccacaggctctcctcgaactcccaaacgcggctgtcttccatggcttctgtcctcttcggcggatcgcagggtgtgaaagggcaatccagcgggatcggatatgttccgagcgcatggagatgcgctcctgcggtcgctggaaccggcgcccccgcctccggttaactcttcgccccgttcaggagagacccatggccgacatcgacaaggcgcgccgcaacttcgtggccacggcgagcctcggcgctgccgccgcagccgccgcacccgcgctggcgcagcagcagccgcagaacccgccgggcgcgcccaccgcgccgcgcgccgccgactatcccaagccgcccttcgcggtgcagacccagccgtggccgggcctcgcctcgcgcatgaacccgcgacccgatcacggcgagaccagctatcgcggctcgggccggctgcagggcaagcgtgcgctgatcaccggcggcgacagcggaatcggccgcgccgccgccatcgcctttgcccgcgagggcgccgacgtggtcatcaaccacctgccggaagaagagccggacgcgcgcgaggtcatcgaactgatccgcgccgagggccgcaagggcgtctccatccccggcgacctgcgcaacgaacggttctgcgcccagctggtggagcgtgcagtgcgcgagctgggcgggctggacatcctggtcaacaccgccgcgcgccagcagccccgccccgccatcgccgacatctccagcgaagacttcgacgccaccctcaagaccaacgtctatgcgcccttctggctgaccaaggcggcggtgacgcggatgcaggcgggcggcgtgatcgtcaacacctcgtccgaacaggccggcgatccgtcggaggatctcgtcgactacgccctgacgcgcgcggcggttctgaacttcaccaagtcgatggccaagcagctggcgcccaagggcatccgcgtgaatgcggtcacgccgggtcccttctggaccccgctccaggtcagcggcggcgccacgcccgaaaagctgcagcagttcggctcccaggcgccgctcggacgccccgggcagcccgccgaaatcgccggcctctatgtcgcggcggccgacccgctgctcagctactccaccggccaggtgttcggcgcgaccggcggcggcggccagccgggctgatccgccatcgcgatcggacacagcctcacgccgaggccgcgtccagcgcccgctgttcgcagcggatgcgcacccacatcatgacggcgttcaacgcggtgaagaccagggcgtagagcggcaggccgaacgccagcggcagcaccgccagttcgcccgccaccacgatgtagttggggtgcgacacgaaccggaacggccctttccgcaccagcgtctcgccgggcagggtgatgatgcgggtggtccagcgccgccccagcgtggcgatcacccacacccgcccggcctgcagcagcacgaagagcagcagcagcggaaggttgaccggacgatcccagaccagcagccaaaggccgatcagccacgccgcatgcagggcgacgatgaagcggtagtgctcggcgccgctttccaccgcccctcgcgccagcagccggcgggtgttggacctcgccagcaccagctcgcccagccgctggagggtcaccagggcgaggatgatcacggccacggtcatgcgagcgcctccagggtcacggtgctgcaggtgaatcccggccccagcgccagcaccaccgagcgcggcggcagtcccgcccgacgcgcgcgatccagcacatgcagcacggtgggcgccgacatgttgccgtggtctcgcagaaccgcgcgttcgtggtccagcgatccgacctccagcgtcagcgatgactccagcgcatcgatcaccttcatcccgccgggatggcagatgaagcgatcgacgtcgtccagcgtccggccctgcccggccagcatcgcctccaccgccggcctcaggcggttgcgcgcgaacggcgggatcgcgcggtcgaagatcacgcccaacccggtggggtcgacccgccagcccatcacgtccagcgtgtccggccaggtgtgctcggcgctcgcctcgatgcgggcgaagccgccgccacctccgctgcgaagcacgcaggcggcggcgccgtctccgaacagggcggtcgccacgacgtcggccttgccgagatcgtcgctgcggaacgacagggtgcacagttccaccacgaccagcagcaccaccgcgcccggcgtcgcgccggccagccgcgccgccaacgccaatcccgtcgccccgcccgcgcagcccaggccgaacaccggaacccgcgccgcatccggcctgaagccgagccgaccgctcgcccgcgcttccaggctgggcgtggcgatgccggtggacgagacggtgacgatcacgtccacctcgccgccgctcagtcccgcttcggccagcgcgccctgcgccgccgcgacgaacaggtcggtcccgacctccagataggcggcggtccgctcggtccagccgcgcggctccagataccagtcgatgggcatggcggtctggcgctggtcgatgccggcgctgtcgaacaccggccgcatgcgctcccagccggagaagcgcccctcgaacatccgctcggcgatctggacggcgtcgctctggcgcatctggtggggcgcgcttgcggtggagagcgcaagcaggccggcgggatgcgggaacttcatccttcaacaaggcgtcacggctgtactggttcacccgcgggttgcgggctgcggcggcggacggatcgcggataggtcctccctttatttcgttcccgccaaggtggaaccggcaggaagacggcacgctcccgaatctcatcatcaacgcggagagaccacgtgaagacgatcctgaccctagccgcctgcaccgccgccctgtcgctggccgcctgcggcgacaacgccgccgaaacaccggccgccagcgactcagccatgggcgctgcggccaccaccgccgaccccatggccggcgccggaaccatgaccgctcccaccgatcccaacgccgcgcccatggccggatcgacaggaaccatgacgacgccgagcgcgacgaccggcgccacgggctcgaccggcgccgccgccagctcgacgcccggcgccgcggccggaaccacgaccggcgcgcccggggccgccggaaccaccggctcggccggctccggccaggccgacacggcgggcgccgccggttctcgccccgccggctgatcgacttatgatcgataaggccccgtcggatcgacggggcctttttcgtgttcgcctatccgacgtcccgcgcgttcaaggggatcagccttcagcgagaaccgccttgaacgatctccgagacacgccgtcaggccagagccgcagtccgacgtttgagccgggcatgggcgggatgaactcggccctcttgcgcaacatcgaggccatgcgccaacgccagcagcaggaggacgcgggcgcgggctttcaggagaagctggcgggcggcgtcaccgccttcaccggcagcatggtgttcgtctacgtccacctggcgatcgttgcggtgtggatcgccgtcaacgtcggcgccgtgccgggcgtgcagccgttcgaccgcacctttgtgatcctggccaccgccgcttcggtggaggcgatctttctgtccacattcgtgctgataagccagaaccgcgcggcgcgtgcggccgaccggcaggccgccttggacctgcagatcaatctgctcaccgagcacgaggtgacgcggctgatcgccctgaccaccgcgatcgccgaccggctgggcgtacacgaggcccgcgagcccgacctggccgagctgaaacgcaacgtcgcacccgaggcggtgctcgacacgctggagcagcaggcgaaggactgaagccggtttcagcgttcagagatcgtcagcgtcgcctcagccgtggccgcctcgccatagacgccgatccagatgtcgtagacgcccgattgcggatcgtcgaacttgaaggcgggatcggcgtcgccgccgctgtcgtcatcgcaggcccactggccgtccggcgtgttgatgaccagtgtggtgtcgctgttggacacggccatgatcgtcagctcgaagtctccggcggtgtagttcagccggaagtccggcgcgtccgcgatgtagccgtcgcagtcgccgcccagcttggaggcgtcgatgctgccgcccgccgtgatggagcgggtgtagggatcgggatcgaagccggcggacagccgcgcctgcccgaacgccggcttggctgaaacatcctgcgcccgccccggtcccgccgaccccatcatcagggttgccgtcacgatcgccgccatccacgtcttcatcgcaccaccctccgtcctgcgacaggctgccacacccgacagagaaagatcaacgttctttccaccgcaacccgagccgcctggccgccccgcccttgtcgcagccgccgcctcgccgtagtcagcgcgtcgagaccgcgacaggcggcgatgagggagtgcgatgggcaagatctatgcggacgtccggtccgcgcttgacgggctgacgttcgacggcatgaccgtcatgtctggcggcttcggtctgtgcggcattcccgaaggcctgattgcggccttgcgcaacagcggcgtcggcggcctgaccgtcatctccaacaatgcgggcgtggacgatttcggtctgggcctgctgctccagacccgtcagatccgaaagatgatctcctcctacgtcggcgagaacaaggagttcgagcgccagtatctggctggcgagctggagctggagttcaacccccagggcaccctggccgagcgcatccgcgcgggcggcgcgggcgtcccggccttcttcaccgccaccggcgtcggcaccctggtggccgagggcaaggaggtgcgcgagttcgacgggcgcgcctatgtcatggagacggcgctgaaggccgacctctccatcgtcaaggcgtggaaggcggacgagcgcggcaatctggtgttccgcaagaccgcccgaaacttcaacccgatgatggcgaccgccggcaaggtcacggtggtcgaggtcgaggagatcgtgccgaccggttcgctcgatcccgaccacatccacacgccaggcgtctatgtggaccgcatcgtcaagacgatcccggagaagcgcatcgagcagcgcaccactcgtcaacgtcctgaagccgccgcagccgggagtgaagtctaatgccccgcacccgcgaacaactcgccgaacgcgccgctcaggaactgggcgacggcttctacgtcaacctggggatcggcattcccaccctggtcgccaactacattcccgaaggcatgaccgtgacgctgcaaagcgagaacggcatgctcggcatgggtcccttcccctatgcgggcgacgaggacccggacctgatcaacgccggcaagcagacgatcacggaaatacccgagagcgcctatttctcctcggccgacagcttcgccatggtccggggcggccacatcgacttgtcgatcctgggcgccatggaggtggccgagaacggcgacatcgccaactggatgattcccggcaagctggtgaagggcatgggcggcgccatggacctggtcgccggcgtcaagcgcgtggtggtggtgatggagcacgccaacaagcacggccagtccaaggtgctgaaagcctgcaccttgccgctgaccggcacgggcgtggtcagccgcatcatcaccgacctggccacctttgacgtcaagcccgacagcgcggggctggagctgatcgaactggccgagggcgtgaccctggacgacgtcgccgcccggaccgaagccgcctacacggtcatcgagggcgtcacgacggcggcctgaccgccgcctcaggccccatcagcggccgacgccctgccgcaccgacgcgggcgccgactggatcgtccagtcggcgatctgggcgtttaggtcccgcgacgcgcggtcgaaggcgtccacgatggccgatacgcggttggcggcggccggctggctgatggagaaggtgcgttcgatcgcggcgccctgctcggggcggatcgcgccctcgccgctgttccgctcgggcgtggttcgcaactgtgcgcgagccgtcaccaccaccgtcggcgccgcattctgggcgccgggcgcatagcgcgcctcgaaggtcgtgaccgtgacctgcagcacatacggcggcgtgccgggctcgcctcggttcagcacgcggatctggtcggcgcgcgaagcgaaggccgagcgcaggtcgtcgtcgaacaggttctccgccgccgtgacccagcgcgcgccgccgatgtaggcggtctcgttgccggtcacgcccaggatgcgctcgcccttggcggcgtccgggaattcgatccggcggatggagaccgacagcggcgccgggcgctgcccctcgggcgagggcgcgtcgacggtgaagccgaaacgatacagctgcgccggttcaggggacgacaaaagggcgcagcccgacagggtcaaggccccgacgcccacggcggcgagacgaagagcggagcggccgatcatggctggacctcgagttccttggaggcgggacgggcgatgaagtcgcgcgggctggcgcgcacgtcgtcgatcagttgctgcagcgagcgcgtggcctcgttcagctcctgaatggtctggctcagctgcggcaggctggaggcggcgaagtcgccgaccggtccttccagtccgctgaccgaccggttgatggaggcgatcgccgtgcgcgcatccgccgtggcctggttgacgttggcgatggcctggcggccgtcgttgttgaccaatcgacgtgcatcgacgcccagctgttcatactcctgcacggcgcgattggcgctcgccaccgcctgctccagttgcaggaagatgcccttgcgcgcctcgagctcggtggtcagcgactccacattgcgcacgctggtggagaaggagcggatgttgtcgtccgacatgatccggttggcgcggttcagcagatccaccgtctgcgccagcaccgtgcccgatccgttcagcaactcggcgatcggggacggctgggactggatcaccggcacgacgttgtcgggatactgatccttcaggatggcgctgttgggcgcgccggcggtgatctggatgtagttcaggccggtgatgccctgcggctccaactgggcgcgcgaggtgacgcgcaccggcgtggtgccgtccagccgcacccgcgcgatgacctgatcgcccttctgcggatccaggttcaggtcggtgacctcgcccacgcggatgccgttgaaatgcacctccccgccctccgacaggccgcgcaccgggccgtagaagacgatgtcatagacgtcgtagtcgttgttgaactgcagccgggccagccagatggtgaacaccgccagcgccgccaggagggcgacggtggcgatgccgacagcggcgtaatgggcgtctctttccatttcgatccgctctcctcaggcggccttctgcccggcgcgtccgcgcgggcccaggaagtattccttgatccagggatggtcggatcgttccagttcctgcaccggcgccttggcgacgatgcccttgtcggccagcaccgccaccttgtcgcagatggcgtacaggctatcgagatcgtgggtgatcatgaagaccgtcagtcccaggtcgtccgacaggttgcggatcagctcgtcgaacgccgccgccccgatcgggtccagacccgccgtcggctcgtcgaggaacagcagctcggggtccagcgccagggcgcgcgccaggccgacccgcttgcgcatcccgccggacagttcgttcggcttcagatagcgcgcctcgggcttgaggcccaccatggcgatcttcatctcggccagttcgtagatctggcttttgggcagatcggtgtgttcgaccaaaggcgaggccacgttctcgagcacgctcagcgacgagaacagcgccccctgctggaacagcacgccggtgcgcatctcgatgtcggcggcctgctgcttggtcaggttcgcgcggtcattgccgaacaggcggatttccccgccgtccggctccttcaggccgatgatggtgttcagcaacaccgtcttgccggtgcccgagccgcccaccacgccgaggacctcgccgcgttccacatccaggtccagcccatcgtggatggtgcgctcaccaaaccggctcaccagcccgcgcacctcgatcagggtctcgggttttcctgcttcggacttctgagcctgcgccggggcgtcctgcacgtcgctcacaggttcagctccaggaagatcagggcgaacaccgcatccaggaagatgatggcgaagatcgcctgcaccaccgccgccgtcacccggcggcccaggctctcgacgtcaccggccaccgccatgccctgacgcgcgccgatggcggcgatgacgatggcgaacaccggggccttgatcaggccgaccatcaggtgctggcccatcatgggatcttcgttcaagcgctgcacaaagaaggcgggccccaggttcagctggctccagcacaccagggcgccgccgaacagcccccccaacatggccacgaaggtcagcagcggcagcatcaccaccagcgccgccaggcggggaatgaccagcgcctgaaacggattgacgcccatgacctgcatggcgtccacctcctggttcatccgcatggagccgatctcggcggcgaaggcggaggccgagcggccggccagcagcaccgccgtgatcaccaccgcgaactcgcggaaaacggccacgccgatcagctgcacggcgaacacgcccgcgccgaagtcagtcagcaggtccgcgccgatgaaggcgatcaccgcgccgatgaagaagttggtcaccaccacgatcggcatggcgtccagcccggcgcgctcggcctggctgacccaggcgggccagcggatgcggcccggatgcttcagggcggcgaccaccgccgtcatcagccgccccagaaaggcgaacgacaggatggtctcggctccgatgtcatagacgccgcgtccaaccttggcgaaggtgcgggtgaaggggtcggcttccttgggcttcttggtcgaggtgcgctcgagcttttcgaccatcttgtagatgcgcccggcctcgggacgcccgtcccaggcgccgtccggcacgccgcccttggaagcctgcgccagcgccagggcgcccgccgtgtcgaaccgccccagttcgctgacgtccagcgccgcgatctcgcgcccgcggagatcagcgttcagccgatcggacattcgtccaacaccggtggtggtccagtcgcccttcagccgcagggtggccgccccgccctgcgcttcctcgatctcgaaatccgccccggtcattcgctcattctatcgagccacggcccggttgcctacggcggcgcttgcgtccccgtggcttgctgaacgcagcgcccgccttttcgttcgcgtcgtccgaacaaggacttacaggctgtggcgaacctgccgcaggtcctgcacgaacttctcgcgctccagcaccctggcctgctcgtccggcaggcgcagcagataggacgggtgaaccgtcagcatccccgtggcgccgtccgacagggcgaccggccggccccgctcctttgtcaccgcaggcttcctgccgaacacggcgaacccggccgtcgcgcccagcgccagcaccaccctgggcttcaccagcccgcgctcctgatccagccaccagcggcaggcggtgacctctccgacgttgggggtcttgtgcaggcgacgcttgccgcgcggctcgtgcttgaagtgtttcaccgcattggtgacatagacgtccgaccggtcgatgccggcctcgtcgagcgccgcatccagcacccggccggccggccccacgaacggcttgccggccaagtcctcctgatctcccggctgttcgcccacgatcatcagccgcgcctctcgggaaccctctccgcagacgccctgcgtcgcgtcgcgccacaacgggcagcgccggcacccctgaacgccctcgccgagttcgggcaaggtggaggcgaccagatcgtccgccgcgcgctcgactgtcggcgccgtcgcgcgaacgaggcgagcgttgggttccgaggcgggcgtggcgaccatgacatcggtgcgaaccgtcgaggccgccaccagttccggtatcagcgcggcctccggcaggttcttccagtaccgcttcgccatctcgccctgcatggtcttcaccttcagccgcgccgggttgaaggtggaggcgtagtaggtcttccagaactcctcgatctcgtcctcggacggcgccatgtcgcgcgtcgccgccggtccgaaccgcagctcctgcgtgtcccagaaggcgctgccgtccggcgtcaggatcgaccagcgcatgttcggaaaccgtcgttggaaaaagggcgcggtccgctccaccacccggtgcgccggctcgaaccaggcgacccacgcctcgccgccctcgtcctcgacctggcggaagcggacaaaggccttcatcttgtgcccggcccgcgacacgttcttggcccgctccagcgcatcggccacgtcgcgatcggacaccaccttcatcaggtccggctcgtccttcagccgccacagcagccggtacagcaggtcccagcgatcgccggatcgatgcagcaccacgtcgcgggccacgtccacaaaggccttggagacggtgaactccccatttgctgaggtggcgggcgccggcgcgtcgaacagtccgcccctaccggccccctccaccacgaagcgcgcctgcgccggctcgaccccctccagccgaaaggcgcgcgcggccttgcgccagccgtcgaagtccgtctcggacgccagcgtcgccgcccgcatcagaacaggctcagttgctgcggctccgccaccggcgccacgcgcgcgcgcaggtcggcggcgtcggtcagcccgcccggcgtccagtccagcgtggtgatgaaaggccgcaccttgtccagcgagcgcgtcagccgcgccacgtcctcgagccgcagggtgcgatagcgccggaccgacacgatcttgtcgaccgacttcactccgagccccggcacgcgcagcagcatttcgcgcggcgccaagttcacatcgaccggaaattgctcgcgccggttcagcgcccagccgagcttgggatcgatcgccaggtccagcatcccgcccttcgccgcctccccgatctcgggcgcggagaagccgtagaaccgcatcagccagtcggcctgatagagcctgtgttcgcgcatcaagggcggcttggccaaaggcaggctggagctggcgtccgggatcgggctgaaggccgaatagtacacccgccgcaggccgtaaccgccgtacagcgaggcgctgcgatccaggatctccgtgtccggcgcgccgtccgcgccgatgatcagctgggtgctctgtccgccgggggcgaaacggggcgggcgggctttttcgcgcttctgcggcttggcctcctcgaccttgagccgcacctgccccatggccttcttgatgacccccacgtccttttgcggcgccagtcgcgcgagcgcctcgtcccgcggcagctcgatgttggcgctgaggcggtcggcgtagagccccgcctcctccaccagcttggggtcggcctccgggatcagcttcaggtggatgtagccgcggaagtcgtggacctcgcgcagcgtcttggccaccagcaccagctgctccatcgtatagtcgcccgagcggatgatgcccgacgacaggaacagcccttcgatatagttgcgcttgtagaagttcagcgtgaggtcgacgacctcctgcacgctgaaccgcgcccgctccacgttcgaggagacgcgattgatgcaataggcgcagtcgtagatgcagaagttggtcagcaggatcttcagcaagctcacgcaacgcccgtccggcgtataggcgtggcagatgcccataccctcggtcgaacccatgcccttgccgccggtcgagtcgcgcttgctcgatccggacgaggcgcaggaggcgtcgtatttggcggcgtcggccaggacggacagcttacgccggagatcgatctgagccattgttccgtttatgttccggaacaacgactgcgtccagcgtagccgttcaggaaatcaacgcagcaggtccagcaacgatgtcgatttcagcgacacgatcacctgcgcggacgcctcgatcgcgacacccgccagttgcaggtcggtgatcgcctgagccggatcatagccggtcttcgcctccagcatcttggtcagcgaggtctgttgcgcctggtggccggccagcgcgctctgcacctggttctgcatcgagccgttgcgggccgtggcggccgtcaccccgacaatggccttgtccagcatctgcatctgcttggtcagaaacgccgtgacctcgtccgacgccgagccgtctatgttgccggcggccgtggtccggggcggcacgacggacggcgtgtaggtgacgccgtcaacggtgaccggaccgccgttctgatagatctggatgttgcgaaacacctctgtcagcgccgccccgacatcatccgccagaaagccggtggtcagggtggcggactcgccgatgcgggacttctgcgcctgccgatcgttggcgaagaccgacgcaacgtccggcgcggcggcgagcgcggcgaggctgtcggccgtcgccggcggtgcatcgcccagcccgccacccagcagatactgcccctggtgcgagaagttcaggccggcctgcatggtctggaaatggccctgcaactcggccatgaggccttccagccgcccggccgcgatggcggtggcgatggactctcgcgccccggcgccgccttcgccgacgcggctcagggcgatgtcctgcgacgccagccgcgcctccaccgcctctcccgaggcgacaaagccggccagccggctctgcgtcgccttcagcgccgtgatgttctgcgacgaccggccgtagcccttggagtccgtggcgatcttttcgctgtccagccgctcctgcgccagctgctgacggccttgcgccttcatcaggtcaagcagcgcggactggtagttgcccatggtcgagacgcgggtcatcagatcatccccagcaaggtgtcgtacatgtccttggccgcctggatcagccgggccgaggcgttgaaggcctgctggtaggtggtcatcatcaccagctcctcatccagattgacgccctcgtgcgaggtctgtcgggcctgcgcctcggtcagcagggcctcggcgctgtttctgcgcgtctcggcggcggccgccttgctgccgatgtcgcccgagaaatcggcggcgtagcgggtgatggaggtcgatgtcgccaccgatcccccggccccatcgaagcgcaccgtggccttgcccgcgtcggccagcgccaacgccccggagccgtcgttgctggtcagggccggcgttcccgccgccgccccgaggttcagccgcgccagcgccagcttcgtcgagtccgcctggatgtcggcgcgcaggctcaagcctcccgttcgcgccgcccgcacgccgccgccgatgccgaacagcgcgctgaccgacacgcccgagggactctggctggtggtgtcgttcagcaccgacagggtcggggccggcgaccccgcgccctggaacgtcagggccccggtggccgcatccagagagaactggccgtagcggcccgcgccggtcgccggattgttcaacgccgccaagaggtcgtccaccgtggccgcgccggcgggggcggcgatggtcacgtccttcagcctggccccgctttccccggtgaagcgcagcgtcagcgctccccccgccgcgagcccgagagacgaggttccgctcaggcccgtctcgtaaaaggccggttgggtcgtggagaccagatcgttcagcccgaagaagtgcgagaagccgcggccgaccttgctggccggcgcagtggggtcgtcagcgatggcgatgccgttcacgcccgtgctggtcaggctcatggtgccgttctggaagcggaaatccacctgtccgcccagcgcggcctccagatcggcctcgaagttcgccgccgaggacgctccgccgttgatggtgatggccccgcccgcgccgaagacgatctcggcccgctgctgcaccacgccgctcgcattggtggtgacgatgttggtggttccggtgaacccggcgatggccgtggcccaggactgacccgtgttgcggccggtcaggctggtcggcgccggaaccgacgcattggcgttgtgtgcgcggttcagttcgtcggcgaccttggacatcagctcgcccaggcgttcagccgcggccggcgcgtccacgtcgcgcagttcgaccagccccttgatctcgccggatgcgacagaatccagcagggcgcgcttctggccgcccggctcggtgatccagacctcgttgaaggcggtcttgccgtccaccgcgcccgcgggcgaataggccagtgtcgcatgaccctgcccggccagcagcgcgcccgtgccggtccgcaccatcacgccgccgttggcgcggcccgtcaccttgatgtccatcagctgcgacagctggctcaacagggtcgcctgggcgttctgggaacccgtggcgtcgtctccggccgccgccgccgaagcgatcgtcttgttcagatcctcgatctggcccagcaggtcgttggcggtgtccaccgccgtgcgcaaccgcccgtccgcctcttcgcgcgccgcctggatgttcttgccgatggccgcgccctgatcgaacagggcctgggcctggtacaggatgtcctggcgcagcggcgaggacgtcgggctctccgacacggatgagaaggccgcgaacaggtcatcaacgtcggtgaagaagctgttgtcgccgctgggatcgccaaacagcgtctgaatgcggtcaaacagctcgtagcgcacgccctgccgcccggcttccgcgccggcgttcaggctcgcggcctgcaggaaccgatcggtcgccagtcggatgcgcgccacctcgacgcccgagccgatgccttgcgtcgccgtggactgctggtcggcgatcttgcggacgtagcccggcgtgttgacgttggcgacgttgtcggagaccacccgcagctgcgtctgcgccgcgtgcattcccgagttggcgatgttcatgatggacgtcagcgacatgcgcgatctcccttgccgtcgcgggcgccgggcaagccgttcccgccgccatgcacatcctgcctagcgcccgcacgagcaggcgcaggcaagcccttgtttttttgagcaaataggtctgatgcagtccacatggcgctgtcacccgcgcaaacggcgggccaacaggcgacgccggcggcccacccgccagccagggcggcaaaaggcgacgctcagggcggcaaaaagcgaccgatggcacaggacgcgatgacgcgttctccgcattttgctgcgccagaaccgagacttgcgccgtttccgcatgtggcccgccgcttgcgacgggacgagggaatgcccaggcgcagcaggcgccgcctcactcttcatatcgaccgcctgcccccccatgtcgctcgccatcgccgcctttgcgccttcagcgcccgcccccgcgcccgccgctcccaacgggaacggcgccgctttcgcgcaggtgttgtccgggcagaccgacggaacggaaaccgtcgcccccgccgtcaagacgacgccctccccgtccgcgcggcgcagccctgctgctgaagaggtcgcgacgactgacgccgcagccgcagcgcccccgccgcagatcgccgcgatcgccgcgcccgccgtcgctgttgatgaacccgattcggacgctccaggcgcggacctgaccgaaaccgaagcggcgtctccggtcgaggcggtgaccgccgacatccctcagccggtggttgcagcccccgtctcctcccccaccgctccggtcctccccgatgctccggcgtcacagccgtcgttgagggccgagatcgccgcgaccgacgccgatccgcttccggccgtgacgccacggttcgacccgcccgcctcaggcgacctgcaggccgcacccgcgccgtcgcccacgcagcctttcggggaagcgatcccggcgcccgtgacgcctgactccggttcgcctgccgcgccggctccgcagacgtcgagcacgtccgccgaccacccggcgtcaaccatcccgacgcccaccgcccaagtgcaaggcccggtcgagcaccgtcccgacacgcgcagcgaagcgccggctgcaaacgcggctcaacctgaggacgcgtcttcgccgtccgccgctgcaagcagcgacgccgcgcccaagcccgcgccccaacccacgcccaaggatgccatgcaggcgctcttgggcgcgacctggtccggcctcgcctcccggccgacgccgccccgcaagccccctcgaccgatccggccgcgcccccgcagaccgcttccgcccccgctccggccgccggcccgcagaccgccgcacccgcctttccgctggggatgatgtccacgctgtcgcaggcgacgatcgagaccacgacgcgcctcgccgcccagatcgccgcacgcttggaaggccggtcgacgcgcttcgacatggtgctgacacccgaagacctcggccgcgtcgaggtcagcctggagatcgacgaaacgggtcagctcgccgcgcgcctggccttcgacaatcccgccgccgccacggacctgcgcggccgcgccgatgagctgcgtcgtcagctgcaggacgccggcttccagatcgccggcgacggcctcgacttctcgcatcgcgaggacgcgcgcggcggagaggccggcggcggcttcgagcggcgcggccggtcctcgctgttcggaagcgcctcccgcctggccgccgaggccgacatcgcctcagcgcccccgccgggcgcctggatcaacctgtcgctggcgcgcgaacgcgtcgatctgagggtctgacgcacatggtcgacgccgtcaccaccgcatccgccgccgccggaaccatctcttcgggcacgaagagcctggcctccaacttcgagacctttctcagcctgctgaccacccagctgaagaaccaggatccgctgtcgccggtcgactccaacgagttcaccgcacagctgacccagatggccggcgtcgagcagcagttgctgaccaacaccctgctgaagagcctgctgggcggccagcaggccggcggcctgtcggacgccgccgcctacatcggcaaggacgccaccggggtctgggccgccaccgagctgaccgatggcaaggccgagtggaactacgagctggccgccaacgcctccaaagcgacgctgcaggtggtcaacggcgccgggcaggtggtctggtcaggcgacgcgcccgacaagaccactggcatccacgccttcacatgggacggcaagaccaccggcggcggtcaggccgacgacggcggcgtctacaccctcaagatcaccgcaaccgacgccgccggcaaggcggtgaccagccaggccttgatccagggccaggtcaccggcgtcgagctctacgacggccagccctacgtcaccatcggcaactccatcatgccgctgtcgagcctgatctcgatcgaacagcgcgcctccaccaactgatctcgcaaaggaaaccgacatgagcatcaacagcgccatgctggcgggcgtttcgggcctgcgggccaactccgccgccctcgcctccatctctcagaacatcgcgaacgtgaacacggtcggctacaagcgcagccaggccgacttctccaccgtagtgaacacccagagcgtctacaccggctattcggccggcggcgtcacctcggtcgcacgtcacaacatcagccagaccggccagcttcagtcgaccacctcctcgaccgatctcggcatcgccggccaaggcttcttcgtggtgacgcagaaggccgagggcctgactcccaccgacgcccgcctgttcacccgcgccggctctttcaaggtcgatgagttcggctatctgaagaacaccgccgggctgtatctgcagggctggcccgtcgacgcctatggggtcatcaccaccgatccgtcggacctgaaccggttgtccaccatcaacgtcggctcggccggcggcacggccgaggccaccagccgcgtccagttgaacgccaacctgaagtccagccaggcgatatcggccgaggcgcgcgacgccgccctcgccgtgcccggccctaacgcctacaacgccgccaccaactcgatggccatgtacgatccggacgccggcacgggcgtgaagccggacttcgagattacggtgccgatctcggactccaagggcggacagcgcacggtcgccatctccttcctgaagagcaccacgcccaaccagtggtacgccgaagtgcgcgccgtgcccgccgacagcgtccagacgggcgccggcctcagcgacggccagatcaagaccggcatggtcgccttcacccaggacggccgcctggacacggccgccatggcggggatggttaacgccctgttccccgatcccgccaacgcgactctgagcttcggcgcctccgacgcggccccggcggcgggcgccgtgtcctgggcgactggcctcggcatcgacgatcagaccatcgcctttgatctgaccaacgcggcgggcggcctgacccagtacgacagcgcctccgtcgttcaggccgtccagaccaacggcaccaacttcggcagccttaccgaggttcagatcgacgagagcggctttgtcaccgccatcttcgacaacggcgtgacccgtcagatcgcccaggtggccatcgccaccttccccagccccgacagcctgagccaggtcaacggcaacgcctaccgcgtcagccagcaatccggagcctacaacctgaagaccgccggcaccggcggcgcgggcgtcctgggctcttcgcagctggaggcctcgaccgtcgatctgtccagcgagttcaccggcctgatcaccacccagcgcgcctactcggcgtcttccaagatcatcaccacggccgacgaaatgctggccgagcttatcagcatcaaacgctgatctctcgctaagtaatcgttagcctcaatgaatcgtcgctcaaatcaggacttcgcgttcgttaacgtgcgggaacggattattccttccttcaccacgacgcttaaacggcctttagccgcggggtcctaccttcaccgaagtacggtggtggaagaggcataagcccatgttgcaagagcgacgcctgaacagcaaaggcgaacaatacgtggtgggaccgacgggctcggccctgaccctcgccgacctgcctccggccaatacggaccgctgggtgatccgacgcaaggccgaggtcgtggcggcggtgcgcggcggcctgatcagcctggaggacgcgctggcgcgttaccgtctgacggccgaggagttcgtcgcctggcagaaggccatcgacaaatggggcatgcagggcctgcgcaccacgcggatccgaagctaccgctcctgagcctcaaggcgcttgcgagcaggcggccgcttccggcgacggaggcggccgttctcatattcagcgggcggccgcgcgcgccgtgtcgaacgcctgccgggcggcctcgatgcggtccaggtgcgtttcggcccatttccacacgccgcagaaggcctcggccaggctgaagcccaggtcggtcaggcgatattcgaccttgggcgggatcacagggtggacggtgcgcaccaccagcccgtcgcgctccatctgacgcagcgtctgtgtcagcattttctggctgacaccgccggacagggcggcgatgcgggtgaagcgcagttccccgttctcggccaggacgtccagcacgatcatggtccacttgtcggcgacccgaccgatcacctcgttgaccagcgcctcaacgcgcggatcgacgggcggatattcaggggcgcatagaggttcggacgccgtcatcgccatttctttccgcttggtaagtacctcacgatccggtgccttcttcctgatcgccagcgcctcttctatctccctgtccatcgcaggcaagcggaagaaggcgcaccatgaacatcgctcaagacaccatcctgatcaccggcggcggctcgggcatcggcagggccttcgccgaggctgtccacgcccgaggcgccaaggtgatcatcgccggccgacgcgaggccgccctggccgaagtcgccgccgccaatcccggcatcgtctatgaggtcctcgacgtctccgacgccgccgacatcaccgccttcgccgagcgcgtcacagccgcccatcccgacctgaacgcggtgatccacaacgccggcatcatgaaggtcgaggacgtgtcggccggcgccttcgacctcggcgtggtggaagacacgatcgccaccaacctgctgggtcccatccgcctgacggccgccctgcttccgcatctgctgacaaagccgtccgccagcatcgtcaccgtgtcgtcgggcctggcgttcgtgccgctcgcggccaccccgacctacagcgccaccaaggcggcgatccactcctggagccagtcgctgcgtcaccaactgaaggacaccaacgtccgggtgatcgagtgggcgccgccggcggtggccaccgacctgatgcccggccatgccgaggaccccaactcgatgcccctggccgacttcgcctccgaaagcgtcgtcctgttcgaggcgggtcacgacgaggtgctggtgcagcgcgtgcagttcctgtcgggtgcggagggtcgcggccagtacgccgaggtgttcgcagccgtgaacggcgcacgctgatcgccgtggacgccggcggctcgaaaaccgccggcgatcggcctatatggcggccatgacgctcgcagagccgctttgccccatcccgaccatcgcccccatgtcctctcaggccgacatggatgcggcgatcgaacaggcgcgcgcggcggtgggcctgccgctcggcagccgcgtggtcgccgccatgtcgggcggcgtggactccaccgtggtcgccgccctgctgcacaaggccggctacgacgtcgtcggcgtcacgctgcagctctatgaccacggcgcggcgctgaagaagaagggcgcctgctgcgccggtcaagacatccacgacgcccgtctggcggccgaaaccatcggcatcccccactatgtgctggattacgaaagccgcttccgcgacgccgtcatcgaccagttcgccgacagctatctgaaaggccagacgccggtcccctgcatccgctgcaatcagacggtgaagttcagggatctgctggacgtcgcgcgcgatctgggcgccgaggccatggccaccggccactatgtccggcgcgccgtgggtccggagggccgcagccagatgcgcaaggcgatcgaccactcccgcgaccagtcctacttcctgttcgccaccacgccggatcagctggactatctgcgctttcccctggccgatctggagaagccccaggtgcggggcgtcgcggcagaactcggcctgcgcatcgccgccaagccggacagccaggacatctgcttcgtcccctccggcgactaccgcaccctgatcgaccggctgcggccgcaggggcgcgagggcggcgagatcgtgcacatggacggccgcgtgctcggccgtcacggcggcatcaccgactacaccattggccagcgccggggtctgaacgtcgccgtgggcgaacccctgttcgtggtgcggctggagcccgaggcgcggcgcgtcgtggtcggcccgcgcgaggccctgctgacctccagcctcacgctcgaggagacaaactggctgggcgaccagccctccatcgcggccgcagccggcgtcggcctgccggtcctcgcgcgcgtacgctcgacccgccaaccctcgcccgcacgcctgtcgctcatgaacggcgcggtgtcggtcgtgttcgacgaaggcgaggaaggcgtcgcgccgggccaggcctgcgccctctacgacccggccgatcccgaccgcctgctgggcggcggcttcatcacgacgacgagcgcggttgccgactgacggctggccggggcggaaccgcgtcgccggcctgtgatttcatccggcatgccgcccgccgatccccatcgccccatcagcccgccgccggccgttggtccacgcggctccgaccttcccgcctacctgtccaacggcatgatcgggcttcgggtgcgcgagaacccgctggaagccggcatgtgcatcgtctccgggttctcgggcgagcaccccgaacgcctcgtcgagggcctgtgccccgctccctacccgctggccggcgatctcggcgtcgacggcgtctggctcagcgacaatccgtccggcttccagcctgtcgatcaggctctggatttcgaaagcggcgagctgaccacccggatcacctacaccgccggcgatgtcaggctcgatgtcgaaattctgaccttctgctcgcgcgaccagcccgcccttgtctgccagcagctgcgcgtcaccgcctccgccgcatgtcgtctgagctggcgcgctcgcatcgatccgcattgggcgcggggccgcctggtgcagcggctcaccgacacgccgggagaagcaacccccgtctgcgacggcgctctgctgtgggcgggcgacggcgatctgtcgcgctgcggcgtcgcctacctcacccaagcgcctgaaggcgccgaacggtccgtcgaccagtggaaccgcaccggcccgctgatgacggaatacgcgctgtccatcgacgccggccgctcggtggtcctgacgcagatcgtcgctcttgttcccagccaactgcacgcccagccgcacctccacgccacgcgcctgtgcgcgcaggcgaagcatctgggcttcgaacgcctgcgcgccgacaaccggcgatgctgggcccgcctgtggcgcagccgcatccgcctggtcggcgccgatgtccgctggcaggctctggccgacgccgccctgttctacctgaacgcttcgacccacccgtcctcgccctcctccacctcgatcttcggcctcgcggcctggccggactaccactactatttcgggcatgtgatgtgggacatcgacgccttcgccacgccggtgctgagcgtcgtgcagccgggagcggccagggccctgctggatttccgcacccgtgggctcaacgccgcccgagacaacgcccggctgatgggacttcccgggcttcagttcccttgggaggccgcgccttcgtcgggacaggaggcgacgcccggcggcggcgacgccatcttccgcgagttgcacatcaacatgcatgtcgcgcgcgccttcgacttccacgccaaggcgacgggcgacggccgcttcctgcgcgaccaggcctggccggtgctctcgggcgtggccgactggctgaccacccggctagaaaccgatcctgacggctcccgccatctgcgcgacatcggcggcccggccgagcgcgagaccacggtggacgacgacgccctgaccctgatgagcggccggctgatgctgcaggcggcgcagggcgcggccgaacggctggatctgcccgcgccttccgcatggctcgaagccgccgacgccatcagcccgccgatccgcgcggacggcgccatcgcctcccacatcggctaccgcaggggcgaggagaagggcgccaccccctctccgctgatggcgatctttccctactggtcgccgttggatccccagacacaagaagcgacccttcgcttctatctggatcagtgggaggactatgttggctcccccatgctggcggcgctttacgggacgtgggcggcctggctcggtgaccgcgacctgtcgctgaagctgatgcacgagggctacggcgcctatatgcacggccgcttcgaacagacgctggagtatcggctcgacaagatggaggggccggcggccgggccgttcgtggccaatacgggcggtttcctgaccggcctcctgtttggactgccggcgctgcggatcgacgacgacccgcccgaacgctggcccgtgcgccccgtggtcctgccgcggggatgggaggccatcgaggtcgatgtgctccacatccatggccgggagtggcgtctgcgagcggtccacggcgccgaccgggccgaactgacgccgctgtaggaccgcgttcgcccgaagtcagcctccgttcaccatcatgcgggcaggctgcatccgtcacccggagacgccgccatgaccgctcgcctgcctcgccgcgccgccgccctggcgcttgtcctgggatcggccctgatgcttcagggctgcctcgtcggcgcggtcgtcggaggcacggcggccgtggtcggcggcacggccaaggccgccggttccgtggtcggcgccggcgtcgacgccgtcaccacctccgacgaggaaacccggctgcgccgcgagcgcgaacagcgcgaatgggaacgcgagcagcgccgctgcgagcagcgtcaacgccagggcaagcgctgctgacgccgttccctgctcgaccgcgcctaaacgtccttcccctcgagccgcttttcgacggcgtagttgtggatggcgacgccctccacctccaggtcgcgacgctgaagagtggtgaagccatgtcgctctaggaagcgccgcgcgggctcgctcgcttcggcgaacagacgcgagacgccttcgcgcgcgcaggcgccctcggcggcctggagcaggcttgcggccacgccccgctcggcttcaggagccttgtaaagaaggtggatgtggccgttcgcctccagatcgaggaagccgacgaccgtctcgccctcaacggcgacgaagcgccgacgcccgtccgccatcagcgcctccagccgctcggcggacggcgccaggcgcgcccaggcggcgcgctgttcatgcgaatagtcgctcgccgcatgcgcctggatcgaccgtgcgtagaggcggctgagcggctcggcgtccgtgggcaggtagggccgcaccctcacagcgtcagcacgcaccgctcgttgatggtcggccgcgccacctggatgcgcgccagccccggccaggccggctgcagccggcgcacgaaccagaggcagaggttctccaggcttggcagctccagccccggatgctcgttcagcaggccgtgatccagctcttcggccgccgccctgagcgcccgatccagcgcccccaggtccgccacccaggcgtgctcggcgtccagagtctccgagcgcaccgtggcctcgacggtgaaggaatggccgtgcagccgccgatagatgctgccttccggctcgtccggaaagtgatgcgcggcgtcgaacgtcgcctgtttggtgatctcgaaaaagggcatcaacgcacgccgatgtacttgtgggtctggacgctgaggcgccactggggatgggtcaggcagtattcgagcgcggcggcggtgttggccgcctggtccggcccgtccatgggctgcagccagaagcgctcgaacggcagatgctcgaaccgctcgggcatggcctgtgcctggggatagaccagtttcagctcctggccgcgcgtctgcaccaccggcgccgacgccttcgggctgacgcagatccagtcgatcccgtcgggcgcctccagcgtgccgttggactcgatggcgatctcgaagccgcgcgcgtgcagcgcatcgatcagcggcccgtccagctgcagcagcggctcgcctcccgtgcagaccaccagccggggatcgctctccctgccccgccacttggacgcgacatggtcggccagaccgtcagccgtggcgaacttgccgcccccgtcgccgtccacgcctacgaagtcggtatcgcagaaggtgcagacggcccccgcccggtcctgctcgcgcccgctccacaggttgcagccggcgaaacgcaggaacacggccggccgccccgcctgcccgccctcgccctgcaccgtcaggaacacttccttggccgaataggtcacgccgacgcccattccgaatagccggccgcgcgcagttcgcaggccgggcattcgccgcagccgtaaccccaggcgcgccggtgcgtgcggtcgcccaggtagcaggtgtggctgtcctcgacgataagctcgaccagcgccttgccgccgatccggtcggccagcgcccaggtctgcgccttcgtcagccacatcagcggcgtttcgatggcgacaggcttgtccagccccagcgacagcgcccgggccatcgcctgcatcgtctcgtgccgacaatccggatagccggaatagtccgtctcgcacatgcctccgaccagcacctccaaccctcgccggtccgccagcgccgccgccgcgaccaaaaagatcaggttgcgcccgggcacgaatgtcgtcggcaggccgcgcgcgtccatctcgatcttgcggtcggccgtcagcgcgctttcggcgatgcgaccatagcctgtcaggtccaccacatggtcgtcgcccagccgtgcggcgagcgccggcagggcggcccgcatgccttcgcgcacggcctggcgcgcctgcatctcgaccacatgccgctggccgtagtcgaagccgaccgtctccacccggtcgaaccgctccagcgcccaggccaggcaggtggcgctgtcctgcccgccggaaaacagcacaagtgcggaggtcgaggtctgggtatcgctcatgacaaacctgcggtcggccacggccgcgcgcatgcaaaagagatggagccgatggaggcggcgggtcaatcgcatacacgacatggaaagccggcgcaaaagcggcggcggcctgtcaaaggcgaagggattaacccttctgcaaatcgttgtcgggcagaaccgaggctcgtaacggagtccccggccagtatgccgaccattgagaccctagttgaacggcccgaaccggtgacaccgggcgcatccggcgccgaggtcttcgcgcgtttcgcgcgcgagccggacaccctggttctgccgatcgtcgacaacggccgtcccgtcggactgatcgagcggacggcttttcttctgaagatggccagccccttcggccaggcgctctacagcggccgctcgataatccacgttatggacgcagagccggtggtggtggaagcgggtctggagacggacgatttctgcgacatcctgctgaagggggggtcgtccgacctgttccggggcttcatcgtcacccgaaacggtctctatgacggtgtcggaaccgccgccaccctgctgcgcgccatcaacgatcggcacaatcgccagagccgcgagatcgccgaacaggcggtcgtgctgaccgacgtccgcacccaggccctgaccgccgcgcgggccaagagccagttcctggcgatcatgagccatgagctccgcacgcccatgaacggcgtgctggccgtggccgagctgctgcgccgccagccgctgaacgacgccgcccaggcgcacgtccagaccattgtcgactcctccgaaaccctgctgcgcatcctgcaagatgcgctggacctgtccaaggccgaggccggcgagctggagctgtcgccccgtcccacgccgctgcgcgccctgatggacgacatccaggcgctgtgggaggcccgcacctcgcaggacggcgtcaccctgctggtcggctacgagggcgacaccgacctgtcggccgagatcgacgacgtccgcgtcaagcaggtgttcaacaacctgatctccaatgcgctgaagttcgcccgcaacggcgtggtcgaggccagcctgcgcgccacagcccacgacgaccgcatccacatggaagggcgcgtgcgcgacaatggtccgggcctggacaccgatcgcgtcgacgtcatcttcgaacccttcgtgcacggatccggtcctgacggcgctggccttggcctgtcgatctgccgccagatcaccgagcgcatgagcggacgcatctgggccgagaacaacgccggcagcggcgcgaccttcgccttcgaactggacgccgaacgcgttcacatcgaagaggccgcgccgtcgaacgtttccgacctgaccgagctggacctgcagtccagcccgcacgtgctgatcgtcgacgacaacgccaccaaccgcgtggtggcccaggccctgtgcgagatgttcggctgcacctccgaactggccgaggacggactggaggccctctccgccgtgcaggaacggccgttcgacatggtgctgatggacatcaagatgccgcgcatggacggcgtccaggccacccaggccattcgcgccctggcgccgccggtcggcttggtgcccatcgtcgccctgaccgccaacgccgatccggaagacgcccggcgctacctggccatcggcatggccgcggtggtggaaaagcccatcaagcccgaacgcctgcgcatggccatgaacgccgccatgtcggccagccaggccggttcccaaggcgaccctaaggcgcagccgggccgcgccgtcgcctgacgatcagtccggccggacttcaaggctctcgtcgtcctcctcgtcatagccgacgagtctcagcgcccgcgccttcatgccgttcagctcggcccagcggcacagcccctcttcgcggccgtgggtgatccatatctcttccggcgcgacttcgcagaaggtggcggtcagctcgtcccagtcggcgtgatccgacaccaccagcggcagctcgacccccttctgccgcgcccgcgcccgcacgcccatccagccggatgcgaacgccgccaccggttcggcgaagcggcgggcccagcggtcctggatcgccgacgggggcgcgatcgccacctctccgcccagcgatcccttcggcagatcgcgcgtcggcaggatcggccccagggccacgccctcgcgctcatacagggcgttcagccgctccagcgcgccgtgcacatagatcggccgctcccagccgacttcgcgcaggtgcttgatgatccgttgcgccttgcccagggcataggcgccgaccagatgcgcccgctccggaaactgccccagcgacttcaccagcctggcgacctccgcctccgccgacgggtggcggaacacaggcaggccgaaggtcgcctccgagatgaagacatggcacggcacgggctcgaagctggcgcacgtcggatcgcgcctgcgcttgtagtcgccggacaccacaatggtcagaccctgccagcgcacctccgcctgcgccgagcccagcacgtgccccgccgggtgcaaccgcacctccacaccgttgatggaggtcgcctcgccataggccgccgcctgccgccgcccggtgaactcctcgccgtagcgttcggccatgatcgccaacgtctgcggcgtcgccagcaccgcgccgtgaccggcccgcgcatggtctgaatggccatgcgtcaccaccgcccgatccaccggccgcaccggatcgacatagaagtcccccggcgggcaataaaggccggccggcgtggggtgcagcaggtcttcgggacggatcatgatcctctaacgcactcgacgccaagcggcgccgtcgccataagacggagcatggtcgacggttttctttccaccatcctgccccagctcgccgccggttcggcgcacacccatgccctgggcttcgtctacgaagggctggatgacgagggcgtgtccatccgcgtgccctatcgcgcggacctggtcggcgatcccgacaccggcgtgctcgcgggcgggctggtgacgaccatgctggaccacgtcggcggcctgtcggtgtgggtcaagctcgaggcctttcgcccgatcgccaccctggacctgcgcgtcgactacatgcgcgccgcccatcccggtcgcgacctgctggccaagggcgtctgcttccgcctgacgccgtctgtggcctttgtgcgcgcctgggcgttcgaggatgatccgtccgacccggtcgccgccgcacaggccgcctatgtcgtcaacgaggaccgcgccgcccgccgcgccgccatcctcgccgcgcgcgagggcggagagtgaccgagcccctgctggaccgcctgccctacgcccgctttctgcagctgcgcaccctggtcagcggcgacgagatcacggtcaccatgccgttccgcgaccagctgatcggcaatccgatgatcccggccctgcacggcggctcgaccgcggccctgctggagatgaccgccatcgcccaggtcgccctgtcatttcccgccgcccgcctgccgcgcccgatcaacgtcaccgtcgcctatctgcggaccggccgtccccaggacgtcttctcccgcgcccgcatcagccgcgccggccgccgcgtcgcccatgtcctggccgaggcctggcaagaggaacgcggccagccgatcgcctccctgaccgcccacttccttctggcggaagacagctaggccggccgccgggcgtccgctctggggtgacgctcagcgccgcagggggtctccacgatcagctctttcgcgcaccaacagggtcaacaaacccctaccgatccacgccaacctatgttaacccttcatttaccatatccaccttggagggctaacatggatcgggttgaagtcgtcgccagcgtcgccggcgatctgcatgccacggaacaggccattgatgcggccatcacccaggcgacggccctggtgcagtcgatgattggcgcgcgcgccgccctgtcgctgtcgcccgtatcggccacggcctctcaagccaaggcgatggagaccatcgcccagctcggcgccgcgcgtgaggccatcgtcgcctgccacgcggagatgcagaaggaccaccgccgcctcggttggggaacctacgccgccggtccgatcaacaagccggatgactggctcgaccccaagcctcgcgaagacacccgtggccttcgcgtcgtcggctaaattcgacgtaacgattgcgatcagccatttccgctgattgcgattcattccaagatcgccctcgcgttctgtcaggcgcgggggcgatttcatgttggacaccctgtatgcacagatcggcggcgccgcggtcatcctgtgctgcctgttcgcctttctgaagggcgaggacctcgagcgcttcggcgccggagcgtttctgttggcgtggttcgcctccatccttgtccagcaggacggcgacctttaccgacctcaggtcggactgttcgcaatcgatgtcatcatggcgatcgtattcgcgggcatggcctggcgctctcgcgccgtgtggccggtctgggccgcggcctttcagcttctgtccgtgatgagccacatcatgaacatgatcgatcttcggacgcccaccgcctcgctctacaccgtcctgaaccttgcgggttacggcgtcttggcctgcatcgtggttggaaccgtggcggcttggcaggagcgcaaggcggccggcttcgaataggtggatattcctattcttcaccgctagattcggcgaatcaccgtcggatcacgccccatgcccctgtcgcacgcccaactctggaaggccgttgatcggctcgccgcgcgtcagggcatgaccgcttcgggcctggcccgccgcgcgggtctggacgccaccagcttcaatccgtcaaagcggttcggccctggcgatccgccgcgtccccgctggccctcgaccgagagcgtcacccgcatccttgaggccacgggcgtgtcgctgtccgagttcgcggccctggccgacgatgtccgtcccgcgcccgccaccgtgccgctgctgggcttggcccaggctggcgaggacggcttctttgacgatgcgggcctgccgaccggcgagggctgggagcagaccgaactgccccgccgcaccgacaccaccttcagcatccgcatcaccggcgactccatgtcgcccgtctaccgagagggcgatcaggtcatcgtggatcgaggtcggccggacgtgcggcgcggcgaccgggtggtggttcgcctgaccaccggcgagacgctggccaaggaagtcaccagcctgacggcgcgccaggtcgtcctgtcctccatcaatccggcctatccgccccgcgtcgtgccccggcgcgagatcgagtggatgagccgcatcctctgggtctcgcagtaaaggaaagggccgctcccctctcggaaggcggccccaaatcccgtcgctcgtcgccgatcagtagcgtgagacgtagttggcgttcacccagccgccgcccgcgatctgcacccagtcgccctgcgaggcgacggcggtgaagggctggccggccgacaggctgcccgcctgacggtaacccgttcccggacccgagcggatgcgcaggttcgaattcgcccggaactgcgacgcgttggcctgagcgatcgcccgtgtgcgctgctggttgcagccgatgtaggagccggccgcggcgccgagacccgcgcccgccaccgtgcccagcgtgcgctcgttgcgcgccacctggttgcccagcacgccgcccagcaccgcgccgatcgcggcgcccgcgcgctggcggccgcccggggcgtcgcagttggtgacgccgttcgcctgggcctgcgccgccatcggcgccagggtcaccagtgaggccatcgcggccgccgtggccaaaccggtcttgaagatcttcgacatggctcttctcctgtccatcgtgttgccgatggagcggacaatgccgcatcgaacctgaaggctcccggagcctccccgtcatcttccgttcatattgcttagctgtcggccagccgcccttcggccccgtcgcggatcagtcgcaccgtctgcgccaggccgtagatcgccgcgaacgagccgaagcgcggcccctgcgacgcgcccagcagcacttcgtacaacgccgcgaaccaggcgcgcagcggctcgaacccatgcgccttgccgaccgcatagacctcgttctggatcgtctcgccatcggtcgtgtcggcgggcagcgcctcaagccgatcggccaggtccagcagcgccgccttctccttttcgtccggcgcccgataggtcttcgtcggcttcacgaagtcctcgtaatagttcagcgcatagcccatcagccggtccagcagcggctcggtctcgggcgtggcgtccggcagatagcgcgctaaataggcccacagcgccgccttgtccgtcgcattcgccacccccaccaggttcagcagcagggcgaaggacaccggcgaggcgtgatccggcggcgatccggcgtggatcgaccacaccgcattgtcgatccgcttggccggctcctgcgtcttgtagctttcgatgaacgacagatagtcgtcggtggcgcgcggaatgacgttgaagtgcaggctcttggccgacttcggcgactggaacatgtaccagctcaaggactccggcgtgccgtagcgcagccagtcgtccatcgtcagtccgttgcccttcgatttggagatcttcctgccctcgatgtcgaggaacagttcgtagttgaacccttccggcggcacgccccccagagcgcggcagaccttggagctttcgcgcacgctttcgatcaggtccttgcccgacatctcgtagtcgacgtccagcgcggtccagcgcatggcccagtccggcttccactgcagcttgacgtgaccgccggtcaccggaacctcggtgcgtccgccatcttcgctcttggcgggatcgacgaagacgatggtgcctttctcgacgttgcgctccagcgtcggcacctgcagcacatggccggtgacggggctgatcggcaggaacggcgaataggtcgcccgccgctcctcgcccagcgtcggcagcatgatggcctgcaccgcatcgaaccgctccagcagcgtcagcagcgccccatcgaaccgaccggaccgataggtctcggttgagctcatgaactcgtagtcgaagccgaagccatccaaaaacgcccgcagacgcgcattgttgtgggcggcgaaactgtcgtgcgtgccgaacggatcgcgcacctgcgtcagcggcttgtgcaggtcttcgcgcagcatctcagggttcgggatgccttccggcacctttcgcaagccatccatgtcgtccgaaaacgcgatcagccgcgtcggccagtggtcgcccgtcagcgcgcgaaaggcgttgcgcaccatggtggtgcgcgccacctcgccgaaggtgcccatgtgcggcaggcccgacggcccgtagccggtctccagcaccaccggccgccgcagggcctcgaaccgggccagcgcctcgtccgccttgcccgcgtcgatcagcgacctggcttcggcgcgctccgcctccggcaaccgcttcttcagcacatgcgccaggaggttgcgggcctgctcgaacggccacgaccgggcctcgcgcgcgagtgtctcaaggttctgaagcatgcggcggggtttggcgcttcacgccgtcgcggtcaacgcttcagcccccgcgcgcgaccagggcctggatgtagctctccagcgtgacctcaccccgctcgtcgggttcgggcgcctgctccaccgtgtcgatggtcgcctgcgtcatgcaggcgtaggaccgcgccgccgcatcggagaagccgtgcttgcgatagtcctcgagccagcggtcgcgcggcagggtctcgacccgcacaggccgccccagcgcctgtgcaaaggcgcgcgcgacatcgttcatggtccgccgctccggtccggcgacgtggcgcacgcccacgtcgtccaggccgctgaccagccgccgggcggccgcggcgcccagatcctccggcgcgaccatcggcaggagaaggtcggccgggaacggcgtgaggaggacgccgccttcgcgcaccgcatccacaagcatgtcgaagttgctgaaatagtaggcggcgcggttgatcgcgaccggcgtgcccagcgctgataacgcctgttcaaaatcgtacagcaccgtcaggtcgccgcacgcctcacccgcccgcgccccgtatgtcgaggccgccaccaccttctcgaggccgactcccctcgcggcctccacgatggcgtgggcggtcgcgctctcccgcgcgtccgtgtcgccgttgatcggcgcgggcgggttgagcagcagcgcgcgccggccggatcgcagaaccacgcggaggccctcgacgtcgcagacatccgccacggcggcgacgcagccttggccttcgatccccgtgaccttctctggatcggaggtgaccacggtgaccgcatgtccgtccgccttcagcctgcgcgccgccgcctgaccgacatgaccggttccgcccaggatgatgaacatggcgcgcctccgctggctcgtgagaccaacacacgggcctgagcccccgttccgagacgcagccttgcgccgtggacgcccgcgcccatgtgcctctgatgcgatcgcttcggaaactcggtctcggcggcgggtgccactggtgcaccgaggcggtgttccagtcgttggtgggcgtggagcgggtacggcagggcttcatcacctccgatccgccgaacgaagccatgtccgaggcggtgctggtcgattgggaggcgaagcgccttccgctggacgtcctgatcgaggtgcatctgcgcacccacgccagcacctcgccccacacgatgcgtggcaagtaccgcagcgccctctacgtcatggacgccgtccaggccgatgcctgcgcggcggcgctagctcggcttcagccggggttcgacgcgccgctgatcacccgggtcctgccgttccgcgcctttcagccgtccgacgcgcggttccagaactactatgcgaccgacccggagcgacccttctgccgcacctacatcgagccaaagctggccatgctgcgccgtcgctacggcgcgagcctcgtcagcccggcggcttcctcaggcgacgaaacaacccgcgcccgctgaacggctcgaacatctcctccggaccttcgggatccagcgcctcgttctcggccagccacgcctcgaccgacgacaggtccggcgtctcgtacggcttcagcgtcttgcccggcccgcgcagccgctcgatggcggcgatcagcgagccggtctcctcgaccgtcgcccgcaccgtctgcgcatccacgcccagatgctcggccatcaggctttcgcgcgtctcacggatggcttccctggccccccggttggcgggaagacgcgcgtcgatcaccacgtcgcactccgtgtccagccgcatcgagcgattgttcatattggacgatccgacccgcaggttcaggtcgtccaccaccgtgatcttggcgtggacgtagatcggctcgccgtgcgtcgtatgcggatgatagacggcgaagcgtttgtgaacgtcgcgccgtttcagcgcctccaccagccgcgcccgcgccgagtccatggcgatcggctccagccagccctcggcggtgaccgggttgatcagcacgatctcgggcccgtccggctcgtccagccgccgagccatcgcctcggcgatgcggcgcgaggcgaaatactggctttccgcatagatgaagcgcttcgcccccgcgatctgctccagatacagcgcctcgatctcgcgcaggcgggctgtcgtccatcagcggcgcagagcgggcgatggcgacgtccacatcggtgaactgcaccgccagatcctccggccagggttccgactgaacctccgcctcgccgacgggggccccgcccgccgcggcccagcgttcgcggaacaggtcccccagcgcccgcgccgccggtcccgccagcgccgtggtcgcatcatgccagggcttggcgatccggcccttgcggtcgcgtcggcccacgtcgccgtcccggtgcgcgcgcgtgtcccagcggtcggccaacatgtcgatgccgccgcagaacgccagccggtcgtcgatcaccacgatcttctggtggtgcgagcccgtcggcgggtggtggccgtccagccgggcgtggatgcgtttgttgcggctccacttgatcagggcgcccagggcgttgcccctcagcaccatcttcaacagcccgacgttccagcgcaggatgaagatctctagctccggccgacgcgcggtcagccagcagaagaagtcggcgatctcgcgcggcccctccacgtcctgcgcgctccggtccaggtccaggtcgccgtcgaagtcccagccgatcagcaggattcgcttttccgcccgcagcatcgcctgccgcgcgtggcggaaatagtcgtcgccatcgacgatcacgctggcgcaggacgcccgctcgatgcgccagcaggtctcgcccggtttcaggccgctatcggtcatgaggcgcaaaccggttacggccaagctggttccgcgcgcttgaccccggccctcagcgccttaaagcgcgcccatgcgcaccgccgatttcgacttcgacctgcccgaggagcgcatcgcccttcgccccgccgaaccgcgcgacagcgcccgccttctggtggtgcgggacggcgcgcttcaggaccggaccatccgcgacctgcccgccttcctgcgggccggcgacgccctggttttcaacgacccccgcgtgatccccgcccgcctgtcgggcgtgcgccatcgcaccggccccgacggcgagaccctcaccgtccctgtcgaggccaccctgcaccaccgcgacgcccccgacgcctggtccgccttcatgaagccgggcaagcgcatcaagcccggcgaccgcatccgcttcggcgatctggaggcgagcgtcgcagccaagggcgaggacggtctggtcgccctgcacttcgacctgtcgggacccccgctggacgacgccatccgcaccgtaggcgtcatgccgcttccgccctacaccgccgccaagcggcccgaggacgaccgcgaccgctccgactaccagactgtcttcgcccagcacgacggctcggtcgccgctcccaccgccggcctgcacttcaccccggcgctgctggaggccatccgcgcccgcggcgtctccacccacgccgtgaccctgcacgtcggcgccgggacctttcttccggtcaaggccgacgacctggccgaccaccgcatgcacagcgaatggggcgaggtctcagccgacaccgccgccgccctgaacgccgtgcgcgcatccggcggccgcatcgtctgcgtcggcaccacctcgctgcggctgctggaatccgccacgaccgaagacggcgtggtccggggcttccacggcgacaccgccatcttcatcacgcccggctaccgcttccgcgccgccgacatcctcctgaccaacttccacctgccccgctcgaccctgttcatgctggtcagcgcctttgcgggcctggacacgatgaaggccgcctacgcccacgccgtcgcaaccggctaccgcttctactcctacggcgacggcagcctgctgttccgagccgacgggaccccgaagcggccgtgacgaacttcagctgagggtggcaagcggacgttgaccaaatcaagtattttggtcaacgcgaacagagctatacatagggcccgaggaagaatgatcatggcgttggccccaagtctactcctggcgacttcacttcagctaggcagccacttgtcttttccgagcatggcctacccgcctgcgcctgacgaagcggagcttgtgcctctaacggcgagccagatcgcttccagatttagcggcaagattcttaggtatcgccagggcccgcagcctgccgaaggccagggtcttttttgcccggacggtacatatctccgcgaagtgcaccgcttgggactgcggttcggcgactacacgattgctgatggggtcatcagcatacagctcaggagtgacgtgagacatcctatcctacagctatcaatttcaacgggcgaaatggacaggttattcgcacgctgggacagccatggctgggcggaaatcgagttcgaagaccctgtcggccagccatgtgctgatgcgccccgcgtaggttcaggagcttcctaggtcaacgatgggtcggaggcgacctgcggctaaagggtggtaaaatgggcggtggcggcgccacggtgtcgcctgaatggagacggctcatggcgacagaggttctcagccctgaacatgatcgacgtgtggtccgcgccgcaacatgggcgttgcggaagattggggctcagcgactggatcagaaatggtcgctgttcggctcgcaggaagtcggtgagcagtatcggatgtcttcagctgggcctctgaccctcactgccgaaacatacatgggcctcgtcctcgatggaccggatgaggtggtgagtcaggtcaggtcgctgattgcgcgacggctcggctagggtccagactcataaccaccacgcgatgatggcggcgagggctatggcggcgatgtaggtgcaggcgagcttgtcgtaacgtgttgcgacgcggcggaagtccttgatgcggcagaaggcgcgctcgacgaggttcctgcgcttgtagggctccgggtcgaagggatgcaggcgctttcggtaaggggcgttggggatgaccggctgggttcctcgggccagcagcagacggcggagcgcgttggagtcgtatgcccggtcggcggcgagggtggctgaggcgggcgcggcctggatcaggtcggcggcgcatcgccgcgctggcccggggtgatgacaaaggcgacccggcgaccgagcccgtcgaccagggcgtgcagcttggtggtcggcccgccgcgcgagcgacctatgccgttggctgaagccccccttttccgctcgtcgccgagcggtgtgccttggcccaggtcgagtccagcatcagctcggcgggcggcccgccggtggccgccagttcctcgaacgcccgccgccagaccccccccctggcccagcggacccagcgattgtagagcgtcttcccgggtccatagaccgccggcgcgtcgatccagcggccgccgctgatcagcacatgaatgatccccgagatcacccgccggtcatccacccgcgccacgcctcgaggcttgttcggcagcagcggtcgcaaccgctcaaactgcgcgtcagtcagccagaactccgaagccatgtcggttctcccgcatccgactgcaggaaatcacgcttcggccaatcagggaatcccgtttatgggtccagaccctagtcgccgggcggcggctccagcgcgtcggggtgaacgggcacgcccgtgaccacgccctgtgacgtcctgaggcggtcgtaacgctgacgcgccccggcccgcacgtcctcggcgtcgcgcagaatggtggggcgaaggaagataaagagggtgcgacgcgtttgagtgtcgcggcgcgcgcggaaaaagccgccgacacccggcagatcacccagcaccggcaccttgctgtcggcgctctgagcatcgtccgtgatcaggccgccaagagtgatggtctctccgtcgtcggccagcaccgtggtctggatgctgcgacggttggtgacgaggtccgccgcgccggcgacggtggcgttcaccagcgacgacacttcctgactgacctccagccgcaccacgtcgccatcatgaacgcgcggcacgacgcgcagggtcacgcctacgtcctcgcgcgtgatggtggtgaagggattggtggtgttgccttctgtcgcaaaggcgccggtgcggaacggcacgttctgaccgacaacgatctcggccggattgttgtccagcaccgtcacgctgggcgtcgacagcaagttggcgctggaggtttgggacagcgcctgcagcagcaggccgaagtcaccccggctgccgaccgccaggttcgcgccttccgacaccgcaccaccacccggtacgcccagcaccgaaagaatctggcccagcgacgcgcccaccgtggtgaaagaggtgccgccgatcacgccgctttccggcacggcgccgccaacggcgagttgcacgcccagccgctcgcccagttcgccggtcacctcgacgatggccgcctcgatggtgacctgcggccggcgcacgtccagttccacgatcaggtcttccagcatctgcacggtcgcgggcgcgccgcgcatgacaatggcgttcagctctccggcggactgcaccgtgacgtcgttcagggcaaaaccctgcggcgtgctggccggctgccccgaggcggaagcggtctgagagggcgcgccctcgctcgatgcggacagcacgctctccgagcggctcgccgcgctgaggctggccaggccggtgcggcgcaggctgcggctgaccgggttggtcgcggtcggctccgcgcccatcaggccgcgcacgatctcgaccacgctttcggcgtcggcgtgacgaaggcgcacgacgcgagtcaccggcgtcgctccgccaggccggtccagcgccgcgaccaagctgcgcacctgggcgatgtctgaggagtcgccccgcaccagcagggtattgctgcgggcatcggcggcgacgcgggcgccgcccccctcctcacccagcagcgtgcccagcgccgccgccacatcctcggccgaggcgtgttcgagcggcagggtggcgaaggattcgccgccgcccgtgtccagagagcgcgcgatcgcctcgacccgccggacgttgtcggcatagtcggtgaccacaacggcgttgggattagtgacggactcgatcgtgccgaaggagttgatcagcggccgcagcgcccgcaccgcctggtcgcccggcagattacgcaggcggatcagacgggtgaccacctgctggctcgatcccgccgccccgccggccgaggcgccgttctggaccacggtggcctgcggcacgatgcgccagaccgcgccgctgcgcaccgccgcaaagccataggtccgcagcaccgacaggaacagctcccacacgccggctgaggacaggggctcggccgagacgacggtgaccacgccgctgacgttcgggtccagcaccagggtgcggccggtcaggcgcgagatctgttcggcgacctcgcggatgtcgacgccgcgcatgttgaccacgacctcaccgccggccggcgccgtgacctgggtgacgccgacagagggcggcgccgcgagcgtcagggccagcaggctgaccgtgcagaggcgaagagtgcgtttcacgatgtgcgcctatcgtagcggaaaggtgagcgtgagggtccggccgtcgcgcacgatctcgacgcgcgcgctgccggcggcggccgcgcgttcgaacagttgctggtcggaagcgagatcgcccaccggacgaccattgagcgaccgaatgagatcgccgggtcgcaggccggcgcgcaacagctgcgccggcgcgtcggggccgaggcgatagccgtccgaggtcgcgctgacgccggccgactgaagcgccgccgcagggttggcgggtgcggcggcgggcgggcgggcgctttggccggcaggggctccgccgccgccggacgcggccggggcggtggcgatgggcgatgcggccgcgagcgccgccgcggcctccgggctgggcggggttgcgacggcgggggtcgcgcccggcgcggcgggcgcggcggcggacgacgtcccaacaagacgcggaaaggtcagcgcctctcggcgaccgccgacgttcagcaccaccacgtccagctcgatgccctcgatcaccgccgagcctatgggcgcctctccgatcgagaagttgcggggcgcggcctctcccaccgcgatcagggcggtggacgcctccggcgaggcagccaggatcacgcccttgagcaccaggcccaggctggtgggcggcaggccggatgcgcccacgccggccccgccgccaaagggcgcgagcgccaggatagaagccagcccgccgtcgccgccgcccaccggaggcagcctgtcgggcgtctcgatcctgctgcggccgtcatcccagccggtcatgcgccacgtcagatgcgcaagcgccacgcccacggatgtgacggcgacaagcgcgccaaggcggatccagaaacgggcggtcaaacgaaggcggatcatgccgacgcctccgcgtccataaagccgctgaggcgggcgagcgacgagccgctcccctcccgcgacaccaagatctcgacggcgatcaggtccggatcgtcggtcgcagttcgcgtcacatcgatacgccagcgccttcccagcatctcgacctcggcctgggcggcggccgggtcgcccaggttcagttcggccagacggttctcggcgatccactgcgccgcgatgcgatcctccagcccgccgacgctgtcgatgtgggcgcgtgtggccagcagcaggcccgtcgaggcgaccgccagcacgaacagcgccaccatcgcctccatcagagaatagccggagcggatcggggcggcgctcatccggccgcgccctgcacgctcagcggcgccgccaccgcgttcagaccgtcgaaccgcacgctccagccgccatcctgctggcgcaggagaaacgtcatgggcggcgccgcgctgtcgggatcgatcacggccgaggccgcgccgtccggaccggtcaggcgcacgccggccgacaggcgatgcggctcggccaccgcgtcggccggcgcaccggcgccttcgaagcgataggcgccgggcgtccaagcgatggccatgggccggccgctgaccagcacctcgtcggcggcgagcttcagccggtccgccaggcggttggcctcggtctgcgccccgtcgccacggcgcagcgatcccagccccagtacgaccacgcccgccgacacgccaacgacggccagcaccaccagcatctcgaccagggtcatgcccccgcgccgtcccggacctttgcgccccgcgcacgtcatcgggcgatcaacgcgtccgttcggtcagatcggcgtccagcccctcgccgccggcctcgccgtcctttccgtaggacagaaggtcgtagcggccgttctggccaggactgcgatagacataggcgcgaccccagggatcggtcggcgcctccggcagatagccctcgctgctccagttcgaaggaaccggcgcggtggcgggccgctcgaccaaggcccgcaggccctgctccgtcgtgggatagtcgccgttgtccagccgatacatgcgcagggcggccgagatcgtcttcagatcggtcttggccaccgtgacccgcgcctcgtccggccggccgatgacgttgggcacgatcagcacggccaccagagcgatgatcgcaaggaccacgatcatctcgaccaacgtcaggccctcgcgccgcgcgaggcgaggtttcaatcgtttcggcacttcaacacgccccgttgcagtagcgatctttcgcgtggggctgctatagcgtcgtcgagcttgggaacaaagccaaatgcaaagtgcttcgcacacgcacgacttgggcgggacgcagcctcatgtgacaggtttgtgtcgcatcattgatgatcgcattgttgcggtcgatgcgctctatgacggacctgtgacagttctggttccatctgaagacgttcttgtcgtcgcggtggatctgcccttcgcctcgcgtcgtcagcgagaggccgccgcgcctttcgccgtcgaaggcctgatcgcccagccgctggatcaggtccatgtggcgctgggcatggaggttgcgcccaatcggcacctgtgcggcgtggttcgtctcgacgtcatggcgcggtgggtcgcgctgctggatcaggccggtcttcatcaggtcgtcctgacgccggacgcgctgatgctggcggcgccgcccaccggggcctggcgtctcatgatcgagagcgatcgcgccctggtgcgcaccgaagacggcgcgggcttcgccatcgacctgcagggcctctccgccgcctgggagatcgccggccggccgcgcctggtttccgcaggcgaccccctgcccgagatcatgcgcgaaggcgtggacgacagcacctttgagctgacgaccaccggcagaccgctgctggtcgcgccgcctctggacctgcgccagggcgcgtttgcggccaggcacgctcgcccccggtcgatggcgcgcaccctgggacgggtcgccgcagcggcggtcgcggcgcacctggcgatccttgtcgtcgataccgtggcgttggaccggtcggcggaccgcgcggaagcccgcacgcgccaactcctcgcggcgcgcgcccccggcgcggaaagcgagcccgatctggtcgcggcggtggatcgcgtggcgccggaggcgtccggcgccggcggcggcccgttcatcgcgacgctggggcgggtctcggccgccctgccgggaacgcgcacccgctttcgggccatcacctatgcgccggaccagccgctggagcttgcggtgtccgcgcccgacgccgcagccctggacgccgccgtccgcgcactgaatcagacgggtcttcaggccacgtcgcgcatcgatcccgtcacgggcggcgcgggcgcggggctgaacgccgccgtcacaatcgctcagaggggagctcagccatgagccgggtgtcggccgtcgccgttccgccggtccaccgcgcggccctggcatggatcgagagccgctcccggcgcgagcagcgtctgcttcaggtcatgggcgcgctgctggttctggcggtggcctggtacggcgtcgccctgccgctgatgcgcgccagagaggcggccacggcgcggatcgagaccgccgcccgattgcagagccgtcttctgaccgcgcccgctagttctaccgccaccccgcccgtcgccgccatcaacggtgatttggcgcaggtggtcacgcaacgcgcgacggcggcggggctggcggcgacgggcgtagaggcgaacggcgacgccttcgccttctccatcgacactgcacgctatgacgccgttatagccttcatcgctgcgctggagggcgcggacggcgcggtgatccggagcctgcgcatcgagggggccggtcagcccggcctggtgcgcgtccggatgcaggtgagccgaccatgaccgccgaaccgctggaaacctcgcccgagccggccgtcgcccttccctatggcttcgcgcgccgcaacggcgtgatgatcgaggagggtccggacggcgccgtgtgcctgcaccgtcgctcggcgccgctgtccgtcttgctggaggtgcggcgtctgcgcggcgcggcggttcgctatgaggcggtggaggacgagcgcttcgacgccctgctgcgcgagcaaaccggcgtcgccgcaggttccgccgccgacatcgccgccagcgaagaagatctggccgccttggccgaggacgccgccgccgtcgacgacctgctggacagccgcgacgacgcgccggtggtgcgcctgatcaacgccatcctgctggaggctatccgcgagagcgtgtccgacatccacatcgaggcggaggagcgccgcctggtggtgcgtttccgcatggacggggtgctgcgcgaggtgctgtcgccgccccgcgcgctggcgccgctgcttgtcagccggatcaaggtcatggcccggctcgacatcgccgagaagcgcgtgcctcacgacggccgggtcaccctgcgcatcggggggctggacgtggacgtgcgcgtctcgaccctgccgacccagcacggcgagcgggtggtgctgcgtctgctggaccggggtgcgacggggctggacctcacgcacctcggcatgtcggcgcgcgacctggaggtgttcgagcgcatgatccgccgcccgcacggcatcatcctggtcaccggaccgaccggctcgggcaagaccaccactctctatgccgccctgacccggctgaacgaccgcaagcgcaacatcatgacggtcgaggatcccgtcgagtacgccttggacggcgttggccagatgcaggtcaacagccgcatcgacctgactttcgcgcggggcttgcgcgccatcctccgccaggacccggacgtcatcatggtgggcgagatccgtgaccatgagaccgccgaggtggcggtgcggtcctccatgaccggccacctggtgctgtccaccctgcacaccaacagcgcggtgggcagtgtgacgcgcctgatcgacatgggggtcgagcgctatctgctggcgcccatgctgaccggcctgatcgcccagcggctggtgcgccgactgtgtcccgagtgccgccgggaggacacggccaccgccgccgacgccaagctgaccaacgacgccgtgccggtaggcgcacgcgtcttccggcccgtgggctgcgccgcctgccgccacgacggctacaagggccgcgcggccctgtacgaagtggtcgaggcggacgctcgcatgcaggccatggtccacgacggcctgtccgaggccgaccttacccgccatgcgcgcacgctgggcccctccatcctcgacgacggcgtggccaaggtcgcccaaggcctgacctcggtcgaggaactggcccgcgtgatccacgaggacggctgagatggcgctctacgcctatcaggccgtggacgcctcagggcgcgccatgagcggcacggtggaggccggcagcgacgtcgccgcgcgcggcatggtgcgcgacctcggcctattaccgaccaaggtgacggcgcaggcccgcgcgggcgacaagggcggcgcccgcccggccatgggcctgttccgccgccgagtgtccgccaagagcctggccgccgcgacccgccagctgtcgaccatgatcagcagcgacatccgcatcgaggaggccattcgcgtcgtcggccaggagcatgcgacccaggccatcggcccggtcctgatggacgtcgccgccgccatcgttgaaggccacagcctgacggcggcgctggagcggcatccgcgcacctttcccgagttctaccgcgcttcggtcgcggccggcgagcagtccgggcggctggccgaggtcctggcgcacctgaccgagttcgtcgccaaccgcgagaagacggcgcgcaagattcagctggccctgctctatcccgccctgctggccgtggtgtcgggcctgatgatcacgctcctgatgatctatgtggtgccggacatcgtgaaggtgttcgtcaaccgcggggccgagctgccgctgctgacgcgggggctgatcgccgtctcctccgggcttcagcggttcggcctgccgctgctgatcgtccttggggtggccggcctggtgctgaaccgctggctggccgtgccgcatgtggcgctcaggttcgcgcggatgcggctgaccacgccgccgctgggcggcttcgtgcgccagctgaacgccggccgcttcgccggcagcctcgccacactggtgcgcagcgacgtaccgctggtggaggcgctgaaggcctcggcggcggtcacgcccaacctctatgtccgcgagcgcgccctgcatgtggcgcagcgcgtgcgtgagggcgcctccctgcgccgcgccatgaccgaggccgacgtctttccgcgcctgctgctggccgtggtcgccagcggcgagcagagcggccggctggggccggggctcgagcgcgccgccgccgatctggagcaggaactggaaggcctggtcgccgccatcgtggcgctggtcgagccgatggtgctcttggtcatgggcgggttggtgctgctgatggtgctggcgatcctgctgcccatcgtcaacctgaacaacctggccgggctgtgagcggagacgcctacagacgcgtctccaacgtcaggggcgtgacgcccggcagcagggccgccgcgcccggcagcactgacagggcgaccgccccgtcgcgggtccgacgcgccgtggcgatgggggcgccgtcgggccccatggcggtcatggccgagccgtccgcgcccgacgacaggttggccgacagcggcggcgtgggccgggccgggccgccggccttggccgcacaggttgcggcgccgctctgcagacgcccttcgccgctcatccccccgcgcagcgcgaggtttgccgccgaaacttgcaggtcgccgtcgcagacgaacggcagggcgggcgccagcgcattgagcagccgcgtcgatcccgcaccctccatccgccggatcaccggcccgttcgggcgcatcgatacgtcgcccatgatgtccgtgtccggtccccgcacggcgacgtcggctacgccggaaagcgagacgagcgaggagaacggccgcgtgctccagccggcggcgaagccaggctcaagcgccgcctcgcctttccacaccgtgcccaccacgtcgcgctcgtcccccagcgccgcctcggcgggcaggaagaccagcagcccagctaggtatgcgccgacgccggtcgccagcagcaccagccgccacggcgtgaccttgacgtacaggcgctcgaactgaaatgcgccctcgccgcgccccccatccccgtcacgaggacgccaaacccggaacatgccctgcctcttcgcccgcgaacgaggtggggactaaaggccggatcgcgcgcgggcgcaacggcttcaccctgatcgaggtgatcatcgcgctcgccctgttcgccttgatcggagtagccgggttcagcatgctgtcaggcgtgctgcagacgcaggaacgcacggacggccggctgcagcggctgtccgacatccagcgcgcggtgttcgtgatctcggcggaccttgatcagatcagcggccggatcgagggcgacggatcgagcctgacctttcagaagaccgacctgtccggtcggccggtcgtggtccgatacggcctgcgcgggccgcagctgtttcgcaccgtctcgggtcctctgggcgagcgggatcagaccattctgaacggcgtgcagtcgctgagctggacctaccaccagcgcggcttgggatggtcgcccaccccgcccccgccgccaacgcctgtcgatccactggcgccgccaggcctcgtcccgcccccgcctcctccgccggttcaagcggtggccatggacctgcggctgctgggcgtcgatgggcgcgaggcgacgctgcggcgggtgatccgcactccggagctggcgccgtgaggcggccgctgtcgcaagcccgagagggcatgatcctgctgaacgtcctggtgatcgtggcgatcgcggcggcggcggtggcggtgatgatcgcggcgcaggacatcgaggtgcagcgcaccatccgcctccgcgacgcctctcaggcccaggcctatggccgggcgggcgagctgtcggccgtggtcgccctgcgccgcgacggcgtcgcggccccgacgctggacgcctacagcgagccttgggcggcgatcgcgcagcgcccgatcagcatcccgaacgggcgcttcgccctgtcgatcgtcgacgagcaggcgcgatacaacttgaaccggctgaagggaggcgacgccgtcgaggcgtcgcgcttcacccgcattgcgcgagccctgggcgtgtctcagccaggcgtcgtcgcggtggccgccgtcatcgccgccgtgggccccttaagcgacgagggcctgctgcgtacggccggcgtcgatccggccgatctggatcgcctgcgcccctttgtgacgtttcttcccgaggacgcggggctgaacctgaacaccatctcgccggagctgctggggtttcttttggacgatgcagacgcggtccgccgcctgctggacctgcgcaacagcaagggcgcgctcacggagcccgatctcgcggccttggggctgcagaacctgggcggtctgacatccagccatttcgccgtggtcaccgacgtgcgtgtgggcgatgtggagcagcgggtgcagagccgcctgacgcgcgtccttgcgccggaacaggtggtggtgtcggtttcctcacgcaggcgcatcgacgccgccaccggcgtctaggcgcacggccccgtgtcgcaaagctgttccgcaacagccggacggagatcaaccggccgtttcgggagacaggcgaacgcgaagcgacgtcagacctcggtcaggcgacgctcggcgctgttcacgctgaaccgcttcacgaccgaggccgtgtagggcttggcggtgatggtcgatacggcccaaagctcggccgtcgcgcgctccggcgtcagtgtcagcagcacgaagcccttggacgcctggtcgcagaagaccacctcgtcgctggccgccgccagcgcctgtccgagcggcagtccggcgacggcgtcgcccggagacgggctggagatggcggaggtcccgaactcgaccgcacgccgctcgccggccgcgtccttcagctcgttgacccagaaggcgtggctgtcgccagccaggacgattggctcgacgccggcggtcttgaacgtctggtacagccgctcgcggcccgccggatagccgtcccagctgtcgaggttgaagggcaggcccagcttgaacagctgcagcgcaccctgaatccggggacgaacctcctccggcaagctcgacatgagctgcgcgatctgggcggcgggaaccatgcgttcgacgtcgggtcccttgacccgcgccatcaccacctgattacccaggatctgccacggccgcccggccgctttggacgcggccagctcgccgccgatccagcggcgctgctcgtcgcccagcaggtcgcgatcggctgcgttgcgcaaggcctcaaaggcggcgacgtccggcgcgcccgccgccgtgcgcggcatatcggcgaaatccagctgctcgttgcgcgccagcagacgcgtctcgaccatgatcaggctggcgaggtcgccgaagtggaagctgcggttgatcgcctccttcaagccgccggccctgggttcccggatgggcatccattcgtagtaggcgcgcagggcggccgccttgcgcacggcgaagtcgccttcggtcgccggctgatggttctcggcgccactggcccaggtgtcgttggtgacctcgtggtcgtcccagacgcagatgaaggcggcgcgcgcgtgggcggcttgaagatcggggtccgacttgtattgggcgtgacgcgtccgatagtcggccagcgagacgatctcatgcggcggctgcggcgtacggttcaggcgcgcgccgttcaccatgccgtagtcgtccggctccgccccgtattcgtagatgtagtcgccgaggtgaaccaccgcgtccagccgttccagcctggcgatggcgtcataggcgttgaacaggccgccggggtacagctggcaggacaccacggccatcgcgacctgcggcgtcgcctcttccggcagggtgcgcacgcggccgacgggcgacacgacgtccgccgccgtgaagcggtagaagtattcctggccgggctcgagcccttggccgtccaggtcgtgcttgacggtgaagtcgcgctcgacctgcgcacgcaggcccgaggatcgccgcaccacgtcccggaactcggcgtcgcgcgagacttcgagcgtcaccgggatgtcccccgaagcaggatcggcgggggtcacgcgcgtccagaacaccgccgaatgccggtcaggatcgccgctggcgacgccgtgcagaaaggcgggccgaccttggaccaaggccggggcggtggcgcaggcgcccgtggcggcccccgctccgaacaggcctagaagactgcggcgatcaagcttcatcggatcggctcctagtaccgcagcttcagggcgaggccgtaggacgccggtcgcccggcgatgaacgtgggcagacccaggctgtcgccggtgttgccggcatccttgatgtactcttcatccaggatgttctcgccaaacgcttcgacgccccaggcgccgccgtcggcttcgtagcggacccgcaggttcagcaggccaaagctgtcctgacgctcgtcctggatcaggtcgggcacgaagttgtcgctctgcagctccggccggtcgttgtcgtcgtcgaagaacatctccgactgccaggtgtaggtcggcagcacctcgatcgcaccgccccgcaccggggtgcgccacacggcgcccagcgacgcgcggtggtccggcgacaggcggaagcgattgccgtcgtagatgcccgcctcgaaccgcgaatggttgtagccataggtcccgaacagctcgaacgcgtcggtcagctgaagcgtcgcctgcccttcaaagccgtaggacagcgcttcgccagcgttggtggtgatgaagctggtgccgtcctgtacagtcgtctggaagttctggtagtcgtagcggtagatggcgccgtcgagccgcagccgccggtccatcagcgccgccttggcgccgacctcgaagctgtccaccgtctcagcggcgacggggctgaatcggggctgaccctgcggtgcggacggcgccgccgcgctgatcacctcgggccggcggccccgggcgtagttggcgtagaggttggcgtcatccgacagcgcgtaccgcgccgtgacccgccaggtcaggccgtcgtcttcggagtcgacatagacgaaatcgccgttgttcggcgtcggctgagccgtcagaccgaagagcggaaaggcggcggctgggagcgacagtacggcagggttggccagggccgccagcaccgccggtatctgcgccgccggaaccgcgccctgctgcacggcgagcagaccgcccaggaccgagcggctctgcaccgagttggcgaagcctgtggtcttgtcgtcgcgggtgtagcgaagccccgccgacatctcgaaccgatcggtgaaggcgtaggtcgcatcggcgaagacgtcataggacgtcagctccgagctgttggtgggcgtctcgatgtgggcgggcttcagattggccgcgatcggaccggcgaaggcgccggcccccagcggggtcagcagcgccgccagagcgccacgcgccaccgtcggataggccgcgagcggaagcgtattgatcccagccgccgtcggcgagccgtccagcagtcccgacagctgcgccagcgccacgcgctcgtcgaactgggtcggcgtgcgctgatagccttcttcctggaaccatccggcgccgacgaagccggtcaggcggccgccgccgtcgaagcccaggcgcaggtcctggctccattgcgtgccgtgcgcgtcctcggccgccgtcaggatcggcagggacacgccatcggcgtcaaaggtctcgtaggagtcgaattcacgataagcggtggtcgcgttcagcgtccactccggcgacaggtcgatgcggctaagggccgtcacgccccagacctcgcggtccagccccaggctcttgccgccgtcaaacgccgcgccacgggtcagcgcggcgccttcccatggcgcgcgatcgcccagaaccacaccggtgaccgggtctgcgggcgcataggcgatcgacttgaacgaggtgccggacgcctgatcggtctgatagttgccgatgacgtccacccgcaccgcatccgtcggggtccaggcgccggacaggcgcaaggccttggtgtcgatggcgttgtagtcctcaccgcccaacagattctcgacatagccgtcgcgcgtcttcatgcgcgcagccaggcggacagcggcgtcttcgccaacgggagcgttgagagcgccctcgaccgagacataaccctcgtcgccggcttccagctcggcataggcgccggtctgtccaggtcgggcgcggttctggacgatgttcaccgcaccaatcagggcgccgcgtccgtagagggtcgactgcggtcccttggcgacctcgacccgctccaggtcgaaaagctcgacataggagccgcgcgacttggagatcgacaccccgtcctggaacaccgacacgcgcggctcggaagtggcggcccccgagtccgaggtgatgccgcgcatcacgaatcccggattgttcggtgactggttctgcaccagaaagcccggcgtgaaggccgacagctggtcgaactcctggatgcccagtcggtccaggaactcgccggaataggcggtcagggcgaacggcacctcgatcgggtcctgctcgcgcaactgggcggtgacgacgatgtcctcgaccgtgccgacggaggcggcgtcttgagcggaagccgctcccgcccagacggtccctatagccgccgccgcaagcagctgcgccttccgaatcgataccgtcattcttgcagtcccccgacttggcgatgtcagggggcttagcgaggcgcgttatcaggacgacgaccgttttgcgcaggcctggcgacgtcctcgcgcacaaaccgcgacaaacatcccgctcacggacattccatacgcgcgccctcgacgagcggcgatcctgcgtgcaaccccagctaggcggccaaatcggacgacgccacgtccgcgccgacgattggccttcgctgctcgacccaaggtcggcggctgtttgaacccatcgcgatcaggccacctcgggcaaccggtccaggtatttgtcgagggtgatcggatactcgcgaatgcgcacgcccgttgcattgtaaagggcgttggccacagcggcgccgacgccgcagagacccagttcgcccacgcccttggccttcatcggcgacaccttgtcgtcggcctcgtccaggaagacgacctcctgatgcggaatgtcggcgtggaccggaacttcgtagctggcgaggtcgtgattgacgaagaagccgatacgcttgtcgacggcgagttcttccatcagggcgccgccgacgcccatcgtcatggcgccgatgacctggctgcgggcggtcttgggatttaggatgcgtcccgccgcgcagaccgccagcatgcgccggatctgcgtctggccggtgaagcggtcgaccgccgcctcgacgaagtgggcgccgaaggtggactgctggtaacgctccgacaagtcgccccactccatggcgtcttcagccaccagatcaccatcccgcgcggcgcggcccagcggcgccgatcgccggccgctgcgcacccggcccccggaaaagtcggcgtcatcggggttcaactccagccgttcggccgccagtcgcctcagcttgacgcaagccgcatagacgcccgaggtcgcgctgttggcgccccactgaccgcccgagccggcggacgccggaaagctggaatcccccagcaccaccgagacgcgatccaggtcgacgcccagcatctccgccgcggtctgggcgatgatggtgtagctgccggtgccgatgtcggtcatgtccgtctcgaccgtgacccgcccgtcggcgctgagccgcacgcgggcggccgacgtcatgttcatgttgttacggaaggcggcggccacgcccattccgaccagccagcggccgtcttgggtcacgcccggcgcggcccggcggctccagccgaaccgctcggcgccctcctggagacaccgcaccagctggcgctgggagaacggccgctccgggttcatcggatcgaccttggtgtcgttcatgacgcggaaggccaccgggtccatgcccagcttctcggccatctcgtccatggcgatttccagcaccatcatgcccggcgcctcgcccggcgcgcgcatggcgttgccctcgggcaggtccagctcggccaggcgcagacgggtggcgatggtggggctaccatagagcagttgcgtctggctcgtcgccgtctccggcccgcctccgggcagatcgccgctccagctttcgtgcgagatcgccttgatgcggccgtcgcgctcggccccgatgcggacacgctgaagcgtcgccgggcgatgggtggtgttgttgctgatgaagggtcgcggcagggcgaccttgaccgggcgacgcacctcgcgcgccgccagcgcggccagcagcacgtccgcgcgcaggaacagctttccgccgaacccgccgcccacatagggcgacgaaatccgcaccttctcctccggaatcttcagcgtcgcggccagatccccgcggccccagtcgatcatctggttggacgtccagacaaacagctcgtcgccgttccaccgcgcgacggaggcgtgcggctccatcatcgcatgactctggtccggggtatggtactcctcgtccagggtgacgggcgccgctgcgaacgcggcgtcgaagtcgcccgaggtcttgtcggcgttctcgccttccggctccttggccgcgccgcgctggtcttccaggctgaagcgcccctgcgagcggccatagctgaccttgaggcgcgaagcggccgcccgcgcctgttcaaaggtctcggcgaccaccaccgcgatcgcctggtgatagtgctgcacctccggcccggccagcagagcggcggtgttgcgctcgcccttgcccagctcgcccgcattccgggcggtgacgacgcccaaaacacccggcgaggccagaacggccgcatcgtcgatcgcccgtatccgccccttggcgatggccgatcccaccacatagccgtaggcggcggtctcgacgccctgggtgtgctcataggcgtagagcgcgcgacccgtggtcttcagcaggccgtcgatcctgtcgtgcggacgtccgacgaccttcatctggtcgatgggattggggccggcggggtgttcgaacttcatgcccgggcctccgagatcgcggcggccagggtgcgcctggccagggtcaccttgaaggcgttgtcgggctggggccgcgcgcccgcgaagacctggtccgccaccgcggccgcgccctcgcgcatcgcgccttccgccgcctccacccgccagggcttgtgcgccacgccgccaaaggccgcgcgtccgctcccgtccggctggatcaccgacgcgacggacaccagcgcgaaggcgtaggacgcccgatcccgcaccttgtgatagctgtgcgtccctccgatcggaggcggcagggtcacggcggtgatcagttcgcccggctccagattgacgtcgcgttgcggggtgtctcccggcaggcggtggaagtcggcgatcggcaggctgcgggtctcgccgctcggcgtcaccgtctcgaccacggcgtccagcacgcgcatcgccaccgccatgtcgccgggataggtggcgatgcaggagtcgcttacgccgatcaccgcaagctgacgcgcaaagccgccgatggccgagcagccggtgcccggctcgcgcttgttgcacgcttgatcggtgtcatagaaataggggcaccgcgtgcgctgaagcagattgccgcccgtggtcgccttgttgcgcagctggccggaggcgcccgccacaatggccttggtcaagacgccgtagtcgcgccgcacgcgcggatgactggccagggcggtgttggtcaccagggttccgatcctgagcccgccctcctccgtatcctcgatgcggtccagcccgaggtcctgaacatcgaccagatggtccggcgtctcgatctccagcttcatcagatcgagcagattggtcccgccggcgatgaatttggcgcccggacgcgccgccaccgccgccgcggcttcggcgggcgtgcgggcgcgttcgtaggtgaaggccctcatgcccgcacccccgccacatcggccatcgcgtctgcgatgttggaataggcgccgcatcgacagatgttgccgctcatccgctcgcgcatctccagcgtcgacatctcgggccggccggccacgtcggcctgcacatggctggggacgcccgcgcggatctcctccagaacggccaccgccgaacagatctggccgggcgtgcagtagccgcactggtagccgtcatgtttgacaaaggcggcctgcatcggatgcatccgctcgggcgcgcccagcccctcgatggttgtgaccttgtcgcccgtgtgcatcaccgccagagacaggcaggcgttgatcctttggccgttcaccaggacggtgcaggcgccgcactgcccgtggtcgcaccccttcttggttccggtcagccgcaggtgctcgcgcaaggcgtccagcagggtggtgcgggtgtcgagctgcagcgacacaggttcgccgttcacctccatctgcaccgacacgacgctgcctgcggccgcgggcgctggcggcggcgcttcgggcgtggtctgcgcctcagccggcagggcgcccatggcggcgccgccggcgccgccgatcagcactttccggcgagaaacctcgagatcgataatgtccggcaccgccgcctacgcttcgcaaccatccgcagggatcgctcagcgagcgcgatgttccgacggaacacgcgtgcttccaactcgctgaaaacacgacccgatcatcccaacgcgcgagcgggcgaaaaggaccacggctgcggctaaaccgaagttcccacggccatcctgttcacgctggaggctgaggggtcgaggccttcgatcagccgctggcgccggcggacggccagttggcttcgaagccccgcctcgccgcggcgacgccgaaggtcgccgggggacgagacgccgccgaacccgcgccgccgccggacagaaccctcagttcgggccttgcgtccgacgcctgcgtggtgaactggcccgccagcgcgaccagctgggtggcctccgtgcgcaaggacatggccgaggcggtggtctgctcgaccatggcggcgttctgttgggtgacctgatccatctggttgacggccccgttgacctgctgaagcccgatcgcctgctcctgcgccgctgcggcgatgtcggaagcgagttggtccatctgcgccacctgatcggtgatcccgttcagggcgctgctggcttcgttcaccagcccgacgccgcgaccgacctcctgcgaggaggcggagatcaggctcttgatctccttggccgcgccggcggagcgctgcgccagcgcccggacctcggaggccaccacggcgaagccgcgcccgctgtcgcccgcacgcgccgcctcgacacccgcgttcagcgccagcaaattggtctggaaggcgatctcgtcgatgacgccgatgatgtcggcgatgctgcgcgagctgtcttcgatgccgctcatggcggcaaccgccgcctgcatgacttcgcgcgagcgctctcccgcccgtcgggccgaggcggcggcgaccgacgcgagccgcgcgctttccgcgctttgcgacacggtggcggtgacctgatccagggccgcggcggtctcctcgatgctggccgcctggcgttcggtgcgtcgggacaggtcgtcggacgccgacgaaatctcatcggcgctgccgctcagcgcgtcggcggcgtcgagaacctgatgcatggcgccgcgcagactgtcgatggcctggttgaagtctcggccgacctgctgatgagcttcgcaaagcggctcttcgatgcgcgcggtcaggtccccgtccgacagtcgggccagctttgtctccagaagcgcgatcaactccgcctgctgcgcctcgcatagcgaacgcgccgcttcattgacggccgccgcctgctgctcggcgctgatgtcgatcgccagcttgatgacgcttcttggcacgccggccgcgtcacgcactgggttgtaggacgcctggagccacacctcgcgtccgtccttggccacccggcgaaaacgctctgccacgaactccccggcgtttagacggcgccagaaggccgcgtagtcgttcgaggcagcttcgtgcggcggcatgaacatccggtggtgctcgcccttcagctcgcagagttcatagcccatcgtcgcggtgaagttggcgttggcgtcgagaatgaagccgttcatgtcgaactcgatcaccgcctgcgaccgccctatggcgtccagccgggcctgagccgacgcatcggcgctctctgcaggcccccgcctgttcaatgtccggagcagcatctcttcccccaatgccgtcacaacgtggggttgagagtggacgccaaaggtttcgacttggtttcccggagcaagcatccgccgccctccgatgtcatcacaagacgcccggggcccctgatcgggccggcgccgcacgacgccgacggatttccttccttggctgcagcccggacaccgaagcgttggttccggctactcctgcgacggcacgtcctcgcccgcttcggtacggtcccgaaacagggctgcgcgcgccagcaggatcagggtgactggcgtggtgatcgtcagaaaaaggccgatcagaacctctcggggcatgaagcggcgctcggctacagtgaaatagatcaccgaactcgccaggacgagcgccatgccgagggtggctccgagcgtcggcgcatggacccgctcgtagaaggttctgagctgcaccagaccaatggtcccgatcagcgacagcccggcgcccgccagggcgagcaccgtcaccgtccatgcggcccaaagcggcaggtcggctcccgtcattcgatcacctcgccgcgcatcatgaatttggccagggcgacggtggcggcgaagcccagcatgccgatgatcagagccgcttccagatagagggagctgccggtgcgcacgccgaacacgacgaccagcaacatgccgttcagatacagcgtgtccatgcccagcacgcgatcctgcgcacggggaccggccatgatcctccaggccgccagcgtcatggcgcagaccaacatcaactgcgccaaacccagcccccagaacaagacggcggcggcggtcattcaaagatctccatcagcctgcattcgtagcgatccttgatcaggcgtatccacacctcctcgtcgacaaggtccagcacgtgcaggagcagccgccccgtggccgcttcatattcgacccaaagggtgccgggcgtgctggtcaagatgatcgcgagcacggcgagcccgtaccggtcgcgaagctccaggggcacatggatgaagccggacacccgcttcttgcgtcggcccgccaggatgatctgagccaccgcccagttggaccgcagcacgtccacggaaacaagggccgccagggcgaggatcgacaggggccggcgaacacgcacgggctcggcgcccagcagccgcatgacgtgcggcagaacaaccgccgccgtcgcagccagggccagcgaaggcgctcccaacgaggcgctcatcaaaatcgaggcgacgaacagccccagcgacaggaaggggtgcggaaggatcgcgctcatcgtccgcccccgctcagaaccgcctgcacataggcttgggggcgagacagccagtcggccgtgtgctcggcgtagatcaaggccgagccgccgaatacggatagcagcacgcaggcgcccagaaggcccgcgatggcggtgaactcggcggcgcccacgaccagacgcggcgcatcctcctcccgcccccatatcgccgcgacgccggcccgggtcaggccgatcagggctcccaggctggacagcgagagcgccgccaccatggtccaggccgtgacatcgccgacgcgcgccagagcgtccatcatcgccagcttgccgatgaagccggacaggggcggcaggcccgcgatcatcaggacgcacacaagataggcgccgcccatcgccgccacggccgccggaatgaccaggccgggttcgttgcgctcgtcatcgtcgaagggatcgcgatactcgtcgtcgaacaccgcccgttgcggacccgcgtccggatctcgccctcgctgaagcacctccgccatcagaaacagggccgcgcacgccagcgtcgatcccgccaggtagaagatcgcgccgctcagcgccgccgggccgccgatcccgacgatcgccagaaccgtgcccgacgacacgatcacgccatagcccgcggcccgcgaaaggtcgcgcgacgcgagcagacccgccgtcccgaaacccatcgtagccaggcctccggccaggagccatccctggccgaagccggccgacgcgccggcgtccgcgccgaacagcagaaggctcaggcggatgatcacatagacgccgaccttggacaggatggcgaaggcggcggccgctggggcgctggcggcggcgtaggtcggcgtcagccagaagccgaccggccacatggcgcacttgatcagaaaggccgtgcccagcaccgccgccccgacatggaacaggccgcgatttccttccgcaatggcgggaaggcgaagcgccagatcggccatgttcagcgtgccggtcacgccatagatcaggctgacgccgatcaggaacagcagcgacgccgtcaggttgaccgcgatgtaggtcagtccggcccggatgcgcgcctcgcccgatccgtgcagcgccaggccgtacgaggccgccagcatgatctcgaagaagacaaagaggttgaagaggtcccccgtcaggaaggccccgttcacccccatcgccagcagcaggaaaagcgcgtgaaagcgcggcccggctcgatcccacctcgccagcgcgaagatcagcgagcaggcgcccagcacgctggtcagggcgaccatgaaggtcgaaagccggtcggcgacagggacgatgccgtagggcgccgcccagccgcccagccggtaaatcctggccgtgtcgccgccgccgctcccgcccgtcgcgctctcgtgcagcaggaccagcgccatgatgaggatggcggccatggcggagaggctgagaacgcccttgatgatgcggcggcgctcgtccagcagcagcatggccgccgcgacgaacagcggcaacacgatggggccgatgacgaggtggtcgcgccattcgatcatgcgtccggctcccgtccatcgacgtggtcgctgccggtgacgccccgggcggccagcagcaccaccaggaacagggccgtcagggcgaagctgatcacgatggccgtcaggacaagagcttgcggcgtgggatcggcgtaccgggcgggatcggtgacttcgccttggagcacgggcggtctccccgagcgcagccgccccatggcgaagatgaagatgttcaccgcataggacagcagcgacaggccgatgatgacctggaaggtccggggtcgcaggagcagccaaatccccgacgcggccagaattccgatggcgagggcgagaaccagctcggtcattccgcctccccttgcccgtcatcgccacgcggccggcgcagcgactggtgcgccagggcgatcagcgtcagcacggtcgctcccacgaccagcaccaccacgccaaggtcgaacgccaccgcgctggccagcggcacgcgaccgagcagcggcaggtcggcgtactggaaccaggacgtcaggaacggatagccgaaaatccaggagccggcgccggccgccaaggcgatcagcaggcccgcgccgatccaggccagcggcctgatggtcagcctcgcctcgaaccggcgagcgcccgaggccatgtactgaagcacgaaggcgatcgcgatggcgacgccggccgcgaatccgccgcccggcaggtcgtggccgcgcaggaacaggtggatggcgagcagaagaacaaagggaaacatccagcgcatgacaacgcgcgggacgagcatggtctccctgagggtgtcgccttcgaccctgttctcgcgccggcggtcggcggcgtcctgaacccgcttctggcccggatcatccagggtgtcgttcgccggccggaagcggcgcagcagggcgaacaccgtcaggcccactatgccgagcacggtgatctcgccgaaggtgtcgaaggcgcggaaatcgaccaggatgacgttgacgatgttgcgtccccccgcctcgctataggcgtgctcgacgaagaaccgcgacagcccctccacggacggccgcgtcatgaccgcatagctgatcaccgcgagggccgttccgccggcggcggcgatgacgaggtcgatacggcgccgccggcgggaacgtcgctccagcagcggcggaagccggatgggctccagccgcttgggcaaccagcgcaagccgagcagcagcaggacggtggtgaccacttccaccagcagctgcgtcatggccaggtccggcgccgacagccacaggaaggacaggcagctggcgatgcccgccccgcccatcagcaccaccgccgcaagcctgtggtacttggcctgccaggcggccgccaccgcacagcccgctccgatcagccacagccctgcgaagctgaactccatgaagctgggagcgggtatcggcgcaagccgcccaaggccgcccaaggccgcagatccaccggcgaccagcgcaaggaggacaatggcgcgaagctgcggctgcatccgcgtcgcgcccgccagacgcacgacgatccgggcaccgcgcaccaagctggtcatggttcgctcgaacaaccagccgccgttcagccgcttccatccccagggcccgcctcgcggattggcgttgatgcggcggccgaaggcgacatagaggcagacgccgcccaccagcgcggccacgctcagcagcagcggcaggttgaagccgtgccagagcgccaggctgtagtacggaagatcgaagcccagcaccgacacggccgcgctcttcaggaacggccccacggtgaccgccggggccacgccgaccaccaggcaaagggcgaccagcacctcgaccggacgccgcatccagcccggcggctcgtgcggtacgcggtccagctgggtcggggccgggccgaagaaggtctggtgaatgaagcggagcgagtaaagcacgctgaaggcgctgccgagcgtcgccaggaccggcagggcgaaactcaaggcgtccgcctcggcgttggcgaccgcctcggccaggaacatctccttggacaggaacccgttcagcaagggaacgccggccatggccgccgccgccaccatggccaggatcgcggtgaacggcatgaagcggaacaggccgctcagccgccgcatgtcgcgggtgcccgtctcatggtcgatgatgcccgcggccatgaacaacgaggccttgaaggtggcgtggttcacggtgtggaagatggccgcgatggcgcccagcggcgtgcccaatcccagcagcagcacgatcagccccaggtgactgatggtcgaataggcgagcagacccttgagatcgtgctggaagatcgcgcaccaggcgccgatcaaaagggtcgccagccccgccgtgccgaccagcagacgccactcctccgttcccgccaggacaggccagaaccggatcagcagaaacacgccggccttcaccatggtggcggagtgcagataggcgctgacgggcgtcggggcggccatggcgcgaggcagccagaagtggaacggaaactgcgcgctctttgtcatggcgcccaggagcacaagcagcagggccggcaggtacagcgggctgtcctggatcgcctcccgtgactcgagaacgacatcgaggtcgtaactgccggcgacgccgccgatgatgatcattccgaccaacagcgccagaccgcccacgcccgtgacggtcagcgccatgcgcgccccgtccttcgccgccgggttctgatgccagtagccgatcagcagaaaggaaaagaggctggtcagctcccagaagaccaccagctggatcaggttgccggacagcaccaccccctgcatcgcgcccatgaaggccagcaggaagcagaagaagcggggcaccgggtccttggacgacatgtagtagcgcgcatacagcaccacgagcgcgccgatgcccaggatcagggcgctgaacagccaggacagcccgtcgagccgcagcacgaggttgacgcccagcgacggcagccaggcgatctcatgcctcagcgtctcgccgtcctggaacaacggccacaacgccgtcaggcagcccaggctgatcagggcgatgatccacgacaggatcgccgccgccgttcgcgcatgacgcggcagacacgccgccgcaatggcgccgccgaaaggaagggcgagaacaacaatgagcagcaggttgaaagacatgaagacgggctgtttctctcccaggatcaaaaagaggagacgctgacctcaacgctcccggcggccccgagccttatcagcggcgcaccaccgacgatagccgagacctggcggctgcacgtcgcacccgccaaaggctgcgccgcgccacgacggcgaaaggccgcatggcaggtgttcaccggcgcttcgcgaatgacaggccccgccgttcacgcaccagagccgtccctctccgcaagttcgctggccgttggaacctgaggcggcgaggatcgggacatcgagaccgacaccgtgtctacgcccttacaaaggatcgtcgccatgatctgttccgcgttgatagcggcgctatgctgagcccatggaaactcctggcgccccttccgccgtgtcgcagatcacccggcgcaccgctcaggccgaaatggtgacggttactaggtttcaggaccttcgccgccaaggcgagccgatggtgctgaaagggctggtggccgactggccgctcgttcaagcggccgctcatgaccgcgcgccggattacctgaagcaaatcgccagcgatgatcctgtccagttcatgcgcggctccggagatccagggtcggctgcattacgcccagggcgcggaaggtcggaacttcgagccgcatcgagcttcgctgcatgcgtttcttgatctgctcgccgcagaagcggacaagccgaaaggcgattcgcttgtgctgcagggaatgccggcggacgagcgcctgcgcggctttttggccgcccatcccatgcccctgctgccgacctccgtcgctccgcgagtctggatcggcaatgccgccacggtcgccattcaccacgacccttcggaaaacatcgcctgcgtggccgccggtcggagacggttcacgctttttccgccggaagcggtcagcgacctctacatggggccgtttcaccagacgccggcgggggttcaggtgagcatggtccatctcaccgacccggacctggagcgcttcccgcgcttcgcccgcgcgctcgaggtcgcccaggtcgcggagctggagcctggcgatgcgctgtatatcccgtaccactggtaccaccacgtggaatccttggctgcgttcaacgtgctggtgaactactggtgggatcccgctcaaccgggctttggatcgccgtgggacgccttgatgcacggcatgatgagcttgcgcgccctgcccccgcagcagcgtcgcgcgtggcgcgcgatgttcgaccactatgtcttcgagacgaacggcgatccgggcgctcatctgccaagcgacggccggggaatcctgtccgcgcccacgccccgcgccgcagcgcagatggcgcggattcgtcgtcagaagctggagcggaactaacgatcggccgggcagacccgcgcaacatagtcggcgtgtgggggcatcgcggccacgcatttggcgatcacggcctccacgccgccgaggaagccggcgatgtcgctttcgtccgtgacgtcgacagaagggtcgtagccggcggggacgacgccctgccccagcaggacctggatccagctttcttctgcaaacagttcgtcgtcctcgcggaaggtacggccgttggcgcgaaacagatccatcttccgctgaagggtttccgaaacggccatgtcgcggcagtatcgccagaacggcgtgtcgttccgctccgtcgccttgtagtgcaggatgatgaagtcgcggatgcgctcgtattcgaagtccgtctgacggttgaactcggcgatcatcgccggatcgaacgacatgtcggggaacatccgcaccagccggatcaggaccgactgcaccagatgcagactggtcgactccagcggctctaggaatcccgaggccaggcccgcggccacgcagttgcggttccagacctggcggcgcttgccggtcgtgaagcggatgcggttcggctcggccatctgctcgccgtccaggttcgacagcaggatgcgctccgcctcctcgtcatccatgtaccggctggaatagacgtggccgttgccggtgcggtgctgcaggggaatgcgccattgccatcccgccggcctggcggtggcgcgcgtatagggggtgaacggctctgtgcgggcgcaagggaccgccatggcccggtcgcaaggcaaccaatgcgtccaatcctcgtaccccgtcttcatggcctcttcgatgatcaggccgcgaaagcccgagcagtcgatgaacaggtcggcggcgatcacctcgccgtcctccatggtcaccgatcggacaaagccgtcctcggcccgcaactggaccgagccgaccttgccctcgcgccgccggactcccgccgcctccgccatctggcgcaggtatcgagcgtacaggcctgcgtcgaagtgaaaggcgtgggcgatgtggcccagcggcgaggtagggcgcttggcgtcggcgcgcttgaagcggttctgcagcgccgccgccgtgttgatggaataggcggcgaggtcggacacccgcccggtctcccgcaaccgcagccagtattgatgcagcctcagccattccaggtcgcggccgatgacgccgaagccgtggatgtagctggagccgatccggtcccaatcgacgaactggatgcccagcttgaagctgccctgggtgcggcgcaggaaatcgtcctcgtccaagccgatcaggctgttgaaggacttgatcgcgggaatggtggcctcgcccacgccgatcgttccgatcgcctcggattcgacaagggtgatgatcttcccccgtaaaagtggacggggttaagccgctttgcgctcggcctcagcggggctgatatagcccagtgctgagtgcaggcgatggggattgtagaagccctcgatgtatccgaacaggtctcgccgcgcctggtctcgggtggcgtagacgcggtgatgaacgcgttcggtcttgagggtgtggaagaagctctccatcggggcattgtcccagcagtcgccctttcggctcatcgacggggtgatgccggatcgggccagggctgatcgataggcttcggctgcgtattggatgccccggtccgaatgatggatcaggccgggcgcggggcgctgacgttcgacggccatgttgagggcgtcgagggcgatctcggtgtgcagggtctggcgcatggaccagcccacgatcttgcgggtgtgcaggtcgaggatggcggcgagatagagccagccttcgccggtcgggatgtaggtgaggtcggcgagccagacctggttgggcgccgccgcctcgaagttccgggccagcctgttgggcgcgatgggataaccgtggcggctgttcgtcgtccgggcgcgacgcggcaaggccgccaagccccgcaggccggcgcggcgcatcagccgctccacgcgggatcgaccgacccgacgcccatgccgccgcagggtggcgtgaacgcgcggcgagccgtaacagccgctgctctccgcatggatcagccggatatcctcggtcagctcgcgattggcgacagaccgctggctctcggggcgaccgcgccaggcgtagtaaccgctggccgacaagcccaggaccgcgcacatcacgcgaaccggccagacctgacgatgctcatcgacgaacccgaacttcatcgggagaccgctccgaagatgagcgcggctttttttaggatgtcccgctccatccgcagctgaccgttctctcgccgcaaccgggccacctccgccgccagatccgacggcgacggggacgacgcctgcgttgtggggcgccgcgacgcccccgtcgcctgcaccccgaactgcgtcatccatcgacgaagcaccgtctcgtgcagcccaagctcgcgggccaccgccccgacgctcaggccgccgttggcgacgcggtcaacggcctcgcgcttgaaagaatccggaaagttccggcgttgaacactcatcagacactcctctccagctccgaaaagctagcatgggtgtccaccaaaccgagggaggatcaaaggctatgggtgccataggcgctgggattcaggtcgatcattctcacccaggtatcgaccagccgggcgtactgcctggtgcatatgtgctctccatcccggctgcggctggggaacagccagtcatcacgccgtcttcctcggcgctccaaccagtgagccagagcttccctcgcggcctccgtgatctcgaacggcacgggccgaccggtcttctgctggatgatcgtcgaccgctgccgaatgacgccgccttgagcaatatcgcccagacggagttttaccagatcacagccccgcagcttggcgtccaatgcgatgttgaacatcgcgagatctcgtgtcgatccaacggacttcaggtgctgacggatcgcccagatgtgctttggcttaagtggggccttcgcaccggtcattcgaccagcgttccagggtttgcggggtaaacgaaacagatcgggctggctcatggccacctcccacgatcaacaccccccctcctcaagatacgctccaaacaacgctgatgcgccagaagcggccactgtcggcgttgcaagaacgcgacttagaagctcgacgtgggtttggttactggttgcttgctgagttctgctctaagcccgtcgccgatgtttgaacagttcagcttcgatggatagcgcgaacgtcagccaaagcgcgataggatccgacatccgcagtgtcaccatcccttcgatgtcgagatagagtttgtttctctctagctaactgatttgttcgcgcccgacgtcatcgacgcaggtcagaacgcgctggtccacgcaccacccacaggccgccatagacgaaggcaaggcctgtcaaaatggctgccaaacctgagacttctgaaaggctggcgcccatggcgttcaggcgaacaaaggcctgaacggcagcggtggacggtgaaaaatgcgcgagccagacgagaccttcaggcatcatgaaatgcggccacgcagcgcctgacaggaagaacaagggcgcggaagtgccgaccagaacctgcaagacccgttcatggcgatcgaaaagcgcgcctagaagcagacccacagcggcgaccgccgctgaaaatatgggcgccagcagtaggacgccgatgaggttgcctgcgcggggatagtcctgaaaccagaacacgaaaccgaaatagaagagactggaggctgtcccaatcgccgtaagcgccagccacagacccaagcgcgcgctgcgtttcagcctagccgcgccggtttctcgacgcacggctgtgatcacgccggctcccagcaatagcgtctgctgcaagatgaaaagactgcccgccggcacggcgtaaccgccgtagccctccgtcgggttgaagagggaaacctgcttcagggtcggcgccaatctgacggcgcgggcgatatcaggcagccctttcaactgcgcctcggcgacctgcgctgttgcggcggcgacggctttgccgaccgctgtgacacgaaccagataaccgccgttcagccagatggccacgcccgtcggcacccccctcaacagatcggcctcaaaacgctgaggcaggacgacgaccccgtcgacaacgccgcgccgcatcagttcaaagccctcagcaggggatgaaatcacggcggcgacctcgatctcgcgcgaagcattcaggtcttcgacaagagtgcgcgtcagcgctgtctgcgtcggtgtcgctatggcgatgggcagtcccgtcgcggcctgtccggcataggcggccggatagtaaaaggcgtaaaggacgacggccaggatcagcaggctgctgaccggccgcgcacgcggcaggtttcggaacgtcgcggcgaaggcggcgataacgccctgttgcgggagaggaaagttcaaattctccggcttggggacaagacgcgctcgtacccggatgaaaagcgccgaaacgatcagaccgatcacggtgacgccgctcagaatcatcaagtctcgccatgccgttgctgaatccgcccccgtgaccagctgacccgtctgcagccgtagatagtgcgtatagggaaggatatcgctccagatccgggcaaagcgcggcccatggtccagcgggagagtgccgttggaaaaggcgatagccgcacccgagtagatggcggtggccgagaacgccatatccacctcgccaagcgcggcgaccagaaaagccgataagacaacgctcaccgccatcaaggcgagtatgccaaggatcagcagcgggagagaccctgccacaccccagccccggacgccgctgagccaagcgatccaggccaacccccacaggctgaagatcacgaagtgcggaatgagtcgcccgatcagagccgtcgttgtgaagccgcccgtctcggtcttgaaacgtttgaaggagccgccctgcatcagccgaccaaccgccagcaccgtggaacaagccgccagcagatgaagaacccccggcgccagaagtccgccgagaaaaagctcgaagctgagttgcggattgccgacgaccgacacctggacagcggggagttgcaaggctgtttcgggcaatcctctctgtcgcgcgcgttcttgcaactgctggccggccgctgatgcgatggccgcgctctgccccaaggccgacaaggcgccgaccgtctggaaggcgccgttgaacgacacggtcacctgttccggccgacgaaatgccccatcagaaaaatctgctggaaaatgagcgacgctgtaaatctcgcctcgccgcatcaaggccatggcctccgtcatcgtcgttggagcatgggtcacgcgaacaccggcgctcgcctccatgttgcgaattgcggcgcggctgaaggccgaatggtcctgatccaccacggcgaccggggcctgacggatcactccaggggccaacatcgccgcgataaccatcagcaggatcagcggcagaccaaaggcgacgaacgcgtcccacggtcgggtcaccaggacgcgcgcctcgtcccgaacggccgatacgaagacggccgcgaggcgtctcaccgtgcggaccaatcgaacagcacgctcatgccaggcctgagtccgttgacagggcgaacaggcttggccttgacctgaaagcttcgcacgtcatagccgctcgactgccgggttgagcgccaagtggcgaactcgccttgaggatggatggcggtgatccggaaggcgacgtcagcgaggccgagtgcgggcacgtcgccacgcacgatcgcgccgattttcagatcgcgaaactgatcctcgcgcacactgaacgtaacccacgggtcgccgatgtccacgattgtgaagactggcacgcccgtgagcacaagctcgccgacattggcgaaacgctccgcaacctcgccgtcatttggagcgagcagtcgtatctcgccttggaggctttggacctcggcgacggcggcctgcgcgcctcgcacattggcgtcggcaacagatttttcctgcggccgtgtccctgccaacgccttcagatactgctgacgggcggcttcggtctgcgaggctgtagcagcgcgggcggccacggcttcgtcacggcgttgggcggaaatcacgccttcggcgaacaggttctccgcccgccgcgcagtctggtccgccaaacgagccgtcgcctgcgcggcgcgccagacggactcgaccgactgcacatcctcgcggcgagcgccttcgcggctcatcgactgaatggcctcactcgactgaagcaaggcccgggcctgagcctcctttgctgcaacctccgggctgctcatcagagccaactcttgacctgccttcacctgatcgccctctgaagccaggaagcgctccacgcgactgggcaccttggtcgcaacagtgaaggtctccgcctcgaccatgccctgaacttgatccctggcaggacgggccgcgaggaagaggcccacgatgatgaagccgatcagcagtacgaggccgacgcccacgatcacaagcagaatacgtcgccgtgcagatgtacgactggccgcgatggtcggcgcaccgtttgtcggggcatcggcaaagggaggcgtctcgctcatggcgcgcttatccggtcttcgcgttgcagatagtcgttcaaggtcagatcgcttcccgacgccgccagcaaggcggccaggctgagatcatattcgtaagctgctgctgcgcgttgcaaacgcgcggtccccagaagattgcgggcgtccacgaccgaggcggctgtggcctcgccttcacggaacccaacctcctgaactctaagattctcgctggcggcctctaggctgctgtccatgctcagaaactgacgacgcgccaactctgcctgattatacgctcgcgtgaccagcaatcgggcgtcgtctcgggcctgtcgttccacctccgcagcagccgaggcctgagcgcgcgctgcgcccagcatgcgtcgtcgatccaccgtcgaaatcagagtgtaacgggcgccgatcccaaccgcccaatccggctcggtcggcagagcgtcgtctggattcagattgtaggttccaaatgcatagacggacggcttcattcgtgacgccgcaagatcggcgcccgcctcagccagatcgcgcccggcttgggcctgcgcaaggcgagcgttcgcctggcttgcctggtcaagaaacacgccggctggaccgactgggtcgcggtttacgaacaggggcgtggtgggaacgacggcgccattggtgtcaacgaccctggcgagggacgccacggcgttgtcgtgctccagttcggccctgttcacctgccgctgcgccgcatcgcgggcgacttcgacctgaagcgtctgggcgtggctgagcacgccttgcgattccagcagtcgagcgttgcgcaaatgcagatcgaagccgtcacgggtctcccgtgcgatcttcagtgcttcggctgccagcacctggccaaagtaagcccgcgccagattcacatcctccaaactgaccgcttcctgctgcttcgcctgcgccagatccacattggccgctgccgctcgtcgtaaggctggaattgcgccgccggtatagatcggctgaagcgccgtcaccgtggggcgaaaggtcgtatcgtcgacctgcagtcggacatcttgcggcaaggcggcgaaaatttcgggaagcgccgcttccagccgctgaccgacactctgcaacacgtcacccggcacgccgggcaagtccgcgatgagcccaggaatggcggcgccgagctcggcctgtgcgcggtccagcgtgtcgcccagcgagagatcgaatgtcttgcgataatggatcaactgagcatcgagcgctacggtcggccgatttagcccggcagccacatccgcctgggccctggcggcctgcatcccatagccggcagcgcgaccgagactggagttggagcgaatacgttgctgagcggccgcataggtcagagcgactgtagcgtcgccttgggccgcctcttggggtgcggcctgaacttgggagaccgccgcaagggcgttcggcgctgatccggccaaaatgcccacagcaacccagccgatccaagctgtacccatagcttcaccccgacgtcagcaagcataactaactcaagcgcagccgttacgtccagcaactggcgttgcgatattgacgtgatggtgtggacgacctccgcctgacgggctgttctgggtgtgtcgtcatcagggacgtcacgtctaggagcggtatcatgcagaccatcgctgtcgtcgggctcgatctggcgaagactgttttccaggttcacggtgtagccacagacggcacggtcgtcgtgagacggcaactgcggcgcggccaggtgctggccttcttccagtcgattgggccgtgcctgatcgggatcgaggcgtgcgcctcagcccaccactgggcgcgtgaactgatggcgatcggccacgatgttcggctcatgccgccggcgtacgtgaaggcctatgtgaagcgcggcaagaccgacgccgccgacgctgaagcgattgccgaggctgtcacccggccgaccatgcggttcgtggctgtgaagtcgaaggcccagcaggcggtgttgatgctgcacaagacccgggatctcctggttcgtcagcgaacgatgctgatcaacgcactgcggggccacctcggggagttcggcatcgtcgcgcctcaaggtccagctggggtgcgggcagcgctgaagagtctgcgtgaagagggtcaggccctgccggatctggcgcatgccgcgcttggcgggctggcagaacagctcgaacaccttggcgcagagatcagccgtatggagcgtcggattctcgattggcatcggcaggatgagacgagccggcgactggcgaccatcccaggcatcgggccgatcactgccagcgccatggcggccagcgcgccagatccgagtctcttccgttccggtcggcagtttgcagcctggctgggactcacgccgcgggccaatagcagtggcggcaaggaacgccagggcggcatcagcaagatgggtgacagctaccttcgacgtctcctggtcgtcggggccacggcggtcctgcgaatggcccggcagcgaggacgcgagggctgggtcggcaatctcctcgaacgcaagaagccgaaggtcgccgccgtggccttggccaataagacggctcgcatcgcctggaccctgatggcgcgacaggaggactacaagcccacagcggcatagagatcgggccggtcttcacccaggaccggcgccgtagacgaaggagtggtgagacgtgatgacgaaccggccgcagccggggatcggtgaaacccagggggtcagagcgcctcgagcgcgttgacgtgattagggagccggtccgcggacttcatcagggccagcagcgcaaacagctgcatcaacaggccgaacacatgactgcactcgaccgagcgccaacgtcgtttccactcttgcgtcttggaggtcgtccacacatgacgtccctgatgacgacacacccagaacagcccgtcaggcggaggtcgtccacaccatcacgtcagctattacccccactcgtcagactggtgcacggaatattacctttatcgagacactgaatgggagacgtcgataacgtgcaacggttcgaacattcacgggacatttgatcccagaggtcgctttcagatggcgaatgttcattccgacgtctcagacagagggcgagctagagaggggatgaaggacagtttgagcgtaagtgggggtcgctgcagtcttgcgcaaagttaccccgctcagggggggacccgggtagaggcggcgatgaacccgccgttgcccgcccctagaatcaccgtcagtctcaaggctctgcaattcaagcaaacgtaggtgttggggcatgtgttggggccccatctatgtcactgcgtttaaatgagcaaattcaaatagatacatagggaagtggcggacagagagggattcgaaccctcggtacgctttcacgtacacacgctttccaagcgtgcgcgatcgaccactccgccacctgtccgttcacgcccgtcgtgcgcgcgctggaggtcgatccagcgggaggcgggcctgatagaacacgtagggcggctgggcaagcgtcgatggcatacccatatacgcagacgccattatttcgtgagacgccccatgctgttcaagaagagcctcgagatgcccacgcgagagaccgccctgcccggccggtccgagccgctgcgcaccgatgaggtccactacgtcaacggccggccgttgaagggtccgcatccggagggctttcagacggcgatcttcggcatgggctgtttctggggcgtggagcgcatcttctggaacctgccgggcgtgtgggtgacctccgtcggctattccggcgggatcacgccgaacccgacctatgaggagacctgcaccgggcgcacgggccacaccgaggtcgtgcaggtggtgttcaatccggacgagatctcctacggcgagctgctgaaggcgttctgggagaaccacgaccccacccagggcatgcgccaaggcaacgacgtcggcaccacctaccgctccgccatctatacgctgaacgacgagcagcggcgcgaggccgaggcgtcgcgcgacgcctatcagcaggcgctgacggcggcgggacgcgacgcgatcaccaccgagatcgagtcggccggaccctattatttcgccgaggactaccaccaggggtatctggccaaaaaccccaacggctactgcggcatcggcggcacgggcgtgacctgcccgatcggcgtgggcgtggaggcctgatccaaggagccgggcggcggggttttcacgcgccgccgcccggcctaatcatcggcgtgaccgccgcccttgagtgatccgtcccatgtccgccgcccccgcgaaccaagtccatcccgacgaaatccgcagccgcttctcggcggcgctttcggccatgtaccgggcggaggtgccgcaatacggcgagctgctgacgctggtcgccgacgtcaacgccgaagtcttgcggcgcgacgacgaggcggctcggaggctggccgcatccggcgatctggcccgcctgtcggaagagcggcacggcgccatccgcgtcggcaccaccgaggagctggcgaccatcgcgcgcgccttcgccgtcatggggatgcagccggtcagctactataatctcgcgcccgccggagtgccggtgcattccacggcgttccggccagtggagcccgaggctctgcgccgcaatccctttcgggtgttctgctccttgctgcggctggagttgatcgaggatgccgtgttgcgggccgaggcggccgagacgctggcgcgccgcgacatcttcacggccggcgcgcgcgagttgatcgacgcagcggagcgtgacggcgggctggacgaggcgcaggccgaccgtttcgtcgacgaactgctggagaccttccgctggcacgcagaggcgacggtggatgcgccgacctacgcgcggctggtcggggcgcaccggctgatcgccgacgtggtcagtttcaagggaccgcacatcaaccatctgacgccgcgcaccctggacatcgatgcggcgcaagcggccatgcccgcgcgcggcatcgcgccgaaggagaccatcgaggggccgcccgcgcgcgcctgtcccatcctgctgcggcagaccagcttcaaggcgctggaggagccgatcgcctttccgtccggcgacggatcgacggccggggtccacaccgcccgcttcggagagatcgaacagcggggcgcggcgctgacgcccgccgggcgcgcgctttacgacgcggccctggcctccaagaacttctcggccctgcccgacaactggtcggcgctgcgccgacaggggctggcgtggttccggtacggcgctgatctaaaggctgcggcgacgcaggacgacgatcttgagggcctgatctccgcgggggcggtcacggccgagccgatcacctacgaggacttcctgccggtcagcgcggccggcatcttccagtcgaatctgggttccgaggcgcgcgacagcggctacgcggccgatcctgccaaggcggagttcgaacaggcgctgggccggccggtgttggacgagatggcgctgtaccaggccgaacaggacgcctccttggccgaggcgctgaacgccgttggacgcagacccgcgacggccgggatcgtctgatcccagaaggttccgcaggcgacgatcggacgccttgcgtcgcggcacggccgccatcatagaccccgcgtgaccccgcccgcctcgccctcggctcgccgctacgacctggactggatccgggtgggcgcgttcggcctgctgatcctctaccacgtgggcctggtctatgcgccctacgactggcacgtgcacagcgcccacacctttgagtggatgcgcgaggcggttctgatcaccaacccgtggcggctgacgctgctgtttctggtgtccggcgccgccctgcgtttcatgaccgcgcgccgcacgccgcgtcaggtggcgcgcgcgcggttcgagcggctggcgcccccgctcctcttcggcgcgcttctgctggtgccgatccagtcatggatcgaggccatggacaaggccggctggcccggcggcgcactcggcttcggacagtggtggacgcacgagttctcgtgggcggggctggccgacggcgttcccgtcaatcatctgtggttcgtcgtctatatcgccgtctacagcctgatcaccgtgaccctgtggcggcggccgggcgttctgccgaggctggaggactggctggagcgccatctcacggggccgcgcctgctggtcctgccgattctctatctgatcgccatccgggtgctgctgttcccgttcttcggtctgaccaacatcctgcacctggactggtacaatcacgccctgtcgctggccgcgttcgtgttcggcttcgcaagcgtgacgcgcgacggagtctggcgggagatggagcggttccgctggatcagcctgggtctggccgccgtcgccctgccgatcatgatggcgcaggtcgcccatcccggcggcggcgccttctggggcatgccgcgggcggtggtctatggcgtcgatcaatgggcggtgatcaccgccgtcctcggcttcggcagccggcatctgcggaaccgtcgcagcccggtgctgacctatctgaccgaggcgacctttccgctgtatctggcgcaccagacggtgctggtggcggcggtctggatcgtgcggccggccggcctgcctgcgggtctggaggcgctgctgctcgtgttgagcacctttatcggcagccttgtcgtctatgaggcggtcaagcgggtcggctgggcgcgtccctggtgggggctcaagccactggatggccgcccttggccgctcgacccggatgcgcccgcccagccccggacctccgcgccgtatcgccgccgccggcttctcctgtgggtcggaaccgccggaccgatcgcggccatggcgatcgtgggcgtggccgccctcgcctatcccgacttcaacaacgccacccagtacctcagcgaactgggcggggagacggcgcggaccccgatcatcttcaacgccggggtgttcctggccggcctgatggcggggatcgcgggcctgggcttcggccttgccgtgcatgcgctcaccggcgcgcgcatcgccggggtggtggtggcggtcgtcttcgtgatcgccggcgcgggactgtcgatgtccaccctgtacccctggcctgatccccggcacatggtgatcaacctgggcctgggcatccagctggcgccgttgctgctgctctggggcctgtcctcacggcgggacctgccgcggctgaagctgtttcttctgctgatcttcctggcgatgctggcgctgacggccttgaccaagcacctgctcttcgccggcctcgtcaacgacgccaacgtcggatggtgggagcgcgcctacgccatcgtgctggtcggctgggtcgcgatcgcggcctgggcgctggaacgcaagctgcgtccagagccgccgctcggcgcctcggcgctcggcctcatcgacggtgcgccctagcgatccaccacttttttggttcccatcaacatcgcgtgattgaaaatcgcgcgaatgtgatcgatgatgcgaggtgctgtgatgcagcacgccgcgccggtccgcctcccctggaccccgtcggtcaccgggagatcttgagcggcatgaacaagctggcgagccggcctgccacgcaggttgaaatcgagaacaccgacttcggtcgttgggcctggctgcctgaagaggcgcctctcgccatgccgcgccagtcgctgagcgcgcccgaagacgtcgccgacgccgttcccgccacctctccgatcaacgtcggcgcgcgccgcctgatgctgctggccggcaccgtggtcctgacgggcctcagcgccatcgcccccttctacctctacgcccgcaagggctgggattcgatggagatgctggcgttcggcatcttcatggtgctgatcaccgccatcgcctgctggttcaccagcggcctgatggggctgtgggtgctgatgcgcggccgcgaccaggccgatctggcgttcgcgcccaatccggcgacgccgcgcacgcgcaccgccctgctgatgccgctgtacaatgaggacgcccgcgcctccttcgggcgtctggccgcaatcgacgcctcgctggcgcgcctgggcgcatcgtcggcgttcgacatcttcgtcctgagcgattcgaccaaggaagaggccgcagccgccgaactgtcggcctgcatgggctttcgcctgtccgccaacagccgcgtctattatcgccgccgtctcgacaacgtcgaacgcaaggccggcaatctggccgagtgggttcgtcgcttcggcggcgcctatgagaacatggtggtgctcgacgccgacagcaccatggccggcgagaccctgctgcgcatggtcgacgccatggagcgcaaccccggcgtcggcctgatccagaccgcccccaccattatcaaggcccgcaccatcttcgcgcgcgtgtcgcagtacagcgtgcggctttacggccgcgtcgccgccgccggcctggcctactggaccggctcggagtccagctactggggccacaacgccatcatccgcacgcgcgccttcgccgcctgctgcggcctgccggtgctgccgggcaagaagccgttcggcggccatgtgctgagccacgacgtggtcgaggccgccctgatgcgccgcgccggctgggccgttcacgtcaccgcctcgctggacggctcgtgggaagaaacgccgccgtcgatcaccgacttcatccgccgtgaccaccgctggttccagggcaacctgcagcacctggggctgatcgcggccaagggcctgtcgcccatgagccgcctgcaactggccatgggctgcatggcctatctgtcctcgccgctgtggctggcctcgctgatggtcggcctgttcatccagatgttctatccggtggactggaccagcttcttctacatcctgaacccgcagctcacccccttcatgctggcgtccttgctgtcgggcgtgctgctgatcggacccaagttcatgggcgcggccctggtgatcagccgtccggccgagctgcgcgcctttggcggcaagcgcgccatcgccaagggcatggccgccgagatcgccctgtcggccatcctggctcccatcctgatggtcgccaacaccaaggcgtttctccagatcgtttcgggccacgacgccggttggacgacgcagcagcgcgactgcgatggcctgtgctggtccgacgccttccgcgccatgcgctggcagatgatcgcgggcgtgctgttctcggccgccctgtgcgtccggcccgacctggcgacctggttcgcgcccatcgtgctgccgctgctgctggcgcccgccgtcgcggtctggacgtcccgcgtgcgctcgggcgacgccgtggccgcaaagggcttcctggtcacgccggctcaggacggcgtctctgtcagcccggccgtgctgcgcaccgttcgctcgccgctgcgggcggtctcaggcggcgtctcgtctcccgccctggcgcgcaccgcctcgaactgaggcgagcgcgccacactcgtcccgcaaccgctccggttgtggctcttgactggatcaagagcttcgaacgggacattctcgacggaccgagggaacatccacatgtccaagccgaaatccgacaacgaaccccgtcccgaccttcgcctcgtggccgccgaggcggaagtctacaacctgatgcgcaagccggagagcaacgccgaacgcgtcaagcgtctgcagctcgaggcgcacgccctggcgcttgaagaggtcgtggagctcgagaagacgctgctcaaggccgccgagatggccagggccatcgccgacggcggcgacgcctatccggttggcgtgcgcgaggtcgcatcgcggatcgccggcgatctcccggtcaaggccgaaaccatccactccatcgccgcgcgcgccggctgaaccttatcggcccgatgcagaacgcaggaaagcgccccggagacgacctccgaggcgcttcttttctttccggggcttagttgaacagccccgcaatgaccgccgtgatcagcccgccggcgaccgcggcgagcaccacgtcgtttccgctgcggacatactggtagccgcggggcggtgggcgcaggccgtagcggccgtagtcgttcaccacatagccgcggctggcgtaagctgccggcagacgttggccatagctccactggcgaacctgatagccgcgcggggcgacatagcggccggcgttgtaacggcgttcggcgcgctgataccgggcgtaggcgcgagcatccgcccggtcctcgcgacgctcctggcgccgctcggcgcgctcattctggcggtgctgctggctatagccgtggcgcgactgcgcctcggcggccgaactcgcaccgacggcgctggtggcgatgacggcggcgacggcggcggtgagaatcttcttcatggcgtatctccgatgtcggaccagcccgaccttgagatcatcatgcgcccaccctgctgaggcccgtctgaacagccatcatcacctgccgttcatgcgccgaccgtccgccgtaaagcttgaggtgccttgccgaagacaggataatggatcggccccgcgactctccgcaaggacaccctcatgcccctccgcttcgacaaccgcgtggccatcgtgaccggcgcgggcggcggcctgggccgggagcatgctttggcgctggcggcgcgaggggccaaggtcgtggtgaacgatctgggcggcgcccgcgatggctcgggcggatcctccagcgcggccgaggcggtggtcgccgagatcaaggcggcgggcggcgaggcgctcgccaacggcgcctccgtcaccgaagcggacgcggtgcaggccatgatcgatcaggcccttgatcgctggggccgcatcgacattctggtgaacaacgccggcgtgctgcgcgacaagagcttcgccaagatgacgctggaggacttccgcttcgtggtggacgtccacctgatgggggcggtcaactgcaccaaggcggtgtgggagagcatgcgcgagcggaactatggccgcatcgtcatgacgacctcctcgtccggcctttacggcaacttcggtcagtcgaactacggcgcggcgaagatggcgctcgtcggcctcatgcagacgctggcgatcgagggcgccaagaacgacatccgggtcaactgccttgcgcccaccgcccacacccgcatgaccgaagacctcggcgcgggccttccgctggaggcgctggataccgccctggtgacccccggcctgctgcacctcgttggcgaagacgcgccgagccgctgcatcctggcggccggcgcgggtgggttcgagcgcgcctatgtcaccttgacccaaggcgtccatatcgtcgggccggacgcgcccgaacaggtcggcgcgcgcttcgatgcgatttcagaccgcaccggcgagatcgtccctgaagcgggggcggcgcaggccatgcttgaactgaccaaggcccaacgcagcctctaggcgggtcggctgaggggtcgcccctagccgatcaaccgcgccgccgccgcccgcgcctcgtcggtgatctcggcgcccgacagcatgcgcgcgatctcctctcgccggcgcgtctcatcgagcgcgacgaccgtggtcgtggtcaggccggccttgtcagccttcatcaccttccagtgggcatggccgcgcgccgccacctgcgggctgtgggtcacgaccagcacctgcgcgccggcggacaggcgctgcaggcggccgcccacggcttcagccaccgcgccgcccacgccctgatccacctcgtcaaagatcatcaccggctggcgggtgtcctcgcggctggccagcgccgccttcatcgccaacgcgaagcgcgccagttcgccgcctgacgccaccgcatccagaggtccgaagtcgcgcccggcgttggtcgcgatctgaaagcgcgcggtctccacgccttccgggccgcgccggccgtctatggcctccagagccacgcgaaagcgcgcccgctccagcttcagcggtcccagctcgcccatcaccgccgccgtcaaacgctccgccgccgcctcgcgcgcggaagtcagaaaggtcgcagccaggtcataggcctcgatcgccgccgccgcctcccgacccgccgccgaaagcgcctcctcgccgtcctcgatcagccgcaactgctcgcgcagacggatacgcagggcgggcaggccgtccaccgtcgtatgcagcttgcgggcggccgcgcgcagggcgaacagccgctcttcggccttgtccagccgccccggttcaaagtcgaaggcgtcggccgcggcatccaccgcagcgatggcctcggccgcctcaaccatggtccggtcgatggcctcgaccgccgcgctcagccgcaagatcaccgggtggtcgccctcggcgcccgcctgccccgccctctggcgcgcatgctcgacggcgcgcagagccgaccccagcttctggctcagcttgtcgccgcccagctggatgcgcgcgtcggcgaggtccgacagcgccttttccgccgcccctaggatggcgcgttcgccggccaattcggtttcttcgtcctcgcggggatcgagcgcatccagctcggcgaggttcagcgcgatctcctcggcgcgagacgccgcatcggccgcctgcgccttcagctccgccagccgcgcctcggccgccttcaaggtcgccgccgccctggcgacggccagcaactgcggcgacagtcccccataggcgtcgagaagacccctatgggtgcgccagtcgagcaggccgaccgtctcgtgctgcccgtgcacctctacgaggtttgcgccgatctcgcgcagcgcggtcacgcccgccggctgatcgttgatgaaggcccggctgcggccgtcggccgagaccacgcggcgcaggatcaggtcctcgcccgccgcgacctcgatacccttgtcggccagcgactgcagcagcgtctcgtcagccggggcggagaagacggcggtggccgatccctgcctggcccctgcccgcaccagtcccgcatcgccccgcgctcctagcgccaggcccagggcgtccaggatgatcgacttgcccgcccccgtctcgcccgtcagcaccgtcagcccgccctccacctcgagatcaaggctgtcgacgagcacgatgtcgcgtatggaaagcgcagtcagcattcaggagcgcggaaaactcgtcgttcgggcggcggtcgcatcatgccgcgccgtgacggcccggcacaagcaccgcggaacaaaaagaaaaccgtcagcccggaatgatgcgctccagccagctttcgcgacggccttcgggggcgacgtcggggcgtgcgccctcgttcgtcagcagggcgtaggcctcggcgtaccaggggctgcctggatagttgtagccgagcaccgagccgttgcgcaccgcctcgtccttgaggcccagcatcagattgacctcgaccaggcgatacagcgcctcgggcgagtgcgaagtgcgctggaagtccggattggcgatcacggccttgtagcggttgatggccgccaggggctggctggcgcgctggtagtagcggccgatgttcatttccttgccggccagctggtcgttgaccatgtcgatcttgacggaggcgtcggtggcgtaggccgtgcccggatagcggcgctgcacgtcgcgcaggcccgccagagccgcttccgcataggcctggtcgcggcccacatcgacgatctgctcgaagttgcagatggcgcgcatgtagaaggcgtaggccgccgacggattgccggggaacagctggatgaagcgatccgccgccgccgtcgcctccgcgtagttggcgttctgataataggcgtagatctgcatcaggatcgcgcggcgcgcccagtccgaatacgggtgctgacgctcgacttcctggaaatagtccaccgcgtcggaccagcggcggctctgcagccggtcatagccggtgttgtacagtagctcgaccggccgctcctcataggccaggcgtgggcggttgcggtttccggcgcaggccgagaccgacagggcggcgagcactgcagccatcgccaccacgccggagcgagaacggcggatgcccgaaagcgaaaaggaagcggacaaggacagacctcatgacgaacgaacgccgtccccgacggcgcccggcaagcgattgcggcgatccctagcacccgtggccgaaacgcgccatgcgccggaaacttgggcgtatggcttgttccccgccgcgtcgctgctaaagagccgccgaccaacgccgtcattggcttggtgatgacggcgaaaggatgaccggccatgaagctgctttccggcaactcgaacaggcccctttcgcaggcgatcgccgaccatctggacgcgccgctgacgcgcacccaggtcaagcgtttcgccgacaacgaggtcttcgccgtgatcgaggaaaacgtccggggcgaggacgttttcgtgatccagtcgacctcctatccggccaacgacaacctgatggagatgctgatcatcaccgacgcgctggtgcgcgcctcggcccggcggatcacggcggtgatgccctacttcggctatgcgcgtcaggaccggaagaccggcggccgcacgccgatttcggccaagctcgtggccaatctgatcacccgcgccggcgccgatcgcgtgctgacgatggatctgcacgcgggtcagattcagggcttcttcgacattccgaccgacaatctcgtcgccattcccgtcttggcccaggacatcaaggaacactatccgcgggggaacgacctgatgatcgtgtcgccggacgtgggaggggtggtgcgcgcgcgcgccttggccagccggctggacgccgacctggccatcgtcgacaagcgccggccgaaggcgggcgagagcgaggtcatgaacatcatcggcgacgtgtccggccgccgctgcatcctgttcgacgacattgtcgattccggcggcaccctggtgaacgcggccaaggcgctgatcgacgagggcgcgaccgaggtctcggcctacatcagccacggggttctgtccgggccggccgtccagcgcgtcaccgacggcccgctgaaggagctggtcatcaccgactccatcgagcagccccacgaagttttgacctgcggaaaaatccgaacggtttcagtcgctcctctcatcggtgaagctatccgccggatcgcaaacgaggaatcggtgtcgaagctgttcgattaaccttcgaaaaaccatttacgtcgcgttataagcccttcagttccggcggccacgcccccttggccgtctcgcgttcttccgggattatgcgttcatgaccaaggcttcccccggccgcggcctgtctctcgccgccatcgccgtcgctgttttcctggccaactgcgccaagcccgagccggaggcgccgcccgccgcgccgccgcctccgccgcccgtcagcctgaacgaaggcgtggcccaggccgcctccgtctacgtcgccttcctgcgcgacgcccagaccatccagcccggcggcttcaccgacgccgagtcgatccaggcggccatccgcaagggcgcggcctatgagccggcgcaactttcgcgcggcctgatcgcctatggttcgatcatcgccctgcagtcgcccgagttcgtcgcgggagtgcgccagttcgcggtcgatccggtccagcgccagcaggtggtggcccagatcgtggccgaccccgcctatgccgcgacgctgcctggggccgccgccgccgccggcctgatcgctgcaaccgtcggccgcgacgcctcggccatggtggtcatcgccgatggcatcgagaacgacgcctacaccatccaggaacgcaacgacccgcgtcgccgctgggccaccacccacctgaccgaacgcgaagcgcgcctggaggccgccaagtccgcctccatcgcgcagatgctgccgtccgccgacgagtccgcccgcctgttcacggcggccaatgcgggcacgggtctggccgtcgaagcgggcgtcagcagcccgccctacacccccgccgtggtgcgctctctggccatcgccgccctggccgccctgggggccgcgggcgacgaggcgcgcgccaacaccgatgcgctgacggtggagtcgaacaacgagttctgcctgaacatgtccaagctgatgctttatcagtgcctggccgcctcgcgcccgagctacgaggacatgttctgcctgggtcgccacatcacccgcgacttggccagctgcaccacccaggccctgcgcccgccgccgatcatcagcgtcggcgacccggtgaccaccagcacggtggccaacgccgttccggttcagacgccggttcagacgcccgccgcgtcgaactgatcgcggcgacaaagaccaaggcccgctcgatcgttcgagcgggcccgtttttttatggtcgggctattcgtagccgtgcgctgcctcgttgatgaccagcggcggcatctcggagaagtcgaccgccaccggctggctggccttggcctgcagcgtgcggatcacgtgggtcatgcggcgccggacctcgcgctctgacgatgttccgtcatccagcgacagcggcgccaggcagaagtcgatgatggcgtcggtttgcgtcagcggttccatgggttgctccttgttcggcccgatcaggccgcgtgcgtgaactgggcggtttcggtcgagtccttgagcgccgtggtagacgactggccgttggagatgaccgtcgccacctggtcgaagtagccggtccccacctcgcgctgatgccgggtggcggtgtagccctgggcctcgttgtcgaactcgcgctgctgcagctcggaataggccgccatgccgcggtcgcgatagccgctcgccagctcgaacatgccgttgttcaggctgtggaagcccgccagcgtgacgaactggaacttgtatcccatggcccccagctcgcgctggaatttggcgatggtcgcgtcgtccagcttggccttccagttgaaggacggcgaacagttgtaggccatcagcttgcccggatgcgccttttggatcgcctcggcgaagcgcttcgcatcctccagatcaggatgcgacgtctcccaccacaacagatcggcataacgcgcataggccaggccgcgcgcgatgcagtgatccaaacccgtgcccgccttcagtcgataaaagccctctggcgtgcggttctcgcggtcgatgaacggatgatcccgttcgtcgatgtcggaggtgatcagctgcgcgctttcggcgtccgtgcgggccaccgtcagcgtcggcgtgccacagacatcggccgccaggcgcgcggcgatcagattgcgctcatgcgcctgggtcgggatcagcaccttgccgccgagatggccgcacttcttctcggacgccagctggtcctcgaagtgcacgcccgcggctccggcctcgataaaggccttcataatctcgaagctgttcagagggccgccgaagcccgcctccgcgtcggcgacgatgggggcgaaccagtcgcgtttggcgccgccctccgcatgctcgatctggtcggcgcgctgcagggtgcggttgatgcgtcggcacagctcgggggcggcgttggccgggtacagcgactgatccggatacatggcgccggccgtgttggcgtcggccgccacctgccagcccgacagatatatggccttcagccccgcccgcaccatctgcatggcctggtttccggtaacggcgcccagggcattgatgaacggctccgtgtgcagcagctcccacagacggtttgcgccgcgctccgccaacgtatgggtgaccggaaccgagccgcgcagacggagcacgtcctcgggcgcatacggcctctcgattccatcgaagcggcccgccggcgaaggcacgagatcggcgaaggtggtcatgttggtctcctggcaagggcggcgcgccgccgcctcaccccaagagaacacgcagcagtcacaaccgatacacctgcggacggcgatcacaggtcatcttgtaccatcgtgacttccacgttttgtcatgatgtgacatcctgcgcatatggacttgacgcccgaccgcaagctgttcctcggcgcacgtttgcgccggctaaggcgcgacctgggcctgacccagacagccatggcgggggacctgcgcgtctcgcccagctatctcaaccacatcgagcgcaatcagcggccggtttcggcgcaactgctgctgcgcctggccgaaacctatgacgtcgacctgcgggcgctgaaccaggcggacggcgcgggcgaagcccaggtgacggagatcctgaccgatccggtctttgcgggtctgtccatcccgcgccacgagttgctgcagctgacggaagaggcgcccacggccgctcaggccttgttgaggctctatcgcgcctttgacgagcgccgagcaagagagcggctggctctggaggcgggcggcgtcgcggacatcggcgcgagccccgccgactgggttcgggatttcgtgcagaaccgccgcaacgcttttttggaactggacgccatgggcgaagcgctggcccacgccttggtgcaggatgcgcctgcgcacgctgacggcttcgagcccgccgctcgcctgcgtctggccgcccgccacgacctggccgtccgcaccctgccggccgaggtgatggtcgagtggacgcgccggttcgatccgcatcgtcgccaactgctgctgtcggaaaccctggggcccgcctcgcgcgccttcgccctcgcctatcagctggccctggccgagcacggcgccgatctcgatcgcatggtcgaggccgccgccccgccggacgtccccacccgctcgctgctcaaggtgtcgctgaccaacaccctggcggcggccatgctgatgccctacgcggcctttcatcgcctggcggaagagacgggctatgacctggcgcggctccaggcgcggttcggcgtcagctatgaacaggcggcgcatcgactgaccaccctgtcgcgcccgtccgcacggggcgtgccctttttcctgatgcgcgtggatcaggcgggcaacatctccaaacgctttgcggccgacgcctttcccttttcgcggttcggcggcgcctgcccgcgctggcggctgcacggcgcctttcgcacgcccggtcggatcgtcacgcagatcatcgagacgcctgaacaggacggaaagcgcgccgcgcgctggttcaccttcgcccgcaccgtcgatcgtcagggccaggacggccttggccagcctcaggacctcgccatcggcctgggatgcgagttgcggcacgcccatcgcctcgcctatgcgcgcggcgtcgatctggcggcgccggaggtcacgcccatcggcccggcctgccgcctgtgccatcgacacccatgcgccgaacgcgccgccccgccggtggaccggcctctggccgtggatgactgggccaagtccatcagcccctacccgttcgcccgcgcctgatcctgtgctagggtcgggccatggccgacggcgccctgaccttgatcctggatgacgcccccgtcgcccgcctcgccgaggcggcggccctcgccggccagacgcccgaggcctacgccgccgaccgcttggccgaaaccctctctccgcctctcgcctacgactggaccgaggcgaacgagcgcctggccgagtacgaccgcaccggcgagtatgtgacgctggaggatgccctggcgagcttccatgatgaggtggaggccgcgctggccgctcgtcggtgatctactcggtccggcttgcccccgccgccgaggcggacctgctccgcctggcgcgctttcttgccgatgtggacgaatcggctgcgaggcgggggcgcgatcggatcgcagatggcctacggtctttggctttcatgccgggccggctgaggccggaggcgagcggcctcagggaactttacatccgcttcggcgacagcggctatgtcgtccagcatcggatggacgccgacgccgtgatcgtcgcccgcatcttccacatgcgcgaggcgcgctgaggcttcgtcagaccagcaccacccgccccgcctccatgcgaaagccgacgcctgtgcgttcgaacaggcgggcgatcaccgccgccggatcggccgcgccctcatccagcagccgttcgacatccaaacgcagcgaggggtcgcgcgagacctccgtcagtgcgtccaaccattcttcacggctgaggacaccgtcccggcgattgtcgtcgatcaggggcttgaggaagtcgagccagtcgccgccggtgacctgtctctgcgcgccctcggccgccatggcgaacacggcgccgcaggcgtagaaggcgcgctgctcgcccctttgcgccgccgtggtcacggatcgcccacgcgccagttcggcgcagtcgtcaacttccttctgcaaggcggcccgatcatcgtaggccgggtcaagcgtcttcagcgcccgcaccgccatcaggtcggcccctccctcggtgatccaggcgtcgcgcgcatattcataacgcaccgtctgccccaaccagaaatgcgcgctctcatggccgatgaaccagcgcgagaccgtcagcatctcggaggtggggttcagcacgcccgcgccctcgaagctcatggtgatcaggcccggcatgacgctgccgcccatgctggtcatctgctcggtcgggccgttccagctgatcatcaccgtggggcgatccgtctgtccaggccccagccggcgcgtgtaccactgcccgacacgcggggcgaagccgcccacctgttcgccgatccagggcggaagcgccgggtccatgatggtggtcagccgctcgccctcgacctgctccacctgcccgaacaagacatagccgttgccgtcatcggtgacggcgcgctccagccgctcgccgcccagcagtacgggaccggccgcgtcgcgccatgtcaccacgggcgcggacccgacctcgacgccgttcagatcctcggggatcgcggccagcgccgcctcggaggcgacggggaagatgtcgaactgacgcgtcggcagggccacggcgccggtggtgaacaccagggtctcgtagccgccctcgatctgggcgtgagcgggcgtgaagccgatccggacttcgcgcggcgccggcccgccatccgtcgaacgcagcacgtcgaaggcgccccaccgctccagcaccacgcccggcgtttcaacccgccactgcttcaaccgccagggaagccgcacctcctggatcagctcggaacgggaaaaggcccagatcggcgcatcctgaccgaagcggtagtccgccgtccagcgatcgccgtcacgcgtcacctcgacggtggtccgaccctgtgcgaacacacggctcgagccgccgccgtcgggcgtgtaagcgcagccggcgaggcctgtgccggctgcgacgccggcggctagagccatggcgcgcgcggcgtcacgaagcttcatgagtgtccgtctcttctctgatccacaaacaacgagccgctcagcctgccgcgtgcagagcgcgaccggcggcggccagttcttcggccatcacggtcttcaacctttgcggctgcaggatgacagcctgctcgccccaggtgaacaggtgccaggccagttcgcgcatgcccgacgcccggaaacgcaccaccaccccaccgttcggctgatcctcgaacgtctgggtcgggtgccagcgccagccccgcgcctcatccgcgccggcgggcgtgatgcggacggccacatcctcgatctcgtcctggtagatgccgaaggactggctggcgaagacgccgaggtcgaagtcgggcggcgggatcgccacgccctcctgcgccgccacatggctcatccggtcgaggcgaaaggtctggatgcgtccgctctcccgatccgccgccaccaggtagttcgcccgcccgaacatcaccccgcagggcgtgaccgagcgccgcctcggctccgcgcctggccgtgcataggtgaagcccagcggctgttgcgccagcaccgccccccggatggaggtcagcatgggctcgtcggcgtgcgcgcgaggaccggcctgcaccgcgatggtctcggcccgcaccagcgcctccaggtccggcgccatacggttcagggtggtcgagcgcatggccgccttcagcttgcgctccagcccctccagcgcctgtgcccgcacctcttctccctgcgcgcgcagggtctgcgcggcctttgtcagctccagcatctcggtcgcggtcggggcctgctcgaacgccgacaggccgccgcggatgcgccagcgcttggtaggcgggtccgacacctcctccaccgtggggaaaagcatcagcacggcgtcgcgcatccgctcggcggtgcggcggcccacacgcatctcggacgccatctcgtccagcgtcagcccctcggcgctggccgccatgcgccgcgccagctcgatcaccatggccgccttgtcgtgcctcacgccacacccttcctcatacgtccgtttctggcgcaatgctgctgtattgtcccaacatcagcaagaggcaatcgcttcaaggagagagacttcgatgggacaggccttccaccccgcagccgccgtgaacgccagccgctacatcatcgtgccgtgcgaggccgacagcggatcggacctggcggtcatctgggaccggctggaggagcaggtggttgacgtcatctccgccgccgccagcgcccgctactccgaggaggacgcgctgtgggacgaggcgcacgcgcctgtgcacgccgacgactggcgcatggcggcctgatcagaccgcgagttcgggccgcgcgacggcgtcgggctttcggctcagacgtccgttgatccagtcgcgccccggcgtctcgatccagcggtatgtcagggccgacaggccgacgatgaaggcgatcaccgctagcgagaacaggtcgttcagccagaccgagcccaggtccacccgcctgccgttcggcatcagctgcagattgcgcgcggcgatcagcatgaccgtgatcaccagcatgtgcgtcatgtagatcgaataggaccaatggccgaggcgaatcatcggccgggccgccagcgcgcgcgagaccgctccaccctcgctggcgaacacccagatgctgagggcgaacagcagcggcgccagcacctcccacggcccgcgcgccagcgacacaaaggcgaccaccgtgaccaggctgatcggctccatccatcccgtcacacgcggcgacagatccggccccgcgctccatagccgatgcacgaggcatcccaggaagaagccataggcggcgcgtggaaacccgaagctgtaggtggtgttcatgaagcgcggtgcgaagttcaacaccaccagcgcgcccgttacggcgatcagcagcgcccatgtgttgaagcgccgcggcgcccaaagcagcagcgcgccgaagacgacatagcagcccatctccacgctgatgctccacgccggcccgttccacgtcaaatacggatggatgccgtaggcctggatcagcagcagattggtcagcagatattccggcgcccggtcacgcgcaaaggccgtgatgtcgtcgaagtggaaccacagccggcagaactccagcaccacaaaaccgcccagcaccgcgacgtgcagcggccagacccgcccgacccggcgcaccaggaagcggcccacgtctcgccccgagccgagccgagcgccataggcgtgggcgatgacgaagcccgacagcacaaaaaagaaatccacgaacaggtagccgtgccgcgtcagggccagcgcatgcaggtggctcgacaccggcaggtgaaacagcaccaccaggagcgcgcacacgccccgcaggctgtccagcacctcgaaccgcgtcgtcttggaaatcatcgcgacggcatagcgccaagcggcgccgtcgcctagcgtaggccgatctgcgcgtcagaacacgtcgacgaaggcggccttggccgggtcgttggtgccgtcggccgtggcctgtccgttcttgaccacggcgatgccgacggggccctggccgccggtcttcttcagggtgcagcgggcgttgtcggtcggcaggcgaccgcgcatggggcctgagcccgtgtgggtgctctggttggtcagggcgccctgcaccgtcaccggccggaagcggcagtccagcgaccagccggcgccctgcggtgcggccacgctccagtgcaggccgccttgcggatcgaccccgcgcaacccttgcgccatcgcggcgggcgcgatggcggacgccacggcggcgatgaggaacagcgacttcataagcaactccggatcaggcgcccgtgcgggcgagccgccacagggcggcggcgatgaacagggggccgagcagcagcatgacccaatcaaacacgccaaaggctcggtcctgagtgatcacgcgcaccagtatgcccgcgaaaaccatcaccacgccgcagtcccgcagacgcatctgcttgacgggcgtccggcccagaaaccagctccacagccacaggccgaaccccagccccgtcgcgatccaagaggcgaaaaccgccagccggaccggatcggcgagcgtctcggccgtcagagcgcgtgctccggcttggtcctgagagcgatgatccccgccacgaccagcacggcggtgcagatcacggccgcgatcaggttgccgcccgggtggaaccacagcgtcaggaacaacaccagcgcggccacgcccagcgaaccccacttggtcaggttcatgaacaggccataggtggcgtgctgttcgttcagcggcatggagccatgcacataggcctgcgcgtccgcatcggcgtgaacggtggcgttctccacgaagttcgcttcgccatcggtgacgacgggagtgtgcgggtcggccatgtcgcggttccgttgagggatcgtgcccgcgactatagcgagcctcgccgtgggctcaagccgcagcggcggctatgacaggtcctcgaactggtcgatcagccgctccagccgattgcatcccacgctccagaaggccggatctcgcgggttcaggccgaatggcttcagcgcatccacataggtacgcgtcccgccggcggccagaaggttgcgatatagcggcgtgaacccggccggatcagcccgcctcgcctccatcagcgccgccaccagaagatcgccgaaggcgtaggcgtagacatagaagggcgagtggaagaagtggctgacgtagctccaccacgtctcgtagccggggttcagcgtcaccgccggtcctagcgaggcgcccatctcctccaaccacagggtgttcatgcggtccggcgacacctcgccggccgagcgctcgtcgtggaagcgcgtctcgaagcggtgaaaggcgatctggcgcacaaccgtgttcagcccgtcctcgatccggccggccagcagcccgcgctgctcgctctccggcgcctcggccagcagacggtcgaacgtcaggccttcggcgaagatggaggcggtttcggccagggtcagcggcgtgtcggccagaagcgtcccctgctcggccgccagggtgttgtgcaccgcatggcccagttcatgcgcaagggtcagaacatcccgccgctcgcccatccagttcatgaacacataggggtggcgggtggcggtcaccgggtggcagtaggcgcccgactgcttgcccggccgcgcctgggcgtcgatccacggccggtcgaagaaccgggccgcacgatcggcgaagtctccgcccagggcgccgaagctgtccagcacgatccggcggccctcccgccaatcgaacacgcgcggcggcgtgccctcgatcggcgcattgcggtcccagtggtccagcgtggccttacccatcgccttggcctttagcgcatagtagcggtgcgacaggcgcggataggcggcggccaccgcctcggccatggcgtccaccgcctcgccgtcgacctcattggccaggtggcggctgtcggccgggcgtttgaagccgcgccggcgatcctccatggctttgtcggcggcgatggtgttcagcaccaacgacatcgtcgaggcgcgctcggcgaaggcttccgacagaccctccgccgccgctcggcgccgctcggccgccggattcgacaagcggttcaacgcttcggccagtgtcagcgtctcgtcgccggccttggcccgaagggccgccatctgctcgtcgaacaggcgcggccactgcgccgtgatcggaccacgctcggcgatgaaggtctccagctcggccgacagctcgtgcggcttggtcgcccgcacccgcctaagccaaggccgccagcgcgccgccgccggatgcgccgccagcgccgcctcgatctcggcctcctccagcgcgttgatctccagcgtcagccacaccgtcggggtggcgatggcggtgatcttctcgcgcaggtccgcctcgaacccctgcgccgccgcatcgtcgcgctgggtcgaggccgacaggaaggcgaaggcgccgagcgcgccgaggtgatccgacgcctgttcgtacaagcttacggcctggtccagccgccgacccaacagcgccgcatcatcgcgcgcggcgacgagctgttcctgaagggcgttcagccgcgccaccaccgtccgcgcctgctccaggtcggaggcgacgccctcatcctcgcgcgaggcgtagaggtcggacaggtcccaaaagggggcgtcggcggtcggggctttgaagggcgcgttcatgcccctgttgtggggttctgctcggccggccgcaaccgggttaaccctccgctcacccaaccgcacaacgcgatcttcacgccgttccgcctagaaccgtcccgaaacgggtcaatgcaccgacccgccaaaaaggcgtttctctccatggccaagaccgttctggtggtcgatgacgatccaacccagcgccgcctgatccaggccgtcctgaaccgtgaaggctacgccgtcgtccatgcaaccggcggcggcgaagcgatcgacaggctcctgcgcggcggcggcgcggacgtcatcctgctggacatggtcatgccggagatgtcgggcatggagtgcctgaccgagctgcgagcggcgggcgtcgccacccccgtgatcatgctgaccgccaacggcggggtcgaggcggtggtcaaggccatgcaggccggcgcccaggacttcttcgtcaagccggtcagtcccgagcgtttgctcatcggcgtgcgcaacgcccttcagctgacgcagctgtcggccgagggcgggcggctgacaaagcgcgcgcagggccgcgccagcttcgacgacatcgtgggcgacagcgcccccatgcggatggtcaaggcgctgggcgcccgcgccgccaagtcctccattcccgtcctgatcaccggcgaaagcggcgtcggcaaggaggtcatcgcccgcgccctgcacggcgcgtcagaccgcgccggcaagccgttcgtggcggtgaactgcggcgccctgcccgccaatctggccgagtccatcctgttcgggcacgaaaagggcgccttcaccggcgcggtggagaagacgctgggcaagttccgcgaggcggatggcggcaccctgttcctggacgagatcggcgagctgccgcttgacctgcaggtcaagctgctgcgcgcgctgcaggaaggcgagatcgatccggtgggcggcaagcggccggtccgcatagacgtccgcatcgtctcggccaccaaccgcgatccggagcagcaggtgcgcgacggcgccttccgtgaggacctgttctatcggctgaacgtgtttccgatcgaggcgccgtcgctgcgtcagcggcgcgaggacattcccgccctggtcgactgcttcatcgcccgcttcaacgccgaggaaggcaagcgcgtcgccggctgcgcgcccgagacgctggcgatgcttcaggcgttcgactggcccggcaatgtgcgccagctggagaacgcggtgttccgcgccatcgtgctggccgatgcgcccttcttgcagccgcatgatttcccggcgatttcgggcgtcgccgcccccgtcgaggccgcgcccgctccgtccgctccatcatccctgatcgacctgccgcccttgccggatcagccgatccgcatcctcgacgagcgcggccacctgcgcacgctggaggacatcgagcacgacctgatccagcacgccatcgccgtctacgccggccacatgagcgagatcgcccgccgcctcggcattggccgctccaccctctaccgcaaggttcgcgaacaggggctggaagggcagttgaaggaggcggggtgatcaggcgtcaagactcctcaagaacgcctccacgcttccctccccgtcatcctcgggcttgacccgaggatcaggcgcccagccgcacagactggggaacaggtccacccattccggattgctgcgctcgatcatctcgagcttccacacgcggttccaccgcttcagcgccttctcgcgccggatcgcctccatgatcctccctcggtttggtggacacccatgctagcttttcggagctggagaggagtgtctgatgagtgttcaacgccggaactttccggattctttcaagcgcgaggccgttgaccgcgtcgccaacggcggcctgagcgtcggggcggtggcccgcgagcttgggctgcacgagacggtgcttcgtcgatggatgacgcagttcggggtgcaggcgacgggggcgtcgcggcgccccacaacgcaggcgtcgtccccgtcgccgtcggatctggcggcggaggtggcccggttgcggcgagagaacggtcagctgcggatggagcgggacatcctaaaaaaagccgcgctcatcttcggagcggcctcccgatgaagttcgggttcgtcgatgagcatcgtcaggtctggccggttcgcgtgatgtgcgcggtcctgggcttgtcggccagcggttactacgcctggcgcggtcgccccgagagccagcggtctgtcgccaatcgcgagctgaccgaggatatccggctgatccatgcggagagcagcggctgttacggctcgccgcgcgttcacgccaccctgcggcggcatgggcgtcgggtcggtcgatcccgcgtggagcggctgatgcgccgcgccggcctgcggggcttggcggccttgccgcgtcgcgcccggacgacgaacagccgccacggttatcccatcgcgcccaacaggctggcccggaacttcgaggcggcggcgcccaaccaggtctggctcgccgacctcacctacatcccgaccggcgaaggctggctctatctcgccgccatcctcgacctgcacacccgcaagatcgtgggctggtccatgcgccagaccctgcacaccgagatcgccctcgacgccctcaacatggtcgtcgaacgtcagcgccccgcgcccggcctgatccatcattcggaccggggcatccaatacgcagccgaagcctatcgatcagccctggcccgatccggcatcaccccgtcgatgagccgaaagggcgactgctgggacaatgccccgatggagagcttcttccacaccctcaagaccgaacgcgttcatcaccgcctctacgccacccgagaccaggcgcggcgagacctgttcggatacatcgagggcttctacaatccccatcgcctgcactcagcactgggctatatcagccccgctgaggccgagcgcaaagcggcttaaccccgtccacttttacgggggaagatcagaggtggtttcgaagtcccgcgacggcaggttgggcgttgcgtggtcggtcacggcgagctccgaatgcggcgatgccgctgaagcctagccgcaacagcccttcccatccacctggatcggaggacacggcacgtcggcataggagcagaatacgcagcagtcgcccggcaacggcttcagcttcacgccgcacccgaggcaatcgtaaaaccagatgcaagcgtcggtgggcatggtctccgtcgcgacatgactgcaatgcgggcaggtcagcgtcgactccagaacgaaggcggccgtcatcgcatcgccgccagtcggggcatggcccagggctcgatgtagggctgccacgccagggacaggacgatcagcacgctggcggtcaccagcagccagaacgccaggcgcgaagggcgccggcatgcgccatccttcttgcacatgcgcagacgacgccaatggagcaaccagccggcggcgaggatgacggcggccaggagcgtcagccagtttctcgcgccagcgatgacggcggccccggcgaaggatacgcccgccaccgacagagcgaggggcagcacgcagcaggcggcccaggcgaacaccgaggcggcggcgccgatggccgccgaggcgctgacggcgacctcaggatctctcggtcggtgttgatcgatggccatggagcctcccgttcgatttctgctagaggctacaacccgtagccactacgggatcaagagccatgtccacacgaagtttgacgatcgggcgtctcgcggccagcgcgggagtgaacttggaaacggtgcgctattacgagcggatcggcctgatgccagccccggcccggaccgacggcggccacaggagctacgagccggaacacgcccaacgcctgcgcttcatccgtcggtcacgcgagctgggcttcggcatcgacgccattcggcggctgatcgcgctcagcgagcccggcgtgcaggcgtgttgccaagttcgcgacatggcccaggaccacctcgccagcgtggacgccaagatcgcggacctcgaacggctgcgattggtgcttaagcaggccgtcgcagactgcagtgagggcggccgagtccggtgtccggtgatcgaagaactgggctcgatcgcatagatgcgggccggagcgccccggggagcggacaggctcacgccagatcaagcgccgataaagcccaggtgctcaagcaggatagtcaggccgagcgcgacgagggcaaggccgccgatcagttcggccattttgccgaagcgctggccgaccgcccgaccgatcagcatgccgacagtggtcagcaaaaaggtcgtgacgccgatagaagcggcgatgacccagatattggctccaatgaaggcaaggccgacgccgacggcggcagcgtcgatactggtcccgacagccgtggcgatcagcccccacggtccggaccggcggggcgcctcgcccgcttcctccgaccgcggacgggtcgcttcccagatcatcttgccgccgacagcggccagcaagccgaacgcgatccagtggtcgatcctttcgacgaggccagcggcgaccatgccaagcgcccagccgatcaagggcgtgatggcctcgatgacgccgaacaccagtcccgccttgaccgcgcctggcagggtcggtcgatgcgaagcgccacggccgaccgctgccgcgaacgcgtcaatggacatgctgagggacaggacggcgatggcgacgggagtcatgacgggcatccaccgggcaacgaacagcgcctcccttcccggccggtgcggcggtgggacgcgctggtctcgctaggcggcggttccgctggccggaccacgcgccaagcgcgagtgtgttgacccggccccgacgatgaatcgccggaagctactccccaacaggaagcggccttctagccggcgttgcgtacagaggtccatcgacaagacgacgcatcatgatcgtgcgcttgttgagatcaccggcccgggcgagggtgcttgggcgacggacatcgtccagcacgtgtcgggccaagccttggcgacgacgttcgcctcagtggcgcgaaggcgtgatcgaggcctcggccgcccggcaggcgccttcgcagcggcggcattcatcggcgcagatgcggcaatgctcatgcatctccgcgtgcttctcgcattcgacagcgcaatcggtgcaaatctcggcgcaggtttcgagcatgcgtttgatcaaggcctcgttgctgccggcgcgccgcgcggcgaggcctgccgtggccaagcagacatccgcgcagtcgagatcgaggcggatgcactgggtcagatccctcaccatctcctcggcgaggcaggcgtcggcgcagatgcggcacacggcggcgcagccgtaggccgcctcgatcgcgcgaacaaggctgtcattgacgctgccgcgcacgtccggatgggtgctgatcatcggttggatttgcatcaggggctccttggctgatcggaatcaaacccgggcgttgaactgatgttccgaacggtggagcctgggaggcttcgcgtttgcgtccgtcgcctacagccctccagccggcagccagaccgcgccctcgggggcgagcgacgcccagccgccgggcgtcgggagaccggctgccgtagccaacccggtcgaggctttcttggcgcggacagccgaacggcagcgcggtcgggagaacgccttcgccagacgcggactttccggcagggacgggcagtttcgcgcgctgctcgcctcgtcacgcataagtccgcctgggctgggacgccaaggagctacgcgagagcggctggagagcaccctgacaacggaaagcattcacctcctagtcgccgccggggccaatcccagcgacgtgcggcggctgcgcgctcgcggggtcgatctcttcgaagcggcgtccgccgccattcggggggaagcgactttcgcccagcaggcgaccctggctcccgttgtcgtcgtcgccgaggcggtgcaggcgcgtcaagccgacggcggcgacgggttcggatcttctatcggtttccgcgtcgtcgaaagcctgaagggagacctgccagcgggcgccgacttcgttgtacgccaggtttccggcgcggacatggatgtgagcaccgatctgcgcccggaagccggcgaccggttcctgctgctgctctcgcgagactattacgaacaactcgtcgcggaagcggggcgttcaccgcgaacaggcgcctatgcccagctgctgccgggtttcgtcgtgaggggcgagcagttgctgccgaccgtgatcggtcagccgcccgtcggctcgctggccgcggcccgaaccgccgcaggtctttaacccggagttccgaatgaagacgctcgtcaccctcgcctcgtgcctgaccctggcgaccgcaccggcgctcgcccagacgccgcccatggagcggaaatgggcctctccgtcggcccaggtctttattcacgtcgaccttccgcccgcctgcgatccggccacccagagggcgatctccacctggaatggccaagggtcgctgtggaactacggatggtcttcgcaaaattaccagaccgactatcaggcctatactggccgcgtaaccttcgccccccagcggctgtcaccgtccgtgccgggccagaccacgcgctaccccagcacaggaacgaccatgaattcggcctggatcgggatcaacgaccagatgctgttctggaacggcagctactatacggcagacggggatctgcagtgcccgcactccggcggggtttcatcgacgcgctacagctacgaatacgtggcgcttcacgaactcggtcatgcgctcggcttcggtcaccatggcgactatagctgcgtcatgagctacggcacctatgcgggggatccaaggacgcgcccctgttcggccgagacgctcgagcttcggaggcagtacggtgcgcgctagatggtcggtcgtcgtccctgccctggcgtcgaccgccctggttctgctcagcggctgcgaacaggaaccggaaggcggctcgatcaccccgccggaatggcgcaccataaccttcgaccgttgctgtgagatcgccctcccccctggtttccgggaaataccgaagccgcccggcgtggtcgacccgagcttcatcgccgtcggcgacgggtcctccgaaatcaccttcgaataccggcctcaggtcggcttcccggaaggtgccttgggccggacgggctggtcgaaagagaccgttctggttgacggccggaacgccgacttggttcggcacgatgcgcaagacgcatttgccggcgggcgaacgcttcgtctcagggtgagactgccggatgtaccgaccctgcagtccgcgcccgccgccgctaatggcatggagctaggcgcgaccggccattgccgggacgaagccagctgcgcgacggtcgaacaaatttatcgatcgatcgatctgccgccgcttcggcgggccgactgactcgaacggctttgtggcgccagggtgccgggccgccgacgagtgctctaccggccccacggcagcagtgcgccagaagcggaacttgggaccgggccgcacagaagaccttcagctgccttggggccgcccgcgcggcgcgctgattctggcctcgcaggccagcaagcggacagcgacctttctatgccagtcagcgccgccaggttgaagactattgcatcacacgcagccaagaggtggcggtcgagttcgttggccggcaacgccgcgattgacgatcgcccgccctcatctccaggcgcgctataggtggcgctaccgccaagcctccgcaacaatcgatcggcacagcgcgccagatcacctcataatcgcaacaaatccatattgaactgcatcgcaaagccgtatacacgcaccatacagacgcgatcgtgcaacgccccgatgggaatcgcttatggaccatttctcgatcatccaggctctctgtcgcgcggccatggccgatgcgtcgccggccctgcgcaagcagatcgagcgcttgcgtgatgcgctggccaaggatggagatgcgaagcaggccgccgccttgaccagcatactgacgaccgcagatcggacgacggagctttcaccgagtcgtatcgagcgttctaaggctcagattcccggcgaagttctgacgcgcaagacccccgtgcccgtcgatcgcgaaacggcggcggcgctagcagacatcatcttcccggcggacatccaaccgaccgcgccgctgttcaacgcgacggtcagccaagccatcgaaaccatcatcgaagaatgggcaaatttcgacgccctatccgagatcgacatccggccgtcgaagacttgcctcatctacggggtgccaggaacgggcaagacccgcttggcgctttggattgcgcagcagctcgaccttcccgttgtcctagtgaagttggacggtctcgtgtcgtcgttcctgggcactaccgcgcgcaacatcggtaacttgttcacgttcgccaaccgccatcgctgcatccttctgctcgacgagttcgacgccatcgcgaaagtccgagacgacccgcaggaagtcggtgagatcaagcgcgtcgtgaatgcgcttctgcagaacctcgatgttcgccgcgatatcggcttcacaatcgggatcaccaatcacccgaagctcttggacaccgccgtctggcgacgcttcgaggttcagcttgaaattcctaagccggacttcgagatgcggaaagcgatcgccgctcatttcatgccgcccgtgaaggctccggacatccatttgcggctgatcgcatggtttactgaaggttcgaccggcgccgagatcgagtcccttgtccgtacgtacaagaaggccaccaccgttcgggaggaggacaagcgtgggctgctcgatacgctccgccagttcgccacgctgaacgccgctcgagttcaaagcgaacgccgcgcgctgctgttcgacgattcgagtaacctgtttcgggccatgcgggatgatccgatccttggcttctcgatggccgacatcggcgagatcgcgggcaaggataaatcgacagtcagccgtcagctcggccgttcagccaagtcgggcgaaagcgaggtgctgaatggctagtccgatccagatcgtcctcaatccggaacactacgaggaagcgcgcgaagctggcggaggcggcggccgaaaggacttcttcgcccaccgtgacgccgaatttgccaagcatcgtgcggccctcacaaaccagatcgacaccatctgcggcgttctcagcgcgcagtcgcaaggcgacgtcggttttgtgaaggtcattctgcgccgtgaagcttgggcgaaaagccaccgaccggttgcgagcctgttccgcaacgatcgcaccccggtcgtcggcggcggcgatctcggcgtcatgatcatcgaagcccgccctgacactctccgccaagtcgcgggcgagatcgccaaggccgagacgcatacgcaaatgcgcttcaacgaacagaagcagaaggatgagcctcacccgtccgcccggaagagcgaaaccggcgccattgaccggatcgaactctacggccccgccgaccgccgcagcttctcggtggaagaggccgtcgcatggctttcaaacccgatgaccggcagcagctaccaagtcgagctgttcgatagcccaccgccccgttcggaatgggatctcctcgacggaggccatcgtcgcctcgccgagagtttcatcgcaggcttcaatgctctcggtcatgggctcgcggtcgagcggctgcccaatcaccgccacaagcagccgatcctctccgtccggctcgaccaatccagcgatcagcccgtcttgcggctgaacgaagccccgctcagtgagcgccgtcgcgagttggctctgttcaaccccgacgtcaaacgccacgctcgcctgcttgccttcctagacagccatccgcttgtccggcgaatcgaactgcccggcatcgtcgtccgggctacaggcgcgaccacgcccgcgccgcgcacgcggccgacgaacctcaccattcctactcgcgacagccgccgcacccatccacggctcggcatcatcgacggcggcatcagtaaagcgctctcggactgggtgatcgatcggtgggacattctcgccgacgaagacgccgacctcgcgcatggcacctttatcggcggcctagcagcggtcggcggcgccttgaacggcgcggaaacctgtcctgagcccgatggcgcggagctggtcgacgtcgccgtgtttccgaatgagcgcaaggccggagccttcgcctcctattatcccgagggcctgccgcagttcttcgacgagatggaaaccgccgtttccgacgctcgcgcccggcacggtgtgcgggtgttcaacatgagcctcaacatcctgcaaccggcggcgccggatcggtacagcccgcacgcagcacggctcgatcagattgccgagaccaacaatgcggtcgtgttcatttcggcgggcaatatccagccccaggatctccgcgccgaatggcccgccgacgcgaccgcagcgctcgccaatctcgtgaacgctcgcaacgacggcttgctcacgccggccgaaagcgcccgcaatgtcgctgtcgccgcgctcaatccgccgggacatgacgggtgcctaccctttgcacccacgcggtacagtcgccgtggtcctggtctacgcgccggggttaaaccggacttggcgcatgtcggcggcgcgggttcccagcatcccatcatcggacacgggctgttttcgatcctgcccgatgggacgatcatagatggctgcggcacgagctacgcctcgcccctcgccgcgaaaaccgccgccgttctggaccacgccattgagggggaagtctcgcgagagaccctgattggcttgctggtccatcactccgaaatgccgaagcccttgcagtccaaggcgctcgcgccgattgcgcgacacatggtcggcttcggcatgccgccttccgccgaccggattctcgaatccggcccgaacgccatcacgcttgtcttcgcttcgcgcatccggcgcgatcagcagatcaacttccgctttgcgtggccggcgtcgctggtgggaccaggcggcaagtgccggggccgggcgaagattacccttgtctccacgccgccactggatgcccggttcggttcggagttcgtgcgggtgaacatcaacgccaccttgcagcaggaacaggcgggcggcggatggaagggtcgccttgaaccgctctacctcccctcaaagcgggaatcaccagccgtcgaagcggaactgatcgaacacgatctgaagtggagcccggtgaaagttctggctaagacctttccacagggtgtcggcccctcgtcgaactggcggctgttcgtcgattatttgacccgcgccggggaggttatgcccgaggacggcgtgccgttcacggcgattgtcaccatcagcgaccccgacgccgaacagccggtgttcaccgatatgcgtcaaaaccttcaggcgctcggcacccaaatcgctgacatccggaccgccgcacgcattacgccgcgcgtctgatcctcatcgatggatgccgccgctcgccggatagcgagaccttaaggagatttgtcatggcgagatcagtgtcactcagaaccggacgagtcttcgagaccgttgcagccgccaaagagcattttacgctcatcctgaacggccaagagttgaagcaggcatttgccggggacgaactggccgacatccgcgccatttacgacgactactgcgcgaagaccgggtgggaattaccgtcccctccggcatccttctatcccacgcacgatcgcggtccgggctacaccacgcgatgctatggtgtgactttcgaagatgggacgactggtaaattctcgcttgagaaggcgctgagggcgatcgcagcatgaggcacattgggcgcacaatcagcaagcgagtccgcaatgtccgatgaattccgacgtctttgggagcaacaagaagcgctgcggcgaatgatgaagccttcgggcgacctgtggcgacatatcgaccccgtgcacgatgcctacaaagggctaggaatcggttcggcaacaatggacttcatccgacaggaagaagaacgccgcagaatgcttgccgatctcatggatgtcggcagcgtcgccaagatcacccaagacttcgagcgacagcgcaagctgctcgaagggccggtcgaggaagcaagacgcctaggtttgttcgaccctaactcggatattcgaaaatctatcagcgcaacaatggaagcgcagcaggcctacgaacgcctgttcagacttccggagaccatggagctcagccggatcgcccaagaggctatggagggggcccgcctcacgcgcactgtgctggggaccgaggatcgactgcaggcggctatggcttccatgcggtcaccctggctccagatcgaggaaagcctagtgtcggccaaggcgttctccgagatcatagcgatgggccgcggtatcgagagtcgccccccgtacgatcatgtttttgcctcagcgctgcggccggggctcggcgattggcgcgacctactgacgccgacacccgagcagttgatcgaccccgtgctgcgttctggcttctatgtggagcggggcttcgatccggatcttaccgatttcaccccgatggctttcggcgaaagcctgaggatcgctggtctgcgggaaccagagacgaccgagagccccgacgagcaggaggatggcttcgtccgtgccaaggaggcgttcgatcaactgcaacgcttcgaagtcgcgctccgtcgcttcatcgagcgtgtgatgcaggccgcttttggcgacgattggatgaagcggcaactccccgccaacatgctcgacgcttggatcgacaagcgagataaagcagtgaaagccggatatcccgagcaaccgctaatcgactatgcggatttcaccgactatcgagcgatcatcgaacgtaaggacaactggcgggcggtgttcaagccggtgttcggccgcgcagaggatgtgcgggaatccttccagcgcctgttccctgtccgcattacgacgatgcacgcccgtctcatcaccagggacgacgaactgcttctgctggtcgagacgaagcgtgtcctgaaggcgatccgaggccagtaactaacggtaaggcacattcggctcgccgaggacggtagccgccgggacaagcggaagatcctgagcgcgtccccccgaaggggacctggcaaatgaccgctaagagtcacgtgccgacattcgaactcacgaaaaagccgcgcgcccccaaagggcgcgcggcgagtttttcctcaatccggcgcggcggctattcggccgcgaacgcgtaggcgtcggcgtcgggcggcgtcacggcttcggccgcctcgccctcgtcgtcttcctccggcgccccggccacggccgtccgcaggacaactggcagccatcccttgccctcgaccagcctctccgccgcctcggccatgtcggccttcttgaacccggcgatccggcccgcctcctcggcgttgacggcctcggtcacggcgtccagcacccgcgccttggacacgcgggcgaagtagctcgccgccgtcgccgaccacgtccccgtcatgtcgaggccgaccgccgccgccagcgtctcggcctgcgccaaggcgccgggccgccggtcgttcgggtcacgcacggcgtagaggccgaccccggcgcagcaggccatcaggtcaagctgctccgagggcgccagacctgtcaccacgctccagaggtcttccgcccgctcgggcaggcgcgcgccccacgcctcgcaccggtcgcgaacccggcgaccggcgggaccgtcctccacccccggcgctagccgctccagtccgctgaccgtcatccgaagctgcagcggcgtccagacgccgtaggtcggatagaagacctgcagggccaaggcgtggaccacggtcgccagcgccgcccccgcatcggcctgcaccgcgtctcgcaggcccatggttctgtgggccgtcaggtcgatgaccagccggtccgagagggccgcgcccgcctcctccggctcggctcggatccggtccgcctccgacccggccccggtcccgacgtcctcagctgctccgtcctcgaagggcggcggcggttcggcgaccgccaccgcgtcctcggccctgaccagcccgcgctcgaagcgggccagaccgtcgtggcccagcaggaccacgatcccggcccgcgccctggcctcgggcgtgtaggcgaagtccgggccgaaggcctgcaaggccttgtcgatctcttccagccgggcgtccacctcgggcggcagcatctccgccgcgtcggtttccgaaaccagacggtcgtattcctccgacagggccgcgatgacggcggcgtccgccgccgaccgctcgaccgccaccggatagacccgtccgaacgcggagaggtccggatactcaagacccgcctcggcccatttccagccctcgcgctcgcgcgcctcctcggccagccccgccagcttgtcgccgaccagccggtccagcagccccacgtcctccagccagccgccgccgtcctcggtgaagaggtcgcgcagcaccgccccgccttcggcctcataggcctcgacgccgacgaagcgcacccgccggtcatcgacgcggaccttggcctcggtcatggcgcggcggatggcgtaggccggggtgtgcggcccgacctgctccagcacttgccgttgccgctcccggtcctcgctgacgcagaaggccgtcaactggtcgagcgccagcgtcccgtcccgataggccgccatcaactccggcgccgccgacccgagccgcagccgctggcgcacgacgtgggccgacaccccgaaccgggcgccgatttcctcggggccgtagcccttctccacggccagccgctggaaggcctcaaactggtcggcgggatgcatggcctcgcgggtcatgttctcgtccagactgatttcgtgggcgtcgttgtcggcgtccacgatcacccgcaccggatgggtgcgcttgatcgccttgcgcttggccagcagccgcagcccctgacggcgcccctccccgatggtgacgagatagttcccggtcgggacgccctccccgtcccgctcgacctcgaccacgggcggctgcaacacccccttggccctgatggaggccgcgaaggcctcgatggtcgccgcgttgtgcggggtcttcctcgcatttttcggcgaagccttgagccggttcagcggcacgatcagttccgcgccgtgctgcggcgcggtcgcctccgtcgcgacggtttcgatggattgagcagtcatgtctgcctcctttgggcatgggttgcaggcacgcgaactgcgcgcctgaaaccctgcccgtcggcgagaccggggtagcaagggccagggcggaccggccggagggggatcgcccgggctgcacaagccgatgatgatgatgatcatgaacagcatgaccgcgcggaaggccggggagaccggccggtccggcggcggagccgcttcaccctggcccgcgcgagggcggagcccttagcgcttccgagcggcgtggcggcgtgcgcctgtggacgagacgtccagccaggcggagtccaccttgaccctgcctcctgttccgcttttgttcttgccatgccctaccgcaagaccgtcattgtcgaatggcagaccgccggcgaccgccgctcctatttcgtgcggcccggcagccggtcccgcccgtggatctggttccgggacggcgacgggccgcccttcgacgaggcttgcgcccgcttcgtggtcgagaagcgcgccggccgctgggtggcggtggagcgggcctgagagcgtcgccgtccggcgaacgggctgacggcgacgcccgcacgccgccatgccgtcggatcgatacgcccctcgaccgctagtcggcggcctccgcctgtgccttgcgggcgtcctccagaatctccaggccgcccctggcggcgatcccggcgacgatgacgccgaccaccaggtccggccaggactggtccagccacagcaccagtccgcccgcgacgatgatgccgccgttggaggcgaagtcgttgagactgaaggtctcggcggcgcgcagattgacgtcgtcgccgtccagccgccgcagcagttgcagacagatcaggttcaccaccgccgcgacgacagccaagacaatcatggtcccgccgatcggctcggcccccagccaccaccgccggccggcgtcgaccaggacgccgacggcgaagatgagcagcaggacgcccgacgtcgtcgccgcgcgccgcttccaggtcagggcccggccgaccgcgaggaagctgatcagatagacgacgctgtcggaggcgttgtccagcgcgttggccagcaaggcgctggagtccgccagcaggccgccgagaccgagcccggcgaacagcaggccgttgaggatcaggacgaccagcagggtcctccgctggcgctcatgccggccattgacggtcacaggggttcctccctcttctccagaatgcgcgcggccagggtcggcagcaccagaagcgtcagcagcgtggcggtcagcaggccgccgatgaccacggtggccagcggtttctggacctcggcgccggccccgaaggcgaaggccatcgggatgaagcccagcatcgcgaccagggccgtggtcagaacggccctgaggcgactgacggccccctcgacggccgccgccaggggcgcggccccttcctcgtaacgctggcgaatggcctgcatcagcacaagcccgttcagcgtcgcgacccccgagacggcgatgaagccgaccgcggccgagatcgagaacggcatgccgcgcagcaggagcgccaccgccccgccgaccagggccaggggcacgccggcgaagaccagggccgcgtccttgagcgagcgcaacgccaggaacaacaacaggccgatggtcaggaagaccagaggcacgatcatcgccaggcgggcgctggcgcgttcgaggttctcgaactgcccgccccagtcgaaccagccggacacaggcgggcgcaccccgcgaccgacggctgcgcgcgcctcgttgacgaagccgccgagatcgcggccccggacgttggcctggacgacgatgcgccgcttgccgttctcgcggctgatctggttggggccctcggtgacctcgaaccgggcgaccgccgaaaggggcactgtcaacgcgcccggttcggccgcttccggcatcaccggcaactgggccatcaccgccggatcgttgcgcagatcgtcggccaggcggacgacgacatcgaagcggcggtcgccttccaggatgtggccggccgaccgcccgcccagggcgatggccaacgcatcggccgcgtcgctggcgtgcacgccttgcgccgccgcgatggtccggtcgacggcggcggtgatcgacggctggcccgagacctgttcgacgcggacatcggccgcgccggggatgcgtcggaggacggcggcgacctgatccgcgctggcctgcatggcggcgaagtcgtcgccatagacggagacggccacgtcggagcgaaccccggcgatcagctcgttgaagcgcatctggatcggctgggtgaattcgtagttgttgccgagcaggtgacccaggttctcctccatgcgctcgaccagctcggccttggccagggaggggttcggccactcgtcgcgcggcttgagcatgacgaaggtgtcggagatcgagggcggcatgggatcggaggccacttcggcggtgccggtccgggtgaagacctgctccacctccggcatcgcctgcagggttcgttcgacctggaactgcatggcctggctctgttcgagcgaggtggacggcacccgcagcgcctggaccagaacgtcgccctcgtcgagcgtcggcacgaactcgcgaccgagactgaggaaggcgagcaatccgacgagaagcgcgagtcccgccccgacgacgacggcacgcgggcggtcgaccacccgccgcaggagcggctcgtagcgggccttggccgcccggctcagccgggtctcgtcgtcgtgccccttgggctcccgcacccagatggcggccatggccggcacgaaggtgaaggacaggatgaaggcgccgagcagggcgaacatcacggtgccggccatggggccgaacatcttgccctcgacgccttcgaacatcagcagcggcgcatagcccagaaggatgatggccgggccgaaggcggccggccgcgccatttctttagccgcgtcgaccgccacggccagccgttcgggcaggctcagggcgcggccgacgctctcgcgccgcatggcgagccgccgcagggtgttttcgatgacgaccacggcgccgtcgacgatcaggccgaagtcgagcgcgcccaggctgagcagattggcgctgatcccgaagcggttcatggccgtagcggcgaacaggaagctgagcgggatgaccagagcggtgataatcgcagcccgcacattgccgagcgcgaagaacagcacggcgataaccagcagggcgccgagggcgaggttgtgctcgacggtgcggatcgtggcctcgaccagttgggtgcgatccagcgccggcttgaccacgacgccagggggcaggctcgcgccgatctccttcagccgctcgccgacgcgatgcgccacggcgcgcgagttctcgccctggagcatcagggccgtgcccaccacggtctcgcggccgttgctgctggccgagccgaggcgcggcgcgcggccgatctcgaccatggccacgtcggagacccggatcacctggccgccgcgattgaggatcggggtctgggccagctcctcgaggctgcggatccgcgcgtcggcccggacgatgtaggcttcgccggcccggttgacatagccggccccggcgatgcggttggcgtgttcgagcgcctcgaccagttgcacaaggcccacgccataggcggcgagacgcgcgggatcgggatggaccgcgtactccttcacatagccgccctggacgtcgatgccggcgacgccttcgacggtcttgagctggggcgcgatgatccagtcctggaccgtgcgcagataggtggccttctcctcgtcggtagtcagacgctcgccctcgggcgtgaggtagacggcgcctgtgcgggcggccggaccggtcagctcgacggtgaagatgaagacttcgccgaggccggtgaccaccggccccatggagggttggacgccttccggaaggtcgtcccgagccgcctgcatgcgctcgttcaccaagctgcgcgcgaaatagatgtcggtccgatcggtgaagacggcggtgatctgcgagaagccgtgccgcgacagcgaccgggtctcgaccaggcccggtaggccggccagcgccgtctccatcgggaaggtcacctgacgctcgacctcctccggcccgagcgcgggcgcgacggtggtcacctggacctggcggttggtgatgtccgggacggcgtcgatgggcagccgcaccagttcgcgcacgccgaagccggcgaggacgatcgcggccaacacgacgagccagcgatagcgcacggcgcccgagatgatccggtcgagcatcagtcgtggtcctccacggcgcccttgccgagctcggccttcagcaggaaggcgttcgcgccggcgatgcgctcggagccggtcaggccgcgaacgatctcgatgcggtcgacggcccgccggcccggaaccaccggctgggcccggaagcccgtcggggtgacgacgaacacgacactggcgccgtcgacggtctgcaccgcctcggccgggacggcgatgccgctttcgccgccggtgatgatcgagccgctcaccgccgaacccggcggcggcgcgacgccgtcggcccgggcgcggatcagggtcgatccggattgcgcgtcggcgcccggggccacggcggtgaccacggccgcatactcggctccgtccgcgccctggaccgtgatgcgcgcaccgggcctgaccgtcgccgccagggcggcgggggcgttgaagaccagttcgacgcggttgggattggcgatggtcgcgaccggatcgccctgctggacgacgccgcctagtccgactctcagggccgtgacgaccccggcgatcggggcgacgatcgtcgcccgcccgctggcgttggggcctccagcggcggcgacccgggcccggctggcgcgggcctgggcctcggcggcggcggcgcgcgcctgcgacgcttcgacgtcctggcgcgcgaccacgccctggtcgaacagattggcgtcgcgcgtccgcgcggcggaggcggcgcgggcttcggcggtcgcggcgtcggcctccgcccgaagggtcgcgccatccccgctgatcacgaccgcgatcggctggccggcgcggacgaccgaacccggcgcgaccagcagccgttcaatgcggccgccgagggcggcgccgacggacgcctgggcgtccggcgcggcctcgacccgtccggcgaggtgggtttcgccgccgccgccggactgcaccgagacgatgcggatgccggcggcctgggcctcggccggcgacagggtgacgacgccgggttcgccgccttcgccctcttcggcatggccttcctctccctcggccgccgttccggccgcgggcgcggcggtcagccgggcggcgccgtaaccggcgccgacggccacgatcagggcggcgaccgccgcggcggtcctggtgcgggtgttcatagttgagctccaaagggggcgcggccttcgaggcgcgcgagttcggcttcggcccgggcccgcatcaggcgagccgcgatggcgacgtcccgggcctgcacgagaccgctgcgggtgctgcgcagttccagttgggagagacggccggcctcgaagccgatccgcgtcaggcggtaggcctcggtcgccgccgtcacggcggcgtcggcggcgacgacgcggctggcggccgcgtcccgccgggcggcggcggcgcgccagtcggcgtcggcgtcgaggcgcgcgcccctaagcctcgcctcggcggcgcgcacctcggcctccgcggccaagaccccgccccggttccggtcgaacagcggcagttgcaggctgacgccggcggtcagcgcggtggcgtcctcggcctcgaaccgccggaccccgacgctggcgcgaacgtccggtcggccgcgcgccgtttcgacgcgcacccggccctgggccgcgccgcgctcggcgacgagggccagaacggccggcgcatcggccgcctgacctactgaggccgtgggcgatcgatcgagcagggagctctccacggaggtgagcggcgtctgtccgccggccagggcggtcagctcggcgaaggccgcgtcgcgctcggcccgcgcctcgtcgagcgcggcgcgcgccgccgccgcttcgctctcgccctggatgccgcgcagcagcggctcccggccctcctcgacgaggatcaaggccgcgcgcgcgtcggcgaccgcgagttcgagcgcctcttcagccagggcgtatcgccgctgcgcggcctccgcctcggcgtaggcgaccgcgagcgcggcggcgacttgcagccggctggcgtcgcggcgccagcgagcggcttcacgttccgattgagccacaccgacacgggcgccgcgacgtccccaaagctccagatcctgcgagaccgtcagggtggtctcggctccatccaccccctggaagggaccccgaccgaggatgttctcgacctcgagccccagttcgggattgggccgcacgccagcctgcgccaggcggccttcggcggcggccagatcggcgtcggcttcggccgcggcgggcgcggtcaatgcctgggtcagcagttgttcaaaggccggcgcggggtcggcccaagccggaaagccggccgccagagccaggacggcgaaggcgcagccgaccgcgcgcggcggccgacagggaggtgacagagacatgatcggggttccagagtttcgacgaaggcgaacgcgccggggcgcgggcgaacgtcaggctctgggcggtcgttctggtcccgcgggcgtgcgggaggggcggtgatccacgaaaagaacggggtgagtcgcgtccgcgctgacggcgcggctgacctcgggcgcgggcggcggcgccgtgaggccgccatggtggcactggcagtgcgtgcagccgcgcggatcggcggcgccccggtcggcgttgtccctgtctccggcgggggcggcgacctgggtcgccgtcacttcgacaaaggacgcgcccgcctcctcggcgatgcaggcggcggcgtcgaccgctgtcgccaggacgaggaacgacaggaacgacgccagaagcgtcgccatcagtcctcgtctcgccaggcccttgcgcatggggccctgtagcacgcgccgccgtgttcgtaaccgcgtcatggccgcgccgcgcgatagaaggtgatcgagcccgtcagggtcggcagcacatgaagttcgcgaacgccgacgaagccggccccggcgatcagggcgggcaggacgccgtcggcgttcggctgggtgttctcgtagccgtcgagcgactggacgatgcggaacagggtgcgcatcgcgcccgtctgtcgcccgtagtcggcgatgtgcagcgtcccgccggacttcagcgcccgccaactcgccgccaggccgagacgcttctcctccatgggcagttgatggaagacgaggctggacgccaccttgtcggcgacgccctcgccaacgagcgaggccacgtcgcgcgcgaagccctggacgaaacggatcggccggcgggcggcttccgccttcaccgccgcccggctgaggatgtcgccgtcgggatcgaggccgatgatgcgcgcgtccggcgcgcggcgcgccagggacacggcgaacgatccggtcccgcagccgaggtcgatgatcgtctcgccggcctccgggtccacctggtcgagcagtcgggcgcgccaggcccgctcccgggtcaacagggcgatggcgggatcgtagaggccgctcagggcggcgtggccgagcgcgggggtgaagctcgcggtcacgccgcggccttcagctcggcgcgcgattgtttcaggatcgaccaggccgactgcaggaagaccaccgccaggatcgcccccgcgatcaggtccggccagcgggaggcggtcagccacaccgccagaccggtgccggcgaccaccacgctctggatcaggtcgttgcgcgtgcacagccagaccgagcggacattggcgtcgccctcgcggtggcggaccagcaggagcgcggccagggcgttggcgaagaagcccagggcgcccaggccggtgatgacgaacccttccggcggcgccccggaggtggcgcgccagatcgcgtagccgaggatgaacagcgccagcgccgcgagactggcgcccttgaccagggccgctccggaccgcacggcgaccgtgcgcccgatcacggccaggctgatgccgtaggtggcggcgtcggccaggaagtcgagggcgttggcccccaaggcggccgagccctgcagggccgcgccgccggcgatggccaggaaggcggccccgttgatggcgatcaccgccatgaggatgcgccgataggccggcgtggcgccgtcgaacttcacggtcgcgccgcagccgcagccggaggccgccggttcagaggataagggacgttcggtcatggctctccacctgtcatcatgaggatgcatcctccagtcgctggaggatcaagcggaaattcgcgcccgcggccgaacctccggactcgccgacgggtcttgatcctccagcgactggaggagttaggatgcggaccgagccggagcgaacccaccatgaggccgatgaacgccgaacagagagagatcgccgcccgctcggcggcggcgatcgcgctgagcgccgcggcggtcgccgccgcctggctatggctgccgcccgcgctgctcggcgccacgccggatatggcgacggccgatcggctggcctacgcgctgaaggcggacctgccggtctttctgtggctcggcggctgtctgagggctgtggccagcatccggttccgatcggacgccgaccggccgggcgcagcctacgggtcgcccagcgcccggctggccgtgccggccgccgtacttcagaactccctcgaacagacggtcctggcggtgggcgcccatctggtcctcgccaccgtgctgcggggcgaggagatgatcctgctgccggtgctggtcgccctctatctggccggccgggtattcttcgccctgggttacgccaggggcgcggccgcccgagcgttcggcatggccctcaccggcacctccaccatcgccgccttcggcgtcgccctcgtcctcatggggctcggccgatgatcccgcgccgggtcgccctccggccatccgtcaaacccgagacgacacaatgacccagccctcccccgcttcatcgggcctgcgcccgatcggcaagctcgccgccgccaccggcgtcaaggttccgacaatccgcttctatgaagagatcggcctgcttcccgcgccgccgcgcaccgccagcgaccggcgcatgtatgacgacgcggcggagcgccgcctgtccttcatccggcatgcacgccagctgggcttcgacctggactcgatccgctccctgctggacctgtccgatcacccggaccggccctgcgccgaggcgaacgtcatcgccgaacgccacctggccgaggtgaagcagaagatcgcccagctcagggcgctgcaaggcgagctctcgcggatgacggcggaatgcgccggtggccgggtctcggcctgcaaggtgatcgaagccctgcacgatcacccggcgtcgctttgagcgcgacagtctcgcggcgcgaatgctaatgcgagccgctcacaactaggtttcccatgcgtcctctgttccacctgctcgccctgctgttcgccatggcgctggctggccccgccctcgcccaggccccgtccgcctcggaggcccaggtggcctggcggctgctcgactatgtggcggtcgactacgccggcgctgtggccgatggcgagatcgtcaacccggccgaatacggcgagatgatcgagttcagcacccagatccggacgcgtttggacgccctgccggccaacccggccaaggccgctctggcgcgcgacgccgcgggcctgcaggcggccatccgggacaaggccgatccggccgtcgtcggcgcccgggcgaaggccctggccggcgcggtgctgacggcctatccgagcccgctggcgccttcgttcccgcccgacctggctcgcggcgccgccctctatgccgagcagtgcgctgtctgccacggcgcgaccggtcgcgccgacggcccgggcgccgaggggctcgacccgccggcgatcgccttcgccgacctggagcgcgcccgccagcgcagcgtcttcggcctctaccaggtgatcgaccaggggctggagggcacggcgatggccagcttctcgcaccttccggccgaggaccgctgggcgctggccttctatgtcggccgcttcgccttcaccgacgccgaagccgccgagggcaagcgcctgtgggacggcgatcccgcggtccgtgcggccttccccaacctggccgccctcacccagaccacgccggccgacctggccacccgcctcggcgaaccccgggcgcgagccctgaccgcctatctgcggcgtcatcccgaggcggcggcgcgcccggccggatcgacgctgaccctggcgcggacgcgcctggcggagagcgaggcggcctatcgccggggcaaccgcaaggcggcgacggacctggcgctgtccgcctacctcgacggcgtcgagccgatcgagccggccctcggcgcccgggacagcgccctgatgcgccgggtcgagaccgctatgaccgagctgcgcgtctcgatcagccggggcgcgcccgcccgggaggtcgcggaccgggtcgcgcgtgcgaacgccctgctggacacggccgagcgggccctcgcgccccaggaggcggacaatctcgccagcttcctcggcgccttcaccatcctgctgcgcgaaggcctggaggccctgctcatcgtggtggcgatgatcgccttcctcaggaaggccgaacgccccgaggtgctgcgctacgtccacggcggctgggtggccgcgctggtcgccggcggcgccacctgggcggccgcgaccttcttcatctccatcagcggcgccagccgggagctcaccgagggcttcggctcgcttctggccgccgtcgtgctcgtctcggtcggcatctggatgcacggcaagtcgcacgccgacgcctggcagacctatatccgcgacaagctctcccacgccctgtccaaacggtcggcctggttcctgttcctgctggccttcgtggtggtctaccgggaagtgttcgagaccatcctgttttatgcggcgatatggagccagggcggccatgtcggcatgctggccggcgccctgacggcggtggcgatcctggccgtggtggcctgggccctgctggcctacagcaagcgcctgccgatcggccggttcttctccctgagctcgatcctcatggctgtcctctcggtcgtcctggtcggcaagggggtggcggcgctgcaggaggcgggctggctcgatgtccaccccctggcctggatcccccgcatcgagatcctcggcctctatccgaccgtcgaaggcgtcgccgttcagctgttgacgatcgccatcctcgtggtcggcttctctcggcatgggacgccgaagggcgcgcggccggcctcttgagcggccgtctccgtctgcggccctcagactgcggcccgtcggcaaggatatcggcgccgcttgggcacgagggcgccgatacccgaacgatccgcggataccaaagatgcggggctgcagccgatggctgtgagagcccagccttggtgtgcggagattaagctccctattctccgcaccatgcgcggagaatagccttgctcttacggcgaataacgcccatattctccgcaaggagtgcggtgaatggcggagtacatccacgagatcgaaggctggccgcgtctggactggcgcgctgacgcgctcgccgatcgcctcgcggcggtccgtcaccgccagggccttctacttggccggatgcatacgctcggcttcgacctgcgcgctgaagcggttctcgagaccctcaccgaagacgtcctcaagtccagcgaaatcgaaggcgaactgctcgacaaggatcaggtgcgatcctcgatcgcccgccgcctcggcatggatatcggagccctcgcccctgcggaccgcaacgtcgacggcgtggtcgagatgatgctcgacgcgacccagaactttgcgtctccgctcaccgaggaccgcctgttcgcctggcacgccgccctgtttccgaccgggcgcagcggcatgacgaagatcgtcgtcggcgcctggcgcaacgagaactccggcccgatgcaggtcgtctcgggccctttcggacgagagcgcgtgcactacgaagcgccgcccgccgcccgtgtgcaggacgagatgcgggtgttcctcgactggttcaatgacgagccgcggacggatccggtcctcaaggccgcgatcgctcacctgtggttcgtgaccatccacccgttcgacgacgggaatggccggatcgcacgcgcgatcgccgacatggcgctcgcccgctccgagaaaagcgcccagcgcttctacagcatgtccgcccagatccggctggagcgcaaggactactacgccaccctggagacgacccagaaaggcgcgcttgacgtgaccctctggctggactggttccttggctgcctcgatcgcgcgttcgacggcgcggaagccaccctgacccatgtgatgcgcaaggcgcgcttctgggaggcgctcgccggtcagacgttgagcgggcgccagagcacggtcatcaaccggctgctcgacggcttcgaaggcaagctcacctcgaccaaatgggcggcgctgacgaagtcctcgcccgacacggccttgcgcgacatcaacgatctggtggatcggggcatcctcgtgaaggatgaaggcggcgggcgcagcacgagctactccctggtcgatcgaggataggcggcctcctacggcgccggcgggactctgggcggggcggctccgctcaagaagcgggtctcaacagggtgaatcgcaattcgccacttctggcgagttacgccaagacgccagcttatttccccagaagtggcgacttacgacctttgccaagcgcgcgacgccccaagccgccgccgacgcggcctcaagcctgacgcgcgatggcgatagccgggagatcggcggcggcgtcgaccggaattccggccgccttgcgctcggaatagcggtccacgagctgggacgcgtggggccggacaaggatggtgaagcgcaccagttcctccatcacatcgacgatgcgcgcatagtaggccgagggcttcatccgccccgcctcgtcgaactcctggaaggccttggccacgctggactggttggggatggtgatcatccgcatccagcggcccagcaggcgcagggtgttgacggcgttgaagctctgggagccgcccgacacctgcatgaccgcgagcgtccggccttgggtcgggcgcatgccgcccaggctcaacggcagatggtcgacctgcagcttcatcaggccggacacctggccgtgccgctccgggctgcaccagaccatgccttccgaccccagggcgtgctcgcgcaactcgcgcaccgccggatggtcgtcgtcgccgggcgcgcccggcaggggcaggtcggacgggtcgaagatgcgggtctcgcatcccatgcgctgcagcaggcgggccgcttcctcgacgcagagccgcgagtaggagcgttcgcgcagcgacccgtacaggagaagaatgcgtggcgggtggtcgtgcggacccaggccgcccgccggatcgctcgacagaaaagccgcgtccagggccggcagatgatccggatccggcagcggccgcagacgcgcgaaggtcatccgagatccttggtgagataggcggccgaggccgggcagatgtccgtgaactcgccggttcgccggatcgcttcgggcgcggtctcccgatcggcggcgacgaagccgcgccggatgaagaagggctcggccgtcgtggtgagcaggtgaagacgttccccgcccatgtcgctcgccacggcttcggcggcggtcaggatgcggcttccgaggccttgcgccttcctgtgggcggatacgaccagggagcgcagcagcaggtcccgcccctgcccttccaagccgacgtatccggccagggcgctgtcgtcgtcggcgcggaagtagcggccggcgccggggtccggcaggccctcggttctgagcgcggcgatcagaccggaatcgtttgcatcgacgcggtgaagcccgatcatcagacgacgtccgccggcggggcggtgtccgggaaccagcgccggcccatccacagcgcgaccgacaccagcaggatcagcaccggcacctcgaccagcggcccgatgaccgccgcgaaggccaccggcgaggtcagcccgaacgcggcgatggccaccgcgatggccagttcgaaattgttcgaggccgctgtgaaggccagggctgtggtgcgcggatagtcggcctcgatcagcctgcccaggaggaagctgaccacgaacatgacgaggaagtagatggtcagcggaatggcgatgcgcagggcgtcgagcggaagagccaccacctcgccgcccttgaggctgaacatgaccacgatggtgaacagcagggcgaccagggtgatcggcccgatgcgcggcaggaagcggcgctcgtaccagtcggcgccccggcgggcgatcagactgcggcgggtcaggaagccggccaggaacggcaggccgaggtagatcagaacggcgccggcgatggtccagacgctgacgtcgaccacgctgccctgcaggccgaacagcggcggcaggaccgtcaggaagatccaggcgtagaggctgaagaacaggatctggaagatcgagttgaaggcgacgagcccggccacatactggttgtcgccgcgcgccagctggttccagaccagcaccatggcgatgcaccgcgccaggccgatcaggatgacgccggtcatgtattcgggctgatcgcgcaggaagatgaccgcaaggacgaacatcagcaccggacccagcacccagttctggaacagggacagggccagcacgcgcctgtcggcgaacacgcgcggcagcgcctcatagcggaccctggccagcggcgggtacatcatcaggatcagaccgatggcgatcgggatgttggtcgcgccgaccgaaaggctgtcgacccaggcgggaaggccgggaaccagggttcccaaggcgacgcccagacccatggcggcgaagatccacgccgtcagccagcggtcgaggaaggacaggcggcgcggcggcgccgcctccgacacgggcgtatcgatcatcgtcccacccgccggccgtcgacgtcgatgaccacctcgccgtcctccttggtgaagggtttgaggccctcagcgggcagaaggtcaagcacggcttcggacggccggcagagcctgacgcccaagggactgacgacgatcggccggttgagcaggatcggatgggcctcgatcgcgtccagaagctgatcgtccgtcaggtcgggattcccgagcgccagttcggcgaagggcgtgtccttctcgcgcaacaggtctcgcagcggcgcgccggtgcgttcggccagccaggcgaccatggcgcgcgacggcggggtcttcagatactcgacgacgtgcggctcgatgccgaggtggcgaacgagttcaagcgcgttgcgcgacgtcccgcaggccgggttgtgatagatgacgatgtccacgggatcctcaggggcagcagggcgcgagttcagccagcagaggctcacacaggtccgcccggcccccgcagcagtccttgagcaggaagaggaccaggtcgcgaagccggtccagatcgacccggtagatgatcgaccggctgcgacgctcggagcggatcagccccgcgcgggtcaggacgcccagatgggacgacagggtgttggccgggatcgccagatggtttgcgatttcaccggccggcaagccgccgggttcgtgacgcacgagcaggcggaacgcctccagccgcgtcgattgcgccagggcggcgagcgccaggatcgcgggttcggtttccatagttccgaattagtcgaaatatggatatgtgcaagccctctccgcgcacaacgcagtaagcctacggtcgagaggttggcggctaggcctgacgcggtctttcgacttcgattcccacgacactgtggagatattcgatggcccaggccgaccccccgctgaagcgtacgatcaagaagccccagttgcgccagatggtgcccctggccgacagcaccatctgggagatggagcagcgcggccagtttccgagacggttcctgctgacgccgcgctgcgtggtctgggatctcgccgaggtcgaggcctggctcgcgcttcgccgggccaagccgatccgcagggctccgccgcccgacgtgcgcaagcgggtcagccgaccggtcagagccgcggatcgaagcgaggaccggccgtttccgggatgacgagcacgggcgtgaacgcccgcccggcctcccaggcgtccacggcgttcgaccactcctgggccatgtgacggcgctgggcctcgaactcggccttgttgtagacgccgcgggacgaccgctcctcgtgggccagacatttctcgatccagtccgagttgaagcccatctcgtgcaacagcgtcgaggcggtgcgccgcaggtcgtggaccgtgaagggctccagcggcaggtctcgctcgcgcgcccgctcggcgatcgccgaggtcacccggttgaaggtcgcccgcgacatcggcgcgtcggcgtcatagcgcgagggcaggatgtaacgggagtttccggcgcaggtcttcagcgcgatcaggatgtcgagcatctgggtcgagagatagacgttgtgcggccgcgaccgcttcatccgctccttcggaatcgaccagaccgcattggcgaagtcgacctcgtcccagacgccatcctgcagctcactcttgcgaaccatgctcagcaggatgaacttcatgccgaggcggatcgtcggcagggtcgccacctcccccagcaggctcagcgcgatccggatctccgttggcgacagcgaccggtcacgtggccggaaggtggcgatcgaggccggccccaccccgtcggcgggattgtcgatcttctccccgtgcaggatggcgtaggcgtatatctgtttgacgatgtcgcgcacgtgcacggccgtcgccggcgcgccccgctcgacgatcgtcttgcagtgggcgcgaagatcgttgggggtgatctcgttcagcaggcgggtgcgccattgaggcaggatttcccggttgaagatggaccgccgcatgttgcgggtgctgtccgccatcggagcatgatccatccatcggatcgccacctgctcgaacctctgggcctccttcagccggcgcttgacccgctgcttgtccagcgccggcgaaacgccttcggcgatctggcgcttcgcctcgaccagcttctcccgcgccctggcgagcgagagcccggtcgggccgtaggcgccgaacgtgaccgtctcgcgccgcccgttgaagcggtagtcgtacttgaaagcgatgccgcctgtcggtgttacgaggacgtacaaaccgtccctgtcggtctttttgtaaggcttcgtttttccacgtgtatttcgcaattcagcgtcggtgagcatgccgttttcactccaaaagaccgtcaggcgttttcgggacctttcgggatctttttcctcagccaaatccgcagcttggctcagaaaaaagaccgtcaggacgccctcggccctatgacggtatggagcggagtctccgcgagcaatggcggcgggaccgtcggagcgaccgacaaaaacgaaagcagcccctcgaaaggtatcgagaggctgcgaaagcatttatcttgcaagtcagtgatttagcgctatatttcaaagcgccgccgaaagacttcgaaagccctgaatcactcccattcgatcgttcccggcggcttggaggtcacgtcgtagacgacgcggttgacgccgcggacttcgttgatgatgcgggtggcggtcttggccaggacgtcccacgggaatgggtagaagtcggccgtcatgccgtcagtggaggtgacggcgcgcagggccagcaccttttcgtaggtgcgggcgtcgcccataacaccgacggtcttgaccggcagcagcacggcgaaggcctgccagatatcgtcatagaggccggccttgcggatctcctccagatagatggcgtcagcgtcctgcagcgtggcgacggcgtcgggcgtgatctcgccgggaatgcggatggccaggcccggtccggggaacggatggcggccgacaaaggcgtcggtcaggcccagctcgcggcccaacgcccggacctcgtccttgaacagctcgcgcaagggttcgaccagcttcagcttcatgaagttcggcaggccgccgacgttgtggtggctcttgatcaccgccgagggtccgccggatgcggacacgctctcgatcacgtcgggatagagggtgccctgggccaggaactgcgcgccctcgatcctggcggcctcacggtcgaagatctggatgaagacacggccgatagttttgcgcttggtctcagggtcggaaacgccagccagctgtcccaggaattccttcgatgcatcaacatgcaccagcgggatattgtagtgttccctgaacagggtcgtgacctgcgtcgcctcatccttgcgcagcaggccagtgtccacgaagacgcaggtcagctggtcgccgatggcctcgtggatcaataccgcagcgactgaagaatcgacgccgcccgacaggccgcagatcaccttggcgtcgccgacctgctcgcggattttcgcgatctgctcgtcgcggtaggcggccatggtccagtcgccgtccagcccggcgatggcgtgggtgaagtttttcaggatcgcggcgccgcggggggtgtgcatgacctccgggtggaactgcacgccgtagatgcgccgcgactcgtcggcgatggcggcgaagggggcgccttccgaggtggcgatgacctcgaagccgtcggggatcgcggtgacgcggtcgccgtggctcatccacaccggttcacggtgatccaccgcaccgacgccagcgaacaacgggctttccctggtgacgacgatctcggcgcggccgaactcgcgatggtggccgctctcgaccttgccgcccagctcggcgcagatcagctgctccccgtagcagatgcccaggatcggcacgccggcctcgaacaccgcgtgatcgacacgcgggctgtcggcctcggtggtcgagcttgggccgcccgacaggatgatcgcccggggcgacatggccgccagcgccgcgcccgccttgtcgaacgggtggatctcgcaatagacgttggcctcccgcaggcgacgggcgatcaactgcgtcacctggcttccgaaatcgacgatcagaaccttctggtgatcgccgggcgtggtcggagcgggggtcatgcggctgtctccgtcagaggtaagcaggcggggtcttggccgacatcggccggtgtttgggggcaggcccggccctgcgtcgtcagcacgtcgacgagccgatcccaggcggcggccaggttccgatcgacatggtgcagggtggaggtccagtcctccagcgccttcaactcggtccggccgtccgacacgccgcgcagggtgacaaggggcacgccgaagctctggcaggcgcgcagaagagcgaaggtctccatgtccaccatctcggcctcgatctcgtcgtaagcctcgccagagacgacgttcgcgccggtcgacaaggcggcggtcggaacgtcggggatcgggtgcggcaggggcaggacaaccggcatgtccagcaacggcgtcacgccgcgtggaaagccgagcgggctcgcgtccatgtcgcgatagccgacggatgacgcctgatagacggcggcgtgctccagaacgcgcgatccgcacgatccgagcgacacaaccgcgtcgggaaggcgtccttcctgttccagccgcgcgagcgccgtcgtcaggctcaccgccgcctccaccgggccgactccggtcatcaacggccggatgcgcgaccgcagatgctcgccgtactcggccggagccgccatgaccgggaggatgcagaccgttccgcaccgctccatgcgcccgccgtcgctcatgcggcgcgctcgtaggcggcgaagaagaagccgtccgtgccggtggacgccggcgaaagacgcagggcgtgccccggcgccttgtcgatcagcgccgccagcgcagcgtcgcctcgcgggatcaggtcggacagcgcgatcgggcggaagtcgccatgggaggcgtcgaaggcggcgaggctggcctcgttctcgcggctcagcatcgagcaggtgacgtagaccaggcgtccgccgggcttcaccagccgcgccgcctggcccaagatgcggacctgcagcgcatgcaggcgctcgacctcttcggccgtcagccgccaggcgtcttccggccgacgacgccaggtgccgctgcccgagcagggagcgtcgacgaacaccaggtcggcgcaatcgttcagttcctcgagcccgccgccgttctggccgatcagcaccagttcagcctccacgcctgcgcgctcgagccggggacgaatgttgttgagccgcttctgcaccacgtctgaggcgaccagcctgccctccccgccgtcggccagatccatggccgccgcaagacccagcgtcttgccgccgccgccggcgcagtagtcgaccaccgtcatgccgggtttcgcacccgccagggcgcagacgacctgactgccctcgtcctggatctcaatgcgccccgcctggaaggcgtccagcgcctggacgttcggcggcggctcggcggcgaggcgcaagccgacgggcgacagcggcgtgtgtgcgggatcgagccccgcctcgcgcaattcggcctccacggcctcgacgctggcgcgggcggtgttgacccgcagatcgatcggcgcgcgcgggaccatcagcccttgcgcctcctccgcccagcgatcgccgaaggtcgccttgaagtcctcgaccacgaactcgggcaggccggcggcgatccagcccggcaggtcccccggctgggccgtcaggcggttgcgctcctgcttggacaacggacgcggtccgtatccctcgccagagtgcagcgcctcgatctcctccagcgacaggccgtcgatggcggacagggagccgatcaccagcgcccgtccgtcctcgcgtccgcccatgatccacgacaggcggccgcgcgcgcgcagcaccttgtagacgcggtcggcgatggcgcgccggtccttggagcccgcatagcggttcgccgcgccccaggccttgagcaccgcttccgccggctggcggctctgggttatggagtctatgacggcgccggcggcggccaatcgggcggcgggagtcacttgggcggcatcctcataggaacagggcggcgaggatcagaaccagcccgatcagcgagacaagccacgccagcgaccggacatagggaacgcccagcgcatacagcggcacatagacgacgcgcccacagaagtagagccccgcgccccatgaggtccaggcgccgttcgccccggcgacatgcgcgataaggaccgcgccgatgaacaccggcagggtctcgaacagattggcctgagcccgctccagcctgtctgtgatcggtcccgccgagcccttggcttcgtcacgcgcgcccgcgttccaagccaggccgaaccgcgccgtccggcccgccgccggcaggaagatctgcaccagcgccaggaccagcgtcagggccagatagaacagctcggtcgtcaacgccgtcagccctgcctgtagttcggcgcctcgcgcgtgatcatcacgtcatgcacgtggctttcacgcaggcccgcgccggtgatgcgcacaaagcgggcgcgttgctggaagtcgtgcaccgtgcccgcgccgacatagcccatggaggcccgcaggccgccgaccagctggtgcagcaccgggctgatcgggcccttgtagggcgtctggccctcgatgccttcggggaccagcttctcagacgacacctccttctggaagtagcggtcggccgagccccgcgccatcgcgcccaccgagcccatgccgcggtatgacttgtaggagcggccttggtacaggaagacctcgcccgggctttcgtcggtgccggcgaacatggagcccatcatggcgacgttggcccccgctgcgatggccttggccagatcgccggagtatttgatgcctccgtccgcgatcaccggagcgcccgagtccctggcggcgcgggcggcgtccagcaccgccgtcagctggggcacgccgacgccggcgacgatgcgcgtggtgcagatggagcccggcccgatgccgaccttgaccgcgtcggcccctgcgtcgatcagggcgcgcgtcgcgtcataggtggcgacgttgccggcgatgatctggatgcggttcgactcgcgcttgatgcgctccacgacctgagacaccgaggcggagtggccgtgggcggtgtcgatcaccaccacgtccgcgccggcctcggccagggccatggcccgctcgaagcccgcgtcgccgacggtggaggcggccccgaccagcaggcgaccctgatcgtccttggcggcgttggggaaggcttgggccttctcaatgtccttcatggtgatcaggccgacggcgcgatagtcgtcgtccaccacgatgacccgctcgatcttgcgggtgcgcagcagttcgcgcgcctcgtcgcggccggcgccctcgcgcaccgtgatcaggtcgccggtggtcatcagcgaggcggccgtgacgcccggatcggactcgaagcgcatgtcgcggtgcgtcagcatgccgaccagctttccggacgcgggatcgaccacggggaagccggtgatcttcttgcgcgtcacgatctctcggacctcgcccagcgtcgtgtccggcgtgaccgtcaccggattgacgaccatgccgctttcgtagcgcttcacggcgcgcacctgctcggcctgctcctcgatcgtcatgttgcggtgcagcacgcccagaccgccggcctgcgccatggcgatggccaggcggctttcggtcaccgtgtccatggcggacgacagcagcgggatgttcagccggatgtcgcgcgtcagctgggtcgaaacgtcgacctcggccggcatgaactcggacgcgccgggttcgagcaaaacatcgtcgaaggtgaggccttcgcgtatctccatgaggagtctccgttttgcgggccgcgtatagcgggcgactcgcctcagcggcaaggtctgtccgttatgcacccgatacattttattggtttgcaaccctgcgcggctgacaccattgtcgttacatggtcggcgtcctgctcagcaccgcacgcaagctcgctttgaagatcgcgtcctacggggtcatgcacctcgtggtcgcgatcctggtggcgttcgccctgacgcgcgactggcgcgtggccctggcggtcggcatggtcgaacccttcttccagaccatcgcctattcgattcacgaccgggtctggcaccgcatcgagcggcgcaggcgcgcatcccggatcgaagaggcggccgaggccttcaccgcccggctggaggtcatgtcgcccgaagagcagcagcgcgcgcacggcggccatcatgggcacagccacgccctgccccgctcgctcaagcaggtggcgctgaagaccgtcacttacggtctgatgcacttcgccgtcgccgtgacggtggcttacgccctgaccggcgacatccgcacggccctggcgatcggcatcgtcgagccgatggtccagacggtgttcttcaccctgcatgaccgcatctggacccgcatcgaggcgcgccgcgccgcccgtcgtcaggcgctgaccgcctagcgccggttcagggccaccaggaaaacctcggccgagtccttccggctggaggcgggcttcacgtatttcaccgtctcgaactcctcgcgcaggcgcgccaggaccccgccggcgtcgccgccctggaagttcttggacacgaaggccccgcccggcttcagcgtgcgaatggcgaagtcggcggcgatctcgatcagggcgatgatcttcaagtgatcggtctggcgatgaccgatggtgttgtgcgccatgtccgacagaaccaggtccggcgggccgccgatggcgtcgatcaactgctggtccacgcccggatgggtgaagtcggcctggatcagggtcgcgccgggaatcggttcgatcggcaggaggtccacgcccgccaccgcggccgcgccccgatccagcgccacctgcacccagccgccgggcgccgcgcccaggtcgatgacgcgcgacccgcgccggatcagccgatgcttgtcgtcgatctcgatcagcttgaacgccgcgcggctgcgccagccttcggcgcgcgccttttccgaccacttgtcggacagctgacgcttgatccactgctggctcgacatcgacttggtgtcggccgtcttcatcttctggcccatgccccgaccggccgccgttccgccgctgggcggccggaccatgcggcgacgctcgggcgcgccttcgggcttttcctcttcgctcatcagcaccacatagccctgacgtgcgttgcgggctatgtcccccgcgcacatccgccacaacgaggagagcgcccgatggccgagaccctgactttcaccctggacaccggcgatggcgaagcccgcgacgtggtcatcaccctgcgtcccgacctggcgccgaaccacgtcgcccgcatcaccgagctggcgtccgaaggcttctacgacggcgtggtgtttcaccgcgtgatcccgggcttcatggcccaaggcggtgatccgaccggcaccggcacgtcgggctcgaacaagccgaacctgaagcaggagttctcgtccgagccgcacgtgcgcggcgtctgctcgatggcccgcacgtccgatccgaacagcgccaactcgcagttctttatctgcttcgacgacgcgaccttcctggatcgccagtacacggtgtggggtcaggtgacctcgggcatggagcacatcgacgccctgcccaagggcgagccgccccgcaatccgggcaagatcgtcaaggcgactgcggcctaagcgccgatcgatacaacggccggccgcccttggcgccggccgctcccttccctctactcctgagctggcgcggccagctcgaacgggaccgccggcaggccgccggggccgtaaaggttgcacagcggactgtcgccccagcagaaccgaaccttggcgtcggacgcacgcgagccggccagaacgacctcgtcgccttccagcgccgcatccacgaagcgacagtcttcaccagcgtcgcagagctggaagcccacgggacgactggcacccaccacgatcaggccggcgtcgtcagcgtatcggacacgcagctcgccgcccacgcgccgaacgccctcgggctggaccgggcgggcgatcgcttggccatccagccgcctcgcctccagcgccaatcgccggccgacctcctgcttgttggacgggtggatgtcgtagcggtcgcccacgtcgatggtcaccgccagccccgccttggcgtcagtggcgacggtgcgccgctgcacctcgcgcagggcggcccagcccgacgcctgcggccggtcggaggcggggccgtagttggccagctgcaccaccagcatgcgcaggtctggattgtcgaagacgcgtcgccaatcctcgaacaggccgggcagcaaggcggcgtagcccgccgcgtcgccggcgttggattcgccctggtaccaggcgacgcccttcaggccgtatggcgcgacgggcgcgatcatgccgttgaacagggtgctgacgcccgatccgcctacccacggcatgcgtggagacggcggcagacccgccagcggcgtcgccacccggtgcagccaggggcggtccagcggcacggacgatccgtcgtcgaagaccagcctcttgtcggccgccggtccccaggcgccgccgccgccgccgctgtccagcacgcccacggcgatgacgttgcgccccgccttcagcgagcccgcgcggatgcggtaacggcgtggcgtgtcccatccctgcatgccgcccagatagcggccgttgatccaggtgctgtcggcgtcgtccaccggcccgatgtccagggtcgcggcctggcgcgcctgcgcccgcgtcagctcgaccgtggtcctcagccagaccacaccgtcaaaggtcgccagatccttttgcgtcgtctcccacgcgccctcggcggcgatggggcgccactccgtctcgtccagccgctcgcggtaccagccgctctggagacccggatcgtggctgcgccaccaggccatggagatgcgctgccacagcgcctcgccctcctccggtgagcggacataggcgtccagcgcctgcaatgacggttgataggcttccatcccgttcagggcgtcccggctcagccagtcctcgatgatcgaaccgccccaggacgcggcgatcaaaccgatggcgacgcctggatcgttgcggcgcagatcgcgcgccatgaagtagcaggcggccgagaaattccgcgcgctgtccggcgtcgtcggcgtccaggcggcgagggcctgcggctcggccgccgcctgcggcaggctgcggcggggaatgttgaacagccggaggctggcgtcgtcggccgcggcgatctcggcgtccgcattggccgcctggcgcagcgtcatctccatgttcgactggcccgaacacagccacacgtcccccaccagcacgtccgtcaggcgctggctcattcgcccacgctgaccaccagcgcatgcggtccgcccgccctctgcgcaggcagttcgatgcgccagcgcccggtcgcgtccgccgtcgccgttgcgttcgccgtattcagcgacaccgtcacgcgcgtacccgcctccgcccgcccccagatcgggatcggccgcccccgctgcagcaccgcatgatcgccaaagaccggatcgagcagcgtcggcgaggcgacggcgatcgaggattgaacgtccgcctcctgcgcttcagcggacgccgcatcccccgccgccgctacgaaaaagagcgctacggccgaaagcagcatgaaacgcaaatgtgtctcctcgcggcggcgatatggatggatcatcggctataccgcagcggccctctccacgccccatcaaagtccaaggcgatgcggcgccgcccttggcgtgacgcggatcaccgccatctccagccggtccggccatcaggatgagtgagcgacacgagtcgttcactcatcgctttctgcgctcgatgggtggtcgtctgagccttaccgcgcaggtgcgacccgccagatcgtattggacacgtcgtcggccaccagcagcacgcgcttcgccggatcgaacgccacgcccaccggccgtccgcgcgcatgctcgccatcgatgaagccggtcaggaagtcgacgggcggcccggcgggacggccgttcgcgaacggcacccaagtgaccttgtagccggacaggtcctgccgattccagctgccgtgctcgccgataaaggccccctgcgcgaactggccgccgaagccgccgtcgcgtgcgaaactgaggcccagcgccgcgacatgcgaccccagggcgtagtccggcgtgacggcgcgggccaccatgtcggggttctgggggcgggcgcgcggatccacggtcttgccccagtagctgtagggccagccgtagaaggcgccgggccgcaccgccgtcagatagtccggcacaagctgcggtcccaactcgtcgcgctcattgaccacggcccaaagggtgctggtggtcggctcgatggcgagggctgtgggattgcggatgccggtggcgatggtgcgatgggcgcccgtcgcgcgatcgatctcccacaccaccgcacgatcctgctccaccgccatgccgcgctcgccgacattgctgttggagccgatgccgacatacaggcgcgttccgtccgcgctggcggtcagggccttggtccagtggtggttgatctcggatggaagcttggtcacctcctgtcccggcgtggtgatctgcgtctggccgtcttggtaggggaaacgcagaagcgcaccctgctcggcgacgtagatcgacccgtcgacgaaggcgagcccgtacggcgcatccaggtcggcgatgaatgtggtgcggacctccggctggccgtcattgttcgcatcgcgcagcagggtgatgcggttgccgggcttcacgctgctcttgcccttggccttgatgacgccggcgatgaaatccttgggccgcagcttgggcgcatggccgcccatgccttccgcgaccaggacgtctccgttgggcagaaccagcatctgacgcggaatggcaaggtccgtagccatggccgttacggtgaagccggcgggcgcagtcggcgtctggccgtcccaccccgcgggcgtcgcgatcttcatgggcggaaccagcgtctcgttccggccgggcagttcggggtttgggccggtctggttgaggttcggatcactgggtcgtccgcaggcggacagggccagcaccattgcggtcgcgccgagaagggacttcatcatcaggcgatctcccgcaccttggaactggaaaaggcgatccatgcgccggcgagagccaggccggccgagaggatcgacagcagcagaccgccggtccccaccgaactccaggcgtcacggctgtgatggaaggcgttggccaggccgaggaaccaggcgacggccagaaggatcacatagacgagctttcgcaccggcctgccgcgccggaaggacaaggccagatcgataacggcccagagaccgaagaagccgccaaacaccagtccgccggtgatcagccaggaggcgaagttcgaccactggatctcggccgagcgcagataggcgacatccgcgatcagcgcgcaggtgaacagcgaaaccagaaaggccagaaggatggcgtgtagcggatgcagaggtcgccccctgtcgattgctgcggtcatgccgtcttcccttccctaaggctgagctttgcgtatcggatgcaaatcccccggggcccgattggttcaacagccttgccggaccgggcccggtcggcgagacgctcaaccttcgcgaaagcctcacacaggcgtcatgaaccgccggaacaagggcgcggcatcgagcccggagtgtttccatgcccctgaacagacgaagcctgatggcgagcggagcggcggcgctggctttctccggtctcgggcggcacgccctggcggcggcgcaggagacctatgtcaacgaggtcgcgggctacggtccgctgaaggctgatcccgccggcatgctcgatttgcccgagggcttctcctatcgcgttctgtcgcgcgccggcgaggtgatggacgacggtctgctggttccgggccaattcgacggcatgggctgcttcccgctggagggctccaaggtcgccctggtgcgcaaccacgaactgaagccgtcgtcggcgtcgcactggacgcgcacggcctgggccgatgacgccggccggctggagcggatcgatccggcgcgcgcctatggcgtgaccaaggacggccgcatcgtgccgggcggcacgaccacgctggtttatgacatggacacaggcgtggtggagcgccagcacctcagcctgatcggcaccagcaccaattgctgcggcggccacacgccctggggctcctggctgagctgcgaggagacggaggatcggccggagaccgccgacgtgtcgcagagccacggctgggtgttcgaggtgccggcgcgcgagaccggcctcgtaaagcccgagcccctgaccgccatgggccgcttcgaccacgaggcggtgtgcgtcgatccggggacgggcgttgtctatctgaccgaggatcggtccgacgggctgttctaccgcttcatcccgaccacgcccggacggctggcggagggcggacgccttcaggccatggcgctgaaggatgcgccctccgccgacacctccaacaggacacagcgcctgtgggcggtcggcgactggcgcgaggtcgaatggatcgacatggaggacgtccacagccccaatgacgatctccggatgcgcggccatgcggcgggcgcggccctcgtctcgcgcggcgagggcgtattctggggcgagggcgaactgtacctgaccgccacatcgggcggcccgatcgagcgcggccagatcctgcgctatcagccggcgggcgaggacggcggccgcgttcagctgttcgtggaaagcacggacgagaaggcgctgaacatgggcgacaacctgacggtcgcgccgtggggtcacctggtggtgtgcgaggacaactattcgccgacaatccacaaccacgtgaagggtgtcgacgcccaggggcacctctacaccatcgcccgcaacgtggtggaggggaacagcgagttcgccggagcggtcttctcgccggacggacgcaccctgttcgtcaacatccagaaccccggcgtgacctatgcgatcaccgggccgtggggtcggatcagcgcctgatccgacgcccggacggcgcggcgaggctgcgcagctcggccacaaaggtcgggtgatccgtcgcttcaccgtcaagacccgacgccagcgcctccgcttcggcgatcaggccgaccacctcgtcttcccccagaccgacgcccaggttcaccagcgaccgggcgcgggcgcgcaacagcagcagagcggcgtgggggtgccgcgccgccagccgcgccgcccaaaggggcgtatcctcgtgcgccccgcgaagctgctccgcgcgcgcaatgatcagcgccgccgcctcgcgcaacgccggccagttcatcaggaaaccgaccgccctcatcacatccggatgcgcggccgcgagctcgaacgcccgatccagggccaccacgtcctcgaagtcggcgagcccttccagcagcgcgcgcagatcgttggccgagagggtgcgttcgaacactcgccatcgggcctctcgcgcgtcgtccagccggccttcggcctccagcaccaagacctccgcctccagccacgcctcggcggccgatgcgcggccggcacgcccgtgcggcggcgcgcccgccgaccggctcgcctccagcgccgccctcgcctcttccgcccgtgcggcaagggcgaagcgtcgcgctatctcgatggtgacttccggcttgcgcaggtcgtcgggcgaataggtctggacccaagcgtcgagatcgccgctgcggttcgccagtcggcgcagcaccagcgccatgcgcccggtcggcggcgggcgatcgtccatgaactcgaccaccagccgacccgccaaatcaggctggagggtctcggccgcatgaccgatccagatcgcccaggcggtcagccgcgtcgacagcgcctcggtgaagacggcggccgaggcgtcgacgccggcgttcacagacagcgcggccaagtccgtcgtcgccgcctcgaacagcagcggcagttcgcccttggcgtcgctgagccgcgcgctcaggcggggatagaggtcgaaccaggcgaccagccggtccagccctaagctggcgtccagctcggccagccggtccacgatgatgcggcgcagggccctgagatcggccagcagcgccggccgcttgcgccacgacacccgcgtcttgctggttgcgagcgcggtcagccgcttgtcgatctccagcgccagatcggcggccccgatctcggccgccagttccatgcgcagtcggcgcttgagattggcgtcagccgaagccgcctcgagcagcagggccgcgagcctgtcggcgcccagtgccgctaggttgtccgaagacaccgtctttctcgccgccgaagatcgcttggccatgcccgggttaagcgcgggggcggcgtccgaggcaaggccggacgcctgatccaggcccggagaccgccgatcaatcctccgcaggatactcgaacggatcgctgggcgtcggctgcgtcggcaacggcatgcgcggcaggggctcgtcgcggttggccgcgttcagcaggaagctggccaggatgaccgccgcctgacgcagatcctcgggtttcaggtggtcgtagctgtcgatgctggtgtggtgcaggcggctggaatagtcgagcgggtcctggatgaactgatatcccggaatgccgacggtctgcatatagacgtggtcggtgccgcccgaggggcgcagcgacacggtggtcgcccccatgctggcgaatggcgccagccactcctggaagatcggggcggcggccacattgccctcggcgttgatgccccgaatcttgcccgacccgttgtccaggttgaagtaggcgaccagatcacggtagcccgcgcgcggctcgatcggccagcggctgcgccaggtgcggttgttcggaagattggccagcgccgggtcgttcgacggtgcgcgcgtcgccaagtgccggtccacataggccagcgagccgaggatgccctgctcctcaccgctccacagggcgaagcggatggtgcgcttgggccggacgcccagcgtcttcaggatgcgcgccgcctccatcaccaccgcgctgccggccgcattgtccaccgcgccgtccgatgcgacccagctgtccaggtgggcgccggccatgacgtattcggtcccgcgcgccgtgccggggatgtcggcgaggatgttgtaggcgttcacgtcctcgtcgtggaagcgaacctcgctgttcagctccagcgtcgggggcgtgtcggtcagggccagccgggccaggcggcgatagtcctcggccgccagctccatgccggctagcttgggagtggcgccgacctgataggtgtagcccgtgccgtgcagcaggccgccgtcgcgctgggagatgcgcacccaggccaccgcgccctcctccgccaggaaggcgtcgagctcggaggcgaagttcgccgtcttcagctggcgctcgatggacgccggcgaatactgcggctgaacatagacgttgcgctcggccagctcggcgctggtccagcggcggaaggccggttccgtgggctccgatcccgtgcccggccgcgacagcatgacgatcttgccggcgagcttgccgcgccactcggcgaagtcctcgacctcggtgatgggcgcgaccaccacgccggcgctgatcaccccgttggtcgagggagtccaggccacgggaatggcgcgcaggtcgatggagcgcgggctggtcatgcgcgcgctggagcggacgatggaccagccccggccgaactcaaagccctcggcgcggacgtcgctgaggccccagtcgcggaagcgctgctgcgtccaccgctccgcttcccgcatctggggcgagttggtcatgcgtccgccgatccgatcggtgaggtgcgcggcggtctgcatgacctcgctgtggttcagcccctggtcgatgatgccgttgatcgcggtgcgatccaccggttgggcgacggccggcgcgctcagcagaacggcggcgacggacacggaggcaagcagacgcagcatgggtgacctcttggaatcggataggccacttcatgaaacttatcgcgcccgcgcaactgcaaaggtgcggcacgacggacgcagctttggtcgcgcagctgcatcggcgccggttggggcagaaaacccgctgatcacgagccgcgcgtcggccactttcctaatcggcaagtttcaacttgacggaatggaaagtcacccccattttccacatcagcaagtcgccagggaggaagcggtgatgatcgaaggtttgtggctgaccggcatgctggccggcatggcgtggtgggtgaagcgcgacgcggaggcgtatcgccgctttcaggcgctgaccctcacccgagatcgtcagcgggtctattggcgctggatcgcccagagtttcgccgtcctggtgggcgcaagcctgatcagcctgtggctggtcggcggactgtcgcccttcagccccttccccagcgcgtttgatcaggcgcatcaggccctgcgcagcccgcaagccgatggatcggccgaatccatggccggcatggcggtcggcttcgccatcggtatgggcgcgctgctgttcatgcaatggcgccggatccgcaagatgctgaagccggtcgccgtccctgccgacgcgctgttgccgcgcaaccggcgtgaggcgatgatcgcggcggtgctgagcctcaacgccggcttttcggaggagctgttcttccgtctggcgctgccgctgctgctgcttcacctaaccggctcgctctggatcgcctttggcgtggcgggcgtctgcttcgggctggctcacgcctatcagggctggaagggcgtgctggcgacgatgatggcgggcggcgttctcacgctcatctacctgtcgcacggatcgctgctgcgggtgatgctgatccatgcggccatcgacatcgtggcgcttctggtgcgcccggcgatcaccgaatggctggcgcgtcgcggccgaccggagatggcgaacgcctgagttcgcccggtcacacccagacaagcaaacgcctgccgccggatcagcccgacggcaggcgccttggagtcgatgtctagaaccgcgccgtcaggctgaccgaagcgctggcgcccaggtcgtagttgttgatgcggatcttgttgccgagctcctgatactcgtcgaagtccgtctgcagcagattgcgcagttcaagcgcgaagccgaggtcccgccctcccgccgtgaagtctttgcggtagacgaaatcgaggaacacgccgggctcctggatgtagtcgggctcgcggttgcccgcctggccggcgccgcgggccgtgatccgctcactgacatagttgacgatgatcgtcgcctggctgcgcgccgcgtcgtcttcccagcccaactgaaggttggcgacgtgttcggactgcccctgcagacggctaccgtcctcgatgaagaaatcggcgggagaagttgcgccgccgcccgagaggtccagcacggtgtcgccctcctccacactcacctcagagtcggagtaggtgtagttgccctgcaccagccagcgcttgttcgagatgaacggcatgccggcgctagggaactcccaatacttcttcacctcgaactcgacgccgtagatgtcggcttcgggcgcgttgacgtaggactgctggcggtcgcctgtcgaggcggcgatgatcaccgactccaccggcttgtcgagggtcttgtagaagacgcccgcggtcacatactgctggcgtgcgaagaaccactcgtaccgggcgtcgacgttcaacagttccgtatcgacgaggaaggggttgccgatgaaggtccggtcgctttccgggtccgtgtaggtctgcggcgccagctcacggaactgaggccgtccgatggtcttggatgcgccaaggcggccctgctggttctcggcgaagttccaggtcgtggtgaaggacggcagccagtactgttcctcgatccgcgtcgccgggaacggcgacgagccgccgaagagatcgcgggaaaccagctcctgctcgccgtcctcgaagcgaacgccgatcgcggtgcggaccagggggatgatctcggcgtccaccatggcgtaggcggcattgacggtcaggctgccgtcataggcgttggcgcccgacacgcccgggatctcccgcagctgcaaggtcgtgggattgatgttgaagtccgacgtcaggaagtcgatgcgcgactcccgctgatcttctgtcagggcgttgacagccgcgaactgaaggtcgcggcgaacggcgtcgcggttgttctccatcgacgccacgccgatgctgaacctggcttcgcgcgcgtccgacagcggcagggtgtagctgaggtcggcgccgcccgagacgacatcgtcgttcagttcggagaacgaaatcaggttaccctgaatgttgtggatgaagtcgccctgggcgttcacgccgtactggaagcgggtctcatacggggcgtcgcgttcggtcttggcgtaggccgcgcgccagtcgaactcaagcgcgccgtccatgaagaagtgctcgccggccaactggctgctgaacagctggcgctcgaaccactcggtgtagtcggtacggatgatcgagccgccggcgtcgaagttcgggccgctggcgctgcgcgcctccttggtggtgttgcggacgtacaggttggtccacttcacctcgtgatcgccgttggtcagcgacagtccgccgaggaagttcagttggacgtcgttctggttggactcgacgtcgtaggtggtgacggggaccagcacgtcgccttggaactggccttcctcctgcacaccctcgcgcaggctccagttgttgtcgtagccggccacgccgatcaggcccagcgtgcccatgcccgtgtcggaggacagaccgcccgacatctcgaccccgaagttcacgggcgtgttgtcgcgttgcagcaggcgcagcggcgcgttcaccagcgagcggcccatgacctgcagctgctcgggcgagaagttggtggtgttgatctgacgaccgctgcggaaggcggcctggatctcagccggcacgtcacgcgtgccgtcgtcgaagctcgtgaagtcggtgcgcgagccgtagtaggtcaggccgttctggccggtcgtttcggagttcacgcccagcgacgtctgcagggtgaagaacggatcgcgcggcgcgtcgatcgtgtgcaggtcgatcacgccgccgccgaactcgcccggaaagttggcggagtagctcttctgaacggtgacgccgtccaggatgctggagggaaacaggtccaggggcacgacgcgctgcagcggctcggggctgggcagcggcgagccgttcagcagggccgatgaatagcgctcgccgaggccccgcacatagatgaagcggccttcaacgatcgacaggccggtcacgcgcgtcagggccgcggccgcatcgccgtcgcccgtgcgttgcagatcttcggcggtcaaaaaggacgcgacctcggcgctttcgcggttcggctcaggaatgtagcggcccagcacgacgatctcgtcgaccgaggccggctcctggctgtccgcctgaggctccgcctgaacggcgggggtctgggcggtcgccgcgtcctgggtctgggccagggcgaaaccgggcgcgatcatcgcgctggtggccaggaggaccccgctcagggtcagagatagcgtcttcatgatctgcgccttgaagggggtcggtcgatatcgaacaggaacggcataggccggcgacgtgaggtcacgccgccggccggatgctttcagcggatcagcaggtcgcgccggcggtcagaccgcaggtccagccctgccaccaggtgtcggccgagttccgaaccgcgccgatgtaggtgacggtgtcgaagaagctgtagaccgacttcggatcgatcgccgtaacggcgttctcgttggcgccgttgatgaaggccaggttctggttggtgatgctggttcccgtcggcgccgtcagggtcgaggttccgttcgccgtcacattggtgttgcgggcgttggtgaacaccgccgtcgagcgcgccgcgttggtgggacgataggcgatgctgcacgacatatagatcgagcgcagcgaaggctggctgttcccatcaaagctggtctgcgtatccacatcggcgatgtcgaagcagccggccgtcgatcccgagacgctggtcgagacgatgttcatcagcgtcggctgggtcccggtgtcgaaatgcatcacagtgtgcgcatcgatcggcgagttgcggcccaccaaggtccagttcgcgatcttgggctgggccaggtagcgcgaggcgtaggcggtcgaggtgggggcggccgagaactcgaacgccgccgaacggctggtcgagttgggcgcgcgctgggtcacgatgccgaactgggcgccgccgcgccagccggtgtcggtgtccagaccatcgtcgtcggcgccgttgatgacgatgtacttgaggttggcgttgccgccgaagatttcgatgccgtcgtccgagctgttgtagacttggacgtggtcgatggtggtgcccgagccgacgccggccagggtcaggccttgcagttcgttgccgaccgagacttcaaagcccgagtacttgatctggacgtagcggaagcggcccgagttgtccgtggccgtattgccgccgtagaacacggcctggccgccctcgaccgttccggtgcaggtcaccggagccgtcagctggcagttcgcctgaggcgcccggccggccatgatgatgccgccccactggccttgcgagctctcggtggtctggccttcgatgttctggcggctggtgaagatgatcgggttggtcgcggtgccttcggcgtaaatctgcgagccgcggttgatgatcagggcgtcgccgccgctggaggcgaacacgcgcacgcccggatcgatcgtcagaatgccttgagaacccgtggtggaggtcgggtcgaggccgcggtcgacgccgacgttcactgcgcccgagatcgagtagatggtgccggcgcgcaccgacagggtcaggttgccggtgacctgctgcggcagctggcagttgcgcagcgtgccgttggcgacggtgccgacgttcgcgaggcccgtggggcagtcggccgctgcctgacccgtccccggattggggttcgggttcgggtttgtcggattggtcggctggttgccgaagtcgccttcgcccggcgaggccacttccgaagagccgcaggcgctgagcgcgagcgcgctggcggcgaccgccagcagagatttcagtcgaaggtcggtcatcatcggtcccaccgtgtctggtcagatttcatcgacaggtgacggccggaacccatgctccgaaccacgaagccgtggcgcccctcctgccctcgccctgcctagagcgacgatgtgacggcgacgctgacctagcgtgacagttgcggcgagtttttttgacaaggaagcgcagctttcatgacgtgtatttgagcaagctgcagtgcacggacgatccgcgtcgccgatgggcgaccgcgacctgccgcatacgcgcgcctgtgcgtgcgtccgcgccagggatcgcccgctgacacgaaatcctcgtcaacgcgcggtagtgtgatcccgtcggtgaagaggcgagccatgactgcgaactccccgggcgcgacggcggccgctctgctggcgttgacgctcgcctggcctcaatctgcgtgggctgagcctctcgccgatgcaccggtggacgacacgccccggcgctatctgatgatgctgccgcagacgcccgttgcggagatcgccgaggaggtgctgggcgagaccctaggcctgccggtgacgacggacgaggcggtggacgcctccatgcccttccgcatcgacggccagtacacgcccaggcagttggcccgcgaactcggctaccggctctggaacgtggacgtggccctgatcgaggaagcgggcggagagttgaagctgatcccggccgccggcctgccgggcgccgtggccgacggggcggaggtggtcgcgccgctggcggtcacggcgcccgccccgacagcggcacctctccaacgcacccccattgtctatggtcgggaccgcttcaacgcgcgggacctgatgatgctggccttgggctggctggggggcgcggcgagcctcggcggttggattgccgtgcggcggcgtcgcgggccccgtcaagccgcggcgccggtcgccctcctggcggcgccgtcttttccgaccgtcgacctcaagcccgaccccttcagcatacccgatcgcgcgggctgacgcctagggtccagactcataaccaccacgcgatgatggcggcgagggctatggcggcgatgtaggtgcaggcgagcttgtcgtaacgtgttgcgacgcggcggaagtccttgatgcggcagaaggcgcgctcgacgagggtcctgcgcttgtagggctccgggtcgaagggatgcaggcgctttcggtaaggggcgttggggatgaccggctgggttcctcgggccagcagcagacggcggagcgcgttggagtcgtatgcccggtcggcggcgagggtggctgaggcgggcgcggcctggatcaggtcggcggcgaccggcgcatcgccgcgctggcccggggtgatgacaaaggcgaccaggcgaccgagcccgtcgaccagggcgtgcagcttggtggtcggcccgccgcgcgagcgacctatgccgttggctgaagccccccttttccgcccgtcgccgagcggtgtgccttggcccaggtcgagtccagcatcagctcggcgggcggcccgccggtggccgccagttcctcgaacgcccgccgccagacccccgccttggcccagcggacccagcgattgtagagcgtcttcctgggtccatagaccgccggcgcgtcgatccagcggccgccgctgatcagcacatgaatgatccccgagatcacccgccggtcatccacccgcgccacgcctcgaggcttgttcggcagcagcggtcgcaaccgctcaaactgcgcgtcagtcagccagaactccgaagccatgtcggttctcctgcatccgactgcaggaaatcacgcttcggccaatcagggaatcccgtttatgggtccagaccctagcggtcgctttgggtcgaaagccgccctaagcctcctccgctccgctgtgccgatgcgggcacccgggccagcagcaagggcggcgtttgccgtcgtgcaggttggaacagccccaggcgatgcgcttccttcgggtctcgggcttcttggcggactcgatccagcagatccattcgttgcgagccagaggcgtgatgtccagccaggtcgacaccgccccggcgtccagcgtcagggctgcctgaaaatcttccggcagatcgtggacgacgccgccgggaagtgcgctctgctcagccatgtcgccttgtcgcagcggccagccaagcctgcaacaggacgggccgcgatcccgctcttcctgctggacgggaagagagccataacccgcccgccctcgcatctgcggcgacaaactcgcgcctgaacaacaccttgggactttctcactccgacttccccgcctgagctcccgcccgtgccatcctgcacccgtcttgtcgcactggaggctcgcctggcctgcgaccttgcgagcggcgggagcggatggagcgggaggggttcggtcaggtcgatcgaacccgccggcgtcggggatcgcccggcgtcgagagggtcgagggggatactcggccggtccagggacagcctcgcagggctgcctgcccgccgcaggcttatggggttaggcgataagaccgccaccatcctccgccccgagcttgcagccaaccacccgcgcggggcgtcgaaccttcgtcgaaacggtacacaactactcaatcttcgggcgaaggcccggcgccccgcccgccctccaaccggatgcatcagcagaccggggctttcgcgcgcctgcggttccgtccgccgtccggagcctgtaggtcacctgtctttacgccgccgcacgccgcatcatgtccgaccccgacgatcttccacccgaccttcgtgccgccctgctcgatgtcggccgggcggcggaggcgctgcacgatccgtggtggatcttcggcggggcggcgctggcgctctatgggatggaggcgcttcacgtgccggacgtggacgtgctgtgctccccgcgcgatgcgcgccgcctgatccaggcactggggggcgagatcgagcccgatcccggcgagggcctgttccgctcgcgcgtcttcggccacgccacgcccgggcgtatgcgcatcgaggtgatggccgagatggacgtgcgctccggcggcgactggacgcccgttgtcttccccacccgccaggcctttgacattcccgatgcggcgggcgaccccgtccgcgtcttcacgccgagcccgcaagagcatatctgcgtctcccgccagttcgggcggcccaaggacctgcagcgcgccgaggcgctggaaagattgatctcccgaccatgacctttcccttcgacatcaccgccaccgagggccgggcccgcaccggcgtgctgaagaccgcgcgcggcgacatccgcacccccgccttcatgccggtcggcaccgccgcgaccgtcaaggcgctgacggtggatcaggtgggggcgacgggcgccgacatcatcctgggcaacacctatcacctgatgctgcgccccggccccgagcgcatggagcggctgggcggcctgcatcgcttcatgggctgggacaagccgatcctgaccgactccggcggcttccaggtcatgtccctggccggcatctccaaggtcaaggaggaggccgtgaccttctccagccacgtcgacggctccaaacatgtgctgacgcccgagcgctcgatcgagattcaggccgaccgcatcggcgccgacatttccatgcagctggaccagtgcgtcgcctatcccgccgagaaggacgcggcgaagaaggcgatggagctgtcgatccgctggggcgcccggtcaaaagcccgcttcggccagcgcgagacccaggccctgttcggcatccagcagggctcgacgttcgaggacctgcgccgccagtcgtcggatcagctgcaggagatcggcttcgacggctacgccatcggcggcctggcggtcggcgagggccacgccgccatgtgcgaggtgctggactatgcgcccgagatgctgccggcggaccgcccgcgctatctgatgggcgtgggcaagccggttgatctggtggaggcggtgtggcgcggcgtcgacatgttcgactgcgtcctgcccacccgcgccggccgtcacggtcaggcctggacctgggacggcccgctgaacctcaagaacgcccgcttcgccgaagatcaggacccgctggacgccgcgatcccctgccccgcctcgtccgcctactcaaaggcctatctgcaccacctcgtccgcaccgatgaaatcctcggcaaggtgctgctcagctggcataacatcgccttctaccaggctctgaccgccgccatgcgcgccgccatttccgagggccgcttcgaggcgttccggcgcgacttccacgcccgccacgtttcgaacggctagggctgctggatgatgatgcgcggcggcgcgggcggctgcggcttgaaccagcgcggcgccgccggcggggcgcagttgcgctgcatgcccacgcccttcagaaaggcgcgccgagcctgaccggcctgatgcgcccgctccgcctcgcgctcgcgccggctggcgccgctgagacggcgggtccagctgcggcccgggatcaggtcggtggcggtgtcgcgaaccgcatccagcgccgcatcggccgccgcgtccgacgccctcgcgctgaggctggaggcttcgggcgccgccggctcgtcgaggtcggggccgagcgcctcgtccagcagcgccacctcctcggcgatggcgtcgcaccgttcgagacccgacatgtcatacggacgaacctgcgcccaggtcagcacgtcggccaggctcttgcggcgcaggttgagatcgtacagaggcgcgctgatcgccgcgccgagcccgtcgcgcacctgccccaccccgcgccctgcggggtggctggcgcacgcggccgtcgccatcgtcgcgccggcgacgaccgaacaggcgcagaggcgataaagacgcggccgatccgccgcgcctcgaacaatcctgccgatcaaccccgtccccgaacctcgtcgcggttggcggcgcgcgtcttggggccctgcccccggtccgcttcggttccgatgggacgattggcgtgatcgccgccggactggacgttcgcaccgcccaggtcgtcgccctcgtccagataatcgccgacctcgcccgccgccggcggcgccagggtcgagtcggccagatcgggcgcggcgtagcggctcggttccgggtgagcggcggcgttctggtctcggccctggtcgttcggcgcctgcttgtcgccgacgccgttctgcgccgtcgcgtccgacgaggtcgtgttctgatgcggcatggatcgctccttctcgaatggcttgcacaacaacccggcccgcacggggcttgttccgagatcagcggtccatggccttcgcccttgacccgggcggcctgacgcgacagaaggcgcgcaccaccgctcggtctccgggaccgcggccacggcgcgtccttagctcagttggttagagcatctgacttttaatcagagggtcctcggttcgagcccgagaggacgtaccagctcttgtttcgcctcagcctccttgccgccatctggcgatgcgaaggcgcggggcttgagcggcgatccttcggtttgacgcacatccggggaacggcggcgcttgcaaagcgttggcgtaaagaagtcggggaaatcaagtcgatgaagcgtattctttttgcattggcctcagcgggcgccttgtctctggccgcctgcgacgacgccgctgatcgggacgcggacggacgacccatggtcgtggaggccgagcccgtcgcgccggccgctgaagattcggccgcgccggtcgtcgcgcccgacgtggtcgaccccgcccccacggctcccccggtcgaaaccctgccgcccgagcccaagacctcggaagagtcggtccagcccgaaagcgaaacccttttctactgaccgcccgcgcggttcgcctcacgcacgcgccggacggtttccggccaagacgaagggttcagtttgacgtcccggccgaagcttttccttgccgcgctggcgctcggttccgcctgcgggtccgccgcccatgccgatccgcgcgcccagatccggggcgagatcgacggcgacctgcgccgccagcttgagcaggcggtcggcgaggtcgatgacgcgccgtccagccgcttcgaagcccgtcgccgcgcccgcgccgccgcggagtccgccgaggccctgctgcgctccgaaggctactatcagccggtgctggaagacatcgtcgagggcgaagagacgccggtcgccgtcgtgcaggtcacgcccggccgccgcttcgtcctgacgccgccgacggtgcaatgggccgccccgccgcccgacgaggccagcgccgccgtcgccctcgacgccattgatctggaggccggcgcgcccggccgtgcggtggacgtcatcgccggcgagggccgcgcggtcgcctccctgacgcgccagggctacgccgacgccgtcgccaatccgcgccgcgtcgtggtcgatcacgccgcctggacagtcgcgccggagtaccgcatcgcctcgggcgagctggtgcgcctgaacggcgtccggctggacaccgagggccgtacgaaccccgcctgggtagcgggcctggccccctggaacgaaggcgaccgctacgatcccgaggatgtggccgaactggagcggcgtctgctggagaccggcgtctacgacggcgtgggcgtggccctggcgacgcaggctcagaacaccgaagcgggcctgcgccccgtcatcatctcgctgcaggaccgcccgcgccgcatccttgaggcgggggccagctactccacggccgagggctcgggcgtggacctgatctggacgcactacaaccggttcgggcgcgccgacaccctgcgctaccaggcgcgcctggccagcatcgacagccgaatcggcgtggatctcagcctgccgcactggcgccgccccggccgcacgctggccatgcaggccgccgtcgtcaacgaggacaccgacgcctacgtccgccaggccctggtgctgtcggccgacctgcgccagcgcatcggccgcacctcctacttcagctacggcatcggcgtcgacgccggccgttacgatgagaatcggttcgacttctcggtggtcccgccgcagccggtggagttcaaccgcgatctcgccatcgtcaccctgcggggctcggcctacatggaccggtccgacgatccgttggacccccgcagtggctaccgcctgaccgcctccgttcagccgacggccgtggccggcgacgacaccgtgctgttcctgcgcaacgacttcgtggccaccggctatcttccggtcacggacggcggccgcaccgtgctggccggtcgcgtccgcatcggctcgatccttggcggcgaggagctgacggtgccggccgaccggctgttctactcgggcggcggcggctcggggcgcggctatgaataccagggcgtcggcccgcgcctgcccgataacacgccgcgcggcggcctgtcgctgttcgagaccgcgatcgaagtgcgccgcgacatcggcgaaagcttccaggccgtggccttcgtcgacgccggctcggtcggcttccaggaaacgccgaacttctccaacatgcgctacggcgcagggctcggggtgcgctacaagctgccgttcggacccatccgagccgacatcgccttcccgctggacgcgcgcgaggacgacgccgcctttcaactctacatcagcatcggccaggccttttgaccgacacgccgcctccccctgccgaccagcccaagcctgagaccccggcggtcaaggcgaagaagaagcgcacgcgcctgcaggtcgccggcctgatcgtcggctcggttctggcggcggtgattgttctggcgctggtcgcctttatcggcgggcgcacctatctgctcagcggcccgggccgcgagctggtcaccagcttcgtggccggcaagaagatcggccgctatggccgcatcaacgtcgagggactgtccggcgacctgttcgacgacttcaccctggcccgcgtcacggtcaccgatcgcgacggcgtctggctggaggcgcgcaacgtgcgcgtggactggagctatcttcagctcgtctttcgccgtttccacgccgacgagatcagcgccgaccagatccgcctgatccgccgcccggtgcccgagccgccgaccggcgagccgccccgccccgcccccatcggcgtggtgatcgacaagttctcggccaatgtcgaactgctggagaacttctccaaggaatacggccgctggcgcctggcgggcgacgcggccattccgcgcttcggctccaagaccgccaacgtcaacgccgacagcctcagccgcccgggcgattacctgcgcctcgccgccagcctgggcagcgagatgtcggacctgcgcctgaacctgcgggcgcaagaagcgcagggcggccccatcgccggcgcgctcggctattcgccggaccagcccttcgccgcccacgccctggtcaacggcgaggtgatcgacgcccgcgtgcagacggggcagttcacgccgctgacggtcaagggccgcttcggcgaaaacggcgggcgtctgtccggctatttcgacttctccggctccgacctgcttgagcccttcgtcacccgtgtgggccccacagcccgcttcggcttcgccatcgtccccgacggctcggacgacgcctttcagggtgtggcttgggtgctggacgccgagaacctgacctcgcgcgctcggggcaagctgcgcaaagaggaccgctcgtctcccggcggcattgcgcttgaggtcgcaacgccctcgctgacccgcctcgcaggaaccgagatcgccggccccaccgcctacagcggcgtgttcaagggcgacgcccagacctggagcctgtccggccaggccagcctgctgaacgcctcgctggccagctatcgcgcgacccgcatcgccgggccgctgaacgtccaggcgcgcgacggccgctatgacatcgacggcgacatccgcgcgacgggcggctcggccgagggcgtgatcggcgccctgctgggttcacagccgcgcgtgcagctggaggccgcgcgcatgaaggacggcgccatcctgctggagcgggtcgatgcgaccggccaggcgctggcgctgaacggctcggggtcccgcaacctgctgggcgggctctccttccgaggccgcgccgagatcaccgacgtgtcgcgcatccgccccggcgcgcgcggcgccttcggcggtccgatccaggcgtcttccgcccgcaccggcgcgccctggtccctgcgcttcgacggacgcggacgcggcctcgtcaccggcttgggcgaactggaccgtgtgctcggccaacagccgcggctgcagctggcgggcctgctgaacggcggccgcatcgagctgaaccagggcgagctgaccggcgccgccggccgcgccgccgcacgcggtctgatcgagcccgagggccgcctgcgtctggcgctgaactggaccgcccagggccccttcaacgccggcccggccgagatcgccggcaacctgcgtggcgaaggcgccgtcaccggcaccctggcccagccgcgcgcggacctgaccgccaacttcgaccgcatcaccgccggcgcgcttcagctgaccaacgccgacctgacgctgagcttccgcaagggcgccgacgcctccgacggccgcattgtcgtcacctccggctccaactacggaccggcgcgggcggcgggcaacttcttcctgggcgggaaccagatccgcctgacgcaggtcgatctgaacgccggcggcgtgacggcccagggcgccgtcgctctgtcgaacaatgtgccctccagcgccgatctgagctttacggcccgtcccggcgcctttttgcagaccggcgaggcgcaagggcgcgtgcgcctgctcgacggcggcggggccgacagcgccatcctcgacgtgaccgcccgcaacgtgaagccggccgggtcggatatcgtcatccgcaatctcgtcctgaacggccgcggcacgctggagcgcctgcccttcaacctggcgctggacgtcggcggcggcacgccggtgcagttcaacgggaacggcctctattcccgacaggggaacaaccagagcgtcaccctgtccggcggcggccgcgtgcgcgagatcgccttcaccacccgcaatccggcggtggtcgccctgtccggcgacgggcgcgtggcgcgcgtagacctgaacgtcggcggcggcgcgctgatgggcgaactgcgccaggattccgactccgccgccatccaggccgacctgaccagcgtggagctcggctctctggcgcccgatcttcggggccgggcgacggggcgcgtgtccctgcgcggcgcgggcgacgacctgtcgggctccgccaacgtccccctggaccagatccgctccatcgacgccccgcgcgggctggcggtcgacggccagctgaacgccaccctgttgaacaacgtgctgcgcatccaggcctcggccgtggacgagggcgcggtgcgcgctcaagccgacctgaccctgccggtggaagcctcggccgcgcccctgcgcctggccatcgcccgcacccgcccgctgtccggcaatgtgtcgatccagggccaggtccagccgatctgggacctgttcctgggcggcgagcgttcgctgtcgggcaacgtcaatggtcaggcgaccattgccggcacgctgaacgccccgcgcctgaacggccgtctcgacctggcggacggcagctatttcgagggctcgaccgggacccgcctgaacgcgctgaacctggccacgcgctttgacgacaccaccgcctatctggagcgcttctcggccaatgacggcgacggcggcacggtctcgggcgaaggccgcatcggcctgcgccagggttcggcctccaacctgcagctggcgctgaaccgcttccgcatcatcgacaacgacctggccgaagcgcgcggctcgggcacgctgacggcggcgcgcgccaccgacggtaagatcgcgctggcgggccggctgaacgtcgatgaggccaccatctccgccaacgacctgcccggctccaacggcatcgtccgcatggacgtggtcgagatcaacaagccgggcggcgacaccgacgagaccgcccgccccgcctccaccggtggtccgcccatcgccctcaacgtcgacctgaccggccgcgagatattcgtgcgtggacgcggcctgaacctggagctgagcctcgccgccagcgtgcgcggcaccatcgcccagccggtgctggacggacgcgccaacgtggtgcgcggcgactacgagttcgcgggcaagcgcttcatcttcgacgaccggggctatgtgaccctgtcgacggacgtgaaccgcatccgcctgaacctggaagcgacgcgcgaggacccggccctgaccgccaccgtgcgcgtcaccggcacggccgcatcgcccatcatcgccctcacctcgacgccccagctgccgcaggacgaaatcctgtcgcaggtgctgttcggccgctcggcctcgcagttgtcggcgttcgaggcggcgcagctggctgcgggcgtcgcctcgctggcgggcggcggcgggttcgacgtgatcggcaacctgcgcgagctggcgggcctggaccgcctgtcattcggcggcacggcctcggccgtgaccgtggccggcggccgctacatcaccgacgatgtctatctggagatcatcggcgggggcgaaggcggggcggcggtcaatgtcgaatggcaggtgcgccgcaacctgtcgctctcgtcccagttcggcggcaccggcgacaccagcctgtcgatccgctggcgtcgcgaaagccgcgaacccggccagcgccaggaccgccgccccaaccgggagcttaggcgctaaagccgacggcgaggcccgccttcacctttgccgtcggcccgtctagggtccgcgccatgcgtatctcgaacccggatcaggccgtgctcgaccacgtcgcggcgcggcgcgaggcgatcatagaccgcgccgtcgcctggtcgaacctgaactccggcagccgcaatgcggccggcctcgccgccgtgctggatgcgcttgaggcggaaggccgtcgcctccccgcctcggtcgagcgcgtgccgacacgcggctccaccaccgtcggcgacgacggcgcggtgcggaccgaggcgcacgccgacgcgcttcggatcaccgcccggccggacgcgccgatccagatcgtgctgaccggccactacgacaccgtctatccggccgacagccgcttccaggctgtcgcgacccgcgctgacggcgccctgaacggtcccggaatcgccgacatgaagggcgggatcagcgtcatgctggcggcgctggaggcgttcgagacccaccctgaccgcgcccgcctcggctggaccgtgctgctgagcccggacgaggagatcggctcgcccgcctccgcgccgctgctggccgaactcggcgcgcgcggtcatctgggcctgacctatgagccggctctggcggacgggacgctggccggcgcccgcaagggcagcggcaacttccacctgatcgtcaccggccgggccgcccacgccggccgcgccttcgacgagggccgcaacgccgtggccggcgccgccatgatcgccgcccgcctgcacgccctgaacggcgagcgcgagggcgtcaccgtcaatgtcgccaagatctcgggcgggggggcgctgaacgtcgtggccgacaacgccgtggtgcgcttcaacgtccgcacgcccgaccgggcgtcggccgactggataacggccgagatcgacgccattgccgccgccccgccctttgaaggcctgacgctgcacctgcacggcggcttcacccgtccgcccaagccgatggatgcggcccagaccgccctgttcgaggccgtgcgcgacgccggcgccctgctcggtcaggacatcgcctggaagccgtccggcggcgtgtgcgaaggcaacaacctgcatgcggcgggcctgcccaacatcgacaccctgggcgtgcgcggcggcgacatccattcggaggccgagttcgcctggcccgacagcttcgtcgaacgcgcccagctcagcgccctgatcctgtgcaaggtcgcctcgggcgagatcgacgcgcccaaactcaagtccctgcgcctggaaagcctctgaatgctggtcgtccgccccgctggtccgcgcgacctcgactctctgctcgagctggccatcctgtccggtcccggcttcaccagcctgccggaagaccccgacgccctgtccgagcggctggagctcagccaggccagcttcgagggccgggtcgagccgcagggcgcctggtacaccctgatgctggaggacggcgacaccggcgacatcgacggagtgggctcggtcaaggcggcggtggggctgaagcggccctttttttcctttcgagtcaacaccaacacggcgtcgtcgccctcgctgaacgtcaagctgacgcaccagacgctggtgctggtcaatgagtgcaccggctggaccgaggtcggctcgctgttcctgaaggccgaccggagaaagggcggcgcgggtcgcctgctcagccagtcgcgctacatgctgatcggcgcccagccggacctgttcgccgacacggtgctggccgagctgcggggcgtcttcacccccgacggcgcctgcccgttctgggatcatgttgcgcacaagttcttccccatggacttcgacgacgcggatcggatgacgggatcaacggacaagcagttcatcctggaccttgcgccgcgtcacccgatctatgtggagctgctgccggagcccgcccgcgccgtgatcggcaaggtgcacccgcagggcgtgccggccatggcgctgctggagagcgaagggttccgccccaatggcctggtggacatcttcgacgccggcccgaccgtcgcctgtgcgcgcgaccatatccgcacggtgcgcgacgcccgcgtgctgactgtcgagatcgccgacagcatcgacgccgaactgcccgcgttgatctccacagacagcatctccgccttccgcgcggtgcgggcccgcgccgacatccatggcgacacggtgcggctgacggcggaggcggcggcggtgctcaaggtccgtgcaggcgacatcgtgcgagtgaaatcatgaacatcctccaatccatcgatcccgccaccgaagacgtcgtctgggagggcgaagccgcctcgcccgcccaggtgcagaccgctgtggaccgcgcccgcgccgccttcgagccctgggccgaccgtcctcgcgccgagcggatcgaggcggtgaagcgctatcaggccgagctcaaggctcgcacgccgcagatggccgaggcgatcagccgcgagacgggcaagccgctgtgggagaccaccgcagagctgggctccatggtcggcaaggtggacatctccattcgcgcctatgaggagcgtacgggcgagcgggccggcgacaccgcgttcggccgcgcggtgctgcgtcatcgcccccacggcgtcgcggcggtgctgggtccgttcaacttccccggccacctgccgaacggccacatcgtgccggcgcttctggccggcgacacggtggtcttcaagccgtcggaggagacgcctctgaccggtcagctgatggccgaggcgttcgaggccgccgaactgcccccgggcgtgctgaacgtcgtgcagggcggccgcgagacgggcgcggcgctgctggacgccggcatcgacgccttgatgttcaccggttcgggtgcggcgggcgcgcacctccgccgcaagttcgccgacgatccgcacgtcatcctggcgctggagctgggcggaaacaatccgctggtggcctgggacgccgccgacgccgaggccgtggcgggcatcatcgttcagtccgcctttgtcaccaccggtcagcgctgctcctgcgcccgccgcctgatcgtgccggagggcgcggccggggacgcgatcgtggaggccgtggccgccctgtccgatcgcctgaccttcgcgccctggaacagcgaccccgagccctacgccggcccgctgatctccgcccgtgcggcggccggagccctgggggcgttgcagcagcggatcgatgcgggcgccaaggtcattcgcgcttccggcccggtcgacaacctgccaggcgcctttgtgcggccggcgatcctcgacgtcaccggcgtggacgtgccggacgaagagatgttcgcccccttcctccaggtcacccgcgtctcgtccttcgaccaggcggtgcaggcggccaacgccactcgctatggcctgtcggcgggcttgatcagcgacgccccggcgaactgggactgcttcatccgccgcatcggcgcgggcgtggtcaacttcaaccggccgaccacaggcgcggccggcgacatgccgttcggcggcctgggcgcgtcgggcaatcaccgccccagcgcctactacgccgcggactactgcgcctatccggtcgccagcttcgaggcggacgcggtcaagagcatcgagggcgagatcaggggcctgcgatgacccacgccgtcgaggccaacgccgacggcctgatcgggccgacgcattcctacgccgggctgtcgccgggcaatctcgcctccagcctgaaccggggcgaggcttccaatccgcgcgcggccgtgctgcagggtctggacaagatgaagcggctggccgacctcggcctgccgcagttcgtgctgccgccgcacgagcggccggacatcccttttctgcgcacgcttggcttcagcgggtccgacgcccaggtgctggagcgcgcctggaaggacgcgcccgccttcgccgccgccgcctgttcggcctcgtcgatgtgggccgccaacgccgcgaccgtaacgcccagcgccgactccggcgacggctgcgtgcacttcaccccggccaacctgcacaccaacctgcaccgctctctggagcacgggcagacccggcgcgcgctggaggccctgttccccgcccccgaccggttcgccgtgcatgacgccctgccggcggtcggccatctcgccgacgaaggcgcggccaaccacgtgcgcctgtgccgcgaccatggcgagccgggcgtgaaccttctggtctggggccgcgacgcgttcgagctctgggacggaccgtatcccgcccgccagacccggcaggcctccgaggcggtcggccgtcgccacggagccagcggcgtggtgctggcccagcagggacgggccgccatcgccggcgggacctttcacaacgacgtgggctgcgtcggggcgctcgacaccctgttccaccacgaactggccttcgaggacaccgcccggacgcgcccggacatccgggatgcggccaaagggttcgagccgatcttcgtggaggtcgccgccgccgacctgccgctggctgacgccatctcgtcctatctgttcaactccatgctgatccgagttccgggcgaggaccggctgacgctgatctgccccgtcgagacacgagagaacgtccgcgcccatgcggtcgcagagggcgtcgcctcgtccaacgggccgatcggccgcgtcgaatacgtcgatgtgcgccagtctatgcgcaacggtggcggtccggcctgcctgcggctgcgggtcgtgctgacggaggcggagctggcggcgaccaatgcggccatgcggctgaccgacgaactgcacggcgcgctcagcgtctggggcgccacctggtatcgcgaccgcctgacgccggcggacctggccgatccccagctactggtcgaaagccgcggcgcgctggacgagttgacgcagatcctgagcctgggcggcggcttctatccgttccagcgcggataggaccgccgaggctcaggctgcgaagcggccgccgcgcgcggcgtagctctgcgtcccgcgggtgatgaggcgatcttccggcagcacggcgtccgcggcgatttcgccccgccccttcaacgcctcatagaccggcccgaaatccttcagcgtctcggccttcagcgcctccaggctgtcgatcacgaaatagacctgctggaaatcgtcgatacggtagagcgtgcgcatcacccgctccagatcgaagccgatgcggttgggcgacggatcgtccaacgcaaacacgctctccgtcgcggatgaaacaatgccggcgccgtagatgcgaaggccttccgcctcctgcatcaggccgaactccaccgtgtaccagtacagccgcgccaggttcggcagcatgccgagcgacgccgcccgctgcccgcccttgccgtaggcctccatataggccgcaaaatccgggttggtcagcatcggcacatggccgaacacgtcgtgaaatatgtccggctcctgaagatagtccagttggtccggcttgcggatgaattggcccgagacgaagcggcggttggccaggtggtcgaagaagacgtcgtccggcaccaatcccggcacgcacaccacggtccagccagtcagggcctgaagcttgggattgatgacgttgaagtctgggatgcctccggcgttcaggtcgagcgcctccaagccccgcatgaaggcgtcgcaggcccgacccggcaggatcttgatctggcgggcgtacagggtgtcccaggtctggtgctcgatctcggtgtagccctgccaattctggggaatggtccagtcggcggcggcgccttccggtggcgcgtcgaacacatgctcgaagtcggacatgaagggctccaaggctctgtcggcggcgctttcccgcgccttgtcgcgccaccttagcgccgcccgcccgcacggtccaagcgggtcagtggatgggctggtccatgggcgcgtgatggccggcgtcatcgacgctgaatcaccggcgctggtcggctctggacagcgtcagggcgtccgacgcgtcgcgcagagcgtcctcggcggcgtaggcgatgaagccgccatcgtctcccatggcgtagacgcggtagaagggctggtcgggcgcggtcagcgcctctccctgcaccgagccgtcgtagacggcgtccacatccaaaaccgcgccttggaaggctccgtcatagtgccggacgatctggccgatatggaaacgggcgctgcggaagtgagccatgcccccaagatacgcccatgttcctgagcgggaggccaaggccgtcgttcatcttcgtgacagattggcttggcgcggagcgaaccggcgggctagagtccaggggaacgggcgccgcttcggaccgcccaaaggatgacacggccatgccggagacccgcggcgcgccatcagggcgcgacgagcggtcccccgcttcctccccgaccgggcggtcgggaggccgggaagcatcgggtcgggaggcgccgctgtatggcgcgctcgatcttgggaccaacaactgccgcctgctgatcgccaggccggcgcgcgacggcggattccgcgtcgtggacagcttcagccgcatcgtgcggctgggcgaaggcctgacgcgcaccggccggctggacgaacgggccatggaccgggcctatgacgccctggccctgtgcgccgagcgcatcgcgcgaaagggcgtggacacgggccgcttgtccgccgtggcgaccaaggcctgccgcgccgccgagaacggcgaagcctttgtggaacgggtgcgccggggcaccggcctgtcgcttcgcatcattgacccggccgaagaggcgcggctgtcggtcgaggggtgcatgaacctgatcgatccggcggccgaggccgtgctggtgatcgacgtgggcggcggctccaccgaaatgtcctggctgacccgcaagggcgacggctggagcgcggcggcctggatgtcggcgccgctgggggtcgtcagcctggccgaacgccaccccgagcccgtcggcgggggcgagctctggtatgaagccatggtggcggacatgggcgcggcgatcgcggccggcggcgtggacgatccggcgttgaagacgctgttcgctggcgaacgggcccacatggtcggaacatcgggcgccatcaccagccgggccggcatccatctgaacctgccccgctacaaccgcgagcgggtggacggcttgtggatgacgcgcggagactgcgaagcggcggccgaccgcctcaaggcgctggggccggacggacgcgccagggaggcctgcatcggcccggatcgcgccgatctggtgctggcgggcgcggcgatccttgaggcggtgcagcgcgcctggccgtgcgagcgggtgcgcgtcgccgaccggggcctgcgcgaaggcctgctgctgcagcggatgcgcgaggatcgccgtccgccccgccgacgccgcaggcggggacgcagcgccggacggagcggtcagggcgcggcctgagcggcctcctcgactggaacctcgatgtcgcacggtgagaagtcggcgcccctcgcctgccgcgcgtgatccaccagggcgcgaaaggcgggcgagcgcgtatccatgacgcgaatcgccggccgttcggcttgcggcaggtcggccgccacccgcacccgggtcatgcggtccggctcgctgacgatgccgtccggattggggctggccttcagcgcgcgcaccaccgacagccccgagatcacccgaccccagacggtgtagcgcttgtccagcgaaggataggcctggcgcatcagaaagaactggctgttggcgctgtcgttcggctcgtcgcgcgccatgccggccacgccggagcaatacaggccccagccgtgaaccttgccgtccgtggtgccaggcatcagcgcgtcaggctgggtctgcaccggcagtgcgcccatgaagcccacaaccgcgcccgccggctcggccactccggcaaaggccgaacccggcccgcgccgaaacgtgaactcggccttcaggtcgggataccagctctggccatcgccggtgcccagcggatcgccggtctgggccatgaaccagtcgatcacgcggtgccaggccaggccgtcatagaagcccttgccggccagcagcctgatccgctccacatgcgccggcgcgacctccggcgacatctccaccaggacccggccccgcgtggtgtcgatcaccaggagattggcggcgtccggcgttcgccattcggtggcgggtggtgcaggcggcgtctcctgagccgcgagcgccggcgcggcggtcaacagcaacagggcaacccccgccatcgccatctggatacgcatggtccctccccctgcttattgcctgcagatcaggcgccggagacctccgccgccggctgaacgtcgcagatgttgaaggctgagcccttggcggcgcgcgcctgcgccagcgtctgcgcaaaggccgcgccgcgcacgtcctggacccgcacggtcggcgcctcgcccgccggcatcgccgaggccatgcgcacccgcgtcatcacgtcgggatcggcgaccgcgccgtcctggctctctgcgccgggcttcagcgcgcggaccacgtccaggcccgagacgatgcggccaaaggccgtatagatcccgttcagcccgtcgttgcggcccgtcatcagatagaactggctgttggcgctgtcgggcgaggacgagcgcgccatgccgaacacgccggggcagaacaggccgtgggcgtcgaccttgaagtccgccgtgatcatcatctgggcgtcgggctgggtctggaccggcagcgtgccgaccaggcctaccaggcctgcgcccgcgttgggcacggcgacaaagcccgcgtcgcggcctcggcggaaggtgaactcggccttgagatcgggcaggacgctgccgccctcgcccgtgccctgtggatcgcccgtctgggccatgaagttcgggatcacgcgatggaacttgagcccgtcatagaagccctgattggccagggtgcggacgcgctccacgtggttcggcgccgccagcgaagacagctccaccaggatgcggcccttggccgtgtcgatcaccaaaaggttttcgggcgcaacggtgcgccactcggccgccgccggtgcttgagccgccgccccctgccccccgccgatcatcatcacggcggccagagcagccgccaccgaaacacgcatcgtctacttcccgttcttgaccttggagcgcacgcgcgcggcgaccgtcgggctgacgaagctgtcgatcgcaccgtccaaacgggcgatttccttcaccagccgcgaggcgatggcctggtggcgcggatcggccatcaggaacacggtctcgatgtcctgattgaggcgctggttcatggccgtcatctggaactcgtactcaaaatccgcgaccgcgcgcagccctcggatgatgacgttggcgtgcagttcctcggcgaaatgcatcaacagggtggagaagggctgcaccacgatctcgccggggatgtgcgacaccgcctcgcgcagcatctccacccgttcgtcggtcgaaaacagaggtcccttgtcgtcgttcttggccacgccgatgacaacacggtccaccagcttggccgcgcgcgcgatgatgtcggtgtgcccgttggtgaccggatcaaaagtgcccggatacagcccgatgcgcatctgcggcgtctccccccagcctgtccggcgcgacgtccatgggcgtttagcaggtgcgaaagccgaggcctagcgggcgaggccgcatcagatcggctggggcggctgggcgacccagcaggcgcggacacggttcaacactggatgatcgacatcgaagaccgcgccgtcgatctcggcgaccggacacatgggcgtggcgctgttgcagatgaacgcggcctcaaaggcgggcagatccggcacggcgatctcgcgcgtctcgcacgacaacccctccgcgcccgatccttgttcgatcagtccctgtgcgaccccgcttagcatcggcgcctgcggccagatgatgcgttcgcccgagacgaagccgatgttccacaggctgccttcggacaggcgaccctgcgcatcgacgaacagggcgtcgtcgaagcccgccgcccgcgcaatgcgccgcgcgcggatgaggccgaatgtcgccagatgcttcagttcggccgcctcgcgctcatagggctgcaccgtcagccgcaacgatgcggccagcggcgcgaccgggcccgccgtcatcgtcatcacgcgcggacggccgatccacgacggagagcgcggccagacctccggcgaaaacaggctgacgcgcagccaggcggcggtgcgcccttcgacggcgcggcgcatcaggcgacgcagctcggactcgttcggcgcctcgccgaacagcgcctcggcggagcgacccagccggtccagatgcaggtcaagcccgcgcaccgcgccatcctcgacggcgaacgaggtgtaggcgccgtagttgaccagggccagataggtcaggtcgtcggcggacgccggcgctccatcgatcaggatgtcggccacgggcctgcgcggccgggcgtcagccctcgccgccctcctcgacatccgacacgacaccgccgtcgccgctttccggcagacgctccaccgagaccacgcgctcgtcgccgcccgtgcggaagatggtcacgccctgcgcggcgcggccggccacgcggacctgtcccacccgcgtgcggatcatctggccgcccgaggtgaccatcagcaggtcgtcgctttcctcgaccgggaaggcggcggccagccgggtgccggcgcgtccgcccaggccgtgcgccgtcagcccctgcccgccccggccggtgcggcgatactcataggccgaagaccgtttgccgaagcccgtgtcggtgaccgacaggatgaactgctcggccgcgcccagttcggcgaagcggtcgggcgagatcggcgcatcggcgtcggcgtcgtcgccgacctcctcctcgatggcttcgggcgccgcgtcctcgatgctctcgccggtggcgcggcgattggcgacggccagcttcagataggcggcgcgctcgtcgggcgtggcgtccacgcggcccagcacggccatggagatgacctgatcgtcgccgttcaggcggatgccgcgaacgccagttgaatcgcgacccttgaagacgcgcacgtcgtcggccttgaagcggatggcccggccgttgcgggtggtcagcagaatgtcgtcctcggcggtgcacaggcccacgccgaccatgtggtctccgtcctccagcttcatcgccatcttgccggcgcggttcacagtggcgaagtcgctcagcttgttgcgccgcacgtcgcccgagcgcgtggcgaacatgatgtcatagttcccccagtccgcctcgttctccggcaggggcaggacgttcatgatgctgtcgcccggctcgatcggcagcaggttgacaaaggccttgccccgcgactgcggattgcccagcggcaggcgccacaccttgagcttgtaggccttgccgttggtggcgaagaacagcacgggcgtatgggtcgaggcgctgaagacgccggtgatggcgtcctcgtccttcatcgccatgccggacttgcccttgccgccgcgatgctgggtccgataggcgttgagcgccacgcgcttgacgtagccgccgtgggtgacggtcacgaccatgtcctcgcgcgggatcaggtcctcgtcctccatctcggcgtcgccttcgccgatcagggtgcgtctggggaccgcgaactggtccttcaccgcgatcagatcgtcgcggatgatcgccaggacgttcttgcggtccgacaggatggtcaggtggccctggatggtgtcggccagacccttggcctcgccgaaaatgtcgtcccggccgaggccggtcaggcgcgccagcgtcagcgccaggatggcgcgcgcctgttcgtccgtcaggcggatcttgtcgccttctacgatgacggtgcgtggatcggcgatcagctcgaccagcgccatcatgtcgccgaccggccagggcttggcctgcagccgctcgcgcgcctcggccggatcggcggaggagcggatgatgtggatcacctcgtcgatgttggccacggcgacggccaggccgaccaggacgtgcccccggtcgcgagccttgttcagctcgaacttgacgcggcggaccaccacctcctcgcggaagtcgagaaagacctccaagagctggcgcaggcccatctgctcgggccggccgtggttcagcgccagcatgttgacgccgaacgagctctgcagcgcggtccagcgatacagctggttcaggatcacgtcgcccgaggcgtcgcgcttgagctccaccacgatgcgcatgccctggcggtcggactcgtcgcggacgtcggcgacgccctccagacgcttttcgcgaaccatctcagcgatgcgctcgatcagggtctgcttgttcacctgatagggcagttcggtgacgatgatcgcctcgcggtccttgcggatctcctcgatggaggcgcggccgcgcaccaccaccgaaccgcgaccgtcgcgcagggcgttgcgcggcgcagtgcggcccatgatctcgccgcccgtcgggaagtcgggccccggcacgatgtccagaatggcctcgtccgagatgttcgggtcattcagcagcgccacggccgcgtcgatgatctcgcccagattgtgcggtgggatgttggtggccatgccgaccgcgatgccgcccgcgccgttgaccaagaggttcggaatgcggctgggcaggacgaccggctccagctccttttcatcgtagttcggctggaaatcgacggtgtccttgtcgatgtccgtcagcagcgccaccgccgccggcgccatgcgcgcctcggtgtatcgcatggaggccggcatatcgccgtcgaccgagccgaagttgccctgaccgtcgaccagcatcagccccatcgagaagggctgcgccatgcgcaccagcgccatgtagaccgaggcgtcgccgtgggggtggaaccgccccagcacgtcgccgaccacccgcgcgcacttcgaataggcgcggtcgggcgtcatgttcaggtcgtgcatcgagtacaggatgcgccgatgcaccggcttcagcccgtcgcgcgcgtccggcagggcgcggctgacgatcacgctcatggcgtagtcgaggtacgaacgcttcagttcgtcctcgatggtgatggtcgaaatgtcgcccgaggcgccgcccggcccggccgggggtgcggcgttggtgtagctgtcgtcggtcaaggaaacgtggctctattcgccggaatcggaacgtgatccgctggtgcggtttctagcatccgacaccccggacgccaaatcgagagcccctgtcgggccgtcagcacaaggactttcccatgcgcacgcttcttctcgccgccgtcgcctccaccctcgccggatcggccttcgctcaggcaccggcccccgcgcctgctccggcgcctcagccggtaggcagcgccatgctgaagaacgcggacggcggcgacgccggcatggtcaccgcctatcacggcccgctcggcgtggtgttcaaggtcgagggcaagggctggccggaaggctggcacggcgtgcacctgcacgcggtcggaacctgcgaagggcccaagttcacctcggccggcggccatgtgaaccatgccgaccaagcgcgtccgcatggcctccttaacgccaacggcgggccggacctcggcgaccttcagaacgtctacgcccacgcggacggcgcggccaacgccgaggtctatctggcggcggccggcctgaacatgcagccgcaggacctgctggacggcgacggcctgtcgttcctggttcacgccaaccgtgacgaccatgtcagccagccgatcggcggcgcgggcgaccgcatcgcctgcggcgtgttccagacctcgcgctaagcggtctcgtcaggccttggccgcgccggcccgcaagccgcgctcggccagggcgacgatggcgacgccgctcatcgccacggccgccccggccaggatctgcggcgtcagcacgtcgcccatcagcccccatccgatcaggatcgagaccacgggcgtggccagaagatagggcgtgacgcgtccggcctcgcgccgctgcaccagccagaacagcagggtggtcgccagcaccgaggacacgatcccggcccacagcagcgacagccagaccaggggcgtggcgttccgcatcgcgtcccactggccgtgctcgaacaccgcggagccgaaggccatgatcggcagggtcgacgccgccagcagcccctgcattttcagcggcgggatcgaggtcgtccgccgagccaccaccgtggtcagcgcccaggccgcgcccgccgcgatcgccaccacgatcgcccgccagtcctccagcgcatgcgcgtccagcgtcatccaggccacgccggcgaaggccaccgccatgccgcccgccgccgcccggctgagccgctcgcccagcagaagaaaggcgaacaggctggtcagcggaatccacagctggttggcgacggtcaccggcgtcacgtcccgcgccagccaataggccacatacagcagtccgtactgcagggcgccgccgaccagcacgatcagcagcaggctcttccagtcgggaaacggcggccgcacgaagccgacaaggcagacggtggcgatggcgaaccgcaaggcgccgaccagcagcggcggcaggctttccgtcgccagcttgcccgccgcgttgttgacgccccaaaccacgatgatcgccaggatcgcgccgatctcgagccgcgtcagggcgtgcggcttgggcgaggcggcggcgtcgggcgtggtcatgtcgcttctatgccacgccgcgctccggccgtcggctcacttcccatgaaccgagatttccgatcctcagaacgggatgtcgtcgttcaggtcatagctctcgcgcgggcccgacggcttgttggcgccgccggtcgagaagccggacgaatagtcgtcgtcattgccgcgtccgccgccgtagccgccgctggaccccgagccttcgccgcgaccgcccagcatcgtcagttcgcccttgaagcggctgaccacgatctcggtggagtatttctcgacgccctgctggtcggtccatttgcgcgtctgcagcgcgccctcgatgtagaccgtcgagcccttcttcacatagttctcgaccaccttgacgatgttgtcgttgaagatgaccacccggtgccactcggtcttctccttgcgctcgcccgaggacttgtcgcgccaggtctcggaggtggcgatcgacaggttggcgatgcggtcgccgttcggcatcgagcggatttcgggatcgcggccgagattgccgatgaggatgaccttgttgacgctgccggccatggctttcttccttttcgtcgtttcgccgccgagacggcgatcagggtcgtggtcgatgggggttccgagagcctagctcaacagcaaagcgactgcgaagcctcaaagatgtggatcactggggcgacggcggcgcggccaccgccaccggcgcgccgtcgatgccgcgctggatcgcgccggggatcgccaggcggccgtcgccggtccgcgccagggcgaagaagcgggcgccgttcagcgactgggcgaagctgacgccctcgcgattgatgaagatgtagcgcccctgataggcgcccgtgatctcctgcttggagccgcccaagcgcaggaactgcacccgcatctcctccaacctcgcggcgcagtattcgatctgtggctggtcgcggaccaggacgttgtaggctggctgttcgcccgcctcctcattgacgtgatagcagacgccgggctcgaagtcgggttcgctggaggcgcaggccgacaggaccagcggggccgaaagcagcagggaagcgagaagaagcgcgcgcatgggtccttacaggctcgggaactgacagttgcggtcctgctcggccagggtgcggaagcggacgttgtcgccggactgctcgacccggcccggcaccagccgcagggtcgagctcccccagcggccgtattgcgcatcgcccggccgcacgcacatgcccgaatacagggcctggacgcaggcgttcaggctcatgcccgaagatatctggcgccagtccgagcccacatggcgcaggcactgctgcccggccgccgccggctgcgcctgcggctgggggctggccggacgaaccgggttctcatagacgggcgcgggctcgacctcgtcgatctctacgctgggcagctcgggcggcggggcgaaggccgccgtgggcgccgccgccagggcgccggacgcatccagaccgacatcgagagcgtcggtggccaggccgttgcgttgggcgcagtcggccagggtcgccatgcccgcgaactggccgtcgacgaagcagcgcagctcccgtgtcggctcaagggtcggcgcctcggccaggtccaccgtcaggccgccgcgagaggcggggggcgcttcgggcgtctggtctccgccgccgctgaacaccagggccagcaccacggcggcgatgatcacgaggccggcgccgatggcgatgatgatgcggttgtcgttggggctcgccatgggctcaataactccggccaagcctgcgtcgtcaaacgaaaaggaatcgggcggacgttacgccgtcagccggctgagcgccgcctgataggccgaggccttgctgttccagtaggcggcgccggcgctgctccccgccgcgacgctgggggcggtcgtggcgctttccggagccagggagcgataggccgagcggatcgaggacagagccgcaaggatggcttccgatgcggttttcaccgccgcggcgtcatccaggctcagcgtagtggaaaggttgaggccgaaggtctcgatcgcgtcctggtcgccggaatccttgaacccgacgtagccggccttgagacccagacctgcgagcgcatccttgccggcgggcccggacgtgatgatcgcgccgcccttgtcctgaaggccggtgatggacaggcgctgaaccggcggggtcacggtgctgtcggtggtgaccgcgaccttgacctgacgacccgccgccgtctcgatgcgcctggccaaggtctcgagcgtgtcggtggcggtgatggtgaggttcgtggcgcgtcctcgcccatcgccgcgcgcgacggagaactggtcgcccacccgcagcgaagtcgccagtgtcaggtatttgggatcggactgcgcgatctggccgctgggaagaccaagccggtccagaacactggcgccgttctccaccaccgcaagggcgctgggagtcgcctggtcgccctcccctctccaggtgcggctgtattcgacggctccagtctccggatcgatccgcgccagataagcacgcgtggggtccgtcgccttggcggtcggcgcgcggtccgccacccccgtgatccagaccttgccgtccgtgatcttcacatcggccgccgtgtcgtcgcccgcgccgccgtagtaggtcagccggtccgtgcccgaggcttgaaggtccgccgaaaggctggcgacaaaggcgtccaagccgccggacgcggccgtggtgatcgttcccgcatccagggcggggttggtggtggcgcccgcgacgatcaggcggccgttctcgacagccagtcccgcgatctcgccgcgcatctgtccgaggtcgcgcgtggcggcgagcgtcgggcggccagcctcgtcgagcgtgaagcgacgcaccaccgcacggccgttctctatcccggcggtgtagaggtcggaaccgctgacggtcatcgcctggacggagtcgtcgcccgtggagccgaactggcgcgtggcgatgttggtggcggtgaacggcgccagcgcattggcctgtcttgacgaataggcctgcacatagccgtcccagccgccgaccgccgaggcgccgctcatcgccgatttggagcgaccggcgacatagaccacgccgtcggcgccgaaggagaccgccgtggcttcatcggccgcccgcgcgccgcgacgctgggtccattgctcctggcctgtcgcatcgaagacggtgacgaaactgtcggccacgccggccgcgtctccgctcttgccgtcatccagcgcgccgatgaccgacccggccacggcgacccgcccgtcgggcgcgaccgccaaggcgtagccgttggcttggctggcggcgcccagaacctggctggaggccacccggccggccttgtccaccttcagcagggcgacatcgctctgtcccttgatcggctgggcgtcgaagccctgatcaaggtccgccaccatccagatagagccgtccggcgccgtggcgctggcccgcacagccgcgacgccctctggcagatcggtccgtgccgcctgcccttccacccagaagctggagttgacgccggcttgcgccggatcggccgttccgccgtccgactggaacttgaccacctgttgggttccgccagcgccggccttttgcatcacatagacagcatcgctggtgtcgggcgccgacagggtcagggtctcgccgatcactccattgatcttcagggaccattgatccggaccggccggcagagtgatggtctgcgaaccggctgcgatcgtgcgcggttcggccttgatctgctgcttggcgaagcgcgtcgccacgccggcttcagacagcttggtgttgatgtggccgatcaccccgtccatcgtccgaggcttgtcgccgaggtcggccaggtcgatgttcagcgtcttcagaccgccgatcgtcttcagggacagggtgaaccgcacgtcgccttcgaaggcctgcaccgactgggtcgcggcgcccttgtggatcggcgcgccctgatagacggcgttggccttttccacgcctgcggtggtcttgctggaggtggccaagagcccctgcaccagccgcacctcctccatggaggccgcacccacgtaggcggaggcttcggccagcccagaggcgaatcgctttctgagctggaccagttccgtcgaagtcacgcctgcctcgccggcgcgcgtagccagcgccgacaggctggtcaggcccttatagagggcgaacagcttgctgtagtcggacgatgcgcctttgacgtccagatcgacgtcggattcggagatcaggctgcgagatcgcagcgcctcgcgcaccagctcgctctgctcggtcttgacgacggtggtggaccagggcgccgtcggctgcttcttgacgacagcgccggcgatggacgcggacatgccgacgcccacgccgccggagacgccgaacaggccgagaaggtagctgttgttgatcattggaggccggctccctgcggcgacgctagggcacggcctctaacaacagcttaagcgttgggcttagttctggaacagcgacaggatcgtctgcggcgcggcgttggcgatggacagggcctggacgcccagctgctgcttggtctgcagggcggtcaggcgcgcgctttccttggccaggtccgcatccaccagattgccgatgccggtctccaaactgtcctgcagcttggtggtgaagatcagctggttgtccagcgacttggacccggtgccgagcttggtcagcgaaccggtgacgtagctgatcgagtcgtcgacctgcttcatcagagcctgccatgcgtccgcgtcggcgggaacgacaggatctgcatcagggtcgccagccgcctccgcacgaatggccgcaaaagaacccgaggcgatgttcatcgccggcgtggcgtcggtatcagctgaagcagcggcggcgtcagcgtgtgacgcgtagagaccgaaattcacgccgctgacgtcgattgtagtcttgccgtcggcgctggcgagcgccttcaacgacttccccgtcagccccgtggtatctgcaagcgcgggagtagcgtcggagtcggcaggatgcttcatctgcacctgcccgtcggcatccagcgccgcgatcatgttgacgccgttgaagctggcgccctggatggtggtggtgatctgtcgcgcgaggttctcgaagtcttcctggtaggcgttcaggctgacctcgtcggtgctgggatccgacgccgccagcaccaggttgcgcatctggcccagcaggtccttgaccgtctcgccggcggccatggcgacgtcgatggtcgattgcccccgctgaagcgactgcttcaccggctccagcgcgttcatctgattggtctggttctgggccacggcccagagggcgccgttgtccttggcgctgttgatcaccttgccggtgttcacccggctctgcgtctcgtccaactgccggttggtggcgttgaggttctgcagtgcgatcagcgccgagcggttggtgttcacgctgttggtcatggtccggcccctagcttcttgggacgaccgttaaccacgaaatatgtgcagagggttaacgcgcggaaaccatcggggtcagcgccggtccgatcaaacgtcggcgacgatgatgcggccctggcgataggtcggatcgtcggccagcttttgcacctcttcacgaggccactggcgcaccacctctccggtctgacggtccacggtcttgtagacaaagccgtcgtcggcggcttcgatgaccaggcgatagcgcgcggcgtctgccgaggcggatgcggcgggcgcaggcgccggaacgggtgaagccgggatgtttgcgggcgttacgctgggtactggagcgacatgatctgacatcatcctccgcgcgacttgggtcgcgccccttcaagaaatgggaagaagagggagacgggcgaacccgcctccccctcaaaggtcttagcggaacaggctgagcagaaccgagctcgacgagttcgcgatcgacagagcctgcacgcccagctgttgcttggtttgcagagccgtcagcttggcgctttccttggccaggtcggcgtccaccaggttgccgatacccatttcaagggtgtcctgcagcttggaggtgaaggtcagctggttgtccagcgacttcgaaccggtgcccagcttggtcagcgagctggtgacgtagctgatcgagtcgtcgacctgcttcatcaggtccgaccatgcagtggcgcgcgtagtttcgcctgcggcattcccggcagctgcgcccgcttcagcctccgcacgaacggcggtgaacgaactggacgcgagcctgattcccgctccggcagtgatgccctcggcggcggtattggcatcagcgagccttgtagctgcggccgctgcattttcgccagcgaccggagctgtgggagcatgcaagccgaagttgacgcccgcgacgtcgatggtgttcttgccatcggcacttgccaacgccttcagcgacttgccggctccggtagcttggggggcgccattagcgtcaaggttagcgaccatgttgacgccgttgaagttggcaccctggatggtcgtggtgatctgcttggagagattcttgaagtcctcctcgtaagcatccaggctggccttgtcgacgcccggatcggacgccgccaggaccaggttcttcatctggcccagaacgtccttgaccgtttcgcccgccgccatggcgacgtcgatggtcgactgaccgcgctgaagcgactgcttcaccgcatccagcgagttcatctgaaccgtctggttctgggcgatcgaccagatcgcgccgttgtccttggcgttgttgatcgccttgccggtgttgatccggccttgggtggtttccagagcgcgattggtcgcgttcaggttctgcagcgcgatcgaagcgccgtagttggtgttgatgctgttagccatcggtagtcatccttctggatcaatggcgccgttctgacgccccgagccttatgctcgcgccggcttcttcaagtggtgggccaaggtcggacaatcagaaaattctgccttttcaacgaaggctgcgtttcatggcccggcaaataggagcaacgcccggcaaaaggcgccgccgcccggcaagtcttgcccccctctcaagggcgatccgcccctcgcctccacggaggcgtcggcgtgtcagcctcagctctccattcgtccgccagtgcacgctcggccaacagggtctcgaccgccagccgccgcgcgccgtcgcaccgaaccagttgctctcctctttggacataggcggcctcaagatcggccagggtggcggcgtccggcagcacggccatttcgcacggcagccgggccgcttcaggcaggtccaggcgaggcgcagccgttgagattgggggcgccgcggcacagctcgcggtcgtgatcgcgcagacggcgcaggcgatcgggatcaaggggcgtttgggcatcgtgggcgctccgggcctgtgcgacggcggtcgcggtcgcccgcgccgcctgtgtggtggtgtcattgaactcatccaggcgacgttgctgaacttcgccgccttgctgttcgagccgtcgcgcgacctgctccgcgcgtccggccgccgcctcggcctgagcagcctccagccgcttgcggtccaagcccagcggatcccagcgaaagcccatgccgcctgccatcgccgcggcgagcaggaccccgccgacagccagcgccagccaccccagcggcgtcagcatcctcagccacgacctcatggatagcgcctccggcaaagctcgaaatgcggaccgtcgcgtagtcgcggccagtcgccgccccagatcagcgtcacgccaagatcgagtgcggaggccctgaacgccttggcgatctgggggtacagcggccaatcccagcgcacctgcccatcgaccaaggccgcgacgtccaccgcatgtccggtcagatgacgagagttcagcgttcggctggcgccggccttcacaagttgcgcctggcgctcggccgaccgaagcccttcggtgatcatgaagtcgatgtcagatcgaccgatagccgcttcgatcacggccacaaggctcgggtgcacgcccttcaggcgttgtcgcgagcgcacggagaggcgaaagctcatgctcgacctccacccgcgatccgcagccgcagattggccgacagggcgaccagttgctgggccgtcggcgccaccaagtaaagcaccagcatcagcgccagcagggtcatcaggccgttggcgatctgcgacatctgctccgggccggcgcgctcgaccagccgatcaagcagccgccacagaccgaagctggcgacgaacacatacagccggcgccacagccattggggctcgggcaaggctgtcatcggccgtcctcccactcagggcgatcgcgtggagcggcggagccggtgaccacccggcagtcgtcttcggtcagatgatccggcgcgtcccaggcctcttcgtccaggagcgcgaactgttcgtcggggctcatgggcggccgctcccgccgaccctaatcggcacgccccggtcgctgtcgttctcccgtcgcctgtcgacaggcggggtgagcccatgcgggccgctgaaatcgttgttcacgcgtgatctccgttgatgtcggagatcagtctgggtcagccccgtaccccggcgagccgaaagggcgcggatgcacgcaaagccggcatttttaccgggatcgccggtctgaactgcgacggctggagacctgaaaggagcaggggaaagcgcggggagaccaggtggaagggctaggtcggcctccccgcgtgacaggactcagctgtcaggcgccgcgcgcaccgagtgaggtcaaatgcgcgcgggagccctgtcagacagagatacggacagccgcgcgatgcggatgcggccgaaagttcgtcaaagcgtctggatgtcgcccgacgcgacgaccggaccgtccggcttgttcggcgcaggcgcatggcccggcgcctccagggagatggccagctgagccacctggccgatctgcgccgacaggccgggcgcgaccggctgacgcgacggctgccggccgttgatggcgcccaccagctgaaccccgccgtccggcagcatcagccagaggtgcggcacgcgcgcgtcctgctgggccgaccgcagcggcgccaggtaaagcgtctcggtggcgctgtcgtagacgacggtggcgaacgcctctccctcgggcgtcgacaaggtcgcgatgcgggcgatttcgggcgtctgcgcggcgggcggggcggcgggcggcggaacaaccgcgtccggacgggccagcatcaccgcgaacgccgccacgctggcggcgagaagccccgtggacgccacggcccagcgacgccagaacgccagcttgcggttgtcattggcgggcgcggccagtctggcctcgatccggctccagacgtgggttgaaggctgcaccggcgcgacgtcgtcgaacaggacggccaaacgcgcctcccaggccgcgacatctgcggcgaacgccggatcggcggcctgacgcgcgcgcgccgccgtctcggcctcgcgatccagcacccgcagcgccagttccgccgcgagcaggtcgccgccgtcgatgtcctgcgcgtctgtcatcgatccaggcagtcccgcagccgcatcagcccacgtcggatccagctcttcatcgtccccagcggcgccgcctcgcgttgggccaggacctcataggtcgctccgtcgaagaaggctgtgcggatcacgcgccgcgtgcggtcgtccagatcgtccatgcaggcgttcagtcgcgcagcgtcttcactccgctcgacctgggcggacgccagaggcgccgtgtccggcacgtgggtcgccgcatccaccgacacggtgcggcgatcgccgcccgtcgccctcagtcgatcgatcgcacgattgcgcgcaatggtcgccagccaggtaatcgggctcgcccttgcgggatcgaaccgatccgccttgcgccacactgtgagatagatgtcctgcaacacgtcctcagccaactgacgatcagccaagatacggaggcagacgcccaacagtttcgccgaggtggcctcatagacgattctgaacgccgcgcggtcgccctcgccggcccgtcccaaggcgtccgccagttcgtcgcgggtcaacgtcgcgctcattcaggaccctgttccagccagagtgcgacttgcgggcgcccgcgcatgtgcgtcaagtcaatcatgcagatagacgatccgtcgcagggccggatcgcgacgaacggtctcctgatgccgctcgtgatcgccggttgcgcgggcgtcggcttcggtgtcctcgacccagtgggtgctctcgatctctttttgcagcgccttggccgccagcagttggcccgggaagaaggtgtccacaatgtccccgaacagcgggaccgagcccgtggcggtgtccacccccatataggccgccatcttggccagggtggaacgcgaagcgccgatcctcagcgcctgaacaatcagccatccgccggtgccgacggtgtacagcgtgccggccacgggaatccatgtcagcagggcgtccatgccgacgccgaagggcccgatcgagatggcgcggtccgacagcttcttgacgccctcgacatcagaccagatcttttcgatatcctgcagactgcgtctggccatgcgtcgttcctcaagcgtcgccttaacgcgtcaacgcttcctgcgttcacccctatcgaggtcgagggcatccatgctcaggcttgcggccaatttgctggcgagcgccgcgtttgtcgggttcggcctgatcgccgcggcggcgctcagccgcatcgggcatcgctgggtggacattctggcgcaattttccgcgccgtcgctggcggccgtcttcgccatgcttctggcctgcctggtccttcggctctggccggccgcgctggtcggggccggagcggccctgctgctgctcctggccgtctggccgcagtgggcgccgccccgcggtcggccggacacccatgcccccgctgttcggctgtattcggcgaacctgtgggcgtggaaccagcagacggaggccatagatcgctcgatccggagcgccgaggcggacatggtgatcctggtcgaactgggcgacgcgccggcggcccagctggaccggatgctggcggcctatccgcaccgggtttcgactccacgcatcgaccggccgaccggcgccgcccgcacagtgatcgcctcccgatggccgatcgttcgcaccgtcgaagacaagcccgacggcctgcacgccattggtgcggtgatcgacagcccgctgggtccgctgaacctcgtcgccgtccatctgacccgcccctggccctatcagtatcagtggggccagatcacccaggtgatggctttgacgaaattgcgcgcgggcctgacggggccggtgatcgtggccggcgacttcaacagcgtgtccagcgcccgcatcggccggcaggtccagtcacaagccggcctgatcccggcgcccggttttcccggcacatggccgacacgtctgcccgcgttcgccggcatcaccatcgaccaggtgtatcgctcgccagacctcgccctggtcagtcgccgcttgggcgaaccaaccggctcggaccatcggccggtcgtcaccgagttccggaaggctctgcgctgatcgccgccaccagcgcgtccagccgcgcctcgtgcccggcatcgggaaagtcgtcggcgatccagctctcttcaaaggcgctcaacagacgcccggtctgcggtcccggcgatacgccgcgcacggccagatcccgtccgcccaccggcagccggggcggcgtccaggctcgcattggggccagcagcggctctgggtcggcgcgggatcgcgcggcggccttcagcaggcgatcctcgaacgcctgcctcccaaggcggtaaagcgccgcgcgcgccgccggctcgggcatggtcggcgagacgtcgcccgccggatcgacggccgcgagtagcctatccctttgcgcattcgacaggcgcaggcgagcggcgacggcggccgcctcggcgtcgggcaacaacaccgacaggcgcagcagcggatcaggcgttagacgcgccaaggtctcgaacacgctgagatccgcctcgccgcccgtcagccgcgccagcccgcccgcctgcgccatcgcccgcaccgccggcgtcggatcgcaagccgacagcagcttcagcaactccttggacacccgctccgccgacagccgctcgacccctgcggacaggcgctcgcaggcggccaggccggccgcgtcaggcgcgcccgttccgtaccaggcgaagaatctaaaaaagcggaggatgcgcaggtagtcttcacggatgcgcgcctctggatcgcccacgaagatgatccgtccttgcgctgcatcggacaggccgccgccggtcggatcgaacacaccccccgccgcaccggcgtagagcgcgttaaggcggaagtcccgccgcgccgcgtcctcggcccagtcttcggtgaaggccaccacggcgcggcggccgtcggtctctacgtcgcgcctcagggtggtgatctcgaacgggcgcccgcccgcgacggcggtcaccgtgccatgatcgacgccggtcgggatcgcccgcagtccccgcgccttcagcgccgccatggtcgcggacggctgaagccgggtggcgatgtcgatgtcgtcgacggactggcccatcaggctgttgcgcacgcagccgccgacgaaacgcgcgcagtcggccccgcccgccgcctccagcgcctccatcaccgcccgcgtttcgggcagcttcagccactcggcgccgaggatcgcggtcacgccgcgtcctcggccgacgccgcgccatacagccgatcgtgcaggcctttcagcatgccggcggttgcgccccagatgtagcgctcctgccacggcatggcccagtaccagcgcgtcatgccgtcgtgcaccagcgagtcccgccggtgattggcgacgttcatcagaaagtcccagggcgtctcgaagacgtcggccacctcgtccggcgagggacgcagcatcggcggggcggcgatccaaccgaccaccggtgtgatcagaaagcccgtcccgctctcataggcgtcggacaggcccagcacctcgacctgatcgggcgcaagaccgatctcctcccacgcctccctcagcgcggcctcgatcgccgtctcgccgggatcgagccgaccgcccggaaaggcgatctgaccagtgtggctggccagggtgtcggcccgtcgggtcagcagcacggtcgcgccctcggctctcgccaccaccggcaccagcacggccgcgcgcctcagcgtgcgcgaagggcgcgccgcctcggggttgaggtcgaagtccgagcggaccgcgcccgcatccgcgcgccagtccaacggcggcgtcaaacgctcaaacagtctgtggcgcagagcggccccgtccacgcctcaggcctcgcccaggcggaacgtcgtaccgcctgagcgcacgataaggccctccggcgagacttccgccatctcgaccagttcgtagaagacgggccgcgcgatgcgcgcccacaggtcgcctcgcaccctcaccgccggctgcggctcgccggtgacggcgtttgtttcgaccatgatcgggtggtccaaatcggctgcgacctcgtccccgacatcggtggtgaagacaagcgtcgcgccgcgccgctccacggttgtggcccgaaacggcagatcctcgacctctatccgcatcttctcgccgggcgtgaccaggtgatagccgtccggatccttgcgcaggatcgtcgagaacagccgcaccagttcacttcggccgatgggagagccctcgtgcatccacacgccgtcgcgccggatcacgatgtcgatgtcgccgcagtgggcggggcgccacagatgcaccggcgccggcccgcgtcccggcgcctgccgcgcggcttgcgcgacgccctcaagacccctgatgttcttttcgtcgcccttgtccatcgccgctgaacctaggccgccggacggcgatgcggaaggcgtcagcccgcgcgaaccgcgccggccgccgacgcctgcgtgattggcgcccacagcacgcggcggcgatccaccggccccggcaacgtcacgcccgacgcggccacgaagccgaaccgctgaaagtatggaggatcaccgaccagcagcacaccgctcgccgagttcgcacgcgcatggtcaaggcaggcctggaccagggccgcgccctgcccgtcgccccgccggccagcgtccaccgcgatcggccccaggaacagcgcgggcgtcccaccgatggtgatcggccatagccgcacagcaccggtcacccggccatgcgtctcgacaacgaagccggctgccgggcgcgcgccttcacgcagccgctccgccgtcttggcatagcggccggggccaaaggcggccgcgaccagggcgtcgaccgcatggccgtggcccgtggtctcaggctggaccagcggattgatggagagggcggcggcggcttgcagcatgggcgcgcgcacctaggcgcaacggcccggcagatcaaccgcccttggagaaatcgggcgcacgtttctggctgaaggccatgaaagcctccatcgcctcggggctgcgcatctgttcggagaactgggcgccctcgcgctgcatcaacgcccagatggcttcggcgtcgcgcattagagccttggtcttgcgcagggagttgggcgcgcgggccgacagcttgttcgccagctccgccgctgcggcttccacttggtcggatggcaccgcccggttgaccaagccccaggccagcgccgttcgcccatcgaccgcttcgcccagggcgaacagttcgaacgcccgctgatgaccgatcacgcccggcagcagcagcgacgaggcggcctcgggcgtcagggccaggttgacaaagggcgccgacagcagcgcgtcctccgccgagaccaccaggtcacagtgcagcagcagcgtcaggccgatcccgaccgccctgcccttcaccgccgccacggcgggcttgtccagatcggccatggccttcaggaaacgaaaaaccggcatgtcggccggcgcggttcccccggccccgagggctgcgaaatcggcgatgtcgttgccggccgagaagctgtcgccctccgcgcggaacagcagcacgcgcacaacgtcatccgcagcggcgccttcgaccgcttgcgccagcgccgcatacatggcctgggtgatggcgttcttcttctcgggccgattcagcgtgattgtcagcacgccgtccgcgagtgttgtcagaacctgttcgctcaccgtcgtctcccgtcgccgcccgccacgcgggttcacgatcgcaacgctccatagcggtcgattgtcgtggccgtccaccgcgcgacgccttgacgcggccacacccgggatccaaggctccgcatcccccccttccaggaggcatcatgcccagctcctttccggccctgaacgacgccctaaagggcgctctggccgccatcctcgtggccgctccggcgttgttcggcgccgccgtgcccgccgccgcgcaaacggctcccgccgcccagaacaccgacggtcggccgcaggcgcagcgcggaagtgcgacgcgtttgcctcgcggggagcggcaacagcgcggcgagaaccgcagtcccgccgcgcccgcccccactcctgaagagaataaggctggcgcgcaggctgccctgaccgccgctggctcgtcctgccaggtgacggaagcagcgctgcgcggccagacggcggacaagaccagtgtctatgaagccatttgcgcctccggccctggcttcatcgtggtgacctccacaccgccggtggcgtccgattgcgtgctgctcgccgcttcggccgaggcggctcgcgccaaggacccggccgcagacgtcggcaccgtctgcaccctgcccgccaaccagaacgcccaggccgtgatcttcggctacgccaaggaagccggtctggcctgtcaggtcgaccagggcgccctgcgcggccagtcttccgccggcacgcccatctacgagatcggctgcgcgggctcggacggcgcctggatcgaacagaccgccggcaacgactgggacgtcacgccgtgcctgcaactcgccgccagcggccagacctgcaacttcaccacggcggacgagcagaacgccgacctgaagaagctgctggcgggcacgcccggcgaagcctgcgacgtccagcagattcgtctgatgggccagaacgcgcgcgggactttcatggaggccaagtgcgcggcggcggacaccggctatgtggtgcgcgtcagcgaaggcgtcgtcggcgacgtctacacctgcgccgaggccgcccacattggcggcggctgcaccttgaccacggccgctgcggcggctccggcggcggctgcgaccgagaactgaccctcgtcgccgacgagacaatgaagacgccgtccgttcgcgggcggcgtctttgtttttgcggcgacgcagcctagccttccgcccatgcgcatcgccacctggaacgtcaactcggtcaacgcccgcctgcccaccgttctcgcgtggatggaggccgctcagcccgacgtcgcctgcttccaggagatcaaatgcgtggacgagaagttcccgcgcgaggccttcgagagcctgggctacaacgtcgagacgcacgggcagaagagctacaacggcgtggccctgctgtcgaagcacccgctgtccgacgtccggcgcggcctgcccggggaagacacggacgaacaggcccgctacatcgaggcggtggtcgatgcgccccagcccgtccgcgtcgcctccatctatctgccgaacggcaatccggtcggcaccgacaagtttccctacaagctggcctggttcgaacggctcaacgcccatgcgcgcagcctgctcgcctatgaggagccgctggcgctgtgcggcgactacaacgtcatccccgaaccgcacgacgtgcgaaatccggacggctggaccggcgacgccctgttccagcccgagagtcggcgggcctttcgcgctctcaagaacatcggcctggctgacgccagcatccttggcaagcagccgccgggatcgttcaccttctgggactatcaggcgggcgcctggccgcgcgacctgggcatccgcatcgatttcgccctgctgtcgccgcaggcggccgaccgcttccgctccatcgagacgcaccgggatgcgcgcgacatggagaagcccagcgaccacgtacccgtcgtcgtcgatctggatctggagtcctgacagatgggcgaggcgttccgggtggtcctgctggtcgggctggtcgctgcgcttctgaccaccggcgcgctgggcctgtcctggtggatggagcctgaccgtcgccttcgccgcgcgctggccaaggcgctgggcggcgcgtccgaggctgaggccgtatcggtcgccgagggcaaggcctgcgcgctcaacttcggcaatggccagctggtcgtcctgtggggccggggcgcgcggggtctggcctacgacttcggcgaggtcgagggcggcgagatcatcgtcgacggccacgtggtcgcccgcgtgcgccgcaacgaggcccgcaagtcgctggaagtgatggtccccgacgccgagcagatcgtgttgcggctgatgttcgacgacgcgcgccatccggagttcgagctggccctgtgggacgccgccgcgcccgcgccgaccggctcgcccgccgaggcgatgcggctgggacggcgctggctttcgcatgtcgaggccttgctgaaggattgagggcctcttccgcacctcgacgcagggcgctagaagccccacctctcctgcaatcgaccaccgccttgccaagggaggccgccatggcccgccttttcgacgcctatgtcgtcgccgactggaccgccgccgagaccaagaagaccggcgacaactcgctgtggatcggcgtggccaagcgcgacgtgcggtttcgcctgtattcggagacgcacaacgtcgccacgcgcgccgagggtgaaaagctgctggcctccatcctggccgaccacagaaagcgcggcgatcaggtgctggtcggcttcgacttcaacctgggctatcccgccggcacggccgcgcggctgaagctggcggaggatcaggcgccctggcgggccatgtggaagttcatcgccgccaacgtcgtcgacaaggccgacaacaccaacaaccgctatcaggtcgccgccaagatgaaccggctgatgaccgacgaggcgtggccgctgtggggcgcgccggccaagcaggcccagcgctggctgaccaccaccaagccgccgcaagggtcgggcgacatccccgagttccgcgccaccgagatcgccgcccgcaggggcaagctgcagcccaagagcgtctggcagatgcacggcgccggcgcggtcggcggccaaaccctggtgggcgtgcccgccgttcgccgcctgctggaaagcctgggaccggcgggagcgggctggccgttcggcaccggctggcgcgaactcacgcccgccgacgtcgagccgctgtcggtgctggcggtcgaggtctggccttcgatcttcgacgccaagccgaaccccggcgagatcaaggaccaggcgcaggtccgcgtggccgccgagacgctggcgcagatggacgaccggggcgaactcgccaaggcgttcgcgccgcccaaggacgccacgcccgaactgatcgcgcaggtcgagggcgaggaaggctggatcctcggcgtctgacgccgaggaaatccgtcaggccagaacgtcgtcgtagtctgggtggcgcttgtgccaagcgacggcatagccgcagcggggctgaagcttcagcccttccgcgcgcgcatgttccgccaggctctgcatgaaacgccccgctgcgcccgagccccgcagcgccggatcggcctcgacatgcaggatcacccgccgctcgccctgcgaggcgtagtcggcccacacgggcttttccccgccgtcggcgtcgaacccctgttcgaaccgctgttcggcggcattgtccttgaacgcgctcatgatcggcctcctgacggcggatcaacccttggcgggacgagcgcgttcccgagcgatcagatcggccgatcgcccagcagcgccagcaggcccagcacgctcttcaccgtgaaccagacgctgagcaggaaccacatcagcaggaacaggaagaagaacggaatgccgatcaggatcagcgaggccaggccgctgatcgccatgccgatccaggccacgatcgtccaccagaacaccgaccagaacaggcggatctgagcctcgatgtgctggcgcgccacgccgctggacgatcctcgcgccacataggaaacgaccagtccgacgagaaccagcacgttcgcgctggggatcgacaggatgaacagcacccacgcagccagcgccgcgacctttccctgcgagggcccggctacggtttgtccgcgatgcaggtctcggtcgctcatggctctgtccttcagatcaaccaggcttggggccgcgcgatcggctggccggccttcagcgtgaacacgccaaacgcgccgcgcgccagcacccacaccgccgccacaaacagcacgatcacccccacattgacgatgatcagcaccgcacccaacgccgccgcggccgccgcgatccacagggtgcgccgctggaacgtgaaatggctcgcctccagcccatcggccggcgccgcgcggtttctgacggccagcaggccgatcacggccgacaccccgatcgtgggcacggccagcaggatcaggatgtagacgccatagagtgctggcgacacagccggagccgtcgccgcacggacaccgagatcgcgcactgcggacgacgagaggcggctgatcgactgcgccggcgtcgcctcctgcgcatgatggttttcacgcagccgaccgcgcagcgacgccgccgaggcgaagccgatgtcggcgtcgtgatcgtggttgtcgccgggttcggccatgcgggagaagacgcttccgtgctggcgcagcctgcgggcggcgcgggggttcggggacaatggcggcgctgggcgtccggcgcaaccgtgtcagcgcgacagcaccacctcgcagcccggcgaggagtggccgcccagcgccccgggcttgtcgatgcgcaccgtcgcccggagcacccgctcgtcctggaggcaagccgccgccagccgatccgcaaaggtctccaccagccccacatgccccgcggcggcgatggcgcgggcggcctgggccacggtctcgtaattgatggtgtcggacagccgggtgatcgcctgcggcgccagctccagcatgacttcgatcacaagggtctgcagccggccatgctcgtggtcatagacgccgatccccgcttcgatgcgcaggtcgcgcacgaagacgcgcaaggcttcgcgccggaagccgtcgctgttctggggggacatgacggctactccaggatgtccggcgtgcgccaggcgaggtgctggccgccgtcgacggcgatcatctggccggtgaccatctccgcctgcgtcagccacagcacggcactcgccaccgcctcggggctgccgggtctcgccagggggatggcggcggcttcggcctggaactcggccggcgtctggtgcacggaggccagcgtggggcccggccccaccccgttgacccgcacccgcggcgcaagcgcctgggccagggtccgcgtcgcccaccacagggcgttccgcgacaggctgtaggaaaagaagcgcggatcgggcttcagcacccgctggtccagcaggttgaccaccgacgccccgtcccccgcctgttccgcgaaggcttcggcgagcacgatcggcgcgcgcagattggtctccatgtggcggtcccacagttcgcggccgaggtcgccgacctggtcgtcctcaaaaacagaggcgttgttgaccagcaccttgagcggtcccatggcccccaccgcatcgggaacgagcgcccgtacggcggcctcgtttgaaaggtcggcgcgcaccaccgtcgcacgacggccgatggcgcgtatttcgccggctagcgcctcggccgcgtccgcggacgcatggcaatggatcgccacgtcatgaccggcgcgcgccagctccaggcagatggcccgcccgatccgcttggcgccgccggtgaccagcgccgcgccgcgccctgcctcagtcaacccggccgaactcaaaatagttgatggcggcgaagacggcgacgaaaccgagaatgatcgcgagggccagcatggcgtgctcctgtgaaggtccaaggcatagggcgcggacggcccggtcgcaagcggcgcctccctccgccctctgctaggatcgtttcatgaaccccgcgattctgccgatcctcgtcgtcatcctcgccggcggcgcgaccgcgcttcaggcgccgaccaatgcgaagctggcgacggcggtgggctcgccagtgaacgccgcctttgtgtccttcgccgtaggcacgatcgcgctggcggtcgccgccgccgttctgcacacgcggccggacatgacggcggccaaggccctgcccgcctacgcctggttcggcggcctctacggcgcctgcttcgtggtcgccgccgcctggggcgtgcctcggctgggcgcggccatgaccatcaccctgatggtggcgggccagctggcgctgagcctgctgctggatcacttcggtgcgttgggcgtgccgcgccagccgttgaacctcggccgcatcgcaggcgtggcccttgtattcgccggcgtccttctggtccggcggtcctgaacctatattccgcccgatgaccgaggagaccctgagcgcgctgtccggcggcgacctgaaggccgccgccctgatccgtgacgaggccagtcgcgcgcccgacaagcccggcgtctatcgcatgtacggcgaggacggcgcctgcctctatgtcggcaaggcgcgctcgctgaagaagcgcatcctgcagtatgctcaggggcgctttcacacccagcgcatcggccacatggtgtctctgacccgctcgatggaactggtggtcaccgcctccgagcgcgaggccctgctgctcgaatccaacttcatcaagaagctgaagccgcgcttcaacgtggtgctgcgcgacgacaagtcgttcgccgagctgatgatccggcgcgaccaccgcgcgcctcaggttcgcaagcatcgcggcgcgcacaccgtgcccggcgactacttcggccccttcgcctcgacctgggcggtgaaccggacgctgaacaccctgcagaaggcgtttctgctgcgctcctgctcggacagcgtgttcgagacgcgcacccggccctgcatgctgcaccagatcaagcgctgctcggcgccctgcaccggcctgatctcgctggaagactacggcgccctcgtcaccgaggccgagggcttcctgcgcggcaagtcgcgcgcggtaatcggccgcctgtcgcaggaaatgaccgccgccgccgaggacatggactttgaacaggccgcgcgcatccgcgaccgcatcagagccttgtcggccatcgccatggagaactccgtcagcgcggaaggggtcgccgaggcggacgtcttcgccctgcacaccgacggcggccaggcctgcgtgcaggtgtttttctaccgcgccggccagaactggggcggccgcgcctacttcccccgcgtggaccgggccgacacggacccggagatcctggccgccttcctcggccagttctacgaagacaagcccattccgcgcctgatcctgtccaacgtgcgcccgcacgagctggagctgctggaggaggccttttcgatgaaggcggaccgcaaggtcgagatcgcccgacctcagcgcggcgacaagctgtcgctggtggatcacgccctgaccaatgcgcgcgaggcgctgggccgacggctggccgagagctcggcgcagggcaagatcctggacgaggtgtgcgaagcctttggtctggaaggccggcccgagcggatcgagatttacgacaacgcccacatccaggggaccaatgcggtcggcggcatggtggtcgcggggccggaaggcttccgcaagaaccagtaccgcaagttcaacatccggggcgaggacctcgcgcccggcgacgactacggcatgatgcgcgaggtcatgcgccgccgcttttcgcgcctggtcaaggacgaggaggcgggcgaggacgtcgaccgccccgacctcctgctgattgatggcggcgcgggccagctggccgaagtcctcaaggtcatggccgagctgggggtgcacgacatcgccgtggtcggcgtggccaaggggccggaccgcgacgccgggctggagaagttcttcatgccgggcaggccgcccttcatgctgccgctgaagtcgccggcgctgtactatctgcagcgcctgcgcgacgaggcccaccgcttcgccaacggcgcccacgccaagcgccgctccatggacatcaagaagaaccctctggacgaaatcgagggcgtaggccccggccgcaagaaggcgctgctgcacgccttcggctcggccaagggcgtgggccgcgcctccgtggtcgatctggtcaaggtcgccggcgtcaaccaagccctggccgagcgcatccacgccttcttccacaaggcctgaggcctcttgtcaccactccagaaggcggagcccgagaatgtcgcggaagtcgtcgccgttgcgcgtcaccagcgtggcgccgtacgtgatggcctgggccgcaatcatgcggtcaagcaccttgcggcgcgagaagccgcagatcgaaatgatgttgcggtaagcggctgcttcttccgaaccgaacggcaggaccggaacggcctccagcaaagcgtcaagccgccggcgacgcacgggcggatcagtctgcgaacgcccgagatcggcttccagttctattctcgtcacgatggacagcagcaggggcggctgcaagctatcgacgagttcgtcgacgacgccgtcgccgtcacgcagatggatggcgaggttcgtgtcgaggagataggccacctacaagccgggcctgtccgggatctccacctcatggcgctccccgatgctggagggcttcggcaggctgcgcagcttggccaacgctgctttgatcgacggccgcttgggtgcgatggtcaccacatcgcccttgcgctcgatttcgacctcgacgcccgggccaaaggagatttccttgggcaggcggacggcgtcgctgtttccactacggaatgttcggctgacgatcggcatgaaccgctccttgtatatacgcgtatacacgatttctccggaacgcgcgaacggctaaggcggtatcatgaccgacgacatcgacgaactgaccgccggctaccgacgttttcgcgccgagaaatggccggaggcgcgggcggagtacggggcgctggcgtccgacgggcagaagccgcacacgctgatcgtggcctgctcggacagtcgagccgacccggccttgatcttcgacgccgcgccgggcgaactgttcgtggtgcgcaacgtcgccaatctggtgccgccctatgagccggacggccagcttcatggcgtttccgccgcgctggagttcggcgtcaaggtgctcagggtccggcgcatcgtggtcatgggccacgcctcctgcggcggggtgggcgccatgctgacgggcgcgcctgaagactgtccggacttcgtcgccccctgggtggcccagggaacgccggtggtgcagcacgtcgccgagaccgtggagccggatcaggtggtgcgcgccgccgaggaggccatcgtgcgcctatcgatcagaaacctgcgcacctttccctggatcgccgaacgggaggcggcgggccagctgacgctcagcggcctccacttcggcattgcggacggcgttctgacggccctgacccctgcgccgcggttcgagcccttgccgaccgactgacgcgccgtggacgtcttctacatcaacctggatcgcgccgacgaccggcgcgccttcatggaagcgcaaggcagggcgcgcggccttccccttcggcgcctgcgcgcgacggagcccaaggacctcagacccggcgagtacgagcagttcgcgaacgcctgggaacgcaagctgacgccgaacgagatcgccctgctgcgttcgcacgccgccctgtggcgaatggcgctggatcggcatgaggggctggtggtgctggaggacgacgcggtcctgtcgccgcgcttcgcacgggtcatcgagcggctgcccgcgggctacgacctgatcaatctcgaggatttcggtcgcgccaaattcttcgcccgaaacgcggaccaatcggacgccgacttccgccttacccgtgtcatccgcgacaagaccggctcggccgcctaccatgtgtcgccctcaggcgccgccaagctgttgaagcggatggagacgacggccgcgccgtccgacgcttttctgttcgccgtcgcgcggctgaacatggcgcaggtggagcccgcgctggcgcgtcaggcccacatcctgaccgagcgcggctttgatcccggcatcaccatcgccacctcgatctgcaaggagcggatcggcgcgcccaaggagcgcaagcggccgatctttgcggctcggcgggttgcgacgcaggttcgtctggcgggcctgcacctgcgccggccgctcgacgtggtgctgcggccggtttcattcgatgacgccgagttccgcgccattctgccgatccgcgtcgatcagccctgatcccacaggcgccgataggcggcgttgaggccctcggcttccacctccagcgagaactgcgtttcgacccggctgcgcgccgccgcgcccgccttggcccgcgccgcatcgtcgtcaagccatcgccccaccgcctccgccatggcgtctgcatcgccgggcgggatcagcgagccggtctctccgtcgatcaccagcttcggaaaggcgcccaccgtagtggcgaccacgggcgcgcccgacgccatcgcctccagcggcgtgacgccgaagccctcccagcgctgcggtgcgacatagaggcaaagcgcgcggtagtaggccggcgtctccagcggtcccacctcgcccggaaacaggatgcggtcgttcaagcccgccgccgccacgcgcgccttcagctcgtccaggaagtcctggtgctcccccgtcgcgcgacccagcaccaccgccttgacgtcgggccggtcgggaagcacccggatcatggcgtccacgaatacgtcggtccccttctgcgcccggatgcgcccgaaacagccgaccagccgtccgatgggcggcagatcggccgggcgcgcttccccggccctcgcagggcggaacaccgccgtgtctatgccgtgcatcaccacgatggaggggcgctgcagataggccgcggtgaaatcggacaccgacaccaccgcgtccatccgcccgatcagaaaccggctccagcccgtgtgctttctttgcgaggcgctggtgaacaccagtttcagcggaaagcgcagcaggtcgcgcaagacaacgccggccagcatttcgacgttgcggcgcgcatgccagatgcgaaacggccgatcgctggggcgtctcgccaggcgcaggaggtctcggaaccgcatctgcgggatttcgtccggcacgacaggtcccagcaccgcaatgcgcaccgaccgggcctgcaccggagcgacgcggaacagggtcgtggtcacgcccgaaagccgccgcttgaagttgggcgcgatcacctgcggatcggagacaagggtcctcatgcgtccttgcgtagcgaagatgcggcgacgctgcatagagaagacttgcgacgatccggccgctagaagcgttggcttcgcagtttccgctgtttctcgaggccgcccgtgaccccgacccgacccaatccgatccccaacatcctgaccgcgatccgcctggcggccggggtggtgatgttcaccatgctggcgggcgcggcgccgggcgcgctggacgcggtcctttctcccgaagcgcagcaggacttcggcgtctgggcgttctggatcttcgtgatcgcggcctccacggattgggtcgacggcttcctggcgcggcgctggaacgctgtcagccgctggggcgcgatcctggatcctatcgccgacaaggtgctgatcaccggcgcgatcctgggcgtcctggcttcgggctccctgcccggcatcgccctgccctgcggcctgatcctgttccgggagttcgcggtgtcagccttgcgtgagaccaccgccggacgcgtccagctgcccgtcaccctgctggccaagtggaagaccacgctgcagatggtggccctggccgcgcttcagctgacgctgctctggccggccttcggcctacagcaggcggacggatcgccgctgtcgtggcaaccggcgtttgaatccttcgccgtattcctgacctggttcgcggcggtgatcaccgtctggaccggctggcagtatttcagcgaggcgcgccgccagatgagcggcgcctagggcctcagcgtcaagcccgcaggcgaggcctcgaagcgcgacagccggcctaggtagctcatgcccagcagcgaatgggccagaccttcctcgaccaccagcgcctcgaccttgcgtacggttgcaccggcaacggacaccgatgcgagggtgacggatgcggccttggcctcgccggatgcggtctgcaccgcccggttgaagtccgccgaggtgaccttcaggcccagacgctgggcgtcctggcgcgtcagggcgaccacggtcgcgcccgtgtcgaccagcacccgcacggcgcggccgtcgatctcggcctccgcccagtaatgaccatcagcgccgcgcaccacctgggccgcgtgaccgctggccggcggcccggcgatgggcgcgacggtcacgaccgctgcctgcgcctgtccgcccgatgacaggtggttcaggccgtaggccgcgccgagcgacgccaaaagggccgcgccgaggacgaatgacgactggatggccttgtcgaacatgagaacccacacagaatgtcgccggtcgtgcgacttcggctggttctagggacttacagttggcgcccgatgaagcgacgtgcctgacgaaaggttacggctcagccgacgtcatccatcctctcccgacgcagcggcagctcggccatgacccgtgcgcggccatcatcgccgagcgcgcgccagccggcgatctcctgcagagtgcggaagcagccgaggcataggccggacgcgccgtcgatcgcgcacacctgcacgcaggggctcgcaatggatttgggcggcctggcgggcggtgcagcggccgtcctcatccctccattttcatccgtttcttgcatttctgtcgcatacctgtcatatcgaacctgacgcgaaacgactgaagcgggtgagatccccccacaagcacgacgcgtctcttttcatcgttctgcgaaaggagacgccaagatgaacgataaggagcgcaacctccagcacgccatgatgtccttcgccctgtggggcgggatgctggtgaacacgcggcacatgccttcgaactcgggtcgggtggtcagccatccctcgaacttcgtgcccatcgagatcaagaagcgcggctgaccccagcctcctgaaaaaccaacagagccccggccccctcgccggggctttttgcatgggcggccttgcatgacgcgacggcgcggggcgaagacgagccaaggcttcaggagaccgccccatgccgctgctcacagaggaacgcctggacggcgcggacgcccgcgtggtcgtcctgacgctggaccgcccggagaggctgaacgccctgcccgatctcggcgacggcgacgaggtcgcggcggcgtgcgagcgggtgaacgccgatccctctgtccgatgcgtcgtgctgaccggcgccggccgcgccttctcggccggaggcgacctgaccgccatgcgcgaccgccgcgacctgttcgagggctcgggcgcgcagatccgcgaacgctatcgccgcgtggtccaccgcatcgtgcgctcgctgtatgggcttgaggtcccgctggtggcggcgatcaatggaccggccatgggcctgggctgcgacatcgcagggcttgccgacatccgcatcgcctcggaccgggcgagtttcggcgtgccgttcctgaagctgggcatcatcccgggcgacggcggctcgtggctcctgccgcgcaatgtcggctatgcgcgcgcggcggagatgctgttcaccgcccgctccatagacgccgaaacggcggagcgctggggcctggtcaatcgggtcgccccgcacgatcggttgatggaggaggcggcaagcaccgcccgccggatcgccgatcagccgccgcaggcgctccgcatggccaaggccctgctgcgccagggtcgcgacgccaacttcgaccagatgctcgagatgtcggcggccatgcaggcgctggcccacctgaccgacgaccacgccgagggcgtggacgccgttctgaacaagcggccggcgaacttcaccggccgctgagcccgcgccgatcaagcggccggcttcatcgcccggtccggaccaacgcccgccgccgcggctcgcggcgcgccggcggtctcccccggcttcatgaacttgaccaggacgcgctgaccgatcagcagcggggcgtcgccggccgagaccaccacctcgaccacgcgttcgtccgtccgctgcgatgggtcgtccgaggccagcttgcgggcgccgaacacggcggcgcgccgcatcaccgatccgatatagacctttgtggcgtcgccctcgggcgagatttccaccgcctggccgtcgcgcaggttgggcagatcgctctccaccacctcggcgcggatgatgcgcggcgcgtccggctccaggtcgaacatggtggacacgttcagggtcgaggcgcccgcacccggattggcgtagcggcggacgatgcggccggccatgggcgcgcggatcaccgtcagctcctggttgtagcgggcctggtcgtactgggcgcgcgccgtctgaaccgccgcctgctgggccccgagctgagcctgggcggtcgagatggcgtcctgagcctggtccatgcgctgcgcggcgacgaagttggtggccaccagccggcccagccgttcatgctcgcgctgagcggtgcggatggcgacgcgggtctgggccatctggctctcggcctgcgacacggcggcggccgcgctttggaccgaaaggcgagcctcgtcatcttcctgacgcgccaggatttggccggcggtgacgcgctcgccttcctgcaccagcacctcgcgcaccacgccgccgcgacgggccgcgacctggatcagtccgccctcgatgtccacgcggccattggcgatggcggcgtaggggctctcgaccttggtctgggcggccttgtccagctcggccttcttggccttgccggcggcctgcaggctcatgaagcccacaaccacgacgatgaccagcaggatgccgatccagaagcgcttcttcttcaaaagggcgggcatgggcgttcggtcctaagtcggtcgtttcagtggtgcaacgccagaacggcgtccggattaggcgtgcggcgctggtcgtccaggatcttgccgtcctcgatgtggatgacccggtcggcccaggcctccaggcgcgggtcgtgggtcacgcagatgacggcggcgccgtgctcggtcgccgcgcggcgcagcaggcggatcaccacctgcccgttctcgccgtccagcgccgaggtcggctcgtccgcgaacagtatcttggggtccttggccaaggcgcgggcgatggccacgcgctgcttctcaccgcccgacagggccgccggccgctgatgcagacgatggcccaggcccacctcctccagcgcggtcgtggcgcgcttcctggcctggcccgaggtcagcccctggaacttcagcaccgtctcgacctgctgcagcgcggtcagcgatgggaacaggttgaagccctggaagatgaagccgcagttatccagccggaacttgtcgatgcggccggtggacagcttccacaggtcgtcgacctccagcgcgtccacccgcccctcttccggcttcagcaggccggacagggcggcgatcagcgtcgacttgcccgaaccggacggacccatgaccatggtcaggtcgccgtggcgcgcgtcgaagtcgacgcccttcagcacctcgacccaggccttgcccgagcggaaccgcttgaccagggaccgggcctcgatggcgaagtcgccgtgcttgccgtgaaccctggcggaggcgaaagatatgtcgttcatcgcagcaaatccgcaggctggctcttcttcaggatgccgagcgacaggagacccgagcccaccgcgatcaggatcaggccgatgccgaccacgatcagcagggtgaacggcagggcgatgatcaccgcgcccgcccgcgccgccagcgccagcagccaagttaggcccacggcggcgatcacgccgaccacgccgacccagaagctcagctccaccacgatgcggcgcagcgatcccatgccgacgcccagcgcccgcagcgaggcgaactccttgatgttggccatgatcgcgccgcgcagcgtctgccaggtgatggccacgccgatgatgacgcccaagaccacgcagccgccgatgatgatcatcaggatgccttcctcgaacatggcgccctggttggcgtcggccagctgctggcgggtccaggccttccactgaccggcgcccgtggcgttcagctcggcggccaccacgtcggcggtggagggatcacgcagcttgatcatcagggggccgactcggggccccgtatcggcctgcccgaccatgcgcagggtgtcgcgcgacatgacgatgccgggctgcatcatgttgggatagccgcgcgtcaccccgaccaccgtcacggtctgaccgttgtagagcgccttgtcgccgagtttgacgcccagcgttctcagcgccgtctcgtccaccgccacggtgtagggctggcgcaacgcgtccacgaggtcctgcgaatagtcggtcggaatggtgaccgagccgggccgcgtgtcgatgatggaggtctggacgaacttctgccgcggcgcgccctgcttggcgcgatccgcctggctggcggtcggatccacgttcttgatgttctgaaaggtgccgccggccccgtccagcggctgcacctcgaccacctcgggatggttgtaggccagggggatgaaccggcgcggcacgcccgaggggccgcccatcaggctcttggcgcccggctgcatgatgaagatgtcggcgcccgatcgttcgatctgcgcggtgaagctcttgccgatgccgatgaagacgccggtcatggccagcaccagcaggcccgacagcgcaagagccatcacggccgccatatagcggcgccactcgaacagcagcgtggaaagcgcaagcgacatcagcgtcatcgtcccccgatcacggttctcatctgcggccatcgtcgtcggcggccaagttaaatcggggtaagcttgcgcgacagaaccgccgattgtgcgcgcctcgcggcggcgctatggcgaaggggcttggcgcggccggcaaggcggcgttagttatgaaataacagcaggagcatccggctcctcgccgggagacctccgccagatgtcgcttcgttcgatccgcctgtccgcctcgctcgccgcgctcggcgccgcgaccgccgtcctgtcgttgcccgccgcgcccgcccgcgccgacgagggcatgtggaccttcgacaacttccccatcgcgacggtgaacgaaaagtacggcacgaacatcgatcaggcctggctggaccgtgtccgcaacgccgccgtccgcctgcagggctgctcggcctccatggtgtctaacgaaggcctgatcctgaccaaccaccactgcgtggtgtcctgcgttcaggacctgtccaccgccgagaacgactacgtcaagaacggctggatgcccgccacgcgcgaggaagaaaagaagtgccccggccagacggccgaaatcctgacggacatcgtcgacgtgaccgaccgcgtcacaggcgcgggcgcaggcctggaaggcgccgcctttgttcaggcccgcgccgccgagatcgaccgcatccagaaggagacctgcggcgatgaccagaagctgacctgtcaggtgatcagcttctatcgcggcggccagtacaagctctacaagttccgcaagtacgacgacgtgcgcctggccttcgcgcccgagttccaagcggccttcttcggcggcgatccggacaacttcaacttcccgcgctatgcgctcgatgcggcgtttcttcgcgcctatgaggacggcaagccggtgtcctcgcccaacttcctgaagtggaacccgaacgcgccagccgagggcgacgtgacgttcgtcgccggcaatcccggcacgacccagcgcctgctgacggtggcccaactggaggtgctgcgcgaccagcagctgccgctcggcctgatccagacctccgagctgcgcggtcgcctgctggagtattccaccagggacgaagaagccaagcgcgtctcggtcgatccgatcttcggcctggagaacggcttcaaggtccagtacggccagcagggcgccctgacggaccccgccttcatggcgaccaagcgccaggaagaggccgacctgcgccagcgggtcgccgccgacccggccctggcgcagcgcatcggcgatccgtgggccgatctggagcgcgtgtccgccgcacagcgcgacctgttcttgccgtatcgtcagctggaaagcgccgccggccagcgctcgtctttgtacagctacgccaaggccatcgtccgcgcctccaaggagcgcgctaaacccgcgtccgagcgtcgcgccggttacggcgacgccgacatcgccaccctgggtcgtcgcctggccactgaaacgccgatctccaacgatctggaaaagatctatctcgatttctggctcagcaagacgcgcgagtatctgacggtcgacaacgccgacgtgaaggcgctgctgggcaaggaaagccccgagcagatcgcggagcgtctggtggacggcaccaagctgggcgatcccgccttccgcgcccaggccttggccatgacgccggagcagctggcggcgtcgggcgatccgatgatcgctttcgtcctcgccaacgacgacgccgcccaggcggtccgcacccagtgggaggcggcggtgtccggcccgaccagccgcgcgggcgagaagatcgcccaggcccgcttcgccgcttacgggaccaacctttatccggacgccaccttctcgcttcgcctgtcctacggtgcggtgaagggctggacctatcgcggcgtgacggtcgagcccttcacccggatcggcggcctgtatgagcgcaacaccggagccgagccgttcaatgcggccgaggattggctggccgccgagaaccgcgtcaacaaggacacggtcttcgacttcgtctccaccaacgacatcatcggcggcaactcgggctcgccggtgatcaacgcccggggcgaggtgatcggcgcggcgttcgacggcaacatccactcgctgggcggcagcttcggctacgacggcgagttgaaccgcacggtgacggtctccaccgccgccgtcaccgaggccctgcgcaccgtctacaaccagccgcgcctgctggaagaactgggcgtgcagtaggacgaccgactctcctccccatcgcctgcgatggggagggggaccgcgaagcggtggaggggtttctccaccgcatgaaagatggggtgtatcaaagaagcccctccgtcacggtgctgacgcaccgcgccacctcctcactcgctctgcgagcatggaggagaaaaggacctgtccatgcgtttcgccctcgccgcctccgccgccgttctcgctctcgccgccgcgtcttcggtcagcgccgaggagggcatgtggacgtttgacaacttccccatcgcccgcgccaaccagacgctggggaccagcatcgaccaggcttggttggacaaggcgcggatgtcgtcggtgaagttcggcggctgctcggcgggcctggtgtccggcgaggggctggtgatgaccaacaaccactgcgtggccacctgcgtcgccaacctgtcgaccccgcaggtcaactacgccgagaccggcttcacgcccaagacgcgcgaggaggagcgccgctgccccggcgcctcggccgagatcctgacggacatctccgatgtgaccgagcggatgcagaaggccggcaagggcctgagcggccaggccttcacccaggcgcgcgacgccgaggccggccggatcgagagcgagggctgcgcgggcgaccccaaggtccgctgccaggtggtcagcctgtaccgcggcggccagttcaagctctacaagttccgccgctacaccgacgttcgcctggccttcgcgcccgaggatcgcgcggcgaccttcggcggcgacctggacaacttctcctttccccgcttcgccatcgatgcggcattcatccgcctgtacgaggacggcaagccggtcgacacgcccgtccacttcacctggaacgccgggcggcccaccgagggcgagccggtgttcgtgtccggcaaccccggcgcgacccagcgcctgctgacccaggcccagctgtccaccgtgcgcgacgtggtcctgccgatggaccagctgatcgcctccgagctgcgcggccggctgatccgcttctcggaagaaagcgacgagaacgcctttatcgccatggaccccatcgtgggcctggagaacacctacaagcgcggacgcggacgccaggcggcgctgatcgacgccgccttcaccggccgcctggccgaggccgaggccgacttccgccggcgtttcgccgccgatcccgccgtggccgcaggcggcgatccgtgggcggcgctggaggcggtgcagccgatccagcgcgagctctatcccgcctacgccctgctggagggacgcgccgggggcgggtcgtcgctgtacggcgccgccgtgtccctggtgcgcgccgcgcaggaacgcgccaagcccagcgccgaacgcctgcccgaattcgccgacagccgcctgcccgcgctcgagcaacgcctgctggccgaacgtcccgtctatccggcgctggagcaggttcagctggaatggtggttgtccaagacgcgcgaatggctgaccgtcgatgatccgcgcgtccgcggcctcctgggccaggagagcccggaagccctgtcggcgcgcctggtcgagggctccaccctgggcgatccggccgtccgccgcgcgctgtgggaaggcggcctgccggcgatccaggcctccaccgacccgctgatccagcacgtgctgcgcaccgacccggccgcccgctctgtccgcgccgagtgggaggagaaggtgcaggccccgaccgaccgcgcctccgaacagctggccgccgcccgcttcgccgtctacggcgacagcgtctatccggatgcgaccggcaccctgcgcctgacctacggccggatcgaaggctcggacgttccgggccagcgctggggagccttcaccaccttcaacggcctgtgggatcgtgcgaccggctcggcgccgttcgacgttgcgcccaggctgctggcggcgcgcgagcggatcgacggcgacacggtgctgaacatggccctgtccaccgacaccatcggcggctcgtccggctcgccagcgatcaacgcgcggggcgagatcgtcggggccaacttcgattcgaccgtgctgacccagcggaacgcctatggctacgaccgggccgtgaaccgcagcgtgatcgtgaccacgggcgcggtgacgacggcgctgcgcgacgtctacggcatggacggcctggtgcgggagctgggcgtcacgcgttgagcgcgctcgctttccgcccggccggcgcgggcgacatcgcgcgactgcaccggctgatcgagagcgcctatcggggcgacgccgcccggcgcggctggacgcacgaggcggacctgctggacggtcaacgcaccgacgccgccgagttgtcggccctggtcgccaatcctgcgcgcgtgctgctgatggccgaacaggagggtggtctgatcggctgcgtccaggtcgcggacctgggcgacggcctgggctatctcggcatgctgacggtcgatcccgagcggcaggcgggcgggctgggtcgtgaactgctggaggcgggggaggcctgggcccgcgaccgcttcggcgcgcgcgccatggagatgacggtcatcgcccggcgtcgcgaactgatcgcctggtacgaacggcgcggctatgcgctcacgggcgagacacggccgtttccgatggacgatccgcgcttcggccttccgcgcgagcccttgttctttgtggtgctgcgcaagcgtctttaatccgtccgggcgcggctggtcaggaacgccttcaacgcggcgggccgcacgggcttgggcatcagcacggcgcccgccgctagggcccgctcggacaaggcctcgtcggtatccgccgagatcagcgccagccgcgctccctgggtccgcccgcccgcgcgcagggcggcgatgagctccagcccatcggcgccctcgcccagatgcagatcgaccaggatggcgtcgaaggggccattcgccgagacggcgctgtccgcgtccgccgccgtcacaacctccacgccccagcggcccaggagggcggataaggcctcgaggatcgccggctcgttgtcaacgcacagcacgcgggttccgaccagcggcgtcttgatgccggctgtaaccacgacggtggcggccggggcggcacgcggcgcggtcagggtgaaggtcgatccccttcctacctccgagcgcagcaacagcggataatccagcaacgccgccacacggcgcacgatggcgaggcccagaccggcccccgtctcatcgccgccgcgcccggccagccgggtgaaggggccgaacaccgcctcctgctgttcggccgggatgccgcgcccggtgtcgtgcacctcgaaacacagggcgccgccgctgcgtcggacgcccaccacgatcccgccctgatcggtgtagcggatggcgttgccgatcaggttctgcagcagcgatcggagcaggtcgcgatccgacaggacccatgtccggctggagacgatgcgcagcctcaaccccttgccgcgcgcctggggaatgaagtcgcgcctgagctcttcgaacaaagcctcgaccgacaggggcgcgaccgccggcttgaccccgccggcctcgagccgcgacaggttgagcagggccttgagcatgccatgcgcgctttcgatcgagcggtcggcgttgtcggccagcgcgcgtccgccctctcccggctgctccttcagggcggcgatgaacaggcgcgcggcgtgcagcggctgcaacaggtcgtggctggcggcggccaggaaccgggtcttggacgccgtcgcctcttccgccagccgacgcgcctcctccagccgttcggtgcggtccgcgacgcgggcctccagcctttcgttggcctcggccaaggcctcagccgcacgccgcagttcggtgatgtcggtgtagctggtgacatagccgccgcccgccatcggcgcgccggtggagcgcagcacgcggccgttcggctgaatccgctcatgactgtgcggaatgcggcgagccagcgcctccagccgccgctcgacccaggcgccgatgtcggccgccggcgcctctccgcgctcggcgttcaggcgatagacttcggccaccggcagacccacgtggacgaagccgggcggcaggtcgaacagctccacatagcgcgcgttccaggcgatcaagcgcaggtcggcgtccaccacgctgacgccctggtcgatgttgtccagcgtggcctgcagcagttcgcggttgaactggacggccagcgacgcctcgtccagcatccgcaccacgtcctcgggtgcgcggcctccgccggccagagccgcggcgatgacccgccgggccgatgaggcgcccaccgcgcccgccagcatccgctcggccgcgcgcgccaggccggcgtctgcggggtccgcgtccttcaaggccaggcccgtctcgcgggcgtgcgcctcgaacgcccgccgcgcggagggatcgccgacgaagcgggccaccagggtcttgaggtcgccgaccgacgctccggacggcgcgctgtcgcgctcgcgccagtccgggctgatccgatcgacgaaagcgcgggcctgcacccggtcgatcaggcgcgggcgcgcacgcctggagacgaccacatagatcagcgtattgatcgaaaggctcagcaggacgccgaggggcaagggatcgtcgaggccgagcggctgtcctcccgtccagcccaaggtcccgccgacctggggccaagccatcagcaccagccagatcacgctgccggccgctatgccggcgatggccccgcgcgcatggccgtcgcgccacagcaccgcgccgaacagggccggcgccagttgcgccagcgccgcgaacgaggtcaggccgatgctggccaggccgctcgagcggtcgatggcctggtagtagagccagcccaggaacaggaccagcgcgatcaccccgcgccgcacctgcaggatcacgccggccatgtccgaggcgtcggccctggcgcgccagcggtcgcgcgccgccaggggcaggatcaggctgttggacgccatggccgacagcgccaccgcctccacgatcaccatggcggtggcggccgagaagccgcctacgaacaccacggtggtcaagaggccggagccgttgcggaacggcaggtccagcacgaacaggtccgggtccgccgcgcccgcgaacagcccgccggccgccaccagcggcaacaccgccaggctggtgatcagcagatagagcggaaacacccatcgggcgcggcgcacatgatccggctccgacgcctccacaaaggcgacgtggaactgacgcggcaggcagaacaccgccagggtcgccagcagcgtgatcgacagaaagcgcgcgtccacgtccggcggtgcggccagttggccgaggctgagcgccgcctcctcgcgtgatgcgcccagcagcagcaccacggcgaacaccgcaaccgcgaccagggccgcgagcttgaccacggattccagggcgatggcgcggatcaggccgcgattgtgctcggtcaggtccgggcgacgcgcgccgaacaggatggcgaagccggcgagcacggcggccatcaccgcgaccgtgggcccttccgagccctcgaccgccgtgttccgcgtcaccagctcccacgccatggaaagcgatttcagctgcagggcgatgtaggggatcgagcccacaatggcgacgcaggcgaccagcgcgcccaggccctggctcttgccgtatcgcgaggaaatgaagtcggcgatggagcccacgttctcgcgccgcgccgccgccgcgatgcgccgccagatgggaaacagcaccactaggccgatcaccggcccgatgtagatcggcagatactcccagccgtttcgcgccgccgtgccgaccgcgccgtaataggtccaggaggtgcagtagatcgacagcgacagcgggtaggcccacggccccagccggttgtgcgcgcctgtcttctgctcgccgcgccaggcgacggcgaacagcatggccatataggcggccaccatcaccaggatcatcaggctgggcattggcttgatctagaaccggcgttcgtgatctgcgcaagcgaagagcgggccgacctctcggccgacccgccctccatccgcgcctgaaagcaggaaatcaggcgttgatgtctacgtccttgccttccttgaccagcaggaagcccagcacgaccgtcgcgacagcgacgatgatcggataccaaaggccggagtagatgttgccggtcgccgccacgatggcgaaggccgtggtcggcaggaagcccccgaaccagccgttgccgatgtggtagggcagcgacatggaggtgtagcggatgttggtcgggaacatctcaaccagcgccgccgcgatcgggccgtagaccatggtcacgtagaagccgaggatgaacaggatcagcaccaccatgggcttgttcaccagggcgctgtcggccttggccggatagccggcggcggccagctgttcgcccagccccgcgtcccaggtcttcttctgggcagcgaagtcggccgccggcagcgtctcgccccggaagctgggcaccacggcctggtcgccgatgcgcacctcggccaccgtgcccgccggcgccgcgacgttggtgtaggtcacgcccgccttggccaggtaggacttggccaggtcgcaggagtggttaaacaccgtcttgccgaccggatcgaactggacgttgcaatcggccggatcggcatagaccaccaccggcgcggaggctgcggcagcggccaggcgcggattggcggcctcggtcagggcgtcgaacagcgggaaataggtcacggccgccagcaggcatccgcccaggatgatcggcttgcggcccaccttatccgacagccatccccagaagatgaagaagggcgaagcgagcagcagcgcgatcgccagcatgatgtagaccagcgacgcgtcgacccgcagcacccgctccaggaagaacagggcgtagaactggccggtgtaccagatcacggcttggccggcggtcaggcccaccagcgcgatcagcaccagcttcaggttcggccacttgccgaaggagtccttgagcggcgtcttggagcccttgccctcagccttcatctgcttgaacgacgggctttccgccagcttcagccggatccacagcgatacgcccagcagcaggatcgagaccaggaacgggatgcgccagccccaggcggcgaaggcttcctcgcccaccgagaagcggacggcgagaatgaccgcgaggctcagcaccagccccgccgtggccgtgatctggatgaacgaagtatagaagccgcgctttccatgcggcgcgtgctcggcgacgtaggtggccgcaccgccgtattcgccgcccagcgcaagaccctggatcaggcgcatcagcaccaggatgatcggcgcggcgatgccgatggcggcgtagggcggcagaaggcccacgacgaacgtcgacagccccatcagcagcatggtcaccagaaaggtgttcttgcgcccccacagatcgcccagccgaccgaacacgatggccccgaacggccgaaccgcaaagcccgccgcgaacgccagcagcgcgaagatgtagccggtggtctcgttcacacccgaaaagaactggaccgtgatgatcgcggccagcgagccgtaaaggtaaaagtcgtaccattcgatcacggtgccgaccgaggaggcgaggatcaccagcttgtcgtttcgatcgacgaccttggtctcgcttccgggcgcgccgatggcgctgtctgtcatagatgttcctcccgtcatggccgttgtcggcgcttgtcccgagccgtggcggcgccgagtttgacgagagactgacagcggcgcttgctgctggagagagcgactttcgtctaagcctgccgcatcttttttgctgcgacagccggtcgcacccttgcgaaacggacaccgatgtccactttcgcatccatgagccggcccgcccgcaaggatgtcgtacagaaccgcacggccttgctgcacgccgcgcgcgaagtgctggccgagcaggggctggaggcgccgctggatctgatcgccgagcgtgcgggcgtgggccgcgccacgctgtaccgccacttcgcggatcggaccgaactggtgctggccgtgctgatcgacggggtcgaggacctgcatcgccgcacggttgaacagggtgacgccccagaggtcttcttctggtttctggacgagctggcggcgctgctgatcaggaacgccggcctgtccggcgtgttgcggacggtgcggtcgcccgatgcgctgacgccgcttcgatccaagctggcggaggccggcgcagggcccctcgcccgcgcccaggcggcggggctggtgcgaaaggacctgggtcccatggacatgcggctgatcgcgacgcttctggcctcgggctttcacaacgcggacgccgccgagcgggaggcggtcagccggcgcacccgcgccatcatcctcgacggcatccgcgcgaggccgcaatgaagccgcgccacgatccggcctgggacgccttcgccgccaccctgcagccgcacgagatgccgatgtttccgggctcaccggcgacgcccgcgcatcccgcccgcaagcggctgcagttcttcttcaccggcctcctgatcgcgatgagcggcagtttcggcaatgcggcggtgaccgccaatctgcagaacctgcaaggcgcgctcgggatcacgcccgtcgaggcggcgtggctgccggtcgtgttcgtcatgaccaacgcctgcatgaacctgatcctggtcaagttccggatgcagtacggcctgcgcctgttcacccagatcgcgctggcggtgttcgtggtggtgaccttcgcctcgctgttcgctcacgactacggctgggcgctggccagccgggccgcatcgggcgtggccgccgcgcccctgaccagcgcgggttttctttacctgatccaggcctttccgcccgcgcaccggcttaagggcctgatcctgggcatcggactggcgggattctccgtgccgctggcgcgtctgacaacgccgcacctgctggagatcgacggctggcgctcggtttatctgctggagatggggctcgcgctggtgtgctgggccgcgaccatcctgctgaggctgccgctgtcccagcgcttccgggtgttcgacaagctcgacttcgtcaccttcgccctgttcgctccgggcgtggcgctgctgtgcgcggtgctggggctgggccgcatcgtgtggtggaccgaggcgtcgtggatcggcctggcgctggtcggcgcgatcgtgctgctgaccctggccgtgatcgtggagcacaaccgccgcacgcccctgatcaacacgcgctggctggccggagcggaccttctgcgtctcctgggcgccattctgctgctgcggatcgtgttgtcggagcagacggcgggcgcggtggggttccttcaggtggtgggcctgggaccggaccagctgaacggtctgttcgttgtgatcctgctggccatggcggcgggcaccgtggtcagcgccttcaccttgaacctggccaagctgaacaagcccatcgccctggccctcgcgctgattgcggctggcgccttcatcgacagccattccagcgcgctgacgcgtccggtgaatctctacttcagccaggcgctgatcgcgttcgcctccgccatgttcattggcccggccatgatgatcggcatcaccaaggtgttgcaggagggcaagcagaacttcatcagcttcattgtcatgttctccttgctgcagaacgtgggcggtctggccggctccgcattgacgggcactgttcaggtcatgcgcgagaagttccattccaatcaactggcggagggcgtcaccctggccgacccgcaggtggtccagcgcgtgcagcagctgtccggcgcctatgcccacaccctgaccgatcccgcgctgcgcaacgctgaaggggtcgccttgttgagccggcaggtgacgcagcaggccaacgtcctcgcctacaacgacgtcttcctgatgatctcggcgctggccgcgctggggtgtctgtgggtgacgatcaaccacctgcgcccgcgctggaaggcgcggcgcgccgcccgcaacgaagcggccgcccaagccgccgccgtcgccgccgctgactgaacgagcccccagatgaccgacaccgcaccgcccgccccgtccgctccagcgcccgcgacagccgccgcaacgccgcccgcaccgcagccgagaaagcgcatcctgtggaccgccgtggtggtcggcatcgcggtcctgggcgtgctgctggtgctgtacgcctggaagctgccgccgttttccagcggggtgcagaccaccgacaacgcctatgtgcgcggccaggtgacgctgatcagcccgcaggtggccggctacgccaccgaagtcgcggttcaggactatcaggtggtgcaggcgggtcaggtgctggtccagatcgacgaccgtatctaccgccagcggctggagcaggcgcaggcggccctgcactcggcggaggccgcgctcgccaactcggcccagagccaggcctcggcgcgcggctcggtggcccagcagcgcgccgccatcgccggagccgaagcgaccctggcgcgggcgcaagccgacgccaaccgcgcccgcacgctgagagccggcggctgggtcgcccaggccaacgtggacgtcgccgaggcggcgctgcgctcggcgcaggcccaggtggcccaggcgcgagcggcggaaggcatcgccgagaccggcgtgacctcggccgtggtcagccgcgaaagtctggtggcggcggtcgagaacgcccgcgccgccgtccgactggccgagatcgacctggccaacacccgcatcaccgcgccgcgcgccggccgcctgggcgaagtcggcgtgcgccagggccagtacgtcaccgccggaacccagctgatgggcctggtgcctgatgcggtctgggtggtcgccaatctgaaggagacgcagatgcgcaacatccgggtcggccagccggtcgagctgagcatcgacgccctgggtcgccaggagctgcgcggccgggtcgagcgcatctcgcccgccacgggatcggagttcagcgtgatccgcccggacaacgccaccggcaacttcaccaaggtcgcgcagcgcatccccgtgcgcatccgcatcgagccgaaccagccgctggccgagcggctcagcccgggcatgtcggtggtggcgcggatcgacacggcggccgaccggagctagccctcgatactggccgtcagcgaggacatggaggtgaacgccgtgcagcctgaacccgaactctacccggtgtccgaaaaaggcgcggcccgcgctcacatgaaccgcgcggcctatgaggcggcgcggacggccgctcagcagacccccgacgccttctgggccgagcaggcgacgcggctggactggatcaagtcgccgaccgagatcaaggacgtgtcgttcaacaaggacgacttccgcatccgctggttcgccgacggggtgctgaacgtctcggccaactgcatcgaccggcacctgccgcaccgggcggacgagaccgccatcctgtgggaaggcgacgatccggcggacagccgcgccatcacctacggcgagctgcacgccgaggtgtgccgcatggccaatgtgctgaaacgccacggcgtccggaaaggcgaccgcgtcaccatctatctgccgatgatcccggaagccgcctacgccatgctggcgtgcgcgcggattggtgcggtgcattcggtggtgtttggcggcttttcacccgacagcctgtgcggccggatcgaggactgcggctcgacggtggtgatcaccgccgacgagggcctgcgcggcggcaagtctgtgccgctgaaggccaatgtcgacgccgctttggagaaggtgtcggtcaacgccgtgctggtggtccgccgcaccggcgcggacgtgccgatgcaagccgggcgcgacttcgactatgcggccgaagcggccgaggtggaggccgactgcccgccagagccgatgaacgccgaggatccgctgttcatcctctacacctccggctcgaccgggaagcccaagggggtgctgcacaccaccggcggctatctgttctgggccgcgtggacgcacgcgctggtgttcgactatcgcccaggcgaagtcttctggtgcaccgccgacgtgggctgggtgacgggtcactcatacgtcgtctacggtccgctggcgaacggggcgaccagcctgatgttcgagggcgtgcccaactatccgaccgtcagccggttctgggaagtcatcgacaagcacaaggtcgacatcttctacaccgcgccgaccgccttgcgggccctgatgcgagagggcgacgggccggtgaaggccagctcgcgcgccagcttgcgcctgctgggcacggtgggcgagccgatcaatccggaggcctggcgctggtaccacgaggtggtgggcgaaggccgcctgccgatcgtggacacctggtggcagaccgagacgggcggcatcctggtctctcccctgccgggcgccaccgacctgaagccgggatcggcgaccaagccgctgccgggggtagagctgcagctggtggacgccgagggcggcgtgctggacggcgcggccagcggcaacctggtcatcaccgacagctggccaggccagatgcgcaccgtctatggcgatcaccagcggttcttcgacacctacttctcgacctatccgggcaagtatttcaccggcgacggctgccgccgcgacgaggacggctattactggatcaccggccgggtggacgacgtcatcaacgtctcgggccaccgcatgggcaccgccgaggtcgagtcggccctggtgctgcacgacgacgtggccgaggcggcggtggtcggctttccccacgatatcaaaggccagggcatctacgcctatgtcaccctgaacacgggggtggaggcgaccgaggacctgcggcgcgaactgatcgcccatgttcgcaaggagatcggccccatcgccgcgcccgacgtgatccagtgggcgcccggcctgcccaagacccgctcgggcaagatcatgcgccgcatcctgcgcaagatcgccgagaacgacatcggcgcgctgggcgacacctccaccctcgccgaccctgcggtggtgaaggatctggtgaagaaccgagcggggtaagccgccgggcgggatgccggccgcgctgacgccctaacctttgacccgccaggtggcgcccttgggtccgtccatgacaacgacgttcagggcgttcaggcggtcgcggatacggtcagcctcgggccagtccttggcggcgcgggctgcggcgcgttgttgcaacaggacctcgacctcggcgcgcagagcgtcggagacctccccctctagccaggcggcgggatcggactgcaacacgccaaggatggaggcgcaggcgatcagccgccccttggcctgagccaccgccacatggtcgcccgccgtcatgccgcgctcgatctcgctggagagggcgaacaggctggccatggcgcccggcgtgttcaggtcgtcctcgatggagcggaggaagtcggcgggcggatcgagctcgggcgcctcgacgccggccgaacggtgcagtgctccgtaaagccgatccagcgccttgcggctctggtccagcagagcctggttccagtcgagcggctggcggtagtgggcgctgagcagcgcccagcggaccacctcgcccggcatcgcctgcaccaggtcatgcaacaacaggacgttgccgacggacttggacatcttctcggcgtccacggtcagaaagccgttgtgcatccagtagcgggcgtattcgtcgtgcggccgatcgccatgcgcatggccgtgggcgcagacgccttgcgcgatctcgttctcgtggtgcgggaacaccaggtcgatcccgccgccgtggatgtcgatgggaaggcccagcgtctgctcgatcatggccgagcactcgatgtgccagcccggccgcccctcgccccagggcgaaggccaggagggctcgccttcctttgacggcttccacaggacgaagtcgtgcgggttcttcttgtagggcgcgacctcgacgcgggcgccggcgatcatgtcgtccaggttgcgccccgacagcgcgccataggccggataggacgagacgtcgaacagcacgtgcccttcggccgcataggcgcagccggcgtcgatgatggccccgatctggtcgacaatggcggggatgtagtcagtgacgtggggctgaaggtccggcggcgagacgttcagccgcttcatgtcctccagataggcggcctcatagcgggccgtgacctcgccgatcggcacgccctcgcgcgcggccttggcgttgatcttgtcgtccacgtcggtgacgttgcgggcgtagatcacctgcggataggtgcggcgcagcagccgcaccagcacgtcgaacaccactggcggccgcgcattgccgatgtgggcgtagtcatagaccgtcggcccgcagacgtagagggtcacccgggccggatcgcgcggttcgaacgggcgcttttcacggcgcagggtgtcgtggatgtgcagcggcatcggggaacggctttgcgttttcttgcgggagggaggctccgtcccatatagcggcctgatagtcagtgagcgctgactgaccaagccagaatcgattgcatgacccctgttcccgccaagcccgtcctggtcagcaccgacggcgccgtcgttcgtcccacgcgcgagcaggcgctggaggcggtgcggaccctgatcgcctgggccggcgacgatccggctcgtcccggcctgatcgacacgcccaagcgcgtggtggacgcctatggcgaatggttcgacggctacgccgccgatgcgggcaaggagctgagccggacgttcgaggacgtgcagggctatgacgacatggtgatcctgcgcgacatcgaggtggagagccactgcgagcaccatctcgcccccttcctcggcaaggcctacgtcgcctatctgcccggcgaaaaggtggtgggcatctccaagctggcgcgggtggtggagatcttcgcccggcgcctgcagaaccaggagaccctgaccaacgacatcgtggacgccatcgaatcgcacctgcagccgcgcggcgtggcggtgctggtcgatgcggcgcaccagtgcatgaccacgcgcggggtgcaccatcgccacgtctcgaccctgacgacccgcttcaccggcgccttcaaggccgatcctcagctggcggaccgcttcctgaagctggcgcgcggctgaatcccgcgcgcggcgacgagaccgctttacaagccggttaaggaccgccaagacacggttcgaggattgtttcagcgcccgccgaccaggctggccacagatttcggagacgtcacgacatgggcgccaaactttccgggcccgctggccagggcggtaagaccatcgagcagaacgcggacatcaacgtcacgccgttcgtcgacatcatgctggtgctgctgatcatcttcatggtggccgcgccgctggccaccgtgtccatccgcctggacctgccgccggccgtgccgccgactaccccgaccgagatgaaggaaccggtgtacatcaccatccaggaatcgggtcagatctacatcgcccaggacgaaatccagctggccaacctgccgcaggccgtgtgcgcggccctgggcggcggcgcctgccgcgaggagcgcgtgttcgtgcgcgcccagccggaagtgcgctacgagcagttcatggaagtgatgaactccatgcaggccaacggcttcttcaaggtcggcctgctgaacgaagacatcgaatagggcttttcgcctgttcgccgggatcagggccgcgctccttcgggacgcggcctttttctttgcccgcgaccttgccgcaggaggcgcatccggttcttgatggccttctcaccgccttgaggaactcgccatgcgccgccgcacattcctgtccgccctgccctccggcgccctggcggccggcgcgctgtccaccggcgccgcgaacgctcagaccggccagccacccgcgccgggccgcccgaccgaggccgcgcctgcgcccgcccgcccgacccttacgccgaggtcggcatcggcgaccggatcaccggacccaagttcgtcggccgctcaaccgtgtggggcgcgaacggagcggcggcgacggcgcatccaaccgcgaccctgatcgggatcgacaccctgcggcgcggcggctcggccatcgacgcggccatcgccatcaatgcggcgctgggctttctggagccggtggccaacggcatcggcggcgacgccttctgcatgttgtgggaccccaagcagcgtaaggtcgtcggcttcaacggttcgggaaacagcccgcgcggtttaagtctggaggtcgcgcggtccaaggccatcgacgggtatctgccccgctacggcgccgtcaccgtcaatgttcctggcacggtggatgcctggtggagcgcgcaccagcgctacggcaagctgccgtggaaggaggtgctgctgcccgtcgccgaattgtgcgagcagggtgcgcccgtgccgcaagtcatcgcctactacctcgagcgcaacatggccgccttcgaccgaggccgcatcccgatcgaggagaacgacaaccgaaagcgcgtctatgctcccggcggcgagacgcccaaggtcggccagatgttcgccaatccgttcctcggcaagacgctgaggctgatcgccgagggcggacgcgacgccttctacgaggggccgctggccgagcagatggagggctacttccgccgcatcggcgggtggctgacccccgccgaccccgccgcgcaccgcactgagtgggtggagccgatccgcaccgactatcgcggcgtcgaggtctatgggctagggccaaatacgcaggggctgtccaccaaccagatcctgaacatctgcgagcagttcgacctgaagggcatgggcttccagtccgccgcctccttgcacgtccaggccgaggccaagcggctcgcgttcgaggatcgcgcccgctatttcgccgatccgcgcttctccgacatcccggtcgagtggctgaactccaaggcctatgcggccgaacgggcgcggctgatccgcccggaccggatcatggaccgcgtcatgcctggcgacgccccgcaccacggcgacaccacctatttcagcgtggccgacaaggacgggctgatggtcagctggatccagtccaactatcgcggcatgggctcgggcctggtccccgacgatgggcggggcaatccgctgggcttcatgttccaggaccggggcgagctgttcgccctgagcgacggccacccgaacgtctatgcgcccggcaagcggcctttccagaccatcatccccggcttcacggtcaaggacggcgagccgtggatggcgttcggcgtcatggggggcggcatgcagccgcagggccaggcgcagatcgtcatcaacatggtcgactacggcctcgacccgcaggaggcgggcgacgcgccgcgctggcagcactacggctcgtccgaaccgaccggccagccgcaggagggcgcgggcgtgctccacctcgaaagcggcgtgccggaagcgaccaagacgcagcttcgcgccatgggctggacgctgggtccgccggacggcggcttcggcggctaccagaacgtcatgcgccagcagaacccggacggtctctggacctacggcgcggccaccgagatgcgcaaggacggcatcgcgctggcctactgagttgcggactggcgaggagggtattacctttccggtgaagaggtaataccatgcgcatcacgtcgaaaggtcaggtcaccatccccgccgacatccgtgagcgggcgggactgctgccgcacaccgaggtggactttcactacgacggcaatgtcgtgaccgtagtgcgaagtggcgaacggaccggcggtcgcggcaggcggctgaccgagcacatggccggtttcggtgaccggctcacgatgagggccgacgaaatcatggcgctgacgcgcggcgaatgagcgttcttgtcgacagcaatgtcctcatcgacctgatcgaccgcacatcggagtggcgggtctggtcgatcgaacaagtcgaacggctcgtcgacgcaggcgaagtcctgctgatcaacccgatcatctatgcggaagtgtcgatcccgttcactgatccagcggacgtggacgccatgcttgcgctactggagcgggaagccctgccgtttgaggctgcgttcgctgccggtaaggcgttccagacctatcgccgccgaggcggcgcccgcaccgctcccctgcccgacttcttcatcggcgcgcacgcgctggtgcgcggccatgggctgctgacgcgcgacgcgagccgctacaggacctatttccccgaggtggagttgatcgcgccgtgacgcgggacgaggtgcacgccctgctgatgagctttccgggcgcggagagcgcagtgtcgtacggtcatccgtcgtacaaggtgcgggagaagttcttcacctggttctggccggagacgcccgactgtctggtggttcagctggacagccgggagcagcgcgacatgctggcggaggccgagccggagacgtttgtcgtcaccgatcaccaccgaccgcatccgatcctgctggcgcgcatcgaccgcgtcgatcccaactggctgcggtcggcgctgacgcggcgctggcgaaagatcgcgccggcggcgctgcgcaatgcgcatccagaccttacgccgaaggaacccggcgcctaactggacccttcccccgaaagagaaggagcctcctgatggcctatggcgaccagcccaccctcacagccggcgaggtggagattccgctgctcggcttcggcacctggcagctggagcccgaggacgcgcgccgcatggtcgcggaagccctgcgcatcggctatcgccacattgacacggccaggatctaccagaacgaggaggcggtcggccaaggcatccgcgactccggtgtcgatcgcgacgacatcttcctgaccaccaagatctgggtcgaggatttcgccgacggcgacctgcagcgcgcggcgcaagggtcggtggatcggctgggcttcacgcccgacctgttgctgctgcactggcccaagccgcagccttcgttcgaggagacgctgggggcgctgaacgacgcgcgggccaagggcctgacccgagacatcggcctgtccaacttcccgtccaaggagttccgccgcgcgcaggcgctgtcggaggcgcggctgctgaccaaccaggtcgagtaccacccctatctgaagctcacgccgctgctggagacggcgaaggacctggggtcgtcgatcaccgcctggtcgccgctggcgcagggcaagatcgccgatgacgcggtgatcagcgagatcgcccgggcgcacggcaagaccaacggccaggtcaccctgcgctggctgatccagcagaacgtcgtcgccattccgcgcaccaccaaggagagccgcgcgcgcgagaacttcgacatcttcgactttcggctgtcggacgaggagatggcgcgcatccacggcctggcgcgtccccacggccgcatcggcgactggattgaccccgccttccgatgggatgatgttgccgcataaggggccgtcgcccgacagagccccagccagggagtgcggccatgggctctgttctggggtttcccggcgtcgatccggcggatgcggcgatcggcgcgcgattgaagcgatggcgggatcagcgcggcgtgacatccgaagtgctggcgcgcgatctcggcgtcacgcccgaggcccttcgccgcatggaggcgggtcgcgagcatctcagcatgctgcaggtcgacgcagcgacccgcgccctgcatctgccggtctgggcgctgatgtcggatacgcgcgcctattgacgccgaggcgcgcccgatgagcgcgcgcctttatcgcgggctgttcgccgccgtcacatggctggcgctggccgttcaggtgctgcttgcggtcggcgacaagggcggctgggatgtcgtggtcagcatcgtccggctgttcagcttcttcaccatcctgaccaatctgctggtggcgctggccttcaccgggccattgctgagcgatcatcggcggctggcgcgctggagcgcaagcgaaggcgtgcgggcgtccgtcgccatgtacatcaccgtggtcggcgtcatctatcacctgctgctggcgccctactggagcccgacgggatggcttctggccgtgaacgtggtgctgcacaccgtcacgccgatcgcctttgtgctcgactggctgctgttcacgcccaagggtcggctgaggtggacggacgcggccaagtggctgatttttccgctggcttacggcgcctggacggtggcgcacggcctcgtctccggctggtggccctatgggttcgtcaatcccggccagatcggctggggcggactggtcgtcagcctcctggccttcgcggccttcttctatggcctgggcctgctgatcgtgggcgcggaccgcctgctgtcgcgccgcgcgagacgtgacagcgcgccctgcgccctttaggccagcgaccaagactggagcgaccgatggcctaccgatccctgcgcgagttcatggcgacgctggaggcgcaaggagagctggtgcgggtgtcggagcctgtctccaccgttctggagatgacggagatccagacgcggctgctgcgcaacggcgggccggccgtgctgttcgaaaagccggtcatgccggacggatcgatcagcccgatcccgtgcctcgccaacctgttcggcacggtgaagcgggtggccatgggcgtgacgctggagggcaagagccgcaccaccaccggcgaactgcgcgaggtcggcgaactgctggccttcctgcgcaatcccacgccgccgcgcggtttcgccgacgccatggagatgctgccgctggccaagacagtgatgtcgatgcggcccaagaccgtgggtcgcgcgccggtgcaggaggtggtgctgaccggcgaccagatcgacctgaccgccctgcccgtccagtcgtgctggcccggcgagcccgcgccgctgatcacctggggcctggtggtgaccaaggggccgagcgaggaccgcgaggacgacttcaacctgggcatctaccgcatgcaggtgctgggcaaggaccgggcgatcatgcgctggctggcgcatcgcggcggagcccagcactacgcccggcacaagaaggcgcgcccaaaagagcccctgccgtgcgcggtggtgttgggggccgatccgggaacgatcctggcggcggtgaccccggtaccggacactctgtcggaatatcagttcgccggactgatgcgcggggccaaggcggagctggtcccctgcaagaccgtcccgctgatggtcccggcgcaggccgagatcgtgctggagggtcacgtcctcttggacgagcatgccgacgaaggcccctacggcgaccacacgggctactacaactcggtggagagctttccggtgttcaaggtcagcgcggtcaccatgcggcgtgacccgatctatctgaccaccttcaccggacgcccgccggacgagcccagcgtgctgggcgaggcgctgaacgaggtgttcattcccctgctgcgccagcagttccccgagatcgtcgacttctggctgccgccggaagggtgcagctatcgcatcgccgtggtgagcatgcggaaagcctatcccggccacgccaagcgggtgatgctgggcgtgtggagctatctgcgccagttcatgtacaccaagtgggtgatcgtggtggatcacgacatcgacgcccgcgactggaaggacgtgatgtgggccatctcgaccaagatggacccggcgcgcgacatcaccgtgattgaatccacccccatcgactatctggacttcgccagccccgagagcggcctcggctccaagatcggcttggacgccaccgacaaatggccgcccgagacgaagcgcgaatggggcgaggagatccgcatggacgaggccgtggtggagcgggtcagcgagatgtgggaccggctcggattgccgggggatgggacgccgatctggaagtagcgtcgctaacctgttataacttcgttgcaacggagcacagccatgagcacggccatccgcaagatcggcaactccgccggcgtaattctgccgaagcccgccctggcggcgctcggcgtccaagaaggcggggcggtggagtttgtctatgaacctggcaagatcagcatcgtgccggcgcgcaaacttccgcgccaaggctgggaagaagacgccaagcgcattgcagcggcgggcttgaccgaagaagagcgtgagtggctggacgcggacctcaccagcgggacggacgcggaagccctgggcgacgactggacggaagacgaactcgccgaattggaagcggcgctcgccgcgaatgaaagcgaaccatcttgatcaagcgcggcgatgtctggctggttcggctggatccgaccgtcggcagcgaacttcgcaagacccggccctgcatcgttgtttccccagatggcttgagccatctgtcggttcacctcatcgtgccgctgactagcggcagcataccgtcgcggtttcgtcccgatgtacatttcggaagccgatcgggcctcctgttgcctgaccagatgcgatccgtggatcgttcgcgaatgatcagacggcttggagcgttgggggcgtccgagatgaaggccctgctcgctaccttgcgggaaatgttcgaagactgacctcatgccccgtctgacggttctttcagtcctggccgcgttcgcggctctcgcagcggatgccgccatgtcccagtccgtcccgaacgccgcgccctgggatcagcctttcctgccgccggcgccggagtgggacggcgcgtccagggcgctgctgcgaaatgcgtccgatccgtgggtcacggcgttcgaggcggacgcggggcacgacttctcgccgaactacgccgacacgcgcgcctggttcgagcggctggatgcggcctccgacctgatccgcgtcgaacagttcggcgtctcgccagaggggcggccgatccatgctgtgatcgcctccagggacggcgcgacgctggatccgtccaagccggtgctgatggtccaggccggcatccatccgggcgagatcgacggcaaggacgccggcatgatgctgctgcgcgacatcgccttctacggcaaggacgggctgctggaccgggtcaatctgatcctgatcccgatcctgagcgtggacgggcatgagcgcgcgtccccctactcccgccccaaccagcgcgggccgcgcatccagggctggcgcaacacggcgaccaaccagaacctgaaccgcgactacctcaagctggatcagccggagatgcgcgcggttcgcggcctgatcctgaagtatcagccggacctttacgtcgacgtgcacgtcaccgacggcatggattaccagtacgacgtcacctacggcttcaatggcgagaacgggaccttcagccgctcgcccgccagctcgcgctggctggatcaggtgttcaagccggcgatgaacgcggcgctggagcggcagggccatatcccgggcgagctggtgttcggcgtcgacgacaacgatccgaagaagggcctgtcggacggcggcctgggcgagcgcttctccaacggctggggcgcggcggcgcacgtgccgaccatcctgatcgagaaccacagcctgaagccgcacgagcagcgggtgctggggacctatgtgttcatggaggaggcgatgcgcctgctggcctcccacggcggcgatctgcgcgcggcgacacagagcgatctggcgctgcgtcccgccgaaatccccgccaacttcgaggccgaggaccagccgtcgtccacgcgcgacttcaagggcatcctgtacgagacctacgacagcccggcgtcggggcggcgcgagatccgctggctgggccgggccgatccggagacgtggcggatgccgttctacggctcgaagccgacgctgacgctgaagcggccgacggcctactgggtgccgtcctatcgcaccgacatcatcgagcggctgcgggcgcacgggatcgagatggagacggtgaacgcgccgcgcgtgcagggcgtgtccatgctgcggctggtcgagcccaggctggagacgcgcccgaacgagggtcacgtgccgatctcggtcgaggcggtggaggtcgagcggcgcgactggacctggccgaccggctcggggcgcgtgccgaccgaccagccgctgggcgacatcgccgtactgctgctggagccgcagtcgaacgagagcttcttcgcctggggcttgttccccgaggtgctgagccgcgtcgaatacatcgagggctacgccatcgcacccctggccgagaggatgatggcggccgatccggcgctgaaggccgagttcgagaagacgctggccgacgatcccgccttcgccgccaacggcgatgcgcggctgcagtggttctaccagcgcacgccgttttatgacgaccgccacctgctctatccggtggcgcgcgaggattgaggccgttgcgggccggggacgcgtccgccatatcggggcatgaccgaaacgcttgacgccgtccccgccgccgcctccgccgacctgctggacgatgtggtgcgggcggcgctgagagccggcgccgatgcggccgaagccgtatccgccgaccgccgcgccctgtcgatcggcgtgcgcaacggcaagctggaggacgtggagcgcgaggaatcccgcgatctcggtctgcgcgtcttcatcggcaagcgtcaggcgacggtgtcggcttcggatttgtcggcggcgacgcgggcgcggctggtggagcgggcggtggccatggcgcgcctggcgcccgaagatcccttcgcgggccttgcacccgaagacatgttggcgcgcgggcccttcctagacctcgacctgtttgatccgacggagcggagcgcggccgagctggaggccgcatcggtcgctgcggaggcggcggctctgggcgtgccgggcgtgtccaagtccgagggcggacacgcctcctggtcgtccagcgactggcggctggtgacctcgcacggcttcgatggacgataccgcggcacggccttttcgctgggcgtcggcgtcatcgccgaaaaggacggagccatggagcgcggcggggagagccgcaccacccgccacctggccgacctgccggacgccgagagcatcggcctggagggcgggcgtcgcgcggtcgcgcgcaccggtccgcgcaagatcgcctccaccaccgcgccggtgatcttcgagaaccgcgtggcgacgcaggtgctgtcgccgctggtaggtgcgatcgcaggcccgtcgatcgcgcgcggcacctccttcctcaaggacaggctgggcgagcgggtgctgcctgagggcgtggacctgatcgacgaccccttccgtccgcgcggcctggggtccacccccttcgacgacgagggcgtgcgggtcgagcggcgcgccctggtggaggacggcgtcctgacaacctggctgctgaacacggcgtcggcggcgcagctgggcctcgcttcgaccggccacgcctcgcggggcctcgcagggccttcgggcgtctcgacccacaacctgcacctggagccgggcaagcgcgatctggacgccctgatgcgcgatgcgggctcggggcttttgatcacctccatgttcggcccgtcgctgaacggcaacaccggcgactggtcggccggggtgtcgggtttctggttcgagaacggcgcggtcgcctatccggtgtcggaggtgacggtggccgggcggctgaccgacctttatgcgcggatggagcggggctcggacctgcggttccggggcggcttcaacagccccagcctcctgttcgacgccgtcgccatcgcgggtaaatgacggacctctgcgccgaccttgatctgatccgccaggcggcgctggacgcgggcgccctggccgtggccgagcgcgcgcggggcctgagcacccgcaataaggccgggggatcgcccgtcaccagcggcgacctgaaagtcgacgccatgctgcgcgagcggctgctgggcgcgcggcccgactatggctggctgtcggaagagacggcggactcgcccgagcggctggagaagcggcgcattttcgtggtcgatcccgtggacggcaccgtcgcctatatgaagggcaagccttggtggtgcacgcccatcgcggtgatcgaggacggccggccggtcgcggcggtgatccatgcgcccgcgctgggcgagacgttcgaggcgacgcgcggcggcggcgcgcgcctgaacggcgagacgatccgcgcctcgcaaacaggcatgctcgaggacgcgcgggttctcgccgacgcccgcgtcttccgcgacgcacgctgggccgagccgtggccggagatgcgctacgaaagccgcaacgccctggcctatcgcatggcgctggtggcggcgggcgccttcgacgcggctctggcgctggcgccgaagtgggattgggacgtcgcggccggcgccctgatcgccgaggaggcgggcgcggtggtcaccgatcatcactgcgcggcctggcgcttcaaccggcctgatccgcgccagaacagcctggtctgcgcggcccctggtctgcacgcggagatcatccgccgttgcgggaccctgccgggttcgccctgacacagcggcgttaaagcggcgccgcggcgttgatccccgcgccgtctcggcctatgccgcccgccaaacgcccctcccgcccaaggacgtcccatggcccccaccaacaccgttcccgccaaccagctctacatcgtcatcggcggcgagctgcgcacgctcaacgagaacgtcttccgcgatctgtcgcacgtcgaatacgtcggcgccttcgccgactatgaagaggccaagaaggcctggaaggcgcgcgcgcaggcgaccgtcgacaacgcccacatgcgcttcttcatcctgcccgcgcacaagctgatcgatccgcacgcggaaggctgatcggggaaccgccggccccggcgcgcgctgggttctcactgacgcgcgccggagccccctctcccatgaccctgttcggacagccgatcgacggcggccagatcatgagcctggtcagcctgttgctggtgctggtgctgctggtggcctcgttgcggggccactccgcctatgcgcgctggttcaggcagtgggacggccggtcgaaagaggcccccgaacccaagcccgcgccgccccaggcgccgatcgatccggcctcccgcaaggggccgtggggctgacgcgcgccgcgcgcgctgttgtcgtcgcgggttgacttggacggcggaccgtccgaccgaaggccgatgagtgcggctccctcctcaacgccagtcaagacgccggccgacttgcccctgtcggcgctgatcgcgcgcatctggcgcgaatatctgtcggacaacaaggccgctctcttgaccggcatggcgtgcgcggcgctggcgggcggcctgtcggcggcgctgctggggctgctggagccggcgatcaacggcctgttcgtgccgggcggcgggtcggtgcggctgttcaacctcgtcagcctgaccgagaaccaggccctgctgtggataccgatcgccatcgtcggcacggccatgctgaggacgcttgcgacctcgacccaggcgcggctggtgaaccggatcggccacggcatcgtcggcgacatccaggtgcggctgttcgcggcgatgatccgggcggacctggcgcggctgcgcagccagcactcgggatcgttcgtgtccacggtgctgtacgacgccaatctggtgcgcgaggccttcacctccggcgtggtcagctacacccagcacggactgacgctgatcgcggtgctgctctacatggcctggatcgactggcggctgacggcggtggtgctcctggccattccggtggtgtcgctggtgctgcggacgttcggcaagcgcacgcgcaaggccgcagccggcgccatgggcgagagcgaggccttgtccaccgccctgatggagaacctggacggcgttcgcctgatcaagatcgagaaccgcgaggcggcggaggaagcgcgcgtggccgaggtggtgcgtcggcgccagcgccacgtcatcaagggcgccaacgcccgcgccctggccggcccggccagcgacatggtggcctattgcgtggtggcggcggtgatcaccttcgccggctggcaggcgcgccagggcgtgatgaacgtaggcgagttcgccgccttcatcggcctgctgctggccgccggtcagtcgctgcggcaggtgaccaacttgtccaccatcatgagcgaggggctgaccgccgcacgccgcctgttcgcgtcgctggacatccagcccgagattcgcgaggcggcggacgccgaacccctgcccgccggaccggcgaccgtgagcttcgacaacgtctccttcgcctatgcgccatcgggcgcgccgacgctgagcgacgtctcgctccgcgtcgcgcccggcgagacggtggcgctggtcggcccctcgggcggcggcaagagcacggtgctgtcgctgttgccgcgcttctacgacgtgacgggcggcgccgtgacggtgaacgggcgcgacgtgcgccagctgaagaccgccgacctgcgcgaccgcgtcgccctggtgacgcaggagcctttcctgttcgacgacacgatagcggccaacatcggttatggccgcgacggcgcgagccccgacgaaatcgaggcggcggcgcgcgcggcggtggcgcacgacttcatcgccgccctgccgcaaggctatgagacgcgcgccggcgaggcgggcgtgcgcctgtcgggcggccagcgacagcgcatcgccatcgcccgcgcctttctgaaggacgcgcccatcctgctgctggacgaggcgaccagcgccctggacaccgaaagcgaggcgctggtgcaggcggcgctggagcggctgatgcaggggcgcgccaccctgatgatcgcccaccgcctgtcgaccgtgcgcaacgccgaccgcatctatgtgctggaggccggtcgcgtggtcgaggaaggaacccacgacgcgctcgtgggccgcggcggcctctattcgcgcctggcgcgccagcagtcgctggacagcgaacggccgaccgtggctgtggtggcctgagctcatgaggccgctgcgcatacccgccgtgcaggcgaccctgtccttcgtgctggccgcgtggatgcggttctgctttcgcaccatccgctggacctatgagaaccagggggtcgccgaagaggtgtgggccgggggcggcggcgtgctggcggtcttctggcactcccgcatcggcctgtcgcccgcctgctggccgctggaccgcgcgacgccggccaaggcgctgatctcgctgagccccgacgggcagttcatcgccaaggcggtgggacggcagggctttcccgccatccacggctccacaggccgcaaggacgcgcccgaacgcgccaagggcggcgcgcaggcgtttcgcgcggcgctgcgtcagctcaaggccggcggcctggccgtcacccccgatggtccgcgcggcccggccaaccagatgggcgagggcctgccgctgatggcgcgcctgtccaaggtcccggtgctgttcataggcatgagctgttcgcccgcgatccggctgaacagctgggatcgcgcggtgctgccgctgccgttcgggcggggcgccatcgtctgggaccgcgaccgctttccggagggcggcgagatggaggcggtgatcgccgactggacggagcgcctcaacggcgtcgaggcccgcgccgatgcgatcaccgggctgaagcgatgacgccgctcccgctgatcgcctatcgctggctgacgcggatgctggagccgctggcgccgcgcctgctggacgcccgtgtccggcgcggcaaggaggacgaggcgagggtggacgagcggctggggatcgccaccgtcgcacgaccgcccggcgatctcgtctggctgcatggcgcaagcgtcggagagaccctgtcgctgctgccgctggtggagcggctgtcgcgtgagcggccggacctgcgcctgctcgtcacctccggcacggtgacctcggccgccatcctgcacgagcggttgcccgcaggcgtgatccaccagttcccgccgatagacgcgccaggcgccgtggacgcctttctccagcactggcgaccagcgctgggcgtctttgtcgagagcgagctgtggcccaacctgctgctgcgggcgcaggcggccggcgtgcggctcgccctggtgtcggcccggatcaccgacaagacggcgaaaggctggacgcgtttcccgaagtccgccgcccatgtgctggacgccttcgacgccgtgctgccgcaggacgacgcctcggccgaacgcctgcgcagcctgggcgcgcacatcgacggcctggccaatctgaagctggcgggcgcgcccctgccgcacgacacgtccgccttcagccgccttagcgccgccatcggggaccgcccggtggtgctggccgccagcacgcacgaggacgaggaggtggccgtcgtcgaggccctgtccgccctgcccggctcgccttgcctgatcgtcctgccgcgccatcccgaacggggcgcgggcgtcggggaggccctgcggatgcgcggccacccggcggccctgcggtctcgcgccgagccgatcgagggctcgggcgtctatgtggcggacaccctgaacgagatgggtctgttcctgcggctggccgatgtggtggtgctgggcggatcgttcgggccggtgctgggtcgtccggcgctgggcgggcacaatccgctggagcccgcgcgcctgggcaagccggtgatcaccggacccgacggggccaactggagcgccgtgaacgcggccatgatcgaggcgggcgggctggtccaggtcgcgggcgtcggcgacctgcccgatgtcgtcgcgcccctgctcatgaacccgtcgacggccaaggcgatgggcgagcgtgcgcggcgggcggcggcggaagccgcctcgggcctggaccggctctgggcggtgctgcagccgctgctgccgcccgcgcctgcgcgaggccggctgtgaagctgaagacgccacaatggtggtatcgccgcgaccgcagccatgcgccggtgacgcgcctgctgctgaagccgctgggctggatttgggcggccgagacggcgcgccggatcaaggccgccgttccggtcgatcccggttgcgcggtgatctcggtcggtaatctgacggtcggagggtcgggcaagaccccggtcgcgggcgaggtgctgcgcctgctgcgtgaacacggcgtcgaggcccaggccctgtcgcgcgggcatggcgggcggctggagggtccggtgcgggtcgatcccgatcggcacacggccgaggacgtcggcgacgagccgctgatgctggcgcaaggcgcgcccgcctggatcgcgcgcgaccgggccgcgggcgcgcgggcggcggccgagagcggggccgatgtcgtggttctggacgacgggcaccagaaccccgccctgatgaagacggtcagcctggtcgtcgtcgatggggagacgcgtggcggcgagtggccgttcggagacggctccatctttccctccggtccgatgcgcgagccgctggcgcccgggctcgcccgcgccgacgcggtggtggtgatcgcgccgacggatgcggacgaagtcagcggcgaactgctggccgccttcggagatctgccggtgttcatcgcgcagctgcgggcgctccagccgcccccctccggtcctctgctgggcttcgcgggcgtcgccaagccctggaaggtcgagcgggcgctgaaggcggccggcgcggatctggtggactttgttccctttcccgaccacgcgccctatcaggataaagatttcgcctttctgcaggaccgagcggccgcgttcggcgcggggctgatcaccacggaaaaggattgggtgcggctgagcgccaatcagcggcggagcgtaaccgcgtggccggtcgtcacgcgtttcgaggacgagtcggcgttcagccgctttttgctgcagcggctgtcgatgcggagctgaaccaggaaagttccgcgctcacgaaagttttatctcgccatcatcagggtcttctcgaagggcagcgccacaatcgtgcgccgatgtccacggacgatgacctgagcagaagccccgcgccgctggcttttcagcatccgtgacatgtctttctcgcccagaagcttcagcgcagggtgacccgccgccggcgagattatgacggttttcaaggcgttggcgcgtcgctccccgccatggctcaggttgcccccgcagcaacagtttgaaacaacacggcccaagaacaaccgcaacgagggcgtcgcatgcggctatcgagacgagggctgatcctgggcggatcggccatgctggcgggctgcgccaccggacaggccaccccgctgatcacccaggctcaggcgccggtcgcgccgccgctgtcggtgatctcgcaggctcccgccccggtcgtcgtctcgatgaacgccgccccgccgctcgatccgcgcggtcaggttcacaaggagctgatggagcgcgcggtcgccgccctggacgtccaccacaagcgcatccccctgcgtgaccggatgtatctggtcgacttccagaagtactcgggcgacgagcgcctgtacgaggtcgacatggtgggcggccaggtgacggtgctgcggacctgtcacggccggggttcggacccggcgcactcgggctacgcccagcgcttctccaacacgccggacagcaacatgtcctcggtcggcgccttcgccaccgccggcgccagctggggatcgcaacaggggccgaacgtgctgctggacgggctggaatattccaacgaccgcgcccgcgaacgcgccatcatcatccacggcgccgactacgccgatcccggcttcctggcccgcgaaggcaagctcggccgctcctacggctgcttctccgtcgcccacgccgacctgcccgccctgcgcgaacgcatgggcgaaggccgcctgctgttcgcctgggcgtagggtctgcaaaaccgtagcggtttgacgctgttgtaggtcaagcatacgctgtgcgacgcccctcaggagagacgcgcatgctgtcggtcaccctcgccgcgctgatgatgttcgcccaagaaccggccgcagcctcgccacctcaggcggcggcttctgcggaggttcaggagcccactcgtctcgaagacatcgacgtggtgggaagaacgctcgacaccatgatccgggatttcgtgggcgaggtggcggctcccaatcgaggtcggggcatcgcccgctgggaggacgccgtctgcatcggcgcggccaatctccagcgtgacgccgcgcagtacatcgttgaccgggtgtcgaccgtcgccgaggatttaggtttgacgccgggcgctccgggctgcgcccccaatgtcatgatcgtggccagcgacgatccgtcctcctttgcggccaagctggttgagacgcgcgcccgcgccttcagaatgggcggttcgggcatggatcgcgggggcgccgcgctgagggcttttcagacgtcgaacaagcctgtgcgctggtggcagcagtccatgcccgtcaactccgaaaccggcgagcgtgcagtccggatcccaggcgagtgcgccaacgcatgcagctctccctatgactatgctcccgtgatcgacaccttcgccgcatctcgcctcacctcgcagatcgccgacaacatcttccgcaccatcgtggtggtcgatgtgaaccaaacctccagggtgtcggtgcagcagctggcggactacatcgccatggtcactttcgctcagatcgatccggaggccgacaccagccggtacgcctcggtgctcaacgtctttgatgcgcccgaggcggcggacgggctgacggattgggacaccgcctatctcaaaggcctgtacgacgccgaacgcacgcgcaagaacgtccgggcgggcacgagcgagatcagggagtccatccgtcggacgcaccaggagctgcgcgccgaaaccgagccgcagccgtagccgctccttcagcgctccagcgcgcgccagccgatgtcggtgcggtggaagccgccgggccagtcgatccggcggatggcggcgtaggcgcgctcgcgggcctcggcgatgtcgtcgccctcggcgcagacgtttaagacccggccgccggcggcggcgagttgaccgtcagggcggcggcgcgtgccggcgtggaagacctggacatgcgggccgaagtcctgttctgcgccgcggatgatggagccctccagcggactgtcgggatagcccttggcggccaggacgacgcagatcaccgtctgcggcttgaactggggggccttgagccccgacacgtcgccgcgtgcgcaggccagcagatagggcacgaggtcgccggccatgcgcatcatcagcacctggcattccgggtcgccgaagcgggcgttgaactcgaccaccttggggcctccgtccgtcgccatcaggccggcgtagagcacgccgcgatagggcgcgccttcggccgccatggcgcgcagggtcggctggacgatccgctcgtccgcctcctgcaccagctccggcgtgaagacgggcgcgggcgagtatgagcccattccgccggtgttgggccccaggtcgccgtcgaaggcgcgcttgtggtcctgggcgcccccgaacagcaccgcgcgctggccgtcgcacagggcgaacagcgagccctcctccccgtccatgaactcctcgatcacgacgcgcgcgccggccgcgccgaaccgcccgcccagcatgcgctcgatctcggcttcggcgtcacggcgatccgggctgatggccacgcccttgccggcggccaggccgtcggccttgatgacgtagggaggatggaaccggtccagcgccgccttggcgtcggccacggtctcgtgcacgccatagccggcggtcggtatgccgtgacgctgcagcaggtccttggaaaaggccttggacgtctcgagctgcgccgccttggccgtgggaccgaagcaggggatccccgccgccgccagccggtccgcgagaccggccgccagcgcgacctccggccccacgaccacgaggtccgccttgatctcgcgcgcaagggcggccaagccttcggcgtcgtcggccttcagctcgggccgaacctcgcacaggcgggcgatgcccggattaccgggcgcggccaccaggcgcgtcagcagcggcgactgcgcgatcttccaggccagggcgtgttcgcgtccgccggatccgacaagcaggatgttcatgatcagccgcaatgaccgcccggcggagggcggtcaagcggccgaaagacttaccggcgccttagcccaatcctcagccttgcggcgtccaggcgggaagagcctgaagctgggcggcggtcagggtggtggtcagggccttctcgccgttctggtcgaccgagctgatctgggcgacgggtacgacgaccttgggatcgccggggccttccagctcgaccacgatgctggtcagggcgccgttcgcgtccagaaccagcgtctcgacgtcgccgagatcggtgttgccttgggccgacagcagatcggcgtcctcgagctcctggcgggtcatgccgaaggcgacggcggcctgggtctgggcaacctgggcctgggtctcggtgaccggctcgggcgcggcgccggcggccggcggctggacgacgtcgtcctcgcggtccgagcaggcggcggcgcccatcacagcgagcgcggcgacggcggtcagggtcagtcggttcatggggtttccttcaggccagaggtcagaacagggccgacaccgcatagacaagcagccccagcaacacgatcgcgccgatcaccagccacaggctgatcgccggcccgccgctgcggcgcgacagctcgcgctcggccggatcgggatcgtccggatcgccctggaggggtgtgttcggcgccatgcgaaacgaacggcgccgctagcgctgcgttcccgcgcggatcgacgcaggctatgatcgcccgatgaccgacgactatgtcttcgaaagcgccgtggaggctgcccccggcccccgcgacaacaatccgcccctgtcgatctccgagctgtcgtttgcgctgaagcgcacgctggaggaccgcttcggccatgtgcggctgcggggcgagatctccaaggtcaatcgtcacggctcgggccacgtctatctgacgctgaaggacgacaaggcctgcatcgacggcgtggtgtggaagggccaggcgcgggggctgggggtccagcccgaaacggggctggaggtcatcgtcaccggcaagatcacctcctatccggcgcggtcctcgtatcagatcgtgatcgagaccatggaggcggcgggcgccggcgcgctgctggcgcagctggagcggctgaaggtccggctgcgcggcgaagggctgttcgatgcggcgctgaaaaagcccctgcccgcctttcccgccgtgatcggcgtcatcaccagcccgacgggcgcggtgatccgcgacatcctgcaccggatcgaggagcgctggccctgccgcgtgatcgtatggccggtggtggtgcagggcgaaagcgcctgcggccaggtgtcggcggcgatccggggattcgagacgctgacgccggacgggccgatcccccgccctgacctgctgatcgtggcgcgcggagggggctcggtcgaggatctgtggtgcttcaacgacgaggggctggcgcgcacggtggccgccgcctccatcccgatcatctcggcggtggggcacgagacggacaccaccctgatcgacttcgtctccgaccggcgggcgcccacgccgacgggcgcggccgagatggcgacgccggtgctggcggacctgcgctacgccgtcggcgacatggaccggcgcctgacacaggcgggcgggcggctgatcgaggatcgccgcacgcggctgcgctcagtggcgcgcggcctgcccgctcgaccggaggacctgctggccttggcgcagcagcggctggacggcgcctccagccggctggagtcggcgctgttgcgcaatgtcgcaatgcatgaacggcgggcgacgctggtcggaggccggctgaacccggccctgctggagcgcgccatcgagcgccgggtcgaccggctggcgggcgcggccgggcggctggcctcgtcgctgagcgccaacaccgcggcgcacgagcggcggctgatccgcgtgtcaggccggctgtcgcccgagccactgcaccggcgtctggaccaacgcgccgcaaggctggactccgtggccgcccggctggcgcctgttctgccgcgcaggctggagcgtgcggaggatcggctgtcggcgctgtcgcgcgcgttggcctctctggaccccggtcgtcccaagcccggattcgccaaggtggaggatgcggagggccgctggctgacctcggccgccgccctgccgtccggtcaggccgtgcgcctggtgttcggcgacggggcccgtgacgccgtggtcgagggcgagccccgccctgctacaccacccgcccccgctcccgccacggtcaggcccgcaccccgcgcgaagccgacggcgcctgggcagggcagcctgttctgatcgctcctccccgcaggcgccgcttggggttggagcttggcttcgcttcctgctaagcgcgcccattcgcccgcctcaaggccaagccgagatcgcatgaccgtccgccgcaccgcccttttcgccttcgcgctcgccctcgctatcatcgtgctggatcagctgagcaaggcctggatcatcggcgggctgtcgctgcaggaggtcgggcgcgtgccggtgctgccgccgatcctgaacttctcgtgggtcgagaaccgaggcgtatcgttcggcctgttcggcgggggcgaggcgcgctgggtgctgagcgtcttttcggtcctcgtgtccatcgccttgggcgtctgggcgctgaaagctgacaggaagctgctgctcgccgccatcggcatggtcatgggcggcgccataggcaacgtcatcgaccgcatccgtttcggctatgtggtggacttcatcgacttctcgggcacgggcgtatttccctgggtgttcaatatcgccgacagcgccatcagcatcggcgtggtgctgctgatcctggacagcatcctgtcggagcgcgcggccaaggttggcgcggcccccgaaaagtcgtaatcacccgctcttcactacgcccatcttcgcgccgctcgcccggcgcctgcaaagcctgagctgatccatgcgtatccgaagcgtcgccgtcttgaccctcgccgcctccacgcttgcgttgggcgcttgcgggacactgcgtgatcgcgccggtctcggccgcgtcacgcccgacgagttcctgactgtttcgacggcgccgctcagcgtgccgccggaatacggcctgcgtccgccgtcgcccggccagccgcgccctcaggagctggctcccgaaagcgccgcccgtcaaatcctgctgggccagcgccaggccgtgacccgcacgcccggggaacaggcgctggtggcccaggccggcggcgagaacgccgatccgctggcgcgctatgtcgtcgacgacgagttcggcgacctggcgcataaggaagaaagcttcgccaaccgcatcctgttctggcgcaaggacgacgcggcgacgcaggcgcccaccgtcagccagaccgccgagggcgccgtcaccatcgacccggccagcgaggcggcgcgtctgcaggccctgaccggcggccggcagggcatcgccatcaccccgcgccgcagcggcggcttcaagctgccgggcctctaaagaaccgacgccatcgctcttcccgcctcacgatcggaaccctgcctgatgcgtcgcgtccctaccttcatgttcgcagcggccctgactgcggcgatcctgcccgccgcggcggacgcgcagtcgtccagccgacagcagcgcggccagagcgcgagcgcccagcaggaagaggggcaaagccgtgcacgcacgccccgcatcgcgccgctcagccgccgcgccaacgccgggccctgccccttcgtcaaggtgctgtacgacgccgcccgctatgtggagctcgagaacaaccgcgcggcagtcagcgccgtgggcttcaccggcgagatcgaggggctgaacgccgactgcacctatcgcggcgaggacccgatccggctggacatgaacatcctgttcaatctcggccgtggcgcgcaggcgacggacgggcagaagacctaccgctactgggtcgccgtgaccgagcggaacaaggccgtgcttgccaaggaatacttcgacctgccggtgaacttcgacggacagcgcaccgcctcggtgacggaggagcgcaccatcgtgatcccgcgcgccgacgccaccaccagcggcggcaacttcgaggttctggtcggtttcgagatcacgccggagatggccgagttcaaccgctcgggcagccgcttccgcgtcaacgccggtgcgcaggccgcgccgatcgaagcccccgccgcgaccccgcccgcgcaataagatgatcgacctcaagacgaccctcagcgaggcggtcgccgccgccttcgccgccgaaggcgtggatgcggcgcgcgccgccgttaccccgtccgatcgtccggacctcgccgacttccagtccaacggggcgctcgccgccgccaaggcgctgaaggccaatccgcgcgatctggccgcccgtgtcgccgaacggctgaaggacgacgatcgcctgctgtcggtggaggtcgcgggacccggcttcatcaacctgaaggtcgccgacgccgccctgtcgcagcgcgccgaggcgatcgccgccgacgccgagcatgcaggcgccgccctggtcgcctctccgcgccgggtggtgatcgactacggcggtccgaacgtggccaagccgatgcacgtcggccacctgcgcagcgccatcatcggtgaaagcctgaagcgcatcttccgcttccggggcgaccaggtcaccggcgacgcgcacttcggcgactggggcttccagatgggcctgctgatcgtcgcctgcggggacgaaggcctggccgacgccttcatggccgagggggacggcccctttcctgaggaaagccccgtcaccctggccgacctggaccggctctatccactggcggccggccgctccaaggaggacccggcgttccgcgaccgcgcgcgcaaggccaccgccgagctgcaatccggccgcgccggctaccgcgccctgtggcgccatttcgtgatcgtcagccgagaggcgctggagcgggagtacgccgccctttcggtggatttcgacctgtggaacggcgagagcgacgccgatccgctgatggaccagatgatcgcgcatctgcgcgagacgggcctgctggtcgaggacgacggcgcccaggtggtccacgtcgccaagcccggcgagacccgcaagaagaagctgcccgacggctcggtgatcgaggcgcccagcccgccgccgctcttggtcatcagctccgaaggctcggccatgtacggcacgaccgatctggcaaccattctggaccggaaacaggcgatcagccccgatctggtcctgtacgtcgtcgacgaacgccaggccgagcatttccagcaggtgttccgcgccgcctacctcgccggctatgcgccggagggctcgctggagcacctgggtttcggcaccatgaacgggacggacggcaagccgttcaagacccgcgccggcggcgtgctgaagctgcgcgacctgatcgacatggccaccgacaaggcgcgcgagcggctgcgcgaggccaagctgggcgatgacctgcctgcggacgcgttcgaggccattgcccacaaggtggcgatcgcggcgctgaagttcgccgacctgtcgaacgcgcgcaccaccagctacgtctttgatctggaccgcttcaccagcttcgagggcaagaccgggccgtacctgctgtaccaggcggtgcggatcaaatcgctgctgcgcaaggcagaggaccaggacgcggcgcccagcgcgatcatgatctccgacccagccgagcgtgacctggccctgacgctggacgccttttcgaccgccgtcgccgacgcctacgacaagcggatgccgcacctgctggccgagcacgcctatcgcatcgcccagtcgttttcgaagttttacgccgcctgccccgtgctggccgcgccggacgcggcgacgcgcgcctcgcgcctggctctgtcggccgcgaccctgcgccagctggagacggcgctggacctgctcggcgtcgagacgccggagcggatgtaggctaggctcgagtgtttcctcccggagcgcctttatgaccctcgacgcgttcatcgccggcctgcccaaggccgagctgcatctgcatatcgaggggtcgctggagcccgagctgatgttcgagctggcgcggcgcaacggggtgtcgatcccgttcagcagcgtggaggcggtgcgggccgcctatgacttctcgaacctgcaggacttcctggacatctactatgcgggtgcggcggtgctgctgacccggcgggacttcgaggatctagccttcgcctatttccagcgggcggcggcggacacggtgcggcacgcggaaatcttcttcgatccccagacccacaccgatcgaggcgtgccgatggcggaggtggtcgagggattgctggccggcatggcgcgggcggaacaggagctgggcgtcacctcaaggctgatcctgtgcttcctgcggcacctggacgaggcggcggcgttcgcgacgctggacgcggccacgccatggctggaccggatcgcgggcgtgggtctggactcgtcggaggtcggccatccgccgtccaagttccagcgcgtgttcgagcgtgcgggcacgctgggcctgaagcgcgtcgcccacgccggcgaggaaggcccgcccgcctatgtgcacgaggcgttggacctcctgcacatcgaccggatggatcacggcaaccgctccatggaggacgaggcgctggtgcggcgcctggcggccgagcggatgacgctgacggtgtgcccgctgtcgaacctgaagctgtgcgtggtcgatgacctgaaggaccaccccgtgcccgagatgctgaggcaggggctgcacatcaccctgaactcggacgatccggcctatttcggcggctatgtgaacgacaactatcgcgaactggcgcacgcgacggggctgacgcgcgagcagctgacgcggctggcccggaacagcttcgagggatcgttcctgagcgaggcggacaaggcgaagcggatcgcggaggttgaggcgtacgccgccgcgcaggcgtgacgaccctcgccgtcaccctcgggctcaccctccccttcgtgcgggtcctccaccgcagagcccgcaggacgtccgatcctcgggtcgagcccgaggatgacggaagggggcgaggacgtcaggccaagagttcggcagcgctgacttccaccacgccacgcgatccgaaactgtcccgcgcctccgccgccgtgttcggcgcgattgcgcggctggcgtcggtgatcaccaccgcctcgaagccctcgcgcatcgcgtcctcggcggtgaagcggacgcagtagtcgtaggccaggccgcacagaaagacgcgcgggacgccgagttcgcgcagcaggccggagaggcccgtcgatgtgcgatgatcgttctcgaagaagccggaatagctgtcgacccgcggactgcgccccttgcgcacgatggccagcgccttctcgaccgccggcgcgacatcgggatggaagtccgcgccgggcgagccctgcaggcagtggtccggccacagcatctggcggccgtaggcgacctcgatctcggtgaagggctgcgcgcccggatggttgaaggcgaaggagatctggtcgggcgtgtgccagtcctgagtcacgaccacgcggtcgaaacgctcggccagccgcacgatcagcggcatgatccccgcgccgccctcgaccgccagcgcgccgccttcgcagaagtcgttctgcggatcgatgatcagaagcgcgtccgacgggccgatgatcatgtcaggcgctcgcgaaggcgtcgatctcgctggccgagcccagggccacggcgatgcgctggtgcagttctgaaggctggacgtccagaatgggttggcggccgtcggtcgtggccttgccgcccgcctgttcgaccagcagggccatcggattgccctcgtacatcaggcgcagcttgcccgcgcggttcggctcgcgggcgtcccacggatagagaaagacgccgccgcgcatcaggatgcggtgcacgtccgccaccatggccgccacccagcgcatgttgaaatccttgccccgccgcccgtccctgccctggaggcaaccgtcgatgtagcggcggaccggctcggcccagtgacgctgattcgacatgttgatggcgaactccttggtgtccgccgggatggcgaggtcttcgccggtgcgcagccactggccgtccgaatccagggtgaaggcggcgacgccccgccccgtcgtcagcaccagcatcgattgcgcgccgtaaagggcgtagccggccgcgacctggctgcggcccggctgcagaaaggcggcttcgtcgatctcgcccgagggcgccggcaggaccgagaagatggtgcccacgggcgcgttgatgtcgatgttggaggagccgtccagcgggtcgaacagcaccagatagccgccttcgccggtgcggccggtcggctccaccgtgtccagttcctccgaggcgaggccgaacaccgaggcgcaggcggccaaggcctcgcgcagcatgtcgttggtgatgatgtcgagcttcttctgctcctcgtcctggacgttgacctggccggaggcgcccagcgcgccgactagggccccgcccgccaccgtccggctgatcgccgcgcaggtttcgcccagcacagccagcacggccggcaggccctcgggcgtctcgagcgcgccgacgtggtcgttcaggcggacgtgggcgatcatcggcggcgctccggggacggtgttcaccgttcttggcgggcgcggccaacgggagcaagtccgccgttgtcagatcggtagcacagctgtgccaaaggcgcgcttcagctcatgcgcggcaaaggtctcggcggcggcggcgtccggcaccaccaggcccatgccgaagaactcgtgcgtcgagccgtggaaggtcttgtgccgcacctcgaccccgttctgctccagccgctcggccagcagttcgccttcggagcgcagcggatcgatctcggcgcagatcacggtagcgctcggcaggccgatcaggtcggcctcgaccaggttgatgcggggatcggcggtccgggacggatcgtcgaaggcgtgccttacgaaccattccatcatcggcttgttcagcggtctggccgtcgcgttctcgatgtaggacggcgtctccatgtcgtcgccagcgatcggatagaccagcaccatgtggcagggcgcctgcagcccctcgtcgcgcgcggcgatggcggtggcgcaggccaggttcccgccggcgctttcgcccatgatggcgatcttgttcggatcgcccccgagcgaggcggcgttgtcgatgatccagcgccacgcggccagggcgtcttcgtgggcggcggggaacctgtgttcgggcgcctggcgatagtggaccgaaacgaccacgcagtcggcgaagcgggcgacgctcctcgggctggcgtcatagacgtcgagatcggcgatcacgaagccgccgccgtggaaatacagcaccaccggcttgacgtcggggtgggcgctctttgggcgatagacacgggcctgcagcggtccggccgcgcctggaatggtgatgtcccgcgtcatcacgcccagtgtcgggtcctcgctttcacgcttggagccgaggagctttttgacggcatcggccggggtcggctggaggcgtgcctcctgcggggtcaaggtctcgatcggcttggggtccagccgggcgtactggtccagcacgcgttgcatggcggcgtccggcctggccgggcggctgcggggcttgccggactcgccgaagatcctggtgatgatggacatggtgtcctctggcgcgggggagagggccgttgcaaaaccaatccacgccgctccggcttgttccgctccgcttgacttcgcgcgggagtcgggcgctaaggtcgcgcgctctcgcgggagagatcggggcggttcgccgccccgacgccgaaggcgcaaccgccccggaaacgctcaggcaaacggaccgcgaagcacacggacgctggaaagtcgcccaggaatcttggttctgggggcgcgccgacggagcaaggccgcagtggcggtcggaatctctcaggcttcaggacagcgggggcgcgagaaccggcgggcgaccgccccgagacgcgaccgcgaaaggctccccgccatggctgaacaggccgccgacgccctgaagaccacgccgctgcatgcagcccacaaggcgctgggcgcccgcatggcggccttcagcggctatgacatgcccatccagtacgaaggcgttctggccgagcaccgctggacgcgtgagcacgccggcctgttcgacgtctcgcacatgggccagtgccgcatcacgggcgaggacgccgtgacccagttcgaacgcttcgtgcccggcgactaccaggcgctgaaggcgggcaagcagaagtattcgctgctgctgaaccaggacggcggcatcatggatgacctgatggccggccgcccggaccacgacggcctgttcgtcgtggtcaacgccggcaacaaggaagccgatttcgaatatctgaagaacaatctggaaggctcggccttcctgatgcggctggacaaccgggcgctgctggcgatccaggggccggaggccgccgaggtcatggccgcgcacgagccggtgctggccgagatgggcttcatggagtgcgcgagactgatgctgttcggctgcgactgcttcgtgtcgcgctcgggctacaccggggaggacggctacgagatctcggttccggccgaagaggccgagcgcatctggaacaccctgctggaggacgcccgcgtcaagccgatcggccttggcgcccgcgattcgctgcggctcgaggccgggctgccgctgcacggccacgacatcgacgccttcaccagcccggtcgaggcggcgctgggcttcgccctgtccaagtcgcggcgcgaggctggaaacttcaacggcgccgagcgggtcgccaaggagatggccgaggggcccagccgcgtgcgcgtgggcttggccgtcaaggaaggcgcgcccgcccgcgaaggcgccgaggtcgccgatgcggacggccaggtgatcggcaaggtcacctcgggcggtccctcccccaccctgggccgcaacatcgccatggcctatgtgcccgcccgcctggcggcgctgggcacggagctgaaggtcatcgtgcgcggcaagcccgccgccgccgaagtcgtcgccatgccgttcgtggcgcaacgctattatcggaagccgaaggcgtaacatccaccccgtcaccctcgggcttgacccgagggccgggcggtcaaccgcttgtgcaaagacatggacgcacgagccgaacaacatcccatcctcgggtcgagcccgaggatgatggtcgaggagaaaagcacatgaagttcaccaaggaacacgagtgggtccgcctcgacggcgaagtcgccaccgtcggcatctccaagcacgccgccgacgccctgggcgacgtggtgttcgtggaggtccccgagaccggcaagaccctgtccgccaaggacagcttcgccgtggtcgagagcgtcaaggcggcctccgacgtctacgcccccgtctccggagaggtggtcgaggccaacgacgccctttcgaccgcccccgagaccgtcaacgccgacccggaaggcgacggctggttcgcccgcatcaaggtgtcggacccctcgcagctggacgccctgatggatcaggccgcctatgacgattacctgaagacgctctgatcgcttttccgctgctcgtgcgaacaaccgacgcacgatccgccccgcatccgatcctcgggtcgagcccgaggatgacggagtgagacccccatgcgctacctccccctgacgcccgacgaccgtacggcgatgctgtccgccatcggcgcctcgtcgatcgacgacctgtttgtggacgtgcccgaaagcgctcgcctggacgcccccgtggacctaccgcgcgtgcagggcgagctcgaggtcgagcgggcgttgtcggccatggccggcaagaatgcgacggcggggaccacgcccttcttctgcggcgccggcgcctacaagcatcatgtgccggccacggtggaccacatcatccagcgctcggagttcctgaccagctacactccctatcagccggaaatcgcacagggcacgctgcagtacctgtacgagttccagacccaggtcgcgaacctgaccggcatgccggtggccaacgcctcgctctatgacggctccaccgccatggccgagggcgtgctgatggcgacgcgggtgacgcgccggaacaaggcggtgatctcgggtggggtgcatccgcactacgtcaaggcgacggagacggtggtgcatgcggtgggcgtggagacgcaggcgctctctcccgctgtcgacgccgaggccgccgtgatcgacgccatcgggcccgacaccgcctgcgtggtggtgcagacgcccaacgtcttcggaaccgcgaccgacgtcacaaagatcgccgaggccgcccacgccgccggcgccctgctgatcgtcgtggtcaccgaagcggtgtccatgggcctgctgaagtcgcccggcgagatgggggccgacatcgtcgcggccgagggccagtcgatcggcaatgcgctgaacttcggcggcccctacgtcggcctgttcgccacccgcgagaagctgatccgccagatgcccggccgcctgaccggagaaacggtggacgcggacggtgagcgcgggttcgtgctgactctgtccacgcgcgagcagcacatccgccgcgacaaggcgacgtcgaacatctgcaccaactcagggctctgcaccctggccttcaccatccacatgagcctgttgggcgagacggggctgcgcaagctggcgctgctgaaccacgagaaggccatggcgacgcgcgatgcgcttgcggccgtcccgggcgtcgaggtgctgaccccgcgcttcttcaacgagttcgcggtgcgcctgcccaagaacgcggccgaggtcgtggatcagttggccgagcaccgcatcttggcgggcgtgccctacagccgcctgaacccggagggcgggccaaaagaagaaagatgggacgacgtgctgctggtcgccgcgaccgagacgacgctggacgccgacatcaagatcctggcgggcgcgctttcgaaggttttggcgggatgacgctccaatctctaaccgtcaccctcgggcctgacccgagggccgggcggtccgcgaaacagatgtcagccactgagcgcacgacgcttccgatcctcgggtcaagcccgaggatgacggggaactgaaccatgagcaccatgaacaccgtcggccgcccgaccacgccgaacgccgtcgatcacgactacaagcacccgaccctgaccggcgggcgcggcctgctgcaggacgagaagctgatcttcgagggcgaaggctgggggaagaccggcgtcgacctgccggagcccaagaccgatgcggcggacctgggggatctgatccgccgcgatccgatcggcctcccgggcctgtcggagcccgaggccatgcgccactatgtgcgcctcagccagaagaaccacgccatcgacctggccatctatccgctgggctcgtgcaccatgaagcacaacccgcgcctgaacgagaagatggcgcgcctgccgggcttctccgatatccaccctctgcagccgcaatcgacggtgcagggcgcgctggagctgatggaccagctggcccactggctgaagaccctgaccggcatgccggcggtggccctgtcgcccaaggcgggcgcgcacggcgagctttgcggcctgatggcgatccgcgccgcgcatgaagccaagggagagcacgcccaacgccgcaaggtgctggttcccacctcggcccacggcaccaatccggcgacggcggcctttgtcggctattcggtggtggaagtggcccagaccgaggacggccgcgtggacgtggccgatctggcgtccaagctggggcccgacgtggccgccatcatggtgaccaaccccaacacctgcggcctgttcgagcgcgacatcctggagatcagccgcctgacgcatgaggcgggcgcctatttctactgcgacggagccaacttcaacgccatcgtcggccgggtgcggccgggcgatctgggcgtcgacgccatgcacatcaacctgcacaagaccttttcgactccgcacggcggcggaggccccggcgccggtccggtggtgctgtccgaagcgctggcgcccttcgcccccgcgccgtgggtcgtgtcggacgcgaacggctatcgcctgatcgagcgcgatgaaggcgaggcggagcaggcgttcggccggctgtgcgcctttcagggccagatgggcatgtatgtgcgcgccctgtcctacatgatgagccacggctcggacggcctgcgtcaggtggccgaggacgcggtgctgaacgccaactatatcaaggcccggctgtcagacctgatgagcgtggccttccccgaaggcccatgcatgcacgaggccctgttcgacgacgaatggctgaagggcacggacgtcaccacgctggatttcgccaaggcgatgatcgacgagggtttccaccccatgaccatgtacttcccgctggtcgtgcatggggccatgctgatcgagccgacggagacggagtccaaggccgagttggaccggttcatcgaagccatgcggctgctggcccaggcggcgaagtcgggagatgtggaacgcttcaagggcgcgcccttccacgcccctctgcggcgcctcgacgagacccgcgcggcccgctcgccgcgcctgcgctggaccgccccggaaggctccaaccaggcggcctgatgccggctgtcgcggcgcggccacggcgccggatcaaatgccgatcatgaccaaagcttcacgcggcggacacggatcggccatcacgcgggtgtgaagaggcggctgtggcgatcgcgtcacggccgccttttcgttgcaacggcaaggatcgggaagccggcgggatcgttgtccctgtgtcccctcactgttcctttctggcctgccgtgacctctgtgagtctgtcctccttcgcctcgtccgctccgcgcccgctactgcgcgtgctgaagcgctggacgatgatgacggcgggcctgcttgtggttctgctgggcgtgctgatcgcgccgctgccgggaccgggcggcgttccggtgatcgcgctggggttggtgctgattctgcgcagctccttctgggccaagcgccagttcatccgcgcccagcatgctcggccgcgctgggtgtatccctttcgccgactgctgcgaaagaagccggagttcgcgccggtgttctggcagtccgcgctgcggacggaacggatgatgctgcggcgcacacaccgtcgactgacccgcacgcgcaagggtttgcggcggtatacgcgaaaaatcttccgctgatctcgcggttgcggtttcgcagctgctaaccacagagttgtgaccgccgttcaccggcggcgggcgtatcctccctctcgcgttatcagagaaccaccaaaggcgttgggaggcgcttcggtcatgatgtcacgcgtacaaaaaggtctggccgcaggcgtggccggaacggtggcggtgtccttactggagctgcccaacatcttcctgaactggtttgatcccaccccggccgtcatcgcccatgtcatcggcatggatgggaacatggccgtgggctgggccctgcacctggccatcggcgttctgctgctggggccggccttcggctacctctgtccgcgcctgccgacggacacgccggagaccaagggcatcgcctttgcggtcggggcattcgtgctgatgatgctggtcgtcttcatgttcggcgatcagggcacattcaccagcggctcgggcttcggcgccgtggcctggatgctgatcaccaacgtcgtgttcggcatcgtcatgggcaatgtctatggccgcctgatccagcgggaccgccagcgcgcccgcgcgatgagcggcatggcggcggcgcactgaccgtcgccgatcggacctgagggttcaagaaaaagggccctgcggcgatccgcagggccctttgttcgtcactgacaagccccaacggcgtcagttcagacggccgccgatctgggcgatggcctgatcgaccagtgggtccttgccctggccggccagacgggcggccagcacggcctccgcctgtttggcggcgagatcggcggcggccgccttgacctcggcagaggcttgagcctccgcctgggcgatgcggcgctcggccatctgctggcggcgggccagggtttcctcgagccggaccttggtttcggcctccatgcggcgggcgtcggcctcggcctgagccatcatatcggcggcctgagcctcggcttcggccttttccttgcgaatctgagccagcagggcttcggcttcggcgcgcagacgggcggcctcgtcgaggtcggactggatcttcaccgccttggcgtccagcgcccgcgcggccagcttgggcacgccggcggcgaccaggatgccgagaaagatcagaaggccgacgccgacccacagttcggcgttggcgaggtcataaaggtgagcgtcgaaaaaggcgggcatctcaggctcccttggccgtggccagttcggcgtcggtcgcgccctgcccggtcaggcgctcgaccatggcgcgggcggtgtccgcggcgatggcggagacgttggccatggcggcgtcgcgcgtcaccgcaatctggccctcggcgtccgcgatgcgggcgttgacgacggcttcctcggcggcctggcgggcgttggcctcttcggtgacacgggccttggcggcggcggcggtggcgcgggcgtcggcgcgagccttggcgacctcggcctgggcggcggcggcctgttcggcggcctcggcctggacctgacgcgctgtggcgacggcggtggagatggtgtcggcgcgctcgtccatgacgcggcgcaggcgcggggcgaagaccttggacaccaggaaaagcagaatggcgaacaggatcagcagataggcgatctgtccggcccagtgctcgaaagcgaactggggcaggccgccttcgccgtgtccggcgacctcggcggcggtgttgttgggcacgtgcccggtctcggccgcgtgttcgacggcctcttccaccggcaggaccggaggcggggatgaagagtttgcggccatggtcgtccgtggtgaaagcgaaagcggcggcgcaagcccctgttcagggcgcgccgccgcgaagatcagcgggtcgggatcagccgagccagatcaggatgccgagcacgaaggccaggatgcccagagcttcggcgagagccgcgcccacgaacaggttgccgacttgcgacgcggccgccgacgggttgcgcagcgcgccggccaggaattggccgaagatgttgcccacgcccagggccgagccgatcatgccgagggtggcgaggccggcgccgatgaacttcgcggcttcaggttccatggtattcaatcctagtcaggtgttggaaatcggggtgaagaactgaacccagccttagtgggcgtgatccaggttgaccacatcgttgaggtagatgcaggtcagaacggcgaaaacgaaggcctgaagaaaggccaccaggaactccagcgcggtcagcgccaccaccatggccagcgacaggccggccaccggcagggtggcgaggcccacgccgccgttggcgaaggcgtaggcgcccagcgacaccacgaagccggcgaagatcttcagcgccacgtggccgcccagcatgttgccgaacagacgaagcgccagcgtcaccggacgcagcaggaacgacaggaactcgatggcgccgacgacggggcgcagcaccagcggcgcgctggtgggccagaacagcttgaagaagccaaggccgttgcgcgcgaagccgacgccgatcaccagaagaatggtcagggcggcgaaggtcgcggtgatcgccagttgcgaggtggcggtgaaggtcagcagcagacccaggatgttcatgcccaggatcaaggcgaacagggtgaagacgaacgggaagtagcgacgtccttcgtggccgatgatcgaaccggtcaggttgtcgatcatgccgaacatctgctcgcccgcggcctgcacgcgccccggcaccaccttgggcgaggacgtgacggccgtcaggaacagcacgatcagaccgaagaccagggtcatcgcgacgtgggagttggtgatggccagatcgaccgggcccaacacgggcaggaccacgtcggggaagtcgacgatcttctggatctgaaactgatgaatcggatcggccatgggcctatcggtcctcgtcttccccggcttcctcgaacgggatcggccttgccgtcacccccgccgccttcgcctgcgccatcagccggttggctgtgcggcgcgccatgtaaatcgacaaggcgaagcccagaaggactccgccgatgatgccccacggggtggttccaaggaaccggtccgcgagaaagcccagccccagacccaccagcaccccgccgatcaggtcggcgatgatcttgtaggcctcccccgtcaccttgtgggcggcgaggtccgcagactcctgctgcgccgtgcgcgcctcgagcgaggatgcgctttcggtgaggcgcttgatggcctcttcgcgcgattcctgcatcggggacatgcctttgaacgatcagcacccgacaaccgccgggaacgggtctgaattcggcgcggaacctatccgcgagggccgacaaggtcaaggctgcgtgaacaggcgctaagttgttgccgcagtgcatctatttttcccatgaaggtgcgccgtggcgaagggccgcgccctggcggcgacgagtcggcgcggatcggtggcggcgagccgcgtgagcgactaggttggcgcgcatgaacgtccacgtcgcgcctcctccgcctcgccgcccgctgcacgtgcggctggccacgccgcgcggcttctgcgccggggtggaccgcgccattaagatcgtggagcaggcgctggagaagtacggcgcgccggtctttgtccggcacgagatcgtgcacaaccgccacgtggtcgagcggctgaaggccatgggcgcggtcttcgtcaaggaactggacgaatgcccggacgaccgcccggtggtgttctcggcgcacggcgtgcccaagtcggtgccggcgaccgcccgctcgcgcgacatgctgttcctggacgccacctgcccgctggtctccaaggtccacgtcgaggccgagcgtcaccacgccgccggccgccacatcctgctgatcggccacgccggccatccggaggtggtcggcaccatggggcagctgccgcccggcgccatcaccctggtggaggacgaggccgacgccgagacggttcagcggccgggcgacgcccccctcgcctacgccacccagacgaccctgtcggtggacgacacggccggcatcctggcgatcctgaagcggcggtttcccgaactgccggacccgcacaaggaagacatctgctacgccaccaccaaccgccaggaggcggtgaagcggctgggcgccggctgcgacctggtgctggtggtggggtccaagaactcgtccaactcggcccggctggtcgaggtggcgatgcgggcgggcgcgcgggatgcgagactggtggacgatgcatcccaggtggactggagctggttcgacggcgtggagacgctgggcgtcaccgccggagcgtcagcccccgagccgctgatcgaggcgctgatcgacgccgtgcgcgaccgcttcgacgcgaccgtgaccgaggacgacggcgcgcgcgagaccgtgaccttcaagctgccgcgcgttctgaccgcctagcggtcctcgcccacgaaatcccgggcgaactccggcgcgtcctcgggctcgagcgggtcctcgtcggcgccgcccatgcggccgggatcgggcacgtcgaagccggcgggcatggacaggtccagcaggcccgccgccttcatctcggccagtcccggcatgtcggacaggttcgccaggccgaaatgctccaggaagcggtcggccgtggcgtaggtcacgggacggccgggcgaacgcctgcgtccccgcaagcgcacgaagcccatctccagcagcacgtccagggtgccgcgcgacagggacacgccgcgcacgccttcgatctcggcgcgggtgacgggctggtggtaggcgatgatggcgagggtctccagcgccgcacgcgacaggcgacgcggctcctcgcgctgctcggtcatcaggaagccgaggtcttcggcggtgcggaatctccagcggccggcgacctgatccagctcgaccccccgcccggcgtagcgttcacgcagccccgcgagagcgccttccacatcggcgccgtccggcaggcgggccgcgatctcggccgcgccgagcggggcggaggcggcgaacagcagggcctcgacctgacgctcggtctcgccggcggtcgtcaaggcgtcagctccagcggctgacccgcgtggcgccgcttcagcagcaggtcgtcgaaaggtcgcgactgccgtacgtccatggcgccttccttgaccagttccaggctggccgacagggtcgaggcgacgtagctggcctgggtggggccgtcctcctcagtgcgccggggcgcgacacgctccagcggggtccagtccaacaggcgcggcatgacctcgcgcaaccagtcccgcgccgcctccagcgcaaaggcctccacgcgggcggtgggggcgtaacggcgccgcacctgcctttcgcgctgggacacataggccgtcatcaggtcgtacaggctggcctcgacccggtcggagggggtgatgacgacctgctctgggtcgccgcgcgtgaagacgtcgcgcttcagctgcggtcgctcccgcaaggcgtcggcgccgcgccggatcgcctccagcttgcgcaagcgataggcgagcgcagccgccatctcttcggccgggggctcctcggccttgccgggctcggtgcggggcagcagcaggcgcgacttcagataagccagccacgaggccatcacgaggtagtcggccgccagcgcgaagttgcgccgacgcgcctcgtgcacgaagcgtagatactgttcggccagttcggtgatcgacagcttcagcagatcgacccgctgatgccgcgccagctccagcagcacgtgcagcggcccctcatagccgtccagatcgaccacgaacgcttccttcggcgcggcctgttcggcggccgaaaagtccagatccggctggaacggctgcatgaaggttattgcgcctcgccgacgtccgggccctgggcggcgtcggtgcggcccgccatggcctgatggaaccgcgcatgggcggcggaggcgtccagcggttcgggcgaccggacgacccgggccatggcggcctccgcgcgggccttcgccctgcccttcagcttgccgacggcggaggcgaccgcctgcatctccgccatgtcgccgttgcagtgcaggacgatgtcgcagcccgccttcaacgccgcatgcgcccgctcgtccagcgcgccggacagggcctgcatcgacaggtcgtccgacaggatcagcccgccgaagcccaactgatcccgcatcagccggatggcgcgtttcgacgtggtggccggacgcttcttgtcgatggcggtgaagacgacgtgcgcggtcatggccatcggcatgtcggacagagccctgaacggcgcgaagtcccaggcgtccagcgtcgccaggtcggcatgcaccaccggcagcgtcttgtggctgtcggcaaaggccctcccatggcccggcatgtgcttgatcaccggcaggacgccccctgccagcagtccctccgccgccgcgcgcgcgagctgcgccaccgtggccggatcggatgcataggcgcggtcgccgatgatgtcgtgagcgccgggcaccggaacatcgaggatgggcgcgcagtccaccgtgacgccgacctcgcgcaggtcgtgcgccatcagccgtgcgcccagccggatcagggtgcgggcctccagcggaccgttcgccgcctgcagataggcggcgcccggcggatatttgggccagtgcggcgggcccatgcgctgaacccggccgccttcctgatcgatcaggaccggagcctcggcatcgccgatcgaacggcgcagatcgtccgtcagcgcccgcacctgttccggcgtttcgatgttgcgccggaacaggataaagccccacggccgcgcctcggcgaagaaggcgcgctcggcctccgtcagccgaggtccggaacagccgtagacgacggcggtcgtcaccggacgatgcagtcgcggcccgccgccttcagcgcgttgcagaaggcggtcgcccgctcgcgcgacaggccggcgaaggtggtgcggtagacggtggagccgttggaggccgtcacctcctgcacccgcttctgcgcgcccgacgcataggagccgaagcgcgccgccacggcggcgtattcccgatcggcgatggcggtggaggaaaaggcgccgatctgcacgcccgacgacccggttgcggcggcggacgcaggcgcggccttttcggccggagccggagccggacgcggcgcggcctctgtcgggcgagccggcgccggacgcgcaggcgcgggcgccgcgacgggcggcaggccctcgccggtgacgggcgcgggcgcaggcgcggccggtcgcgcctgaggcgtttcgggcggggcggtgaaggtcggcgcggcgtcggccgcttcggtttcgtcgcgatagacccgcacgccctcggccggatcgaccggctgggcctccagcggcgcgggcgtggtcatctcgccgaccggctggcccacagccggcggtgcgtccgtcgaggagcgcaggcccgagcgatagaagaagatcaccgccacgatcagcagcagcagcaccgccgcgctgacgatcagggtgacgggcggcgccttgcgcgcgccggtcgcatagccgcgctcctgacgaggatcgaatgcgttgcgccggaacggcaggtcgtcgtcgtcggtcggcggggtataagcaccgcgctcgcgatcctgattccgatggttgtcgtcgaatgacatggtcgcgctccgcctcgatccccgcgcgaatcgccgcaggggtcacacagtctagcccgccatcccccgcttacgaatcacagatccagcgcgaggtcgaggctgaacagcttcttgtgcacctcgatggcgtagcggtcggtcatgccggcgatgtagtcgcagatggcgcgggcgcgagcgtcgcggtcctcggtgcgggcgggatcgccccactccggcggcatcacctccggctcctccatgaacagctgaaacagctgggccagcatgcgccgcgcctggctgcgggtgcggttgacgcagtggtggcgatacatccgctcgaacaggaagcgccgcagcacgcccagttcggccttcagcgcgggcgagaagtccaccagcgtgcgcgcggccgtgcgcacgtcctcgaccgagccgatgcggtcctgctcgatccgccgcgccgtctcgttcagcacgtcgtcgaccatgacgccgatcatgcgccgccccgcctccagcctcagcatgcggtcatcgacgcccgaccagtcgcgccgcgcctcgctgaggatcggtccgatgatcggcacatcggccagctcgcccagggtgatcagccccgcctgcaccccgtcgtccacgtcatggttgttgtaggcgatgtcgtcggcgatggccgcgcactgcgcctccagcgaggcgaagccgcccagccgcaggtcccatcccgccgccccgcccgccgcataggcgcggactgaggaccaggccggctcgtccagccgctgggtcaccgggccgttgtgcttgatcacgccctccaccgtctcccacgacaggttcaggccgacgaactgcggatagcgatgctccagctcggtgacgacgcgaaagctctggacgttgtggtcgaagccgccgtggccctccatctgcaccaccagctcgtcctcgccggcatgggcgaagggcggatggccgaggtcgtgcgccagggcgatggtctcggccaggtcgtgatcgaggcgcagcgcatgggccagcgagcgcgcgatctgcgccacctccaggctgtgcgtcaggcgggtgcggtagtgatcgccctcgtgcgccacgaagacctgggtcttctccttcagccggcggaaggccgtcgcatggatgatgcggtcgcggtcgcgcgcaaaagcggtgcgggtgcggctggggggctcgggaaagcggcgcccgcgagaggcgtcggcgcgttcggcgtagggggcgagaggcgtctggctcaaagggtcacgcacgcaatgtgatggccgcgggccttggcgctcgcccgcctgcgcctcatatagagcgtcgtgagcagcgtccaatccacagaaccgtccacacccgccttcgccgtctccgcacgcgcgcccgaaggcatccgcctggcctccagcgcggcccggcggctggccaagctgtcgcagatcgagggtcgcgccctgatgctgcgcgtcgcggtggacggcggcggctgctcgggcttccagtaccggttcgagctggtcgagggcgccgaggccgacgacttgcgcatcgagatcgacggccagacggcgctggttgatccggtctccatccccttcctgaagggttctgagatcgcctttgtcgacgaactggccggcgcgcagttcgtggtcaacaaccccaacgccgcctcctcctgcggctgcggcgtcagcttctcgatctgagaaacaaccgaacagacgctcgtggacggccgaaaatcgattaggggcttgactaatcatcggcagtgattagcttagctgctaattaggagttatcctatgaacactctgttcaaggcgctgtcgcatccggtgcgccgccgcatcgtcgccatgctgcgcgccggtccgttggcttcgggcgacatcgccgccaccttcgacatgagctggccgaccatcaccggccacctcaacgccctgaaggaagccgggctcgtcagcgctgagcgcgatggccagaccatccgctatcggctcgagatctcggcgatcgaagaggccatggcctttctgatggacatcgccgggacaggtcagccggcgacggtcgcgaccaaggcggcccgccgatgaagcatcgcctctccctgatcgatcacctgacgatcggcgtcttcgccatccaggccgccttcgccctctacatcggtctttatggccccgccacgccgatgccgatgcattggaacagcgactgggaggttgaccgctggggcgaccggatcgacttcgcggtccagtccggcggcctcgccgtgatcggtctattggccgcgggcggcctgggcctcggcgcgatccgggccgccgcagagggcgatgcggcgcgctgtcgctcgttgcgcatcgcacaggggatcagcctgttcaccttcgcggcgatcggcctcttgatcgtctggaccgggctgggccatgcgacggcggagaccggcccggccgtcgccatggccggcgtgtcgatgatccttctggtcacgggcgcctttctcggccgggtcgcccccaatccgctggtgggggtgcgaacgccgtggagctacaagagccgtctggcatgggatcgctccaaccgcctggccgggcgtctgctctgcctgctgggcctggcgggcctgatcgccgcgcccgtggcaagtcagccggccggaacctacggacttgtcgggggcgcgatcctcagcgccgttctctcgatctttgaaagctggcgtgtctggcgcgccgatcccgaccgccagcccttctgatccaccaaaggagaccgcccatgtccagcctcgccgcctccgccgcctccgccgccctggtcgtcctgatggccggccctgtcccaaccgagatcgccctcccagcccaacccgcgccgctgcacgggacgctgttggccccggagggcgaggtggcggccgtggcggtgatcctgccgggatcggggccgaccgatcgggatgggaacagcccgctgggcattcgggcggcgacctaccgcctgctggcggaaggcctggcggaggacgggatcgccacggtgcgcatggataagcgcgggatcggcgccagcgccgccgcgggcgggagcgaggccgatctgcgcttcggtgactatgtcgcggacgcccgcgcctggacgagcgaagccgtgcggcggacgggcaagccttgcgcctggctgatcggccacagcgaaggggcgctgatcgcgacgctggcggcggagaacaatccggaggtctgcggcctggtgctgctgtcgggcgccggacggccggcgatcaccgtgctgcgcgagcagttccaggccgtgcccgagccggtgcggggtcaggccctgacgatcctggatcggctggagaagggcgagacggtcgcggacgtgccgcccgctctggccgcagccttccggccgtcggtgcaaccctatctcgccagctgggcgccgctggacccggccgaggcgctgggccgctatcgcggtcctttcttcatcggccagggcgaaaccgatctgcagacccgggaaacggatgcgcaggcgctgaaggcggctcggccggacgccacgttggtgatctggcccggcgtcaatcatgtgctgaagaccgcgccggccgatcggcaggccaacatggccgtctatgtcgcgcccgacctgccgctggctcctggcgtcgccgaagacgtggcgggcttcatccgcgagcacacgccctcgcactgaggcgtcaggcggccagcgtctcggtgaaacgcaccggccggccgtgcgcctggccgatcagttcgccgtcctgcatcaccacccggccccgcaccaccgtggccatcggccagccggtcgcctccacgccgtcgaacggggtccagccgcagcgagtcgcctgctggtcgtgggtgatggtgcgcctggccttcagatcgacgatggtcaggtcggcgtcatagctgaccgccattcggcctttgttggccgtgccgaagacccgctgcgcccccgccgaggtgaggtcgatgaaccgctccaggctgaggcgcccgttggcgacgtgcgtcagcatcagcggcaccagggtctgcacccccggcatgcctgagggcgaggccggatagggcttggccttctcttccttcgtatgcggcgcgtggtccgagccgagcacgtcggccaccccctgctgcatgccccacaaccacagcgcatccacgtgctcctgcgaccgaatcggcgggttcatctgggcgtaggaaccgagtcgctcatacgcctccggcgcgacaagggtcaggtgctgaggcgtgatctcgaccgtggcgacatccttgtggaagcgcagatactccatctcgtccttggtcgtgacgtgcaggacgtggatgcgcgcgcccgtctccttggccaggccgaccaggcggcgggtcgaacgaatggcgctctcggcgtcgcgcacctccgggtggctggtccagtcgcccgcacgggccaggccgcgccggtccgccaggcggtattcatcctcggaatgaaaggtggcgcgccggcgcacgttggacagcaccttgcgcacaccgtcgtcgtcggcgatcagcaggtcgccggtcgaggcgcccatgaacaccttgacgccgcagcagccgggcagccgctccagttcgccaagatagtccgcgttctcgtgcgtgccgccgacgtagaaggcatggtccgtccacatccggtcctttgcgcgcgccagcttgtcggccatggtgtccggatcggtcgtattcggatttgtgttcggcatctcgaacacagcgacgacgccgcccagggccgccgcgcgtgatccggtctcaagatcttccttccattccagtcccggctcgcggaagtggacctgggtgtcgatcacgcccggaaggaccgtcagaccggaggcgtcgaacacctctccggccgaggcctggctcaggtcgccgatgaaggcgaccttgccatcgatcacccccacgtcggccatgccgcgccccgcgtggttcgccacttcgccgccgcgcacgatcaggtcataggtctgggtcatgccgtgacctgtaaccccgcacgcgcgcggcgagaagacgccccgtcgccgaaagggctgtgctagaggcccgcgtaatggagccctgcccgtgtccctgccgctgatccccgaccgcacctgcggcggctgcgtggagtgctgtcgggtcattccgctggacctgccggaactggccaagccgacgggcgagctgtgcgcctattgcgtgccggacgccggctgtggggtgcacgccatccggccgcagacctgccgcacctggttctgcctgtggcgggcggtcgagctgtcggacgactggcggcccgaccgaagcgggatcgtgatccgacccgacggggtggagcatggcgagatcaccctgttcgtggtgcgccgctccgatttcctgcagtcggaagaggtgttcgagacggtcgcagggtggatcgatgccggcatccaggttgcgctgagcgtgcccggcccgatcgggacctatccggcgcgggccgtggtcaccgactatctgcgtccggcggtggacgcgggcgacgccgagcgtttccaccagctggtcgcgcgttcgctggacaagctgggcgagcacgactggcaggccgacgggatcgaggcgcgctaccgcgtcacctgacaggggcggcgcccgcgcctatctaggccgcatgacacgcatcgcccgcctggacagccgcgccctaatctccgtctcgggagacgaggccaggccgttcctgaacaatctgctgacccaggacgtggagacgctggccgacggagaacttcgtttcggcgcgctgttgtcgccgccgggtcggctgctgttcgacctgttcattgtgggcgaaggcggcggcgtgctgcttgacgtggcggcggaccgaagggaggcgctgctgacgcgcctgtccatgtaccggctgcgagccagggcggacatccgcgccgacgaccgccccgtgttcgccgcctgggacggcgaggcggcgggcttcatcgtcgatccgcgcgcgccggaactgggcggccgggcgtatggcggcgaacacgagacgaatgcgagcgaggacgatcacaagacccatcggctgtcggtgggcgtgcccgatccggcgatcgacgccccctcggacaagacctatcccatcgaagcgaacttcgacctgctgaacgggatcgacttccacaagggctgtttcgtcggacaggaaacgacctcgcgcatgaagcggcgcggcgcgattcgcaaccgcatgctgccgatcgccttcgacggttcccctcctccgttcggcgccgaggtgttgaacggcgaccttcgggccggcaaggtgctgggcggccgggagggtgcggccatggcgttgctgcggctagaccggctggagggtcagctgacggtcgacgggcggccggtcacggcgcgtcggccggactggatgcctgcgacctgagctactgcaccgactggcgcggttgctggccggcgtcgcccgcattgtagggctgaggaccgacggggggcgccgcggggcgaggcgcgctttccgtccggcgagccgtggtttgcggacgcggggccgggcgcggcgcttggcgcgcagcggggcgcggcgcggcgggcttggcctccggaacggcaggctgggcggcgggcgtcggccccggcgtcgcggcgggggccggagcgggttcggcggcctgggcggcggcggcgcgggcggccatctgctgagcctggaagcgggcggcgagcttttccgtcagttccttggcctgagccggggacatctggaccatgatggcggccagggtgcgcggacgcatggcggcggcgactggcagacgcacccggtcttccagcgaggccagcaccggcgccgcctccttgggccgcatggcggagtagacctgcaccagacggtcgatctcggccttttcgcgctcgtccacctggccgagcaggccctgcatctcggccttcagcgcctccagcgccttgaccttggcgtcgatcttctgctcggcggcgaccatcagcggcagggtggtggcgaagtcctggtcgcgtgcgtccagctcggtgcgacgggcggacagcgactggatgatcttcagttcggccggcgaaatgcccgcctgctgggccagctggtccggcgacagggcgcaggcggcctgggcgggcttgggcgcggcggcgccggcgggggcggccccctcggccccggccttggccccgctgaacaggtcgggcgcaacgcccaccgcgcgcacggcgaccaccccgccgatggcgatggcgatcaggggcagcaggcggggaatgcgggccatgggcttcggtctcgtggcgccctcaagccgcttcgtcgtcgcgcggcgaagcatggggcggtgtaatttggtcaggcggcgaacaggtcgtcgtccaggctacgacgggcggcgttgaggctttgtttggcggattggttagcggtcatcgcctgaagaatggcggcgacgttgccggcgcccgggttctgctccggcgccgcggcggcccggcggctggtggccaggcccgcgaggccctgaattcgctcggccagggcggccatgcggcgggcgcggtcgtcgtcttcgaccgaggcggcgaccggggtcgcggtctcagcgccggcggccgggcgctcctcgatccgcgtcgcaatggaagccgtcggcgcgcgggcgatcagcgtctccagctgcgccttcacctcgcgcgccttgatgatgcggtcgtgcagcagatcggtctcctggccggacgcccgcagggtcgcgagcgcggcctcggcgcggcttgcggccgagttcagctcggtcacggcggaggcgaacgccagttgccccgcccgcagggccgtcagcttgcgttccagcttgacgccgtagccgaccgccgcgaccagcagcagcatcagcacgccgtccatgatgaccccggtcatgccctgctcctcatgctttgcgcggcttcgacgctgatcggcgcctcgacgcggatggcgatgttctggcccttgcggcccatgcggccggtggtcagggggatggagccggcgcggatcgacacctcgctgtcaggggtcgcgttcagcatcagggtgtcgcccaccttgaagtccagcacggtgctgagcggcgcctgctgctcgtccaagaccgcccggacctccgtctcggtggtccagagctcggtggcgaggtggccttcccagatgttgtcgcggccgaacttctcgcccatgaactgctgcagcagcatcttccggatcggctccagcgtcgcatagggcagcagcagttcgatacggccgccgcgatcctccatgtcgatccgcagcttgatcaggatggcggcgttggccggccgcgcgatggcggcgaagcgcggattggtctccagccggtccaggttgaagtggacgggggtcagcggctcgaacgcctgacgggcgtcgttcagcaccacctcgaccatccgctgcaccagcacccgctcgatggtggtgtagggccggccctcgatccgcagcgccgccgtgccgcgccgcccgcccagcagcacgtcgacgatggaatagatcaggttggaatcgaccgtcagcaggccgtagttgtccagctcttccgccctgaacaccgccaggatcgccggcagcgggatcgagttcagatagtcgccgaaccggatcgaggagatgttgtccaggctgacttcgacgttgtcggaggtgaagttgcgcaagctcgtggtcatcagccgcaccaggcggtcgaacacgatctccagcatcggcaggcgttcataggacaccagcgccgagttgatgatggcccgaatgcccgaccggccagcgccgtcatcgccgccgagatcgaagcccagcaggctgtcgatctcgtcctggttcagcacgcgctcgcccatggtcgagccggcgtcgccgcccagcgcgccgaatgcgtccatatcggccaggggatcggtcatcgggctactggaccagcatctcttcgatcagaacggcgtcgaccttgcccggcgcggccagcaggttgacgcggcgcaggatctcggcgcggatctgataggatccggcggatccggccaggtcctcgggccgcagctcgcgcaggaagctctggaacatgtcctgcatgcgcggggtctcttcctgcagatgggccgcgacctcggcgtccttcatctccagcgtcagagtcagcttgaggtaggtgggccggccgtccggcgactggatgttcgccaccatgttgggcagggtgtagaaggtcacgccgtccggcccctcggaaatcttgccgagcgcgggatcggcctccccttccttgccgccgccgtggccgcccttttcttccttcttttccttgccgtggcccttttcggccttctcttcgccgtgcccgtccttggcctcttcgccgtgggcctcggcgggcttgggcttcatcaggatcatggccgccgccccgccgccgcccagcacgaccagcgcggccggaatggcgatgaacagcagcggcagcttcttcttcttgggcgcggcgtcgcccccctcgccttccgtgacgacgggcaggttggcgtcggccgaagccgcgtccttctttttcttgcccagcttcaacatggccgcactcgccccgcaggatgtcgcggcaacagtgtccccgtttggttaacgcgccgtttagaagcggcaggatttgccgggctgcacaggcgcaggcgctgcggagagcccgccgttgctggattaaccctgttggcacgggcgttgcgacaagggtcggcgaaggagccgcccttttggaaaacgccgcctacatcggattgtcccgccagatgacgctgcgccgcgagctcgacatcgtggccaacaacatcgccaatgcggacaccaccggcttcaaggtcgaacagctgatgctgggcaccgaggtgggcgagcgcgcccgcaacgatcaggtgcggccgggcgtcagcttcgtgctggacaagggcgtcggccgcgatttcggccagggcgcgatgcagcagaccggccggccgctggacttcgccatcgacggcgaaggtgccttcttcaccgtcggcgacggcgcgaacggcgaggcctacacccgcgacggcgccttcaccctggacccggaaggccggctgaccaccaagtccggcgcgccggtgctgggcgacggcggcgagatcgtgctggacccggcgctgggccccgtgtccgtcggcgcggacggaaccatcacccaggacggccagaccaccggccgcctgtccgttgtgcgcttcgaggcgctgggcgtgctcgagaagggcggcgacggcctgtatcgcaacacctccaacgcccagacgatcgacgcgcccgacgcccgcatccagcagggcatgcttgaggcggccaacgtcaatcctctgatcgaaatcaccaatctggtcgagatcagccgcgcctacgaaagcgtgacgcgcatgatcgagaacgccacagacctcagccgccgagccgtcgagcgcctcggccgagccgcataagaaggaccccgacagatgcgcgcactcagaaccgcagcctcgggcatggccgcccagcagctgaacgtggaggtcatctccaacaacatcgccaacatgaacacggtgggcttcaagaagcagcgcgccgagttccaggacctgctgtaccagaacgtcgagcgcatgggcgcgcagtcgtccagccagggcacggtggtgccgaccggcatccagatcggcgcgggcgtcaaggccggctcggtctatcgcatcaccgaacagggcacgccgacgcagacgggcggccgctatgacctggccatcgacggcaagggctatttccaggtgacgctgccttcgggcgaaaccgcctacacccgcgccggcaacttcgccgtcaaccaggaaggccagttggtcaccgaagacggctacgccatcgagccggccatcaccgtgccgcaggacatggtggacatcaccgtctccaaatccggcctggtgcaggtcaccaccgatggcgcgaccgagccgaccacggtggggcagcttgagctcgcgaccttcttcaacgaggcggggctggaggcggttggcgacaacctgctgctggagaccgccgcctcggggccggccaccgtcggcacgcccggcgacgtgggttacggctccctgctgcacggctacaccgaggcgtccaacgtcgatgcggtgtcggagatcagcgcactgatcgtcgcccaacgcgcctacgagatgaactccaaggtcatctccaccgccgacgaaatgctgtccgtcgccgcccaggtgaagaactaggccatgaagaccgtgatctgcatcgcagccgccctgctcgcctccgccgctcccgcatgggccgcagaggtcgtcctgcgcgccaatcccgtggacgccgatggccgggtcaccctgggcgacatcttcgagggcgcgggggcagcctccgaggtgatggtggcgcagcgcaacggcccgtccgtggtgctggaggccggccagctccaggcccaggcccggcaggcgggtcttcagtggtccaacccgaccggcctgcgccgcgtggccgtgcgccgcgccgccgccgcgctctcggccgccgcagccgtcgaaccaaccgttccttctgccactgtctcgcctcatcgcgaggccccgtcggccgccggcgggtcagccgtgatcgcccgcaacgacatgattcgcgtctcctacgaggtcggcggcgtccggctcagcgtcatgggcaaggcccagcgcagcgctcgcgtcggcgagcccgtggccgtcctgaacaccacctccaaccgcaccatcgacgcggtcgccaccgggccgggcacggccgtggccgccggcgccgcccaacagttcgcgtcccgctgaggatttctcccatgcgtaaagccgtcttcttcgccgccctcgccgtctcggctgctccgctggctgcctgctccaccgccatcgaggcggtcaaggggccggaactggcccccatcggctatccggccgccctggtcccggtcagccaggcctatctgccggccagcgccgtgcgctcggaagcctcgcccgccagcgccaacagcctgtggcgcaccggcgcccgttccttcttcggcgaccagcgcgcgcgccacatcggcgacatcctgaccgtccgcatcgacatcgacgaccgcgcccagacgcagaactcgacccaacgccagcggtcgaacgacgcctcggcgggcgtgtcgaacttcctgggcttcgaatccaacctcggcaaattcttccccgacacctttgatcccaatcgcctggtgggcatcgagggcgaactgaacgcctcgggctccggctcggtcagccgctcggagaaggtgtcgctgaccatcgcggcggtggtcaccgacgtgctgtccaatggcaatctggtgatccagggccgccaggaggtccgcaccaaccgcgaagtgcgcgagctgacggtcgccggcatcgtgcggcccgaagacatctcctcggccaacaccatcgcccacacccagatcgccgaagcgcgcatctcctacggcggtcgcggcgacatcagccgggtccaggcttctccggccgcccaaagcctggtggagcgcttcagccccttctgagggcgatgccggggcgccacaccctggacgtgcgtcagctgagccgtgaaccgtccgcgcgaaccggcgttataccccggaacgcgagcgcatccccatgttcaaggtcctgatccccgccgtcgccgccctcggtctggtcgccttcaccgcccagacgcaggaggcgtccgcccccgcccagcccggtatggcctggcacctggtgcaggaaggcgagatggccaagctcgcctacggcatggccgattccgaccagctggcgctgatgataacctgctcgcccggcgatcgcacggcggtcgtctatggcgacgtgcagccggtcggcgcgcggaccctgacctcggctcccgcgccgatggaccccatgagcggcggcgatgcggacgaggcgcgcatctcgatcaacgactccaatcttgcgaatctggcgcgtcgcggtgcgatccgcgtcagcggcgaaggcggcgagaccgtgctgaccgccacgacggccgagcgccggggcgtgcggggcttcctgtcctattgcggttccgctcgcgtctgaggatgatcggcgcgggcgcggtcgggtcgcctgatttcggatgcttgcatgaagccggtcctcttctgcatggccgccctgctgcttggcctgaacgccgcgccggacgccgtgcatgcccagtcccgtccggccgaccggtgggtctggtctttgtacgagagcggcgggtcggtcgtgctggccaatgaggtcccggacaccacgcagctgagggcgacgctggagtgtacgcccggcgagggcatggcggtcttgtcgctctatgaccctcaggccgggcccggctttgcgcgcgtgacggcgggaacggcggcgagcgcggtggaggtgcgggccgcgcgcggcggcaaggtggagacgaccttgcgcctcgaccatcccgtcttcgccgcattcgtcgcgggcggcgagctgacggtggcgacgggcgagcaccgcacggaggtgcgcgccgaacccgagtttcaaggcctgctgcgccgcttcggcgagcgttgcgcgggatcgcggtgatgaggcgggcctttgcggcgcgcccgacgatcgtgacgctgggcgtactggcgctgagcgcctgcgccacgcctgcgacccgcgcgccggatgctgttgcggacagcggcgctccggccccgacgctgggccttgagtggttcgaccacaaggatggagacgccctgtcgctggcttacgggcgcgaaaccagcgacgacctgcgtcttcggctggattgcgacgccgggtccggaacgttgacgctgaccgctccggcggaaggcgccgacggcatgatccacctcgagtccggcggtgacaccgagcggttcccggcggtgagggagtcgtccggcctaggcgacggcgatctgctgatcgcgtcggacgtcgccttgcgccagccggtgtttcagcgcttccgcgcggttggctggatcgccgtctggcgaggggatgcgcgcgaggtctatgcgccgcacacggggtccaaagcggcggtgtcgcgcttcttcgacgggtgcgacccgggctgaccggcggctcttgacgacgccctcgccctcgggtgctgtccccccgcgcgaacggggaaacgatcatgaaggctctgcaactggctttggcggttctgctggcgacgggcggcgcggtcccggtcgcggcctcacagacggcttcggccgtccgccccccggtcgatccggcgctggacgcgatcgtgcgggattacgaggcctatctgaagtcggtcgatccgatatcggcgggatccgagggcgatgtcgaggcgcagggccgcctgcccgacacttcgcgcgcctttgagctggcgcaggtccagccgatgcaggccttcgtggctcgcctcgaggccctttcgcccagcagcctgagcgaagccggccgcatcgatcaggcgttcctgctgcacacgctgaaacacgccctggccggcgttccgctggacgccggacggctatcgttcgactccgagggcggacccggaagctgggccctctacatgggccagagcacgcggctgtcctccgtcgccgaagccgaggcgttcgtgcgtcgcatccgaggcttccccgacatctaccggaacgcggtcgacaacgcccggcgtgggctggagaccggccttatgcagcccgcctcggtcgtggacagcgccatcgccctggcgcgcaacgacgtggccataatgccgggcgacgagccgctgatgcagcccttcgccgccctgccctccaccatcccggcggccgagcaggcgcggttgaggcgggaggcgcaggccgccgtcgcgggcgtggtgcaggcccggcgcgagtggctggcgttcctgacggacgactatcggcccaaggcgccggacgcgcccggcctcgcaaaccgccccggcggcaaggcgctatacgcccatctggtggctggccacaccaccaccgacctctcgcccgaccagatccaccagatcggtttgtcggaggtcgcccgcatccgcgcgcgcatggagaccgagatgaaggccgccggctggaccggcgatttcgcaggttttctggcctttctgcgcaccgaccctcggttccacgccgccagccgcgaggacctgctggaaaaggcttcggagatggccaagcgcgccgacgacggcctgccggccctgttcggcgtcctgccgcgcctgccctacggcgtgcgcccggttccgcgcgagatcgaggagaactacaccaccggccgctacaatcccggctcgatcgtcaatggcgtggccggcggctacatggtcaacacctcgcggctggatcagcgaccgctgtatgagctgccggccctgacgctgcacgaggccgtacctggccaccacatccagatcgccctgcagcaggaggcggaggaccagccctacttccgccgccaggccaacgtcagcgcctacaccgagggctggggactctacgccgagttcctgggcgaggaaatgggcttctatcgcacgccctttgagcggttcggccgcctgtcctacgagatgtggcgcgcctgtcgcctggtcgccgacaccggcctgcactggatgggctggagcaccgaacaggcgcgcgcctgcttccgcgacaactcggccctggctccgcacaacatcgagaccgagcttcagcgctacatcggctggccgggccaggccacggcctacaagataggcgaaatccgactgcgggacatccgcacgcgtgcggagaccgcactgggcgaccgcttcgatgttcgcaccttccacgacgctctgctggtggacggccctctgccgctggacctgctggaccggcgcatggacgcctggatcgccgaacaggccgcgcgctgagccgtcaggcccagggcggcgtcggcagcccccgcgcgcgcaggaagtccgggttgaacagcttcgcggcatagcgggcgccgccgtcgcacaggcaggtgacgatcgtcttgcccggaccgagctcgcgcgccagccgcaccgcgccggcgatgttgacccccgccgagccgcccagcgacaggccctcgtgctccaccaggtcgaacaggatgggcaggaactcggcgtcctcgatgcgataggcgtggtcgggccggaagccctgcaggttgccggtgatgcgcgcgacgccgatgccctcggtgatcgaggagccttcgcccttcatctcgccgcgggtgaaccagctgtgcatcgccgcgcccgccggatcggccaaggcgatgcggacctcgggctttctttcgcgcagatacgccgacacgcccacgatggtgccgcccgatcccactgcgctgacgaatgcgtcgatcactccgcccgtctgctcccagatttccggcgcggtggtgcgatagtgggcctcgcggttggcgacgttgtcgaactggttggcccacagggcgccgttcggttccgacgcgtccagctctgaggccaggcggcccgaatagtggacgaagtggttggggctggagaagggggcggcgtccacctcgatcaggcgcgcgccgaggctgcggaccgcctgcttcttttcctcggactgggtccgcggcatgaccaccaccaccggatgccccagcgcggcgcccaccagcgccaggccgatgcccgtgtttccggccgtgccctccacgatcaccccgcccggcctgagcgcgcccgacgccctcgcaccctgcacgatggagagagccgcgcggtccttgatcgagccgccagggttcaggaactcggccttgccgaggatttcgcatcccgtctggtctgacaggcggttcagacggatcagctgcgtgcggccgatcaggtcgacgatggagcgggtggcgatcaagggttcagaacattctcagaggctggccagccctcactgaccccgacgcccttgcttgtccatgcaaagccggttgtctcgggcgcgcttataggttttctgcaaggcatggcccgaccgatgctgccgctgaacgccctgcgcgcctttgaaagcgccgcccggcatctgaatttctcgcgcgccgccgacgagctgtcggtgacgccgggcgcggtcagccagcagattcggattcttgaagacacggtgggcgcgcccctgttccggcgagaggcgcgggggctggtcctgaccgatccggcgcgtgcggcccatccgctgctgcgcgaggggtttgaacggctggccgaggcttcggccctgctgcgcgagccgccacggcgacggcaggtggcgatcagcgtcgcgccgtcgttcgcctccaaatggctgatgccgcgcatgaacgacttccacgccgcgcatccggacgtggaggtctggatttcggccgacatggagccggccgatctgaacgagggcgcggtcgacctggcggtgcggtacgggcccggcgactatcccggctatatcgtcgagcggctgctgaccgagacggtgctgccggtctgcgcccccgccctgatgcgaggcgagcatccgatccgccggccggcggacctgatccaccattccctgctgcacgacatgagcgacgacggcgatccgggccgtccggactggcccatgtggctgaaggcgcgcggagtgcgccatcccgatccgcgccggggctcgcgcttttcgcagtccggcctgttaatcgaagcggcggcggccgggcgcggggtggccctggcccgccacaccctggcgcaggcggacctggcgtcggggcggctggtcgcgccctttccggacggcagccagagcgtgggctacgcctatttcctggtgcagccgcgcgcgcggccggcgtcgctcagcacgcaggcgttcgtgggctggctgcggcgtcaggccgtcgatcacgacaacaacctggaccaactctgagtccgaaggatcagtggccgatcagattaggaagggtctgatagacgatgccgatcaggccgatcgcgccgcccagaaccccgagctgaaggctgaaccgctccacctccgcgcccgtcccccggcgcagcgccatcgccggcagggcgatcgccacaccgcacagaagggcgcaggcgacgctgaacgccaccccgcccatgcgccaggcgaaatcgtccgacgtggcgaccacatccgcgacgctggagatcagatagacgccgaggaagtgcagcgcccagatcgacagccccgccagcatcagcgtccacagccggatggtcatgcgcccgctccggggaacaggcggaccagcagcacgcccagcgcaccttgggtcgccgaaaacatcaggaacatggcgatcaggtccaccgtcgaggggaaccggtgcgacatgcggcgcgccgcccatcgcagcgccacgaatagagccatcagcaggcagatgcccgaggactgggcctgccaggcgatcagaaagccgacggtcgcgccctggctggtgtcggtggggcgcagtccggtgtcccaccagctgaagccgtccagcagcagggcgcccgtcagcgcggcggcggccatcacgatcaggccggccgccaggccctgccaggcgcggccctcgcggcgggtcgcgcgcgtggcgaaccaggccgcgcccgcgcaggtcgccagcagagccagcacgccgatcagggtgaggacgtcgggtggcgcgatccacagatccggcctgcggctccacaggaagacataggagaagccggccatgaccgtgatcatgcccgacacgatcagggtgatggccatggcccaccagccgtgactggtcggaccggacacataggtcggcaggatcacgccgccgcctacgtccacggcctcaagctcattgggcgcatccagcttccaggcccacttcatgatgcagtagatggccaggacgccgctgatcagcgacacaatgtaggcctgcaccgtcaggatcaggaagaagccggcggtgaaaaccgcgccccacagataccaggacgatggtcgcggcatccgcagcacgtactgcggctcggcgttgatcgggctggtgacgatggtctggcgctggttcagcggcgcgcccggcaggaaccagcggccgtcctcgacctgcttggacagttcgggctggtcccagacgggatacaggctcttcaccacggggatggagcgcagcgagtagaggccggccggcagccactccaggcccgggccgttgtagacgttgcccgcgtcctttccgaagggccggaagttgcggcacatgtcgatcacccacaggatcaccgccagcgccgtcaggaacgagccgaccgtggagatgaagttgagcaggtcccagccccgccccggcagataggtgtagacgcgcctgggcatgcccatcagcccggtcaggtgcatgggcaggaaggtgatgtgcatgccggcgaacatcagccagaagatccacttgccccaccgctcgctgagcggtcggctggagctcatcgggatccagtagtagatcgccgcgaacagcggaaacaccatgccgccgatcagcacatagtgcaggtgcgcgacgatgaagtagctgtcgtgcgcctgccagtcgaacggcaccatggcgaccatgacgccggtcagcccgcccatgacgaagatcaccaagcctccgaccgcgaacagaccgggcgtgttgaagcgcatcttgcccgccgccagggtggcgatccaggcgaacacctgcacccccgccgggatgctgacggccatggaagcggccgagaaatagttgatgctgatctgcggcatgcccgtcgcgaacatgtggtgcgaccagacgccgaaggagatgaagcccgtcgccagcatggccagcaccaccagccggtagccgaccagcttcgtctgggccaccgccgggatgatggtcgacatggcgcccgcggccggcaggaagatgatgtagacctcggggtggccgaagaaccagaacagatgctgccacagcatcgggtccccgcctttgatggcgtcgaagaagggccagcccagcgcccgctcgagctccagcagcagggtcgacaggatcaccgacggaaaggcgatgatgatcatcaccgcgaagatcagcatggcccaggcgaagatcggcagcttgtccagcgtcatgcccggcgcgcgcgtcttcagcacgccgacgatgatctcgatggcgccggcgatggccgagatctcgataaagccgatgcccaaaagccagaagtcggcgttgatgcccggcgaataggtcgtgttggtcagcggcggatacatgaaccagccgccgttcggcgccaggcccacgaagatcgagcagaagaacgccagtccccccaccagataggcccagaaggcataggcgctgaggcgcggaaacggcaggtcgcgcgcgcccagcatctgcggcagcagcagcacgcccagcgcctcgaccgccggcaccgcgaacaggaacatcatcaccgtgccgtgcatggtgaatatctggttgtaggtctcctgcgccaggaagcctgtcatcggcagagccagctgcgtgcgcatcagcaccgccagcactcccgccaggatgaagaacagcatggccgcgccgacatagtagacgccgatgaagttgttgttgatggcggtcagccactcccagccggagcgcggcccgcaccaggtttcttccagctgctccagctcgccttcagggcggtcctccggcgtcgggaagcggtcgtagagcttggggtcccagccggtctccgaactcattggaggctgtccagataggcggaaacgtcacgcaggtcggcgccggtcagcaccggatacgacggcatgcggttgccgggcttgatgccctggctgtcggagatccagccggcgagcgtgccctgattgttcggcaggatgcccgcgccgaggctctggcgcgcgccgacgtgggtcaggtctggcccggccagaccattgtattcggttccgcgcacggtgtggcaggcgccgcagccgttggcgtcgaacaccgcctgtcccctggcgagttgcggcatggcgggcgcgacggcgggtcccgcctgtttggctcgccactgcgcataggccgccggttcatgcgccacgacgacaaagcccatcagggcgtgcgggccgccgcagtattcggcgcattggccgccgaatacgcccgcctcgtcggcctgcagccgcatgaagttgcgccgaccgggaatcatgtcggtcttgccgcccagacgcggcacccagaagctgtggatcacgtcggcgctttccagctcaaacaccaccggctggccaacggggatgtgcacctcgttggcgtcctggatcacctcgcggccttggtcgtccagataggcgacgcgccaccaccacatctcgccagtgacgcgcacccgcatctcgccgggctggggctcggccgcgaccctggcgctgacgttcaggccgtagatcagcaggccggtcagcacgaccacgggaaacgccaggccgccgatccagacgatccgctcgccgcccacgcgcctgcgccactcgcgtggaccgaacagggcgacgcccagcgcgatcagcacgatcgtcagcacgacggcgcccatgatgaacagcacccaggacacgacctcgatcggccccgcgaacgggccggcgggatcgagcacgggcgggggccatccggacaggccgggcgcggtctcagtcttcatcgagcgtgtacagataggccgcaacgtcgcgggcttggtcttgcgtcaagggcatcggcggcattccggtcgagggatcaagcgatggcgcattgatgatccactgcaccaatacgtccggctggttcggcaggcgacccgagatcagggggcgggcgccgaaaccgcccagcgatccgccgcttcggccctcgggccagccgacgcccggcacaacatggcacgccgcgcagccgacccgctcgacgatgcgcaggccctcggtcgcatccgcgcctacgatctggcgcggggcgttggccttgtccgcacaggcgcacagcaaggcgagcggaagcgccgcgagcacgcctcgcctcacgtcctgcactcgacgactgaatgggcgcgtcgcatctctcccccaagcttgacctttgaaaagccccggctcggctgcggttccaccctgcggcgcgacgccacgccgaatctcgacagggaacctctgccgtaagccgtcgttcgccccttgtgcgcctgctcctgcctctcttcaccgcccccttgttgctcgccgcctgcgacactacgccgggcgagacggaccgcgccttttcggcgaccggagaggtgatcgcgctgagcggcgggccgggcggcgccaaaaacgcctgtttcacctgtcacggcatgcagggccagggcgacggggtgtcggcgccgcgcctggcggggctggatcagggctatctgcagaaacagatggaggactacgtttccggactgcgtccacatgaccagatgaccgccgtctccaaggcgctggatcatcgcagccgcaaggccgtggcggcctactatgcggccatgccgatcccggcggaggtcacgtccgacacggccggcgcgccgccgccgatctatctgatgggcgacgcctcgcgcggaatcacggcctgcgcatcctgccacggtcagaacggcgaagggggcggggcgggcaatccgcagatcgccggccagcccgccacctatacggttgagcagatccggctctggcaaaagggcgaccggcgcaacgatgcgcggggcgtcatgcaggcggcggtgcagaggctttcggacgaagaaacaaccgccatagccgtttggctgtcgcggaaacccgcttctccagcgcgcggtagcgccgctgccagcgcgtccgccggggtcgaagctgcggcacgaccggcagcatcgcgtgaaacacgtcgtccctatcgatcagatggtgcttcagggcggcgcccgcatgaatcgggatcatcagaagcaaggtgatgatcagcccccagtgcatccactctgccgcggcctctacggcccacaactgggtgttggacaggttctggaatggcagcaggggccaggggatgaagccgccggcggtaagttcctgatcgcgcgccgtcgctgaaatcatagcccagccgctgagcggcagaccgaacagacaggtgtagaagacatagtgagtgatgtgggccgccgtgctctcccagcccggcttgtcggcgtcattgatcaggttgggggccatcaacctccacgacaaccgaccgatcaccaggatcagcatcagcacgccgaccgcgaaatggacgtcataggccgcgaccatgccgccgcccacgccttggcgcacccgcgccatccacaggccccatcccagctgaaagaacaccatggccgccatggtccagtggaaccagatgccgatgggcgagtagcggccctcgtcgtggtggcccgccgcccattccagcagctggcgaaatagcttctcgatcatgcggcggcgccctcggcaggcgggctcagcatgcgcccgagacgccacagcgcggcgaacaaatacagcgccgccgccggcgcccacatgatcaggccggcgttctgctgatcctccagtggcgtcaggccgtagagcatcgtggcgccgaaatgcggcgcatagatcggcgtgcccgcgaacgtcagcagcgcgcccagcagccccatcagcagcatggccgccaacagcgcgatcaccgccgccggcgcgctcgccgcccgcgccgcggcccagaaccacacgcccgagccgatgatgctgagctgcatcagccagtagacgccgtcgctggacagggcggcctcataggcctggggcgcatgccaggcccagaacaccgccgcctgcaccgccgtcgccgccgccagcgacccggtgcgggccttgggaagggccagggcgatcagcggcgccgccacggcgatcagcagcacgtggtgcacggtccgcgccgagaacagcgccgaactgagcgcgcacaggggcgaaacaaagccgatggcgagaaccgccaacgccagaacggccgcgcgacgttcaagagggccctttcgccacgtccacaaggcgacaaagctcgccgccagcgccgcaagcagccagggatccaggttccagttgcgcgccagaaccgacggatcgggcgcttggccgcaatagggcgtccagatgacgtcggcgttcatacgatcccctgccttgcgcccgagacggcgccttccgtcgtcaacgcgccagacccgaagcggttgagcccaaccttcaccgtgcggctcagggtcgcgcgatcgatgtcacaccacctgccgcttggccagctttcgggccagggtgcgccggtgcatgccgaggcgccgcgcggtctcggagatgttgaagccggtgtccgccagggtctcgtggatgcgctcccactccagcgtcttgatggaggtgggccgggcgcccaccggcgtgtcggtggcgccctccgagcggccaaaggcggcctcgatgtcgtcggtggaggcgggcttggccagatagtgcgaggcgcccagcttgatcgcctccaccgccgtggcgatgctggcgaagccggtcaggaccacgatcaccgtcgtctcgtcgtgcgcgtgcagggtttggatgcacgacaggcccgacgcgccgcccagcttcaggtccaccaccgcatgggtgggcgtcgcggtcttcagcacctcgaccagaccgtcgtggctctgcgccgtcagcacgcggtagccgcgtcgctccagcgaacgcttcagcgtcttggcgaagacctcgtcgtcctcgaccagcaccaggaggcggtcggcctcggtcatccgatcctgtccggcaggaccagggccgccagcggcagccgcagcgtcacggccgcgccgcccccgggccggttgctcgcggaggcttcgccgcccagctttcgcagcacattgaccagcaaaaacaggccaaggcctgcgccgtgcctggccttggtcgattgatagggctggccgaagcgggccaggatgtcggggctgaagccggagccgtcgtcggtcacggtgatgatcaggacctcctccgcagtttcggccaggacgtcgatccgttttgcgccggcttccaccgcattgtcgaggacgttgaccagcacctgctgcagcgccgtgtccgagaccgcggggcgatcctcgcccagccgctgctggtattgcagatcgatgccctgggccgagcgccaggtcgcgaccatgtcgccgaccagggcgtgcagggtggtgaccgccggcgcttcccccctcgcctctccggccgagagcaggatgccggtgacgatcttcttgcagcgctcgacctcggcctgcatgccggccagatcctcgatcagttccggatcacggttgatggcgggcgtgcgccgccagtcggacaggatgaccgatagcgaggccaggggcgttcccagttcgtgcgcggcgccggacgcgagcaggcccatgcgcacgatgtgatcctcttccgccgcacgctggcgcatctcggccagataggcgtcccgggcgcgcagatttccgctgatgcgcgtgacgaacatcaccagcagcaccgcgatcagaccgaagcagaccagtccgcccttgatgtagagttcgaagtcgtgacccagcagccccggcggcaggagcatgggccggtaggtcatgctgagcatcagggcgcacagactggtcacggccaccagcgcccaggtcaggatcggccccagcaggaccgcgcccagcaccacctgcaacaggaacagcgacatgaagggattggtcgcgccgccgctgaggtaaagcagccaggtcagggccgcgacatcggccatcagggcgacgaacagctcgatgcccgacacattggcgctgaagcggatgcgcgccatgctgagcagattgaccccgatcagggccgccggggccgccagcatcagcagaagcggcaggcgcacctccagcacccactcgaccgcatagatggccagcacctggcccgccaccgccagccagcgcagctggatcaacagctgcatgttgcgtccgcccgcggccgaggcggcgtcggcgctcagcggcggccagcggcgcagcgcgccaagcgcggcgggccgggtcacgtcgcgtcggagccttttccgcgtctgcgctcgcgcagcaccaggcccatgccggccagcgacagcaacgccatcccgaaccaggtcagggcgtagaccaggtggctgttgggaaagcggatcaccgtcagccctccgcgcggccaggcgcccggatcagacgccgcatccgcgtcgatgaagtacggagcaacgtcggcgagaccgcgcgcacgggcgatggcctccacatcgcgcgagcgccagcggttgctggcgggatcgttggcgcggaggaagccgccattgggctcggtgacgcgcaggagccccgtcaccgtctgctcgccgccgccgccggcgccggcgcgcagggcggggtcgcgacgctcaggcggaacaaagccccggttgatcaggacggtgaacccttgatccgtccgcagcggcgtcatcacccagtagccggcgcccagggccgtcgcggcctggctcagggtctcgcggtcgtgcagaaacacgccgtgcacctgcacccgccgatactgatcgcgcgcggccgacacctgcggccactccgaaggaccgggcggcgcaacggcggccgcatgcacgcgcgcatcgacctgggcgatcaggtccagcttccagacccgccgctcgagctgccagacgccgagggcgacgaaacccgcggcggccagcgcgagaagccccagcagcaacaccgagccgaacggctggcgcggcctgcgccgctgggccgccggctcagacgggtcggcggggttcagggcgccgcgctcatggccgcctcgacatggcccggcatcatgttggtgtcgaggtggtacatgacccacagggtgcccacgagcgagatcaccacgatgatcagggtgaagatcaccgccagcatgacccagccgccctcggacttggagttcatgtgcaggaagaagatcacgtggaccaccatctgcaccgccgccagggcgacgatgatcaggcccgtcgcctggaacggcagggcgccggtcatcaccagccagaacggaatggccgtcagcaccaccgaaaggccgaagccgatcagatagcccttcatcgagccgtggttgtggccttcgtgacccaggtgatcggcgtcgtgcgagtcggcgctgtgatcgtcggtgcggtcgtcgccggtgatcggcggatgcgcgctcatcgcagcattcccatcagatagacaaaggtgaagacgccgatccagatcacgtccaggaagtgccagaacagggaaaggcacatcaggcgccgctggttggcctcgatcaggcccttcatcgacacctgcaccatcagcacgaccagccagatgatgccaaaggtgacgtgcaggccgtgggtgccgaccaggataaagaaggccgagaggaagccggaccgctggggcgtggcgccctcatggatcaggtgggcgaactcatacagttcgatgcccaggaaggcggcgccgaacaggccggtgatcgccagccacatcagcgtctggcccttggccttgcggtccatggccagcatggcgaagccgtaggtgatcgacgagaacagcagcatggcggtgttgatcgccaccaggttcaggtcgaacaggtcctgcggccccgggccggcggcgtagttgcccccgatcaccccatacaccgcgaacagcatcgcgaagatgaggcagtcgctcatcaggtacatccagaagcccagcatggtgctggacccctcggcgtggtgcggctcttccttcaggtagaagaccggctcttcggcctcagaagcgcccgtgggggcgtcggccgtggcgacattggtgctcatcggttcagccctccctcagccctgcgccgccagggcgcgggcgcgcgcctcggtttcggtgacttccgacgcgggaatgtggaagtcgcggttgtagttgaaggtgtggaagatggcgtaggcgacgatgccgacgaacgacagcacggccagccaccacatgtaccagatcaggccgatcgcgcaggccacggccatcaccgacaggatcacgccggcgccggtgttccggggcatgtggatgtcgcgatagccgccctccggcgccttgtagccgcggtgcttcatgtcccaccaggcgtcgccgtcgtggatcaccggcgtgaaggcgaagttgtagtccggcggcggcgacgacgtggaccactccagcgttcgcccgccccacggatcgcctgtgaagtcgcgcagcttgtcgcgattgatgatgctgacggcgaactggatcaacatggccaggatgcctatggcgataatggccgcgccgacgcctgcgatcacgaaccagatctgcagcgacggatcgtcgaacacccgcatgcggcgcgtcacacccatcaggcccagcacatagagcggcgcgaacgccacccagaagccgaccacccagcaccagaagctgaccagaccccacttgcgatccagcttgaagccgaaggccttgggccaccagtagttgatggccgcgaagatgccgaacagcacgccgccgatgatgacgttgtggaagtgagcgatcaggaacagcgagttgtgcaggacgaagtcggcgggcggaacggccagcagcacgcccgtcatgccgccgatcacgaacgtcagcatgaaggcgatcagccacatcatcggcagctcgaaccggatgcggccgcgatacatggtgaacagccagttgaagatcttcgctcccgtcgggatcgagatgatcatggtggtgatgccaaagaagctgttcaccgaggcgcccgagcccatggtgaagaagtggtgcagccacaccaggtaggaaagcaccgtgatgaccacggtggcgtagaccatggaggtgtagccgaacagcttcttgcccgagaaggtcgaggcgacctccgagaagacgccgaacagcggcaggatcaggatgtagacctcggggtggccccagatccagatcaggttcacgtacatcatcgggttgccgccgagatcgttcgtgaagaagttggtgccgatgtagcggtcggcgcccaggagggccagcaccgcggtcagcaccgggaaggcggcgacgatcagcacgttggcgcacagcgaggtccaggtgaagatcggcatcttcatcaggctcatgcccggcgcgcgcatcttgatgatggtcgcgatcaggttgatccccgacagggtggtgccgacgcccgcgacctgcagcgcccagatgtagtagtcgaccccgacatcgggactgtagccgatgccggacagcggcggataggctagccacccggtgcgcgcgaactcgcccacgaacagcgacatcatcacgatgatcgcgccgcccgccgtcatccagaagctgaagttgttcaggaacggaaaggacacgtctcgcgcgccgatctgcagcggcacgatgtagttcatcaggccggtgatcatgggcatggccacaaagaagatcatgatcacgccgtgggcggtgaacacctgatcgtagtggtgcgcgttgaggtagccctcggacccgccaaacgccatcgactgctgcaggcgcatcatgatggcgtcggcgaagccacgcaggaacatgatcagacccaggatcatgtacatgatcccgatcttcttgtggtccaccgtagtgaaccactccttccagagatagccccacagcttgaagtaggtcacggcgccgagcagggcgacgccgcccagcaccaccacgataaaggtcgcggcgatgatcggctcgtggaacggcagcgactcgagactgagccggccgaagatgaactgcgcgatggtgtcagcggacattggagacagtcggtccgatcaggattggcccgcgcccgccggagcggtcgcgcggaacagggaaacggaaggcggggtcaggcccgcgccggtcaggggcccggtctgggcgagcgtcagtgcgcgcggctgcacgccggcctcggcgtccacgccttcgaccggatcgcacagcgacgccagatagctgggctggtcgccgaacaccgcgccacgccggccatgcttgtcgtaggtcagcggcagggtcatgcgggcgctttcgatgcccaggccgcccttgtcgtccagcgccatcatctcgtgcatgcacatcttgccgggctcgacgcacatgccgacgacggcgttgaacaggcccggctccaccgagccgaacagcatcacgggcgcgttctcgctgggtcgctccagctgcagatagccggcgcggtcaagcgagccgccgctggcgcgcacgcgggacacccagctgtcgaagccggcgggctccagaccgtggaagtcgaaacgcatgcccgagaagcccgagcccgagtagttggcggagaggcccttgtactcgcccgggcggttgatcaccgcgtgcagcgtcgtctgcatgcccggcatggcgtagatctgccccgccagcgccggaacgtagaacgagttcatcaccgtcgacgaggtgatgctgaactggatcgggcgatccaccggcgcggccagttcgttgacggtggcgatgccgtattccgggtagatgaacagccacttccaatccaaggccaccacattgacctgcagcgggcgcaccgcctcaggcgtcgggcggcccggctcgatccggtcaagcggacgataggggtccagcaggtgggtgccggcccaggtcagggcgcccaaggcgatgatgatcaacagcggcgcgccccagatcgccacttccagatgcgtggagtggtcccaatccgggcggtagtcggcgtccttgttcgactgacggtacttccaggcgaagaacacgatcatcaccatcacagggatgatgatcagcagcatcaacaacgtcgatatgaccaagaggtcgcgctgctgagcggccacgtcgcccgagggcgcgagcaccaccgcattgcacgcggacagcagcgcaaacgctggcagaaggatcagcggcttaaggcgccgcagggcggttccgagggaggagttcggcatggtggcggcgccataatgggttcttcgcagcaacgacattggacaatctgccctatctcttttctggacgtttggccgcatcaggcgctttcatacatacaccaccccggcgcgcgcgtccgcgcgcctcatgacgaaaacggagcggtcatcccatgagcgccacaacgggatcggcgtcctcgacgtcgctcgatcgcgacgccaagcagatcaacgcccgccacggcaaggtggacgccggcgagatcgccatcggcgtgatcatcggccgggcgtcggagttcttcgacttctttgtctacgccatcgcctcggtgctggtgtttccggcgctgatctttccgttcgcgggcccgcttatgggcacgctgtactcgttcgccatcttcgcgctggcctttgtggcgcgcccgatcggcacggtgatcttcatctggatcgacgaggcgtttgggcgcggggccaagctgacgatcgccctgctgctgctgggaatctccaccgtggcggtggccttcctgcccagctatgcgacgctcggcggctggtcgatcatcctgctggcgatcttccgcatcggccagggcatcgccctgggcggcacctgggaggggctggcttcgcttctggcgctgaacgcgcccgaagaccgcaagggctggtgggccatgatcggccagatcggcgcgcccatcggtctgatcgtcgcctccgccctgttcgcctatttcgtgtcgctgctgtcgcaggccgacttcctcagttggggctggcgctatccgttctttgtggccttcgccatcaatgtggtggcgctgttcgcccggctgcgaatctcggccacgccggcctttatcgagtcgtttgaaagccgcgaactgcagccgacgcccgtgctgcgcacggtgcgggcggaagggcgcaacatcgtcatcggcgccttcgcgccgctggccagctttgcgctgttccacatggtgacggtgttcccgctgtcctatgtcctgctctacaccgacgagccgcccgcccgctttctggtgatcgagctgatcggcgccgtggtctgcctgtttgcggtgatgctgtcgggcgtgctggcggaccgctacggtcgccgcaacctcctggccatcaccgccggcgcgatcgccgccttcagcggcttcgcccccaccctgctgtcgcagggcgaggtcggcggcgtgatcttcatgatggtcggctttgcgcttttggggctgtcgttcggccagtcgtccggcgccgtcgcctccaacttcacctcgacctaccgctacaccggctccgccctcacctcggacctggcctggcttttcggcgcgggcttcgcgccgctggtggcgctggctttgacgtcgcagttcggcctgttgtcggcgggcgcctatctgctgtccggcgcggccggcacgctgatcgcgctgtggatcaacaaggagatgggccggacccgccgggaggcggcgcgcgccgcccaagctcagccggaataactgcgatcccgctttgaaagacgaaaggccgccgcgaacctcgcggcggcctttttcttgcactctgaaccgaccgcccagccggcctagtccgcgccgatctccatccagatcgaaagagtgcggcccggctccagcacgaccagtccgctgtcgctgctgcggcgggcgtgaaccgcgtccggccggtgcgtcaccggttcgatgcagcagaacgcccgaccctcgggcgcatagacctgagcccagcgcgcgttgggcgaggcgtccagccggaccgctccctcaccgctcgacagctccgcctcgccgttccagccgccgtagcagtgatccacagccggggcgtccgccactctcggattggccgaccagtcgaacacggccgaaggcggccccactcgcgcggggatgtcgcggtcgtccagcagccacaccgcgtctgtgtccagccgcagccgcgtctgttcgtcctttgggaaacagggatgaagccccagtccggcgggcatgggcgcgtcgtccagattgcagaccgacaggtcgatccgcaggccgcgttcggacaaggcgatggtctgcaccgcgcgatagcgccacggccaggcgtccggctcgtgatcgagcgccagcgtcgccgcgtcctccgcctgatcctgaagcgaccagacgctgagccacccctgaccatgcaaggcgtttggcgcaaaggcgtccagcacgggaagggagacgcggcgcccctcgaactcgaactcacccccggcgatgcggttggcgaacggaaccagcggaaagcacgccgtcagcagcgggtcggccgcgtcctggggcatcgggcgcaggatcgtgcggtcatcccgggtcagatgggtcagggcgccgccaagctcgggccgcacgcctgcgcgccagccgccggatcgaagatggatcatgcggcgactataggccttccgccgccgcaacgcgaagccgttcggcatgctcgcgcaggtttgcgacgcttcgacatttccgtcacccgccggagccaacgcctctccggctcgttcagaaggccctccccttagagacgtgcgcttgtgccgaatagacggttgaatctccttgtcgccgagagcgagcccggcgaagcgcgcgaccagcgccgcgaaagcgtcgggcgaagctcgggcgagacctacgaggccgttctggcgcacatcgcgcttggcgccgacatccagcgcatcaagcccgtcgacacgcccggcgagataccggacgccgccggcctcgccgacttcgacggcgtattcctgacgggctcacccctgcacctgtacaaggagacgccggagacgcgccgggtcgtggagttcatgagcgcggtctttgacgccggcgttcccgcctttggatcctgcgcgggactgcaggtcgccacggttgcggccggcggttcggtgcgcccgatgggcgaaaggcgcgaggccggcttcgcacgccgcatcttcccgaccgaggccggccgatcccatccgctgctgcggggccgcccgccggcctttgacgccccggcgatccacagcgacgaggtcgccgccctgcccgacggcgccttgcgtctcgcgtccaacgcgacgaccgaggtgcaggcggccgagatccgctgcggcgacggcgtcttctggggcgtccagtatcatccggagatctcgctgttcgaggccgcggccgccctgcggcgacaggcggacgatctggtccagcaggggctggcgacgtcggtggcggcggtcgaagaacaggcgcaactggtcgaggcgctgcacgacgcgccccagcgccgcgatctggcctggcggctgggcctcgaccctcaggtgaccgagcccgagcggcgctccgtcgagatccgcaacttcatcgaacacctcgtcctgccgacccgctccgggcgcggccgcggctgaggcgccggccggtcagcccccgacgatccggccggcctccatccgcaccctctcctcggcgatggcgtcgatgtcgcgcgggtcgtgggagaccaggatcatcggcgtgcggccttggtccctcaacctcagcagataggggatcagcgcggcgcggcgcccggcgtccagtccggtgaacggctcgtccagcagcagcagccgggggtccgagcacagggcgcgcgcgatggcgacccggcgcatctccccgcccgacagcgacgaaggccagcggcgttcgaacccctgcaagtccagcaactccagtatgggtcccatggcgagaggatcgcgggcgaagcggcgtccgaaggcgatgttgtctcccaccgacatatggggaaacaggcgcccatcctggaagacgtagccgattcttctccgatgcgacggcgggtccaatccgacgcgggtatcgaccaccggcgcatcgtccagcaccaggcgcagtcgactcggcgccagcagcccggcgagcgcgtgcagcagcgtggtcttgcccgcacccgacgggccgacaagcgccagcacctttcgctcggtccgaaacgccgcatcgacggtgaagccgtcgcgctcaaccaccacatggcattcaatgctcatgacgtctgacgcgccttgtgcagacgccggttgcaggcctcggccgcgaggatggccccaaccgccaccgccaccgagatcacggccagccgcaccgccgaggtttcgccctccgccctttgcagcgaggcgtagatggcgacgggcagggtctgggtctcgcccggaatcgatccggcgaaggtgacggtggccccgaactccccaaaggcgcgcgcaaagcccagaaaggcccccgccacgatccccggcgcggccagcggcagggtgatgtgggcgaacacccgccaggggggcgcgccgagcgtcgccgccgcctgctccaggcctcggtccacggcttcgaacgacagccggatcgggcgcaccaccagcggaatcgccatgacggcggcggccaaggccgcaccgagccaactgaaggccagggtcacgccgaaggtctcgcgcatccaggcgccgacaggcccctgggcgccgaacgccagcagcagcagcaggcccgtcaccaccggcggcagcaccagcggcaggttcaccaaggcctccagcagccacttgcccggaaagcgcccgcgcgccagcagccaggccagagccactcccagcggcgcggtgaccagcagcgaggcggcgccaacgcgcagcgaaagcagcagggcctcgacctcgaagggcgtgagcggcgcgaacacctcaatcgccgccgaggttcgccagccgccgcagcgccggcccggccgcggccgtcagcaccgtctccagatgctggaactcctgcaccaccgcctcgcccgtcgatgtcaggcgcgcgccgccgccgcccttcccgccctggctggtctccaccaggcgatggccaacggcccggctcgcctcgtccaccaactgccaggcgcggcgataggacaggcccgccttgcgcgcggcggccgacagggagccctcctcctgaaccgcacgcagcagccgaaccttgcccgggcctatcgcaccctgcggcccatccaggcgaaaccacagctgcagcggctgggcggtcaccgcgactggccgaagcccgcggcctcgaacgccgctcgagcttccggcccctccagatatgccatgaagtcgtcggcgccgggcttggcgtccttcagcagggcggccggatagacgatgcgcggctgctgctccggcggcggcgtcagcaccacgcgcacgccctgcgcgcccaccgcgtcgctgcggtagaccacgcccagcgccgcctcgccccgctccacgaaggtccgcgccgcgcgaacgtcggcggcggtgacgaggtgcggctgaaggccgtcccagcgcccgatcccctgcagccaggtgcgggcataggcgcccgccggcacgctttcgggatcgccgatcaccagcttgcggtccccgtccgacacccacgccagcggatcggcgacctgcggcgcatcggcgccgatcaccaccagggcgttggtcagaaggtccagccgcgtgccgggctgcacacgtccggcctcttccagccggtccatccacggctcgtcggccaggatcacgagatcggccggcgcacccgactgcacctgccgcgccaccgcgccgcttcctgcaaaggataggcgaaccgcctggccggtctcgcgttgataggacgcggccacgctttccagcgcgtccgtgagggaggcggcggcgaacacggtcagcggttcggtcggcgcctccggcttgggggagcaggcgaacagcaggacgccggcgaagacgcctagcagggcgcgtctctgagaggcgaaagaaatggctgggctcccggggacggatcgctatgttcaatccagcatgacggtggtgatctcctctgacaagccgcgcccgcgaagcttgggcgcttcgcctctgatcgacccgttcgggcgcgtgatcgactatctgcgggtgtcggtgacggaccgctgcgacctgcgctgcacctactgcatgctggagaagcagacctttcttccgcgcgccgagctcttgaccatcgaggagctggatcggctgtgctcgaccttcatcggcctgggcacgacgcggctgcgcctgacgggcggcgagccgttggtccgcaagggcttcatggacctggtcgcgggcctgtcgcggcacctgcaagcggggcggctgaaggagctgaccctgaccaccaacgggacccagctggcccgccatgccgaggcgctcgcccgctacggcgtgcggcgggtcaatgtgtcgatcgacacgctggaccccgacgactaccgccgcatcacgcgcggcggcgacctgggcggcgtgctgcaggggctggaggcggccaaggcggcggggctccgggtcaagatcaacgccgtggcgctgaaggacgacaacgccggacagctggccgacatgatcgcctgggcccacgcccgcgacatggagatgacgctgatcgagaccatgccgctgggcgagatcgaggccgaccgcactgaccagttcctgtcgctggcgcaggtgcgatccgagctggagcgtcgctggacgctgacgcctatggcgcggcgcacgggcggcccggcgcgctatgtccgtgtcgaagagaccggcggcgtgctcggcttcatcaccccgctcagccacaccttctgcgaggcctgcaaccgggtgagggtgacctgcaccgggacgctgttcctgtgcctggggcaggaggaacagaccgacctgcgctcggtgctgaggtccagcgacgacgacgccgcgctggaggccgccatccgcgaggcgatccgaagaaagcctcgtgggcacgacttcgacatctctcggcgcggggccgcgcccgccgtgtcccgtcccatgtcgatgacggggggctgaaatggccagggtgaccctgttcggcgcctttcaggacatggccggctggcgcacgcgcgaggtggacgccgggacgttgggggcgctgcgcgaggcgctgtcgaccgagcatgcgcctctgggcgaacggctggagcacgccagcaccctggtgatcctgaacggggcggtcgcgccccgcggacgccacgccgacgacacgcctttgtcgcctggcgacgaggtcgggtttggcccgccggtcagcgggggctgagcgcatgatccgcctcgccgatcggcccatctcggccggcgatctgctgaacgaattctgcgccggccgcaccgacgccggcgccgtggtcagcttcaccggcctgacgcggatgcagaccgccggcgccgccgtgtcgcgcctgacgctggacgcctaccccggtttcaccgagaccgtgatggcaggcatcgaagcggaggcgcgggcgcgcttcgacattcaggatgtgctggccgtgcaccgctggggcgcgctggaggtcggagaaccgatcatcttcgtggccgtggccgccgagcaccgccgagccgctttcgaggccgccgactatctgatggaccagttcaagactcgcgcccccttctggaaaaaggaggacggcccggacggcgcacgctggatcgacgcccgtccgcaggattatcaggacctcgcccgctggggcgacacggagaccgccgaatgacagacacgctcgccgacacgcccctgcccgcccccggcggccgactgatcgatgcgcccatcaagccggtgcggatcgcggtgttgacggtgtcggacacgcgcgacgaagagagcgacacctccggccagatcctgtccgagcgggtggtcgaggcgggccacgcctgcgccgcgcgcgctctcgtggccgacgaggtggaggcgatccgcgcccaagtgcgcgcctggacgacctcgggcgagatcgacgcggtgatcaccaccggcggcaccggcctgaccgggcgcgacgtgacgcccgaggccttggagcccctgttcgacaagcggatcgacggcttctcggtgatcttccacaccgtcagctatcagacggtcggcctgtcgacgctgcagtcacgggccacggcgggcctgatggatggcgtgttcgtcttctgcctgccgggctccaacggcgcggtgcgcgacggctgggacaaggtgatccgctggcaactcgacagccgccaccgcccctgcaacatggtcgagctgatgccgcgcctgaaggagcggtgatgggcgagctgacccacatcgacgccgacggccgcgcccgcatggtggacgtgtcggacaaggcggtcaccacgcgcgaggcgcgggccgaagggcggctggtcatgcgggcggagacgctagccctggccctgtccggcggcgggaaaaagggcgatgtgcgcgccgtggccgagatcgccggcgtgatggcggccaagcgcacggccgacctgatccccatgtgccatccgctgatgctgagctcggtcaaggtgacggtggagcctttagacgacggaagcggcctcctggtcacggcgacggtgcgcaccaccggcccgaccggggtggagatggaagccctgacggccgccagcgtttctcttttgacgctctacgacatgctgaaggcggtcgatcgcggcatgaccatcgaggcggtgcgcctgctggcgaagtccggcggcgcgtccggcgactgggtgcgggaatgaagctgccgacggtggaagcggcgctggccctgatgctggaggccgtgcgccccctgccgccgcaggacaccccgctggcgcaggccgacggccgatggctggtcgaggacgtcacggccactcgggaccagccgcccttcgacgcctcggccatggacggctgggcggtgcgcagcggcgacgtcgcgcccggggccgtgctcgacatcatgggcgagagcgccgcggggcacgcgctggacgcacggatcggccccggacagacggcccgcatctcgaccggcgccgccctgccgcccggcgcggaccgggtggtgatccaggaagaggcggaccgggaaggcgaccggatcgtgctgcgcgcctcggccgacggttcccgccacgttcgggcgcgcggctgcgacttccgtgaaggcgaggtgctgcttcgggcgggtctgcgcctgaacccctggcgcatcgcgcttgcggcctcggccggacgggcggtgctgcgctgcgggacggcgccccgcgtggcgatcctgtcgaccggcgacgaactggtcgagcccggtctgtcggcaggtccgcaccagatctacaactcgggcgcgccgtcgctgtccgccttcaccgcgcgccacgcgggcgccgctcatgtgctgccctcggccggagacgatgtcgacaccatcgcccacacgatcggagaggcggcgttcgacctgctggtcacggtgggcggggcgtcggtcggggaccatgatctggtcaagccggcggtgcgcggcctgggcggcgtactggcggtcgagggggtggccatgcggccgggcaagccggtgtggttcgcccttctgccggacggccgccctgtgctcggcctgccgggcaatccggcctcggccctggtcggggccgagctgttcctcgcgcctctgctggcggcgctgcagggcggccgggccgagaaccggttcgagacggcggtgctgggccaagctctggccgccaacgggccgcgcgaccactacatccgcgccgaggcgagccccggccccgacggcgcccgcatcgtgcgccccttcgcggatcaggactcctctctggtcaccgtgatggccgccgctaacgccctgatccgccgtcgtccgcacgcgcccgccgcggaggccggcgaggtggtggaggtgctgggaccgacgctctaggcgttaggcccgccgcgtcaggtcctcgggccgatccacgtcgaagacgacgccggggtcgtcagtgaacacccccgccacccgaggtccgagcgtggacagcagcgcgcgtgcgccctgatccgccgtgaggcaggccagagattcgaacatctcacgggcgaaggccaccggatgcgccggcccgtgcggcgagatcgtccgcgccgcgacgtgcgccccgtccaaggcgtccagcagctggtcggccagtttgtccgggatcgccggcatgtcgccgaggaagaccaccgccttcgccgcatcggccggcaggctgcgcacccccgcgctcagcgaggcgcccatgccttcgctccagttgggcgcggcgacgatcctgaggcgggaatcctcgagcgtcgcgaccgccgccgtcaccgccgccgcatccgaaccgacgaccagggtcaccgagtccacccgcgcggacagcgcccgccgcacggccgcgagcaccaggggttcgcctcgccagtcagccagcagcttgcgcccgccgaaacggcttcccgcgcccgccgccagaaccagcacgtggcgacccgtcatgaccgaagggcggcgatgatttcggctgtcaccgaggtggcgacttccgccggtgagcgagcgccgatcgccagcccgatcggcgccttgaggcgcgccagcaccgcttcaccgacgccgtccgcgcgcagccgctccaggcgctcgggcaatcgccggcgcgcgccgagcacgcccacatagccagcgtcggacaacagcgccgccttcagcaccgcgtgatccagttcgccctcatgcgtcgccgtagccaccgcggtccaggcgtctggcccgagacgctccagaaggatttccggcgcttcgcggctgtaggtcacggccagcggcggcggcgcctcgggtcccttcggccggcacagcaccaccgaccagccctgccagagtccggccgccgcgatcgccagggcgaaggcgtcgccgccgaacacgaccaatcgcctcggcggcgcatagagcttgcggcaagcgtcgggtcctgcatcccggtcgccgccgaaatgtctgcatcgcccgtttgagacatagacgcccggccgacggtcgctccaggcctcgcgcactgcgatcaacgccgcatcagccggctcaagccgctccaccagcagttccagccgcccgccgcagggcagtcgcgcgtccacgaacgggctgccccggccatagaccaggcggcgcggctcgccatcgacaaggcattcgcgcgcatgcagggccacgtccgcctcgatgcagccgccggacagaaagccgcccatgtcgtcggccgtgaccaccatctgtgcgcccacgccgcgcgggccgccgccctccgctgcgacaatggtgacgagagcgaagggccggccgcgacccgccgcctcaaacatgcgcgggcgcatgtcgtcttccatgccggccggataccagtcgctcatctgcgcaccaccgctccttcaccttcgtcgccggcgagcggccttgttcggacacggaacacgtccccgcgccgaccgttgccttaacgaccttttccccacggattaactcatgatcaccgcgcacaaaccggcgttgccctacgatcccgccgacgaggaactcgagaaggacgaggcggagaccactcgggaactgatcgaaaccatgcgcgacatccagcaaaaggtgctggacgacagcggccatgccgagcgcagcgtgcacgccaagagctatggcatcctgcagggcgaggtaaaggtcttcgacgaccttttgcccatgtatgcgcaagggatcttccggccgggcgcgacctatccggcggtgctgcgcatctcggccattcccggcgacatcctgcccgacgagattaccgcgccgcgggggctgtcgctaaagctgttcggggtcgagggcgcgcgcctcgaaggctcggaaggcgacacgacccaggacttcgtcatggtcaacggccatcacttccagacgcccaccgccaaggcgttcctggccaatctgaagttgctggagaagaccaccgaccgggtcgagggcgtcaagaaggcggcctcggtggtgaaccgcgcgctggagcaggtgctggaggcgttcggcggcgagagcgccaacctgaagggtctgggcggcgcgccgatgacccacccgttgggtgacagcttctacagccagtccgccttccgctacggcgaccatgtggccaagttcgcggtggcgccggtcgatcccgctctgatcgccctccacgacaaggccgtggacatcaggggccgcgacaacggctatcgcgagctggtgatggagcatatcgcggcgcatggcggcgagtgggacatccgcgtgcagcttcgcaccgatcgggacatgccgatcgaggacgcctccaaggagtggtcgcaggacgacagcccctacgttccggtcgcccggatcaccgtcaagccgcagcccggctggtcggaagcgcgctccaggaccgtggacgacggctatgcgttcagcgtctggcacggcgtcgaggcgcaccggccgctgggtcgcatcaaccgcgtgcgcaaggacaactacaaggcggcggccgaattccgcggacgcgccaacggctgcccgatgcacgagccccggtcgtggcagggcctgcccggctgatccacaacccagcaggcagacaggaaagccgccggattgctccggcggctttcttcatgttcaggccgcttccgttcggctctgcatggccgagcggctgaggcgcaccggcaccgccttgtaggccggcgtgtgcgcctgcttgtcgtggtgcgccagcggcaccaatgggttggcctcggggaagtaggcgccgatgcagccttgcgggatgttgtagggcacgatgcggaagccctcgatcatccgcgtcacgccgtcgtcgatggccgtggtcaggtccacgaactcgtccttggcgaagctcaatcgggcgatgtccgcctcgttcatgaacaccaccatgcgcgtgcccttcacgccccggaagcggtcgtcgtagccatagacggtggtgttgaactggtcgttggagcgcagcgtcataagctgcagcacgtcggccttgccgaagctgtcgacatcgcccgcgaacatctgtgtgggcacaatgaagttggccttgcccgtgcgggtgttccacttgcgctcgcgcgccgccagcggtcgcgccacgccgcccggatcgaacagcttctcgctgaagttcgggaaggtggcgggccaggtcttctcgatcgcctggcgcaccagcccgtagtcgccgacccactcgtcccaggggacgcgggcgttcggctccagcgtcgccttggcgatgccggcgacgatggcgggttcggagcgcagatgggggctggccggtttcacgtgtccgcgcgagccgtgatagtgcgccaggctgctttccatcgacaccgcctgacggccggtcgcctgctcgtcgatctcgatacgccccaggcacggcagcacgtaggcgacctgtccgtgcaccacatggctgcggttcagcttggtggcgatggagacggtcaggcgcagcttcttccaggcctcctccaccgcacgcatctcgggcgccgcgcggatgaagttgccgcccagcgccacgaacgccttgacctcgcccgtgatcatcttctcgcaggccgtgacggtggtggtcccctcatgccgcggcggctcgaaaccgtacatgtccttgagcacgtccagcggggccagttccggcttttcggtgatccccaccgtgcgctggccctgcacgttggagtggccccgaaccggacagattccggtgcccgccttgccgatgttgccgcgcagcagcagcaggttgaccaccatctgcacgttctgaacccccgccacatgctgggtcaggcccatgccgtagatgcccatgcagcggtcggccttggcgtagtcgcgcgccacgccctccagcgccgcgcgcgtcagccccgacacccgctcgatctcggcccagtccgccgcgcggcagtagtcggcgaacgcctcgaagccgtgggtgtgttcccggatgaagtcgtggtccagcaccttgcggttctgcttgttcgccgccgccgccttgatcgagaagccgccgtcgtcctccgtctgcgccagcagggcctcgcggtcggtggcgtgcgcctcgcccttggccgcctcggcgtcgtccatggcgatcagcgccttgcacacgccggtcagggccgcgatgtcgccgccggcccgcacctggtggatctgcgaggcgatctgcgtctcgcccagggtcagcatctgcttggggttctgcggatcggtgaagcgctccagcccccgttcgcgcaaggggttgaagccgatgatgctggccccgcgatccaccgcatccttcagctggtgcaggatgcgcggcgcggacgtgcccggattgtgggcgatgtagagcatcaggtcggtctgctcgaagtcctgcagcgtcaccgtgccgacggacaccccgatgctctcgggcaaggccacagaggtcgattcgtggcacatgttggagctgtcgggcaggttgttggtcccgtacatgcgcgccatcagctgccacatgtagctggtctcaagcgacgcccggccgctgacgtagaagacggtctggtcgggatcgccgcccagcgcccgcaactcgctcccgatctcctcgaaggcgctttcccacgagaccttttcgtacttgtcggtttcggggttccaccgcatcgggtgggtcagccgccccgcctcctccagattgtagtcgagccaggtctcaagctccgacagggtgtgcttgtcgaagaaggcctcgtcggcgcggtgcttggtggtctcccaggcggtggccttgatgccgttctcgcagacctccagcgggtggggcttggcgggcttgccccaggcgcaggacacgcacatgaagccgtcggccttgttctgatgcagcatcgtctccgagccgctgaccggcagctgctcccgcatcagtatctcggcgacggatttcgccgagccatagccgccggatggtcccctgtacggcttgatggtgggggtcttgctgggtgcggtcatgcggcagggctcctgcgagggtccggatagaacaggccgggcctttcgaggatgcaagcctgtcgcccgttttcttcgccgccctcgcccgcttctccctcgcggcctaagatggcggtatgagctccgccgccgaagaagacgccaaagccgcacctgcgctccgctggtgtcaggacacgccccggcgtcgctggagccaggccggcgtcgagaacggggaacggcgactcgcggaggaaaccgccatcgccattgtgcacgacgcctccaccaccgccgtgctgatggcgaccccccacgacatcgaggatctggcgctgggcttcagtctgaccgaaggcgtcatcgacagcctggaccaggtgcgcggcctggaggtggcgcagtcgaatctcggtgttgaggcgcggctatggttgacgccggatcgcgccgaacgtctggccgcgcgccgtcgtcgtgtcgccgggccgaccggctgcggtctttgcggcgtcgacagccttggcgaggcggtgcgcccgccgcctcgcgtcacgcaggcgttgcgggtcacgcccgacgggttgctcgcggccatggaggcgctgtcgggtgcccaggcgctcggacgcgacacccgcgcggcccacgccgccggcttctggacgcccgccgacggcctcgtcgccgcacgagaggacgtcggccgccacaatgcgctggacaagcttgcgggcgccctcgcccggatggatgcgccggccgccggggtcgtgctgctgacaagccgcgtttcggtggagatggtgcagaagaccgccgccatcggcgcgccgatcctgtgcgcggtctcggcccctacggcgctggcggtgcgcaccgccgaggaggcgggcgtgaccctggtcgccgtggctcgccgagacgggttcgaggtgttcacgggcgcacacaggatctccggatgatcgtcggtctactgctggcgggcggccgatccagccgcttcggctcggaaaaggcggtgtttgagttcggcgccggcctgatgatggacggtcctctctccgcgctcgacgctgtctgcgccgcgatcgcagtctcggctcgccccggttcaggcgccgagacgcaggcgaggatgcggggcctgccctgcctccacgaccggcccggagacccggaggggccgctagccggccttcgcgtcggcttggactgggccgcggctcagggcgcggcatggctgatgaccgcgccctgcgacagccccggcatcacgaccgcctatgcgcgcgaccttgcgggttcggcttcaagcacaggcttggccgccatcgccctttcgccgcgcggaccggaacctcttcttgcggtctggcccgtgtcactctctcaggagcggatttcagtggagttagacgccggtcagcatcctcccgtccgcgcgattttggaggctttgggtgcgcgccccttcgccggctacgacggcttgaacgtcaatacgcctgcggaccttactggcgtctgacatccggaggtctcgaagttgagcaaccacaacgttgaggtcggcgccgacccatgtgggctctagacgcacgaaagccccgctttttggggcggggctttcatgtttgtcgagtttgggtgcgggagcaggatttgaacctgcgaccttcaggttatgagcctgacgagctaccgggctgctccatcccgcggcgaacggaggggcgtgagggaagaacggttcgagcgggtcccgccctcaagcaggccgaaggccgatagggcaaggattgtgtttgtcatattcggctgtccgccttgtagacccggcggcgacctactctcccgcgccttgagacgaagtaccattggctctggagggcttaacgaccgagttcggaatgggatcgggtggggaacctccgacatagccaccgggtcaacgaggcggacagcggaatatgagaagacattgtctgcgatcgttctggtctgaacgatcatcgaatgagttttgctgagaaacgatcaaaccgatcggattattagtaccagtaagcttcacgcgtcgccgcgcttccacacctggcctatcaacgtggtagtcttccacgatcctcagcgaagccttgttttgaggttagtttcccgcttagatgctttcagcggttatctattccatacttagctaccctgctgcacagctggcgccatgacaggtccaccagaggtatgtccatcccggtcctctcgtactagggacagatcctctcaagcttcgaacacccacggcagatagggaccaaactgtctcacgacgttctgaacccagctcacgtaccactttaaatggcgaacagccatacccttgggacctgctccagccccaggatgtgatgagccgacatcgaggtgccaaactttgccgtcgatatggactcttgggcaaaatcagcctgttatccctagagtaccttttatccgttgagcgatggcccttccacgcgggaccaccggatcactatggccgactttcgtctctgctcgacttgtcagtctcgcagtcaggcgagcttatgccattgcactcgacgagcgatttccgaccgctctgagctcaccatcgcgcgcctccgttacactttgggaggcgaccgccccagtcaaactacccaccacgccatgtcccgggaccggataacggccctcggttagacgtcaacgacagtaagggtggtatttcaaggatgactccaccagagctggcgccccggcttcatagtctcccacctatcctacacatacggtcgctaacgccaaggcgaagctatagtaaaggttcatagggtctttccgtctgaccgcgggaaccccgcatcttcacggggaattcaatttcactgagcctatgctggagacagtggggaagtcgttacgccattcgtgcaggtcggaacttacccgacaaggaatttcgctaccttaggaccgttatagttacggccgccgtttacctgggcttcagttcgacgctttcacatctccctttaaccttcaggcaccgggcaggcgtcagaccctatacgtcgcattgctgcttcgcagagccctgtgtttttgctaaacagtcgctaccccctggcttgtgccactcagtcctgcttgcgcagggtgagtcacgcttattccgaagttacgcgtgcaatttgccgagttccttcagcatagttctctcaaacgccttggtatgctctacctgaccacctgtgtcggtttcgggtacggtctctgctggagttatttccagggacaacgcccccgcacgcacaatccaataagtgcgtacgagttatgccatccgtcacttccagctggtgcaggaatatttacctgcttcccatcgactacgcttttcagcctcgccttaggggccgactaaccctgcgcagattagctttacgcaggaacccttggtctttcggcgggagtgtctctcacactcctatcgttactcatgtcagcattctcacttccgatacctccagccaggctcacgcctgaccttcactggcttacggaacgctccgctaccgcttgcagtaaactgcaaacccatatcttcggcgcacggcttgagccccgttacattttccgcgcaggatcgcttgatcagtgagctgttacgctttctttaaaggatggctgcttctaagccaacctcctgattgtcaaagcaatcccacatcgtttcccacttagccgtgacttgggggccttagatgatggttagggttgtttcccttttcacgacggacgttagcacccgccgtgtgtctgcccgatagttctcttgggtattcggagtttggttagtattggtaccgctcgcgcagcccgcaaccatccagtgctctaccccccaaggaattcgtcggacgctctacctaaatagatttcgcggagaaccagctatgtccaggtttgattggcctttcacccctatccacaagtcatccgaggctttttcaacagtcaccggttcggacctccagttggtgttacccaaccttcatcctgctcatggatagatcacctggtttcgggtcgtcatacgtcgaacttagcgccctattcagactcgctttcgctgcgcctacacctaacggcttaagcttgctcgacacatgaagtcgctgacccattatacaaaaggtacgccgtcaccgcgcttggcggctccgactgcttgtaggcttccgatttcaggatctgtttcactccccttgtcggggtgcttttcacctttccctcacggtacttgttcactatcggtcgtagaggagtacttaggcttggagggtggtccccccatgttcagacaggatttcacgtgtcccgccctactcgagtcttctgctgtttgacggctacggggctgtcacccgctatggccgacctttccaggtcgttcgcctttatgtcacagaagcactggcctggtcccggttcgctcgccactactacgggagtctcggttgatgtcctttcctccgggtactgagatgtttcagttccccgggttcgcttaatgatgcctatgtattcagctcattatacctttcaacaatccgccaatcgccgtccccgaaggaacagagttggaagactgtaaaggtgggtttccccattcggaaataaccggatcaaagggtgctagcgcctccccggttcttatcgcagcttgccacgtccttcatcgcctctctacgccaaggcatccgtcagaagcccttcaacgtttgatcgtttctcagcaaaactcatgcgtggtttattccacccgactggaaagatgccgggggaccacgcctgattttgtcagacaatgtcttcttctcgaacagtgacctagaagctcaggggagccggtcgcgttcttccttcacgatttcaatgccggtcggcgagcgccgacaggcaatccttgatgcgatctgcgagccttggcggggtgcgccaccgctttcaaagcggggcctcgggtctattccccggccgcgggcgcggcctggtggagccagacggagtcgaaccgacgacatcctgcttgcaaagcaggcgctctaccaactgagctatggccccgttccagccggaacagtgcgaagcccaggagagctgtcggacgatctgcttaaaggctgaagtccagcccccggcttgccagaggtcctggtaggcccgggcagactcgaactgccgaccttacgcttatcaggcgtacgctctaaccacctgagctacgggcctatggcagcgacagccgggtgcgaaacccaggctcgcgatcgcgtcaccgtcgatcacaacccgtatggctgcgtcgatgatgacgaaagtggaaagagaaacggagacggcggcgttccgcatgatgtgctcggcgctgtgaagcgcttcgctatgcggagcgtcaatagaacctcgtgagaggcgctggagacgcatccttagaaaggaggtgatccagccgcaggttcccctacggctaccttgttacgacttcaccccagtcgctgaccctaccgtggtcgcctgcctccttgcggtcagcgcagcgccttcgggtagaaccaactcccatggtgtgacgggcggtgtgtacaaggcccgggaacgtattcaccgcggcatgctgatccgcgattactagcgattccaacttcatgccctcgagttgcagaggacaatccgaactgagacgacttttaaggattaaccctctgtagtcgccattgtagcacgtgtgtagcccaccctgtaagggccatgaggacttgacgtcatccccaccttcctccggcttagcaccggcagtcccattagagttcccaactgaatgatggcaactaatggcgagggttgcgctcgttgcgggacttaacccaacatctcacgacacgagctgacgacagccatgcagcacctgtgtcccagtccccgaagggaaagccagatctctctggcggtccgggcatgtcaaaaggtggtaaggttctgcgcgttgcttcgaattaaaccacatgctccaccgcttgtgcgggcccccgtcaattcctttgagttttaatcttgcgaccgtactccccaggcggattgcttaatgcgttagctgcgtcaccgaaatgcatgcatcccgacaactagcaatcatcgtttacggcgtggactaccagggtatctaatcctgtttgctccccacgctttcgagcctcagcgtcagtaatgagccagtgtgtcgccttcgccactggtgttcttccgaatatctacgaatttcacctctacactcggagttccacacacctctctcatactcaagacacccagtatcaaaggcaattccgaggttgagccccgggatttcacccctgacttaaatgtccgcctacgctccctttacgcccagtaattccgagcaacgctagcccccttcgtattaccgcggctgctggcacgaagttagccggggcttcttctccgggtaccgtcattatcgtccccggtgaaagaattttacaatcctaagaccttcatcattcacgcggcatggctgcgtcaggctttcgcccattgcgcaagattccccactgctgcctcccgtaggagtttgggccgtgtctcagtcccaatgtggctgatcatcctctcagaccagctactgatcgtcgccttggtgagccattacctcaaccaactagctaatcagacgcgggccgctctaaaggcgataaatctttcccccgaagggcacattcggtattagcacaagtttccctgagttattccgaacctaaaggcacgttcccacgtgttactcacccgtccgccactaaccccgaaaggttcgttcgacttgcatgtgttaggcctgccgccagcgttcgctctgagccaggatcaaactctcaggttgagttgacttctgacctaagcttaagaccaccaaaatggccttggcattagttctacgtattcttgacgagttcccacgtcatcgatcccaaaaaggaaccgacgcatggtatcttcaaaaagaccgcagatgtcagtgtcgattgacgttccgaagaacgtcgctagaacaccgccgcctgcgtttctctttccagatcaacgatttcaaagacccaggaaccgatctctcagtcccgccgtttatcgcccggctgcggcggaggcggcgatttagtcgcctcggtgatccgtgtcaagcggttctttttgcgaagaacctctttcaccaaccgacccgggaaactcccgaaaccggcggaggcggcgatctaccgaccctccaactccccgtcaagctgttctttttacaaaagaacctctctccgaagacccagcccgaagaccggaagaggcggcgatctacagacccccgatcccctcgtcaaccggcttttccaaaccgccgcaaaaccccggagacaaaccccgaaacccgcagaaaaccgcccccgaacccagccaaaaggccatgccccagacaaaacaaacaatagcgattccgtcgaagcgcgaaacctagtgggcgactatcaaaagatcaagagcgaaccgctccgaggcccttgatgtcgccgcccggtcccgagcgaggcggctctatacggagccgcctcgaccgccacaacctctttctcgcagaacagtgacgtttctttggcggacgcgtgaacgccttcagccgagccgcgtcagcctggccagcgggccaatcgccaggatgccaacaacaaagcccaccgcatgggcctcccaggcgatgcccgcgccgcccgcgcctggggcatagccgataagaccgaccacggcgttcactgccatccaggcgatcgccgcctggatcacgcggccatcgcttagcgccaatacctggccgcgcccgtccatcagccgcgtggccgcgccgatcaggccgaacaccgcgccggacgcaccgaccatcggctgggtcccgccccagtggatcagtccatatcccaacgccgccaacaccccgcatcctacatagaacagcagaaacagcgtcggcccccatcgcacgttcaagagacgcgcgaccggcgcgccgaacgccagggccgccaccgcgttcatgatgacgtgcgtccagccgccgtgcagcagcatggaggtcaggaggccgccataccgcccctgctgcagatcgacgggggcgaacgccatgccgagcccgccgtccggcaatcctagttgcaccatgaacagcagcggcatggacacggcgatcagcagcgccatgggcggggcgttgaacatgcgctcgcgcggccggtgcggatgatcgttggcggacatggggtgcagatgcgcgcgaacctgcgtgatctcaagcggttcttaataaccctaatgcaggatgcgggctgatcgtgcgcgacgatctcgttttcgcgcgagcagggaagctgtgaacatgaccatgcgccgggccgccttgccccttgccacagcccttctgctgtccgcctgcgcaagccccgtggccggtccgtccgggcggtacgccacgcccatcggcaatgcgccggtgacctccaatcccacgccctactccaccgccctgttctgcctggcggactacgcccggcgctacgacctgccgtcgccgcgcatggccgtcggccggatcagcgactacaccggcacggtgtcggcggacggcgggcgccagatcaccggcggcgcgtccctgatggcgacctccgccttggccaaggcgggcgcccgcatcgtcgagcgctatgacacttcggtttcggaactggagctgcgctacgccaacaccaagctgatcggcgacctggcgccggacgccaagagcccggaggacacccagtaccgacgcatcctggccggtcaggtgccgggctcggacttctacatcgtcggcggcatcaccgaggtgaactacaacatccgctcgggcggcttcgaggtgggcggcgccgaggccgacaccgacaccccgctgtcaggcgcgatcggctaccgcacattcgtgatgaacatcgccatggacctgcggctgatccagaccaccacgctggaggtggtcgacgtggtctcctatcagaagcagatcatcggccgcgaaatctcggccggcgtgttcgacttcctgaacggcaacgtcttcgacatctccgccggctccagcgggaccgaaccggtgcagctggccgtgcgcgccctggtggagcgggccaccatcgagttcatggctaacctttacggtgcgccgggcccggaaatctgcctgaacgccgccaacgatccgctgggcggcagcgcggtcggccccacgggcggtttctatccggcctatccgacccaggacaccaacaacggtgccacccgcgccgatcccaaccgctggaacgatcggcgcgacggggcggttcgcgccagccgctactgagcccgccgtcgcaacggccgcttgttgaggcggccgccatcgcctaacgctctgatggccgcccgggggaggcggcctttccggagtgtccgatgcgtcctgtccgccgcctgcttctgctcgccgcctccagccttgcgctgtcgacggccctgcccaccctggttctggcgcaggccgcgcccgtggcggccgaggcgccgtcccagccctgggcccaggccgccagcgacattcccgccgatcccgccgtgcgcttcggccagctgccgaacggcatgcgctacgccctgctgcggaacgccaccccgcctggccaggcctcgttccggctgcgcatcgacgccggctcgctgatggagcgggacgaccagaagggtctggcgcacttcatggagcacatggccttcaacggcaccaccaacatcccggagacggagatgctgcgtcggctggagcggctgggcctggccttcggcgccgacaccaacgccttcaccagcttcgaccagaccgcctatgtgctggaactgccgaacacccaggccgagacggtcgacaccagcctgtatgtcctgcgcgaaatgatgtcggaggcgttgatggcttcggacgccatcgacgccgagcggggggtgatcgtgggcgaggagcgcacgcgcgacacgccgcagctgcgggtgctgaagacccagctggggctgctggcgccgggccagcgcctgtccgagcgtctgccgatcggcgacctggaggtgatccgcaccgcgccgcgccagcgcttcgtcgacttctacaacgcctattaccgcccctcgcgcgcgaccttcatcgccgtcggcgacttcgacgtcgacgccatggaggccaaggtgcgcggagccttcgagagctggacgcccaaggcggcggacggggcagagcctgatctcggacaggtcgccccgcgcgagcccgagacccgcatccaggtggagccgggcgtgccctcctcaatccagctgaactggatcaccgctccggacaccgaccccgacacggtggcggaacgcgccgagtcgatccggcgcggcctaggcctcgccgtcttgaaccgtcgtctgggcgagatcgcgcgagcggacaatgcgcccttccttggcgccggcggctcttatcagacgctgttcgacagcctgagcctgggtgttctgtcggtcgccttcaatcagggcgcctggaagccggcgcttgagcgcgtcgagcaggaaagccgccgcctggcgcagtacggcgtcaccgacgccgagctgcagcgcgagatcaccgaggggcgcaccgcgcttcagaacgccgttgcgaccgccgccacccgctccacgcccgccctggccgcgggcctgctgaacgcggtcaacgaagacgacgtgttctcgaccccggccaccgcgctcgccatcttcgatcagacggtcgagggcctcaccgccgaccaggtcaacacggcggttcgcgccgtgttcgagggcggtggaccactggtcctgttcaccagccccgtgccggtcgagggcggagaagccgccgtcaccgccgcgctggaagcgtcgcgcgccacgccggtcgaagcgccggccgcccaggcgcagctggaatggccctacaccgacttcggaacgccggcgacgcccgccagccgcacggaggtcgccgacctgggcctgacgctggtgaccttcgccaacggcgtgaagctgaccatcaagccgaccgacttcagggacgagcaaatcctggtcaccgcccgcaccggcatcggcgaactggccctgccgacggatcgcgcgacctccatggccttcgcctcgacggtgatggggccgggcggcctgggcaaattgacggcggacgagctgaaccgcgtgctcgccggccgtgtcttctcggtgggcgtctcgcaggccaccgaggcctatgtcttctcaggcgccacgcggcccgaggacctgcagctcgagatgcaggtgctgaccgcctatttgaccgaccccggcctgcgggccgcgccgttcgagcaggtcaagggcgtctatccgcagatcctggaccagctgagcgccacgcccggcggcgtgttccagcgcgacgtgacaggcctcttggccggcggcgacaagcgtgaaacctcgcccaccgctcaagaggtcgccgccatgaccatcgaggaggtgcgcttgggcgtgcgcgcgggcctcgcctccggcccgatcgaggtgacggtcgtgggcgatgtcgatgtggacgcggtgatcgccgccgtgggctcgacactgggcgcgctgcccgcgcgcggagaagcgccggcgccgctggcgggatcggaccagcgccgctttccctcgcccgccgaagctccggtgcgcctgacccatacggggccggccaaccaggcgctgggcttcgtcgcttggccgactcgggatcagatcggcgaccgcacggaggcccgccagctgacgattctggccgacgtgctgcagctgcgtctgaacgacgaaatccgggagaagcgcggcctcgcctattcgcccaacgccggctcgaccgcctcggacgtctttcccggctacggctatctggcggtcacggccgagacgccgccggaggagttgaccacgctgttccaggccgtggacgccatcgccgccgacctgcgcgacaggccggtggaagccgacgagctgaaccgcgcccgcctgccggccgtggagcgcctgcgccgcaaccaggccgacaacggctactggctgggccagctcagccaggcccagtcggacccgcaggcgctggatcagatccgcagcaacgtgcaggacttggagtcggtcaccccggccgacattcagcgcttggcccaggcctatctgaagccggagacggcctggcgggcggagatcgtttcctcccagccggcgaccgccgccgcgcctgcggctcccgccgcgcgctgacatcgccgtccgacaagagaaaggccccggtcctgctggaccggggcctttttcgtgtcgccttgtcagagcgaccggatcagaacacccggccgccgacgccgccgtccagggtgatggcgctggtgatcaccgccgtggtctccaccacttcctcgcggtactcggtgtattcctcttcgcggaacatggtcagcaccttcacgcccgcgccgtagcggcgcagcagcgaacgctcgttgcagtcgcgctcgggcttctcgggccggcattccagcttgccgccggcgccgtaccacagcgcctcgtgcttgcggcaggtcaggctttcgccgccgtcgaaccgttcctcgccctgccagtccgcgaaggtggcctgcagccaggtgcccgccaggcagcgatacagctcgccttcatagtcctcgccgacgtcccggcccggacgcacctgtgacgccgggtgcggcaccgaacggtcgtcgatgcagacggcgcggatgatcacctgcttcatctcgcgacgccaggcggtgaagggggtgcggaccacctgctggatcggcgcctccacgttcaggccctgaaccgtggtcggatagggctggtccaccgacacataggccgacccgccgccgccgcgcccaaagcccagcccggccgcgttcgacgacgaccagcttcgcgccgaagcacgggcccgcgagagggcgttggcctgggcgttcgcctcggcgttgaccttcacattgacgttcacgttgacgttgttggtgttgcagctgccgttcatgcagtccgcaatcggaggaggcggcggctggcagccgtagtcgcagggctcgggttcgggctccggctcgggcggcggcggctcgggctggcagccctgatcgcagggcggcggctccggcggggggcagaccaccggatcgccgcacgattgcgccgcggccgcatcggccagcgccatgacggcgaagccggcggccaagcccagcaaccacctgttgatccgcaaccgcatgggccgccctccagacatgcgggcgcgcccacgatgcgcgccgctccatctggcatctgaccgcaaaacccttgagtttccgtgaagccggccacagcgaggggatggcgcagagctgcccgcctctgctaacaccccgccatgaccgtgcgcgccctccgccagacgattagccgcccggcgtagcgcttccgggctcctcgccccgcgctcgccgggagactgcagcacgccgccacgatccaaactcacgacgccgagaccgcccccatggccgattccgccgacaccgcccccgccggccgcgactatcgcgacaccgtcttcctgcccgacaccccgttcccgatgcgcggcggcctgcccaagaaggagccggagatcctggctcagtggggcgacctctatgcgacgctgcgcgccgagcgtcagaagcagaacgcgccgctttatgtgctgcacgacggcccgccctacgccaacggcgacatccacatcggccatgcgctgaacaagacgctgaaggacttcgtggtccgcagccggttcctgctgggctacgacgtcgactacgtccccggctgggactgccacggcctgccgatcgagtggaagatcgaggagcagttccgttcaaagggccgccgcaaggacgaggtctccaaggaagaattccgcaaggcctgccgcgactacgccgccggctggatcgacatccagcgcgagcagttcaagcgcctgggcatcaccgccgactggtcgggacgatacgccaccatggacttcacgtccgaggccgccatcgtcgccgagttccacaggttcaagaactccggccagctgtatcgcggctccaagcccgtcatgtggtcgccggtcgagcgcacggccctggccgacgccgagatcgagtatcacgaccacacgtcgcccacgatctgggtcaagttcccggtcaagacctatgacgaggaccgctacagcgtctcggacgacgagcgcggcgagaacgtcttccgcctggcgccgaacgacgcctccgtggtgatctggaccaccaccccatggaccatcccggccaaccgcgccatcgcctacggtccggacatcgcctatggcctctatgaggtcgagacgatgcagtcggacctggcctttgagccctggtccaagccgggagaccgcctgatcctggccgacaagctggccgaggacgtgaagaaggcggccatggtcgccgaatggcgccgcgtctccgacgtcgactgcaccgggatgatctgccgccatccgctgtgggaacaggacgagggcttcggctatgaggtgccgctgctgtcgggcgagcacgtcaccgacgatgcgggcaccggctttgtgcacaccgcccccggccacggggcggatgactatcaggtctggctcgccaacggcttcaccgaggtgccggacacggtggatccggacggcgcctactatccgcacgtgcccttgttcgcgggtctcaaggtgctggagacagagggcaagaagaccggcaagttcggcgcggccaacggcgcggtgatggacaagctgatcgaggccggaaacctgctcgcgcgcggccgtctggagcactcctacccgcacagctggcgctccaaggcgccggtgatcttcaggaacacgccgcaatggttcatccgcatggatgagccgatcgaaggcggccagaccctgcgcggcacggcgctcgcttcgatcgacgccaccgatttccatccggcggcgggcaagaaccgcatccgctcgatggtcgagggccgacccgactggttgatcagccgccagcgcgcgtggggcacgccgttggccatgttcatcgacaaggcgacgggccagccgctggtcgatgcagacgtggacgcccgcatcaccaaggccgtggccgaacacggcgccgacatctggttcaccgcgcccgacagcgacttcctcggtgacctcgacccgtcagcctacgaaaaggtcaccgacatcctggacgtctggttcgacagcggctcgacccacgccttcaccctggatccgcgcacgcctgagcacggctacagcggcgaccggccgtcgcactggcccgccgacctctatctcgagggctcggaccagcaccgcggctggttccagtcctcgctgctggaaggttcgggcacgcgaggacgcgcgccgttcaaggcggtgctgacccacggcttcaccctggacgagaacggggagaagatgtccaagtccaagggcaacaccgtggacccggcctcggtcatcaaggaatccggcgccgacatcctgcgcctgtgggtcgccctggtcgactattcggacgaccagcgcatcggcaagcagatcctgcagaccacggtcgacgcctatcgcaagctgcgcaacaccgtccgctatctgttgggggcgctggcaggcttcgacgatgcggaacggctcagcgactacggccagatgccgccgctggagaggttcatccttcatcgcctgcatgagttggacgcacaggtgcgcgaggcctaccgcacctatcgcttccaggacgtggtgcggccggtgctggacttctgctcaaacgacctttcggcgctgtatttcgacatccgcaaggacagcctctactgcgaccgctccgacgctatccgccgccgcgccgcccgcacggtgatggacgaggtcttcatgcgcctgaccgcctggttggccccgttggcgcccttcaccatggaggaggcctggaccacccgtttccctgatcggggcacgaactgcgcgcgcatcttggcggaggttcccgccgaatggcgcaacgaggccgaggccgaacgctgggccggcgtgcagagggtgctggaggtcgtcaccaacggccttgaggaaagccggcgcgccaagaccatcggcggggcgctggacgcctggcccgaggtgcgcctgcccgccgacgccgccgccctgttcgccgacctcgatgcggcggaggtgttccgcaccagcggcgccgacctcgtcgtcgacgacagcggcgtgatctcggcggtgatcaacacggccggccatccgaaatgcgcccgctcctggcgtcgggtgccggacgtcggctcggactccgaatatccggacctgtcggcgcgcgacgccgacgccgtgcgcttcctcgacgcacaagcggcgcgctgaccgccctctcctcctcatcggcgatggggaggagagccgaaggcgtgctccgtcagagcacgccgatcatgctggccaccagcgggtggcgcacgatgtcgcgctcggccaggcggaccacggcgatgtcgtccaccgcctccaatcgcgccgagatgtcggccaggcccgagacgccgggcagcaggtccgactggtgcggatcgcccgtcaccaccatggtcgagtgccagccgagccgcgtcagcagcatcttcagctggacgtaggtgcagttctgcgcctcatcgacgacgataaaggcgttgttcagcgtccgaccgcgcatgtagccgatgggcgcgatctcgatcagtccctcggccatcagcgccttgacccgcttcatcgacagccggtccgacagggcgtcgtagagcgggcgcagatagggagccagcttgtcctccatgtcgccgggcaggaagccgatcgattcgccggcctccaccgccgggcggctcagcactatgcggccgaccttgcccgcctccagcgcctccaccgccttggccaccgccagataggtcttgccggtgccggccgggcccagcgccatgaccaggttgtgggcgtcgatcgcctccatcagctcggcctggccgtcggacttgggcttcagcgtcttcagataggcctggtcgcggtcgtcgttcgagggatagggcgaccagccgggccgtggctcgggcccatgcagccgccgaaccttggattcctccatgaactcacgcgaatcgagcaggccgtgctcgcgagactgacgccgggttgccgcacgcttggtcatggacgcctccagggcatgaaaaaaggcgggcccgaacgagcgccgccttggatggacgtggggaggaaagaagcgagcttggcgacgccgcctggatcgccggagccgtatcggccggggacgcaccccggcggcgagccgatctccagcggacccccatgcgtcacgcgcacgctccgacttcagaccggaccgggcttgatccggcttcggattcgccgcgacgcgaggccgcctcgaatcacttcaacagaaggatgctaacgtggtttgcagacccttgaagcgatattccggtcacaaagaggagacgccgcgatgacgatctacgccctgggcgaccagcaaccgcaactgcccgcgaacggcgatgcctggatcgcgcccacggcttcggtcatcggccatgtgatcctggaaccgggcgccagcgtctggttcggcgcggtgctgcgcggcgacaacgagccgatcaccataggccccgacagcaatgtccaggacggcgcggtgctgcacaccgatccgggctcgccgctgacgctggggcgcggcgtgacggtggggcacaaggccatgatgcacggctgcgtcgtcgacgactattcgctgatcggcataggggcggtgatcctgaacggcgtgcgcatcggaaagaattgcatcatcggcgccaacgccctgatcacggagggcaaggtcattcccgacaactcgctggtcatggggcagcccggcaaggtggtgcgcgaacgcgatcccgaccagatcgccgtgctgaagatgtcggccgagcactatgtcgccaactggaggcgctacgcctcgggccttcgccctatcgcttgaggatgtcgcgagctcgggcggcgtcgatgtcgatctgggccttcagcgccgccagcccgtcaaaccgcgcctcgccgcgcagaaaggcgaccagctcggtctcgaccacctggccgtacaggtcgccctcgaagtcgagcagccagacctccagcagcggcgtctccagctggaacatcggccgcacgcccaggctggcgacgccgtcgacgatccgcccgtccgccagccgcgtgcgcgtggcgtagacgccgtaggccggccggacgtagtcgcccagggccacgttcagcgtcggcacgccgatggtgcgcccgcgcttgtcgccgtggatcacctcgccttcaatggcgagggggcggcccaggatcgccgccgcgcccgccatatcgccggccttcagcgccgcgcgcaccgcgctggacgacagcttcagcccatccaagccgtcgtggcgcggaacggccgacaccgaaaagcccagcgtctccccatagcggcggagcgcctcaggcgagccggaccgtcccttgccgaaggtgaagtcaaagcccacggccgcatggcggacgcccaatccgtcggccagcaccttgcgggcgaagtccgcgtcggacagcgccgccatctcggcgtcgaacggaagaagatacagccgctgcacgccctgcccggccagggcgcgggccatctgatccgtcgacatcaggcgaaacggttcggcgtccggctggaaccagcggcgcggatgcggatcgaagctgacgacgcccagcggcgcacccatccgatcggccgccgccctcgcctcggcgatcaccgcctggtgcccccggtgcacgccatcgaaagcgccgatcgccacggccgcccccttcagcgtcgcaggcggcccgcgccagtcgcggacgatctccacggtcagcgggcggacggcttgcggcggcgcggcacgcgaacgaccgccacgccgtccatgatcagggtgtcgccgacaaagccctcgcagctcagtttcacccgcgcgctatccccctcgatctcgatcacagtgatgcggatgcgcacctcgtcgtcgatccggaccggctggtgaaatgaaagggtctgggagatgtagatcgatcccgcgcccggcaggatcgttcccaccaccgccgatccgaacgaggcgctgagcaggccatgggcgatgcggccgcgataggcggtcttggaggcgaagccctcgtccaggtgcaccggattgaagtcgtccgaggcctcggcgaacaggcggatgcggtcctcggtggcgaccacgagcttctcggcggccatgccgacgtgaagttcatccaggatatagcccccggacggatgctgctgaaccagatcgaccatccgacaggccttagcgcccgtgtgacaaaatggcgagccttcgccgttcgcgggtcaccacttcaggtccagcgtggcatagcgggcataggcggtctcggccttgagcaaggcggccgccccgctcgcgtcgagctcgccgtcggcgccgcgcgccgcatcgccgtggatgccctgcgccacgaacaggcagtccagcccctgcgcattggcgcccagcacgtcggtgaccacgccgtcgccgatgcacagcacgcgtgagcgatcgacggggcgccccagcagggcctcggcctcctcgatggccagttcatagatcgggccgaagggcttgcccgccatgatcacgcggccgccgaggtcttcgtagacgtcggccagcgcgccgccgcagtagatgatctggtcgccgcgctgcaccacgcggtcgggattggcgcaaatcagctcgaggtcccgggcgacgcccgccgccagccgctcgcggtaatcctcaggcgtctcgacggtgtcgtccaccgggccggtgacggagatgaaggcggcgtcggcgacgctgtccgcccgctgcaggtccagcccggcgtagagcggcgcgtcccgttcgggtccgacgatccagaccggaccgggcgcccggcgttgaagctccatccgggtcgcgtcgcccgaggtgacgaacgccttccagctgtcgcgcggcacgcccaggccgtccagctgcgcgatcacgtcgtgcgccgggcgcggcgagttggagatcaggacgacgtgcccgccttcctggttgaagcgggtcaaggccccgcaggcgtccggccagctttcgcgcccgttgtggatcaccccccagacgtcgcacagcagaatatcgtaatcggcggagaccgcgccgagatgaggcagaggcgtgggaagggtcatgccggctgtctagccgccggcggcggaccgcgaaagcctcagccgaagcggcggcgctgctcggcgctgcgcagggtggagcgaaggaagtcggcgggcgggtcggtttcggccagcacctgttccttgatggcgcgcggctcgccgaacaggtggccctgtcccatgccgatctcgaggtcgaggatgtcgacgacctggcgctcgctttcgaccttttcggcgaccacctcgacgccgtagcggcgggtgagcgcggcgaagtcggcggcctggatgtcgggcatggagcgcaagggcgcgccgccgtccaggtccagaagctgctcgatcagcaggtcggcggcgaccttgacgaacttgacgtccgaacgctgcaggtcggcgaagtcgaggtccagcgtctgcaccttgtccaaggagaagcggaagccgagatccgccagcttggccatgttgcgggcctcgacggcgccgcgcgcgtcaaaggtcgcctgccccagttcgaagatcagggcctgattcaggtcgcggttctcgctgagaaaatccaggaactgcgggaaaaaggtctcgtcgccaagcgaggtgagggcgacgttgcagaagacgccgacctttcggtcctgccgcgccagccggcgcacgatctgggcgcagcggaacagcaagaggttgtcgatggcgggggccagcccctccgtctcggcggtggccagatattccgccggcatcatcacccggtcggaagcgtcccgcagccgggtgaagctttcatagaagacggtgcggcgctgcggcagcgagactaccggctggaggtacaggtcgacccggttctcgctgagcgcgtcgtgaatggtcttcagcagcacgttcgactgctggtgacggcgaccctccggcgcatccagcgcgggggccggcgtctgggccaggcggtcgtcgatgctttcgctcatctgctggatcagcgtctccaacatgcgcacctcggaggtcagctcctccgtgcgggagatggcgccgctttcgatggcctgggccagttcggtcagggcgccctgcgtcgactccatcgcatcggccaggaggcggtgggcctctcggacctggccgatctccttcttcagggcgcgccgctccatcgcgccggtgatgatggcgtgaaaggcgccgagcaggcccagcgcgcccagcgtccccgccacgcccgcgccgatccccagccccgcccgccacagaaaggcgcccacggtgagcccgaggaacagataggcgaaatacagaaagccggcggtgacgttgcgcatcggtctcggttcggctgccttcccggatggaatcggccggagatcagcgtatcagggaagctggcggagcacagcgcggaaatcaaccggacggcccgcaggaggaaagacgcatggaactgttcgacctgtccggcaagaccgccatcgtgaccggatcctcgcgcggcatcgggcgcgccatcgccgagcggctggccgagcacggcgcccgggtcgtgatctcctcgcgcaaggccgcgccgtgcgaggaggtggcgcaggccatcaatgcgcggcacggcgatggacgcgccatcgcggttcccgccaacatcgcctccaaggaggacttgcagcggctggtcgatgagacgatccaggcgttcggccaaatcgacatcctggtctgcaacgccgccagcaatccctacgcggggccgatggcgggcatctcggacgagcagttcgagaagatcctgcgcaacaatgtgctggcgaaccattggctggtgcagatggtcgcgcccggcatggtggagcggcgcgacggcgcgatcctggtgatctcctccatcgggggcctgcggggcaatgcgctgatcggcgcgtacaatgtgtccaaggcggcggacatgcagctggtgcgcaacctggcggtggagttcgggccgtccaacgtgcgggtcaactgcatcgcgccagggctcgtccagaccgacttcgcccgctacctgtgggagaatcccgaactgctgaagcaggtgacggaccccgcccccctgaagcggatcggccagccggacgagatcgccggcgccgccgtgttcctgtgcagcaaagcggccgcctatacgaccggccagacgctggtggtggacggcggcctgaccatcgcctggtagatcaggcgctgggctcaggcgcgctgggcgtcggtggcgcggcggaacgggccggcgtagccgaactcgtcgcgcctgcggcggcacgggccgaaataggtgtcggtctttacgaacgggcgcggcttgaagacgaccgcattgatgcggtccaggatggccttggcggtgatcggcttgaccacgaactcggtcacgccggcgtcgcgggcgtcggtgacgcggctgcgctcggagtggccggtcatcatgatgatcggcagatagacgttggggctgtccggggtggtgcggaccaggcgggtgaaggcgcagccgtccatcgggaacatgttgaagtccacgatcgcgagatcgatcggatactggcgcagcagggccatggccgccgtgccgtccgccgcctcgcgcacgttgcgaatgcccgccgactgcagcaccgcggacgcgatggtgcgcatgtgctggttgtcgtccaccagaaggacgttgagcgactggaaggcggacatgacaagcgcgttcttgaggtgatcccggagcgtagagagccaatggttagcgagccatgagcgcgtctacgccgagccgggaatcatcggggttccggcgatgccgccgtaggcctggggatatccttgatcctgtcgacgtcggcaagatcgggcgcatcgtccgccgcccctcgcaccgggcgggccggctcgggcgccgcgcccatgcggtcgatcagcttgaacacaaagggattaatcgagatcgagagaagcgcgccggccaggatcaggtcgtgggtctcgcggctcatggcgcccagggccatgccgagtgcggccaggataaaggagaactccccgatctgggccagggaggcggcgacggtgaggctggtcctgcgatccagcttgaacacggtggtgatggccagcgccgccgccgacttgccgacgatgatgatcaggaggacgctcagcaccgcgcccggctcgcgaaccagaatgcccgggtcgaacagcatgccgaccgagacgaaaaacagcacggcgaaggcgtcgcgcagcggcagcgaccgttcggcggcgttgtggcccaggggcgtgccgttcagcaccaggcccgcgacaaaggcgcccagggcgaaggaggcgccgaagacctcataggcgataaaggcgatgcccagggcgatggccagcacccccagggtgaacaactcgcgcgacttggtgtgggcgatgcgcaccagaagccatggcagcatcttgccgccgaccaccagcatcagggcgacgaagacggccaccttgaccagcgtccagccgatgttggcggccagggcgcccggatcgacggcggttccggccggcaccacaaccagcggcagcatgaccagggcgatgacgatgaccagatcctcgacgatcagccatcccacggcgatcttgccgatgtcgcccttggactggcgacgctcctcaagcgcgcggatcagcacgacggtggaggcgaccgacagggcgaaacccatcagcagggcctccacgttcggcagaccgagcgcgaaacggcccagcacccaacccagagccgtcgccgccgagatctggaccagcgccccgggaatggcgaccttgcggacctgcatcaggtccttgggcgagaagtgcaggcctacgccgaacatcagcaggatcacgccgatctcggccaattgcggcgcaagctcggtgtcggcgacataaccgggcgtgaacggccccaccacgacgcccgccaccagatagccgaccaggggcgacagcttcagccgattggccaacatgccgaacacgaaggcgaggacgaagcccccgaccagggtgagaatcaggctgtcggcatgcggcatcggcgctccttttgacggtgagctcggttcagtgatgggaagcgttacagttggtggcgcggccgggtaaaagcaagccgcaaacgcccatggcgatgtcgggtcgcaggcgcgcgaaagccccggtgtgcgtgatgcatccggttggagggcgggcggggcgccgggccttcgcccggagtgtgagtagaggttaccgtttcgacgaaagctgacgccccgcgcggatgattacgc

SEQ ID NO: 4 - DNA, 272075 bp, brevundimonas massiliensis
  source 1..272075: mol_type = genomic DNA
tggaccacctccccttcgacgccgtcgaccgccaccgcgccgggctgctgtccgtggatggccgccagtcccgcgcggcacacgcgccgcaggtcggccgccgacagcacggccggcgcggcgggcggcgcctccgcaggcggtagagccgccggcaccctgttcgccggcgccggccgcgccccgcgccccgcgccggtcgtgcgctgcagccgctgatcaagaagctggacgagacgttcgggcgcggcgccgcggcgctggagccgcgctgggtggagatcgtcggcgagcggctggcccgcgtctgccgcccgcagaaactgaccaagggacgcggcggccagcccggcgttctggagctgcgcgtcgtcggcgcagcggcgctgctggtccagcaccagtcggccgagatcctgtcgcgcgtgaacctgttcctgggcgcaggaacggtggatcgcctgcggatcgcccagggtccggtgaagcccctgcccgtccccgccgccaaatccaccaccgcacggccgcctcttccggccgcaacggaggccgaactgttcgcatcgctggcggacgcgcccgacgcgctcaggaccgccctgcacgcgctgggccgctcggcgatggcgcgcgacgccgaggagcgttgacaaaccttcgccgcacctgttctcgatgatgaacaaggacgcgcagttccgggggagccgcgccgccgactagacgccaaaggatgccccatgcgcgctgaacgtccgtcccgcctcgcccagatgagccgccgtgcggcgatcaccggagcggcgctcgccgccatggccctgtcggcctgcggcgggaacaagggcggatcggccgagggcgacatggcgctgggcgcggccgacggcgccaaggtcacggtggtggagtacgcctccgtcacctgcggccactgcgccctgtggcagcagaacacctggccggccttcaaggccaagtacgtggacaccaacaaggtccgctacgtgttccgcgagctgccgacgccgccggtggacgtggcgacggccggtttcctggtcgcgcgctgcgccggcgacgccaagtatttccaggtcgtgcaccagctgctggccacccagcaggagatggtcaccggctcgccgcgcgactggctgctgcgcaccgcccaggccgccggcatgaacgagcagcagttcgccgactgcgtttccgaccgggacgccgtggccgcgctggagaagcgcatccagcaggcccaggcgcagggcgtcaccggcacgccggccttcttcgtcaacgagcaggaagtgatcacgccgggcagcagcgaagggcccagcctggccgacctgtccaccgccatcgacgccgaactggccaagtgagcctgatgcgccgtcatcttctggcgctggccgtgctggcgacgaccgcctcttcgggctcggccttggccgccgacgtgccgccggtgacggcggcggaccgggtgctgggccgcgccgacgcaccggtgacggtgatcgaatacgcttccttcacctgctcgcactgcgcggccttccacaacgaggtgctgccggcgttcaaggcgcgcttcatcgacagcggccaggttcggctggtgtaccgcaatctgcccacggcgcccgtcaatgtcgcggcggcggcctcggccgtcgccgtgtgcgcggcgcctgaccggttcttcgacgtcgccgacgccttcatgaagggtcaggcggggctgtcgaccaccggcgccaagccctggttcgacgccggcgtcgccgccagcggccgaacgcgcgagcagatcgagacctgtctggaggcgcccgccacgcgccagacgctggaagcgcagatccagggcgcgcaggacgccggcgtggacggcacccccacactgttcgtcaacggcaagcgcgtcacggatcactcgctggccgccctcagcgccgccgtcgagccgctgctgacccggtgatccgctgatcccatgcagttccagcggctgcggatcgtcggcttcaagtcctttgtcgacgccgccgaggtgcagatcgagccgggcctgacgggcgtcgtcggtcccaacggctgcggcaagtccaatgtgctggagagcctgcgctgggtgatgggcgccaactcggccaaggccatgcgcggccagggcatggacgacgtgatcttcgccggcgcgtccggccgcccgccgcgcaaccatgccgaggtccagctgaccatcgacaatgcggaacggcgcgcgccccagccgttcaccgacgcccccgtgctggaggtgtcgcgccgcatcgaccggggccagggctcgacctaccgcatcaacggccgggcggtgcgggcgcgcgacgtgcagttgttgttcgccgacgcctcgaccggggccaactcgcccgcgctggttcggcagggccagataagcgaactgatcgccgccaagccgcagaaccggcgccgcatcctggaagaagccggcggggtcgccggcctgcatacgcgccgccacgaggccgagcttcgtctgcgcgccgccgaggccaacctggagcggctggacgacatcggcaaggagctggagaccgcgctgaaccggctgaagcgcgaggcgcgtcaggccgaaaagtacaaaaaggtctccgccgacatccgcgcgttgcaggccgccctgctgttcgtgcgctggaacgatgcgcggatggccgccgaggccgcggccgccgatctgcgggaggccgaccgcatcgccgcggagacgacgcaggccgccgctcgcgcgtcgaccgaggcgttgcgggcccaggaggcggtcagacccgcgcgggaggaggatgcggtcgccgccgccctgctgcaccgcgcgacgctggagcgggaccggctggacatggcggaacaggccgcccgagccgaggtcgagcgactgcgcgccgaggtcgcccgtctatccgccgaccaggagcgcgaggcggcggtcgccgccgacgccgcacgcgagctgtcgcgcatcgacgccgagctcgagcgtctgcgtgccgagatcgcagccgcccccgcgcgcgggcccgagctggaccgggcgacggaggcgacggagacaacccggcaggcggcggacgccgaggtcgagcgcctcgccgccctggcggccgcgacggaggcccggctgaacgcggaggccgcgcgccgcaaggaggccgaggcccgtctgtcccggctggaggctcagcacgaggcggcgcggcgcgaacacgaagccatagggccggcgcggacgtccgaggtcgaacaggcgcaaggggcgctgaaggcggcgcaagggtcgctcgccgccgcgcgcgccgaggttgaggcggccgagacccaccgcggtgattgcgcccgcaccgaaggcgacgcccgatccgctgcgcgcgcggccgaggatcggctgggtcggctgcagaccgaggcgcggggactggcgcagttgctgaccaccacgcggcgagaccatccgcccgcgctggatcaggtgtcggccgagcgaggctatgaggcggcgctggccgcggcgctgggcgacgatctggacgcggcgctggacccccgcgcgccggcgcactggaccggaggcgcgacgccgacggtggagtggccgcaaggcgtggagccgctgggctcccgcgtgacggcgcccgacgccctgactgcgcgtctggcgctctgcggggtcgcgccgcgcgacaggatcgaagccatggccaaggccctgccgcccggcgctcgcctggtgacggtggagggcgacctttatcgctgggacggctttgtcagccgggccgaagccccgcgtcccgccgccgtgcgcctggcccaacgcacgcggttggcggagctggaaagcgccatcgacacgggacgtccggacctcgcgcaggcgcaggaggcgctgaaggcggccggcgaggcgctgcgcgcggcggacgagcgggtccgggcggcgcgccagcaacccttcgccgcagacaaggccgtagcgaccgcccgcgaccggctggagacgctgaaccgggaggaggcccggcgcgaggcccgcgcggcggcgctggacgagaccctgatgcggctgacgcgggaacgagacgaggcgcgcggggcggtcgccgtcctcgcctctcccgacgccgcctccgccgacgggctggcgacgttgaagactgacctggcgaacgcgcgcatggccgccgatgcggcccgcgacgcggccatgcgcgcccgtagcgcccgcgacgccgaagcgcgcgagcgcgcccagcgcgaacagcgccttggcggcctgatccgcgcttgggaaggctgggtcgtgcgatcctccggcgcgacaaaacggctggccgaactgggcgccgacgccgaggcggcgaacgcccgcctcttcgccgcccgccaggcgccggagggcttcgccgagcagcgcgcccgactgatggacgccctgatcgcggccgagacgcggcgcaaggcggccggcgacgccctggcgacggcggaggcctcggcgaccgaggcggatcgcgccggccgcgccgccgacgccgccgcctctcaggctcgagaggcgcgcgccggcctcgccgcccgtgcagacgccgccgctgaacggctaggcgaggcggaggctaatctgcgagagggcgccggcctgtcgccggaggaactggagcgcaagctgaccgccgatgcggtggcgcgcccgccggacgcggccggcgccgaggccctgctgatcgggctggagcgcgaacgcgagcagctgggggccgtcaatctgcgggccgaggacgaggcagtggagtacgcggagcggctgaacagcatgcgatccgagcgcatcgacctgacccaggccatcgcccgcctgcgcgacggcatcgatgaactgaacgccgagggacgtgagcgcctggtggcggcgttcgacatcatcaacgacaacttcaaggccctgttcgccgccctgttcggcggcggcgaggccgagctgaagctggtggaaagcgacgatccgctggaggcgggcctcgagatctacgcctgcccgcccggcaagcggctgtcggtcatgagcctgatgagcgggggcgagcaggcgttgacggcggcggcgctgatcttcggcgtctttctggccaatccggctcccgtctgcgtgctggacgaggtggacgcgccgctggacgacgccaacgtcgaccgcttctgccgcatgctggacgagatgcgcaagcgcacggacacccgcttcatcgtcatcacccacaatccggtgaccatgagccgtatggaccgcctctacggcgtcaccatgcccgagcgcggcatgagccaactggtcagcgtcgatctgacccaggcggaaaggatggtcgcatgatcgcaccggccctgattctggccccggtggtggctctgacgtcgccgagcgaaccccggctggtggagacgggcgtcgggcggtttgccgtgttcgccgacaccgcctcgatccggcgcgagggcgacgtggcctatatgcgcgagctgcaggtcgtggagaccggcttcgaggtcggcggaacaatctatgtcggcggctggtcgcgctgggcgtttgactgcgtcgccggcacggcggaccggctggacttcgcctcgctgcggagcgacggaagcgaggggccggccacacccgatcccgccccggccttcccggcggcgccgggcggagacgccgccgaactgatggctgtggcgtgcggcggacaaaccgcgccacatgcgctgagcctatcggaggcgatcatccggggccaggctgcgctggccgagtgacgccgtctcaggcgtgccgctgtcgggacttccgccgggtccgctgagcggccggtcggcgggaccggacggcgtgtgcggacgctcttccccttgcggccactccaggcgatcccgcggcagggcctcgcggcattcgtcgcgcatgaaggccatcagcttttcacggatctcgcaacgcaggtcgaaggccaccggcgccgagcgcgcgctggcgaggcagcggacctgcagcacccgctcggtgatgtcggtcacctgcatcacctgcacgtcgccgtcccacagcctggagttcttgacgatgtcttcgaacgccgcgcgcagccggtcgatcggggcctcgtagtcgacatagaagaaggccgttccgatcaggcgagcgttgtcgcgggtccagttctggaacggggtggtgatgaagtagctgagcggcagcaccatgcgacgccagtcccacagcttgaccaccacataggtggcgctgatctcctcgacattgccccactcgttctcgacgatcacggcgtcgtcgatgcggatcggctgggtcagggcgatctggatgccggccaccatgttggtcaggatgggctgcagggcgaggcccgcgatgatgcccaccacgccggcggacgccaggaggctgacgccccactgacggaaacccgagatcgtcatcagggccaggcccacggtgacgatcaccaggatcaccttgaccacccgctggaggattcgggtctgggtcaggtgcttgcgcgccaggaggttgtcctcgacagcgacgttgtaccgcttcaggtggaccacggtccacatgtccagcacgcccgacaccagccagccggtggcgaggatgaagaggaacagcagcaccgaacgcacgagggcggatggctccgggttcagcggcgagacgctgaccccgatgccgatggcgacgattacaagaaggacccgcagcttgatgcgcgcccgctcgaccacgccgcgccagaagacgtcgcggttcttcaccagccgccgcaagatggcgaaggcgatgcggtgcgccagcagaccgccgccgacgaacacggccagaacgattagcaccacggcccactcgggaagccagtcgaacctgtgccacaagcgcgacgtttctcgcgtcaggtcggtgatccatgaaggcatggccataaggacgcgccatcgccccaacggttcccgccaagcttcgccgatccgtgtgacgcggacgatggctgtgacctagcggccggccacgtgctcggtcaggtcggcaaggcgcacggcggcgtcggggatggccacggaacgcgcgccgtccgacatggccgtcagtcggctcggatcggacaggatctgctgcagggtcaccgccagccgctccaccgtcagggcgtcctccaggatgacctcggcggcgccggcgtccaccagggcctttgcgttcaaacgctggtggtcgtcggtggcgatcttcaacgggatcagcacggacggcagggcgcacaccgccagttccgcgcaggtcgaggcgcccgcgcggccgatcaccaggtgcgaggccgacagccggctggccatgtcgcggaagaagggcgccacctccgcgtcgatcccggcctccagatagatctggcgcgcctcgtccatgctctcgggccgggcctgctgatgcacgatcaggcgacggcgcaggccctccggaagggcggccagcgcccgcggcgtggtttcggccaggaggcgggcgccctggctgccgcccgtcaccagcacgcggatcggaccgtcctcggcgggcggggcgtaggcgccgtcgaacaccgcgcggatgtcggcgcgcacggggctgccgaccacatgggcgcggccctgcaccttctccggcgcatgctgcagcgtcggaaaggaggaggcgacggccttcatatagggggcgaggatgcggttggtgcggcccagcaccgcgttctgctcgtggatcagggtgggtcggccctgggtgatcgccgccaccagcgccggcgccgagggatagccgccaaagcccaccaccacgtccgcgcccagccggtcgaacgcggttcgcgcctgcatcacgccccggaagatggccgagccggccttgagcatgccgagcgggccggacgccgtggccgcatccagcgacagccgctcctcggccggaaagccgtgggcgtagacctcgcccctgtgatcgctggccagcaccacccgccagccgcggccgatcagttcgcgcgccagcgcctcggccggaaacatatggccgccggtgcctccggcggcgacaacgcagagcttggacatgtcccgcccttacagcaagcgccgccgtgtcccaagggtcgcgccgggctcataggcgccaggcctgcgccgtgtcagcgccagcgccagccccatggttagccccatggccagcatcgacgatccgccatagctgatgaagggcaaggtcatgcccttggtcgggatcaggttcaggttcaccgcgatgttgatgcaggcctgcagcccgatcagcatgaacagccccgccgccgccgtctgctcgaacgggtcgttcagcttcatggccttcttcatgccgcgcaggacgataaaggcgtagaggccgatcatgatcaggctcaggatcaggccgaactcctcggcgccgaccgaatagatgaagtcggtgtgcaggtcgggtacgcgccgcttcatcaccccttcgcccacgccgcgcccgatcaggccgccggcgcggatggcctgcgaggcgctgtcgatctggtgggtgtccgtggtctcgggcgagaagaagcggctgaggcggtcgcgcatgtgcccgaacacgaaatacagagacaccagccccgccatgccaaggctcgccagcaccgccatccacttgaacggcacgcccgccatgaagaagacggccatgaaggtggtggtgatcagcagcgtctggccgatgtccggctggatcagcagcagacacacggtcagggcgtagaagccgaaggcgatggtgacgccgggcacgccctgccccttctgcgcctcggcgaacatccaggcggcgaagacgatgaggccgggcttggcgaactcgctgggctggaggctgaacggccccaggttcacccagcgcgctgcgcctttcaccgtgtcgccgatgaacggcagcgccgccatgaccacgatggcgcccagcagggccagaatggcgatgcgccgcacgcccttgggagacaacagcgacgagcccagcatcagggtcagacccaggccggagaagaccatcatccgccaggagtagtggaacgggtcggagatcgattcgtcggccaggatggcggcggggctggaggcgaagctcagcgccacacccagcgccatcagggccagggccgcgctcaagaggccgcgatcgacggtccagaaccatttggcgagcgcgctctggtcgttgcgcgagaaggcgggggcgtaggaactgctcatgccgagggctccggtgcggcgccgaggttcaggacggcggctctgaacgcctcccccctggcctcgaagtcgggatactggtcgaaagaggcgcaggccggcgagagcagcaccacctgcgggccgccttcagcctgcgcatcggcggcggcggcctggacggcggcctccatcgtgcgggcgacgaggtgcgggatcgcgccgagcgcaccggcgaagtcttcggccgcctcgccgatcagataggcgcgggcgatgtgggaaaacaggtcgcgcaggtcgtcgatgccgccggccttggcccggcctccggcgatccagaatatcctgtcgtagctggccagcgcctggcgtgccgcgtcggcgttggtcgccttggagtcgttgatgaagcgcacctcgccgagccttccaaccgcctccatgcggtgggcgagaccggggaaggtcagcaggcccgcgacggcctgttcgtgcgacacccccacggcgcgcgccgccgcataggcgaaggcggcgttctgggcgttgtgccgtccggggagagagcgtgaagcggacaggtcgacctgctggtcgccaatgatcaacgatccgggccgcgccagatatccttctcccctcgggggagaaggtgggcccgaagggctcggatgaggggacctatcctgcgaagcctcttcggaagacgaacccgccctatgcggcccctcatccgtctcgctgcacgatccaccttctcccccgaggggagaaggctccgtacatacgggttcgaccctgcgcccctgcgccgatagcgttcgcgcgatctcggcgccccatgcctcatccaccccgaccagcgccagtcccgcatgggtgaagatgcgtcgcttggcggcgacatagccctccatgccgccgtgccggtccaggtgatcgggcgagatattggtcaggatggccacgtcgggcgcgaagctgtcggtcaggtccatctgataggacgaggcttcgatcacatagacggcttggggtgatggctccggcagggccagcacgccgatgccgatgttgccgccgacgtgcaccgtcaggcccgcctgcttcagcacccagccgatcagggcggtggtggtggacttgccgttggtgccggtgatggcgacgacctggggacgccgggcctggggcaaggcggcgacggcgcgggcgaacagctcaagatctccgatcaccggaacgtccgcggcccgcgccctatccaccgtccagtgcgggcgcggatgggtcagcggcgcacccggcgacagcaccagggcggcgaagccggaccagtcggcgctcgtcaggtcttcgaccgcaaaaccttccgcctgcgcctgcatgcgccccgagacgccgtcgtcccagaggatcggaatcgcgccgccggccgcgagcgcgcgcgcggccgtgatccctgaccggcccaggccgaccaccgcgacgcgccggccttcatatcccggaacggggatcacgcgggggtctttccgtcatcctcgggctcgacccgaggatcaaagggtccgccgctggcgcgcggatacaggcgcacagcccaatcggcgcccaatcctcgggtcaagcccgaggatgacgatgaaagaagcgtcatcaccgcagcttcagcgtcgacaggccgaccagcgccagggcgccggcgatgatccagaagcggatcaccacggtggactccggccagcccatcttttcgaagtggtggtgcaccggggccatcaggaagatgcgcttgcccgtcagcttgaagtagccgacctggatcatgacggaggcggcctcgaccacgaacaggccgccgacgatgcccagcaccagctcgtgcttggtggtgacggcgatggcgcccagcgcgccgcccagcgccagcgacccggtgtcgcccatgaagatcttggccggcggggcgttgtaccagagaaagcctgcgcccccgccgatgatggccgcgcagaagatcgacagctcgcctgcgcccggcacgtggtggatctgcagatactccgaaaacacgaagttgccggccagataggagatgacgccgaacgccccggccgcgaacatcaccggcaccgtcgccagcccgtccagcccgtccgtcaggttcaccgcattggagaagcctacgatggtgaaggcggcgaaggccacatagaaccagccgacgttcagcagcaccgccttgaagaacggaaaggcgatggaggtctccagccccggcgatgtcggcgaataggtcatccacgccaccgtcatcaccccggcgaccagcgacaccagcgtctgggccagcagcttctgcttggacgtgagaccggcggaagtctgcttggtcaccttggcgtagtcgtcgatgaagcccagcactccgaaagccgccgtgacgaaggacacgatccaaaggtaagggttggtcaggtcaccccacagcagcacgcccgccccgatgccggccaggatcatcagcccgcccatggtcggggtgccgaccttggacaggtgcgacaccggcccgtcctcgcggatcggctggccgcggccctgcttggcgcggatccagttgatgaagcggctgcccatagccacggcgacgatggcggcggtggccagcgccagcgccgtccgcaccgtctggtactggaccaggttcagcagcggatactggtgcgccacgtcggcgtagtagaggtagagcaggtagaacatactggattttcctccaccgtgtcaggcgagagacaggtcggcgagcgcgcgggcgaccagggcggcctttgagccgttggagcccttgaccatgaccacgtcgccggggccggccaaaagcgccgcttcggccgccagctcggccgccgtctcgcgccagacgccgcgccgggatgtcggcaggacgtcgtagagccagcgcatctgcggtccggcggcgtgcaccatgtccaggcccgcggcctcgatggcttccgacaggccttcgtgcaggctacggctctggtcgcccagttccagcatgtcggtcagcaccacgacgcgccgcccgtccgtcggccgcgcgcccagggtgcggaaccccgccgccatggacagcggattggcgttgtagctttcgtcgatcagggtgaaggcgccgcccggcgcgtcgacggtccgcacctgccctcggccgaccagcggctggaacccggccagggcctccagcgccgtgtccagcggcacgtcaagagcctccagcatcaggatcaccgccaggctgttcagcccccagtgcgcgccgctctgcgccaggcgatagtcgatgcgccggccatgcagttcggtcgagacgcgggcgccttccgcatcggcctggaagtccagaagccgggcgtcatgggcgccgttcgcgccgaatgtcgccagacgggcgccgaccgctctggcgtgctcggccagcaccgaggcctgagccacatcgccgttcgccacggccaccccgccctcgaccagaccgtcgaagatggccgccttttcgcgcgcgacgcccgcctcgccgtcggcgaaggcctcgatgtgcaccgggccgaccgtggtgacgcaggcggcgtgcggccggaccatgcgcgacaagggcgcgatctcgcccggcgcgttcatgccgatctcgaacaccgcgcgttccgcgtcgcgcggcatgcgcgccagcgtcagcggcacgccgatgtggttgttgtagctcttgatcgagccgtgagcgcgtccggccagatccagacccgcgcggatggcctgggtcacgctggtcttgccgacgctgccggtgacggcgccgcgcttcacgcccgggctgcggtcccgcgccgccgcacccagcgcctccagcgctttcagcgtatcggagacctgcacgaacggcccgccttccaccggccgctcaaccagagccagggccgcgccggcctggaaggcggccgccgcgaactcatgcccgtcgcgcgcgcccttcagcgccaggaacaggtcgcccggcgcgatctcgcggctgttgtaggtcaggccggtcacggcaacgtccggaacggacaggacgccgcccgtggcggcggcgatctcggcggccgtccacagcgggcgcgattggggatcaggcatggacggcgagagcctcggcagcgacagcggcgtcgtcgaaggggtgggtcacgccggcgacgatctgaccctgttcatgcccttttccggcgatcaccaccacatcgccgtcgcgcatcatctcgatggcgtagccgatggcgctgcggcggtcgccgatctcgaccgcgtcagagcagccggccttgacctcggcgcggatggcggccgggttttcgccgcgcggattgtcgtcggtgacgatggcgtagtcggccagacgtcccgccacctcgcccatcagcggccgcttgccccgatcgcggtcgccgccggcgccgaacaccacgatcagccggcccttggcgtggggacgcagcgccttcagcaccgtctccagtccatcgggggtgtgggcgtagtccacatagacctcgccgccgcactgtccgccgtcgatgcgctgaagccggccgcgcgcgccctgaagctgctccagagcgccgatcaccgcatccggccgctcgccggccgcgatgcacaggcccgccgccaccagggcgttggaggcctgaaaggcgccggccagcggcagcaggatgtcgcgggtgtcaccacgcacgtccagcgtcagccgctgaccctcgggcgtcgcacgccgggccaggagggtcaggtcgcgcccgcgctcgcccacccccatcacccccagcccggccatgatggaggccgaggcgaaggccccataggcgtcggagtcggcgttcagaaccgccgtgcggccgcgcggcagcagcgtctcgaacagccgcatcttggccgtgcgatagctgtccatgtcgccgtgatagtcgaggtggtcctgcgtcaggttggtgaaggccgccgccttcagcgccacgccgtccagccgccgctgatcgatgccgtgggacgaggcctccaggcagacgtgggtcacctccttggcggccagttcggccatcaggcgcgcggcgtcggcggcgtcgggactggtcaggccgggatcggtcagggcgtaggtcttcggccccttctgccccaccacgcccagcgtgcccatgctggcggacttgtagccgaggctggcccagatctgacggctgaaggcggcgaccgaggtcttgccgttggtgccggtcacggccacgcaggtcctgggctgggcgccgtagaagctgcgcgcggcgatggcgtaggcgcggcggacgtcgccggaggtgaccagcaccggcgcgacctcgaccggggtgtcgaccggcgccagcacggccgccgccccttgcgccagcgcttgcggaataaaggcgcggccgtcggaggccgagcccggcagggccacgaacagggcgccggggccgaccttgcggctgtcggcggtcacgccggtgatcaccggatcggccgcgacgtcgcggcgcagcaggtcggacagtcgaagcgcgctcaacgaccgtctccctcgatgtcctgaaaggccgggaccttctcgccggtggcggtgcgatagcgatcggcccggcgctccacgcccaggaagccggcgatgcggtcggcgatgcggccgacggccggcgccgccacatagccgccggtctttggatactgcgacggctcgtccatcaggatcaggatcgaatagcgctttgcgctgaccgggccgtccgccgggaacaccgccgcgaaggagcccaccgcgtgcgatgggtcgtagcggccgcccaccagcttgttggccgagccggtcttgccgcccacccgcaggccgggcgcgtccgccagcccgcccgaaccccgcaccacgttgcggcgcagcaggtccagcatggtcagggaggtctgttccgacaccgcctggcgcggccgggcgcccggtgccccgcccttcctgaggctcaagggaatgtagcggccgccgttggtcagggcccccatggccgccgacacctgggccggcgtcgccatgatgccgtagccgaacgacagggaggcgagggtcgagttgtcccacttgcgcggcaccaccgggcgggccgattcctttagttcgatgggcgccgccgccaagaggcccagattggtgaaataggtccgcatcacgtcgggccccatctccaccgccagctgcgaggtgccgatgttggacgagtggagatagacctcctccagcgtcatgacccggttctgggcgtggaagtccttgatcttgcgcgtgccgatctggaaggcctgggaggcgtcgaacaaggtgttcatgtccgcccgcccggtgtcgatgccggcggcgacggtgaagcttttgaacaccgaacccatctcgtagtgggcggagacggcgcggttcagcgtggcgccttccgaggcgcgggcgcgctcggccgggttgaaggtcggccatgacgccatgcccagcacttcgccggtctggacatcggcgatgatgccgacggcgcccttggagccggtctcggtcgcggcgcgcgccagctcgttctccagcacgccctggacccgcaggtcgatcgaaagggggaagctctcgccgcgctgaccggcggcgcgcacctcgtcgttgaaggccagttcggcgcccgcgacgccctgcccgccggtgtcggcgtcgccgatcaggtgaaccgccgaggttcccagcggatagacgcggcgatcctcgggctcgaacgacaccccgcccagcgccagcgcatgaaccgcctcgcgctcggacggcgtgagccccgtcagcacgatcaggcggcggtcgccgtcgagcaccttgttcagccgcttggccggcaggcgcggaatggcgcggcgcagctgggtgaaggcgagacgcttgtcccagacttcggccggatcgatgtagaggccgtagtgggtgatgttggtcgccaggagctcgccgttgcggtcggtcagatcgccccgcaccagggcgtgtggattggcggccgcccacagccgtcccttgtcggcgaacagggctgcgtgggtcgcccccagagccagggcgccgaacaccaccgaaaagacgatcagcaccagaaagatgcggacgcgcgtgtcctcttccggccgcgcatcggccttggcccgctcgaacccgtgctcgagccgccacatgacctcggacagccagcgccagaagggcgacagccgatcggagacgctgggtcccggcgcggggcgatagccgcgatgatcgtggtgaacggtcattgcgcctcctcgacaagcggcgcggcgggcgcggcgtcctcgatcggagccggcgcgggtggcgcgggcgccacggcggtgtcggacagatccgccttcggcgccttcagcgccggcagggccgcctcgtccgcctggcgatgcacgtccaccggagccatgccgatctggcgcgagaggctttccaggcgcgccggttgctccaggcgggcggcctcggcgcgaagcaggcgcacgcgctggccgttctcggcgatgtcctgctccagctgggcgatgcggctgctttcccgcgccgctcccgccttggccgcatagaccgaaacgatcatcacggcgaccaggaccgcgccgatcagctcgacccagcgcacgccgcgcaccttcatctcgaacaggcgaacgagagcgtcgcggccggacggcggcagggcgttcatgcggcggcctttccatggaagcggccccaggcgggggcgtcggtgcgtacggcggcgcgcagcttggccgagcgggcgcgggaattggccagccgttcggcctcgcccgcctcgcgcgcgcccttgaaggcgagatcgaacgagggacggcgcgggtccaccgcgaccggagcatggcgggatccggccggcgcattgccggtgcgctcggtcaggaaggccttgacgatgcggtcctccagcgaatggaaggtgaccaccgccagccggccgccgggcgacagggcggcctccgccgcctccagcccgcgcgtcagctcgcccagttcgtcgttgacggctatgcgcagcgcctggaacactcgggtcgccggatggatcggcgcgccgcgacgcccgcccagcgccttttccaccacctcggccaggtccagcgtgcgggtgaacggctgttcggtgcggcggcgcaggatggcggtggcgacgcgccccgactggcgctcttcgccgtacagcttgaagatgtgggccagcggcccgtggtcccaggtgttgacgatctcggcggcggtctcgccttcatccgacatgcgcatgtccagtggcccgtcgcgcatgaaggagaagccgcgctcggcctggtccagctgcatggacgagacgccgatgtcgaacaccgctccgtccagccgctccgcattcgagccttcgaacgcctcggccaggccggagaagggcgtgcgcaccagttcgaaccgctcgggaaagtcgttggcgagggcgtcggcgtgcggctgcaccgtgggatcgcggtccagcgcaatcacgcgcgcacccgccttcaggatcgcgcgggtgtagcccccggcgccgaaggtggcgtcgatcatcacctcgccggggcggggctgaagggcctccaggacctcggcgagcagcacgggggcgtggggcgcggcgtcggtcatgcgccgcctcccgccgccagcttcatctgcgcctgcagcttcagcgcgccgacctgggcgaggcccgccttggccagggcgcgctgttcggcgcggcgcgcccgccacttgtccttgctccagatctggaagcggtcgtccaggccgacgatcatcacgctgtcgcccccgtcggcgcccaggcccgcctcttcacacagcgcctcgggcagggtgatccggccgccggcgtcgaagttcaggcgcgtctgctcgcccatcacctgccattccagcgccgaacgctcggccgagccgaacggaagggcgcggatcatctcggcgtagacggcgaacagccggtcgccgccggcctccaggcagtcagcttcgatcgatgggaagatgaagatggcgctctcggcgccattgtcggcggtgcgatagtcctgagggatcaggaggcggcgcttgccgtccagctgcttctcgtaggtcgagagaaacacgccctgcccatcggatcttccgacccgtccctgaaaccgaaaaatgcaggcgcccgagacgcgcgcctctcaccccaactcacggcggatgggatatcatgggatgaaatgggcctcaatgggattggtagccttgctttaaccatgaacggcagtgttgcgcccgatccacgccgactagatcggaacatacacagaacatgacaagtattcacagtctgtggaacagcttagtgaaggcccatcgcgcaagggttaacggcgcctcggcctgtggacagccgccggttgtgggtgagctgcacgcccatcccattcaccgagaggaaaaaagtggaaaagccagacggcctgtaagccgggttctgttccgcctcgaaaggcggcgacgatcattcctctggaccgcccattgctgagcggttctcgcgacctacccggacgtctggggcggtgaacccttgcggagcggaccccgcgcgacgtccctatttggtcttgctccaggcggggcttgccatgccgtcgacgtcgccgccgacgcggtgggctcttaccccaccctttcacccttaccggtctcgcgaggccggaggtttgctttctgtggcgctatccctcgggtcgccccgggcggaagttatccgccgcctcttcaccgtggagcccggactttcctcgacaggcgcagggcccgccgcgaccgcccggccgtctggcggggcagtagatgcgctgcccggcggatgcggtcaacatcggatgcaatccgaacccaaaggccgtatgttgcccccatgtccgatcctgcagtccgatctgcaccgcacgaaagcgaagaacagcgcgcacgccgccttgcgtgggaacgcgagcgccttgccgaggccgaaaaggacattgctgccggtcgagtgatctccggcggcgctgctctggactggttggaccggtgggcggcgggcgaagatctcgacgagcctgatctgcactgatggataccgagtacgctgtcgtcttcgccgcgcacgggcgagccgacctcctcgcggtacgtcgatggctcaatcagccaggcagcggcctcagagcgcggctgcgacttgcaaagatcagccgcgcgttgactgagctgcgttttgcgcctcatcgctggccgatcggcgaccatccgggcgtgcgggaacgtgcggtggaaggtcatcgcatcttctacagggtggacgaagtccagcgtacagtgaacgtgctgcgcgtattcggcccgttccagaaccgagcgccgtctagttcaaaacgccagtgaccgtctcgacctgcgacagctgcagcaggcccacgaggcgggcgcgcgtgtcgccgtcggccacgccgtcgacacggatgggccgccagtgccgctgaaaggcgcgcacggccatctcggtttcggcgtcgtagtcgccgcccggcgtcaggccgtagcccagccggtgcaggcctgagcgcagcaccaccaccccgaggccctggtcgccgggctgcagcaggccggtcaaggccgcgacgcgttccggcgccggctcgaaccacaggccgtgcccggcccgagccagcgtcttccatggaaagcgctcaccgggatcctgcttgcggtcaggggcgaggtcggagtgggcgatgatgcgggcgtccgggatggcccagcggctccgaatatcgccaagcagggcgcagaccgcctcgatctgcgcagccggaaagtcgcgatagccgaactcgtgccccggattgacgatctcgatccctatggaggcggcgttcatgtccgtctcgccccgccagctgccgcgcccggcatgccaggcgcggcgctcttccggaactaggcgaaagaggcggccgtcctcctcgaccatgtagtgggccgagaccttggctgagggatcgcgcagacgctcaagcgccgcatcgcccgtctgcatgccggtgtagtgaaggacgatcgcgtccggcggcgcgcgccgggcgtcgaagttcggagacggcgcctcgatcaggtccagcgccacggctcagcgcccgcgcggctcccagccgtaggcgacccaggtgccgtccaccttgcgcgcctcgatcacgccctcgggcgcggcgcggacgggcgacagcttgcggcgagcccgcaccacgaagccggccaggaacaccaccatgcccgcaaacaaggcgatcaccgcaacggctgcggcggtgaacaccgccagcaccgccccgatcgccatggcggccacggcggccagggtgctgaccagccagatcacgggcgcgaacaggccgtcggagcgacgacgacgcacgcggccggacaaggcgacgggttcggactggagcataatgatcctttcaggcgctccaaggaacgccggaaagccaatgtcggtccatcaggcccggccgtcaatgcgtcgcccggtcacggcggcgtcatgaagagacttcagggcagcggctggtcggccagcaccgaggcgcccccaacccgcatccgctcgccttcgatgcggcgcagcacgctctgcgcctgagggtccgccatgaccccgcccagcatgaccagggcgcgcgcggcctcgctctgcacgccgaacgcctccgacagcgcctcccacggcgacttctgctcggggaagcgcttgaaccgcactgactggtccgccgggatgcgggccagttccttggccttggcgacggcttccgtaaccccgcccagttggtccaccaggcctagcggcagcgcctgcgcgcccgtccacacccggccgcgcgcgatctcgcgcacgcgttccgccggcagcttgcggcccgtggagacgcgcgcgatgaagtcttcataggtgcggtccatgccggcggcgaaggccgcgcgctgcgacgggctgaacggctggctggcggagaaggcgctggcgtagtcgccgcccacgccgatctggcgggtgtcgacgccaaagcgggccagagcgtcggccagaacgaacttgccgccgaacacgccgatggagccggtcagggtcgagggttgggccacgatccagtcggcttccgaactgatccagtagccgccggacgccgcataggcgcccatggacaccaccaccggcttgccggcggcgcgcgcggcgcgcaccgccgccaggatctgttcggatgcttccggggagccgccgggcgaggagacgcggaagacgatggcctttacgtcgtcgtcctcaatggcgtcgtagatggcttcggccgtgtcgtcggactggatggaggagccgccgccaaagcttccgcccccgcgtccagtgacgatcgcgccctcgccgccgacaatggcgacggcgctgcggcccgagccctcgcgctctccgacgttgaaggcgtagtcggcgaactccacgatctcgccgcgcgcgccggcccggcgcttggcctcggcctcggcctcttcgacctggccgacccggtcgatcagacgggcgtccagcgcggcctgagccgaatagggaccggcctcgatcacgccgcgcagggcctgcggcgtcatgccccggccacgcgccgcgtcgctgacggcgccatcatagatggcggtcatccaggcggtcatggcctcgcggtgtgcgggcgtgaagtcgctctgggtaaactgattgacggcgttcttgtattcgtaccgctgctcgaactcggcatcgacgccgtatttctcgaaggcgcggcccaggaacatctcgtcggtcgagaagcccgccgcgccgaaggtcgcggtgttctgcatccacagctggtcggcggcggcgcccaccatgtagctggatacggccgtgccgaccggcatccatccctggctgtgggcgatcaccggcttgccggacgccctgaagcggcggatcgcctggctcagctcacccgccgtggcgggcgtcatgcccgtttcgggcgggcgccccagcagccccttgccgttgcggtccccgcccgcctgcgccagcacgtccaccacgcgcatcaccgaaagccccgccccgccgaagacggcgaagggattggacgacggctggtcgctgagcccctcgcggagatccagttccagcaccgtctgcgcgggcgttgcgggcttggacgaggtggccaaggccgccgtcagcagaaccaccggaacgacaacaaggaacaggatcagcccggtgaagacgccgaggaccgtcaggaagaactgcttcatggccgaaccatagagccgcaaagacagccgtcaaatgaaggcgatgtcacacaggaggcgtgcgattgccgcccccgcgcgaaatccctatatgcggcgcctgcgagcgggggcccatgccccgcgtctgccccgggaagacgaccgccatgctggtcaccctgatgaagtccaagctgcaccgcgccacagtgacccaggccgacttggactatgaaggctccatcgccatcgacatggacctgctggacgccgcgggcatctatccgcacgagcaggtcgatgtgctgaacatcaccaacggcgcccgcttcaccacctacgccatcgaggcgccgcgcggctcgcgggtgatcggcgtcaacggcgccgccgcccgcctggtgcagaagaacgacaaggtgatcgtcgtcacctacggccagccccctcaggaagaagcccgtcagtggtcgcccaacgtcgtgctgctggacgaccgcaacgagatcaagccggcggcttgagcctctcctccccgccacatggcggggaggattggacttgccgcgatcagcgcgccaggtcgtagacgccggtgacgtcgatccgtaccgtcagttcgccggcggccacgggggtggaggacatctcggccatggcggcgcgggcgtacatcaccggggggcgtggcggctggggagaatagccgccgccctcggtcaggctgcggatcgaacccagcggctggttcagcgcctgggcgtagagcgcggccttggcctgcaacgcgcgcaccgccagctgacgcgcctcgttctcggccgccgtcgggtccttaaggccgaagccgatgccgtcgatctggttgacgccggcggctaccacggcgtcggcggtggtcccgacgcgttccaggtcgttgatggtcaccgtgacccggttgacggcctgatagccccgcaggcgcggcggctggttctcctgatagtcgtactgcgcctgcaggttcaggccagaggtctggacgtcgcgctcattgatcccggcgcggcgcagggcggccatgacgcgcgtcatctgctcggcgttctgctgcatggcggcctgggctgtcggggcctcggtctgcacgccgaaggtgatggtcgccatgtccggcgcggtcttgacctcgccataggccgacaggttcagcgacggccgctcggtcaccgcctggatggtcaggggcgcgccgccgatcggctgcgactgggcctgcgcagtggcggcgatagccgtggcggccagaagggcgccgccaagcgtcaaggcgcgggaggtgcgggtcatgggaggtctccttcggatcgagcggcgaaggccgcgcgtcatgcggcgacctttgccattgttcatctgaatgaacgcagcaggcccgctgtcaggttccgttcatcgcgcggtgttggccgcatcgcttggcaagctgcgcccgcgcctgctaggcgtttccgcccgcgaacggcggcgggcgcgtagctcaatggttagagccgaccgctcataacggtctggttgggggttcgagtccctccgcgcctaccacccctcgcctcccgttccgaaaggcgcatccatgaagccggacctgacaaagcggctgctgctgggggtggcgatccttggcatcgtgctggcggtgttcggctcgggggtgatcgtgctgcgcgcctttcaggccggcctgtagagagagcgtttccatgagctacgtcgcccgcgacgaccgccccgccgacaaggccgatcgctatgccgaagtcgaggccgagatcctggcggttctggagggcgagccgaacctgaccgcgcgcatggccaccgtcgcctcaatgctggccgacgccttcgagcattatttctggaccggcttctacgtcacggtgccggacaaggcggacgagctggtggtcggtccctatcagggcacgctgggctgcctgcgcatcccgttcgggcggggcgtctgcggcgccgccgcgcgtacgcgccagacccaactggtcgaggacgtccacgcctttcccggccacatcgcctgcgacagccgctccgaaagcgaaatcgtggtgccggtgctggacacctcgggcgacctgatcgccgtgctggacgtggacgccaccacgaaagccgctttcgatgcggtggatcaggcggcgctggaacggttgatggccaaggtcttcgccggcggctgacgccaggcgagcgggagggatgcggatggacggacgggtcgttgcggtcacgggcgggcacggcgtgctgggtcgtgcggtggtgcaggcggcgctggcgcgcggctggcgcgtcgccgtcatcgaccacgccatgggccattcggcgccggacggcgcgctggagatcggcggcgtcgacctgaccgaccccgcccaggcggacgccgccgtgggtcgcgtggtcgagcggttcggccgcctggacgccgtgctcaatatcgcaggcggctttgtctggcagacggcggacgacgcggcgcccgcctgggagcggatgttcgcgcttaacctgtccaccgcgctccacgccagtcgcgccgccctgccgcatctgaaggcgtcggacgccggtcgcatcgtcaatgtcggctcggccgccgcgctgaaggcgggcgccggcatgggggcgtacggcgcctccaaggcggcggtgcacgccctgacgcagagcctggccgaggagctgaaaacgaccgccgtcaccgtcaacgccgtcctgccctccatcatcgacacgccggccaaccgcgccgacatgcgggacgccgatccggcccagtgggtcgcgccggccgatctcgcggcggtgatcctctttctcgcctcgcccgaaagccgagcgatgaccggcgcgctggttccggtgacgggtcgcgtctgatgcgcgcccgcagcgtcctgttcctgccggcctccaatacgcgcgcggtggaaaaggcgcgcaccctgccctgcgatgtcgccgtgctggacctggaggacgcggtcgcaccccaagccaaggtcgaggcgcgccgggcggccgtggacgctctacgttcaggaggcttcgcgccgcgcctgggcgtgcgcatcaatgggctggacaccgaatggggcgccgacgacctgcgcgccgtggccgacgcgggcgccgctctggtgatcgcgcccaaggtcgaaagcgtcgccgtggtccacgacctgtcttacggcctagctgaaggcgccgccctgtgggccatgatcgagacgcccgccgccgtgctgaggctggacgccatcgccggggcgggggccgcgctgagcggcctgatgttcggcgtcaacgacctgtttaaggcgctgggctgcggcgaggcggccgaccgcgaaccagtcaagccgtggctggcggcggccggggccgccgcccccgcccctggtcttctggccgtcgatggcgtgttcaaccgcatcgacgatgcggacggcttcgatgtcgaggccgctcagggccggctctacggcttcgacggcaagagcctgatccacccgtcgcagatcgagccggcgaaccgcgccttttctcccaccgaggccgagatcgcccacgcccgcgccgtcatcgccgccttctccacgcccgaggcggagggtcgcggcgccatccagatcgacggccgcatggtcgaacgcctgcacctcgatatcgcaaaggccgcgctggccaaggcggatgaggcttgacgtgaccccgcccgccgcctcgccttccgctcccacgcctgcctgggtctgcgcgcccggcgtgctgaaggtcccgttccttcaggccttcctgccggaatacgacctgcgtcgcctgccgggcgcggagattgaggcggttctggggtggggcatgaagccctcggccgcggccggtcggcgctgggcggcgaagcatgatcgcccctatgtcgcactggaggacggctttctgcgctcgatcggcctgggcgaggcgggcgccgccagcgtcagcctgatcgtcgacgacgtcggagtctattacgacgcaacccggccgagccgcctggagcggctgatcgcggacgcgccgaactggtgcgacaccgcggtggaagcgcgcgcccgcggcctgatcgaccgcatcgtcgcttcgggcctgtccaagaccaacatgggcgggccgcttgacgcttcggtgcttcagccgcggcgccgcatcctgctggtggaccagacgctgggcgacgcctccatcgcctgcggcctcgcctccacccaaagcttcgccgagatggtcgccgccgcgcggcgggacgagtccgacgcccagctgatcgtcaagcgccacccggccgtcgccgcgggccgcaagcagggctgcatcgcggaagcggacctgcacggcgtcaccctgatcgacgctgacgttcgggcggcggacctgctccgagcggtggacgcggtctggtgcataacctccgcgctcgggttcgaggcgctgctgcggggtttgcccgtccgctgcttcggcgcgcccttctactccggctggggcctgacgcaggatgcggtcgacaccgggcggcgaggagcctcgcgcaccatcgaacaggtcgcggccgccgccttgatcgcctacacccgctacgtcgatccggtcacaggccggcgctgcgaggcggaacaggcgctggatcggctgatcgcctttcgagatcgggccgagcgtctggcgggatcgtggtccgccgtcggcttcgcccccgccaagcggccgcaggtacgccgcctgctgaacggccccaagacccgcctgcgctacttcatgtcgccgcagcgagcggcccggcacgcgagcgaaagggacggccggctgatctggtgggcgggaaaggagagcgcggccacgcgcgaagcggccgagtgcttcgacggcccgacggtccggatggaggacggctttatccgctcgcgcggcctgggttcggatttcgtcggtgcgctgtccgtcgccctggacgaccagggtgtctactatgacccgcgccgcccctctcgcctcgagaccctgatcgagacgacggagccagacgcggatgagctggcccgcgccgccgccctgcgcgcccgcgtggtcgaggccggcctgtccaaatacaacatccgtggagaaccacccgccggctggccgacggaccggccggtgctgctggttgtgggtcaggtggagaacgacaagtcgatcctgctgggctgcgaaccggacctccgcaccaattccgcgctggtcgaggcggcgcggcgcgaccatccggacgcctttctggtctatcgcaaccatcccgacgtgctggcgggcaaccggccgggccggctggatcatgcggcgctggaggcggtggacgcttcgggcgacggcttggacatcatcgattgcctgaacgcctgcagccgcgtcgccaccctcacatctttgacggggttcgaagcgctgatgcggggcaaggcggtgtcgacctacggccggcccttctacgccggctggggcctgacggatgatcggcttgcgttcgagcgccgcagccgccgcgccacggtgaatcacctcgttctagccgccctgatccgctatccgctctacatcacgccggacgggtggccgtgcgaggcggaggacctggtggaggccctgatcgccgcccgcgaccgtcccgttccgcctccgccgcgcggtcaggtgcgccgctgggcgaccggcgtgctggccagcctcgaccggcgtcctccgccgtcctattgacgcgatcgaagacgaaatatctccaaggccgcgagaccccgcaggtcgagcgacaggaacccacttcctcaagcagcgaggcgccgcgcgccgagcgataggaaaacaacaaagtgccccacgccgtcatcgccgcgaccggcctattcacccccgaacagtcggtctccaacgccgaactggtcgaaagctacaacgcctgggccgagcgctggaacgccgcccattcggacgcgatcgcggcgggcgagctggaggccaagacgccatcctcggccgagttcatcgaaaaggcgtccggcatcaagagccgctttgtcatggacaaggccggcgtgatcgaccccgagcgcatggcgccccgtatcgcagagcgcggcaatgacgagctgtcggtcatggccgagatggccgtggccgccgcccgccaggcgattgcggcctggggcaagccggtcagcgagatcggcgcggtcttgtgcgccgcctccaacatgccgcgcccctatccggcgcttgcggtggagatccagcaggcgctggagatcgacggcttcgccttcgacatgaacgtggcctgctcctcggccacattcggcatcaagacggcggcggacttcatcggcggcggctcggtcaaggccgtgctgatggtgaaccccgagatctgctcggcccacctgaacttcaccgaccgcgacagccacttcatcttcggagacgtggccaccgccgtgatcgtggagtcgtccgacaccgccggcccgggcggttgggacatcctgggcacccggctgaagacggtgttctccaacaacatccgcaacaacttcggctttctgaaccgtccgggccgcgacaccgaccagctggacgcgaccctcgccgacaccacccgccagaacgacaagctgttcgtccagcagggccgcaaggtgttcaaggatgtggtgccgatggtgtcggagatgatcgtagatcacgccggcgaactgggccttgacccgcacgggctgaagcgcctgtggctgcaccaggccaacatcaacatgaaccagctgatcggcaaaaaggtgctgggccgcgagccgacgtcggacgagaacgtcatcatcctggacgaatacgccaacacctcctcggccgggtcgatcatcgccttccacctgcaccacgaaggcttcaagcctgggaacaccggactgatctgctcgttcggcgccggctactccgccgggacggtgttcgtcaggaagcgcggttagacgcgcggagtcagcagggcccagtccaggctccacaggccgggaccctgcaccatcagccagaacaggatggtcatcagcagggtctcgggcaggtccagatagctggacagccgatagccgaggctggtcccctccaccgacttgcgcgtgaccgtcagcaaggcgaccaggctgatgatgaacagcacggcggccgcgagcgtggtcatcaggcccaggatcaacagggcgccgcccacgaactcgcacaccgagacgaagcgggccgttttgcgcggcgcggcgatcccggcctcgaccatggtcttctgcatcttttcggcgctctgggccgagaacagcttgtagaagccggacaggaagaacatcccgccgaccacgacccgcgtcacgaacggtgcggcctccatcaggtgcggccaacccagggcgacgccgcgatacagctcgatcatctcgatcctccagcaagcgccgccgtaatgatcgagcggcccgtgagttgcgaaacctgacaaacgagcgccgcaattcaccacaatcgatttggttccattcacatctgtgtggctacgcttgaatccgtcgagaagatttgcgaggcgtgaggggtcgagaacagggagttcctggatggctcagacgagaacaccacgcagcggactggacagtctggcgcgcgacatcgccctggtgctggagcgcatggggggatcggcgcaccagaccgtggtcatcgactgcgtcgccgccttgaagcgacaacgcggcgagcaggtgactccggacctcaagacccgcatcatcgaagtcttcgaacactaccgcgacctgttcttccgccccttcggcgaaggctccaaccgctgggcgctggcgggcgacttcgcctgacgcccctgccgacgtgaaaacggcgcgcctcgcgggaggcgcgccgtttcgtcgtctgagatcaaagacgatcagaacttgcgcacgaagctcaggccgtagctgtcgttctcgccgtccgtgccgttgaagtcgcggcgcgtccaatcggcccgcacgccgttggcgccgtccaccagataggtgacgcccgcgccgtagttccagctgtccgagccgatgtccgacgatccgccggccagctcgcgcttcagctcggtgtggccgtagccggtgcgcacaaagacttcgaggttgttggacaccgggtacttgccgacgatgtagcctgcggcgtcccactcgtgctcgatcttgccgtcgacgccggccacgttgatgtcgtggtccttgacgcccaccgaggcttcggtctccagcgcgatgaagcggttcaggttcacgcccagtcggcccgtcaccgcgcccgtgctggtgtcgtcaagatgagtgtatccaaggttgccgtatccccgaggttccgaagccgactgcgccagtgcaggcgcggcgatagcggagatggcgacagcagcgataagaatgttacgcattgtttctattaactcctagatgcggcgacctgtgttgatcgccaaccccatccagcgagtgcataaatgatagcccgcatcgggcgttccagagcccaaggtgacttgcgttcagctgtgcacgtagggacacatacatcgttccgccaactgtgacgaagagatgacggtcgcggcgcagccccatgcaaaagggcggctccgaagagccgccctttgctgaaccgcatctctgaagaggcttagcgatccttttcgcgttcttcggacaaggcggcttgggcggcggccaggcgtgcgatgggcacgcggtagggcgagcagctgacgtaatccagccccacctgttcgcagaaggcgatggaggacggatcgccaccatgctcgccgcagatgccgagcttgacgtccgcccgctcggcgcgcccgcgctctgcggcgatgcggatcaggtcgccgacgccgtcctggtccaggcggacaaaggggtcggtctcgaagatgcccttgtccatataggcctgcaggaaccgcccggagtcgtctctggagatgccgaaggtcgtctgcgtcaagtcgttggtgccgaacgagaagaattgcgcgtgctgggccaggtcgccggcgcgaagggccgcgcgcggcagctcgatcatggtgccgaccagatagtcgacgctgtcgccggcctcctcgaacaccgccttggcggtgcggtcggtcagctcgcgtaggaacttcatctccagccccagcgcgaccagcgggtgcatgatctccggcgtcggagcctggccggacgtggtcttcacctccagcgccgcctccaggatggcgcgcacctgcatctcgtagatttcagggtaggcgacgcccagccggcagccgcggtggcccagcatggggttggtctcgtgcagctcgcgcgcccgccgcttcagcttgtcggcgtcgatgccggaggaagcggccagggcgtcgatgtcctcgtccgtgtgcgggatgaactcgtgcagcggcggatcgagcaggcgcacggtgaccggcaggccggccatgatggtgaacagctcgacgaagtcccccttctggaacggcgcgatcttggccaaggccgtgcggcggcccgcctcgtcgtccgccaggatcatctcgcgcacggccgcgatgcgggtgtcgtcaaagaacatatgctcggtgcggcacaggccgatgccctcggcgccgaagccgcgcgcggtgcgggcgtccagcggcgtctcggcgttggcgcggaccttgaggcggcgcacgccgtcggcccagcccatcagggtctggaagtcgccggtcagctccggctcgatcatcggcacggcgccgtccagcacctcgcccttggagccgtcgatggtgaccacgtcgccagccgagaaggtgcgtccgcgcgcggtgaaggtccccgccgcctcgtcgatgtggatctcgccggcgccggacacgcagggacgccccatgccgcgcgccaccacggcggcgtggctggtcatgccgccgcgcgcggtgacgacgccgcgcgccgcgtgcatgccgtggatgtcctctgggctggtctcctcgcgcaccaggatcacggcgtcgccggcctgggccatacactcggcctggtcggcgtcgaacaccaccttgccggtcgcggcgcccggagaggccggcaggcccgccgcgatcacggtgcgcggcgcgtcgggatcaagcgtcgggtgcagcagttggtccagcgccgccggctcgacgcggctgacggcctcctgctgagagatcacgccctcgctggcgaggtccacggcgaccttcagcgccgacttggcggtgcgcttgccgttgcgggtctgcagcatccacagccggccctgctccaccgtgaactcgatgtcctgcatgtcgcggtagtggctctccagcgtgccgaccacctcgacgaactggccgaacacctccggcatcgcctcctccatggaaggcgcggtctcgcccatctcctcgcggccgatcttggtcaagctctgcggggtgcggatgccggcgaccacgtcctcgccctgcgcgttgatcaggaactcgccatacagccgcgcttcgcccgtcgaagggttgcgggtgaaggcgacgccggtggccgaggtctcgcccatgttgccgaacaccatggactggacgttgaccgccgtgccccagctttcggggatgtcgtgcatgcggcggtagaacttcgcccggtcgttcatccagctttcgaacaccgcgccgaccgcgccccacagctggtcctgcggatcctgcggaaaggcttggcccagttcgcgctccaccacctgcttgtagtcctcgaccacacgctcccagtcggcggcctgcaggtcggtgtcgaccgtgacgccgagacggtccttgtgctggtccagcacctcttcgaaatcgtcgtggctgaggcccagcacgacgttggagtacatggtgatgaagcggcgatagctgtcgaaggcgaagcggcggtcgccggacagacgcgccagcccctcaaccgtctggtcgttgaggccgaggttcagcaccgtgtccatcatgcccggcatggacgcgcgggcgccggagcgcaccgagaccagcagcggattgtcgacgtcgccgaaggtcttgccgaccacgccctcgaccttggccagcgcggtcttcacctgcgcctccagatcggcgggataggtctcgccgtgggcgtagtaccaggtgcagacctcggtggtgacggtgaagcccggcggcaccggcaagcccaacgaggacatctcggccaggttggcgcccttgccgccgagaagattcttcatcgacgcgtcgccgtcggcggagcctccgccgaagccgtaaacccactgagtcatgttcggtaagcccctgagccgtgttctgatcggcgggggtggccccgctcgggatgcggcatgactagcgcgcatgcgacagcttgaccatgccgcatgtaacaatacgtgagcagccgaacaggttcccctcaccggcgggggcggcgggccgccgcaaagaaaaaggccggctcgcgccggccttttccatcagctgtccaggaaggaccgcagcttgcggctgcggctggggtgcttgagcttcctcagcgccttggcctcgatctggcggatacgttcgcgcgtcaccgagaactgctgaccgacctcttcgagggtatggtcggtgttcatgccgatgccgaaacgcatgcgcagcacccgttcctcgcgcggcgtcagcgacgccagcacgcgggtggtggtctcgcgcaggttggactggatggcggcgtcgatcggcaggacggcgttcttgtcctcgatgaagtcgcccaggtggctgtcttcctcgtcgccgatcggtgtctcgaggctgatcggctccttggcgatcttcaggaccttgcggaccttctccagcggcatggccagcttctcggccaactcttccggagtcggctcgcggccgatctcgtgcagcatctggcggctggtgcggacaatcttgttgatcgtctcgatcatgtgcaccgggatgcggatggtgcgcgcctggtcggcgatcgagcgggtgatcgcctgacggatccaccaggtggcgtaggtcgagaacttgtacccgcgacggtactcgaacttgtccaccgccttcatcaagccgatgttgccctcctggatcaggtccaggaactgcaggccgcgattggtgtatttcttggcgatggagatcacaaggcgcaggttggcctcgaccatctccttcttggcctgacgggcttcacgctcgcccttctgcacggtctggacgatgcggcggtagtcgtcgatcggcaggccggcctcggttgcgaccgcggcgatgtccgagcggatcagggcgatctggccggattcgttttcgctgaacttggtccagcgcacgcccatctccttgacgcgctcgctccaggtcgggtcgagttcggcgccgaagtaggccttcaggaactcgggccgggagatgccgtaactgtcggcgagccgcagcaggcgcccctccaggccgatcagccgcttgttgatggcgtaaagctgctcaaccagcgcctcgatgcggttgttgttcagcttcatcgtcttcaggcggtccgagatcgccgtggtcagcgtctcataggccttctggtccttggccgagagctgctcgcccttcagccggctttcgaccagcttgtcctgcagcttgcggaagccctcaaagtcggcggcgatggcgttcagcacctccatcacgccgtcgcgcagctcggcctccagcgccgagatcgacatgccgccgccgtcgtcgaagtcgtcgtcgtcctcgtcgtcgctttccggcttggcctcggcgggcgcggcctcctcctcggtctcctcgccttcaggctgggcggcgcccggcacggaggaggggttcagcacgccataggtggcgtcaaggtcgatgacctcgcgcagcaggatgcggttattctccagttcgtcgcgccacaccatgatggcctcgaacgtcagggcgctttcgcacagccccgagatcatggcgtcgcggccggcctcgatgcgcttggcgatggcgatctcgccctcgcggctgagcagctccaccgagcccatctcgcgcagatacatgcgcaccgggtcgtcggtgcggtcataagcggccttggcgggcgtctcggcgacggcggtgccggcggcggcggccacttcggtcgactgcgcctcctgcgcgtcttcctcggcctcgacgacgttgacgcccatctcggacagcatggccaaggtgtcctcgatcgcgtcgggggtcacctcttcgctggggagaaccttgttcagctcctccatcgtgacatagccgcgcgccttggcctgcttgatgaacttcttgacgccggcgtcggtcagatcgagcaggggcccgtcggtcgaaacctcggcgtcctgcgtctcggtctgagtgctcattcagtgtctctccggccagcgggggtgatcaggccccatggcaaaaatacaacgcctgccgacttcgttgcttacgaggtcgaactgttatcccaaatcgttccggtcttgatggcccggcgcaaggcgtcgcgctccgccttcacgcgcgcgaaggccgaggcgtcgaagaccaggtgggcctccgacttcgctgacgccagcgcctgctccaacgccgccacgcgggttgaggcatcaagcgcctgcgaccaccggatccgcgcctcggcgaggggcttgtcggaagccaggaatggcgcgccggacttcgccgccgccttctcgacctcgcgcactaaaacatcgtgacccgattgcgccagatggcgacgcatggccgcagagtcaagcggaacgcccgacaaccgtaagcgcaccaactcctgcgccagcccgtccagcgccggatcgccgaagccgtgggcggcgacagcctcgaggtgatcgtccattcgctcgggatcgtcgatcgcgccgtgggcgagggcggccggcaccggctcgatcgaccggctgagcgactgcatggccgcggcgccttcggcggtctggccctgcatgggcggcggaccgaaacgtccacgcccctgccccggcgtccacgggcgggcgcccgcgcgagggacactacgaggaaacagggcgtcgaagcggtcgaacaggtcgcggcggtactgctcggccaggtccttgtcctgaatggcggcggcggcctggcgcaggcggcctttcagcccggcccggcgttcgggcgtgtccagcggctcgacctcgacctcgcggcgaaacagcacctcggcgaaggcgcgggtgtcgctcagcgcttggcgaagcgccggcgcgcccctgtcgcgcaggatgtcgtccgggtcctgtccgccttccagcagggcgaagcggaaggatcggccggatttcagtagcggcaggccgcgttcgatggcgcgataggcggctctgagccccgccgcgtcgccgtcgaagcacagtaccggctcgtgcgacacgcgccacagccgctccatctgctcctccgtcagcgccgtgcccattggggcgacggcggggaggcccgcgcgctggcaggcgatcacgtccatgtagccttcgaccacgatgatcgactggtcggtcttgctttcggcgcccaaaatgcgccgcgcctcgggcaggccgtagagggtcgcgcccttgtggaagagcgggctctccgggccattcagatatttggcgcggtcgtccgggttcatggcccggccgccgaacgagacgatccgcccgcgcgcgtccagaatggggaacatcagccggtcgcggaagcggtcgtacggctggccgccgccgtccggcgcgatcagcatccccgcctcgaccagctccgccgggcgtgcgccgcgctggaccagcgcctgcttcagcccctcgcggtcgttgggcgcatagcccaggccgaaccgctcccactgatcctcgggcaggccgcgcctttccagatattcgcgcgccgccttgccgggagaccgccgcaggttggccgcgaaccacttctgcgccaggtccatccagtcggacaggccctgcttcttggcctcgcgttcggccgcctgcggatcctcggccggcaaggccaggcccgcctcgcccgccagcctctgcaccgcctccacaaaggacaggcgctcggtctcctgcaggaaggagatgatgtcgccgtgcttgccggacgagaagtcgtgaaagaagcccttgtcgtcgttgacgaagaacgacggcgacttttccttggagaagggcgacagcccgacgaactcgcgcccctgacgcttgagcttcaccgtccgcccgatcacgtcggacgggcgaaggcgcgccttcagttcatcgatgaagcgttcgtcgaagcgcacgcgcggtgtttatcgcagcgaaggcgtttggtcgatgcggagaggaacaggccccgcccttgccttcccctgcgtcgctgagcacaagctacgccgcgatgacatatccccgcctcttcgccgccctagcgctcctggtcgccgttctggggaccggcgcctgccaaaccttgccgagggacagcttcacggccgagcacctggcccaggccagcccgccctaccgctacgacttcaacgaccgcgcgtcgctggcgcggttcgaggcggaccgcaccagaatcctcagcgggtcggacagcgacttcgaccttctggcgttgtcaggcggcggcgcaaacggagcgttcggcgcgggcgtggtgatcggctggcgcgaccggcccgagttcgacatcgtcacgggcgtatccacgggcgccctgatcgcaccgttcgtgttcgggggacatcgcttcgacgccgcgctggagcgggcttatacgtccggccaggcggacggcctgctgaaacctcgcgggctgctggcgttgttcctgccgggtgtgttcgacccccagccgttgcgtgacctggtgctgaacaacgtcaccgacgaactgatccgcgcggtggcggccgagcacgccaagggccggcgcctgtatgtcgccaccaccagcctggacacccagacgcagatcgtctgggacatgggtgcgctggccagccgagcagatgcgcagtcgcgcctgctgttcgtcaacgtgctgatcgcctcggccagcatccccggcgctttcccgcccgtgcccctgacctttggcccggaaggcgacaccgtcagcgagctgcacgtggacggcggcgcgaccgccaacttccttgtggcgcctcagcaggtcatgatcgcccaaaccgcccgccctgcgccggaacagaacggacgtctgtgggtcctgatcaacggctcccccaacgccgtgttcaaggtggccacgatcagcggcgcacgcattgcggagcgcagcttcgacaccgtgctgaaggccatcacccgggcggacctcgccaatgtcgcgcagttcgctcgcgccaacagcctcgaacttcaggtcgccatgctgaaggatcccgaagacgacgacgccctagacttcagccgcgagaacatggcgcggctgttcgccatgggacgagccgctcagggccaggatgaggcgttcgagaccatcgtgtcggcggagggcggccttcgcggacagccggccggcgctcctggcgtgaatacgggtcaggcctggtagtcgccgggcgccgatcaggcggcctgtccgaacctcccccgaagtttgaacaggccgccgcatcgcggatcgggcgcctgtcgccccggcgtcccccgacacctgggctaacgcgttcctaacgcctcgcggacgctcatctggcgcaagcttgccgaggttgtcgagcgaaggttacggcacagctgtcgaaacgtggcgatactgtgtctttttggctaccgttcgccgaacggaacaaccttgttttgcgcatcatggccgatgtcggcggaaccgagataggcgacgcccgagcgcaggcaccagtatctggcgatctcttcgggcgtctggccgaagtcgggatcgttgggagtgacatccgacacgcggccgaggcggatgcccgccacgcgccggatcgaggcttggccggtcagatggaacatcatccggtcgacgcggtacagcgcctccgacacctcctccagcatcaggacgtggccggagaggtcgggctcaagcgcggttcccaccagttgatccaggatggtcaggttgaaggcgacggcggggcggggatcggcgtgcagcgacggctcccaaccgttcgcctcgccggtggtcagccagtccagcgcgcgccggcccgtgtcgtcatggcgcagggcgtcggacgccatcggcccatgcgccagatgtcgaaatccggccctgtacatgcccgccagaaggctgcccgcatccgaatagccgagaaagcgcttggccctggccacgtcgttcagccggggcagcacggcctcggcgatccggcaggagccgtagccgccgcgcgcgaaccagacggcgtcgatgcgcggatcgttggcgaactcgacaaaggcttcggcgcgggttcggtcgtctccggcgaagtggccgtgcttcagcaggcaggcggggtggaacaccagggcgatcgagcgatcgggtacgacctgctccatccatgcctcgatcgcctgcatgcgatcgaggctgaagcgggagctcgcgcacaccacgccgatcttgaagggggcgctcttcatggatggttcctcgcggttcgcgtgctagtcagccgccctgagcgccctgcctttccggtttccgttccatgaatcaagacagctcctacttcttctgcggcgtcggcggctcgggaatgctgccgctggccatgatcgtgcaggcgtcgggcgcccgtatcgagggctccgaccgcgcgctggaccagggccgcacgcccgagaagttcgactggctgcgcgggcacggcgtggtgctgcacccgcaggacggctcaggcgtttcggcggaccagatcgttgtggcgaccggcgcggtcgaggacacggtgccggacatcgccgcggcgcggcgcgcgggcgcaaccgtgttgacgcgccccgaactgctgagccgcctgttcaacgccgcagaaacctccgtcggcgtggcgggcaccagcggcaagtccaccatcaccggcatgatcgcctggatcctggatcagacgggtcgtcgccccacggtcatgaacggcgcggtgatgaagaacttcgccgacgccgagcatccgttcgccagcgccctgatcggcgatccgaccctgttcgtggcggaggtggacgaaagcgacggctccatcgcccgctacgatccgacggtggcggtggtgtccaacatttcgctggatcacaagtcgatggaggagttgcgcgacctgttcggcggctttgcgggacgggcgaaaaccgccgtgctgaaccgtgacaacccggagactcaggcgctcgcccagatgctcccgcccgatcgggtgatcaccttctcgctgggcgaggaggcgacgctgtcggcgcatgacctgcagccgctggcgcacggaatgcgattccgcctgatcgagggctggaccgagcacgatgtggaactggcgacgcccggcgcacacaacgtcgccaacgccctggccgccataggggccgtgcaggcgctgggcgtcccgacggccgaggcggtcgtggccctcaaaaccttcgccggcatccgccgccgcatggaggtggtggggaccgcaggcggcgtcaccgtcatcgatgatttcgcccacaacccggacaagatcgccgccacgctgaagacgctgcacgccttcgacggtcggctgctgatcctgttccagccgcatggcttcggcccgctgaagctgatgaaggacgaattcatcgacggcttcgctggcctgctgcgccctgacgacatcctgctgatgcccgagccggtctactatggcggcaccaccgaccgcagcgggtcgtcgcaggacatcgtctcgggcgtgcgcgccgccggccgtcaggccgaggctctgccggatcgggcggcctgcggtcagcggctgctggaactggcacaggccggcgaccggatcgtggtcatgggcgcccgcgatgacaccttgtcgaccttcgccggtgcgcttctggagcaactgtccgaaaaactcggctaaggcggcgaaccgacgagcgacatctgtattgtagcggccgatgttgcagcttccccctccccccgccccgcccgttcagctcgaggaggtggtggtcaccgccgcccgtctgccgcccgccgacgccgacgccgccttttcggtgatccggctggacgagcagcttttgggacgctcgacccggctggacgaggcgctgcgcaccgtgccggccgtgtccttgttcaggcgcaccaccagcctgtcggccaatccgaccacccaaggcatctcgctgcgcgccatcgcgccgtcaggcgcgggacggaccctggtcacgctggacggcgtgccggtcaacgatccgttcggcggctgggtgatctggtcgcaggttccgaccgagtcgctggaaagcctggacatcgtgcgaggtgcggggtccggcccctatggcgcgggggccctgaccggaaccatcctgctgcgcgagcgagagcgcggcgcggtgctggacgcctcggtgctggagcgcggcggcgcgcggctggcgggttcgggctctcggcaggtgggcgcggtgaacctgacgggttcggcgctctacgagaccagcgacggctatgtgcccgtgcgcggtccggccgccggcgccgccgacaccccgctcgatctgcgcacccgcagcgcctctgtccgcgccgacgtgccggtgggaaccgccaacctgtctctgcgcgccgccgcctatgacgaggaacgcggctcggggctgggcgacagccgctccaccgccgaaggccatgtgctgagcgccaccgccgcccgggcgccgacggacggcggctatggctggcggctgcaggcgtggcggcgcgagagcaacttctccaacaccaccgccacggcctcgaccgatcggtcgaccacgacactggtcaacgaccagtaccgcacccccgcgaccggctggggcctgaacgcggccctgcgacgcggtgcgcaggacttcggcggcggacagcttcagtgggaggtcggcgccgacggccgcttcaacgaaggcgagaccaacgagcgcttcggcctggccttcacgccgcgcaaccggcgcgcgggcggcgagacctcggtcgcgggcggttatgtagacggatcgtggaccgggggcgactggctcgtcgcgggcgggctgcggctggaccgatgggagaacgagggcggctttcgcgaggagtacaccctcgccactggcgtcgtgacgctggacgaggtcgaagaggcgcgctccggcgaggtggtcagcgcgcgtctggccgtccagcgcgatctgggcgacggctatgcggcgcggctcgcgggctattccggcttccggcccgccacgctgaacgaactccaccggcccttccgcgtcggcgacgacgtcacggaggccaacgccgggctggagccggaatcgctgcgtgggatcgaagcgggcctggccttcgacgaccgcgcgggcctgacctggggcgcgaccctgttctggaacgagatcgaagacgccatcgtcaacgtcacggtgggccaaggccccgcgaccttcccccgcgccggcttcatcccggccggcggcgtgctgcgccagcgccggaacgccggaaccatcgaggcctggggcgtggagctgaacggctcggcgtcggtctccgagcggctgtcgctcatggccgcggtgtcctggacggacgccgaggtcgacggcggatcggcggcgccgcagttgaccggcctgcacccggctcaggcgccggaatggagcgcgacggccggcgtcgactggcgcgcgaccgatcggctgaccctgatcgcggccgcccgctatgagtccgaccggtacgacgacgatctgaacagccgggtgctggaagccgccgtcacgctggatgcgcgggcggaatgggcggtgaacgaccgcgccctggtctatgtcgcgctggacaacgtgacggacgaggatgtcgaggtatcggaaaccgggctcgggatcgccggctatggtccgccgcgcaccctcagcgcggggctgcgtctgacctactgagcggctgggacagggcggcgcaatcgccgctattgaaaacggttcgcaacaatggcacagccgtcggcgtgaccgatctcgccgctccccgcccgccggaacgcgccgccacgtcccgcgcggcggtcaacgcgcgtcggtcgttctggctgaagcagttgcaccagtggcactggatctcggcggcggtcagcctggtcggcatgatcctgttcgccgtcaccggcgtcaccctgaaccatgcggcgtcgatcccggccgaacctgtcgtcagcgaacagaccgccgtcctgcccgcgccgctgctgcagcggctggagacctttccggccgagaccacggaccccgtacccgatgcggtggcgcgctgggcctccgacgccctggacgccgagatcgccggccgcgccagcgaaaccacgccggaggaaatctatgtcgccctggccatgccgggcggcgacggctgggtcaccatcgaccgcgagacgggcgaggcgctgcgggaaaagaccacgcgcggctggatcgcctacctcaacgacctgcacaagggccgcaacgccggcgcggtctggttctggttcatcgacgtgttcgcggtcgcctgcgtgatcttcgcggtcaccggcctggcgctgctgtggctgcacgcacgcggccgaccctcgacctggccgatcgtgggcctcggcctgctgatccccgtcgtcatagcccttctgttcatccactgacgagttcgcccatgcgcctgcttcccatcgtcgtcaccaccgcagggctcgccgccgcagcccccgccatggccgcggacatctccgtggccgtggagttgccgcgcatcgccacagcctcctaccaccgcccctatgtcgccatctgggtcgagaagcccgaccagacggcggtgcagaccctggccgtgtggtatcagcagacccgcaacagcgagggcgacggcaaggactggctcaaggacctgcgcacctggtggcgcaagggcgggcgcgccatgaccctgccggccgacgggatctccggggccacgcgcgccgctggacgccagtcgatcaccgtgcccgcggcgcgtctgcgggggctccagcccggccagtacaccatggtggtcgaggccgcgcgcgaactgggcggccgtgaggtggtgcgcgtgcccttccgctggggcgcggccaacacggccaacgcctccggctcgtccgaactcggcgccgtgcgcgtcaccgtctctcgctaaggacccgcaaccatgaagaagaccctggcccttctgtcgctcgccgccgccctcgccgccccgctcagcgcccaggcgcaccgcgcctggctggcccccacctccaccagcctgtcgggaacggacgcctgggtcggcttcgacgccggcatgtccaacggcgtcttcattcccgatcacgccgcgatgcggctggacaatctggtggtcactgcgcccgacggctcaaccctccagcccgagcacatgatgcagggccagtaccgctccacctttgacgtgcacctgacgcagaacggcacctacaagatcgccaacgtcggatcgggcctgacggccagctacatgctgggtggagagcgcaagcgctggcgcggtccggcgagcgacttccccgccgccctgcccgccggcgcgacagaggtgcaggcgaggcgcaacaacagccgcgtcgagacctttgtcaccctgaatgcgcccaacgagaccgtgttcaagaccaccggcgaggggctggagatggttccggtcacccaccccaacgacctcgcggctggcgaggccgcgacctttaaactgctgcgcgacggccagccggcggcggacctcgaggtcacggtggcgcgcggcggcctgcgctatcgcaacgcgccggaggagatgacgatcaggaccggcgcggacggcgccttcaccgtcacctggccggaagccggcatgtactggatgaacgcggcggtgcgcacggaggcgcagggcgacaccctggcctccaacacctcctacgtcggtgtggtcgaggttctgccctgacccgagcttcgaaagccgcaccgcctgtcgtcggcatcggcggcgatgtaacgcccgaccgggcgggcaaccgggtcctgatccccgtcggcgtcggcctgcccgagcgcccgcccagcgacatcgtctggagcctatccggcgtcagcatgggcacgacctggaccgcgcgcgtcattgcgccgccgggcgccgacaaggccggcttccaggcggccatcgaggctgaactggctggggtggtcgccctgttcagcccatgggagccgtccagcgagatcagccggttcaacacggctcccgccggcatgtgggcggtgtcgcaggggttctgggacctgatggatgcggccatggacctgggcgacgagaccaacggcgcggtcgatccgacgctcggctccctggtcgacctgtggggcttcggcccgccgggtccgcgctcgccgctgctgcccacgcctgctgacgaagagatcgaggtcgcgctcaaggtctcgggctgggggcggctgcgcctgaaccgcgaggcgcgcggcatgatgcagctgggcggcatgcggctggatctgtcggggatcgccaaaggtcacgcggtggaccgggtatccgagcgcctccacgccttgggcgcgacttcgcacctggtggaaatcggcggcgaactgaaggcccgcggcgtcaagccggacggccagccttggtgggtcgaaatcgagcagccggagggctcgccggcgccatgcacggtctgcgccctgttcgatctggcggtcgcgacctccggcgactatcgccgggcgttcgagcacggtggccgacgctatccgcacacgatcgacggctccacaggccgtccggtcgacaacggactggcgtccgtcaccgtcttccacgccgaggcgatgaaggccgacgcctacgccaccgccctgaccgtgatggggcccttcgagggacctgagttcgcccgcgacatgggcttggccgcgcacttcgtcgagcgcaccccgcgcggtctggtcgagcgcatgagcccggcctttcaggcgatgatggacgagggcgcgtgacggacgatcccggtcggctgctgtggacgggggtcgccgttctgctgtggctggcgctggtcgcggtcgtcgtctggcgcgaagcccgcgcacgccatcaagcccgacagaggcttgctgcgccggacgcgggtcggtcggttcttgtcgccttcgccagtcagacggggttcgcagaagaactcgcgaggatgacggccgaagccttggcgccgggcggggtcgcgcctcgcgtctccccgctggaccagatcgacgccgtgacgctccagacctgcgggcgcgcgctgctgatcgtctccaccaccggcgagggcgatccgccggacaacgccgcgcgtttcgtgcggcgggtgatgaccgaagccccccacctgtccggcctccgctatggcttgctggcgctcggcgatcgtgactacgaccggttctgcggcttcggccatgcggtggacggctggctgaggcgcgccggggcggagccgctgttcgacctggtcgaggtggacaacggcgatgcgggcgcgatccgccattggcagcatcagttgaacggactgaccggagccgtcgacgagccggactggaccccgcccgcctatctgccttggcgactgacgcatcgccgtctgctgaatcctagcagtccgggcggcgaggcctatcacctgcggctggagcccatcggccaccagccaggttggcgtgcgggcgacatagccgaggtcggcgcgccgccttcctccgcccatccttctcccggcgcgcgggagtattcggtcgcctccctgcccttggacggaggcgtcgagttggtgatccgcctggcgcgccacgccgacggcacactcggactggcgtcgggctggctgacgcaggactgccctatcggcggcgaggtggccatgaggttgcgcgccaacagcggctttcacggccccacgcccgagacgccgctgatcctgatcggcgctggcacgggcctggcggggctgcgcgcccacatcaaggagcgcccggccggctgcgagacctggctgctgttcggcgagcggacgcgagcgcacgacgcatttttcgacgaggagcttcagggttgggtggcgtccggcgtgctcacgcgattggaccgctgcttctcgcgcgacgtcggcgacggccgctacgtccagcatctgatcgccgcccatgcggacgcgctttccgcctgggtcgcgcgcggcgccgccgtctacgtctgcggcagcctggagggcatgtcgcgcggcgtgcatgcggcgcttgaggcgatgctcggcgaggaggccgtcatcgagatgatcgaagagggccgctatcggcgcgacgtctactgaagcctacttctgacgcgggctctccaggccttcataggtggtgaccagcttgccgtcgcggcgcgcccgcacggcgcgggccagctgttctgcggcgatgcgcacctcggcctggatgtcggtgtccttgtccagcgcctcgtggctggtggcgtagggctcccagtagccgatgtagcgatcaagctccgcgtccggcccggcgggctgtagcttcatgaaccgcagccagtcggacagcgagcgccgcacgttctcggccccctccacgtcgccgtgcaccacgaccgagaactgccgtccctccaggtggcgggggtagtcccagccgtccaactcgatctgcttggcctccctggcctccttgccgtgggtggaggacggatcgggattgccgccgtcgcagcacaccatccggtccatcatcagcttcatcgggctggacacctgataccagttgaccggcgtgacgaggaacacgccgtgcgcctcgacccacatcggatagatgtcgttcatccagtcgtggacctggcccagcgaatagttggggtagcagctgcaggggaagtggcacagcgccgccgccgtcgagaagcacgacttgcacggatggatttcgcatccgaactcgctggtcagccgcgacaggtccagcaccgtggtctcgaatccgccctgcccgtcgaacacctcgcgagcgatctgcgtcagccgccagctcttggacatctcgccggggcagctgtgctccgagcgcgacgagccgttgaccagaaggatgcgcatcggtccgtcccgatcgacgtgccgcgccttggccgcctggatcatgtcgttggcggcgatccagtcgatcgacaggtcgtagtcgggatcggcgaagccgtcgcccgccttgcgcgtcaccggcgacttgcgctggttctcataggcgtcccaggccaccgacacgatgcggtcgatctcgggcgcgaggccgttgaaggcaggatcgtgaaagcggctgcgatagcgcgcctcgaaatccgctcgctccagtcgcggcgacggcatgcccttgcgcggctcgggcgcggaccggggcggtgatgagtccatgaagacggctttctgcttgattgcatgggaaaacgccccgcccggcggggctgttcctcagcccggcggaaccggggccggacgcggcggttctgttggcggacctgtcaggagagccaccatgagaatccgcgacgtgatgagccgcgacgtgcgcgtcgcccgccccggagacaccctgcaggacgtgtcgcagtggatggccgagggcgacttcggcttcgtgcccgtggccgatggcgaccagctggtcggcacgctgaccgatcgggacataacggttcgcgccgtggcgcgtggcgcaggccccggctcttcgatcatggagtttatcagccgcgacgcctggaccttgcgcgacgacgacgacctgaaggtcggtctggacctgatggccgagcggcaggtacggcgcgcgcccgtgatcgacaagcatggccgcctggtcggcgtggtctcgctgggcgacctgtccactcgcgtaaaggagaagtacgcgggcgaggcgctggaggacatctcgcgcggctgatcgccccccgcttaaccacgtcggcataccggccgctaaggcggcggggctaagcctgcacgatcaaggtggaggcgatgaatggcgcgcgcgcagttccagaaggggcaaaaggtctgggtcgagtgcgtcggcgcctgggcgcaaatcgaacaggtccagcccgtctgggccaagggcttcgacgagcctgtccgcgtgacctatgacgtggggctgggccgcgacttcgccgcctccgaactgttcctgccgagcgaggatcctgcgtccgccgacctgggaagctggcgattgctgcgcgcgcgcaacaagtggcagacgccggaggactgcgtccatcatccctatcccggcacctatccggtggtggtcaccgacacggccgactggggcggatggcgtgtgcccggcgccgagtacgaccgcgacccggccaagatcgaagcgcaggcgcgactgatcgccgccgcgcccgccctgatgcaggtggcgcaatcgctggtcgatctggcggccgaagcgcccgacgatgcaccgcccgccgtgctggccctggcccgggaggcccgcgaggcgctgaagccggtcaccaacgtcttggatacgcctgcattccttgatggaccggcggaggtccgcgccgcctgacgcgttttggttaacgaaccctcgacaggaatcgccgatacagcctagattccccgcatcgctgatttggtccggagatcgccttgcggggcatggagcgccgcgtgaacagccaggggcggcgggcctctgaccaggagccgggctctcccgcctggttgcgcgtggccgtgctggcgctggcgctggcgatcacggcctatgtgctgctgacctcgcggcaggcgacccgcccattgcgagacgtgcaggcctatcaggaactggctgtaagccaggacgcccggcttctggcggcggagacccgcgccctcttgttgcagagcgacgccgcggccgatcagctgtcgcaaaccctgcctcgtccggccgccgcgccagaaggcgtggacctgcggctggtggacggcgaaggcctgatcgtcgcctccactcggatcgacgaaatcggacaagcgctcgcccaggcgctgggcgccgctgctccggccgccgacggtcgggcggcggctctcgacgccaagggcgagccgacgctggcggccagcgttcccgtgggggcgcgggggctgttcgccgtcgccacccgtccgtcacctcagcgcgggggtgtgatcgacgacctgtggctgctggtcacgcctctattgctcgggctggcggttctgatcctgatgacgatccagcacttccgtcgggctcaggaaagccgggcctgggccgcctcggagaagcggttccgggtggccgtcgaggcggcgcagtgcggcgtctgggagtgggatctcaagggcgaggaagtgaacctgtccgactacatggcccagatgctggggttcgacacgggcggcgtggtcagcgccgcggcggtcttgtcgcgcgttcatccgaaatatcaggaagaagtccagcacgccttgcgccaggcggcggcttacggcgcctttgaagtcaccttccccgtggccgatggagacgggaaggcgcgctggatagacgctcgggggcaggcgcgcggggagcgcggcgaaggcggcttcttctccattctcggcgtcgcgctggacatcaccgaggcccgccgttcgaaggcccaggcgcaggccgccgagagccgcttgcgcgacggggtggaaagcatctccgacgcctttgtcctgtttgatcggcaggaccggctgatcctgtggaacgacgccttccgcgacgccttcggcctcggtcctgacgtggtgcggcgcggtgcgcggaaggacgacctcaaccgtatcgccgccctggccatcaagtcggatctgaacgccccggacggacgtgtcggggcccgcgaggtggaactgcacgacggccgctggctgcaactgaacgagcgcttcacctccgacggcggctcggtgatcacggccgccgacatcaccgccatcaagcgaaaggaggccgaacgccagcgagccgtcgacgtcctgcaggtcgccgtccgggagcttgaagcgagccaggccaagctgagccagctggcgcgcaaatacgaggtggcgaagacccgggccgaggcggccaatcaggccaagtccgagttcctggcgaacatgagccatgaactgcgcacgccgctgaacgccatcaacggcttttccgagatcatggcgggcgagatgttcggccccctggggcacccgaaatataagggctacgccggagacattcatcgctcgggccagcacctgctgagcctgatcaacgacatcctggacatggccaagatcgaggccggcaagatgaagctgcattatgagcccgtgtcgatcgccgacgcctgcgaggacgcggtgcgcctgatgcgcggcaagatcgaggatgcgcgcctgcgtttctctcttcacgtcgactccgcgcccgagatcgaggcggactaccgcggggtcaagcaggtgctgctgaacctcctgtccaacgccgtgaagttcacgccggagggcggctcgatcacgctcagcgtgcgccggatcgtctccgacgatggagaggagcgggtgcgggtctcgtgcgccgacaccggcatcggcatcgcggccgaggacatcgagcggctggcgcagccgttcgaacaggtcgagggccagcattccaaaacaacccagggcacggggctggggctttcgctcaccaaggctctggtggaactgcatggcggggccctgaccatcgaaagcgagttgggcgccggcgccaccgtcagctttgaactacctgtacgccgccccaaggatgacgcgacacaggaccagtccccgattcaggcgcgcgcggcctgacatccgggccgaaacaaccgccggagatgcaggagacaggccgccgatccggatcgccgctacttctggaacctaacgcgccgacgccctttcgaaacctcatgattgacgacaccaaggactcgctcgccgcccggacgacggccagtgcgaaatcggatcgcgatcaggcgatcctgaacagcgttctgggctttgcgatcatcggcatggaccgggacggcgccatacgcgagtggaacccgggcgcgcaggccgtcttcggatggaccgccgaggaagtcgccgggcgctccgcaggcctgatcttcacgccggaggatctggcgaacgatcgacccggcgaagagatgcgcctgtcgatcagcgatggccgcgccaacgacgagcgatggcatatccgcaaggacgggacgcgcttctgggcgtccggcgaaatgacgccgctcctgggcgtgggcggcgatcatctgggcttcgtcaaggtggtccgagaccgaacatcggaacatcaggcgcggcgggctctggaagaggccgaggagcggctgcagcgcgcccaggaagccggcggcgtcggcctgttctgggtgtcggcggcggacaacatcatccatgcgacgccggagttctgccggctctatggcatgcccgagacgccgcaagccccggcggagatcttcgagcgcctggttgtctccgatgatgtcgaactcgtctccaatgcgttgagccgtcaaaccggccaggcgccgcttgacgtcgaatatcgcattcgacgcgccaacgacggcgcgctgcgctggatcgcgcgcaagggtgagctggagttcgacgcggaggggcgtccggcgcgcttcgtgggcgtggccagagacgtcaccaaccgggtcgcaggcgagcaggcgctgcgtgacgagcgcgagcagttggcgcagatgttcgcccaggcgccgacgttcatggccctgctgcgcggacccgagcacaggttcgagcgggtcaatcccggctatgtgcagttgatcggtcaccgggacgtcgtcggtcgaagcgtgggcgaggcgctgccggaggccgtgtctcagggctttgtggagcttcttgatcaggtcttcgcgaccggcgagccgtttgtggcgaacggtgtcaggttcgaagtgcagccgacgcccggcggtccgttgcgggagcgctttctggatttcgtctaccagccgatccgcgacgcgagcggcgtgatcaccggcatcttcgtggagggcgccgacgtcaccgagcgcacgctggcggcagccgcgcttcgggacagcgaaacgcgatacaaggccctgctgaacaccaccgacatcggcttctgcatcatccagatgaaattcgacgaggcggatcgccccgtcgactacaggatcgtggagggcaacgccgcctacgagcggatgacgggcctgcacggctcgaccggcaaatgggtctccgacatcgcaccgggcttggagcagcactggttcgatctgtatggccgcgtggcgcggaccggagaaaagatccgtttcgagcagcccgccgcaaccttcggccgctggtacgacgttcaggcgtttcggatcggcgatcccgaccagaaccgcgtcgccatcctgttcaacgacatcaccgcccgccggcgaagcgaggcgcggcaggagaccctgctggcgctcgccgacgcgttgcgcgacctcaccgatcccgccgagatcgcccacgccgcctcggaggtgctgggccgggcgctgggggtcagccgcgtcggctacggcatcatcgatcgggtggcggaaaccgtctccatcgaacgcgactggaacgcgccgggcgtccagtccatcgccggcacgctgaacttccgcgacttcggctcctacatcgacgatctcaaggtcggccgcaccgtggtcatcggcgacgccgccgaggatccccgcacgcgcagcaccgccgagcagttgagcggaatcagcgccgaagccttcatcaacatgccgctggtcgaacagggtcggttcgtggccctgttcttcgccaacaacgccacgccgcgcccgtggcccgaagacgacatcacgctgatgcgggaagtggcggatagggtgcgcgccgcgtccgaacgcgcccgcgccgaacaggccgtccgcctcagcgaggcccagttccgcgccttcgcgcaggcggtgcccaatcagatctgggccagtcggccggacggcttcctggactggttcaacgccgcgctccacgcctacaccggcaagacggaagaagagcttgcgggcccaagcggctggacggccattgtgcatcccgacgatctgccccgcgcccgagccgcctgggaggcggcgcttcgaaccggaaccatctacgaagtcgagttccgcatccgtcgtcatgacggcgcctggcgctggttccttgtcagggccgaaccgatccgcgacgcggacggcgtcatcacccgctggatcggggccagcaccgacatagacgatcggctgcggcaagccgccgagctcgagcagctgaacgaaacgctcgaggaacaggtcgccacgcgtacacgcgagctgatggccgccgaagaggccctgcgtcagagccagaagatggaggcggtgggccagctgaccggcggcatcgcccacgacttcaacaatctgctgaccggcatcacaggcagcctggagatcatgggcaaccgcatcgcccagggccgcttcaacgagatcgaacgctatacgacggcggctcagggcgcggcgcgcagggccgcggcgctgacgcaccggctgctggcgttttcgcgccggcagacgctggatccccggcccatcgacgccaaccggctgatcggcgggcttgaggagctgatccgccgcacggtgggtccgcaggtcgaggtcgaggtggtggccgccggcggcctgtggaccacgctggtcgatccgaaccagctggagaacgcccttctcaacctgtgcatcaacgcccgcgatgctatgccgacgggcggacggctgaccatagagacgggcaaccgctggctcgacgcgcgcgccgcggagcagcgcgacatggagcccggccagtatatctccgtctgcgtcagcgatacgggaaccggcatgagcgccgatgtgatcgccaaggcgtttgatccgttcttcaccaccaagcccctcggcgtcggcacggggctgggcctgtcgatgatctacggcttcgcgcggcagtcgggcgggcaggtgcgcatctactccgaagaaggcgacggctcgatggtgtgcatctacctgccgcgtcacctgggccccgccgaggcggcggagccggttccgaacgtggccgagacccaccgcgcgcgcgtcggcgagacagtgctgatcgtcgacgacgagcccaccgtgcgcatgctggtgctcgaggtgctggaggagctgggctatgcggcgctggaggcggcggacggcgcggcgggcctgaagatcctgcagtcggacgcccgcatcgacctcttggtcaccgatgtgggcctgcccggcggcatgaacgggcggcagatggcggacgccgcgcgcctggtccgtccgaacctggaagtgctgttcatcaccggctacgccgagaacgccgtcgtcggcaacggccaccttgatcccggcatgcacgtgatgaccaaacccttcgccatggaagccttggccagccgcatcaaggcgctgattccctcgggctgatcgaccgcgtcagatttcgaggtcatgcgatggagcgtcttggctcgcctcgccgttgatgaccgcaccctgaagcgagacctccgtggcccaagacaaacgcgacccgcacgcccccgccctgaccggcgaagcgcccctgatcgacgggcctcagccccaggtcgaggagccggagcgcgcggcccgacggcccggcgcggcggcggtcgcggcccggctgctgcgggcgttggatccgaagacgccgctgaccgtcctggtcaccaccagcgagcggcgggcggacgagatcggccgcgccctgtccgccttcgccggcgaccgcccgctccgcaccctgatcctgccgccttgggactgcctgccctacgaccgcgcttctccctcccgcgagagcatgggccggcgcatggcggtgtttgaacagctggcgcgcgacgcggccggatcggtggtcctggtgtcctcgcccgacgccctgatgcagcgcatcccgccgcgcgcggtcctggccgaacggttcgagatcgaggcgggggcgccgctggatcgcgacgccctgtcggccttcgcccaccgcgccggctatgtgcaggacgaccgtatcgacgagccgggggagatcgccatcctgggcgaggtggtggacgtttatccgcccgcatccgccgcgcccgtgcggatcgccttcgacgaggagggcaaggtcgccgacatccgccgctacgatcccgtgacgcagcgctcggacgacagcgtggagcgtctgtgcctgacgccggcgtccgaactgctggtcgggccggacgatgtacgcacgcccggcgaggagcatcgcatggcggaacgctatgatgacggtctggtgagcctgctcgccctgctgtccggcgcctgcgtcctcacggaagacgaggtcgaggaccgctgtcgccgcttcgccgatcagacggaggaggcgcatcaaacccgcctcgccttccgcgacgaggacgcgcgtcccctgcctcccgagcagtcgtatctgtcgctggaggagacattggcttttcttgatcagggccagcgactggatctggacggcctgtccggcaatccgtccttcgcggtggagcgctcgccgggaaaggcgctcgcatccttcattcaggagcgccgagacgccggacggcgcgtggtcctggccggtctggcgcacgaacatcggatggtcgcgcgtctgctgaggcgcgccaaggcggaggcgcccgagacggccgcgagctgggacgcgcttctggaggcgccgcacggcgcctttgtcgccctgccgctcgatctcgacgtcggcttcgacgatgcggagctgggcgtcaccgtgatcacgccgaccgacgcggtgggcggccgcgtggcgcgcccggcctcgggcaccgccgaactgctgggcgagccggaactgcgggccggagacgtggtgatccacgaggaccacggcgtcggcgttctgcaggcgctggagcggatcgcggtcggcgatcaggagcgggacgtgctgcgcctcgaatatcacggcggcgcgacggtgctggcgccggtcgaggagttcggccgcatctggcgctatggctccgagccgtcggccgtgacgttggaccggctgaacaccgacgcctggctgaagcgacgggcgcagctcagcgccgacatcgacatgacggccagacagctggtcgagatggccaaggtgcgcgaagaagccacggccgaaccgatccggccgcccaagccggcgcttgcccgcttcgccgcgggctttccctaccctgagtccgtcgatcaggccgccgccatcgaggcggtgctggacgatctcgcctccggccgcccgatgaaccggctggtgtgcggcgatgtgggcttcggcaagacggaggtggcgctgagggccacggccgccgcggccttggcgggcaagcaggtgatcgtgtcggcgcccaccaccgtgctggcgcgccagcatttcgagactttccagcgccgcttcgccggcacggacgtggtggtggcccagctgtcgcgcctggtcgacagcaaggaggccaaggccgtgaaggcggggctggcgtccggcgagatcacggtcgcggtcggcacccacgcgctgggcgccgacgacgtcacgctggccgagcccgggctggtcatcatcgacgaggagcagcggttcggcgcggccatgaaggacaagctgcgcgccaaggcgccgcacctcttgtcgctgaccgccacccctattccgcgcacactgcaaggcgcccttgtcggcattcaggacgtcagcgtgatcgccagcccgccggcccggcgcaggcccatccgcacctttctgacgccattcgatgcggcgtcggtccgcaccgccctgctgcgggagaaggcgcgcggcgggcagagcttcgtggtcgtaccccgcatcgaggacctggagccgatgcaggcgcgcctggccgaaatcgcgggggagctcagcgtccgcaccgcccacggcaagctgtcgccggaagagacggacgcggtcatggtcggcttcgcggacggcgagggcgacgtgctgctggcgaccaacatcatcgaaagcggtctggacgtgccacgcgccaacaccatgatcgtctggcggcccgaccggttcggcctggcccagctgcaccagctgcgcgggcgggttggacgcggccggcgacagggcttcgcctatctgctgcacgccgaggacgaggaactgcccgaggcgactcgggcccggctatcgacgctggaggcgctggatcgcctcggctcaggcttcgccatcagcgcgcgcgacctcgaccttcgaggcggcggcgatctggtcggcgacgaacaggccggccacatgcggatgatcggcgccagcctgtatcagcgcgtgctggaaggggctctgcgcaccgcgcggggcgagcggccgctgaacctgggggagccgatctattccggtgaccccaaggcggccctgccggaggactacatccccgaccccaccacccggatcaatctctacgcccgcctggcgcggctctccaccacggcggagatcgaggcgttcggcgacgagctggaggatcgcttcggccccctgcccgatccggccgccgccctgatcgccaacgcccggctgaacgccctggcgcacgaggcgggggtggaggccatcgcctcgggacccaaggcgacggccttctccttcggccgcgccgccgcatcggtctccaaacggatcaaggatgacgacgcccgccattggaaggacgaccgcctgatctatccggcgggcgacacgccgcacgattcggccttcatcgagagcgttctgaccgatctcgccgcctgatcggatcagtccgccaaaaaggcgtcgaccaaggctgcgaaacgctccggctggtcggccatgatgaagtggcggctgccgtcgacgcggatcaggcgcacgtccggcaaggccgcatactcccgcgcccatagggcatccgccatggcggacggagcgccgccctcggcgtccgcggcgtagagggccgtcactggcgtggtcatggcggccagaccgggccgggcgtcggtggtcatgacgtcgcgcagggcggcggcgaaggcgtgacggtccgacgccatcgaccagcgcactatctgcgcctgcatggcgggcgtccgtgacaggccggcggctgaggcggtctgttgcgaccgcagcgtggcctcgtccgccgaaaggacgccggccgccgcctgctcggcgaagggcctggcgctctccggcgtcgctgtcggtccgaacagggcgctgtagaagggcagcgaatccaccgagagcagccggtcgaccagctccggatggctctgcgccagcagaagcccgcttaaggcgcccatagaatggccgatcaccgccggacgctgcagtccggcttcgcggatatagcgggccagttcttcgaccgccggctcgacgaagggaccatcgccgtggctccacggctcgcctgcgaagccggccagttgcaccaggtgcacccggtgggtcgccttcagccggtccgccgtctcgcgccacacctcccgcgaggagacaaggccggggatcaggatcacgtcgggcccctgccccgccacctcgaccgacagccgatctgaggcgaaggccgacggggcggcggcggcggacggcgccgcctgggcgtgcgcccgctgcggatcgagcgccgagaggatggcgaacagggcgccggcgatcagcatgaggcgggcgcggcggggcgcgcacgcccccttcagggttgcgtggaacatggtggtctaccttttcggggttgtggcgaccgcctcagcggccgtgagggttctcgaagatggtctcgaccggccgctcgaagatcgcggcgatccggtaggcgaggtccagcgacggatcgtgcttctccgtctccagcgcattgacggcctggcgggagacgccgagctcccggcccagctgctcctgcgtccagccgcgctcgacgcgcagcagcttcagacggttcttcatcggctggtccgcacgaacggcgagatgacgccgaacgccgcccagaacagcggatagatcagccatcccggcgcatggggcgcgtccgcatagctttccgcgaagccccagacgcagaacacggcgaaggcgacgccggtcgcggcgacgaacgtcttggtcatcaccgcccgcacgaactcgtccgcctcgttcagataggccagcgtcgcccagatctgggcgatgaccggcagggccaccgcgatcgccagcagccaggccgtccagcccgcgcgtccatcgaacaggccgaacatcgcggcgatgttgatggccgcgtagacgcccatgaaacccatggtccgccgggcgtagcgcctggccgccggcgtgttgtccctcgacgagctccacatggatcgtccctccccctgatgtaaggctgaccttacatcaggtgcatgtcatgtcaacctgacatttcgtcaggaggacgtgacatcaacatgcgcttgatcctgatcggcttagagcgcaggcgttcagggatgaccatcaccgatcccgccgccttcatcacggccaacacccggcttcagcctgtgccgcatgcgccggaaatctcgctgtggctggcggacgaggtgacgccgatctggcgactgacggaggaggagctgggcgaaatgggcctgccgccgccgttctgggccttcgcctgggcgggcggacaggcgctggcgcgctatctgctggaccatccgcatgaggtcgccggcaagcgggtgctggacttcgccgccggctccggcctggtcggcatagccgccatgaaggcgggcggcgcctccgtgctgtgcgccgacatcgatcccttctgcgaggcggcggtgcgggcgaacgcctcggccaacggagtccgtctggacttcaccgacagcaacctgctggacggcgaaccgcccgcggtcgacgtcatctgcgccggcgacatcttttacgaacggccgatgaccgaggcggtgctggcttggctcgaacgcgcgcgggcgcggggaacgcaggtgctgatcggcgatccgggccgcacctactttccccgctccggcctcgatttcctggcggaatatcgggtgcccaccacgcgcgagctggaggaccaggagatcaagcggtcctccgtctgggccatgccttaggtgatcagcgggcggcggcctgctgcgtctgctcggtctgtccctggtggcggccttcggcgaactcctcgatcatcttcctgttgaaggccgggatgtcgtcggggcagcggctggtgaccagacccttgtcgaccaccacctcctcgttgacgacgttggcgccggcgttcctcaggtcggtgcggatgctttcgaacgccgtcagggtgcggccctcgaccacgcccgcctcgatcagcagccagggcgcatggcagatggcggccacaggcttgccggcctcgaagaaggcccgcacgaacgccaccgcgtccttgtcggcgcgcagctggtccggattggccacgccgcccggcagcagcaagccggcgtaggacgaagcgtccgcatcggccaccgctttgtcggccgtcaccttgtcgcccggcgtcagatggtcgaagccctggaactcgccggccttcaacgacaggatctcgacgctcgcgccggcctccttcagcgccttaaccggctcggtcagctccaccagctccacgccgtcggtggcgaggacggcgacggtcttgcccgaaagggtctgggccatggtcttgctccgttttctatggggaaggaggcaggacaacccgtgcgccgacgacaggttgcggctccgcttgcctcggcccaagcctccctatctgtttgctcatgttcacgcgcatcgccctcgccggcctgatcgccgccgtcgcctcccccgtcccggcccagacctggacgccccatgtgtcgccatacgcgggttatccgggcggcgcgccggccgccatcgccgaccagcatcgctacgagacggagcggctgcgcagccaggccgagacgcgcgatctgttcgctcgccagcagcagctggagacgcagctccgtcgccagcggatcgagggcgcccgacctctgcccttgccgaacgagccggcctatcgcccgctgcgttcgccggccgaggagcgtgcgcttcgcgagtccgcgacgcagcggcgcgaaaccctgggatcgggcgtgggccagatcgacgcctggctggaccgacgcaccgaatagagcccgcacgcatcccttcgcctcccctccgcgttacggccgggcttgagctttggagatgagcgatgcgctggcagggcggacggacgggcggcgggatcgaggatcgtcgcggcatgggcggcggcgccatcgccggcggcggcatcggcgtcaccgtgatcgccctgattggctattttgtcttcggcatcgatcccaacaccacccagcaggtcgccagccagttcggcggcgccggcgcggcccagcagcagggcgaggtcggcacgcccgaggatcaggcgggtcgcttcgtcgatgtggtcggaaccaacgtcaacgacgtctgggccacgaagcttcagggctatcagccgcccaacaccgtcatctacgagcaaggcacctcgaccggttgcggctacggtcagtcggccatgggacccttctactgcccgaccgaccagacggtctacctggacctcggcttctggcgcgagatggagacgcagttgggcgcgtccggcgccgatttcgcccgcgcctatgtcatcgcccacgagttcggccatcacgtccagaccctgaccggcgcctcccaacaggtgcgtcaggcgcagcagcgcgcggcgggccaggccgaggcaaaccgctattccgtcgcgctggagctccaggccgactgctacgccggcgtctgggccgccaatgcggcggcggtctccaacgggcaggtggcgctggaggccggcgatctgcaggaaggcatgcgcaccgcccaggccatcggcgacgatacgctgcagcgtcgcggcggcggccgcgtctcgcccgaaagcttcacccacggatcgtccgcccaacgcgtggagtggctgcagcgcggctaccaggccggcgatccctccgcctgcgacaccttccgagggctctaatcccggcgtggtctccccacggtgacgtccatggcctcggacaccagcagcctcgcgcggccgatgtccatcaccacctggcgaccggcgaaggcctccatgcccagcagggcgcgcggaaatccgggcacggacacgtcggcgaagatggcgacctcggcgtcctccaccagggtgtcgccgaaggtgacggtgcgagcccgcacgatgtccgcccgcgtcgcgccgcccagcacgatgctgacgccctggcggctttcgcgaccgttcagaaggcccgccccttccgccgcctgacgactgacggccaggagcgccgaggcgccggtgtcgaccaccgcctcgatctccgcgccctcgaccgtcacggctgcggacaggccgcgatccgcccgccgcacctctatggggaccagacccgtcggcgcctgatggtcctccggccggctcagccgcagccgtcgccccacggtgtcgagatccaggaccagttcgcgcagcacgtcctggcccaggatcaacggcgttcccagtccgcgttcggacgccagcggccccagttgcagtatggcggcgcgcaatccgttcagcctcagctcgcccaccgccacatcgatcgtcgccccgcgtccaagctgagggttgccgcccacgccataggcgatcagcggcatcgagaaggtctcggccaggcccagatcggcgaacagggcggcgtcgatgaccgagaactgcgcgccgctgtcgaccagggccgcaacgcgtcgtccgccaacctcgacctcgaccgtgggcgtcgccgcccgccttcgcgcatagggcagccagccgctggaaccgccctcagcgtagccgatctgcggccctcgccagatcacattgtcgcgcagccaccaggccccgccgatgccggcccccagcaggcccagccggaccaggatgtcgcgtcttctcatgcacagggacatggaccctgcggccgccccgcgccagcgacgccgatgtcgcaacaatcccacgcccgctcgcaggtttgcggatgacgcaggtccgccgggccgataccgtccggcccatgcttcccgacagcgcccattatctctcgacacgcggccaggcgccgcgcgccgacttcgccgaggccttgatgcgagggatggcgccggacggcggcctctacatgcccgaggcctggccgactttaccggcgcgcgggatcgaagcgggtgcggactacaaggcgatcggcctggacgtcctgcctgcctttgtcggtgacgcccttccggcgggcgcgcttgagcgagcgctggatgcgctgatctccgggttcgaccatccggcggtgacgcccctggtgcagttggaggacgggctgttcctgctggagctgttccacggccccaccgccgccttcaaggatctggccatgcagttggtggcggccctggcggacgaggcgctggccgcgtccggtgagcggctgatcctgctgacggcgacctcgggcgacaccggcgccgcggccgtgcgggcgttcgcgggcaaggaccgcatccggctggtggtgctgcatccgcttgaccgcgtctcggccgtgcagcgccgccagatgacgacggcggatgccgacaacgtgctgaacctggcggtgcgcggcgacttcgacgactgtcagcggctggtgaagggtctgctgggcgaagagtccctgcgcgaacacagtcgcctgtcctccgtcaactcgatcaactgggcgcggctggcgggacagatcccctactatgtctcggccgtggcgcagctgggcgggcccgcgacctttgtcgtgccgaccggcaacttcggcgacgccttcgccggggttgccgcgcgccgcatggggctggagatgcacgggatcgtcgccgccgtgaaccagaacgacgccctggcccgcgccatcaaccacggcctctattcacgccgtccggcggttgaaagcggcagcgtctccatggacgtgcaagcgccgtccaacttcgagcggctggtgttcgaggcgtcgggccgagatgcggaacgcactcgagacgtgttcgagacctttgctcgcgacggcgcggtcgccttcaagccggacctcctggccgccctgagagccgaggtttcggccgtctccgtcgacgaaaccgaaacccgcgccgagatcgcccatgcccatcagcgctggggaaaggtcatctgcccgcacaccgccgtggcgctggccgccgcacgccgccatgatcgcaaggaggggccggtgatcgccctgtccaccgcccacgcctccaagttcggcggcttcgtttcggaggtgctgggtttcgagccggagccagcgccggtgatccaggcgctgggcgatcgccccgagcgcctgacgatcatcgacaaggcgcccgatgcggcgctttcggccgtccgcacctttgccgcctgacggcgcttaggccaccgcctccagcgcacgccacccgtcgagccggcgcagaaacactgccggatccttgggcgtcaccagcttgctcggatcgtggaagatgcggtcgtgcagccgcgttagggtgaaccgcagcgccgccgcctcgcccagacgcggcagggcctccgcttccgccggcgtcagcggtcgcacgctctcatagccgcgccggaaggccgcgatcgcgcgtgcgtcgggatgaccttccgcatcaaagccccaggccgacagggcgatggccaggtcgtaggcataggcgtcggtgcagccgtaatagaaatcgatcacgccggcgacctgatcgccctcgaacagcacattgtccggaaagaagtcggcgtggatcggcccgtacggcaggtcgcgcggcggcccacccagacgctccagcgccgcctccacccggtccagcagccgccgatcctctccggtggctgcgatcgcgcaacgctcggccagagccagccaggcggccggccccaatgggttggcccgctcctcgggaaagtccgcgccctgcaaatgcagtcgcgccagggtcgcgcccgccgtcgcctgggcctggaggctgggggcccgcagccagtcgcccggcttccattccaccaaggcggcgtcacggccattcagccgccccagccagcggcccgcccgatccatcatcggcgtcgcggccggaaaaccccgcgccgccagatgcgccgtcagccccaggcagaagggcagcacgtccgcatcggtccgctcctcgaacaacgtcaggaccaaacgttctttgtcggtctccacccggtagttggtgttctggatgccctcggcaatggcttcgagcgccttcagctcgccgagatcataggcgcccagaaaaaagcgcgcgtcggcctcggtcaccggcgtgaaaacggccatgtcgcgctctccttctgaaggcggcgccggtcagttcagaccggcgtccgcgcgacgaattcgcacgatttcggccaggtccgccatcaggctttcggtcgtggcccagcgcccggcgccccgtccccggcatcgccacacccgaccgtccgcgccgtgcaccttcagcgcattgccctcacctttcagagactggaacagggcgtcgtcggcgtcggcccgcagacgcacggaggcgtcaagccgctctccatcccggcggcaggcgccgatctggcgcagggcggcgtccggctgcgtctcggccgatagcgcgtcgcgcggcaccgcatccgcctctggcgagacgccgaacgcctcataggccaggagccgcaccttggccgccgcgtccagcccctccagatcggcggagggatcctcttccgcaaagccggccgcgcgggcgtcggcgagcgcctcggcgaaggccgcgccctcgcccagccgttccagcatgaagttgacggtgccgttcagcacggcttcgaagctggcgatctcgccggccgcgcgggcggcgcgcaccgtctcgatcatcggcgatccgccgccgaccgaggccgaccagaagacgcggcggccatgcgcatccgccagggcctgcagcccggccggatcgcggctgaccgcctgtttgttggcgctggccacgtcgcagccggcctccagcgcggcccggatcacggcgtggccggcctctccctcggacaaggcttccaggaggatgtccggctggcgcgacaggagatcagctgcgctcgccgtgaacagttcgggcggacagggcacgtcgcgcgacttcttcgggtcgcggaccagcacgccgacgacctggtagcgcgggtcgcccagcagccggttcagcacgccgccgcccaccacgccgcagccggccaccgccaccttgagcggctgaagcgcgggcgcgggacccggaggcgccgagcgttcgccgatcaccgtgccgtccgcacgatccagcgccgccacctcgatctccaccccgcgcgcctcgcccagatcgatggcgtcgcgctggaccagcgatccacccagccgccgcgccacgtcccacgacgccctgcgataacgcagggccggggccgcgtggtcgttggggtcgtggtcatagaggccgtcgacgtccttcaccagccgcgcccgatccaggcccagctcggccgccagaaacaccgccgtcagatccgatcccccgcgtcccagaagggcgatccggccgtccggccgcaccgcgccgaagcccggcacaatcactgcctcgtggcgttccagcgcctgcttcaggtgatccggacgcaggccgcacggccgcgcatgctccggctcgccctcggccaagatccccaactcacggaccgacagggcacaggcgtccagccccacccggtcacacgcgatggccgtcagcgccgccgccttttcctcgcccaacgcgacatagcccggcaggaggttgttcgaatgcggcaggcccaggacccgcgcctcggccagcagggcgtccgtgtgcccggcaaaggccgacaccaccgccaccacctttcgccctgcccggacatggccgtagatggcggaggcgacgcgcggcgcatcctgcggcccgcgcaggatcgagcttccgaatttcagcaccacgacctgtgcaccctcgggcgcaggctgcggtttgggggcgtcggagacgagggcgaggctggctgaggcgggcatggaggcggctttcgggtgaggtctgaaaagaggctggatcaagaaaaacccgccgggcggggcgccgggcggtgggttttgcgtattcgccgaccttggcgcgctaaccgtctcccgcccgcgagggcatggtggtggtcccgccgatcgtcatgccgaagccggtcgcggccagcgcgacgacggacccttcagcgatgaacatggggcggcgagacacgtggaaggctccggatggctgttgacccgagcatgttcggcgaccctcgccgccgtcaagtccccacgcacgattttttcgttaaagggctcgaacccgcagccactccggtcaatacgcacggcagcgccgatgaaggggtaaaacatttctcttgacccgcgctccgtctccccacaccgtagggtcactcatcaagaccggctgagggattaggccctttgacgccggggcaaccatcgggttccgcccgaaacggtgccaactcctgcggggtccctatcgggccgcgagagatgagtggagcatcgacgaggcgacgctccacgatctgtcaccgcaccgagccttgctgagcgagactggtgcgagacgacgatgaccctgacggaaaccctgctggaagagccccgctgtcgccccgctcggcgaacggcgccgacgcgtgcggcgacgcccggccgcggcgcccacgacatcgtcacccccatccccgagactttccgcctgcaatcaggagagcggctgggccagcgcagcatcgtcggtcggctgcacggccgcgccggcgcgccgctggtcatcgtggccggcggcatctcggccggccgcttcgtgcaccgcacggaaaccaacggcctgggctggtggtccggcgccgtttcggtgcgcggcccgatcgatctggaccgcctgcaggtgctgtccgtcgattttgcgcccgaagccgaggcgggcgccaggcccgtcaccatcaccacgcacgaccaggcgcgccttctcgcacttgtgctggaccggatcggcgcggacgcggccgccgcattcgtgggctgctcctacggcggcatggtcgccctggccttcgccgagctgttccccgcccgcgtcgagcagctgatcgtggtctcggccgcccaccgcgcccacccgcaggcgaccgcctggcgtggcatccagcggcgcatcctgcagttcgcggtggcggcgggccggcccgaggagggcgtcgccctggcccgccaactggccatgaccacctatcgcacggccgaggagttcgacggccggttcgaaggcgcggccccggcccacgccggcggcgcctatcccgtctgcgactatctgaccgcgcgcggcgaggcctatcgcacccacaccacgcccgcccgctggttgtcgatgtccgactcgctggatcgccaccaggtgacgcccgaggcgatcaccacgcccgtgaccctggtcggcttcgcctcggatcggctggtgccgatcgacgacatgcgcgagctggccgcgcgcctgccgaacctgtggcgcttcgtcgaggcgccctccctctacggccacgacgcctttctgaaggaggacgctctggtcggcgacatcctccgcaccactctcaaggacatcgccgcatgacccaccgccccgccagcccgcacaccattgccgcccgcacgggcgtggacacggacgcggcgcacggctcggtcatgccgccgctgtatctgtcgtccaactattccttcgccggcttcgaccagaagcggaaatacgactacagccgctcgggcaatccgacccgcgacgtcctggccgagaccctggccgaactggagggcggcgcgggcaccgtgatcacggcgaccggcatggcggcggtggacctgccgctgtcgatgctggagcccggcgacctgctgatcgcgccgcacgactgctacggcggcacctgtcgccttctgaacgcccgcgcgcgcaagggccatttcgagctgaagctggtggatgagggcgatccggaggcgctggaacaggcgctggctctcaaacccaagctggtgctggtggagacgccgtccaacccgctgctgcgcgtcgtcgacatcgccgacatctgcacccgcgcccatgcggccggcgccaaggtggtgtgcgacaacacctttctgtcaccggcgctgcaacagccgatcaagctcggcgccgacttcgtggtgcattcgaccaccaaatacatcaacggccactcggacgtggtgggcggcgcggtcatctccgcagatgcggcggatcacgaagagctggcgtggtgggccaactgcacgggcgtcaccggctcgccgttcgacgcctatttgaccctgcgcggcgtgcgcaccctgttcgcccgcatcgagcggcagcaggccaccgccggccgcgtggccgaggttctggcggcccacccggcggtcaaggccgtccactatcccggcctgaagtcgcacccgaaccacacgctggccgcgcgtcagcagtctgggcccggcgccatgctgtcgttcgaactgcacggcggcgccgaggccgtgcgcgacctggtcgaggcgctggaggtcttcaccctggcggagtcgctcggcggcgtcgaaagcctgatcgcccacccggccaccatgacccacgccgccatgacgccggagcagcgcgccacggccggcatcggcgacggcctggtgcgcctgtccgtcgggctggagcatgtcgaggacctgctggccgacctcgcgccggcgctcgatcagctcacgtcccgcgtgcgccaagcggcctgatcgtcgagccgttactgccacgcttggttgccagcgttaacttgtggttaaccactaaggcggaagtcggcgcggaagcacctgatttaccgcacattcttcgggactgatggaactatccacaagggttgtggttaaccatacgttgttcacggcgcagaagcgctctttcgcaccgttccgagtcctgaagaatgttcatcgccatcacacgtccggcggttgagccccgaggccccgacgccgtcgccgtccccggctcgcccgccatcgccgaactgtcgccccgcgcgctgcacgccaagctgctgtccaacgccgccgcccgccgcctgcggggtctggagcgcaagcaggcccagcgcttcgacgacgccgactattggctgcacgccgcgccggtcgcggtgaagaaggccagcgccctgcgtgaagacaagagcttcctcagcctgccctgacgccagcctggaattttagcccatcagttcggcgaaacggtcgaacagatagagactgtccgtcggcccaggcgacgcctccgggtgatgctgcacgctgaagatcggcttgtccttcaccgccaggccgcagttggtgccgtcgaacagcgacacatgcgtttccgtcaccgcatccggcaggctgtcgcgatccacggtgaagccgtggttcatcgacacgatctcgaccttgccggtggtcaggtccttaaccgggtgattggcgccgtggtgcccctgatccatcttcacggtcttggcgcccagcgccagcgccagcatctggtgacccaggcagatgcccatcaacggcttgccgctgtcgaccagcttcttgatttcgggcacggcgtaggcgccggtggcggccgggtcgcccggcccgtttgacagcaccacgccgtccggattgcgcgccagcacctcctccgccgtggtgtcggcaggaaccaccgtcaccttgaccccggtcgaggcgagcgcccgcagaatgttgcgcttcacgccatagtcgatgaccaccaccgacttgcgcccttgcgtcttcgggtgcccttccggccaggcccacaggccctcgtcccactcgaacgactgcagcgtcgaggcgggtttggcgagatcaagacccaccaggccggtccactcgcgcgcctgctgaaccagggcgtccagggcgaagcggccttcgagatcgtgcgcgatcaccgcatgcggcgcgcccttgtcgcggatggccttggtcagggcgcgggtgtccaccccggccagccccaccacaccacgccgcttcatccaggcgtccagcgagccttccgagcgccagttggccggatcggtcggcaggtcacggaagatcgcgcctcgcgccgaggtgtcggaaccgccgcccatctgttcaatgtcctcgacgttcaccccgacgttgccgacgtgcggaaaggtgaaggccaggatctggctcatgtaggaggggtcggtcaggatctcctgatagccggtcatggcggtgttgaagaccacctcgcccagcgccgagccggtggcgccgacgcccaccccttgcaggatcgtgccgtcggcgagcgccagaacgccggtcgcgccgggaagaagcttcgtcgtcatggcgcggtccttggcggctgaggtgggcggctgatggtggcgggcaaacggcggcgtcgttaaagaacgccgctgttcaggtcaacgcgtgctgcgctatcggccgtcgctgacgctgggcggcccgaccaggcggaaggtcgccgtggacccgccttgcgcatgcggagccagccagacgtcgaacaggccgggctccacgcgatagcgctcgtccgccccgatgaagcccagttgcgacgggtgcagggtgaaggcgacgcgcttgctctctcccggccgcagcgccacgcgcttgaagtccttcaacagccgtcccggctgggtcaggctggcgacccggtcgtggatatagagctgcaccagctcttcggccgcgcgctgtccggtgttggtgacggtgatcgccacttccagttggccggcccattgcaattcggccgcagccatctcgacctcgccataggtcacctgtccgtaggtcaggccgtggccgaaggcgtaaagcgccgtgttcggcgtttcgcgatagcgggacacatattcctgcgtctcgagcgccggatcggcggggcggcccgtggtcttgcgatcgtaggaatagggctgctggcccgacctgtgcggaaagctgatcggcagtcggcccgtggggccgtggtcgccgaacagaacgtcggccaccgcatggcccatctgctcgcccaggaaccagctgaccaccagcgccggcgcgttgcgcaccgcgcccgagagcgcaagcgcccgcccgttcctcagcagcaccacgaccggcttgccggtggcggcgatcgcttcggccagcgcctgctgcggcgccgggatgacgatttcggtgcgggactgggcctcgcccgacatgcgggtgctttcgccgatggccagcaccacgatatcggcgccctgcgccgccgcgaccgccgcctcgatcccgccggccagcggctcctcgacgtccgacccgcgcgcgatggtcagcagcgacggatcgtccatcgcggctctgaaaccggtttcaagcgagacccgacgctcggccgccccccagatcgtccagggcccccagacgttgtccacgtcgtccgcgaagggtccgatcagggcgatgcgctggccgctcttcttcagcggcagcaggtcgccgtcgttcttcagcagcacgatcgacttgcgcccggcctcgcgcgacagggcgatgtgttcgcgcgatccgaccacggccttttcgcgccgctcgtccgtgccgcgataaggatcgtcgaacagccccagcgccgccttgacggtcaggacgcgccgcaccgcctcgtccagccgcgccattgacacttcgccggactgcaccaggccgggcaggtgctccatgtagaggcccgacaccatgctgacgtccaccccggccaggaaggccagacgcgcggcgtcgcggccgtcctcggcgaagccgtgggcgatcagttcctgctccgaggtgtagtcggacaccacaaagccttcaaatccccactcgccgcgcaggatgtcggtcagcagcctgcggttgcccgaggcgggaatgccgttcacgtcgttgaaggcgctcatgatcgacagcgagccggcgtccaccgacgccttgaacggcggcaggaagaccccgcgcagcgtctgctcgctcatgtcggtggtgttgtagtcgacgccgccgatagccgccgaatagccggccatgtgcttggccgtggccagcaccgcgtccggcgcgtccagtcccttgtcgccctggaagcccctcacccgcgccgtcgccagcaggttgttcaacagcacgtcctcgccgccgccctcgacattgcggccccagcgttggtcgcgcgccacgtccaccatgggcgcataggtctggtgcacggccgaggccgcggtctccacggccgccgcccgcgcggtgcgataggccagctccacgtcgaaggcggccgcttccgcgagcggcaccgggaagatggtcgagagcccgtggatcacgtcggcggcgaacagcagcgggattttcagccggctttcctcgaccgccacgcgctggatctcgcgtccggccttggcgccgatgccgttgaacaaagagccgaccttgccctcgcggatcaaggcggtgacccgcgccggatcgcccgtcccgtccagcggattgaccgccatgggcatccagcggaacggatcggccagcagattcagctgcccggccttctcctcgatcgtcatcgcggcgatcaacgcctcgatacgctcgcgatgacgcatgatcgttctcctgatctcggcgcgagcctcggcccgcacgggaactgcgattacgctcgcacccaacgccgtcaagaggccgagccccgagagaacgcgacgacgatcggtcatggcggcgtggcgctttgtggaaatcatgatctcgcggcctcctcgaagaagcgtcgtcgggtagcggcccagcgcctgctcgtccagccgacatgagggcgcactgccgaacaggccgcactggagaggccgacgcgccccctcagggcctggcgagaaaggctgcgatctccgcggctatgcgatccggctgttccaggtgcagccagtgggtcgcgccttccacgatcgtcagcctgccgtcgtcgcacaggtccagcgcggcccgcgcgacatggtgttccagaaaggcgtccttttcgccccacaggatcagcgtcggagtccggatgcggaccggcgtctccggccgcggccgctcccgcagagcgcggtagtagttcagcatggccgtcagcacgcccggccgagaccacgcctcggcatagcgctcgaggtcatcatcgctgaaggcgccggcatgcgcgctccgggccagcatggtcttcatgccggcgaaattcagcgccgccagcgtcgcctccggcagccacggcgcctggaagaagccgacataggcgcttcgcagcatctgggtcggatgcttcagcgccgggccgccccagacatccgggttcggagcatccatgaccaccagccgacgcaggcgctcggcatgccggccagccacggcccaagcgaccaccccgccccagtcatggccgaccaggtcgaacctgtcggcgccgaacgccgcccccaaggccgcgacgtcatccgccaggatgtgcagccgataggcggacagcgcctccggcgcgtcgctgagattgtagccgcgcatgtccgggaccacgacgtggaagccggcttccaccagcggtgcgatctgcaaccgccaagcccaccagaactccggaaagccgtgcagcaggatgagcagcgggtcgccctccctgcctgcatcgaccacatggaggttcaggccgttgacggggaccccgcgttcccgccatccgggctgcaggaggtcgccgttcatcgacgcgcgcgatcaggcgaagctcgccacgccggcgatgatcaggatcaggatcatcagacctgcgagaacgtaccagaccttgggcgtcagccgcaggcccggcccgtcggtctccggtgtcgcattcatcggcgatgagggagcggcggccgcctccgacggcggagcggcgggcgcgccgccagcctccgcatcggtacccagcggcgacaggccggggtcgaagacgggcgtcgcgccgttggggcgctcgcgccattgttcgtccttggtctgcagcgggttgctcatgcgaggctaaccggtccgcccgtccgaggttccgtctccgtctcagcccttgggaggccgcgaacccgcctcatgacgtccgccttccggtcgccgcgcggacaggtcgaagctgtcgccgctggacagcacatgcatgcgcacgtcgaagagggacagggcctgctccggcttggcctcggcgatgttgacgtggctgacgccgcccccgtcgaccacataggccgcgccgctgccgatgacgtcgaaacgctcgctctcgaccaccagcgcggtgttctcgtcgacgcccacgcccaagaggcgcggattgtgcgccaccgcgcccagcagccgaccgaagcgtccgcgctcggcgaaatgctggtcgatgatgacgccgccaagcaagcccagccctggcgccatgtgcagctcgccgatgcggtaggagcccttgctggcccccttcaccagcatggtctcgctcatggccgaggcgccggccgaggttccggccaccacgccgccggccgcgtgcagcgcctggatgcgagtctccaccgccgttcgcccgatcaggctggacaggcgcagctgatcgccgcccgtgaagaacagcccggccgcgccgtccagcacggcgacggccgaggcgatctcctcctgcgagcgatcctcgacatagagttccaccaggtcggtcacgcccagggcgccgaaagccgagacgtagctgtcgaaatagccctcgcgcgtgtgcgaggccacggtcgcgatcaccaggcgcccgccgttcaggcgctcggccacggccttcaggatgacgcgctggtcctccttgtcctcgtgcccgccgatgatgatcaggggacctgcggcgtcagccatggggcggctccagagtgacggccggctgatcgccaggccggaagttcagcacttgacgccagaccgcgtcgatctgggtgggggtcagcaccaccacatcgccgggcctggccatggcgaggcagtgatcgacggcggacgcctcgatgcgcacgccctcgatgcgatcggccgcgcctccggcggagagcgcgccttcgctcatgaggcggatcacttcgccggccgcccgtcctcgattgtccggcgtttcccgaaacacgatgcggtcgaaatccgcggcggcgatggcgcccatctcgacgatttcggcgtctcggcggtcgccaggtatgctcagcatggcgatgcgccggccgcccggcggcgtgatggcgcgcgcggtccgggccagcgcccgcaggccgtccggattgtgggcgtagtccatcacgacccggaatccatgggcgtcatggatgttcagccgaccggggttttgctcgaaggtcgaggcgaagctcgagagcgccgaggcgatcgcctcgggcttgacgcctacgccataggtcatcaaggcggcggccatggcgttggcgacgttgaaccgcgccgctcctcccagggtcgcgggaatgtcgtccgcgtcgcacagccggatagaccggctggcgtcgtgcagggtcaggcagccggtcgcctcgtcgaacaggcaggccaggcctccctcctcgacatggccgcgcagaacccgggggacgtcccgaccgccgctcatcgagaaccagaccggccggcccggcgtcagccgggccatgcgccgggtcagagggtcgtcggcgttcagcacgcacacgccgcgccggctgacggtgcgcgcgacaatggctttcacccgcgccaggtcctgcagcgtgtcgacgccgcccaggcccagatgatcggcctgcacgttcagcaccgcacccacgtcgcaccggtcgaaagccagcccttccctcagcacgccgccccgcgcgcactccagaaccgccgcctccacggtcggatcgcgcaggaccatgcgcgcgctcttcggcccgctggcgtcgccggcgtggacccgctcgtcgccgatatagacgccgctggtgttggtcagcccgaccgtgcgcccgtcggccttcaggatgtgggcgaccatgcgcccggtggtcgatttgccgttggtgccggtgatcgccagcacggggatgcgggcgcgcgagccggtgggataaaggctgcggatgatgggctcggccacatcgcgcgcctggccggcggacggctccagatgcatgcgcaggcccggcgcggcgttgacctccacgacgccgccgcccgtgtcgcggatcgatcgcgtgatgtccggcgccagcagatcgacgccggccacgtccagccccagcgtcagggccgcgcgccgggcgatggcggcgttgtcgggatggatgtcgtcggttcgatccaccgccgttccgccggtcgacagattggctgcaccgcgcaagggcacgaaccggccggcttccggcacggagtccggagtcagatcctgctgcgccagtatgtccagcgcgccctgggccaggcggatgcgcgtcagcatcttttcgtgaccctcgccccggcgcggatcgaggttcacccgctcccccagttccgcgaccgtatgttcgccgtctccggccacatgcgcggggatgcgctcggccaccgcctcgacctggccggcgaccaccagcacgcggtggtcgcgtccgggcagttgctcctccacgatcacacgggcgctgtgctggaccgccagatcgaaggcggcgcgcacgcccgcctcgtccgtcagccccgtcgtcacgccccgcccgtgattgccgtccagcggcttgaccaccaccggcgaggtcagctcccccgccgcccgccaggcttcgtcggccgagcgcaccaccgtcccgcgcgcgaccggacagccgatggcctgaagcatggccttggcgcgcgacttgtccccggccagttcggtggcgatcaggccggtgcgatcggtgacgctggcgcggatgcgtcgctggttggcgccccatcccagttgcagcaggctttgctcgttcaggcgtgtgaccggtatccgccgcctccgggccgccgcgaccaaggccgcggtgctgggcccgaacgatcctcgcttcaccgcctggcgcagcggaccggcggccgcctccgccgtctgcaccgcctccacacggccgtcgtcggccgtgagccgccccagcccccgcgcgccgcgcagatcgtcgggcagcagcgcgtcgacgatctggatcgccagccgtccggccagcagccccgccgcctcgtcctcataggcgtagagggcgtcgtagacgccgggccgctcccggaccgaccgcgtcttgccccgcgtcaccgaggcgccggcgcgcgcctgaagctccagcgccacatgttcgatgacgtgccccagccaggtgccggcctcgagccgccgcaggaacccgcccggcgccccgtagcagcagccgtgctgctggagccccggcagttgctcgaccagcgccgcgttgaagccgggaagacgatcgctcggccacgcctccagcgcgccgagatcgaggcggatgcggatcatgggcagacgcccatacaggtgaggcccccgatagacgctgcgttccagtaccgtgagcggcgccacgggcgtgtcgggggtcatgcggccagacggtcctgaggctgatccgcgaccgtcatgccttggcagagcgcgcgcacgaccagcgccgcggccgccgcccgggtcgcggtccgaccttccccgcacgccacgccgtcgccggcccgaacgatgcgccattgccagccggagcctggggcggggcgcacggtccacgcatatcctggatgagacacatcgccctccggccctgggccgccacgttcgggatggtggaaaccccccagcaagacggcggttcctgtgtcggcccggcgttcgacaatgctggccggaaccgccgacagggcggcggattgatgccgctcgccctcttcttcccgtttgccgaaggacccgccgatgaccgaagacgcgcttgttcgattgctgcgcgagctgggcggtcgcggctacagcttcgtcacgccgacaccctcgacccatggccgggttcgaaggcgcatggatgcgcaggacgcggacctgctgcgcgacgtcttcggctggagccgctcgtttcgcgccgagcagatgcccgatcccctgctccaactcctgaaggaagcggacgggctcgagcccgccggcgatgatcggctgcgggccacgatccgcgtcagcagcctggacgagcgcctttacgtccactccgcgcccacgaacgaccaggatgcggtcttcctcggccccgacagctatcgctatgtgcgcctgctgcaccgggaactcgacaagcgtccgccgatccgcagcggcctggacatcggcgcgggcgcgggggtgggagcgctgaccctggcggcctctgcgccggaggcgcgcgttctgggatccgacatcaaccccaaggccctgcactacctgcgagccaacgcccgtgcggccgaactgcaggtcgaggcggtggaaggcagcggcgcggccggagacggcgctttcgacctgatctgcaccaatccgcccttcatcgccgacgacgccggacgcacctatcgcgacggcggcgaggacctgggcgcggcgctggcgctggactgggcgcgccaggccttgccgcgtctgacggacggcggccggttcatcctgtataccggcagcgccatcgtgcgcggcgaggatcgggtgcgcgacgcccttcaggcgctggcgtcgggcgccggcatgaccctgagctacgaagagatcgatccggacattttcggcggcccgctgaacctgccggcgtatggcgaggtggagcgcatcgccgccgtcggcgccgtcatctccgccgcctgaggttacggccgcgcgtcggtgggcgagttgttcaccgccgcgccgtccccgcgcacggccgactccccgcgagccgcgtcgcctgttccattaccttcaaccgggctcggttgcgcgggcgcggcgggtcggggttcgggaacggccgccggctgaaccacggcgctgcggctgtcgctggtcgcctccggattgcgccacaacgcctccgccgcgatcagccaggccaccagggccgccagcaccacgacggcgagccacacccacggcccccggccttttcgccttttttccacggctcttctccagttctctccggctggtaagcgtcgtcatcgcgacctcgttccgctcagaagaagcgcagcggcatgcccaggcccggctcaataagctgaaccatgcaagtggtggtgaataccacgccgcaaccttcgccgtatcgagtatcgaagccgacaacatctacaacggctttgctgttgttctgaagcgtcgccttacggaacggggccggctctcgcctgttgcctttccgccattcggtgcattcaccaaaaggaacagggctagaccatgtattatacagacaagcttcttcaatatcccgttcgcgtcgagaaaccggaccccgtgttcgcccgcgcgctgcaacaggcgatcggcggcgtcgaaggcgaaatccgcgtctgcctccagtacttcttccaggcgtggggggcgcgcgcggtccggccaagtaccgcgacatgctgctgaccaccgcgaccgaggagatctcgcacatcgagatgctggcgacggccgtggccctgaacctggagggcgcgccgctgtcggtgcaggaagacatctccaacgacaccgccggcggttcggtgctgaacggcatggacatgcgccatgtgctgtccgccggcctggccgccctgccgaccgatgcgaacggcgtcccgttcgacaccagccacgtctacgccagcggcaatctggcggccgacatgatcgccaacgtcacggccgagtccacgggccgcgtgctggccacccgcctgtacaacatgaccgacgatccgggcatgaaggacatgctgtcctatctgatcgcgcgcgacaccatgcaccagcagcagtggctggcggcgatcgaggacatgggcgggctggcggccaacctgccgatccccaacagcttcccgcaggagcaggaaaaccaggagttcagccgcgtcttcctgggcttcaacaaggacggctcgccgccgccgcagggccgctggacgcaaggcccgtcgatggacggacagggcgagttcacctctcgcgccatggagccgctgggccaggagccgaagctcgccccgccccgcccggacgccggcgcccagacgcagcagatggccgaaggctcgacaccgcccggatcggtcaagccgcgcaaggccaaggacggcggcggcctgatggacgcggtcaagcacgcgctggattgatcaagctggcgggcgcggctcggtcgcgcccgcctcctttcccgacaaggagatcgcgatgggcgacgagccgaactggaacaagaccgcgtccgagctgagagcgccggacgccaagcctgatgaacacctgccgcccggcgtcgcccgaggccaccagccaggcgacaccgcccggcaggaccagctgactgacggcggcgtcggccccggcgcggccggggcgggaccggacccggccacacgtccgctgcaggagggctccagcttcgcgcgcgaaggtcaggatccagccgcctacgaacccgttcccaaggcgccgggcgaaacctgacgtcctagagcctcgcccaacgccgggaagaggaccggcgacagcgaggccatcttcgctgcgctgcaacaaacatgttgcggaagcgcctcagctgcgttcagtctgcaacggttgatcgcagcgggggcggatgacgaaggcgtttgacgagatgagcggcgacggatcggggcggatccgtgaaagctatcggacgctggccgcctggctggagcaggcgccgcccgacctgcttcaggcccgatcccggcaggcggagctgttctttcgccgcatgggcgtgaccttcgccgtctatggcgacaccgagtccaacgaacggctcatccccttcgacgtggtgccccgcatcatcgacgcggcggaatgggcgcatgtggagaaagggctgaaacagcgcgtcacggcgcttaacgcctttctgcgcgacatctacggaccccaggaatgcctcaaggccggcatcgtcccggccgagctcatcctcaccaatccgcagtatcggcccgagatgcaggggcgccggccgcccggcgacgtctggtgccacatcgccggcgtcgatctggtccgcacgggcgaggacggcttctacgtgctggaggacaatgtccgcacgcccagcggcgtctcctacatgctggagaaccgcgagatgatgatgcggctgttccccgacctgttcgcagaacaccgggtgcggccggtggacacctatgtcgacagcctgttgcgatcgcttcaggcctcggcgccggcccgggcgggcgaggaccccgtcattgtcgtgctgacgccgggccccttcaactcggcctactacgaacacagctttctcgcggacaagctgggggtggagctggtcgagggcggcgatctgttcgtcaacgacgacaccgtcttcatgcgcacgaccgagggacccaagcgcgtcgacgtcatctatcgccgcatcgacgacgacttcctcgatcccctgaccttcaggccggattcggcggtgggcgtgcccgggctgatggccgcctatcacgcaggacaggtcaccttggcgaacgcggtgggaacgggcgtggcggacgacaaggcggtctacacctacatgcctgaactcatccgcttcttcaccggcgaggaggcgctcctgaagaacgtgcccacctggcggtgccgcgagcccgacgcgctgaaggcggtgctggaccggctggaccagctggtggtcaaggaggtcggcggctcgggcgggtacggcatgctggtgggcccggcggcgaccagggccgagatcgaggcctttcgcgccaagttgatcgccgatcccgacgacttcatcgcccagccgacgctgagcctttcgacctcgcccaccctggccggcggtgcgctggccgcgcggcacgtggaccttcgaccctttgtgctgaccagcccgtccgggacgcaggtgacgccgggcggcctgacgcgcgtggcgctgaagcccggttcgctggtcgtcaattccagccagggcggcgggaccaaggacacctgggtgctgaacgactgatgctttcccgtaccgccgacagcctctactggaccggccgctacatggagcgggccgacttcctggcgcgcatcctggaggcggccatccgcctggccgccctgccggccagggacgacgccgccgtcaccgcctgggccagcgcgatcgcgtcctcgggagtgaaggcggccttcgacgccggcggccgcacgccgtcggagacgtcggtgcgcgacttcctcgccttcggaagcgacaatccgacgtccatcaaggcctgcatcacccgcgcccgcaccaacgcccgttcggtgcgcaccgccctgacgatcgagctgtgggaggcgatcaacggcgcctggaacgggttgaacgagatcggcgaaccgagccgccgcgacgacttcgttcacttcctggatttcgtgaaagcctccgccctggcgatcgagggcgcgacctcgcggacgatgctgcggaacgacgcctactggttcctgcgcctgggcatggcgatcgagcgggccgataacaccgcccgcctgctggatgtgaagtaccacctgctgctgccgccaggcgagcgggtcggcggccagctcgactacttccagtggaccaccctgctgcgcgaagtgtcggccctcaccgcctatcgctgggtgtatcgagaatcggtgcggccgtggctggtggcggacctgctggtgctgaaccggcagatgccgcgttcgctggccagctgccagggcatgatcgtgacctatctggagcggctggcgaccgactatggtcgacgcgggcccgcccagcgtctcgcctccggccgcctcgcccgcttcaacgaggcgcgcatcgaaaacatcttccagtccggcctgcacgaatacatccaggcgttcctggacgagaacaacgcgctcggcgcggcgatccacgagcagtatctggtctgagccatgcggatacggatcgaccacaccacgcggtacggatacgcacgggcggcgcgcttcatcgtccaggtgctgcggctgacgccccgctcgtgcgacggacagcaggtgcgggagtggcgcatcgagtccgacgtcgatgcacgtctgcgccggaccgaggacgccttcggcaacatcgtccacaacctctacaccgagcagccgactagcgccctgaccatccgggtcacgggcgaggtgtccaccgccgacaccggcggcgtgctgcgcgggcaggtcgagaagctggcgccgaccgtctttctgcgggacacggcgctgacgcggccggatgccgacctgaccgcctatgctcgaagcttcgagggcggtcggacgctggaccggctgcatgcgctgatggcggcgatccaccgggacgtggcgttcgaggtgggcgccacttccgccgcccattccgccgccgacgcctttcggctgaggcgcggcgtctgtcaggatcacgcccagatcttcatcgcctgcgcgcggcgtctgggcgcgcccgcccgctacgtctccggccatctcagccgctcggacggcgtctatgaacaggaggcggcgcacgcctgggccgaggcctatgtggaggatctgggctgggtcggctttgatcccgccaacggtgtctgccccaccgaccactacgtccgcgtggcggtcggactggacgcgctgggcgccgcgccgatccggggcgccagctacggcgggggcgccgagagcctgtcggtcgccctgcatgtgcggccggtgcaacaggggcagcagcaacatcagacacgaggctggtcgtgatcgccgcgccgaacgaatctgctagcgtgcggtgatgccgatcgcggggagcgaagcgctgtcatgacctattgcgtcggcatgctggtggacgaaggcctggcgatgatcgccgacacccgcaccaatgcgggcgtggacaatgtgtcctcctaccgcaagctgcatgtctacaaggcccccggcgagcgcatcctggcggtctgcaccgccggcaacctgtcggccacccagaccgccctggccatggtggcggaaggcgtgaagctgccggactccgtaacggaggagacgcttgaaaccgcacccacgctgtttcgcgccgcccagatcctgggccatgccctggcccgtgtgcgcgcgaccctgaacaccccgccgacgccgaccgccgacggcctgaacgtcaacgcctccatgctgctgggcgggcagatcggcggcggcaagatggggctctacctcatctacggacagggcaacttcatcgaatgcggcctggacacgccgtatcttcagatcggcgagctgaaatacggcaagccgatactggatcgcgcgttgcgcgcgggcacgccgctgtcggaggcggtgaagctggggctcatctcgttcgactcgaccatccgctccaacatcgcggtgggaccgccgctggacctgatcatcatgccgcgtgggcgcctggtcggcatggagcggcgcatagcagccgacgacgcctatttccgcgatctcggccagcggtggtcccaggccatggccgatgcgcaccgcgccatgccgaaccccacctggctgaacgccgacgccgcccagcctgcgcacgacgccgtcgcctgaacccctcgacctgctcgctagctgccctcgcttttcttcgcgggagccttacaggaacagcgccgcccggcgtcacgttgaccggcagccattccaaccgagcccctcatgaaactacgcacccgcgccgagctggtttaccgcttcgatccgccgaccgacgccatctacaagatccaggcggcgcactggcccggtcagcacatcgtcgaagagacgctgacctttgatccccccgtcgagtttcaggaggacgaggacgccgagttcggcgcccgcaccctgcgctgccatctggagggcgaggtgaccctgacctatgaggcggtggtcgacaacggccgcctgcagggcctgccgccacaggtgtcgcagcacgactggggtgatctgccggcggaggtgctgccctatctgtcgcccagccgctactgcccgtcggatcagttcggccgcttcgtcacgcgcgcgttcggcgatacggcgggcggtgcgcgtgtcatcgccattctcgactggatcagcgccaacatcgactatgagcacggggtgtcggacacggagacgacggcggcgcgcaccttcatcgaccgcgcgggggtgtgccgggacttcacccatctgggcatgaccctgtgccgggcgtccggcatcccggcgcgggcggtcagcgcctacgctcaccagctggagccgccggatttccacgccgtcttcgaggtctggctggacaacggctggtggctggtggaccccacccgcctggctcccgtcgaggggctggtccgcatcgcctgcggccgcgacgccgccgacatcgcctttctcaccacccaggggcgctgcgaactggtgcgccagacggtgacggtcgagccggcatagacgcgcctcagccgcccgtcgccggctcaacgcccgccgaaggagggcgccggcaggatcacgccttcgcaggggccgaacccgatcggaatgcgaccgggcgccgaggcgcgggccgaaagggcgatctggtcgccgtcctcgacaaaggtgcgtgcgccgccgggaaccgcgaccggctctgcgccgcccttcgtgatctccagcaggcttccgaagcccgagcgttccgggcccgatatcgtcccggtgccgaggaggtcccccggattgagggggcaaccgttcgatgcgtgatgggtgacgatctgcgcgacggtccagtacatgttggtcgccgagccgtgactgagctgaagcggagcctcgcccctgtcccccatctcccggctggcgaggtgcaccttcagatcaaccgacagcgcgccgccggcctgatccgcctcgtcccacaggtagggcagcggatgcggatcgtccgacggacgctccggctgggcggtgaagaagggcgccatggcttcaagcgtgatgacccagggcgagatggtcgaatgaaagttcttcgccaggaagggtccaagaggctggtattcccaggcctgcagatcgcgggcggaccagtcgttcagaagacagaagcccgccacatggttcatcgcctccgcgatagggatcggctgtcccagcgcattgccggcgccgatccagacgccgagttcgagttcgtagtccaggcggcgcgacggaccaaagctcggcgtctcggcgtccggggcccgggtctggccgttcggacgcaccacgggcgttcccgacacccggatcgaggaggcccgcccatgatagccgatcggcacatgcttgtagttgggcaggagcggattgtcgggccggaacagcttgccgacgttctcggcgtgccggatgccgacatagaagtccgtgtagtcgccgatcactgcgggcagatgcatccgcacgtccgccgccggatggagcagaggccgcacggaggcttcatgctgttgttcgctcaacaggcgcgccaaggagcgcctcagcgccagtctttgctccgccggagcgcccatataggcgttcagcgtccggccctccatcacggtcgccggcggcccttgcaccagccctgcggcggatgcggcccggagatcgagcacgaagtcgccgatggccacgccgatgcgcggatcgccctcgccatcgcccggcgagaagacgcccagcggcaggttctggattggaaagtccggatgaccgtcggccccttcgacccagctggtaaggtcgggagcgtgggtctcgtcgatggcggggcggcttgcgctgcgcgtcactggccgggggttcctttctcgaagttcgaccagacgtcgtcgtagtcgagctgcatcgtcggggtctccatggcgtagtccgtcgtgcggatgaccgagcggctttcgaacatgaaggccatggtgttctcgatcttgtggggcttcagctccgccttgacggcgccgtcatagctggcctgatccggcccgtggccgctcatctggttgtgcagcgaggcgccgcccggcgcaaagccccccgccttcgcgtcgtaggcgccgtggatcaggcccatgaattcgctcatcacgttgcggtggaaccagggcgggcggaaggtgccttcggccaccatccagcgcggggggaagatgacgaagtcgcagttggccgtgcccggcgtgtccgacggcgaggtcaggacggtgaagatcgacggatccggatggtcgaagctgaccgtgttgatcgtgttgaagcgccgcaggtcatagcggtagggcgcgagatcgccgtgccaggcgacgacgtcgaacggcgagtggtcgagcgtcgtcgaccacaacccgccctggaacttctggatcagttcgaccggtgcgtcgatgtcctcataggccgcgaccggcgtctcgaaatcgcgcgggttggccaggccgttggagccgatcggacccaggtcaggcagccggaacagggcgccgtagttctcgcagacataccccctcgccgcctcgcccctcagttcgacacggaagcggacgcctcgcggaatcacggcgatctgctgtggttcgacatcaatgatcccgaactctgtgaccagggtcagttcgcccatctgcgggacgatcaacatctccccgtcggcgtcgaagaacgcccggccggccatggagcggttgcaggcgtaaagatggacgccgatcccgactccgtccgccacgttcccgtttccgccataggtgaccagcccgtcgacgaaatcggtcggctccgacggcggcggaagcgggtcccagcgcaggcgattgggcgaaggcgggcggtgaaacggagccgtctccagccgcgacggcgtcgtgtaaggcctgaacgccgcatggttggcggagggccgcagccgatagaaccagctgcggcggttctcatgccggggagccgtgaacgccgtgccggacagctgttccgcataaagaccgaagggggtgcgctgcggcgaattgcgcccgaccggcagggcgcctggcaccgcttcgctggcgaagtggttgccgaagcctgaaagatacgagcggctgtcggcgcgagtgctcgagtccatcgcggccaccgcgacatgatcattcatcggcgcaccctccagcatgaaatctgcgaaatcagtctggacagacccccaactagtgtcaagtgtaaccagatgagcgacaccgccgatttccgccttgaggcctttctgccctatcagctgtcggtcgcgaccaacgccgtgagcgatgcggtcgcctcggtctatgcgccgacccacgggctgcggacgcccgagtggcggttgatcgccgtcctggccgaggcgggaccgctgaccccgctcgcccttggacttcgcacgcgcatggacaaggtgacggtcagccgcgcggcgatcgccctgaccgagcgagggctgttccagcgcacgcccaatccgcacgaccagcggtctcaccttctcaacctgacgccatccggacgcgcgctctatcgggacgtggcgccccgcgcgcttgcggtggagacccgcatcttcgccggtttttcggccgaggagcgacagacgctctcgcgcctcctcgcccgcgccgaagccgccgcgctcgcggcgccggacggtgcttgaaggacgtcggactccgcgccatggagcggtcccggccgtcctgtccgcgtgcgcgtgaaagcggcgcgacacggcgcgacggacggccggtcgaagaagcgtccttgatcggaaccgccgaagcggaccccggctcgcgccctagaagcggcggcccacgcccacggagacgacccacgggtccaggtccacgtccgcggccagcgcgccgttgttgacgtcggcgtcggtgttgaaccagacgcgcttgacgtcgacgttcacgctccacggcccacgcaggccgatgtcggcgccggcctgcagcgcatagccgaagccgtcgtccagatcgacttcgaagccgttcttgtcgtctccgccgtaaaagaccatggcgttcacgcccgcgccgacataggggctgatgttgccctgcgtcagcggtctgtattgcagcgtcacgaccggcggcagcacccaggtcttgtggaccgccacgtccgtgtcgccgccctgcgcgcggatttcatgccgcgtcgtgcccaggatcgcctcgaccgccagatggtcggtcaggaagtaggtgaagcccagcgtcggcatgatgctgtcgctgacatccacacgaaggccgctgtcagcccccgcggcggtgacgatggcgtcgtcggtcgtcggcgccacgtccgtgacgcgcccggtcacgatccagtcgccagcgcgcggcatggtccagtcgccagaggtctgcgccatggccggggcggccagtcccgccacggcggcggccaggagcagggtcttgatgttcatcttgctgtatcccgacgcccggcgccgcgagtgcggccaggaagttcaggcgtcgaaggagtgatgcgccggatggccaagcttcgccttgatccagcgcaaacctgatctcaaaccacgcgggcgtggtgccttgcgctcgcctgcaccagaggatcaaacgcggcgcagaccgcccgcacgaacggtcgtcccgcctcggtgatgcgcacggtcccatcgtcgatgcggaccagacggtcagcgacaaaggcgtccagcgccgcgcgcacgcggctggccgcgcacaggccttgacggtgtcgcgcggcgaccgccgtcacgtccacggcgaagtcgcacatcagccgctcgatcagttcggcgatgaaggcgtcgcgcggcatgatctccaccccgcgcgtgaccgacagccgcccctcgcccaccgcggcccgccagtcccgctcgaccgtcaggttctgggcgtagccttgcggcgaacggctgatggccgaggcgcccaggccgatcagcagcggagccgtgtcgtcggtatagccctggaagttccggcgcagctcgccgcccttcgccgcgaccgccagactgtcggtgcgcagggcgaaatgatcgatgccgatcgcgcgccagccgtgggcgatcagaaagcggcgcgcggcctcgctctgggcgaagcgcagatcggggcccggcaggtcctcgtcgcggatcagcttctggtgcggcttcatccacggcacatgggcgtagccgaacagggcgatgcgttcgggccgcagcgtggcgacctgctccagcgtcgccagcacctcctccacgccctgcaggggcaggccgtacatgaggtcaaggttcagcgaagtgacgccgccggcccgaagcatggccgccgaatgcgcgatgctgtcaaagctctcgggccggttcaccgccgcctgcaccatgggagacaggtcctgcacccccaggctggcgcgcgtcagacccagcgccccggccgccgcgatccactcgtcggtcagcacttccggatccagctcggcggcgaactcacccaagcccgtcaggtcgaagacttccgacaggcccgtcatcaaccggcgcaggtcgtccggagacagcatgttgggggtgccgccgcccaggtgcagccgtccgatcctgatgcgccgccccgccgcccgggcggtcagcgccgcctctttcagcagcagatccacataggcggagatggactccgcccggttcatggcccgggtgttgcagccgcagtaccagcacagccgcttgcagaaggggatgtgcacatagagcgaggcgggctcatccggcgcggcggcgagccagccggcccaggtctcggccccgacggcgggcgtgaactgcgccgccgtcggataggaggtgtagcgcggcgcgtgggcgtcgtagcgggcgatcagctcgcccgtggacggcgccgcgccagggtcacagcgggacatcggtctgtgcatcctggtccgggaccgacaggccgggatcgccttcgtcgaacaggtggaactcgtgccagacgccgttcaggacgccgaagcccaccgcgaggccaagccccagaacccaagcgaaataccacatggctttgtcgcctttctgatcagtagaggtcggggttggtgcgcagcgcggcggtggtcgagcgaccccacagcaccttatagacccacgaggtgtagagaagaatcagcggcaggaagatgatcgtcaccaccagcatgatgaacagggtcacatggctggaggaggcgttccatgccgtgaggctggactgcggatcgatcgagctgggcaggatgaaggggaacatcgacaggcccgccgtcgagatgatgcccagcgtgcccgccgacgatccgccgaacgccagcggctcggagcgacgccccaggccgaccagcgccgccgccgtgccgagaaagcccagggccggcgcgatccccatccacggatagcgtccgtagttgtccagccaggcgccgggcgccgcctcgaccgccgtgcgcagcggattggaccagccgttcggatcgacctcgccgacgatgcggaagcccagaggcccaaaggcgacataaaggccgccggctgcgaacagcaccaggctgaggatcgccgcgatggtgccgtaccggcgggcgcgatctccgatcacgccgcgctcggccttgagacccagccaggccgccccgtgcagcaccagcatggcgaccgacagcaggccgcagatcaggctgaagggcgtgaacagacccagcagatgaccttcgtagaaggaccgcaggttgccgtccaagcggaagggcgcgcccagcagcacgttgcccaccgccacgccgaacaccagggccggcacgaagccgccgatgaacagcgcccagtcccacgccgtgcgccatttcccgtgcggccgcttggaccgatacttgaaggcgacgggccgcaggatcagggccgacagcaccaggaacatggccaggtagaagccggaaaagctgacggcgtagacgaaaggccaggcggcgaagatcgcgccgccgcccaggatgaaccaaacctggttgccttcccaggtcgcgccgatggtgttgatcacggcgcggcgctcttcatcggtcttggcgacaaagggcagcagggcgccgacgccgagatcgaagccgtccgtcagggcgaagccgatcagaagcacgcccagcaggccccaccagatcaggcgaagcgtggcgtagtcgagagggagttccattggaggatgtcctaaagggatgtcgtcaggccacggcgggcacgggcacgccgtcctgggttccggtcaggtcggggccgccggccggtgcggggcgatccagttcctgctgttcgtggaacgggcccttcttgatggcgtgcaggatcaggccgacctcgaccacggccagcgcgccgtagaagacggtgaagccgatgatggtggtccacagctgcggaaccgtcaggctggaggcgcccatgaaggtcggcagcacgccttccacggcccagggctggcgaccgtattccgccacaacccagcccagctcggccgcgatccacggcagcgggatcgccagcacgcacagccgcaggaaccagcgcgtttcgtgcttgcgcagcgtgcacagcacaaaggcgacggcgaaaagggcgatcatggcgaagccgatgaaggccatgaggcggaacgaccagaacatcacgggcacgttcggcacggtgttccaggcggcgaccacgacctggtccggcgtcgcctggcgcggatcggcgacatagcgggtcagcatcagaccgtagccgaggtcgcggcggtgctgctcgaactgggcgcgggcggcgacgtcgttgggatcggccttgatcttctccagggcgtcataggcgatcacaccgctttcgatgcgggtctgcgccagcgccaccaactgcacgatgccgtccacgctgccgtccaggctgcgggtcgagatcaggcccagaacccagggcacctgcacttcgaagcgggtttcgcgcgtcttcatgtccggcatgccgaacaccgacaggctggccggggccggctgggtgttccacatggcctcgatggcggccagcttcatcttctggttgtcggtcagcgcatagccgctctcgtcgcccagcacgaccacggacagcgaagacatgagtccgaacgccgccgccaccgtcatggagcgcttggcgaagcctttgtggcggcccttgagcaggtaaaaggccgagatgcccagaacgaacaccgaggcgatcacatagccggccgagacggtgtggacgaacttggcctgggccaccgggttgaacagcacggccatgaaatccacgacctccatccgcatggtctcgggattgaaggtcgaacccacggggttctgcatccagccattggcgatcaggatccacagcgccgacagattggtgcccagcgccaccatgaaggtgacgaacaggtggacgtgccggctcagcttgtcccagccgaagaacatcagcccgacgaaggtcgcctccaggaagaaggccatcaggccctcaatggcgagcggcgcgccgaagatgtcgccgacgtagtgcgagaagtagctccagttcatgccgaactggaattccatggtcaggccggtggcgacccccagcacgaagttgatgccgaacagcacgccccagaagcgggtgatcgttcgccagatcgggcggcgggtcatcacatagatgctctccatgatgaccagcatgaaggacaggcccagcgtcaggggcacgaacaggaagtggtaaagggctgtcagcgcgaactgcagccttgataggtcgacgaccgcaaggtcgatcatggcgaggctccatggcgctggcccccacgacctgcgccttatggaacacgccctagggttcgggagggcgccgcgccttgatcgagatcaaagagaggcgggcgcggatcggcgtattcgacggtcatgaccgcacagcccctcgctccttcgcttgcgccgcgcccctggctgtccggcgccgcgcgtccgcatcggcgcctcgccggcatggccgccctggcgacgatcgccgacgtggcgcccgccgtgggcttcgcgggcggtctggcgctggcggtccaccatctgccgcagtcgccggtcgccgccgctccctggatcgccctggccgtcgtcgccctggcggcgcgggggctgctcggccagggcgcgctggtgctgtcggcgcgactggcgaggcgggtcaaggcggacgcccggacgagggccctgcaggctctgttcgcctcgccaggctcggccgacaagcggctgacggcggcggtggagggcgtggaggcgctggacggatattacgcgcgcttcgcccccgcgcgcacggccgcggccctgtcgccgctgctgctgatcgccgccgccgccctggccagcccgatgtcggccgccatcctgcttttcaccctggtcccctttatcgccggaatggcgctggccggcacggccgccgcggccgaaagccgccggcagttcgacgccctggaacgcctcagcggcctgttcctggatcgcgtccgagcccttcccgccctgctggccttcggcgcggaggcgcgcacggcggccgagatcgagcaggccgccaccagcctggccgcgcgcacctccagggtgctgcgggtcgcctttctgtcgtccggcgtgcttgagttcttttcggccctttcggtggcgctcgtcgccgtctactgcggcttcaacctcctgcggcttctgccctttcccgcgccggagacgctggatctgccccgcgccctgttcgtgctggcgctggcgcccgaggtctatgcgcccatgcgccggctggccgccgcctatcatgaccgtcaggcggcggaggcggccgcgccggcccttcagacgccccccgtccccgctcccgcgtcgacgaccctcggccgccacgcgccgggcgtctcctttcgatcggtcgcaatcggctatggcgcggcgcccgtgatccaggatctcgacctcgaagtccgccccggccagatcgtcgccctgaccggagcgagcgggtcgggcaagagcagcctgctgcacctgctgctgggtctggtccccctcgccgacggcgaggtggaggtcggcggcgcgcccatgcccccggcggggttcgccggacagatcgcgtgggccagccagaatccggtcgtgctgccgggcacgctgttcagcaacatcgtcctggctcatccgcaggccagccggcgcgaggtcatgcgcgcggtgggcctggccgggctgcacggcgatcttgatcgaccgctggacgagcgcggcggcggcctgtcgggcggggagcgccggcggctgggcctcgcgcgcgccctgctgaagccggcgccgctgctgctgctggacgagcccaccgccaacctggatcccgaatccgaagcccggatcatcgccgtgatccgccgggccgccgagggccgcacgaccctggtcgccacccattccccggccgtcacggccctggccgatcgcgtggtgcgcctgtgaacgcctccggaagaccatcccccgtccgtcgtctgctggccgccgagttccggctgcagcgcccccggctggtcgccgctgcggtgaccggcggtctcgtctcgaccgcctccgtggcgctgctgggcctgtccggctggttcatcaccgccgcagcgctggccggcgtggcgggcgccgccgtcgcccacgccttcaactatcttctgcccagcgcctttatccgactgctggcgatcgtccgcacggcggcgcggtatggcgagcgggtgaccgggcacgaagcgggtctgcgagggctggcggccctgcgccctcgcctgttcgccgccctcgcctcgagccggcccgaccgggcgctgagcctggcgtccggcgaggcctcggcgcggatggttcaggacgtggacagcctgctgacgctgttcatccgtcgctcggcgccgtggagcgcgggcgcgggcgtcgccgccgccgccgccatggcgctgctggccgtcccggccgccgccgccgcgaccttggcggcgatgggcctgggcgcgttcggagcggtcgtgatcggacgacgtcgggtcgagcctgtcgccgcgtcggttcccccggccatgggggcgctgaagacccgcctgtcggcgctgtccgccgccgcgcccgaactgcgcgcctacggcctggacgcctgggccctggcggaaggccaggccgccgggcggaatctggacgccgccaatcagaagaccgccacggccgcggggtggctgatggtctggcaagccgcgaccaccgcggcgggcctggccgtggtgttgctggccgcccgcgacgcatcccagccgctggcggccttggcggcgctggccctggtgatgggaatggagtccgcctccggcctcgtcgccgccctgcgccaggcgggcgcggccgaggcggcgctggatcgtctggacgccctgttcgacgccgatccggacctgcccgcccgggacctgacctccgacaccctctccctcgacggcgtcgtcgccgtctcgccgcctgcgcgcctggcgctcacgggcccgtccggcgtcggcaagacaacgcttctggagcaggtcatcggcctccgttcggccacggcgggcgtcactctgggcgggatcctgatcagcgacctcgcgccggagcggcgccgcgccctgttcgcctacgccgcacaggacgtacggctgatcgacggctccgtgcgcgacaacctgcgcctcgcggacccgaacgcccgcgacgaggcgctctgggccgtgctggaggatgcggcgctgtcggtgcgcttccggaactcacccctcggcctggacacgccggtgggggccgacggccaggcgttgtcgggcggcgagcggcgccggctcggcctcgcgcgtgcctatctgcggccggcgccctggctggtgctggacgagcccaccgaggggctggacttcgccacggaggcgcaggtgctgtggcggcttcagcagagactggcgcgcaccggccagggcctgctgctggtcagccaccgcccctcgcccgccgccctttgcgaacaggtggtcgggatcgagggtgtcgacggggaacgtcggatgcgcctggcgccgaggcgcaacgcgtctcagccctcgccgctggcgatggcctgaagctggtcgggccgcagcacctgaagttcgtgcagggaaaccaggcgcaccacgccggacgccttcagccggctcagcacccggctgaccgtctcgatggtcaggcccaggtagtcggcgatctcggcccgcgtcatgggcaggcggacgtggttgtcgggggcggagcggctgggatcgtgcgacggcaggtccagcaggaacgaggccacccgctcctgcgccgtcttgcggccgagcagcagcatctgattctgcgccgccgccagctcatgcgaggtgcgggtcagcagcgcctgctccaggtccggcgtctcgcgcaccagcgtccgatacgcgtcgcgccggaagcggcacaggctggagacctccatggcctcggcggtaaagccgaaggcctcgccgccggccagccccagaaaatcgcccgcgaacaaaaagccggtgatctgtcgtcgtccgtccggcagcagcttgtagacccgcagcgacccggcggtgacgttgaaaagatgacgcgccggatcgccctcgcgggccaggacgtcgcccggctgcagtgtgaccgtttccgccagggcgttcagccgctccagatccggccccttcacatcgcgacagacgctgaaggcgcgcgcgccgcagcccgcgcagccgtcggcggcctcgcgacgtgcacaagcggcggacaccgagatcatgctcatgccccttcctacaactcgcacggttgagatcaaagtcgttcagccctgacccgctgctgcacgctcgccgcagagggcggccttggtgcgggcggccgggctcgaaccggcaagggcttgcgcccgacggactttaagtcacacacgccagcatcaaccagctgatactttttgctttttaccacatcacgcctggcttgtgtaagaccttgtgtaagtcgggggcgagtgtccgaggatcatgctagggcgtccgccgtgcatgaggcccgcgcggccgcgcgggatcgcccatcaagaagcgcccgcttcagccgccggcgaccaagcgataccccacggccggctcagtcaggatcatggtcggcgtcgcggcgtccttctccagcttttgccgcaactgcccgatcaccacgcgcagatactgagtgtcctcggcgtgcgccgcgccccagacggcgatcagcaggtcacgatggccgatgaccttgcccgcatcccgcgctaaccgggcgagcacgtcatactccttgggcgtcagacggacaggctccccggcgcgcgtcacccgccggtgttccacatcgatggtcacatcgcccgtctgcagcggtccggtcggctcgggccgcccggtcgcctggcgcaggttgacccgcagtcgagccagcagttctcccaccccgaacggcttctcgacatagtcgttcgcgccaagatcgagcgccgcgatcttctcggcctcgcggtcgcgggcggacaggatgatgatggggccggtatagaattcgcgagcgcgtgtcaggacgtccttgccgtccatgtcgggcaggccgaggtcgagcaccacggcgtcgggcgaccacagggcgatgccgcgcagaccttcctgcccgctatccgcgcgcttgggctcatagccggcggcgtccagcgccggggacaggaagcggtggatctgaggctcgtcgtcgatgacgaggatcgcgggacggacggcggacatgggcggctatagcaggtcggggtgggtcgcgatcgccttgggcaggctgatcaggatgcgcgtgccgtggccctcggcgatagggctggccgcggcgatgcggccgcccatggcctcgacgaagcccttggcgatggcgaggccaaggccggcgcccttttgccggtcggagggctcttccatgcggcggaacttgtcgaagacgcgctggagttcaccggtcgggatgccctttccctcgtcctcgatcgagacgaccacggagccgcgatcttcgtaggccgccagctcgatggtggagccgtcggggctgtaggcgatggcgttctccagaatattgaccaccgcctgctccagcagggcctgatccagcatgacaaggctcagtgttgccggaaaatcgcgggtcatgtgacgggtctccaggcgtcgcgagacccgttcggcggcggcgttcagcacatcgcgcacatcggtccagtcggcacggacactcagcccgccgccctccagccgtgtcatgtccagcaggtcgccgacatagcggttcaggcgctcggcctcttcgcggatgctgagcaggaggtcggctcgaacggacggcttcagcgtttcaccgtagtcgatcagcgtcgtcgaggcgcccagcacggtcgacaggggcgtgcgcagatcgtggctgaccgagttcatcagggcgccgcggaagcggtcagcgcggcgcaggctttcggtctcgaccgcctcgccggccagacgcgcgcgctccagcgcgacggcgccctggtccagcagcgccagcgccaaacgctcctcgtcggagccgggcgcgagcgccgccgcctcgacgcccgccacgccggcgcgaccgcgcacgccctcaagcgggcggaaggtccaactggtgttgggcagagtgccggtgccgtggccggctggctcgccatgcgcccaggcccagcgggcggcggccatggcggctgagccgaggttctcggtctgcggcgcgctggcggccagggcgatgtcctcgccctcgggcagcaggacgacggcgcgggctcccgcggcggcggcagtctgttcggccagcacgcgggcggtttcgaagacgccgtcggcgttggtcatggtctggctggcggccagcagggccgagacggccgaggcgcggcgctgggccctctgcgcctgatccctgacacggcccgccagatagccggtgaccagagccacgccccagaacaccagcagggtcagaatgtccgtcggtgacccgatggaaaagctgtaccggggcgacaggaacaggaagttgtaggtcaggaaggcgaccgtcgccgccgccagcgcgggccggaggccatgaatgacgcccgccgcgagcactgcggacaggtagacgacgcccagatccacccgctcgaacgaccgatcgagcagcagggccagccccgtggcgaccccgacgaagccggccccgatcgcataaccggaccatccacgggtgagcggtttcggcggtcgtgcgggcggcgccgcttcctcttggtgatccgtgacgatgtgaatggccacgccgcgggaggcgcgcagcagttccgccgccagagaacggccgaacagttcgccgagccgactgtcgcgtcccttgcccagcacgatctgggtgacgttgttgcgatgggcgtagtccatcacagtgcgcacgatgtcgtcgccggtcagcaccaccttgcgcccgcccagttgctcggccagcttcagggcgtcgctgacccgtgcgttgcgcacggggtccgccgcgctggcgctgggccggtcgatgtgcgtcacggtccagggggcgtccatcatcatatcggacagtcggcggccggtgcggaccagatcgggcgtcatcccgtccccgccgaccagcaccaggatccgggcggacgcggcccaggggccctgcacccccttttcgcgcagggtcgcgacgaggtgatcgtcgaccgtctgggcggcgcgccgcaacgccatctcgcgcagggcggtcaggttctcgatcttgaagaagttctcggaggccagccgcgccgtctcgggcacatagaccttgccctcggccagacgcttgcgcagctcctcgggcgtgatgtcgaccacctcgatgtcgtcggcgttcgacagggccagatcggggatggtctcccgctggcggatgccggtgatgcgcagcaccaggtccgacaggctctccagatgctggacgttcaaagtggtccagacatcgacgccggcggcgaggatctcctcgacgtcctgccagcgcttcggatgacgcgagccgggcgcattcgagtgcgcgtactcatcgaccagcagaagagcgggacgccgggcgatggcaccgtcgatgtcgaactccatcagggcgcgcgccttgtagtcgatcggccggcgcgccatcacctcaagcccgcgcagcaggctttcggtctcgcggcggccgtgggtttcgacgacccctacaacgacatcgtcgctctcggccttccgacggcgcgcggcgcgcagcatttcataggtcttccccacgccgggggacatgcctagaaagaccttcagccggccccgctttcgcagggccggcctcgtcgggtcggatggaccggtgtccggcaagatcagggggccggaatcgggaagcgggcgtccagcgcccggttcgtcaccagcacattgacgtgcggctgaccgatgaagcccagaagggcgccttcagcttgctgatcgatcaccgcctggacctcctgaaccgacgcgccgcgcgcggtggcgatgcgtcgggcctggaggcgagcgtattccggcgagatgtccgggtcgaggccggacgcggacgcggtgacggcgtccgccgggatcgctccgaccccgttctgggcccggatcgccatggcgccttcggccacgcgggtcttcaggtcctcgttcagcggcccgtagttggagcccgaggacgcggaaccatcgtagccgtccccggccgccgacggacggggatgaagatacaccgcgcctgcaaacggttggccgatcagggccgagccgacgacggtcccgtccgcattgcggatcaggctgccgttagcctgggcggggaagacgccctgcgcgatgcccgtgatcgccagcgggtaggcgagcccgagcatcagtgtgaacaatgcgaccatcacgatcgccggacggatcgaccggatcatcagaaggtcgccttcaggctggcgacggcgcggctgccgtacgcatcgccaaaatcatgctcgtcggtgtcgtggtagcggacatcgaacaccaggttgtcggtcagggcatatgcagcgccgatattccaggtggtgtagtcgaagtccgacgacacccactgccggcccagggcgcccgacacggtccagcggtcggccggagcgaaggcggcgttgacctcggcataggtcgcttcgtcttccgaagcgccgaagaagtccggcgaccagaagactgcggcgccgatggtggccgggccgaccggtcgcgaggcggcggccttcagctcgacgtagtcgtaatccagcgcgccaggctcgtcatacaggtagccgacgacgccgaaatcccagttggagccgccgaacactgggcgaacgccggcgtagaggtcgacctccacgccggtgtcgccgtcgccggcgaaggagacgttcgacacccaggccccggcgtagaaggcgccgctggtcatgtcgacgccggcggagacggccgcgtcttcctcggtctggctgacgccgcggaacacatagtccgaggcgacggcgacgttggccgaccattgcgggccctggatgggagcgggggcttcctgggcgtgggcgtgggtggcggggccgcagatcacgaggccgacgaggccggcgccgacgaaccatgcgtcgttccggcccgaggccttccagcggcgtttgcgggtcatggcggtggctttcataagggtcattcgaggggtcatttcagtgttgggtcagtcgctcaggccagtccgaggccggagatcaccaggtcgatgagcttgatactgatgaacggggcgacgaggccgcccaggccgtagatcagcaggttgcgggacagcagggcgccggctccgaccgcgcggtatctgacgccgcgcagggccagggggatcagcgccacgatgaccagggcgttgaagatcaccgccgacaggatcgcgctttccgggctgtgcagacccatgatgttgagcgcgcccagagccggcaggccgaccacgaacatcgccgggatgatggcgaagtacttggccacgtcgttggcgatggagaaggtcgtaagcgccccgcgggtgatcagcagctgcttgccgacctcgacgatctcgatgacctttgtcggatcgctgtccaggtcgaccatgttgccggcctcacgcgcggcctgagcgccggtctgcatggctacgcctacgtcggcctgggccagcgccggggcgtcgttggcgccgtcgccgcacatggcgaccagccgacccttggcctgttcctcgcggatgaggcgcagcttgtcctcgggggtggcctcggcaaggtagtcgtcgacgccggcttccgaagcgatcgccgccgccgtcaccgggttgtcgccggtgatcatgatggtgcgcaggcccatgcgacgcaggtcggcgaaccgctccttcacgttcggcttgaccacgtccttcaggtggatgacgccgacgagcacatcgtcctgcgtcaccgccagaggcgttccgcccgagcgcgcgatacggtccaccgaagcctggaactcggccggagcggtcgtctcgtccaggttcagcgacttcagcaccgcgtctacggcgcccttgcgccacgaggccgcgccgacttcgatgcccgactgccgggtgacggcgctgaacggaatcaccttcgcgccctccggcagttcgatgacgatgctcgcgttgcggcccagttcgacgatcgaacggccttccggagtctcgtctgccagcgaggcggtgatagccgcgcgcagggcgagttcgggacgcacgcccggaaccgggatgacctcggtggccatgcgattgccgaaggtgatggtgccggtcttgtccagcaacagggtatcgacgtcgcctgacgcctccaccgcacggcctgaggtggcgagcacgttcacctcgagcaaccggtccatgccggcgatgccgacggcggacagaagccccccgatcgtggttggaatcagggtgatgaacaaggcgcccagcacgatgggatccaggtccacccccgaataggcgccgaggccgagcagggtcagcaccgcgatcaggaacaccagcgtgagtccggccagcagaaccgacagggccatctcgttgggcgtcttgcggcggtcagcgccttccaccatcgcgatcatgcgatccaggaaggtcgcgccaggggccgaggtgatgcggaccttgatccagtccgacaccacagtggtgccgccggtcacggccgagcgatcgccgcccgcctcgcggatcaccggcgcgctttcgccggtgatggccgcttcgttgaccgaggccacgccctcgatgatctcgccgtcggaggcgatgacatcgcccgcctcgacgaggatgatcgagccgatctcaagctcgctggcgttggtgggaacaaccgcgccggtcgtcgggtcgacgatcagcttggcgctggtcgtgacgcgggtcgcccgcaggctgtccgccgccgccttgccgcgcccttcggcgatgctttcggcgatgttggcgaacagcaccgtggcccacagccacagcgccagttggatggcgaagccggccggctggccgccggcgaccgccgccacggccgagatggtcgccaggaaggcgaccatccaggtggcgaagatcaccgggttgcggaccaggtgaacggggttgagcttgacgaaggcctcgcctagggcgcggccgatcatggcaccggtcatgccgcccgccagcggcggctgccgggggcgatcgcccgccaggtcttcagggtttgcgaaagtcatttcacggatgtccggttcacgccgcggccgcaccggcgagcatctggaagtgctcgacgatgggtccgagggcgagggcggggaagaactgcagcccgcccaggatgatgatgacgccgaccaccagaccgatgaacagcgggccactagtcggcagcgtgccggtcgacggagccagtttcggcttggccgccaaggcgccggcgatggccagaacggcgacggcggggccgaagcgaccggccagcatggcgatgccctgggtcgtgttccaccacggtgtattggcgctcaggccgccaaaggctgaaccgttgttcgccgccgccgaggtgtaggcgtacaggatctccgagagaccatgcgggccgtcgttcagcaggctctcgagcgccgtcggatagacggcggagaccgcgctgaagccgaggatggccagcggaaggaccagcaccgcgatcatggcgaactggatctcgcgcgcctcgatcttcttgccgaggtactccggcgtgcggccgaccatcaggcccgccacgaacaccgccagcatggccatcacgaccatgatcgcgatgcccgagccgataccgcccggcaggatctcgcccagttgcatcaggaagatctggatgcccccggccagcggcatgtagctggcgtgcatggagttgaccgaaccgttggaggcgccagtcgtcgatgcagcccaagcggtggatcccggaacgccgaagcggacttccttgccctccatattgagcggctgctcgatgccggcggcgaccagagccggagccggctgggtctcggcggcatagattccgaccgtggcggccgacagtagcacgaaggcggcgatcacgagggcgcgaacgtccttcttcgccagcacgctgcggccgaaggcgaagaacgccgcccagcccagcacgttgatcgcaacggcggtgatcaggttggtcagggcggttggattctcgaatggatgggccgagttgacgttgaagacgccgccgccgttgatgcccaactgcttgatggccagttgcgaggcggtcgggaacagcgacagggtctgctgtccgccctcgacgccggtggcgctgaccgaggcggccatgctctgcacgacgcccaggccggcgagcgcgatggcaaggatcagcgaggctggcagcagcagccacagggtggtgcgggtcatgtcggcccagaagttgccgacgccctcgctgcggttggcgacgaagccgcgcgccagagccgcagcgatggcggcgccggtggccgcggacaggaagttctgcaccgtcaggcccagcatctggctgaaggtcgacatggtggtttcgccaccatagctctgccagttggtgttggtgacgaagctgacggccacgctgaacgcctgatccggggtcagggcgccgaagccctgcggattaagcggcagcacgccttgcaggcgcatcatcgcgtacaggacgacgaagcccgccagattgaaggccagcagggcgccagcgtacccgagccagccctggctacggctcgggtcgacgcccgaagccttgtagaagacgccttctacgggacgcaggaccgggtcgagccaggtcttctcgccattccaaacgcgcgacagatagatccccagcggccatgcgattagcacggacagacacagagtaagggcgatctccgcccagccttgagttgtcatgaacgcggccccctcagaaccgctcgggtcgcaggagggccgcgaccatatacacggcgacgacgaccgcgccggcgccccagagtatgccgacaaccatcgtcacacccgcttcaggaaaacggcgagcgcggcgaaggcgagaaacgccgcgccgccagtcgccagaaagatcagatcggccatgccgacgcctccgactgttggaagctggacaggaccgcgaaaccgcataagcgcgccattggggttcagggctggcgcataaggaaaccataaggggagcggggcgaagcttacggccggcttatgcgggcgacggcgatccgcatggcgcgcttacggccatcggcgctgcactggcggccctcgaaaggaggtctccatgacccgcaatcacctgctcagactgtcaacccgggcgcggccagcgaaccagctcgtcgtctggcgcatgaccatggatctgctcggcttggcctttggtgcggccccgagccgccgggagcctcgccgatgatggccggctactgttccgaccgccatagccccgcagccgacggctcgcgccgctacacggtcgtgccccgccccggcggctggagcgtctcggtcaatggagcctgcacccggccgttcgccagcaaaggcgcagcccagcgcatcgcggcgacgctgcaacgtcaggcggacgccctgcgaggccgccgatgacagcacgctccgccgaacctccctcctggatgatcgtccgcttcaccggaaaactgtggcgggtcacctcgaatgacgggtcttaccaggggactttcatcgatcgccgcagcgcggtgcgggaggcgatcgccgaagccgaggcgcaccgcgcttcctgaggcgaggctgccgctggcttccgaattgtgccggtgatcggtgtgtcctgccgtggtgcgggcggccggactcgaaccggcactccatcggacccgagttttaagctcggtgcgtctaccatttcgccacgcccgcgcgtctcagcgacaccaccgtaagtttacggaatgtcgctacgacgaggagcgactaaactcgccccacatcgacgctatacagcgagcgagcgtacaggcgcgcgattttttaagtccgttgcgtctacctgtttcgccacgcccgcgaaccggcgctccagcctataacggaagccggagcgcctcgccaacgcggttcagggggttgtcgtcgcggtccgcagagtccggaaatcgacgtcggagtcggcgatcagccagatcagcccggcccaggcggccacgttctgggtcagttgcgccgggtcgatcttgtccagggtgtcgtcggcggtgtggtgcaggtcgaagtagcgcgtgccgtcctgagccagggtgaagacgggcacgccggcttccgccagtggaccgatgtcgacgccgccgtgcagctcgggctcggccgaggccagaacgccgatcgggcccagcacgcgggaggcggcgcgctggaactccgtgcccgcgcccccgggcggcaggcgcagggcgtagacgcgatcggcgccgaagtcgctttcgcccgccacgatatggtcggacaccgcctcgccgatcccgcgcacataggcgccgccgccgttgccggtattggtcggctgggacacctcttcggatccgtaaagcaccacgcgaatggtgcgcgctgggcggcggccggactccatgatcgtcttggccgccgcgatggtgatgccgccgccggccgcatcgtcgatggcgccggtgcccaggtcccagctgtccatatgcgaacccagcacgatcacctcgtcgggacgcgagcggcccggcaagtccgcgatcacgttctgcgaggtcgtctcataggtgcgggcggtggaagacaggcgcaggcgcaccgtctcgccgcccgcgaccatgcggctgatctggtcggcgtccggcgcgctgagcgcaaaggccggaagggtcgggcggccctcgacgtagcgggtggtgcccgtgtgcggcatgcggtgctcgtcggtgccggccgaccgcatcacaaaggccgccgcccccttcttcatcgcctcggcgggaccggcgctgcggatgcgcgacagcacgccgtagccggagccgtcctgcatccgcaccatctggccggcgtcgacataggcgatccggccggacagcgatccctcaggcgccgccatcagggcctcaaggctgtcgaagcggaccacgtcgccttcgacgccgccggccggcgtggcgggcgaatggcccagcgccgccgcgacgatccgttgcggacggggcccgatgatcgctgcgctctcctcgccccggtcccagccgaccaggggaaagctctcgatgcggacgtttcggaaacccaattccttcagatagtcggcggcccaggcggcggcctcctgctccgaacgcgacccggccgggcgcgggccgaagcgggtcgtcagccgggtgacgtagtcgagcgccacattctccttcagcgccgcatcgcgcacggcggccgcgcgctggacggtctgggcgtcctgggctgcgacaggcgcggcgacgaggccgagcgcaagcgcgctgacggccgacagcagacgaagagacatgggcgaacagctccggattcggaaagccgaaccgtagccccgcgttcaagccggggtaaagccctcagccgttgcggaagtagggctcgaccggcccctgcagcttgacggtcagcgccttgccgcgccggtccacgcccttgccgaccgccagccgcacccagccttcggagacgcagtattcctcgacattggtcttgtcctcgcccttgaagcggacgccgacgtcgcgctgcagcacttcggcgtcatggaacgggctgtcgggatcgacggacaggcggtcgggcggagtgtcggacatgaggcagacctcggaaacggcggatcggcgggctgaatagcggcggcggcgcgccctgccaaccgatcaaccgcgcatcaggcctcggcggcccggcgcagaccttcggcgatggcctcgtgcacgcggcgcagggcgttgcggtgcttgtcatggaacatctcgccccgaagccccgagaagatcaggccggaggcgacgatgcagctgcccttctccagttcctcgatctcgaaatagcgcacggtgttgaacagaaagcagcgtttctccgcccacaccagctgggcgcgcggctgccattcgcccacgcgcccctggacctggcgctcaggcaggcccggcaggcgctcggtcatggtcaggacgccgccaaaggcgatggtcccgctcacgtccgtctcatgcgggttccatcgatcccaggacggcaggtcggagatcagctcccagattcggtcggaggtggcctgcacgccgacgcgcttttcgatgcgagtgtccatgggtgtgatttcgcacgcctttccggcgagggaaaggcgtcagccgccctccaccagcgtcagcgccggcttgccccggcgcggatcggccaggcccagccgcgccttcacttccaggaggtccgcgccgccgggcaccaccagcagcgcctccggctgggcggtgttcaccgccaccaccgcgcccttgggacacaggccgaaacagtcggcgccgaccacggccagttcgtgcttgcggcccttcttgcccttgggcagttgcagatagcggcgcagcgcctttttcagcgtcagatcgccgtcgggaccaaagcctccatccagcttcttggagcatttgcggcagaccagaacgacctgccgccaatccgtcgatgcgctcttgatcgccatgaaccgaacatcgggtgcgccgggcgcctcgacaagcgaagctttcgtgtctcagccgccgagaacgcccagccgcgacggcgccgtctcgatcacccggcggtagatgtcggtcagctccagaagttcggcggtcggcccccgctcgtcgatctggtgcatggtctggccgaccagccccagctccagcaccgggcacaactggcggatgaagcgcgcatcggacgtgccgccggtagtggaggcctcgggccgacgccccgccacggcctcgaccgcgtcctgcaccgccccgacgaaggagccggactgcgtcagaaaagcctcgcccgagcactggtgctcaaggctgatcgacaggcccgaggccgcctccgcctcccgcgcaaccccatccagccactgcatcagcccaacgcccgtatgcgcgggattgaagcggatgttcagccgcgcgcgcgcctcggccgggatgacgttggtggcggtgttgccgatgtcgatggtggtgatctccaggttcgacggctgaaaagcctcatagccttcgtccagcacatgggcgtccagcgtggccagcaggcgagccaagaccggcgccggattggccgcgcggtccggataggcgacgtggccctggcggccccgcacggtgatccaggtgttcagggagccgcgacgaccgaccttgatcatgtcgcccagcagttgggccgacgagggctcgcccaccacgcaggcgtcgatgcgctcgccctcggccaggagctgctccaccacccgcttggtgccgtgcagcgccggtccctcctcgtcgccggtgatcagcagggacagcgacccttgcggctcgccctgcgccagcacgcgcgagacggccgcgacccaggcggcgatcccgcccttcatgtccaccgcgccacggccgaacagcacgccgtcgcgaacctctccgtcgaagggccccacgctccactgggcatccgctccgaccggcaccacgtcggtgtggccggcgaagcagaggttcggcgccgtcgttccccgacgcgcatacaggttctctatgtcctcgaaccgcatccggcggcagacaaagccgaggcgcgtcagcacctcctccagcacgtccatcgcccccgcgtcggcgggcgtgaccgacggcctgcggatcaggtcgcggcacagttcgacgggatcgatcacgggaaggggtgcgcggctcatgcccgcatgctttagggggatcgcaccgccgcgagaaggcttcgcgccgtcccgccgccaggagttcgcatacagccccgtgaccgacgccgccgcccaacccgccagcccgccgcccgcctcgcccgagggcccctccagcccctgggcgatccgcgacttccgcctgctgtggctgggccgcgtggtggcggtgctgggcatccagatccagtcctcggccctgttgtggcaggtgtatgagatcgcgcggcgcgaccatccgatcgagcaggccagcctgtatctggggctggtcggcctgtgtcagttcctgccgcttctggcctttacgctcccggccggcgccatggcggaccggcgcgaccgcaagcgcacggtcgccctgtcgatcatcgtggaggcggactgcgcgggcgcgttcctgctgatggcgctgcacggatcgccgcccctgtggggccttctggcggtggcggccctgtttggcgcggcccgcgctttcctggcccccgccagccaggcgttcttgccgatggtggtggggcgaaaggccctgccgcccgcgatcgccgcccagtccatcgcctttcagaccggcgccatcgccggcccggcgctgggcggagtgatcgtcgggatcaacgtgccgctggcctatgcggtggccatggggctgttcctgctgggtgtggccgcgtttctcctgatccgcaccagcggcaagccggtggtgcagccgaacgctccgtcgccggtcgcggccgtgcgcgaaggcctggcctatgtctggaagaccaagatcgttctgggcgccatctcgctcgacctggtcgtcgtgctgctggcgggcgtggcgctgctgacgccgatcttcgcgcgcgacatcctgcacgtggggccgcaagggttcggcctgctgcgcgccgccttcggcgtcggcgccctgctgatggcggtctatctcagccgccggcccatcgtgcggcacggcgggcgctggatgttcgccgccgtcgccctgttcggcctgtgcaccttgaccttcggcctgtccaagagcgtgtggctgtcgggcctggtgctgttcatcggcggcgcggccgacatggtcagcgtcaacatccgccagaccctgatccagctggccacgcccgaccacatgcgcggacgggtcagctcggtgtccatgctgttcatcggcgcgtccaacgaactgggcgaggcctattccggcgtcgcggtgcgcttcctgggtcccatcggcgcggcggcgttcggcgggatcggcgctctcgccgcgacgggcgtctgggcgaagatgttccccagcctgcgcaaggccgacaagctgacctgacgccggctcaggtcagcagcgccttcagcaccccgtccagcaccggccgtccccgctgcgtggcgaccagccgctcgccctcgatccgcaggaagccgtccgcgatcaggctctccagcgcccctccgcccgcacgcagcccaagcggcgcaaggttcgccagcggcacgccctcgacggtgcgcaggcccagcagcgcccgctcctccgccgcctccgccgcgtccatcgtcgcctgctcggcccaaggcgcgcccgtaacgacgcccgccacatagtcgccgatccggcggtgggccacggttgcggtgcgggcgccctccagcgtcagccgcccgtgcgcgcccggccccagacccagatagtcgccgcctcgccagacatgcagattgtgcgccgaccgcgcggccgtcccccgcgcatgattggacacctcataggcctcgaaccccgccgcgctcagcacctcctgcgtcgcctcgtaaagcgccgcggcttgatcctcgtccggcgggatcagggcgccgcgacgcagcgccctcccgaacgccgtctccggctccaccgtcagctgatagggcgagacgtgttcgaaaccgagcgccagcgcttggatcagttcggcggtccagccctccaccgtctgctccggcctcgcatagatcaggtcgatcgacaggcgcggaaaggcccggcgcgccgtctccaccgcccggatcgcctcgcccgccgagtggttgcgcccaaagaaccgcagcgaggcgtcgtccagcgcctgcacccccatcgacagccggctcactcccgcctgcgccagttcggcgaaacgtccggcctccgcgtcggtgggattggcctccagcgtgacctccaagcgaccggagggctcaaacagccgccgcgcctcctccacgatcctcgccaccgcctccggcgccatcagcgacggcgtgcctccgccgaagaagatggaggctagtcggcgcgcccccagcatcgccgcctgcgcgcgcaggtccgaaaggatggcctcgaccagcgccgcctgctcctccgcccgcccccggtcccgcaccacgttgaagtcgcagtaggggcagatgcgcgcgcagtagggccagtgcacatagatggcgacgtccgttcccggatcgggcgtcgcgcgggacggctcagtcaatcagcgccgccttcagcttctcgaacgcgcgggcgcggtggctcatggcgtccttggcgtgcggctccatctcgccgaaggtgtggtcgaagccgtccgggcggaagatgggatcgtagccgaagccccggtctccgcgcggcggaaaccccagctcgccatgcacctcgccctccaccaccacgcacggcccgtccggccaggccaccgccagggccgaggtgaaccaggcgcgtcggtcggtcgcgccgacctcctccagccgctcctcgaccttgcgcatggccagggcgaagtccttggtcggtccggcccagcgtgcggagaagacgcccggcgcgccgtccagcgccgccaccgacagacccgaatcgtcggccagcgacacctcgcccgacagccgcgcggcgtgccgcgccttcagcatggcgttgccggagaaggtgctctcggtctcttccggttcgggcaggttcagctggccggccgtgacgatctcgtaatctccgcccagcagagccgcgatctccgggaccttgcccggattgtgggtcgccgcgacgatccgcatgcccttgatcagcttcatcatttccgacgggcctctcgcattgccaaaacgtaataccgataaacgatatgtaacgtgaataaagccccgggcgggactactcattagctcaaggacggagaacaaaccgcccccgcttcagatcagaacctgaaacagattttcgacagacctcaacccacgggcatgaaccgcccaatcgaaagagacccgccatgcacacgatgaacgcctcgctgatgatggacaagttcggcgcagccttcctgaacaccgtcctgctcgccgccctgccgaccgccctggtcgctgtgctgttccaggccctctgatcggtcgcttcatcccttccgatccacgagagctttgacgatcttgcacaagacagcgatgaatggcgccgcgacggggttcgccggaccccgcgcggcgatctcgccccgtcttccggcctgaagaggcccgtcccgccccatgcgcccgcccaagctgttgcggatcagatcgggagagacgcatgcgccgaggcggatggacccggcctggatgcggaacgtgcggaccatgggtcccggttcgctgtccagcttcctcaaggtcgtgctggacgtggcctgggtgcttctgggcctgatcaccggcgcgcttttgatccttctggtcgtggcgatcttcatccccatgaccaacctcaacatcaccgtgtccagcggcggcgacggacgccagctgccgctgacccgggccctgctggtcttcggcgtcggcgccctgaccgcctatttcggcggcttcatgctgatcctgcagggcctgcggaagattttccgcaccctgaccgccggcgaccccttccaccccgacaatgtgcgccgcctgcgccagatcggcctgaccctggccctggtcaccggcggcgtctgggtggcgcaaggctttgtcgccgcccggctagcccccggcatcatggacccgcaagggttcggagagctgctgacgccgatcttttccgttttgatcgtattcgtgctggccgaggtgttccgcgaaggcgcccggctgcggcgcgaatccgaactgacgatctgagcggactggtgtaggcgacaggacgaccatggccatccgcgtgacccttgaccgcgttcttctggaacgccgcatgtccctgaccgagctggcggatcgcgtcggcgtgaccgtggccaatctgtcgattctgaagacgggcaaggcgcgggcggtgcgcttctccaccctggacgccctgtgccgagagctggagtgccagcccggcgacctcctggcgcacgagccggggccgcccgccttcgacgacgatctggaatgagccgccgacgcggccccgagcgtgatgcggacggcctgacctccgaggaccggcgcatctgggcgcgcgtgtccggcacggtggctcaacccaaggtccgcaaggctcagcgcgtgccggtcgccggaccggaggtcggaacgcccgccgaacccgcagcggcgaaaccgcgccgcaccgccgccgcagaagctccgccgccgtctgtcctcgaccctgtcgcaccccgcctggccaagccgcgcgccgctccggagacgctggagccgcgccgtcagcgccggctggtgcgcgagcgcgaacccatcgaagcgcgcatcgacctgcacggcttcggccgcttcgaggcggaggatcagctgcgcgcattcctgctgggcagccaggcgcgcggcctgcgcgccgtgctggtcatcaccggtcagggtcgccggggcggcggcgtgatccgcgcctctttcgaggaatggctgcacgcggcggcgctgcgcggcgtggtgtccggcttctcgtccgccggccgccgtcatggcggcgaaggggccttctacgtcaccctgaagcgacggacctagccgaccgtcagcccatgctgcgccgccaaatccttgagcggcgtcatcggacgcggaccccagtgggcgatcacttccgacgccgccagcgaacccagggcgccggcctgatccagcggcaggccgcgcgcgagacccagcagcaccccggcggcgtactggtcgcccgcgccggtggtgtccaccaccttgtccaccgggaaggccgcgaccgtcgcccgctcttcagcgcgcaggatcaccgagccggccgcgccgcgtgtgatcgcggcggtctcgacgatcgcggacagcttctgcgccgccacgtcgaagtcatccgtctcgaacaacgccgccagctcgccctcgttggccaggacgatgtcggccgaggcctcgataaaggccagcagctcggcccgccagcgcgcgaccacgaaggtgtccgacagggtgatcgccaccttgcggcccgccgcgtgcgcgatctcggccgcacgctcaaacgcggcgcgcgcgtgaggcgggtcgaacaaatagccttcgaggtagacgatggcgctgtcgccgatcacgtcggcgtcgatgtcgtcggggaacagctggttggccgcgcccagaaaggtcgccatggtccgctggccgtccggcgtgacgttgatcaggcaacgcccggtgccgaaaccgcgctcggccccgtcggcgagcgcgggcgtttcgaagtggaccccaaccgcgcggatgtcgtggctgaacacctcgcccagcgtgtctgcggcgcccttgccgacataggctgcgcggccgccgaacgatccgacgcccgccaccgtgttgccggccgatccgcccgacgcctcgacgcccgccgccatggcgtcatacagcgctgcgctctggtcggcgtccaccagttgcatcgagccgggggcgaggccctgcgcggccagaaaggcgtcgtcgcacgggctcagcacgtcgacgatggcgttgccgacggcgcagacgtcgaagcgggcggaaggaatggtctgggtcatgcgccgcccatagcgggccgcacgcctgcgcgccagcacccctaggcgcgcagccccgtccgccctatgcggagccgacgtcccgccgcaggagccgcctcgatgaccgcgatcgccgtcttcactcccgatcccgccgatccctcctacgccggccagtggccgtcggttctggagcggctgtcgcaggccctggcgcgcgaggggatcacggccgcgcccacgccctggaccgaccatgtggagggcgcctcaggcctgctcgcctatccgctggtgctgccggtggtgtcctggggctatcaccgggatcacacgcgctggcttcagggttgcgaaacctggacggccgcgggcgttccgatggccaatccgacctcggtgctgcgctggaactcggacaagacctatctgggccggctggcggagcgggggatcgccatcccgccgaccctgtggcgcaccgacgtgacggccgccgacctcgacgccgccttccggcagaccggcgccgaaaccctgatcgtcaagccgacggtgtccggcggggcctggcgcacgctgaagatcgggcgcggcgatccgccggccgacctgcccgtcgggtcggtgatgatccagcccttcctgccgaccatccagaccgagggcgagacctccatgctgttcttcggcgggcgcttcagccacgccgtcaacaagcgccccgccgccggcgacttccgcatccaggtgcagttcaacgggatctacacgccggtccagccgcccgcaggcgcgctggccctggccaaacaggttctggccgccattgacgagccgctgctctacgcccgcatcgacacggtgcccgacgcggacggccactggcgcctgatggaggccgagttgatcgagccggacttctacctcggccacgatcccaggggcggcgcaggcttcgcccgcgcggtgcgcgagcggctggagcaagcctagggccgcgtctggcctgtcccgcgcaccacatatttgtaggtcgtcagctgctcggcgcccaccggcccgcgggcatgcagccgggcggtggagatgccgatctcgccgccgaagccgaactcgcccccatccgcgaactgggtcgaggcgttgaccatgacgatggcgctgtccacgcgggcagcgaagcgttcgcccgcctccgcgtctgtggtgacgatcgcctccgtgtgccccgagccgtaggtgcggatgtgcgcgcaggccgcctccaggtcatcaacgatccgcacggccaggatcggcgcgaggtattcggtcgtccagtcgctgtcggtcgccggaaccatgccgggaaccagcgccctcgcctcagcatcgccgcgcagctcgcacccggccgccatcaggtcggccgcaaccgcgggcagtaggcgcgcggcgcccgccctgtcgatcagcagggtctcggtcgcgccgcacaccgacacccgccgcatcttggcgttcagcaccacggcgcgcgccaccgcctcgtccgccgcgtggtgcagataggtgtggcacagcccctccaggtgccccagcaccgcgacccgcgcctcgtcctgcacccgttggaccaggctcttgccgccgcgtgggatcagcaggtcgatggcgccgtccaaccccgtcagcatcagccccaccgcctcccggtcggcggtgtccaccagctgaaccgcctcgcgcggcaggcccgcctccgccaacgcctcgcccaccgccgccgcgatcgccagcgacgactgcagacagtccgaaccgcagcgcaggatcgccgcattgcccgagcggatgcacagcgccgccgcgtcggccgtgacgttgggtcggctctcaaagatcacccccagcacgccgatgggcgttcggacccgcgcgatgtccaagccgttcgccggcgtccagcgcgccatctcggcgccgagtggatcgggctggtccgcgatctgctcgacggcatggaccatgccttgcacgcgtgcccgcgtcagcgccagccggtcgatgagggcctcgctcatccccgcctgccgcgccgccgccacgtcgcgcgcattggcctgcaggatggcgtccttcgcctcgccgatccggcgcgacagcgctctcagcgcccgcgtacgcgcctcggccggcgccgaacggagggcctccgccgcctctctggcctcccggcccatagccagcatccggtccttcatcacgcctccagcaccagatcgtcgcggtggatcagggcggcgggacccggatagccgagcagggtctcgatctcgtcgctgcgccgcccccggatcagcgcggcctcgcgcgccccgtaggcgaccaggccgaccccgacacgccgccccgccgcatccagcagccgcacgctgtcgcccttgccgaaggcgcccgccaccgccgtcaccccggccggcaaaaggctgcgcccggcccggagagcccgcacggcgccatcgtccagcgtcagctcgcccgccggctgcacgctgccggcgatccaggccttgtaggcggccatgggggtgtccggcgcggtgatcagcgtcgcccgcgcgccctccttcagcgccctcagcggcgacggcgcctcgcccgaggtgatgatcgtggcgcatccggccgcccgcgcgatggcggcggcctgcagcttggtcgccatgcccccctgcccaccccgccacggcgttcgcgtctccgcccatcgccatgatcgcgggcgtcagcgcctccacccgcgccagatgacgcgcgccgggatcgcggcgagggtcggcggtgtagaggccatccacatccgacagcagcaccaacaggtccgccctggccagttgcgcggttcgcgccgccagccggtcgttgtcgccgtagcaaatttcctcggtggccaccgtgtcgttctcattgaccaccggtacgaccccgtggcccagcagcgcttccagcgtcgcccgcccgttcagccagcgcctgcgccgctcggtgtcgtcgcgggtcagcaggatctgtccgaccaccagcccgtgcggctccagcgcctcctgccacgcctgcatcagcagcgactgaccgaccgaggccgccgcctgcttgtccgccagccgcagggaaccgccgctcgccagccgcgcccggcccagcgcgatcgagccggaggagaccacgatcacctcgcgcccttcacctctcagccgcgcgatgtcggcggcaagcccggtcagccacccgcgcgccgcgcctgcgccctcccggtcgatcagaagcgccgagccgaccttgatcaccacgcgtcgcgcgcgcgccaaggcgtcgctcggcccagcagcgttcaagacggcgtcaatccccatggggccagcataaacgccgcgtcccgccttgtctccgccgcgcaagggcgccaagccgcgaccggcccgtcacgcggctgagacatccgcggcctagacggcgccgacagtcaggattgttcgcccatgtttccctcgcgccgcgcccttgcgctcagcctctcgcttctcgccatgccgctgccggcgctcgcccagacggcgccggtcccggccgcgcagaccgccccttcggcgcccaagctgatcgtgacggtcgtggtggaccagttcagcgccaacctgttcaaccagtatcgcagccgcttcaccggcgggctgaaggccctggccgatcagggcctggtgcacgccaatggctatcaaacccacggcctgaccgagacctgccccggccactccacggtgctgaccggcatgcacccggccaccaccggcatccccgccaatgactgggtcgatgcaaaaacgggccaggaggtctattgcctggccgcaccgcagaacacgctggcgcacgggcgcaacaccgacaacgggccggtcggccccgatcagctggaggtcccgaccttggccgactggctcaaggcccagagcccccagagccgcgtcttcgccgtatccggcaaggaccgcggcgccatcaacctgaacggccacaccggcgacggcgcctactggttcaccgaaggcttcggcctgaccacctatgtcgagcccggccagacggccgaggcgcggcttgagcccgtcgccgccttcaacgcgcgtctctccgagacgctgaaggcccagccgccggcctggacctacgcctttgaagactgccgcgcgctggagggcgactggaccatccgcgacgtcgccttccactcgaccgttccgcccgccaactacgccctcgacagctcgccgcagctggacgagatgacgctggaggccgccgaatatctgctggagacccaggcgctcggccggcgcggcgtcaccgacatgctgggcgtcagcctgtccgcgaccgaccggatcggccacggctacggcacgcaggggccggagatgtgcgagcagatgcatcggctcgacgccgccctgggcgagttcctgaccaaactgtcgaatgtgcccggcggcgccctggtggtgctgaccgccgatcacggcggctccgatttcgtcgagcggctggccctgcgcggctatccgcaggcgcaccgcgtcgatccgcagggcatgcgcgacgtcaacgcccggctgcgcgagcgcttcgacctatccgccgatccgctgcaatccggcggaagcggacttctggtcgccgacgcccagcaccgcgccctgcccgagcccctgcgcacgcaggtggccgaagccgccgtcgagctgctgcgccagacgccggacgtggctttcgccgaaacgcgcgagcgcctgctggccgaacccatgcccgcctcgaccctgaaccccgagatgctgacgctgcgcgagcgcatgcgcctgtccacggtggcggaccgttcgccggacatcgtcttcgcctgggcgccgaacgccgtctccggcggtcgcgtcggcggggccgtcgccgggcacggcacgccctgggactacgaccggcgcgtgccgatcctgttctggtggccgggcgcgaccggccaggagcgtttcctgccgatccgcaccatcgacatcgccccgacgctggcccacgtcatgggggtgcagacgcctcggctcgagggccgctgcatcgacctgggcggcttcggaaccgcgccctgccctgcgcccgggccgtaaactgttgtttccgaggcgccgcgcggacttacctcgcggaagtttcgttggcagaaggccgcaagcctgaacgccgaccgcttggggaagcgggcgtcaggatcgaggacacgccatgaacagagcccgccgcgcccgcatcgtcgccaccctggggcccgccagccgcgcccccggcacggtgaaggccctggcccaggccggagtggacgtgttccgcctgaacttcagccacggctcgcatgacgaccacgccgcggcgctgaaggccgtgcgcggggccgagatggcgctgcagcgcccgctgggcgtcctggccgacctgcaggggccaaagctgcgcctcggccgtttcgccaatgtcgagatcgcggtgaagccgggccacaccatgcgcttcgacctggatcccacgccgggcgacgagacgcgggtgcagatgccgcatcccgagatcttcaaggccctgcgccccggcatgctgctgctgctggatgacggccgcgtccgcctgcgcgtgggcgagcgcacagacgagtgggccgacgtcacggtcgaaagcggcacgaaactcagcgaccgcaagggcgtggcggtgccggacgcggtgatccccgtctcggcgctgacgcccaaggaccgcgaggatctggccttcgccctgcggctgggcgtcgactgggtcgccctgtcgttcgtgcagaagcccgaggacatggccgagctgaagcagctggtgaagggtcaggccgcgtgcctcgccaagatcgaaaagcccgccgccctgacggacctcgaagccattctcgactactgcgacggcgtcatggtcgcgcgcggcgacctgggcgtcgagatggacccggaagaagtgccggtggcgcagaagctgatcgtgcgcgccgcccgcaatcgcggcgtgccggtaatcgtggcgacccagatgctggaatccatgaccagcgcccccgcccccacccgcgccgaggccaccgacgtcgccaacgccgtctatgaaggcgccgacgccctgatgctgtcggccgagaccgcctccggcgactatccgctggaagcggtcggcatcatggaccgcatcatgcaacgggtcgaaaaggaccccctgtggcccaccctgatggcgtccgaacacctcggcatcgacgaggacgtggacgccctggtcggcgccgcgcgaaaggcgacggatgcgccctccaccgcctgcgtggtcgccttcaccaccctgggcggcaccgcgcgccgcatgtcgcgcgaacggccgctgaagccgatcctggtgctgacgcccaaccccaacaccgcccgccgtctggcgctggtctggggacttgagccgcgcctgggcgagcagccggactcgctggaggccgtgaccgacgacgcggtcaacagcgcggtgaagttcggcctggcccagcccggccagcgcatcctgatcctggccgggacgccgttcggcgcgccgggcgccgccaacctgctgcgcctcgcccacgcgcctcagccgaggacgaaaaagccgcgccgctgaagccccgactcgcgcgaacggcctcgcccgtcctatgctgaagacggtgacgcggggccgggcatgatcaaatacatcggctccaagcgggcgctgctggcgccgctcaccgccgccgtgcgcgccgtgttgccggacggcggccaagtcggcgacctgttctcgggcacggcgcgcgtcggccatgcgctgaagcggcagggctacggcgtctggtccaacgaccacaacgcctatgcgcacgccctggcgaccgcctatgtccaggccgatcgcgagcgatggctggagccggccgcacggcttctggacgaactgcgagacgtgcctcccgaagccggctggttcacccgcaccttttgcgaggaggcccgcttcttccaccccgacaacggcgcccggatcgacgccattcggaaccgggtcgaggcgctggacctgcagccggagcttagggccgtcgccctggtcagcctgatggaggccgccgatcgggtcgactccaccgccggtctgcagatggcctacatgaagcgatgggccccgcgcgctctgaagccgctggagctgcgcctgcccgaccttctgccggcggcgaccacgccctgtcgggcgacgcaggccgatgcgctggagatcgcgcccgagatcgacgccgacctcgtctaccttgatccgccctacaaccagcactcctatctcgccaactaccacgtctgggagagcctggtgctgtgggacaagcccccgacgtacggcgtcgccaacaagcgggtggacgtgcgcacccgcaagagcgccttcaacagccgccccggcatcggtccggcgttgcgctcagtgatcgagcgcctgcgcgcccccaatctgatcgtgtcctttaacgacgagggctatctcggccgcgacgaagtgaccgccatgctgtccgaccgcggctatttgcaggtcatcgaaatcccacacccgcgttacgtcggcgcgcggatcggcatccataatccccggggtgaaaaggtcggcgccgtcgggcggcttcgaaacgtcgagcacctgttcgtggtcacgcaacgtcgggtggagttgtccggcgccgcctgattcgttgatttttcttaagaagcggagccgggaactctccgcgatcggcctcgttagcaaccgtatgcaaccgcccgtcgaacgccccgaccttaactcccgcacggatgacctccgtctgaggcggatggacgtggcgcgcgggcacgaggcctatgtcgcggccgaagagcggtcctgggcgccgcgcgcgaccgaaatcccccgctcgatcccgccgtccttccacgatcgcgggctcttcacccacacggccgccaacttcggccgccgcgtcgaggcggagccggcggcggtcgaggagatcgacgtcgaaccccagctgccgccccccccgcgctggatgctgatgatgggcggcgccgccatcgcggccctgatgggcgcgctgctgggcgggttcatgcacatctgagccgccgcgctcaggcctcttccagcaaggcgcggatcggcgaccagcttcggcgatgcgccgggcacggtcccatcgccttcagcgccgcctgatgcaccggcgcgttatagcccttgtggctggcgaagccgtagccgggatagacgccgtccagctcgatcatcaggcggtcacgcgccgttttggccaggatcgacgccgccgcgatcgacaggctgagcccgtcgccgcccaccaccgtgcgcacgtcgcacggcagcttgaagcggtagttgccgtcgaccagggccgcggccggctgcaccgccagcgcctcgatcgcccggcacatcgccaggcccgtcgcctgcaggatgttgagctcggcgatttcctccacggaggcgaagcccacgccccacgccagcgcccgggccttgatctcgccctccagcgtctcgcgccgcagcgccgtcagggccttggagtcgtcgacgccttcgggcaggtcatgggggttcaggatcaccgccgccgccgacaccggcccggcccagggaccgcgccccgcctcgtccaccccgcacaccggcccgcccacggcctcggccgccagggtctccagcgtcaaggtcggcaggggccgcggggtcttggctttgagaggagcgggcacgcgccgcccatcgcatgatccggcgcgggacggaagcggccccggcccttcctatttcgcgaaggtgtcctggatgttgatgatcgccggccccaagatcacgataaacagcaccggcaggaagaagaggatcatcggcacggtcagcttggccggcagggcggcggccttcttctcggcggccgacaggcgcaggtcgcggttctccttggccatcacccgcagcgccgcgcccaggggcgtgccgtagctttcggcctgggtcatggcggtcgccaccgacttgacgcccggatggttggtgcgcttgcccaggttctcataggccgtgcggcgatccggcaggtagctgagttcggccgcgagcagcgacagttcttccgccagatcgatggaggaaccgccgatctcctggctgaccttctggatcgcggcctcgatcgacatgccggcctcgacgcagatcagcatcaggtccagcgcgtccgggaacgcctgcatgatcgaggtcttgcgcttggagatgcggttggaaaggtagatgttcggcgcatagaaccccgccaccgccgccgccatcacccccgtcacgcgcgacatcaccggcaagccgaagtcgttgacgaagaacaggtacaggcccgcgatggtcagaaagacaaaggggggggcgaagcggaagaagtagaaggtcgtcagcggtcgggggccgcgaagccccgcctgcatcatcttctcggccacctgggggtcttccagaaggcgcgacaggtcgagcctgtcgacaacccgcttcttgaagccctcatccgtctggcgaaggccgccctggctggagccgaccgccgcgcgcgatcgccgcttcagctcgtcccggcgttgcgacaccgccttcatccgcttgtccaggtccgcgccgccggtcatcgaaccgagcagcgtcagcagggtgaagaacaccagcacgcctatgacgatgctcagcagcgtctgcggattggtgatcgcctggatgaggtcgttcatgctccggctcccatcagaacttgaacgcgatcatcttcttcatgacgaagacgcccatgcccatccaggtgacgccggccaacagcatggcctgcccgcgcatgtcggtgaacatcagcatcatgtaggcgggcgccgtcagcgtcacgagcagcatgacgaccggcggcagcgagccgatgatgccggccgacgccagcgcctcggacgacatcgccttgatcttctcccccatcatccgacgggcgcgcagcacggtggacaggttgtgcagcgcctcggccaggttgccgcccgtcttctgctgaatggcgatcacaatggtgaagaagcgcagttccggcgagggcatgcgctcggacatgcgctccagcgtctgctccagcgtcaggcccacagccagtccttcgaccagcttctggaactcggggccaagcggcgccgggctctcgcgcgcgatgatcttgaagcactcgtgcaccggcaggcccgaccggatgccccgcacgatcacgtccacggcgttcgggaactccagggcgaacttctttaaacgccccttggcgatgaagccgagtatccagcgtggcaggccgagggcgaacaccagcccgattccgatggcgacgaacaggttgaggcccagcaccagcgcgggaagagccatgaccaagccgacaccgccgctgatcaggtaaaaggtcctggggttcatcgacacgccggcgtgcttcagtcgcgcgtccagcgtcatgcgggccttgcgctggcggcgctcggcgtcctgcaactggtcgatgatctgcttgcggcgggcctcgggcgtattggccagcgccgcctttcgagccgccgcctccttggccttgccgccgccgaagctttcggcgcgcttcaccgccttggccgaggagtcatcgccgcccaccagcacccagcccaggctgccgatggtcacaaaggccaggatcgccgcgagtatcggaagcatgggcccttactccgccgcgtccagcgcatcggccagctcgcgctccagcccgtagtagcgcgcgcgatcccagaagcgggggcgtgcgatgccggtggagcggtgccggcccagcacgcggccgttctcgtcctcgccggtgatctcgtagacgaacaggtcctgggtcacgatcacgtcgccctccagccccaccacctcggtgatgtgggtgatgcggcgcgagccgtcgcgcaggcgcgcggcctggacgatcacgtcgaccgagcccacgatcatctcgcggatggtcttggacggcaggccgtagccgcccatggtgatcatggactccatccggctgatggcctcgcgcggcgagttggcgtgcagcgtgcccatggagccgtcgtggccggtgttcatcgcctgcaggaggtcgaaagcctcgggcccgcgcacttcgccgacgatgatgcgttcgggccgcatccgcaggcagttcttgactaggtcgcgcatggtgatctggccctggccttccaggttcggcggccgcgtctccaggcgcaccacgtgcggctgctgcagctgcagttcggccgcgtcctcgcaggtgatcacccgttcggtggggtcgatgaaagccgtcagagtgttcaagagcgtcgtcttgcccgagcccgtgccgcccgagatcaccagattgcatcgcgacgcgccgatgacgcccagcacgcgcgcgccttcggggctgatggaggcgtactccaccagattgcgcatggtcagcttgtctttcttgaacttccggatcgtcagcgtggggccgtcgatcgccagcggcggcgcgatcacgttgacgcgcgatccgtccggcaggcgggcgtcgcagatggggctgctttcgtccacgcggcggccaacctggctcacgatccgctggcagatgttcatcagctggccgttgtcacggaagcggacgttggtcagctggaccttgccgccgacttcgatgaacacccggccggcgccgttgaccatgatgtcggcgatgtcgtcgcgcgccagcagcggttccagcggcccgtagcccaggacgtcgttgacgatgtcctggaccaggttctcctgctcggccaccgacatggagacgttcttgatcgccaccagctcggcgacgatgtcgcgaatctcctcggacgccgccttctggtccagctgcgccagctgtcccaggtcgatggtgttcatcagcgcgttgaagatcgtggtcttcgtggcgtgatagtagtccgactgttcgcggacgatctcggcgacggcctgggccttcttcagctggtccaggcccttggtcggcttggggcccgccgcggccggagccgccggacgcggcgcggcctccggcgccggcttgggtctggacgccagcgcatccagccggtctgtcgccttcgcggtcgcggtggccactgaatcgtcaggacgggcgaagccctgcaccgcgcccgtgggggaagcgaagcccgcgccggccggcgccaaggtcatcacctcggccgcgccggacgcaggggccggagcgggagccggacggaggggcgcgatggtcgcgccggcctgacctgtgcgcttgccgaacaccgcgtcagcgcttcttgaacaggccggcgaacagcgacttagacgccttgtcggatgcggccttgcccggcgccggcagggcggcggcggccttggccagcttgcccttggtcgcgaccggcagctcacggcgcgacacgatctgcgccagggtctggaaggcctcggccgacttggtcttggcccccgcgtccaggatcatctggccgttgttggccgcagcgccgaaggtcttggcgtcgaacgggatcaccaggctgggcaggacgcccagggccgcgccgaagtccttggccggtatctcgggccggccgggcacgccgacctggttcagcaccaggcgcggcggggcgtcgttggggcggctcgacttgatcaggtcgatcatgttcttggcgttgcgcagggacgccagatccggcgtcgccaccaccaccacctcgtcggccgagatcagggtgcggcgcatccaaccggaccacagatgcggcaggtccagcaccacgaacggcgcgggggagcggatgcgggtggtcacctcttcgaaggcgtccggcgagatgtcccagtcggcgtccagcgtcgcgggcgcggcgaacaggctcagcttgtcggtgcagcgcaccatcatccggtccagcagcgtggcgtccagccggtcgggctgacccagcgcgtcggccacgccgttcagcggatcctggttgaagtccagccccgccgtcccgaacggcaggtcatagtcgacgatgacggtgttggcgccgatccgctccgagatcgcataggcggtgttgtgcgcgaccgcgctggcccccgccccgccgcgtgcgccgacaaaggccacggtgcggccgacaaagggctgggccgggtcgttgaacagccccccgatggcgccgatcagctgcagcggctgcaccggagacaccagatactcgctgaccccgcgccgcatcagttcgcggaacagcaggatgtcattggtcggaccgatcacgatgaccttggtgccggcgtcgcacacattggccagctggtcgacctgccacagcagggtctgcgggtcctgaaggcattcgacgatgatcagaggcggggtcggctcgtgctgataggcctccaccgcggcgggggcgccgcccacccggatctgggtggtggcgcgcgacagccggcggtcctgtcccgcgcgctcggccgccgccagcgtgtcctgccgttcggcgaagacgtgaatggcgatgcgcggaaccgacacctcgccgatcgccggcgccagcgccgactgcgccccggccatcaggtcgccgaccggattgaagctcgccgccgccggagcgacggccgtcatcggcagcggctcacgtggattgatgtcgccttccagcagcacgggctggaccggcgcgacgggcgcgacgggctgcatgcccaagggcgcgggcttgtcgccgaactccagctcgaactcgtcgtcgaaatcgtagccctgagcggcgttgtgggcggcgttgctggtgctcatgatcctattccaccgcctcggagatgcgaccttccaccaacggctccagctcggcggacgtcacctctccgatccggtaggcgtccagcaccgtggcccgacgcggcgcgtcgggggccgtcatgtcgcgcgggatcacaatgtcacgcgggttggcgatctgggccgccatgttggcggtgacggcgcagccgaagccggtgtccggctcgttgctcgcattccgggccaggtcgccgatgcgtccggcgcactggggcacatgagcgcgcagggtttcgaaaccgaccaggacgggcgcccggggatcgggcgcggcataggcggcgaccacgatgcggtccatcggcacgcccagcgccgccaccgcgtcgcgcgcggcccaggcgaaggcggccgcggcggggtcattcccgcctggcgcctcaacaaccacccgtggcgcgccgctcatggcgaaccggtgagtcaggtcgctcaaggcggcgttctggttgtgcgacacgccgtcgggacggaccgccagcgcgatccgatccacgcccggctcgacctgcagaacatagcgcgaggtcggcgtcagcggctggcccgcgcctggttcaccaggctgcgtcgcgcaggcggcgagcagggttacggctccggcgagcgacaccacacccaaggctcgactgcggttcgcatggtgcatcatggcgcgtctcattcgatcacatagcccaccggcccctgccagcccgcggccgggtcgggggcgggcggcgggctgccgtattgctggttcaactggccgaacagcagggtccgggcgtcgttggcgatccgcagcccgtccgccggagtttgcaagcgcccgggcgcggtcggcgagacgatgtaggcctcgacgatgatgaccagttccgtctggcccgaggtgtagtcgcgcgagcggaacagggcgcccagcaccggcaggtcgccggcgcccggcagcttgtcgatgttctggcgcatctcgtcgcgcaacaggccggcgatcatcagcgatccgcctgacggcagctccaccgtcgatgaggcgcgacgcacgttcagagccgggatcaccagcgccgagtcggccgaaggccgaagcgtaaaggcgccgtccgtggtcagctccgacacttcggtcgacagctgaagcgatatccgaccttccgacagcacgaccgggcggaaggcgagccgcacgccgaacggcttgaactctacggaaatgttggttcgaccatcgtcgtcggaggcgccgacagggatcgggaactcgccgccggccaggaattcggcgctctcgccgttgacggaggtgaggttgggttcggccagggtgcgcaacagccccgtgcgctcaaaggcctgcagtcggctgctcagcgagccgtccgcgccggcgttgacatagccgagggcgcctccgccgagaatgccgccgctgacgccgaaggtggcgttttgcgcaaaactgaggccgtcgccgacggtgttcagcaccgcgctgacgtccagccccagttgcttcacggccgagcgctgcacctcgaccacgcgcgccttgaccatgacctggtcggaaccggcgacgttcagcatgttcagcaccttttccggcgccgacacaaaggcgcgcgcaatggtctgcgcttgcgtcgattgggcggggctcaggaccgaaccggtcaggatgatgctgtcgttgaccgcctctgcgcgcaccatcgcgccgggcaggacgcgcgccagggtgtcctgcagggcgctggtgcctgcatcgaccctcacgcggagcgtcaggatggtgcggccagcggcgtctaggaagacggcgtccgtctcgcccggctgcagcccgatcaccgtgatgcgacgcggcgagtgcagcatggcctcggccacctgcgggttggacacgatcacgtcgcgggcgtccgccggcagatcgacggcgaaggaggtgccgcgcggcaggttgatcatctgcggcgcggtcgatcccatggccacggccgcgcgggtctgcgccagcgtcatcgagggcgaagcagccgacagcagcgccagcgcgcagactgcggcggatcggatcatgcgaaggctcattgcaccgtcaccacttgcggttcgccgccgcgatagaccttgaccgcacgcggcgccgcagccggggcggcgatgcgtccggtccggccggatggcccggcgttgtcggcataggagcgcagcaccagcgacaggtcgccttccgccttggccagcgccagcgcctcggcgtcctgcggcccgacctccagcgtcgccgtcgcgccgaccacggcctgggcgtcgtcgccggcgcgggtctgctggtcgatggccagaaccttgaggttgcgcatcacggttgtgacgctgaacttcggccccggcgcattgtcgccgccgccttcgttttctcgcgacagcaccacgtccacccggtcgcccggcaggataaagccgccggcggcggtctccaccgtcacgccgatggccatggcgcgcatgccgggctccagataggcggccaggtagccgctgtcgccggcgcgcacgatcttgcggccgacaatcggttcgcctgcgagaatggtctcgcgcaccaccgagccgaggtagtctgacttcaggcccttgccggcggcttcgttggcggcgcgagccacggtttccaccgcgccctccaccttcttttcaggggtggcgtccttgggggcgctgggcgccgaggcgtcgatgatgaaggtgggatcgacctcgtcggcgggccagtccttccaggtcatgtcgtcgtcggtcaggcgcttgcccggctggatgtccttggcggcgaccaggatgcgggtcatggcgcgctgctcgaccggggcggcggcggccggcgccgccggctcgttcgacgacgatcccatggcgcgaaccaccagggccagcccgatggcggacacggcggcgacgcagatgacggcgatgcgggcaggcttcatccagacggtctccggtcgggcgcgggatgcgaaacgcgattcccgggcgccccctcgttaacgatcatggagcgggcgggttaacgccgccctaaacgctgtttggcgatcacaacccggccgagaagcgcgccaccatgtcgctggcgggaaaggccaacagggcgccggcggcgatggccacgccgtaagggatgtcgcctttgggctgcatcaggtgcgtgacccagccgggcccggcgaccaaaagcggcgccaggtgcttgcgcgcggtcagcaacaacagacagaaggcgccgccgcagacgcctgtgtagagcagaaagacgcccgatccggtcaggcccaaccacaagcaggatgcggcgatcagcttggcgtctccgccgccgatccagttcagcgcgaacatgcccgccccgatgaacagggccagcagccccacgcccacgtgagccgcgaccgttggcaggtccaggcccaccagaaaagcgacgggaaagaaggtcacgatcagcagcactgagatccagttcgggatcttcatggtgagcaggtcatgcagaccggcgacgatagcaagggccgggaggaggccgagcagcggaagggtcagggtgtccatacgtctatcctgctgacggaactttaagttcgcgtttccaacaagtctccgcattagccccctgaggtcacatccgggggttcggccatgttggagccgatgtgctcgagagcctgctttagctggggaccgaaggcaccgagcacagcaatgacgacaaccgccatgagtgcgccgatcaggccgtactcgctagccgtcgctcctgcctggttgtggccaaggcggtgtgcaaattctctcatcattcggtagattcctgcctcggttacaaacggatgaaggccggcggcatcgccaccggcctccaacatctcactgcgcgacctactgcatcaggtgccagcagtgatatcagtgtccttcgcgtcttcgagcgtggctccgaggtctgcgaacgccgtcttcaacttcggaccgaaaacagttaggcaggcgatgacagcaacggccatcagggcggcgatcaggccgtattcgatggcggtggcgccggactcgtccttgacgaaacgcgaaacgaagttggtcatgtgtgtgtccttctagacgtggttagcaggcaactggcggggggagccggtagcccgcttgacccccaaaacgcagggtgaccatcgcagcccgaagttaagggcgagtcgccggatgtggttaccgcctgatttacctcgatttttctccaagatcggtttcagactttcttgagatttcaggcgcacctttcgcgcgtcgcctcgtgcgcgccgcatctatcaggcgctcgcgcctctcaatcgaaggtcgccatgcctcctcgctcccttaccgctgccggcctaatcgccctggccttggccgcggcatctccggtcctggcgcagtcgcggccgctcacggtcgagatcgaccgcgcacagcgggtgcagctgaacggcgccgccaccgcggtggtggtcggcaatccgcagatcgccgatgtgacggtggtggacgccaacaccctgttcgtcactggcaaggcttacgggaccaccgaggtcgtggcggtggacgcgatcggccgcaccctgtttcagggcgagatcagcgtcacctccggctcctcgggcgcggtgcgcgtctggcgcggcggccaggcgaccgagatggcctgcgcccagacgtgcgcgcccagcattcgcgcctcgtccaacggcccggccgccaccgccgcgccggcgccctgatccctgcagcctgaaccatgatgcgccgaccttccctgcgccgcctgcgtccgccccgcttcgccgggcggctggcgcgcgaccgaaggggttcggccgccgtcgaattcgccatcgtcagcctgccctttttcgccatgatgttcatggtgctggaaatcggcttggcctttctgatcgattccaccctggagaccgccgtcagcgagagcggacgcctgatccgcaccggtcaggccgaggcccaggggttcgaagtcaaccggttcaagcaggaggtgtgcgagcgcatgagcgtgttcgccgctgactgcgccagtcgcgccaccatcgacgtgcaaacgatcgccagcttcgccgcgccgcctgcagatcccatcgttgatggagaactgcaggcgcagaactgctacaacggcggcacggccggcgacctggttctggtgcgcgtctggtatcggcagccgatgatcgctcctttcctgcgcgacggcgtgatgcggctgaacggcacaaccgtcctgctgaagggcgccaccgtgttccgcaacgaaccgtggaccccctccggcgtgccccccgtgaagacctgcgcatgacggcgccgtccctgtttcggcgcttgggcgcggaccgccgcggtgtttcggcggtggagttcgcgctgatcgcgcctgttcttcttctgctctacttcggcctgaccgagttctgccaggcgcagatggctcagaaacgggtgaaccacgtcgccgccaccattggcgacctgatcgcccagaacggtcagctcacccgcagcgacgtcgacagctttcttgacgcaggtgacctgatcatgtcgccctacgcccccgaggacctgcagttgcgcgtcagcagcgtccggcgcaacggctccaagtacacgctggtgtggagcaggggttcgcgctggggcggctcgctcaccgcgacgccggcgatcggcgacgacatcgtggcggacggcaagacggtgatcgtggccgaagccaagtacagctacgactcgccgacccgatatgtcatgggcgacgggttcgagttcacccacaccgcctatcttcaccctcgcgacggcgacgtcgtgctgaaggactgatctccggccaaggcctcggccatggccctgatcttgacctcggtttcggcgcgttcgcaggcgggcacgctgtcggccacgatcccggctcccgccagcgtgcgaaagcgccagcccgtctcgtcccgctcgaagctggccgtgcggatcagcaccgaggccgtcatccgcccctcgtccagcatgaacagcgacccgcaccagggccctcgcggcggctcgtgggcggcgatcaccttcatcgcctgatgcttgggcgcgccggtgatcgagcccggcggaaaggtcgcctccagcgcgtcggcggcatgaagccccgccttcaaccgcgcgctcacggtcgacaccagatgatgcacggtggggtggctctcgatctcgcagagcgcctcgacccgaaccgatccgggctcggccgcgcgcgccagatcgttgcgcatcaggtccacgatcatcaggttctcggcccggtccttcgcgcttgacgccagttcggccgtgagcgcccggtcctctacgacattcccgccgcgaggccgcgtccccttgatcggccgcgcctccagccgagcgccatccaacgacaggaacagttcgggcgagttggacaccaccgcccgctccccgaccctccagaaggcgccataggccgaggctcgctccgcctgcagccgcaggaacacgtcgaacggttcggccccgcagcgcaagcgaccgccccacgcccgcgcgatgttggcctgaaacagttcgcccgccccgatgcgagccaccacgtcggccacggccgcttcgtagtccgcgcccgaggtttcctccaccagggcgtcggccggcggtccgggcggcgacggcgggacggcccgtcccaaccagcctgacgcccgatccgccgccctccccgcggcgatcgcatcgacgcccctgccgatcacctccaccgttcgggcatggtgatcgaagcgcaggatggccggatagcgcgccagcatcaggtccggccacaccgcctcgcgcgagcccgtcgccggtcgcgccccggcgtcataggccgcgaggcctatgacgccgacgctgaggaccggatcacgcagggcttcgaacaaggcctttcccttgccttccaaggtcaggatcaggtccggatcggccgccacgagggaccagcgcccccccgccgcagcgccattggcgaccagcgccgcgagtcccggcgcgtttcggagcccggtcgccacccagaccggatccgtccagggcgccacgcgacgcacacaggcggtcaggggctgggcgtctgcggagtgactcatcaaccgcgtcttagccggacggcgtcacccccgccatggcgtcgagataggcgacaaaggcgtcgcgtcccgcctccgtcatgaccgcctcggtcagcggcttgcgtccctggaagctcttggtcaccgtgacgaagccggcgtcctccagcttccgcaggtgcaccgacaggtttccgtccgtggtctgcagcctggccttcagggtgttgaagtccgcccgctccgcacccgccagataggccatgatccccaaccggatgcggccatgaatgacttcgtcgatacgattgatgtcgaagtcatccgccatcagacgatcctcgacggttcctgacgcatcaggagcaggccggggaccagggcgacggccgccagcaccacggtgaacaccagatagatcgcgggatcgtcagcaaaccagcccaccgccaccgcgcccgcataggacagcagggccgtcagggacatccaccgtgtcttggtcatggcggccgccaccatccacgccgagccgtaggcgaccagaaccaccgtgggcatgaccgacatccacgaccagttgtccgtcctgaccgacattgcgaccagacctagccaggtgacgaagatgccgtagcccacgccctcccaggcggctccgaccgcccggttgcccgtggcgttatagcccggtcggcccttcatgcgtccgatcagcaccgtcagggccaccgcgaacaccacacccgcaccaatccataggccaagctgcgcccagggactgacgtccagcacgtcggcctgaatcgcccactgtccgaggttcgccgtcccaaagaccaagcccgccgtaaccagcatgggcccggccagcagcggcgcgtgccgcccctcatgggccagcgcccgcatataagcgatgtcgtcctggatggtctgtgtctcgcgcgtcatgacgccctccccttgttgatgacaagaggatgcgcaattcgctttgtgatgtaaagttcttttcagccctaccggaacggcggctcatcaaaggcgcgcagcttgcgcgaatgcagccgctgcccctcagcccgcatcaggtcgatggcctggatgccgatctgcaggtgttcggagatggagccttcgtagaagcggttcgcctgacccggcagcttgatctcgccgtgcagcggcttgtccgacacgcacagcagggtcccgtagggcacgcggaagcgatagccctgagcggcgatggtcgccgactccatatcgatggcgacggcgcggctctggttgaagcgcagcgccgacttggaatatcgcagctcccagttccggtcgtcggtggtcaccaccgtgccggtgcgcaggcggcgcttgacctcctcgcccggcatgccgctgacggacttggtggcgtcgtagagggcgcgctgcacctcggcgatggaggggatcggaatgtccggcggcagcaccgcatccagcacatgatcgtcgcgcagataggcgtgcgccagcacatagtcgccgatcgactggctggcgcgcaggcccccgcagtggccgatcatcagccagacatgcggacggatcaccgccaggtggtcggtgatggtcttggcgttggacggccccacgccgatgttcaccaccgtgatgccctttccgcccggcgcggtcaggtgataggctggcatctggtgcttcttccaggcgttctcgctcagcgccgcatccgggtcggccgtctcgcgcgtcaccaccacgccgcccgcgcacgacagcttgtcatagggactgtcgggcgccttcagctgctcgcaggcccagcgcacgaactcgtcgatgtagcggttgtagttggtgaacagcacataggactgcatgtcctccaccggcgttccggtgtagtgccgcagccgcgccagcgagaagtcggtcctcaacccgtcgaaatgcgacaagggaaagtcgcccgacggatcaaacaggccgtcggcgatctcgtcgccgatgtgcgccaggtccgtggtcggaaaccaccgcgccagccccgctgtcatcgaccggtccagcgccacgtccagcccgtcggtcacataggggaagggaatttcctggcgggacagcccgacgtcgaaggtcgcgccatactcccgctccagcaggctcagctgctcggtgagataggcgcggaacagttccggccgcgtgatggtggtgctgtaggttccgcgatgggccagccgggcgtaggcgcgaggctccagcgcctgggtgcggtcgccgtcccacagcactcgcagctcgggataggcgaacagaccgtcggcgcgctcggccgcatcggggcgagcgccggtctccacgaaagcgcgcacggcgcctcgcagattgcctacggactggttgtagagggtttcgaggcggtccagcgccgcctcagccgtcatcggctgtgtgttcagttctgtcatgacctcctctagccgaggatcgtgactttggcgagacgccggcgttccgcatgacgcatcgtcacagtccggcggttgcgatcatccgccgcatggcgcatcgggcgcccatgaccgcttccgccgccctccccgcccggcgcgagcccggcttcgtcgagttcgtttgtcttatcgccctgatgatggcgctgaacgcgctcgccatcgactccatgctgccggccctgccgcacatcggagaggacctgggcatcgccaacgagaacacccggcagtgggtggtgaccgcctatcttctcggcttcggcggggcacagctgatctacggtccgctggccgaccggttcgggcgaaagcgcgtgctgctgacgggggtgggcatctatgtgctgttcagcctgctggcgacgctggcccccagcttcgaaaccctgatcgccgcccgcgtcggccagggcctaggcagcgcctgcacccgcgtgctggccgtctccatcgtgcgcgaccgctatgaaggccgcaccatggcgcgggtcatgtcgttcagcttcctggtgtttttgggcgtgccgatcctggcgccgtcgataggtcagctgatcatgctggtcggcccctggcgctggattttcgcagggctcggcctggtcggggtctgcctgatcgtctgggccgcgctgcgcctgcccgagacgctgaagcccgaggatcgcctgccgatccaggcgcgccgccttgtgtccgcctaccgggtcgccctgaccgaccgcacggccgtcggctacaccctggccatgaccgccattaccggcgccctgttcggcttcatcaactcctcccagcagatcttcgccgacgtcttcgacgcagaagcgcagttccccgccgtgttcgccttgatcgccgggggcatcgcagtggcctctctggtcaacgcgcgctgggtggtgaaactgggatcgcgccgcatctcccacaccgcccttctgggcttcaccaccatcgccgccgtccacgcggccgtggcgctgagcgggcatgaatcgatctggacctttgcggtgctgcagaccctgaccatgttctgcttcggcctgatcgccggcaacttcggctccatggcgatggagaccatgggcaagatcgccggcacggcctcgtcggtccagggcttcatctccaccatcggcggctcgctgctgggctttgcggtaggtcagcagttcaacggcaccgtcgccccgatgaccctaggcttcaccggctttggtctggtcgcactgacctgcgtcctgttcgccgagcgcggcaagctgttccgcgcccagcacgcggcaacgccggccaaggcttgatctttgcggtcatccggggcgttgtccgtgctcgaaacagcaggatgacctctacgatgatccgcactcgcgccggcctggtctcggctctcgctctcgccgccgccctgggcctctccgcctgctccaccaccggagggtccgacatgccgcccctgccgccttccgccaatgcgccggtcgactacgcgcgcgacgtccactcctacgctcggcccgagatcgcgcgcgttcgccacgtcgcgctggaccttcaggccgactttgcaacgaagactctgtcgggcacggcggcgctggacatccagggcgttcccggcgccaacgagatcatcctcgacatccgcgacttggacatccgttcggtgtccgacgcctccggccagccgttgcagttcgagacgggcgccaacgatccggtgctgggccaggcgctgaccatccgcatgcccgccctctcggtcggagagacgcggcgcatcgtgatcgactattcgacgcgaccgaacgccgccgccctgcagtggctcagcccgcagcagaccgcgggcggccagaagccctacctcttcagccagggccaggcgatcctgacccgcacctgggtgccgacgcaggacagccccggcattcgccagacctatgacgcccgcatcaccgcgcccgccgacctcacggtggtgatgagcgccgaaatgctgaccaagggcggagaggcggcggcggacgggcggaaggcctggcgcttccgcatgaccaatccgatcccgccttacctgatcgccttggggatcggcgatttggccttcgcgccgctggacgagcgcaccggcgtctggaccgagcccggccgcctgcccgccagcgcccatgagctggagcccaccgccgccatggtcgatgcggccgagaagctctatggcccctaccgctggggccgctacgacctgttggtcctgccgccctccttcccgttcggcgggatggagaacccgcgcctgaccttcgccaccccgaccatcatcgccggcgaccgctcgctggtcagcctggtcgcgcatgagctggcgcacagctggtccggcaatctggtgaccaacgccacctgggcggacttctggctgaacgagggcttcaccgtctatttcgagaaccgcatcatggaggcggtttacggccgtgaccgtgcaatgcaggagcaggtgctgggctacgacagcctgcaggagacgctggccaccctgcccgccgccgacacccggctgaagatcgagctgcagggacgtgatcctgacgacggcctgaccgacgtcgcctacgaaaagggcgccctgttcctgcgcaccatcgagcgcgtggtgggccgcgagcgcttcgacgcctggctgaccggctatttcgaccgcaacgccttccggccgatgaccaccgagcagttcctggccgacatccgcgagcatctgacgcgcaacgatccggtgctggagcagcagctgcagatgaacgcctggatctatcaacccggcctgccctccaacgctgtcgcccccacatcgccggcgttcgcgccggtggatgcggcggccgtggccttcttccgcgacaagggaccggcctcggccatcccctggagcggctggaacacccagcagcgtcagcgcttcctcggctggcggccggagggcctgcgcgccaacgccgactggctgacggccgcgcagctggcggacctgcagtccacgctgaacctgaccaatgaaggcaacgctgagctgaccttcgcctggctgcagatcgccatggcgcaccgctaccagcccgccgtgccgacggtggagcgcttcctgaccgaacagggtcggcgcaagttcgtcctgccgctgttcaccaccctgtggggcgaaggcgactggggccggacgctggcgcggcgcatctacgcccaggcgcggccgctctatcacccggtcaccaccggctcggtggatcaactggtcgggcggtcctagggcttcagggatgcccgagcttccggaggtcgagacggtccggcgcgggcttgagccggtgctggcgggcgcgcggctttcgcgcgtccgcatcaaccgtcccgacctgcgctttccctttccagaccgcttcgccgagcggctggaaggggcggtggtccagcgcatcgagcgtcgcgccaaatacctgctcctgccgctgtccacgggcgagacctggatcgcgcacctcggcatgaccggccgcttcaccctggatgggatgcagctgggcgagttcgaggagcccgcgcccatcgccggcaagcacgagcatttcagcgcctgcgcgatccgcgacggctcggccaccggcatcggctttgcggacgcgcgtcggttcggcttcatggggctggcgccgaccgatcaggtcgaggcgcatccgtggttcgccgctctcggccccgagccgctgggcaacggcttttcggccgcgcacctgcacgccgccttcgccggtcgcaagcagtcgatcaaggtctcgctgctggaccagaggatcgtggcgggcctgggcaacatctatgtctgcgaggccctttatcgcgcccgcatctcgcccacggtcgccgccggcaaggtttcgcgcccgcgcctggagcggttggcgatcgaggtccgcaacgtcctggatgacgccatcgcggccggcggctccacccttcgcgacttcgccaacgccgagggcggtcagggctattttcagcaccgcttcgacgtctacggccgcgagggcgagccctgccggggcgaaggctgttcgggcgtggtcgcccgcatcgtccagggcggccgctccaccttcttctgcccgtcctgccagaagcgctgagacgccctgtcgcggcccggcgtcaaccaaaggccgcgatccgtcgttaggggcggatcatgcgccgcatcctccttcttcttctcgccgtcttcgccgtgggctctcccgccgccgcgcaaggtgccttccgttccgaccgcatcatcgtggagacgcgggggcgcggcccggacgtgatcctgatcccaggccttggctccaccgcgacggcctgggggccggcggtgaaccggttggacgaccagtacaggctgcacctcatcaccgtgcgcggctttggcgacaccgccatcgcgggcaacgccgagggcggcattgaaggaccggtcgccaacgagatccgtcgctacatggccgaacagcggctgaaccgccccgccctgatcggccactccatgggcggccagatcgcgctgcgcgtcgccgctgacgcgcgcgagggcgtcagccgggtcatggtggtcgattccgcgcccttcttcccggccctggtggacgcccgcgccacctccgcccagatcgagccgatcgcccaggtcatctatcaggccctgatgctgttcggagactccgccctgtccagccagatcggcggcttcggcggtgatctcggcgcggccggcgacatggtgttcggcggcctgggtcttccgggcggcgaccgccgcatcctggcgcagggcctctatgaggtgatgaccgtcgatctgcggcttcgcctgcgcgagatcaccgccccggtcaccgtggcctacggctggagccgcgacgagaacaatccgcgcagcaagctggaggccctgttccgttccggcttcgacaacctgcgcacgcccgcccggttcgagcccattgaaggcgccgagcaccaggtcatgagcgaccagccgcagcgcttcctcgccgccgtgcagcgcttcctcgcgtcctaaaggaagaagggtggcggcgccgcgagagccgtaaagaacagtttgaatcctctcgagcctggataaccaggtgggcgccatatacccaggccctcgagcccggacagggacagctcccttcgagtgaattaaggccgcgaggatatgtcgtcttcctcgagcaccgcagcatgacccgccgtccaccaagataggcgtgacggcgacgcccctcaagcggtacggtcagccaaatccagggagatcgcgatgagcctgctgaacgccctcatgggcaacgccaacaccctcgaagccgccgcggccaccgccgaactcacgcacatcctgatccccggcgagcgggtggagcacgcctacaagctggtgcgcgacctgatcgtcttcaccgacaagcgcctgctgctggtcgacaagcagggcgtgacgggcaggaaaaccgagtaccactccgttccctacgcgaggatcagccacttcagcgtcgaaaccgccggcacgctggacatggattcagagctgaaggtggcggtgtcgggcggcgcggtcttcacccgcaccttcggccgcggcgtggacatcggcgacgtgcagaaggttctggccagctacgtcctggcctgattggtcagtccggttcgcgctcgcccacctccgtcggccgcacgatccgcagccagccttccgcaaggttcagttcgggcgcggcctccttggtgaagggcaggtaccaggtcggcccgccctcgaccggggcgatctccagcatgtcgtcggcgccgaagttctgcaccgacttgaccgtgccgattgccttgccctcggcgtcgcgcgcctcgatccccagcaggtccgccaggtagaactcgtcttcctcgggctccgggaaacggtcgcgcggcacgtgcagcttcaggccgcgcagcgcgtcggcctcttccttggtggtgatttccttggcgcgcccgaccacgccgttcttgtccggccgcgcctgcgtcagcgtcagcccgaccgatccgtccgcccgcagcagcggcccatagtcggtcagcgccagcggatcggcggtgaacgccgtcacccgcacctcgcccttgaccccgaaccccccggccacctgcccgaccaggatcagtctgctgttctcgcgcatgaagcctccggcgtcctccccgcctacagggtaggaacaaaaaaggcgacgcccgatggacgccgccctgattgaagcaagccttggaaagcttaggcctgttcttcggccgtctcggcggccggagcctcttcagcagccggagcctcttcggcggccggggcgtttgcggcggcttcggcggcggcggcggcttcagccttggcggcggcttcggcctcggcgcggtcggcttcgcgctgggcgcgctcggcggcgcgttcctgggcctttttgccaggctggcccttgttcgggttgttgctctgcgtccacgtcaccttggccgacaaggtctcgtcctgcgacaggaagcgggccacgcggtcggtcggctgggcgcccttgccgagccattcggcgatgcgctcggacttcagggtgacgcgcggctgggcgccgtccttgggcagcatcgggttgtaggcgccgaccttctcgatgaacttgccgtcgcgcggcgagtgcgagtcggcgatgacgatgtggtagtaggggcgcttcttggcgccgccgcgggccagacggatcttcagcatttcggtctctttctaatcgaagtcagttctttttcgggaagcccggcaggcccggaaggcctcccggaagttgtccgcctcccaggccggcgaagcggtcctggatggctttcagttcgtcggccgagggttcgggcatcttgccgccgcccatggccttgaggcggttcaggtcgggcccgcccatgccgccgccgccgagcccgcccagcatggcggccatctgctgcatcttcttggggccgccgcgcgccatcgacttgaccatgtcggccatctggcggtgctgcttcagcacgcggttgacgtcctgcacgtccacgccggcgcccgccgcgatccgcttcttgcgcgacgcgttcaacaggtcgggcttcttgcgctcagccttggtcatcgaggagatgatggcttcctggcgcaggatcatgcggtcgtcgatgccgctctcggccatctggcccttcatcttggccacgccgggcagcatgcccatgatgccctgcagaccgcccatgcgcttcatctgctgcagctgaccggccagatcgtccaggtcgaactggcccttggccagcttcctggccatcttctcggccttggcctgatccaggtcctgggcggccttttcgaccagggccacgatgtcgccctggcccagaatgcggccggcgacgcggcgggcgtcgaacacgtccagcgcatcgaccttttcgccggcgcccagatatttgatcggcaggccggtgacggcccgcatcgacagcatggccccgccgcgcccgtcgccgtcggcgcgggtcaggaccaggccggtcagcggaaggcgctcgtggaaggccttggcggtgcgcaccgcgtcctggccggtcaggctgtccgcgaccagcagggtctcgaccggcttggcgatctcggcgacctcggccacctcgttcatcagcccttcgtccagggtgatgcggccggcggtgtccaggatcaggacgtcgaagccctgcagcctggccgactgcagcgcccgacgcgtgatctgcaccgcgctttcgccctgcacgatcggcagggtggcgacctcgatctgcttgccgagcgtagccagctgctccatcgccgccgggcgacgggtgtccagcgaggccatcatgaccttcttgcggtcgaactggctcaggcggcgcgccagcttggccgaggtggttgtcttgcccgagccctgcaggccggccatcagcaccacggcgggcgggttggcgttggggttcagcggaaccggctcttcgccgcccagcatctcgatcaggccgtcatagacgatcttgaccacctggtcggccggcttgaccgagcggatgacctcctcgcccgtggcgcgctcggtggcgaaggcgatgaattccttgacgaccggcagggcgacgtccgcctcgagcagggccgtgcgcacctcgcgcatcgcctcggccacgtccttttcggacagggcgccccgcccggtgatccggtcgaagacgcctgtcagccgctcgttcagagcctcgaacattcactacctcgtttggcgggtgagaacggctccatacgacaacggcccctgtggacgatcacgtcgacagggggttctcgccatcctcgtccatccaagatggggtcgtgatggtggagacgcgaggttcacttgcgccggaagcggcggcttatggcggaagagtccgcgaattgcaacacggcggcctcaccccagcgcgcccggaacggatcacatccccttggacggatcgtcgctcggggtgttcgggtccagccggcggctggccttgcggttgcggaacttggaaaaggccagcgccagtcccagcaggatcgggccgccgatcacgacaaaggcccagggtgcggcttccgccatcgcgtctctccttacatgatgtcactggaacaacgacgggatgcggggtttgatccgaagccctcctccccgccgccgcgagacctgatcatgagccctgccgccgacgacctgctgcgcgaagaggtccgcctgctgggcggcctgttgggcgaggtgatccgcgacgagggcggcgacgaactgttcgagcgggtggaggcggtgcgtcaggcctccgtcgcctaccatcgcgatccgaactcgcacccggcagggcggctgcagaagctgctgaccgccatgagcgcggatcaggcggccggcctggcgcacggcttcgccctgttctcgctgctggccaacatcgccgaggaccgggcgaccaggcgccgcgccgaggggcaggcccaggccggggcgcgtccggacacgccggaagggatgctggctcgcctcgccgaacagggggtggattgctccgccgtccgcgctctcttgcagggcgccctggtctcgcccgtcctgaccgcccatccgtccgaggtgcgccgcaagagcgtgatcgaccgcatcgccgccatcagcggcattctcgacgcctgcgatcaagccggcctcgcctgcgcgccggatcagctgaccgcccgcctgcgccgccagatcaccatcctgtgggccacccgtctggtccgcacccaagggctggtggtgcaggacgagatcgacacggtggtctccttcctcgaccgcatctttctgcatgtcgcgccgcagcagctgggcgcctggcgccggctgctcgacgctcccgacctccagcccttcatgcgcgtcggcacctgggtcggcggcgaccgcgacggcaatccgaatgtcgacggcgccgtgctgagcgccgccttccgcagccagagccgggcagtgctgggcttctacatggacgaggtccacgccctgggttccgaactcagcctcgccgccgaactgaccgaggtgacgcccgagcttcaggccttggcggaccgggcgcgcgatccctcgccccatcgctcggacgagccgtaccgccgcgccctgaccggaatctacgcccgtctggcggcgacgcacgaagccctggccggcgccccgcccttgcgccgcgcggcggtggaggccgagcgctatcccggcccggacgccttcgaggccgacctgcgcgtgctgcacgacagtctggccgcccgtcacggggcggtgttcgagggcgaccggctgaccgacctgctcaccgcggtgcagatcttcggcttccacatggcgaccctggacctgcgccagaacgccgacgtgcacgaacgcgtggtggccgacctgctgcgtgtcgccggcgtctgcccggactatctcgcccttgatgaagagggtcgcatgcaggtgctggcgcgagagctgacctcgacccgccccctgttcagcccctacgccgaatacgccgaggagacgctgaaggaacgcgccatcctgcaggcggcggcgcaggccctgtccgacttcggcccgcaggcgatccgcacccacatcgtctccaagaccgacgccgcctccgacctcctggaggtctatctgctgttgaaggaggtcggcctctaccggcccgaagaccccgccgcctgcccgatccaggcagcgcccctgttcgagaccatcgaggacctgcgcgccgcacggcccacgctggagcgcctgctgcgcgaaccctccgccatggccgtcgcccgcgcgcgcggcgtgcaggaggtgatgatcggctattccgactcgaacaaggacggctcctacctgacctcgggctgggagctgcacgaggcgtcgcgcgccctggtcgacgtcaccaaggcggcggggctgaagcttcagctgttccacggccggggcggcacggtcggccgcggcggcggctcggccttcgccggcgtgctggctcagccggagggtacggtgcagggccgcatccgcaccaccgaacagggcgaggtcatcgccaacaagtacggcgagcccgagatcgcgctgcgaaacctcgacgccctgacctgcggcgcggtgctggcgtcgcttggcaagggccgcgaccaggccttcaccgccgagcacggccagctcctgtccgagctgtcgcaggcctcgatgaacgcctatcgccggctggtctatgagacggacggcttcaacgactactaccgcgccgccaccccgatcgccgagatcgccgacctcaagatcggctcgcgcccgtcctcgcgcaccgcgtcgcccaagatcgaggacctgcgcgccattccgtgggtgttcagctggtcgcagtcgcgggtcatgctgcccggctggttcggcttcggctcggcggtcgacgggcgcgacatggccgagctgaaggccatggccgaggcctggcccttcttccgcaccttggtccagaacatggagatggtgatggccaaggccgacatgaccatcgcccgccgctacgccacgctggtgcccgatccgtcactggccgcccgcatctacggcgagatccgcagcgaatgggaccgcacgcacgccgccgtcctcgccatcaccggccacgacaagctgctgggcggccagcccgagctggatcggctgatccggctgcgcatgccctatgtggagccgctgaaccacgtccagatcgagctgatccgcaggcggcgcaacggcgacgacgatccgcgcgtgcgtgaaggcatcctgctggcgatcaacggggtggctgcgggacttcgcaacagcggctgagccgctctcgcatcttcatacgcaccgtcatcctcgggcttgacccgaggatcggacgcggagcggtctgtgcgtcgccttcagcgcaatgctgcggaacacccggccctcgggtcgagcccgagggtgacgttcagctatcgggtgcgacctacagccacttcgaccgcttgaagctgagatacagccccaggcacaccgccgcgatcgcgcccagggtgatgaagtagccgtaacgccagtgcagctcgggcatgttgtcgaagttcatgccgtagatgccggcgatggccgtgggcgcggcgaggatggcggcccaggcggccagcttgcgggtgatcaccccctgccgctgctgctccagcaggttggccacctccagcaccgagcccagcgcctcgcccagcccctcggcccggtggttcacccgccgcgcatggtcggccagatcgcggaaatagggacgcacctccgggtcgatgcacggcaggtccagcgtctccagcttcgatcccacatcttccatgggaccaaggatgcgccggaacttcagcaactgacgccgcaggcggaacagacgcttgatctggagccgcgaaaggaaagcatccagcgcctcgcgctccatctccagcgcgcgatcctcggccttgtccatgatcggcccgtatccgtcgaccacgaagtccaggatggcgtggagcacgaagtccggcccgtgcctcaattggcgcggcgaggcttccagctgtcgccgcagcgccgcgtgcgacttggccgaaccgtgccgcacggtgatgatgtggttggcccctacaaagacgtgggtctcgccgtaggtgatgcggtcgtccttgagctcggcggtgcgggcgactacgaacagctcgtcctcataggcctcgaccttgggcatctggtgcgcggacagggcgtcctccaccgccagcggatgcaggcggaaccgctccaccagggcgcccatctccgcctcgtccggctcgtacagcccgacccacacgaactcgcccggctgaagctgcagcccctcgcccgtcaacggcgcctcgcgcacccgcgcgccgtctcggtagacgtaggaagcgacgacggtcatgcgcgatctccctcttctctcctccccgtcgcgcagcgatggggaggtggcgcggcgcgtgagcgccgtgacggaggggttccgacgccggcgacatcacccctccgtctcgccggcttcgccgtcgatccacctccccattcgccaagcgaacagggaggacaaagcactcctagccctgcctcaagcaggccgctcagatggcctcaagtagcccgaagggcggtaggcccccttatgaagtcgggaagccccgcaccttgagcagcgccgccacgtccgggtcgcgcccgcggaaggcgcgataggcctcgccccggtcggtggtgttgcccggcgccaggatgatcgccttgtagcgcgccgcgatgtccggattgaacacgtcgcccgactgcacgaagtagtcccaggtgtcggcgtccatcacctccgaccacaggtacgagtagtagccggccgaataggcgtcggaggtgaacaggtgattgaactgcggcaggcggtgccgcatcacgatctccttgggcatgccgatgcgggccagcgacgccttttcgaacgcgtcgatgtcggtcggcggcgtgctttgcgtgtgcaggtccatgtccacgatggccgaggacaggtagctgaccgtcgcatagccctggttgaaggtggcggcggcctcgatcttgtcgaccagcgcctgcggcatcgactggccggtctccacgtttttcagatagccgtccaggatcgggcgcgacagcacccagtgctcgtgcacctgggacggatattcgacgaagtcgcgcggcgtgccgcccagcgccggatagacgacgttggacgaataggcgtgcagcgtgtggccgaactcgtggaaaagggtctcggcgtcgtccagcgagatcaggatcggctcgccgtccggcgccttgacgaagttgttgttgttggaccccagcgtgttctccggcccgtcataggtcgagtgcgaccggtaggtcgtcatccacgcgcccgagcgcttgcccggacgggcgtagtcgtcggtgtagtacaggccgatcggccggcccgcgtccttgacctcgtacaccgtcacgtccggatggaagaccggcaccgagccttgcggcagcttctcgaaggtgaagccgtacaggcgctcggccatgtagaaggagccggcgcgcacattgttcagctcgaagtacgggcgcagctcgttctgatccaggtcgtacttcgccttgcggaccttttcggcgtaatagaggtagtcccacggctcgatctcatggccggcgacgccgcgcatgtcggcgacctcctccgccacccgcaccttggccggcgcccacacccgctgcatcaggtcgctggccgcggccggcgtcttggccatggtgtcctgcatgcgccattccgcgtggttgcggaagcccagcagcttggcgcgctgatcgcgcagcttcacgatctcggcgatggtcgagttggtgtcgtttgcgtcgccgttgtcgccgcggttgacgaacttgttccacacctgctggcgcagggcccggtcgtcggcgaaggtcaagaacggatccacgctggagcgggtgttcaggatcgcccagccctgcaggttgcggctccgcgccgccgccgccgccgccgtcttgttggaggccggcaggccgcgcacgcccgcctcattggggatcagggtccagctgttctcgtcggccaccaccttctggccgaagcgggtgaaggcgttggacagcgccgtgttgatgcggccgagttccgccttgccggcggcgtccagcgccgcgccgttgcgcacataggcgtcgcgcgcgcgggtggcgatgcgcgtctgctgcgggttcagccccgcggcctgggcgccgtcggccaccgccttgatgcgggcgaacagggcctcgttgaaggtgatctcgtccgacgccgccgacagcaggggcgaaacctcgctgtccagcgcctcccactcgtcgccgccgatgttggaggtcatgacgccgaacacgctcatcacccggtccagcggctccccggccatctgcatggccaccgaggtgttggcgaaagtgggcgcatccggattgttggcgatcgccgcgatctcggcgcgctgcagctcgatcccttccaggatggcttcgcgcaccttggccggcgtcgcccggtcgaacggcggggtgccgccatgggcgccggtccattcctgcagcagctcggcgcgcggcgtctggcgcggcagcacggcgcgcgcgatggcggcttcctcggaaagcgtcgcggccgacggcgccgtcgcgttcgcctgacctgcgcccatgccgttcgcgctggcgcagccgctcagcaccagaaagcccgcaccgccgagaagaagctgtcgtctttgcatcgatatgtccttgcttcgatcatctggcgcggaccctagccccatcgtccgcctcagtgacaggggcgggtgcggaatttatcgtcgcggtccgttcgccgccgcgataaacgctggcgcatggccataggcgttttcgactccggcgtgggcgggctgaccgttcatcgcgaactgacccgacgcttccccgagcgcgacttcatctatctggccgaccaggccagcgcgccttacggcgggcgcggcggcgaggacatcgtggagctcacgcgcgccggctgcgagcggctgttccaggccggcgcctcggtggtggttctggcttgcaacaccgcatcggccatcgccctgcgccggctgcagcagacctggatcccgtcgctgcgcgaacggctgggtcggccggtcaacgtcctgggcatcatcgtgccgaccatcgaggccgccaccggcctgccgtggacctatgaggccgaagccgtgcccgagggcgacaaggtcgccgccatcgacatcaccggcgtcttctgcaccgccgccaccgcgctgagccgcgtctacgagatcgagatcgacaagcgccgccacgacctcgccgtcttcgccgagccctgcccgggcctggccggcctgatcgagctgggcgctcccgtcgaggagctgagcgtggtggtgtccgaccacgtcgacgccctgcgccgcaagatcgggcgccatccggacaaggcggtgctgggctgcacccactacgagatcgtcgccgagctgttcgcctcggccctgcccgccggaaccgaactgatccaccagccgactgcggtcgccgattcgctggagcgctacttcgcggcccatcccgaatatgcgctgggtgatgcgggccgccgcgacttcctcaccacgggccagccgggaccccagtccgccctggtcgcccagttctggggcgagccgctgacgttcgagcaggcgtgaagccgaaggctcctccccctttttggggaagggggaccgcgcccgcaggcggggtggagggggaatgcctcacagcctcctccgtcacatcgctccgcgccgcgccacctcccccagaaggggaggatcatccgtcacgccttcttgacgaactcggtccgcagcaccagcccgcgcaccttttccacattggcctcgatctcgtcggcgtccgtagtcaggcggatgttcttgaccagcgtgccgcgcttcagcgtcaccccgcccgatcccttgaccttgaggtccttgatcagcgtcacgctgtcgccgtccgacagccggttgccgttcgagtctttggtcacatcttcgctcatgggcgacgtctaggcgtccggcgtgttcgcctcaagctcgtccagccacagccgcgccgtgccgtccgacggcgcgcgccagtcgccgcgcggcgacaaggagccgcccgtcaccaccttggggccgttgggcagggccgagcgcttgaactgcgccgtctggaagaaccggtgcaggaacttgctcatccagtccttgatgatcggcagctcaaaagtgatgcgttcggcctccggcgtgccggccggccattcgccgcgcccggcgtccttccacgcctggtgcgccagatacgccaccttcgacggcgccatgccgaagcgggtgacgtagaacagaaagaagtcgttcagcgcatagggtccaaccgcgctttcggtcgactggatcttgccgtcctcccctgctggaaccagctcgggcgagatttcggtgtccagaatgccgtacagcgtcgggctggcgtccgcccccaccacctgcttgtccgccacccagcggatcaggtgccggatcagcgtcttggccaccccgccgttgacgttgtagtggctcatgtggtcgcccacgccgtaggtcgcccagcccagcgccagttccgacaggtcgccggtgcccagcacgaacgccttgttctggttggccagccggaacaggtagtcggtcctgagacccgcctgcacgttctcgaaggtgatgtcgtacaccggctcgccgcgcccgaaggcgtggccgatgccctccagcatggcgcgcgccgccggcttgatgtcgatctcggcgccggtgatccccagcgcgttcatcagcgcccaggcgttcgacttcgtgccctccgacgtcgcgaaccccggcatcgtgaagcccaggatgtttgtgcgcggcagctccagccggtcgaacgcccgacaggcgaccagcagcgcctgcgtcgaatccagcccgcccgacacgccgatcacgatgcgctggccgttggtggccttgagccgccgcatcagcccctgcacctggatgttgaacgcctcgtagcagtcctggtccagacgctcggctcggtcgggcacgaaggggaagcggtcgacgccgcgcatcagctcgccccccggcccctcgcctgcctcgaacggcacgaattcgtaggcgtgcggcgcgacctcggcccgcgcgcagtcggcgaaggtgccggtgcgcagccgctccagcccgatccggtccacgtccacgtcggcgatcgtcagatggctttccagcgagaaccgctcgccttccgccagcttcgatcccagttcgtacaccgtcgcctgaccgtcccaggccaagtccgtggtgctctcgccccagccggaggcggtgaacacataggccgccatcgcccgcgccgattggctggcgcacagcagggcgcggtcgtccgccttgccgatcacgatgttggaggccgacaggttcagcaggatgcgcgcgcccgccatggcttggcgcgtcgagggcggcagcggcgcccagtagtcctcgcagatctccaccccgaaggtgaagcccggccggttgtcggcctggaacagcaggtccgtgccgaaccgcaccgcttcgcccgcgatccgcacctcccgctcttccggctgcagatcgaccgccggcgagaaccagcgcttttcatagtattcgcgatagttcggcagataggtcttgggcacgacgcccagcaccgacccgttcgccagcaccacgccgcagttgtagagccggtctccgctgcggatcggcgcccccaccaccgccacgatgcccgtcttcgcggtcaacgcagccagcgccgccacctgccgctccacctcgtccagcagcgcgccttgcaacaacaggtcgtcgatggcgtaggccgacagcgacagttccgggaacacgatcaggtcgcagccctgctcgcccgcctgtcggatcagcgcggcgtgctcctctgcattggccttggggtcggcgatgtggctgacgggggtggcggcggcgacgcgcacgaagccgtgcgtggcgggcgaatgaaaggggtgcgtcttggacatcggctctccgcatcgccgttgttcggctgatagagacaacgccccgcccgccgcttggatcagccgcttatagctgaaccgcgacgctcgagaacaaacgcgccgcgtgacctcgcgcgcttgtggcgctaaggcgatgcgcatgaccgatacgggtaaaaaaggctggttccagcggctgagccagggcctatcgcgctcctccaagcagatgaccgatcaggtcgtctccgccttcgtcaaggagccgctgtccgaggcctcgctggaccgactggaggagcatctgctggagagcgatctcggccccgccgcctccgcccggatcgtggagcggttccgcacccttcgcttcggcaaggacgcgcccgagcgcgaggtcaaggaggcgctggccgaggccgtggccgctgagctgctgccgcgccaggcgacgttcgacccgctgtccgggcccaagccctatgtggtgctgttcgtcggcgtgaacggctcgggcaagaccacgacgctcggcaagatcgcggccgacctgacgggcaagggcgccaaggtgatgatcgtcgccggcgacaccttccgcgccgccgcccgcgagcagctcaaggtctgggccgagcggtcgggcgcgcatttcgaaagccggcgcgacggcgccgacgccgccggcctcgcctttgacgcctacaccaaggcgcgcgcggaagacttcgacgtggtgctgatcgacacggccggccggctccagaacaagtccgccctgatggacgaactgctcaagatcgtgcgggtgctgaaaaagatcgaccccgacgccccgcacgagacgcttctggtgctggacgccaccgtgggccgcaacgccctggcgcaggagcagatcttcggccgcaccgcattcgtgtccggcatcgtcatgaccaagctggacggcaccgcccgcggcggcgtcctggtgcccgtcgcccaggcgtcggacgcgccgctgaagctgatcggcgtgggcgaagggatcgaggatctccagcccttcgacgcccgcgccttctcccgctccctagtcggactggacgactgatgacccaatccgccgccgaccgtaagcgccagtccatccgccaggccgtcgatttcggcgccctggtcgccttcatgatcggctacgcggtcaaccgcttcgtgcgcgggctggagggccaggaggcgctagttcaggcgacttgggtgctggtcggcgcctccgcactggccctcctgatcggctggatggtggagcgcaggctggcgcccctgccgctgctgaccggcggcttcgccctggtgttcggcgtcctgacgctggtgttccacgatccgacgctgctgaagatcaagctgaccatccagaacgccgccctggccgtggtcctgctgggttcgctgccgctgcgccgctatccgttcaaatacttgctgggcgaggcgttccagctgaccgaacggggctggcgcggcctgaccctgcgttacggcctgtatttcgccgccgtcgccatcgtgaacgaggtcgtctggcgcacccagagcgacgacgcctgggtcagcttccggggcgtgctgtggatcgcctcggcggtgttcggcgtctggcaggtcttcttcatcatgaagcacatggtcaaggacgacgaagccgcccccgtgtcacccgacaccggcctgtaaggctccgcacggacgaactgtcgccaaaccgacgcacgatccgcgtcaaaccgtaaagcgccgctgttacctgtgccgcaaggcggaggtcggatcatggtcaaggcgggcaaggcggcgaaaaaggtcgggccgctggcgaattcgcccagccacctgatgcaccgcgcccttcagctggcgctcgacatctatgccgaggaggcgggttccgacggcctgacgcagcgtcagttcgcggtgctggaggccgcctcgctcaaggccgggctgacccagaccgagctggtgcgcctgaccggcatcgaccgctcgaccctggccgatctggtggcgcgcatgaccgccaagggcttgctggagcgcgaacgctcgacgctggacgcccgcgccaaggccgtgcgcctgtccgaggccggccttgcccggctggaggccgcccgcccgcgcgtcgaggccgccgaccgccgcatcatgggcctcttgccaaagggccaccgcgacggcttcctgaagcaactgaccgaactcgccgccgccgccgacgacgcccctaccctcgccaaggctcaggccaaggccgccaagaaggcccagaagctggcggacaaggaggccaagaaggcggaaaaggccgctcgcaaggaggccaaggtcgaagacgaggcggttgaggacacgtcgcccgaaacggtctgatccgagccgcgctgcggccctgcagccccttagacccgcgcttcctccgcgaacgccgtcacgtcgcggatcaacgccgggatcgccgtgtcgatgatcctctggcccttttccggactggcctgcgccgggtccgagccgatgcggccgtcggggaagcgcgcgcggtagtccagcgcgtcgcggatcgggccgttcggcgcgatgcggggctgatagtcggcggtcttgatgcggtcgggatgggcggcctgggtcaccgcgatctcggacggggtggcgtgcgcgccgtggccggtggggaacaggctgttgcacaggcccagcacgcccggcaggtcccaccagttgcgcagcttcagagaaaaccccggctgttccccgccaaagctccagtccgcgtagatttcgctgaacgtcgcttcgatggtggcgacgttgccgccgtgcccgttcaggaaatagatgcgctcgaacccgtgccggctcagcgacgagacccagtcgatgatcgccgccatgaaggtcgagggcctgagcgaaatggtgccggcgaaggccaggtgatgctgggccatgccgatgttgaaggtgggcgccaccaccagccgctcgtcgcccttctccgccgcgtgggcgatgatctcggggcacatccagtcggtgcccagcaggccggtcggcccatgttgctcgttcgacccgatcggcacgatcgcggtcctggacagcaccccgccgtcgctcagtcgcgcatcgatctcgggccaggacgacaggtgcatcagcatgggcgaactccttttcggggaccgcccgcgatctaggccgaccgctcgcctgcgtccaccggcgcgaaggcgcgcacgaagcgcgccgccgcctcgcgcgcgcggaccttgcgctgctcgggcccgatctgggggatgtccagcacggcgcgcagatggccgtgacccagcaccatgccggtaaacatctcggccgcctcgtccggatcgggggtgtccagccgccccgcgcgcgtctggtccgccaaccacgccgacaaccgcttcaggctctcgcccggtcccgcctgatagacgatgcgcgagatctcgggcgcatccgccgacaccaggcagacgccgcgcagcgacgccgtcttttcgggcgcgcagacccgctccagcagcgacagcgccagcgcctccagcaccgcctccggctcgccgccgcctttcagcggcgcggtgacggcggcggaccgctgctcggccagggcctgtgcgatctcggacttggaggcgaagcggttgtacagcgtctgcttggacacgcccgcccgcctggcgatctcgtccatggaggcggccaggccccggtcggcgaacagggctcctgcggccttcaggatcgcatccgtcttggcctcatccacctgtccgggcaggcgcggcatcagtgggcgtccgagggcggcgcggagccttgcgcccgcaccggctgggcgaacagggtgacaaaggccgcgactgcgcaggccacggccagaagcgcgaaggcgtcgccgaacgccagcgtcgtcgcctgccgctgcaggatgccccacaccgccttcagcgccgaggcgtgcggatcgatggagtcggcgaacctctgcgtcaggcccgcgatcattccctgcacgccctggctgccttgcggaatggcctgggtcagctcgcccatgtgcaccgccgtctgggtggtgatggaggtgttcaggatcgccaggccgaaggcgccgccgacgttgcggctgaggttcaccaggccggaggcgttcttgaccatgtgcggcggcaaggtcgccatggtcacctgctgcgaggcgatcatggccagcatgacgcccaccccgcgcagcgcctgcacgcccgcgaactgccagaatccccattcgctggtgaccgcatgcgcatcccacatgccccaggcgcacagcatgaagcccacaaacatcaggacgcgggcgtccaccttgcgcaccagccgcccggcgaagggtcccgtcgcgaacatggccaggcccgacactaccatggtggtcccgacctcggccgccgaatagtcccgcacccgccccaggaacagcggcaagaggaacgtcccgccgaacagcgccgcccccacgatgaaggtcataatgacgccgaccacgaaattgcggttgccgaacgccctcagctccacgatcggattgcgataggtcagcgagcgccagacaaaggccggaaacgccaggcccgcgaccaccgccagcagcaggatctcgtcgtcctggaaccagtcgttcttggccccctcctccagcacgaactgcaggctcatcagaaaggcggccatcaggaacagcccccaccagtcgaagcccttggcgaggctgggatcacccttgtcgaagtcggcgtagcgcccaaccaggaacagcaccaccacgccggggatgacgttgatgaagaacagccagcgccagctcagccactcggtcagatgcccgcccagcgtcggtccgacggtcggcgccagcgtcacgatcaggcccatgaccacgctggccgtgacccgcttgtccggcggaaaggcggtgaatgcgacggcgaacacggtggggatcatggccccgccgacaaagccctgcagcgcgcggaacaggatcatgctctcgatcgacgacgacagccctgtcgccacgctcatgatcagaaagccgacgcaggaggccagaaacagcttctgcgtgccccacagccgcgacagatatcccgacagcgggatcatcacgacttccgggatcagataggcggtctggatccagctgatctcgtcggcggaggcgcccacgcccgcctggatctgcggcagggacgccgccacgatctggatgtccaggatggccatgaactggcccaccaccatgccggcgaaacccagcagcaggacggtccagttgatctcgggggccgaggcgccggccggaatggccgggctggcggcggtcaccgggctgcggcgccgttcgccgccatctgcgcgccgccggcttcggcgaagctgtggccgccctcgctcttcagatcgaccttgacctcgaccgacaggccgggccgcagcgacaggccctggttgcggtccaccacgatgcggacgggcacgcgctgggtgatcttggtgaagttgccggtggcgttctcgaccgggatcagggcgaactcggacccggtcgcgggcgcgaagctgtcgatgcggccatgcagggcgcggcccttgaaggcgtcggcctcgatctcgacagtctggcccagccgcagccggtccagctgcgtttccttgaagttggcgaccacataggtgtcgcccagcggcaccagcgacagcagttgcgcgcccggcccgacatactgcccggcgcgcacgctacgggcgccgaccacgccggccgagggcgcgcggatcaccgtgcgctccagcgccacgcgggccagttcgacctgggcccgcgcctgctgcacggcggccacgctgcgctcgcgggtcgatcccagcacgcccgagctgcgctgctcggcggtcagggcggcctgggcctgcgccacggtggcgttggcgcttcgggcgttggcctgctgcgtctggatgcgctgctgcgagacccagccggcgtccgccagctggccatagcggttcagttcggcctgggcgaggccggcctgcgcgcgcgcctgctcgaccgcagcggcgcgggcggcgatggtggcctcttcctgcgcggcctgggcgtcgacgttgccgacggcggcttccgccgcctgcagattggcctcggcctgcgccagctcggccttctggtcgctgtcgtccagccgcaccaggacctgcccggcttcgacccgctggttgtcgcccaccagcacctcgaccacgcggccggagatctgcgggctgaccagggtggtgtcggcctcgacaaaggcgttgtcggtcgcctcccagcgctggccgttgatccaccacacgacgccgcccccgaccacgatcacggccgcgactccggcggcgatcagcggcaggcgtttcttgacttgaggcgacatcgatccgtccggtgcgacactttgaagcgccgcataaatggacaccgtcgtccagaaatcaacggtgtttctcatcaggcttgaacacgagcggtttccgcgtgttttcagtaacccatgaccgacgcctccgcctcttcgcccctgcccgcccacgtcgatgtcgcggtgatcggcgcgggcgcggccggcatcgccgccgctcgccggctgtcccggcccggcctgtcgctgctggtgctggaggcgcgcgacagggtcggcggacgggcgcacactgttccggcgcgggacggccagggcgccgcgcacggcctcgacctgggctgcggctggctgcactcggccgaggacaatattctggccgcccgcgtcgagcccgagggcctgagcctcgacaagaccccgccgccctgggagagccaggccttcaaccacgaaatgacctcggccgagcagtccgagttccgccaggccttttccgacttcgaggaccgcgtcgcccaggcggcgcaagcaggcgaggacccgcccgcctccaccctgttcgatcccgactgccgctggaacgcgcgcatggacgcgatctcgggcgccctaaacggcgcgcgcttcgccgaggtctccacgatcgactacgacgcctatcgcgacaccggcgtgaactggcgggtgaaggaaggctacggccggctggtcgccgagctcgcgcgcgggatcgacccggccgctctggtgctgaactgccccgtgcgccgcatcgaccgctcgggcgcgcctctgcggatcgagaccacgcgcggcgcgcttctcgcccgcacggtcatcctgaccaccccgaccagccttctggcgtccgaggcgatccgcatcgatccgccggtccccgccctgctggaggccgcctccggcgtgccgctgggcctggcgtccaagctgcacatgacggtggaggggcccgaggactttccgtccgacagccagctttggggccggcgcgacacggcggagaccggcggctatcatctgcgccccttcggccggccgatgatcgagggctatttcggcgccgatctagcctggggtctggaggcgcaaggaccggccgccttcttcgacttcgccgtggacgagctggtctcgctgctgggttcggacatgcgaaagcggctccggccggtctctgcctcgatgtggggcgccgatccctggtcgcggggcgcctattcccacgccctgccgggccgcgcaggcgaccgcgcccggctgtccgcgccgatcgagaaccgcatcttcatcgccggcgaggccactgcgctggatttctacggcacggcccacggcgcctggaccgagggggagcgcgcggccgatcaggccttggccgccctcggccttgacccggtccgcgcccccggcgacagcgaggcatgaaggccagaaccgctcgacccaagaaggccgcacccaaacgcccatccgtcatgaccggcgcggccatcccgatcctggcctggccgccggacgaagacagggtcgaggcgatcttcacccgcctgtcgggcgtcatgcccgacccgaagaccgagctgaacttcagcaacgccttcaccctggtcgtcgccgtcgccttgtctgcccaggccaccgacgtgtcggtcaacaaggccaccgagcggctgttcgccgtcgccgatacgccggcaaagatgctggcgctgggcgaagagggcctgatcccctttatcgcctccatcggcctctatcgcggcaaggcgcgcaacgtcatcgcgctcagccgcatcgtgcaggagcagcacggcggcgaaacgcccctgacccgcgaggcgctgcaggccctgcccggcgtcggccgcaagaccgccagcgtggtcctgaacgaactggggatagagccggccatcgccgtcgacacccatgtgtttcgcgtgtcgcaccggctgggcctggccaacgcctccacccccgacaaggtggaggcgcaactgcaccgcattgtgcccgacgaatggctgcccaaggcgcaccactggctgatcctgcacggccgctacacttgcacggcccgaaagcccgcctgctcggcctgcgtcgtctccgacctgtgtccgtcgcgcgcgggcctcgcggctttgggcgaggcccgctgacgccctaccgctgcggcaaggcgtaggcgatgacgtagtcgcccttgggcgtctccatgaagtggtgcccgcccgccatgatcacgaggtactggcgcccgttctgctcatagatcatcggattggcctggccaccggccggcaggacgtccgaccacaccgtcttgcccgtctcgatgtcgatggcgcggatcaggtcgtcggtggccgccgcgatgaagatcagcccgccggccgtcaccaccgagccgccgttgttgggcgtgccgatctccagcggcaggtgcgagggaatcttccacggcccgttcttgcgcgccgtgccgaacgggcggtcccacagggtgcggcccgtgcgcatgtcgatggcggtgatcccgccataaggcggctccttgcacagcagacccgtccacttcacccgccagccggcgttgacgtcgatggcgtagggcacgccgatctgcggatcgcccgcgccttcgcccttggacaggctgccgccgcgttcggccgcttccttctgctgctggatgtagcgaggatcgtcgcgcgggaaccagcccttctcgttcgcctcctcgcgcggaaccaggcggttgtagttgggcatgtcgttgtagttggcgacgatcacgccgcgccgcggatcgaccgccaccccgccccagtccgagccgccgttgtagccgggatagttgatgtagtggttggtcgagggcggcgtgtaatagccttggtagttcgccttcttgaagttgatgcggcacatcatctggtcgatcggcgacatgccccacatgtcgcgctcggtcagattcggcttgcgcagggtggcgaacagcgagaacggctgggtgggcgagcgctggccctgctcggccccgccggtggtcggaactggccgttcctccatgccgtgcagcatccggccggtcgcccggtcaaagatgtacatgtcgccctgcttggacggcagcagcacggcaggcaccacgccgtttgccgtcgggtagtcgatcagcgtcgcctgcgaccccagatcgaagtcccacacgtcgttgtgcacggtctggaaactccagcgcggcttgcccgtggtgacgtccaacgccaccagcgaggtcgaatactgcttctccagcggccggcgcgacgatgaccagtagtccgccgacgaattgcccatgggcaggaacaccaggcccagccgctcgtcgcccgtggccgtggtccacatgttgggcgtgcccggcgtataggtctggccttccggcggggtagtggtgatgtccgggcgcatcatgtcccaggcgaagcgcagggcgcccgtctcgacgtcgaagcccttgatcacgcccgaagcgttccagcgcttctggccgtccagcacctggtggccggtcacgatcacgccgcgaacgatcaccggcggagaggtgatggacaccatgcccggatattgctcgcccatgccttccttgatgtcgacggcgccgttttggccgaacgccgggcagggccgcccggtgcgggcgtccacggcgatgatccggccgtccagcgtgccttcgatcaccttggtggcgcagggctgggccgcgtcggcgcccgcgcgcgcatgataggtcacgccccggcaggctgcggtgtagggaatgttgatgtcggcgacctgcggatcataggtccagcgctgctgccccgtcgcggcgtccagggcgaacagcttgttgcgcgccgagcagagatagacggtatcgccgaccttcagcggcgtggtttcggcgccccagcgctcctccggcagatcgcctgtgcggaaggtccaggcgcgctccagttgaccgacgttgtcgcggttgatctgggtcagaggcgtatagcgctgcgaactgtcggtcccgccccaggcgggccagtcggcgcccgtgcgcatcatcgccggatcgtcgtagttcagctgcgcgcccggcaatggacgctcgacctgcgcgcgattggcctgagccacccccacgccgaacaccgccgtcgccgcgaccaacgctagggcgctcacgcccgccagcttgcgtccgccgcgccccttcagggccggcagggcggcgatgaccaggaacatcagcaccagcgggccgaccagccggggcaccagcgcccagccgtccagacccttttcccagaacgcccagatcagggtgccggcaaaggtcgcggcatagagccaggcgccgcgcacgtcgcgcagcacgatcagcacgccggaaaccacaagggccagacctgcgatcagatagtaccaggagccgcccagcgccgcgagctgcacgccgccgatagtcagcaccacgccgatcagcaacagcaagacgcccagaacgacagtcagccaccctcccgcactgcggggttggttccaacgcggcatggggatctcctacgacgatacggcgaagcctccgtaacgccttggaagcggagcggttcctcggtgtcgcaccccggaacctttgtggcgttctgcaaagcgctcctctggcgcagagaagaaggctgaacaccgtgattcagcgcaagatttctccgccgacccgcacgcaggcgggggcaaaagaaagatattgcctcactggcgtggccttgttcattatggcggcgtgacccacaagaccatcaagcccggcgggacgtttgtcctcgagcctcgtcgcctgtccaaggcctcggccgagctgcgcgcacgcggcttcggcgaaattaccttgccgccgtccaccgaaaaggcagaggcgcaggccgcgcgctgcacagactgcggcgtgcccttctgtcagaacgcctgcccgctgcacaacaacatccccgactggctgcgcctgtcggccgagcatgaggcgcgcgaagcctggcgcatcgcctccctgacctcgaccatgcccgaaatctgcggccgcatctgcccgcaggaccgcctgtgcgaaggcgcctgcaccctgaaccagtcgggctgggaggccgtcaccatcggctcggtcgaggcctggctgggcgatcaggcgtttgaaaacggctgggtcgagcccatccgtccggcggtcgagcgcagggaaggcgtcggcgtcgtgggcgcgggccccgccggcctggccgccgccgaccgcctgcgcagccagggctatcaggtcacggtctacgaccgccacgaccgcgcgggcggcctgctgatctacggcattccaggcttcaagctcgaaaagcgggtggtgcaacgacgcgtggaccgcctgatcgacggcggcgtccgcttcgtgctggattgcgaggtcggccgcgacgtgtcgctgacggaactgcgccaacggcacgacgccgtgctgctggccatgggcgtctatcagccgcgaatcctgtcggcgcccggacggggaccgggggccaccgtcgccgccctgtcctatctgacgcaacagaaccgccgcgacctcggcgacgccgagggcgacggctggcacgaggcgcgcggcaagcgcgtggtggtgatcggcggcggcgacacggccatggattgcgtccgcaccgccgtgcgccagggcgcggcttccgtcacctgcctctatcgccgcgaccgcgacaacatgccgggctcggcccgcgaggtcgtcaacgccgaggaggagggcgtccgcttcgaatggctggcggcgcccaaggccctgctgtcccacgccgatcaggtggtgggcgtgcgcgccgcccgcatggccttgaccgagccccgcacgggcgaacgggccgacatcgtccccgtgcccgactccgacttcgacatccccgccgacatcgtcatcgaggcgctcggcttttcgcccgagcccttcgccgcgcatgagccggacctgcgcctgcgcgaggacggcacgatccgcgtgggctcggtcagcttcgccaccagcctgcccggcgtctatgcggcgggcgacgcggtgcgcggcgcatcgctcgtcgtctgggccgtccgcgagggccaggacgccgccgccgagatcgaccgtcacctgatgtcccgcaccgaggaggtcgcggcgtgaccgattggctgacccagtatgaagatacccggcaacggctgatcgacgcccacgcctatgatcccgcatccgagcgcgacgcctgcggcgtagggctggtctgctcgatcgacggctcgccccgtcgtgaggtcgtggactacgccatccgcagcctcaaggccgtggctcaccggggcgcggtggacgccgacggcaagtcgggcgacggcgccgggatcatggccgagctgccgcaggacttcttcgcaggccaggtcgcctccatcggccagaccctgcgtccgggcccggtctgcgtcggccagatctttctgccgcgcactgacctgggggcccaggaccgcgcccgcgccattgtcgaaaccgaggctctgagggccggcttctggatctacggctggcgccagactcccatggacctgtcggtggtcggggccaaggccggcgcaacccgccccgagatcgagcagatcatgctggccccgcccctggacgacgccggcgcgccgctggacggcgaggctctggagcgcgaactgttcctgtgccgccgccgcattgaaaaggcggttcaggccgagggcgtctcgggcgtctacgtctgcaccctgtccgcccgccagatcgcctacaagggcatggttcgggccgaactgctgggcgagctgtatcccgacctggaggacccccgcttcgtctcggcctacgccgtcttccaccagcgctactccaccaacacctttcccgagtggcggctggcccagcccttccgcatgctggcccacaacggcgagatcaacacgctgaagggcaacctcaactggatgcggtctcacgagatccgcatggccgcctcggccttcggggagcgagacggcgaggtcaagccggtggtccagccgggcggctccgattcggcctcgctggacaatgtgttcgaggtgctggtccgcgcgggccgtcccgcccccatggccaaggcgctgctgatccccgaggcctgggccaaggacgatgtggtgatgcccgagccgcaccgcgccttttacgcctactgcaatgcggtgatggagccgtgggacggccccgccgccatctgcgccgccgatggccgctggatcgtcgcgggcaaggaccgcaacggcctgcgccccctccgcgtcgtcgagaccgtggacggcctgctgctggcggggtcggaggccgggcttgtctccctacccgagacccgcatcaagcgccgcctgcacatcggccccggcaagctgatcgccgtcgatctgaagcacggccgcctttacgacgagcacgaggccgtggacgccctggccgccgcccacccttacggcgactggctcggcaacatggtcgatctggagccgctgatcggccccggccccgagccgcgcgccgcatccggcgaggccctggtgcgccgccagatcgccgccggcttcagccgcgaggacctcgacctcctgctcgatcccttggtgcgcgacggcaaggaggcggtgggctccatgggcgacgacgccccgcccgccgtgctgtcggcccagccccgcccgctcgcccactatttccgtcagaacttcagccgtcaccaaccgcgtcgaccccgcgcgaagcgggggcgatgagcctgaagacccgcttcaagaacctcggcaacatcctggccgaggaggaggcccagaccgccgtcttcgtgctggacagccccgtcctgaccaccggcatgtacgagcggatgctggacgtggtgggcgcgggctccaccgccgtgatcgactgcgcctatccgttgccggccgagggcgcgcggacgggcgcggggctccgccaggcgctggaccgcatcatggacgaggcggcggccgcggcgcgtggcggctcgggcctgatcgtgctgacggacgaacgcgcggaccccgcccgcctcgccgcgcccatgatcctggccacagccggggtgcacaagcggctgaccgatgcagggctgcgcacctattgctccatcgtggtccgcacggccgagacgctggacccgcacgccttcgccgtcctgatcggcgccggcgccaccgccgtcaacgcgtggctggcccaggacctgttccaggagcgtctggaccgggggctttatcccggcatgaaccttcgcgacgcctgcctcaactacaagcagggcatagaggccggcctcatgaagaccctggcgcgaaagggcgtcagcgtcatctccgcctatcgcggcggctgcgagttcgaggtgctgggcctgtcgcgcgccctgaccgccgagttctttcccggcgccccgtcgcgcatttccggcatcggcctgtcggggttggagcaggcggccatgcgccgtcacgccatggcctggggcgaggcgcggccggtcccctccatgggcggctttttccgcatccgcgcgggcggcgaggcccacgcccacgaggcccgcaccattcacctgctgcaggacgcctgcaaccgcggcgactaccgccgcttccgccagtattccgaggcggttcgacagcagccggacctgtccctgcgcgacctgctcgactttcgcgacggccggacgccggtaccgctggaggaggtcgaaagcgtttcggacatccgccgccgcttcctgacccaggccatgtcgctgggcgccctgtcgcccgaggcgcacgagacgctgaacatcgccatgaaccgcatcggcgcgcgctccgtctcgggcgagggcggcgaggacccggaacgctacctgccccgccccaacggcgacgacgccaactcggcggtcaagcaggtggcctccggccgcttcggcgtcaccgccgaatatctgaaccagtgccgcgagatcgagatcaaggtcgcgcaaggcgccaagcccggcgagggcggtcagctgccgggcttcaaggtcaccgaattcatcggccgcctgcgccacgccgtgcccggcaccaccctgatcagtccgccgccgcaccacgacatctattcgatcgaggacttggcccagctgatctacgacctcaaggcgatcaatcccgacgccaaggtgacggtgaagctggtgtccgcctccggcatcggcgccatcgcctccggcgtcgccaaggccaaggccgacgccatcctgatcgccggccacaacggcgggacgggcgcatcgccccagacctcgatcaagcacgccggcctgccgtgggagatcgggctggccgaggcgcaccaggtgctgacgctgaacaacctgcgcgactcggtgtcgcttcgcgccgacggcgggctgcgcaccggccgcgacgtggtgatcgccgccctgctcggcgccgaggaatacggcctgggcaccaccgccctgatcgccatgggctgtctgatggtgcgtcagtgccattccaacacctgccccgtcggcgtctgctcccaggacgagcggctgcgcgagaagttcaccggcacgccggacaaggtggtcaacctggtcaccttcatcgccgaggaggtgcgcgagatcctggccgcgctgggcgcgcgcaccctggacgagatcatcggccgcaccgacctgctgcgccaggtgcggcgcggcggctcgcatctggacgacctcgacctcaatccgctgctggtccaggtcgaggcgggctcggccggccgcctgtccgacaagggccgtcgccccgtgcccgagagcctggatgcgcgggtgctgcgcgacgccgtgcgctttctggatcgcggccagacgctggagctctcctacgccctgaacaacacccagcgcacggtgggcgccgccgtctcctccgccatcgtgcgccgttttggcgcgcaagggccggccgggcggctgcgcctccagctggagggcgtctcgggccagagcttcggcgccttcgccgcgcggggccttgagctgcatctgaccggcgaggccaacgactatgtgggcaagggcctgtccggcgccgacatctccatccgcacgcccgactggcgtgagggccagctgatctgcggcaacaccaccctttacggcgcgacctccggccggctgttcgtggctggcatggcgggcgagcgcttcgccgtccgcagctcgggcgccgaggccgtggtcgaggggctgggcgcgcacggctgcgaatacatgaccggcggccgggtcgtggttctggggccggtcggctggaacctggcggcgggcatgagcggcggcgaactgttcgtgctggatgcggacggtcgcacgcatgcggccttgaacggcgacctggcgggtgtggccgagatggatgacgaggcggccgatcgtctgcgcgcactaattgaggcgcacggcgcggccacggcctctccgctggcgcggcggctgctgggtgactgggcgaacacagtgcggcggttcgtgcgcatccttccgcatacggcgattgtcagccccgcggaacggcttaagacctccgcctgaagcttcaccgtcccgcctcctccccgagaccgacgcccatgaccaaagccaccgccgcccttgtcgtcacgggcgcgtctctgctcgccgcacctgcgctggcgtcgcccgcgctgctggcgcaccaggcgccgcttgcgatcgacaacgccgccacagggtggatcctgacgtccacggccctggtgctgctgatgaccctgccgggcctcgccctgttctacggcggcatggtcaggaaaaagaacatcatcagcgtcctggcccagtcggccgccgcctttgcggtggtcagcgtcctgtggttcctcctcggctattcgctgtcgttcgggcggggtcccgaggcggtgaacggcctgatcggcggcgtgcaggccgcctttctgaacggcgtcaccgccgagaccgcgcacagcctgctgcccggcctgcccgaactgctgttcgtagccttccagatgaccttcgccatcatcaccccggccctgatcgccggggccttcgccgagcggatgaagttctcggccagcgtgctgttcttcgccctgtggcacctgatcgtctatgcgccgatctgccaccaggtctggggcggcggctatctgggcggcatgggcgtgctggacttcgccggcggcgcggtggtccatgtaaatgcgggtgtcgcggggctggtctgcgccctcgtgctggggccgcgccacggtttcggccgcgacaacatggccccctccaacctggcctacagcgccatcggcacgggcctgctgctggtcggctggctgggcttcaacgccggttcggccggcgccgccgacgctctggccgccaccgccgccttcaacaccattctggccgccgccgccgccgccatcggctggacggcggtggaatggatcgaacgaaagcgtccgaccctgctgggcctcttgtccggcgtcgtcggcggcctggtcgccatcaccccggccgccggcttcgtcgatcccaagggcgcattctggatcggcctgatcgccgggcccgcctgctacgccggcgccgtctggctgaagcacgccctgaagtatgacgacagcctggacgcattcggcgtgcacgggatcggcggcatcgtcggcgcgctgctgaccggcgtcttcgccacggccgccgtcaacccgctggccgaaggcgcgaccgtctggaaacaggccgtgggcctcgccggcgccatagcgtggagcgcggccggcacctttgtcgtcctgatgatctgcaagttcaccaacggcctgcgcgtctccagggacgaagaggtcgagggcctcgactacacccagcacggcgagacgctgcactaacgcccgttccctccgtcaccctcgggcctgacccgcgtgtgacggaggataagcgcgggcgcttccgaccgttgtcgttcgccctcccactccccatcttcatcgggtccggacgtcctgccgacttcggggggcgattgccggaaggtcgcttgttcgaggaccccagatgacgacgcgtacgatcctgttcgacagcccctttctgctgggcttcgaccacacccgcgccctgatcgaccgcgccgccaaggctgcggccgagagctacccgccctacaacgtcgaacagacctccgacaccggcgtgcgcatcaccctggcggttgcgggcttcaccccggacgagctggccgtcaccgtcgagggccgtcagctgacggtcgccggcaaacgcgacgaggcgaaccggggcgagcaggcctttctgcaccggggcatcgccgcgcgcggtttcgtgcgcagcttcgtcctggccgatgggctggagatcgcgggcgcgaagctggagcacggcctgctgcacgtcgatctgatccggccggagacggagcgcgcggtgcgccgcatccccatttccgtcggttgatccacaacttggcgaactacccggcgggtccgggcgttgcctatctgtaaggaggcggtcctatgacgccgatgatgatgaccaaggaagacttcaagggactgggcgcccccgacctcgtctatgtgcgcccggtcaaggcgtcggacctgatggcggatgcgggcgaaatgcaggatctggagatcgatcccgagcagtcgctgtatgcggtccacagcgccgacggcgagcgtctagccgtcatggtcgatcgcgacaccgccttcgccgccgccgtggcgcacgagctggcgccggtctcagtccactagcccgtgggttcaggcggcggcgacggccgccgcgtcgctgacgaacagcgccctcaccgcatcaaccgtccgcgcctgccgcacgcgctcgcgcaactcggccgaccgcagtgcgcgagacacggccgccagcgcccgcagatgttcggtcccgcccgacggcggcgcgaagagggcgaacagcacgtccaccgggcggtcgtccaccgagtcataggccaccggctgatccagccgcaccagcacgccggtcacccggtccagccccttcagccgcgcatgcggaaccgcgacgccgcagcccaggccggtggaccccagctgctcgcgctccatcagcgcctcaaacacctcggcctcgttcagacccagcgcctgagccgccgcgcccgccgccagatgcagggcctgacgcttggacgacgcgccggcgcgcagcttcacgccttcgggcgcgagcaggtcgctgatgtccatcttctgaagtccccgactcaataacaacggccttcgggtcgcctgtcgacgacccgggccgcgccttaaagctctattgtgacgatccgttcccgttggcgtgaccgttcgcaactgtccgctcgggatcgatccagccgacgttcccgtccgggcggcgatacaccaccgacagcccgccgtgcgccgcattgcggaacagcaccaccggatatccggtcatgtccagttcggccacggcgcgccccacggtgatggtgcggatttccgactgcgtctcggcgatcaccatgccgaccggcggcggaccgtccgcctcgcccgcatcgccgaagtcctcgtcctcgaccgtgtcgggatcgcgcagcacgatggagcgggccacctcgcgcgcggcgtcctcggtcttttcgggcgacaggcccttgggtccgatgtggtggtccttcagccggcgcttgtagcggcgcacccgcttctccagcttgtccaggctttcggtgaaggccgaatgggcgtcggcgcccagcccggtcgtcaccagcgtctggccggacgccagcctgacccagcagtcgaccttgaagccgtgaccgtccttggcgacgatcacctcggcgtcctggccgcctcgggcgaagtacttgccgacgccttcttcgagttcctgggagatgcgcgagcctaacgcttcgccgacatccacttgctttccactgacttggacttgcatgcacacagaacgcgacgcgccggctttggtgtcaaccggatcaccgttttgtggtcgggctcagccggccttgagcatgcgccggcgctgcaccgatgagggaatccgcagcgcctcccggtacttggccaccgtgcgccgggcgatgtcgacgccggcttccttcagcacctcgacgatgcggtcgtcggacaagacgtcgccccactcgccctcgccgtcgatcatggtcttgatccggtgacggacggcttcggccgaatggctggccgcgccgtcggtcgcggcgatcgcggcggtgaagaagaacttcagctcaaacaccccgcgcggcgtcgagacgtatttgttggaggtgacgcggctgacggtggattcgtgcatgccgatggcgtcggccaccgtcttcaggttcagcggccgcaggaactccaccccgaacgccagaaacgcgtcctgctggcgcacgatctcggacgacaccttcaggatggtcctggcccgctggtccagcgacttcaccagccaactggcctgcaccgcgcagtcggccacgaacgtcttttcggtctcggaccgcgcgcccgccgccaccaccccgtgatagcgcttgtcgaccaggaggcgcggcagggtgtcgctgttcagctccaccttccagccgccggccggatcgggccgtacatggacgtcgggcacgaccgtctgcgccggttcgccgccgaaccccgcccccggcctaggcgtcagcgccttcagctcaccgatcatgtcctgcagatcgtcggcgtccaccccgcatactcgccgcagacccggcaggtcacgcctggccagcatctccagattgtccagcagcgccgccatcgccggatcgaagcggttgcgctccatcagctgcagcttcaggcattccggcacggaccgcgccatcacccccgtcggctcgaacccatggcacacggccaacaccgcctcgatccgctcgaggccgcagcccagccgatcggcgaactcggcaagctcgccgcgcagatagccgccctcgtccgtcgcatcgatcagcgtgagcgcaatgccttggtcggccggcgaaaaccccgccgtcgccgcctgcgcccgcagatgctcccacagcgacagggcgcgcgtgtccggccgctcgctgtcatccccttcgggcaggcccccgcccgcgccgacgcgcgaccagtccgacaggcccggctgcgccggatcggccgcatccgtcatgcggtcgccgccgcgctcgcccggcgccgcgtcaccatagagatcgtcggatgaggcgtcgaccgcccccagggcctcgcgcccctcgtcgccgttgaagctcagttcgccgtcggcggcgggcgcctcgcccggcgtctcggctgccgcctccgcctcctcgcgctgcaacagcggattgcgctccagctcggcttccacgaactcgtccagctcgaggttcgacagttgcagcagcttgatcgcctgctgcagctggggcgtgatgaccagcccctgcccctgcctgacctccagcctttgcccgatcaccgcgcctggtccccgccgggcgagatggcccggaacttgctagaggctcagattgcgcgggatcggttaacgcgaggcgaacgcggccgcccgcctcgcctctgcgggatcagtcggccaggtcggccggaaccttgccgccgttgtcctgcagcttcttcagcacctgcttgtgcagccagatgttcatggccgccgagtccgacttgtcgccggtgtagcccagctcgtccgccagctccttgcgctcggacagagagctttccaggccgaccagcttcatcaggtcgacgatggaggtgcgccagttcagcttctgggcccgctcggcgttcagcccgtccagcaccgcttcgatgtccaccggctgagcggcgggcgtcgccgcctgcggctggggcgtgggtgcgggagcggcttgcggctgcgcctgaggctgcacctgcggctccatgcgcggctgggcgccttcgggcgcggccttgggcttgccgtggccgcccggacccgacttcgcccgatcccagatgccgccgaggatttttccgaaaatgctcatccgctgctccttaagcttgaagctgaaggagcggtctgcgcgcgcgtcggttcccgcctcgagagacggcgtcgcaacggctgttcgatgaagggaaggggtggagaccgacacgacccgaaggggaattcgttgtggctgctgccttccggccctgaccagattggcgaagccttcgcccgcaccgatctccgtggcggcatatggcaggcggcgcgagcgctttcaacccttctccccgcccgccggcccgcgctagatgaggccatggcttcccccaacaccttcgccggctcccccctcgaccgcgcgggcgaccttcgcaacgatccctactggctggccgagcaggaggcgaacccgcaggcgcgcgcgcttgtgctgtgggagggccggccgctgctgggcgaggacggcggcctggtgtggctgtcgttggctcatgcgcgcgacatcgttcccgaccgcgacctgttcctggggctggacggcgaggcgccggtcttcgccgtcgagatcgagggctcggccgatccggcggagggaccgctgaagggcgcgggcgccttttccgacctgcgttcggccgccgccgtcctgccgggcgcagaggcggccatggcgggcgcggccaagagcctgttcgactggcgccgacgtcacggcttctgccccgcctgcgggatcgagagccgcaccgccgccggaggctggaagcgcaaatgccccgcctgcgggaccgaacattttccccgcgtcgatccggtcgtcatcatgctgccggtgttcaacggcgggcccgagcccctgtgcctgctcggccgccaggcgtcctggccgcccggccgcatgtccgccctggcaggcttcttggagcccggcgaaagcatcgaggaggcctgcgcccgcgaggtcgccgaggaggccggcctgcgcgtcacggccgcccgctatcactccagccaaccctggccctttccctcccagctgatgatcggcctgatcgccgaggtcgacggcgaggaggcccgccccgaccagaccgagctggaggccgtcgcctggctgagccgggatcaggcgcgcgcggtgctggcggcgtcccaccccgactatgtcgcgcctccgccctccgccatcgcgcaccggctgatccgcgcctgggtcgacggcttcgaggcctgatcgatcgcgtcgatcgcggcgcgacccgtcgccgcatcgggtgaaccgcactggcgctgaacggattgcggctgcgacgcgccgcgtcgggcggcgacaacggaattcaaagccatggccgatctgcctcgccgaaccctgctgaccgccgccgccctcgccgcccccgtcgctgtcgcgggggcggcgagggcgcaggatcaggcccctcctcgaccggcgggcggcaagcccctgtccggcaaggtcgccctggtcaccggcgcggcgcgcggcatcggccgcgccatcgcggtggagctggcgcgcgagggcgccgacgtggccatcctcgacatcgccaccccccgcggcgtcgcgggcgtcgacgactatccgctggcgagccgggaggatctggacgagacggaacggctggtgcgcgccgagggcgtgcgcgttctgccgatcgtcgccgatgtgcggaatcttgagctgatgaccggcgccgcgcgtcggatcggggccgagttgggcgggctggacgtcctttgcgccaacgccggtgtgaaccgggcgaccgacaatctggaggcttgggaccaggatacgctggagccgatcatggccgtcaacgtcggcggcgtcgccaatacggtcaaggcagccttgccggtgatgacccggcgtctcggcggccgggtcatcatcaccagctcgatcgccggccggcgcggctccagcggcctcagctattcggcctccaaatgggcggtgaccggcctgatgaagtcgctggcgcaggagctgggcaagcagggcatcaccgtcaacgccgtggcgccgtcgggaacggacaccgacatgttctttcgcggcttcaccggcacgggctcgcgcgaggaggtggcggcccgcaccctgcgcgacagcccgctggccggagtgggcgtgctcgagccgaaggacatcgccgacgccgtggtctttctcgccggacctcgcggcggccgcatctccggcgtcaccctcgacgtcaacgccggccgctcggccagcaacctcggctgaaatcacgcactgtcgtcttctccctccccgcctgggaagggagaagtaaaacgatcttcccccgctcgtcgggggaagtgtcagctcgtggagcggagcgacacggctgacgatgggggaagtctcctgtcgaacgaagactcccctcagcgaccctgaaccgcttcccgatcaacgggctacctctcccgcgaacaggagaggtataagtcgccgaccagcgcgtcatgagcgataaaccctcatggtatcagacacttaatccttttccgccccgacttactcgcctgagttccgacccgtgacatcctgcacaggtctcgtcgcactggagggctcgcctggcctgcgaccttgcgagcggcgggagcggatggagcgggaggtcgtcgggggttcgcctctgccgacgccgggcgcgggcatggtgcgcgtccgagagggtcgagggggatactcggccggtccggggaggatgctcgcagcgtcccctgcccgccgcaggcttaggacttaggcgataagaccgccaccatcccacggtcctggcttgcagccaatcatccgcgcggggcgtcgaaccttcgtcgaaacggtacacaaccactcacactccgggcgaaggcccggcgccccgcccgctctccaaccggatgcatcagcagaccggggcctcagcctgcctgcacagccgccaacgctcgcgcagcctgcaggtccgccggattgtccaccgacagcggcgccgcgtcgatcacccttgcccagatctgcatgcccccctccatcgcccgcagctgctccagcttttcgcgcgtctccagcggcgacggcggcgcggcgcagaatcgcatcagggcctcgcggcgatagccatagaccccgacatggcgccagatcggaccatcgccatacagcgtcgagcgggtgaaatagagcgcccggccctgttgcccgccctcgggcaaggccagcaccgccttgaccacatcgggattggtccggtccgacggatcggcctcggccgaaaccagggtggcgatgtcgcacgacggctcgacctccagcagttcggcgcaggccagggcgaagccgggatcggcgaaaggcatgtcgccctgcacattgatcaccgcgtcgtggcggccgtccggatccagcgcctgcagcgcagcccggatgcggtccgatccgctgggcaggccgggatcggtcaggatggcccgaccgccggccgcctccaccgcctccacgatctccggatcgcccgccgccaccgccaccggcaggcccgaggccgcggcctgcgcccacgcccgcacgatcatcggccgcccgccgatgtcggccagcggcttgttcggcagccgcgtcgcggccattcgggcggggataaggatcaggggattcatggccgggcgcctcgtcttcgacgccatggcctcgacatgggcgccggcgcggttgcgaaggtggcgctagcgtgccagacacgcctaagcaacacgcgcgatcatcgtctgtcgcgcggggctcaaagggatgggatgcggccacggcatgagcggcgatctgaagtggaacaagattttcggcgcagggctcgggacggccttcgtcatcctgctggtccagcaggtgtcgggcgccatctatcataccgagccccctgaaaagatgggctatttcgtcgacgcgccggaagaggccgccggcggcgccgaggccgagctgccgccggactggggcacggtgctgcccgtcgccgacgttgcggccggcgaagcggccttcgcccgctgccaagcctgccacaacatccagcagggcggcgccaacggcatcggccccaacctgttcggcgtggtcggcggccccgtcatgcacgcggccggcttcgcctattcggacgccatggccaagcacaaggccgaggccccgacctggggctatgaccagctggaccagttcatcaccgcgccgggccgctacgtgccgggcaccaagatgtcgttcgccggcatccgcgacacccagacgcgcatcaatctgatcgcctatctgcgctcgcaagggtccggcggcttcgccatcccggcgcccgatccggcccgccagccgggcgcgaccccggccgaggccgccgcggccggcgaaacgcccgtcgcgccgggcgctggcgaggcggccgcgccgaacggcggccaggtcggcggcgcgccggacacgggcgccgcggcccagcccgaaagccagacctccaaccccgcgccgctgagctcggaagccaacgccacgggcctaggccagaacagcccgcagcgctgaggctctaaggcaagaaaagaatcaggaggcggctcttcggagccgcctttttcgcgtcagctaaggcgacgaacgaccggcgcctcgaagccggcggcgcgatagcgagcatcgacctcggccagcgcttccgtcaccacggcgccggcggcgctactggcgtggatcaccgtttgcgcatccagcaggatgccggcgtgcccgccccaaggctcgacttcgccggagcgccagacgaccagatcgccccgccgcgcctggctgatctccacggcgacgcccagctgggcctgctcgcctgcgaaacgcggcccggccagtcccgccgcatacagcgcctgctgcaccaggccgctgcaatccgtcccctcgcccgtccggccgcccagccggaacggcgcaccgatgaagcgttcagcgctcgcggccaggtcacgctcgaaaacgccgaagtccgcaagatcggccgaggcgatccagcccaggcctgcgacctcgaccaggccgtcgcggcgccccgcgtcacgaaccagggcgttcatcggcagggtcgcgatcagtgcgccgccggagggaccggcgaagacatcggcgcggacgggggccacccggtgcgtcggcgcatcggccggcgccgccagcgtctccacctcggcccagccgaccacgcccgaccgccgcgagcggccccaggccagcgttccatgccgctccagcacgtcgaacagttcgccgaacaccagctgatccacgacctggccttccggccggtctcggatgtcggccgcctcgccgccgcacgtcagcggcgtcgtcgccgcatagcggtctgcacgcaccagcccctccagcgcctgttcggcgaggtcggagcgggccagcaaggcgcccggcggcaaaaggtcgaagcggtcggtcaagaactcgcggcccagaaaggattgagccggcatcctgcgccgcgaagccgaagcggccgttaacgcccttcgcttttttcgccgaaacgatcctgcagatagtggaagcaggctctgatcccctgcgcctccccgccttcgggccagcccggccggccgcgcgggttccaggcgaagatgtccatgtgcgcccaggctccggtctccggcgcgaaccgctgcaggaacagggcggccgtgaccgagcccgcctgcgcccatcccgccggatcgttgcgcaggtcggcgatgtcggcctccagcgccccgcgatagccgccccacagcggcatccgccacaggggatcgcgcaccgccgccgccgcctgcagcagccccgccgccagcgcctcgtcatcggcaaagagcggcggcagctccggtcccagcgcgatccgcgccgcgccggtcagcgtggcgaagtccagcgtcaggtccggccgatgctcgccggctcgcgtcagggcgtcggcgaggatgagccgcccctcggcgtccgtattgccgacctcgaccgtcagcccctttcgcgtccgcaggatgtcgccgggccggaagctgtcggccgagacggcgttctcaaccgccgccacgatcaccaccaaccgcacgggcagatcggcctgcatgatcagccggcccagcgccagggcgtgcgccgccccgcccatgtcctttttcatgttgcgcatgccggcggccggcttgatgtccagcccgccggtgtcgaacaccacccccttgcccaccagcgccaccagcggcaggtcggtctgctccaacttccagccgatctcgatcaggcgcggctggcggtgcggcgcggcggcgcggcccacggcgtgaaccgccggatagttcgcctccagcagggcctcgccctcggtcaccgtgatctcggcgcgagcctcctccgcaatctcgcgcgccaccgtctcgatctgcagcggccccatatcggcggccggcgtgtccaccatctctcgcgccagggcgcaggcggccgcgatccgcagcacggcctcgacgtccacgccctccggcgccgccagccgcgcccgcccccgctcgggccgcgccttgtagcggtcgaacaaataggacccgagcgcgaacgccagcgccgcctgcgccgcctcctcgccctccacgttctccaggcgccaaacgccggccggcaggcgcgccgccaaggcgcgcgtcgacatcggatcgaagcgctcgcccgcgccgaacagcgcctgcccgaccccgccgtccgcgcccggcgtcagcagcagctgtcccgccttgccggcgaaatcctgagcggcggcccaggcggcgacgccacctggcagcgtctcgccggaccggacgatccggacggcgcgatcgccttcgccggccccagcggcggagatcaggacttcggcatgaacagcggacatgggcatgacctcaatcaggcgcgggcggcgccagttaaccaagagttgacgcggacaggcgaccctttgcgcctcatcaaggctcgtccggacctccaccatgtcgcgcatgcccgtcgccatcgcaaccatcgcggccctgctcgtcggcggcgccgccccggccctggccgccgatcccgcagcgccggcgaaggcgtccgccgagatccgcgcggcctatgaccggatggacgccctgtcgcgctcggtcttctgggccaacgaacagcaggtcgatccgaacgatccggtggcgggcgtgaagctgtcgcaggcgctgcgcgagctcggcaagttcgatcaagccgcgcaggcggccgaggcgacgctgacggtgcagccgaacaatctggacgccatgctggcgctgggccgcgcccacatcgcgcggggccaggccttctacggcgtcgcgccgctggagcgggcgcgcgatgcgcagccgcgcgactggcggccgctgtcgcttctgggcgtggcctatcagcaggtgcgccgcttcgacgacgcccgcgcggcctggaaccaggcgctgaccctgtcgcccgacaatcccgacgtcctgaccaacgccgccatggcggccatggccagcggcgatgccgccggcgccgagaccctgcttcgccgagccgccgcccagccgaccgccaccatccaggtgcgacagaacctcgccatcgccctcgggctccagggcaagaccggcgaggcggaggccatcctgcgccgcgacctgccgcccgaacaggccgaacgcaatctcgcttggctcaggaaccgcgcgaactcgacctcggcgcaggcgcccggccaaacgccggacgccgcccgcacctggggctcgctgggcggttgacgccttcccgcgccgccgccgccgccctatctttcacccatgatcgacgatctctacagcgcccgcatcctgtcgctggcggccaacctgccgcacagcgggcgactgcctgcgcctgacggcaccggcgagcggacagccaaactgtgcggctccagggccatcgtcgacgtgacgctggacgacgacggccacatcgtcgacttcgcccaggacgtgcgcgcctgcgcgctcggccaggcggcggccggcgtggtgggcgaacgcgccatcggcgcctcgcgcgacgagatcgccagcgcccgcgacgccctcttggccatgctgaagtccggcggcgacggtccggatggccgcttcgaaggtttgcgcgtgctcaagcccgtcgccgactatcccgcccgccacgcctcgaccgccgtcgccctcgaggcgacgctggaggcggtggatgcggcgcttcttgctcgaactcgtctcgccggagcggcctgacgcagggcgtctcggttgatcccccgggctccacgggggataagcgcggcgaaccgcagaacagtctgtttccggcgaagaggcgcgatgtctctctatgaacgcggcgtccgcgcggcccaccagggctacaagctgacgctgtccccctggttcggccagtcgtgccgcttcctgccgacctgctcggattacggacgcgacgccctgatccggcatggaccgatcaaggggggatggctcaccgcgcgcaggctctgtaaatgccaccccttcggcgggtcgggctacgatcccgttccgcctgcccagcaccgggctgagaagacgaaatcatgatcgacctgaaattccccgacggcgccgtgcgccagtatccggccggctccacggcgcgcgacgtggcccagtccatctcgccctcgctggccaagaaggcggtgctggccgaactgaacggccagcaccgcgacatgggtcgggtgcttgagacgggcggcgacttccgcctcatcatgcgcgacgatccggcggcgctctacaccatccgccacgacacggcccacgtcctggccgaagcggtgcagacgctgtttcccggcacccaggtcaccatcggcccggccatcgaggacggcttctattacgacttcgcccgcgacgagccgttctcgaccgacgacttcgccgccatcgaaaaagagatgggccgcatcatcgaccgcgacgccaagttcgagcgcgaggtctgggaccgcgacgaggccatcgcgttcttcgccgcagggggcgagcggttcaaggccgagctgatcagcgacctgcccgccgacgagaccatcaccatctaccgccagggcgagtggctggacctgtgccggggcccgcacttcccctcgacccgccacgtcggcaaggccttcaagctgaccaagctggccggcgcctactggcgcggcgacagctcgcgcgatcagcttcagcgcatctacggcaccgcctgggcgaccaaggaggacctcgacgcctatctgaagcgcatcgaggaggcggaaaagcgcgaccaccggaagctgggccgggccatggagctcttccacatgcaggaagagggccgcggcatggtcttctggcaccccaagggatgggtgctgtggcaggtgctggaggcctatatgcgccgccggctgacggccgccggctatgtcgaggtcaagacgccccaggtgctggaccgcaaattctgggaggcgtccggccactgggacaagtaccggcccaacatgttcgtctgcgaaacggtggagggtgaaaccctcagcctcaagccgatgaactgccccggacacgtgcagatcttcgaccatggccagcgctcctatcgcgagctgccgctgcgtatggccgagttcggcgcctgccaccgctatgagccgtcgggctcgctgcacggcctgatgcgggtgcgcggcttcacccaggacgacgcccacatcttctgccgcgaggaccagatcgtcgaggagacggccgccttcatcaagctggcccgcagcgtccacgccgaccttggcatggagacggcctatatcagcctgggcacccgccctgagaaccgcgccggcaccgacgagttctgggacaaggccgagtccctgatggccgaggcggcccgcgccgccgggaccgagccggtcgtcaccgaaggcgacggcgccttctatgcacccaagctggacttcatcgtcaaggacgccatcggccgcgaatggacctgcggcacgatccagctggactatgtgctgcccgaacgcctggacgccacctacatcgccgaggacggccagaagcatcgtccggtcatgctgcaccgcgccatcctggggtcgttcgagcgcttcatcggcatcatgatcgagaactacgccggcgccttccccttgtggctggcgccggtgcaggcggtggtggcgaccatcacctcggacgccgacgactacgcccgcgaggtccaggcccgcttcaaggccgctggcctgcgtaccgaaatcgacctgcgcaacgaaaaggtgggctacaaggtgcgcgagcactcggtcggcaaggtgccggtcatcgccgtggtcggccgaaacgaagccgccgaaggccaggtcgcgatccgcaggctcggctcacaggcccagacggtggtcacggtcgaggaggccatccgcatcctgaccgaggaagccaccccgccggacttgcgctgaacgggggtgaagacgggctttgtcccgtcttcaccgtatcttaggtcatcgagcggcagtctctttcggaagttccgaaggagcggcgatgacgcactccctgcaatccgcaagctcctcatcgacgctgaccaagcgcacgacgcttcagcggctgatcgcggccggcaatctgcgctactggatcatcgtcagctgggcggtggcgctcgcgaccacggcgcctccggcgatggccttggggtggatgatcgtggctctggcctccggcctcgcccgcaccgtggtggagacgcgcatcaccctcagcgatccggttcggcacgcgcgcctgaagctgtttaccgcctttgtctcatgcgcggcctgggccgcggcgccggtgatcgccttcacctatggcgaactgttcggtgacgcgctggctgtgggcctgcttgtcgccggctacaccctggtcttcacccagatgcgcgcggcgccaagggaggcgctgatcgtctcggcgccctattccgcggtcacggccctgctgatcgccagccagtggggcacccaggccttctgggtgctcgcggcgatcgtccccgtcatgggcctgtcgctgctgatcaaggtcgtcgtcacccagatgaaggacgacgaactgacggcggtgaacgcccgccaggcctcgctgatcgccgagcttcaggccgcccgcgacagggccgacgccgccagcgccgccaagtccaacttcctgggcgtgatctcgcacgaactgcgcacgccgatgaacggcgtcctgggggcagcccagttgctggagttcaccgaactgacggagcggcaaaaggagtatgtcggcgtgatccgcgcctctggcgacggcctcatggtgctgttgaacgacatcctggacctgaccaagatcgaggccggccgcatggacctcgcccccgccgacgtcgacatgtcggacctcacgccgcgcctgatcggccccttcaaggcccaggccgaggccaagggcctcgccttcgagacgaccgtcgccggcgagatgccggaccgcctcaggctcgatccgctgcgtctggcgcagatcgcgcacaacctcctgggcaacgccatcaagttcaccccccagggcgtcgtgcgcttcagcctgaccggcgaacggctgtcggacagccgggcgcgcctgaccctggccgtggccgacagcggcatcggcatcgccgcctccgacgtcgagcgcctgttccagcccttcacccaagtggacggctcctccacccggcgcttcggcggcaccggcctgggtctgagcatatgccagcggttcgccggcatgatgggcggggagatcacggtcacctcgcaacccgaccaaggctcggtcttcggcctgtcgatcgaggtcgaggcgctggcctggcccgctgtccggctgcagagccaagccgcctgaccgcggacgcgcctaaagccccagcggcccaatcagccaggtcagccagattccgagcgccagccccggaccgaagggcatgcgatcgctccccgaggccgaccgccgcacgatcagccgcgcagccacgaggctgaagcccagggcgcaggcccagagcagcacgctgggaagcccctgccatccgccccaggcgccggctccggcgaaaaggaaggggtcgccgtcgcccaggccgtcgcgtccccgcgccagccgatagccccaggcgaccagccacagcgccgcaaagccgacgccggcgctcagcaccccgtgccacccctgccccagcagcacggaggcggccagtcccgtgccgatcaacggcagcgtcagcacgtccggcagcagcatgtgctcggcgtcgatcaccgcgatcagcaggagctgccatcccagcaccgccgtgatcgccgccatggtccagtcgccgaacgccagccccgcccagccgccgatcagacccgccgccgcctccaccgccggatagcgggcggagatgcggacgccgcatcgcgcgcagcgcgccctgagcgccagccaactgaagaccggaaccagctcccaaggccgcagccgacgttcgcagctcatgcagtgcgacggcctggacaccacatccacgccctgcggcaatctcacgctgaccacggccaggaagctgccgacgatcagccccagcccgccgagcaccacagccgtgatcgccggcgtcgtcatggcaaggtcagtcgcgcagcaactcgttcacgcctgtcttggctcgggtctgagcgtccacgcgcttgacgatcaccgcgcagtacagcgacggtccgccgttcgcatccggcaaggctccgggcacgaccaccgaataggccggcacctcgccccggaacacctcgcccgtcgcacggtccacgatcctggtcgaggccgacagatagacgcccatggccagcaccgcgccctcccgcacgatcacgccttcggccacctcggcgcgcgcgccgatgaagcagccgtcctcgatgatggtgggattggcctgcagcggctccagcacgccgccgatgcccgcgccgcccgacaggtgcacgttcttgccgatctgcgcgcatgagccgacggtcgcccaggcgtccaccatcgagccctcatcgacataggcgccgatgttgacgaaggacggcatcagcacgacgttcctggccacaaaggcgccctgccgaacgatcgcgccggggactgagcggaagcccgccgcctgatagtccgacgccgtccagtcgccgaacttgttgggcaccttgtcgaagaagggtccgacgccgggcgccgcgctggccgcgccccaatcgccggcgcgcatcaccacattgtcgttcagccgaaacgacagcagcaccgcctttttcagccactggtgcgttgtccaggcgccatcggctccacgcgaggccacccgcgcctgcccggaatccagcagcgccagcgcccgctccaccgcctggcgcgtctcgccccgcgtcgatggcgacaggtcggcccgcccctcccaggcggcttcgatcacggattcgagttgggcggcttcgctcatgcggcggcgtccttgaacgacagagagaggagaaaattcagcagatccggcgcctgatgatcgatatgcggccccagcggctttccatgaccgtcgccgatcaggaccgtgcgcatgcccatcgccttggccggttccaggtttttcggcgtatcttcaaagaagacagccctatgcgtgtccagcccaaagcgctcgcacatccgacgaaaggtggcgggcgcgggcttgggcgtcagatcggcatcctcaatggcgaacacgtcatcgaagcagtcggccacgcccagccgatccagcacccgacccgcatactcgcgcgcgccgttggtgaagacaaagcactggcccggcagccgcttcagcacttcggccaaccgcgggttcggctccagtccatccagcggcacatcgtgcacctcatggaggaaccgctccgtatcgaccgcatagttcgccatcaaccccgccaaggtcgtgccgtgctcgtccagaaactgccgctgcaacaccgccgcttcttcaggcgcaaggcctacagcctcgaccacgaacgcgttgatccgcttctgcaccagccccatcagcccctgctcgggcggataaagcgtgtcgtccatgtcgaacacccagaagcgaacgtccgacagatcgggcgcggcgaccatcacccggccgtcaccagggtgccggcgccgtattcgctgaacagttcgaccagcatggcgtgcggacggcgtccgtccaggatcaccaccgcctcgacgcccgcgcgcaccgcggccatcgccgtctccagcttggggatcatgccgccggtcgccacgccatcgtcgatcagcccttgcgcctcttccagcgtcatctggcggatgatctcgccgtcagcgcccttcacgcccggcacgtcggtcagcagcagcatccgcttggcgcccagcgacccggccacggcgcccgccacggtatcggcgttgacgttataggtctggccgtcctcggccaccccgatgggggcgatgaccggcacccagtcctcggtctccgaggcgatcaggcccttgatcagcttggggtcgaccttggtcggttcgccgacgaagcccaggtcgacctcgtgctcgatcatgctgtcggggtcgcgcttggtgcggcgggtcttctcgaccgtcagcaggccggcgtccttgcccgacaggcccacgccgcgcacgtcggcctccttgccggccatggtgatccagtgggcgatctccttgttcacggcgccggacaggaccatttcggccacctccatcgtcgccggatcggtgaccctcagcccatcgacgaaggcggacttcacccccgccttgtccagcatggcgctgatctgcggcccgccgccgtgcaccacgaccgggttcacccccatcagcttgagcagcaccacatccgcggcgaactgcttggccaccgcgctctcgcccatggcgtggccgccatatttgatgaccacggtctcgcgatcatagacctggatatagggcagcgcctcggcgagcgtcttcgccgtctcccagctgcgttcctcggactggcgttcggtttcattcatcacgcgcgcgtgatagcgggggatgggggtgaagtcacgacctcagtctgtgatcaggcccgcgtctgtatcgtcaatctcgaaacgccgcctctgaccgtcgatctggtcgagaaactcgcgggtttcgctcccgcgcgcgaaggcggtgagcgttgcgaagacctccagggctggaggatggtcattgccggagtcttcgcggtgatgctgaaggtcgggcgaaaggaaacctaaaatacgatcagcgacgctcgggtcgtcgagggcgaaatcgatcgatgctaggttttcgattttggccagttgagtccgccaatcggagaggaaatcagaccacctaatccaggcgcgggcctgccccctggtgaagcgttcggcatctagcacgtgccttagccacaatcttgcagcatcggcaggcgagatgccgttgcggaactccaaggacgcttgcacctgagccgggtgtcgaaagataagaatcgcgagcgggtcgtagcccgaacgctgaagcacctctctccagaacggataaaggcggcatatgcgtggatatttcagaacaagagtttgggcttgcccgaactcggattcgaggacatcgcggccctcatcaacgaagggaacagcaagccgttcggagaaagggcgtgaatcagaccaagcagaaccgtaggacgccaagattctatcgttgagattcatcgccgataacgtcgtcgagcacgaccaccggtgcgcgctgaactgacgcgccgttgtccctaaagctgtcttccagctctgcgtaaggaagcgtccaagtcccaccgggattgccgaggtccagattccaaccgatgaaaatctcgcccggagcttcgccgaccgcagcgttgaccaacgtcgccctgtcggaaagccgttatcgtaaaacgttcgcgacagggcctcaaacgtgtcctttcgaggttcgaaggagaatatacgcccttccggaccgacccgcttggccgcattggcgaaaacccatccgatgttcgcccccacgtccacgaacgtcattccagtcttgaccaggccacggataaacttggtctcgagcggctcaaaaccgccgctcacgcaatggcgagaacccccagatctccgagatcggcccacaacaggaggtcagccacttccacccgagcccaggtcgaaggcggatagttaggtctgagcttctctccgctatggattgagcggaactcttcgctcgcggagaaccgagcgagaatatccttcagttcgtcttcttcctccggctggcatgaggacagttcaaactctgcggcggcggcgacatcaggttcgcgacgaagaaggccgcgataggcggcgcgcgtcagagcttcctttgcgagttgaaaagcttccgacatggcgacgctccattctaccgccccggtcacggagcttcgcaagccggaatgccatgaaatccgaggccgacaaagggtcgttcaccggaggtagttatgcctcgacttgccgcctcgggctcgttaaggaacgtcaaaatcagcaacaaccaatgatatttcggctcatcatgatcgagcgtttccgtgcctactccctcagaaaatccgcgatgcggtcaggtaaggcgcagcgctggaataaagcgatcgagcgctatgaagctctggttaagacaggagttgtccgtccctccgacggcgttcgccatgcccaggcgctcgaggcggtcggtcttatagatgccgcggcgcaagttcacagggacaacgtcgggcgctttcccctcgagccgaatgtccatcgccagacaggcctgtttctgctgaggcagcacagagaggcggaggcggcgttgagcttggcgaaggctcttgtgttggcgcctacggacgacgtgctgaaagcggatatcgatcgcgtggggatcgcagacgatcgtgtcggcgccgtcgcccttgccgccttttacgcatcgccagcgcctcagcctccacggcctggcccgctgaagcggttcttcgcgcgtcgtgcggccgcacgggcgaagatgctgcgtcagtccggggattggacgaaagcgttggcggcgcagaggacgatcctgacgaacaatcccggaaatgcatcggcgcaaacccgactggggcatgttctgaaggagcttggggacgttaaaaacgctgagacggcgtattggaagggagtggcgctggcgcccaagcacgcggacagttacctgcaactcggccatggcctcaagctcgctcatgggccaaaagccgccctgcctgcctatcttctggcccagcgccttcagccaagtcatgccgaggccggtgagggggtcaagcaaggcgggctatcggatcacgacgccaccagattctccgacctgttagccacagccgatctcgaggcgatcctcggcttcaccgagacgtctaggtcacccgagacccacccccctgaaaaccgcaaggtcgtgccggtctttcggcgtcctcggccacgcgctatcgatgtgcgggcggcggccatcgcgggggacatcgcgcggaccgttggggtaaacctatgaaaatcgtcatcgatctccaggcctgccagaacggcagccatggccgaggcattggccgctatgcgatgtccatggcccgtgcgctggtgcgcaacgggcgagaccgtcacagcttccggatcctgctctccgatcggtttcccgcgcgcgttgatccggtccgcgccgccttttccgatctactggagccgcacgagatcgtcgtcggcgccgttccgccacgcgtggaaagcgctgatatgcatctcgcctggcgcacccgtgcggccgaagtggcctggggcgacttcatcgccggcttccagcccgacgcctattttacgccgagcctgttcgagggcttctgggaagacgcggtgacctcgatcgagccggcctcccacattcgcgccgcgacgatccacgacctcatcccgctggccgatcccgacttctatctggtcggcgaaggcaacaggcgcgcctatgctcgcaagatcaacgccttgaggcgctgcgacttcctgttctcggtgtccgaattctcgaaacaggacgcggtcgagcgcctgggcatcgatccaaagaaaatcttcgtcatgccgctaggcgtcgaggacgaattcagccccggggaagtaccggacgaacggcgggaggagctcctgcggcggcacaggctgaaggggcgggtcgtcatcaacaccagcccccttgaggccaggaaaaacatcccccgcctgatagcgggcttcgcccgcgtgccagccgacgtccgggcgaacacccagttgatcatcgccggcaagatgagcgagcatgaccgcaacgaaatagccgcgatcacggccgccgaagggctggctaagaccgacgtcgttctcccgggcttcgtgccggacgaggatctgatcgatctctatcgcctgtgcgaggtcatggtcttcccgccgttcagcgaaggcttcggcctgccgccgctggaagccatggcttgcggagcggccgtcctcgcctcctcggccaccagcgttcctgaggtggtggggcgcaaggacgtcctgttcgacccgaccgacgccggggatatcggccgtgccatcgcacgcgttctgggtgatcccgcctatcgcgacgaactgcgtgcgttcggacccaggcaggccgcgacgttctcgtgggatcggtcggcccaatcgatactgaaggttctggaaggcgcgccgcgccacggtgtggccgagacgccgccggccgcgccagcgcggccggcggtcaaattggccgtggtggcgacgggcggcataccccacagccgtgaaagcttgctggtcaaggactatgtccgccgcctatcggcagcctatgatgtgacccttttccagctcgatggcgacctgggccacgatgtctccatcccgctggaacggcgaagcctggacgacttcattatccacggtggcggcttcgacagagcgctctacatcctcaacagcagtcggaccgacatcgctctgccgatcatggcggcgcgtccgggcgccctgatcctgtacgaacaggcggcgccggtcgatccacgcagcatgtgcgacagccaggtagccgatcagcgcgccagcggcggtctgaacgccgcgccgaaccctcagaggctggaagagacggcctggaagaagggcgccgcagcggcggcccttgcccacgggctggccgttgaaggcgattccatcctggccggccgcgccggcgtggcgaccgtgacgccgaggcttcaccgcctgcctgccccgaccacgatcgacttccggcgggcgcgaggaattccactcgatgtggagctctgggcggccttcgctgcggatgacgaaggcgcccggcatatcctgcagacgttccgccagcatcgcccggcggcccgggacaaggtgtggctggcgctcgtcccggcccacagcaccatgaaggaggggcatctccaggggcgcgtctatgtcatgcccaacgggttcacagagccgtacgccgaactgatgagcgctgcctccgccgtcctgatcgacgaacaattgccggcctcatcgcgtcgccggctcgaagacgatgcgcgcgctttcggtctttcgctcctgtcggcggacctgagcgcaagccggagggggggagacgcgggcgccgaggccgcggcaggcggcttccacggctggcctccggccgaggacgcagccttcctcgcggcgatcgagtccatgctggaacagacgccgcctccgctggcggcttcgccttcaatgctcgatcgaattcccgctatggccggcgaccgccgcccggaaccgcaggacatccgggatcttggcgcggcgttggcgcggaacgccgagtttggcttgcctggacgcattctgatcgacgtgaccgcgccgcttcgcgagaccgccgccgggctttccggcccgacgcggcgctttctcagggcgctgctgtccacggagcaggatgtgcagctcgtcgccaccgacggagaggcctatttcaccgccggcggcttcatgagcgtgctgctggggatcaccaccttccacgacgaggccctgagcttcagggccgatgacgttctggtgggcgtcgatcttctcgacggcgcgacggacgccgagtcgttcgacgcgggcgcccggcgtgtccgcgtgcaggtcgccgacctcgtcttcgaccgccccgatctgagctccctggccgctgcggctctgatcgaagccgtcgataacgaacgatccggcgcccccgcgaaggccgccaccgccggaccgctccaacgaagcgtggtggaaggcgcggttcatatccgtctgcacgcccccacatcccgtgccaagaccgccagccttggcccggcggtcgccgccctggccaaggccgcgttggcgcccccgccccgcgcagacagccgcctggacacctccttcaccgttcaggggcatgtctggggaacctacagcctggcgatcgtcaatcgccggatcgccggggtcttgagcgaagcctatccgggccgcgtcgatttcgcgcctgtcgagacggtccccgtgactgatctgaccgcggttccggaccctgaccgtcctctcatccagtcgctgctgaagcccgcccgccgagcaaaggtccacgccaccgtcagccaacactatccgatccagccgccgctcagccgtaccgaggtcggcatggcgctggtggcgtgggaggagagccatctgccgccgaccatgatcgatgcgctgaacggggccttcgacggcgccttggcgcaggtgcggaccgttcagaaggccttgatcgattccggcgtctggattccgtcggtcctgaccggcctgccggccgagatcggcgactatgagggcgcctgccggcgcaagggtccagcccggaccttcctgcatgtctcttcgtgttttccgcgcaagggggtggacgtcctcctagaggcgtggggccgggcgttcaccgcgaaggaccgggtcaaactggtcatcaagaccttccccaatccgcacaacgatgtgcaggagcgggtttgggaactgtcgcgacgctatccggcgatggcgccaattcaaatcctgaaccgggacatggagcgtgacgaactgatcgacctgttccgggacgcggacgtcatggttttgccgacccgaggggaaggctacaatctgcccgcactggaggccatggcggccggccttccgctgatcgtgaccggccatggcggtcatcgcgacttctgcagccccgccgaggcccgtctgctcgattacgacttcgcgctgtcggccagtcatgtgcgagagaccgtctcctactgggcggatccttcggtggacgatctggtcgaagcgctgcgtgaacagatccggccggaccagcaatcagccatcgaggcccgccgccgccgcgccctggccagcgcccgcaaggccgtcgatccccgtcgctggagccggaccgtcgccgacttcgcccagtctctggcggggcctgtggagcgcgggccggtccgcaccagctgggtgtccacttgggcgattcgctgcggcattgctgagtactctcgcttcctgatcgagcaggcgtcgcccgagtggcgcgaggtattggaggtggtggccgacgatcggaccgacgcggaacccgatttgaccacccaccgactgggctggagcatgggatgggattattcatcggagcggttgctagaggacatcagtcgcgccgatcccgaagccgtcgtcatacagcatcaggacggcctgatcttttggcgcggcctggcggagttggcgaatgacccccgcatggcggcgcgcgtcaccgtcgtcaccctgcacacggtgcgcagcctagacgcgctccccgaggacgagcgtcgacacgtggtcgagtcgctgggccgctttgatcgcattctcgtgcacaccgtcggcgacctgaacgacctcaaacgtcatgggctgatcgacaatgtcgctctgttcccgcatggcgccatccggcccagcacgcccgcgccggcggttcgcgccctgagcgcgggctcgaatccggtgatcggctgtcacggcttcttcttcgaccacaagcgcatcgaccatttgatccgcgccgccgccaagctgaagccgcaatggccggggctccgcctgagactggtcaacgcccagttccccagccctatctcggccagcgctatcgcccaggccaaggcggtcgcagccgagactggcatggagggctccatcgactggcacaccgatttcctgccggtcgaggacattcaggccctgttggcaggatgcgatctgctggttctgccttacgacgagaccggcgattccgtcagcggcgccgtccgcgtcgccatgagcagccaggtcgcgacactgaccacgccggtcaagattttctccgacctgggcgacgccgtcgcctcagttccgaccaatgagcctgaaaaactggccgaagcgatcaaggccctcctggagtcgccggaggaccgttcggagcaccagaagcggatgcaggcgtggctggagatgcacgactggaagcgcatgagcgccaacctggaaggcattgtgaaggccttggcttacgcacgccgtcgcgaggttcggcagtcggcggaggagatgtccgtggtggcagcggagtgacaagggaaccctttgggtttgttcaaattagaagatgaggaagcagtcgcccttggatcattgtccgagcacctggcgggctttttcatctgcataggtctggcggaaggcgtgaaatgacgggaatgtcgaaagcgttgcattccctcaaaagaggcgtgctgacgcgtattccgaggagcggacgcaaggccgaatcggcgagagctatcccgatcgaaagctcaggaacattccgcgaagacagcgtgtccgcatcttcgttcgaagaaaaatggctgctgatctcgaactgccagacccacggcttggccagggcgctgcagatggtcaactccaacttcagtgtcacgccgatggactattggaccgctatccgcgatcctgaggcggcgcgacgcgaagcgctcgaaggggggtattttcgcgtcctggtctccccggagatcgaggaggccggcattgatctgaccggagcgccgcacctgacccgcatcccgcgcgtggtcttcaccgcctaccaccctgactgcgtctatggcctcagcgatgggaagcaggcaaaggggccgctggacgcctatcattcgatgatcgtcatggcggcgcaccgcaagggcatgaaggccgaagacgcccagcgcctgttcaacggcgccttcttcgagaaggtcggctatatggactactgggttccccagcgtaaccgcctggtcgccgaatacgcccggttcggcctggacatcagcgtcggcgtccgccgctggggccggacctcggcgttcatgcacacggtggaccaccccaagatgacgtgcctttacgacatcgcccgcgccatctttgcctcgatgtgcgtgcccgaccaaggggccgacatcatcccgcccgacaatctgtgctcgggcgtctccttcgcggtctatcctgaggtcggcgaggccttgggcgtgccgggcggctatcgcttcaagcgcttcaacgactatcatcatatcgggctcgagcagttcatcgccgagagctatcggggctatgacgccctgcccgagatccggccggacgacgggtccatgcccgccttcaaccgcgtcctggaggccatcggatgacgaatccctacaagggtctgcccgaccatcagttctggcggcgcggcgttgcgggggtcgagcaccatcggctggatccgatcgttgcgcccaagttccgcatcggccgcaccgaccgggtcgccaccgcaggcagctgcttcgcccagcacatcgccaagcgcctggcgcggacgggcttcaactatttcgtcaccgaggacggcgccgatctgacgccccagcaacgggcgaagcggaacttcggcgtctattccgcccgctacggcaatctctacaccaccacccagctgcgccagctgttccaggaagccttcgaccaccgccagccggaggaccgggcgttccgccgcccggacggtcgcttcgtcgacgccttccgccaacagatcgagccggacggccacgagaccgtcgaggccgtggcccaggcgcgcgccgaacatctggaggcggtccgccggatgttcctggagtgcgacatcttcgtcttcaccctgggtctgaccgaggcgtggcgctcccggtcggaccagtccgtctatccgatcgcgcccggcgtcgtcggcgacggcttcgacccggatcggcacgaattcgtcaacttcgacctggccgccgtcgagggcgacctggaagccttcctggcggacctgaagcggctcaatcccggcgtgcgggtgctcctgacggtgtcgccggtgccgctgatcgccacctatgagccgcgccacgtcctggtctcgaccacctacagcaagtcggtcctgcgggtcgccgccgaacaggtcatgcgccgccacgactgggtcgactacttcccctcctacgaaatcatcaccggcagctacgccggcggcctctattacgaggacgacttccgcgaggtgaacaatctcggcgtcgcccacgccatgcgctgcttcctgcgcaactacaccgagggcggcgcgcgccaggacgacgcggccgccgaggtcgccgcccgccgcaccaccgacatcgtctgcgatgaggaagcgatagctgcgacggtctagggtcatccccgccgggcgcgctgcgcctcatagaagcgcacgtcctcggccagcagatcggccagacccgccatgcggcgcatgtcggcgcggatcgccgccctttccccgtcgccgctggcggtgggatcgtcgtgtcggtccggctccagctccaggccggcgatggcgttcaagcgtgccatctccggcccgcgggtctcatgaaagccgatgaagtcgaaccgctccatgtcgtagcccccgaagaaggtgtccgagctcaggccgcgaatcggcggccaggtcgcgaattcctcgatcgtcggctgtcgtccaggaaccggcggtgcagcgcctgtccctcgtgcggcatggtgcgccagaaaaaatagaacgacagcaacatcggccgggccttagtccgaaatcctctcgatcgtggcgccgtgaaaatggacctgtccgtggaacgccccctcatgcaagaacagtcgagcttcgctggcctcgtgtcttggccattcgtgttccagggcgatctcgaatagacctgctcttccaggcgaaaactcatgcgcggcgtatgaatcgccgctgccccagtgtatctcatagcgcttcggggccgcgtcctgatcaaagcccagccgaatagtggcccgccagactccgggcgtcaggaagatgtaaggaccgaagacgacaagccgaggccggccggttatatcgaccacccccacagagtcgctgacggttttccaacctgcgtaatggaagactgctggcgaccattgggcgcgaccctggtcaagaaaccgcaacgcattgcggaaggtgtcctcgagcggactgagcggtcgctctgatctctccggcgttggcgtgttggcgaacggctcgggcagccgatccaagcctaggcggacacgttggccctcaaaactatgcgctgcggcgatctttcgcgtcacatcaagaatgcgaaacggccgttgcccatcctcgcacccttcaaggcctacgaagggagagccgagaagaacgaccgtgtccgccggctgcgcccctgcaagacgggcgacatccaaatcctgggccagaccgacgcttccgtgaggaaccgtctcggtccctgcgaggacttccaccacaggcacgccttgcgccgacgcctgctgcagaagggcgcgccgccaatcatccgcctcctcggccggcggcagaacgtaccaacggaaaggcaggctcatcacgccgccctcagccatgtgtacacgtcgacagcctcggacacgtcgctgaacatcttggcgcgtccgctctcaatcaccagggcggtgtcgcagtagctcgcaacaaggtggacgtcgtgagaagccatcaagaacgcgcggttggcgcgatgctgaaacagctcctcctggcacttgcgctggaatctggcgtcgcccaccgcaacaagctcatcaatgaggtagcagtcgaactcgatcgccaacgaaagcccgaacgcaaggcgagcgcgcatcccggaggaatagtgcttgaccggccgacgcaacgccgatccgagttcggcgaaatcgtccacgcggtcacgcatctccttgtaatcgcgctcatagaggcgggagaggaaacgaatattgtcaaggcctgaaaggctgccctggaatccaccatggaagccgataggccatgaggacgacatccgccacgcgatgcctccctcggacgggcggtccacgccgccgagcatccggatcagggatgacttgccctgtccgttacggcccaagatcgccagccttccatctcttttgagagagaagctcaggttggtgaacagcggcttggccgcaccgcgaaacgtccgactgaggttgtcgacacgaagccctacctcggtttgcgcaccctgcattaatcttgccgatgctcgcggacgcccgccaagaccaaccatccaatgccgtagagcagcagcgacgtcgccagtaccaccaggatggagatcaatcggcgcggctggctcgggcgatccggcaaactcgggttgacgactcgttccaagtacagcttctgtcgacgggcttcttgttcagcgctcaagagcgtcgccgtggcctgggtcagctctcggtcggccagttcacgctgaagcatcagatcttcgtaagctccaagcttgcccgcaagcgagtcggcagaaccagcgatcttggctcgctcggcctcaatctgccgttcgtaggcggcgattcgattatccaggagcggcagctgcgggctgctgggcgcttccgccgccagctgagcgcgctctgcccgcaaagttgcgaccgtcgcgagaagattgccgatcaattgaccgccctccgtggccgaacgcgcaggatcgataaactgttcgcgattccggaacgtcgtcagctgttcctgagcaaccgtgagccgttgacgggcttcgtctcgtaccgcacgagcatcgctgacagcgtcagcggcggcgcggtcattgagacgattcaccagccgttcgcccccattaagcagagcttcagcaaggcgttgcgcatcggcgggcgcaaagccttgaacacggagcgtgctgatgcccgtcgttgaatcatagccaatgctgacgaagcgggacaatgcagcttccagcgagcgatccgaccgatcctcgcctagcctcggccaccccgtgatcacatcgcccccccgcggccgcagcatcgaagacaggtcgaaacgccgcttcaattcctcaatgctgtcctgcgagagcgcatattcgtggaccgcgaaggcatcggtggaggtggtcgataagcctacaccctgcagggcgaagcccaaagatgtaggttgtggctgattggctgcccggacgatgaagcgggcttccgagacgtagcgcggcgatgcgatcagcaagaaatagatggccgccacgagcgtcgggagaacgaccaccaccacaaaagcgagcgggatcttgcgccaccacggcgtcgccgcatgggacgacgtcagcaggtccggcagcggaccgacgtagttgagcttagggtcgttcatcattttagcaagaaccggttcattctctattcagcctcgatgcggtcgcgcgcggtcgcaatcaacagcaagcctataatgttgagcacaatagcccatcctaacgggtaaagaggggagtaatgcgtcggaacatactcgccgaaaacgcccaccctcatcatttcaacgcaatgaacaaacggtatcatcagatagtatttctgtaccgccgacggaaaccaagaaaccattgcaaaggcccccgacaacgggatcatcaaatatccaatcaaccctgtaatccgctcaacaaactcaaatctgatcgaaagccctgtcagtataagcgcaaagcctgccgaaagaaacccaagcgtgaaccagccgtaataaaacaggagataatcatgaggaagctttacctgaccaatcatgatcaggaccatatacacaataaagtaagcagttgtcgcgcccccaaactctaggagcagccttgaggaaagtatatggagtggcgtcacgtgccggtgataaaggatgccgatattggcttgcagcgcgacggtcaggtaactgataaaatgtcttatcaggatgattgacagataaccggtcatcacgaacggcgcgaggcggacgccatgctcgtagctgggcttggtgacgctccagagcgccatcaccccaaaggtgaaaatgagcggctcgccaataagccaggcgaacccgagcccttcccgaccaaagcgggtaatgacctctctcatcatcaaggcggtgacgatgcgcgtgttgcggcgcacccccgcccaaatggcgaagagggacggtcgcgaagaacgcggagagaaagtatttagagacattcggcctgaaggtaacccagacgacggtattacgcgcccgagggcgtaacgccaatggcggaataggcgcccagaaggcgatcacgataggcttgagggttgaacttggcggcttgacctcgcccgcacaactccagttcagccctcaagccatcgtcgccgtcgagcgcttggatgcccttagctatggcttgaacatcgtaaggatcaacaatcaccgctgcatcccctgcgacctccgaaagagcgccgcccgtcgaggtgagcacggccgtcgaaagagccatcgcttccagcacaggcagaccaaacccctcgtagagggacggaaacaacactgccttggcgccacggatcatgctgatcagcagagggaacgacatgtagtcgtactgaagaatgcggcctgcggcgggaacgccgtcccttttcacctgcgccagcagggccgtttccccctcgtctagccatgatcgccctcccaccaggaccaaggggcccgtcacgccggaagaaagataggcctccacgatgcggccaaggttcttcttcggctcgaccgcgccaaagtgcaggaaatactccttccaccccagattgaagacgcgctccagttccagtgcgacctcgtcttggctccgcgccagcaactccttgggaaaatcgacggcctgatatgtattcgtgacccggccttcgtcgacgccaagcaggcgcacgacgtcttggcgggtcgtttcagagaccaccacgatgtggtccgcccgcgcggccatctcgagactcaacgccatatagcgggatttatcgcccagggtcgtgtgcggcagacgcagagggatgaggtcgtgaaaggtgtatatgttcggacagcccctagcgtaaaccgggactagggacgtccagtgcatcacgtcaggaggaagcgcctcagccgcagccttgaacgtgaccggcgtcgcacttccgtagcgctgaaagcatcggttggcgcgcgcgaaaatatcctgggacatccaaaaaaggtcggccgcagggggtgtccccaacggccagatcacctcgcccgaaggggttatgggataggctgaccggccaaactgcgagagcaatgtctccccaaaacgcttgaccttgtcacgacgcgtggctttcggcgcgatgggtcgcgcgtctacaagcagcgcctcgttcagcacgttggaagccgcatgtttggctggcggcccgtagagaacttgcgtccccaagcccgaagccctcgcgacgtccagcagattcctgccataggtggcaatgccggatccctttggcatcgccaagttgaagccgtcgatgcagatcgatgccatcgatatcctgccatgagaggtcggccggccatggacgacacacggtcggcctggtcaaccccaagctatagattcaacagcgccggatccccaccctgcgcggcgatattgatgctcaccgccttttccgctgcatagcggatcaggctgttcgggccgcccgccttggggccggtgcccgacaggccctcgccgccgaatggctgaacacccacgaccgcgccggtgatcgagcggttgacgtagacgttgcccgcggggaccagcgacatgacctcgtcggcgaaggcctcgatgcggctgtgcacgcccagcgtcaggccgtagccgcgtgcggccagcttgcccgcgaccgtcttcagctctgacggatcatagcgatagacgtgcagcacgggtccgaacacctcgcgctccaagaagtccggggtcgggatttcggcgatggtgggggcgaacaggtcgcccttctccgagcccatcggcagggcggcgcgggcgacgatcttggcctcgcgcgacaggcgctcgacatgggcctccagcgcgcgccgcgattccggatcgatcaccgggccgatgtcggtcttcgggtcggcggggtcgcccaccgcctgcaccgccagggcgcccttcagcccctcgatcagggcgtcggcggaatccctgggcgcatagaggacgcgcaaggccgagcagcgctggccggccgagccgaaggccgacaggatcacgtcgtcgatgacctgctccttcagcgcggtggtgtcgatgaacatgccgttcaggccgccggtctcggcgatgaagggaatgatggcgcccggccgcgcggcgatcgagcggttgatggcggcggccgtgtcggtgccaccggtgaaggcgacgccgtcgacgccccgatgcgacaccagcgccgcgccgaccgtctcgccacggcccgggacaagggccagcagatccgggttcagccccgccttgtgatacaggcgcaccgcctcggcggcgaccagcggcgtctgctcggccggcttggccaggacggcgttgccggcggccagggccgcggcgatctggccggtgaagatggcgagcgggaagttccacggcgagatgcaggcgaagacgccgcgcccgtgcaggaacagctggttggtctcgccggtcggtcccttcagcgtctcagggcccgcgaagtcgcgctcggccagaagggcgtaatagcggcagaaatcggccgcctcgcgcacctcggccacgccgtcgttcagggtcttgcccgcctctcggctgagcagggcgaccagccggtccaggtcggcctccagcgcgtcggccatggcgcgcaaggtcacggcgcgcttggcgccgccctgacggtcccatttgacctgggcgttcgcggcggccacggcggcggcgtcgatgtcggccggctcggcttccgagacgtggcccagcacctgcgaccggtcgaaggggttggtcacggcctgagcgtcgacgccggcgcgcagcttgccgccgatgatcggacccgaggtcagcttctcgcggtccaccaactccagcgccttcgcatgccgctcgcggtcagcggcctgggaatagtcgcggccgagggagttctgacgatcgccgtacatgtctttcggaaccggaatcttggggtgacggtcgggcgcctgctcgaccagggagacgggatcggccgcgacggccgcggcgggcacgcgctcatccagcaaggcgtggacgaaggaggagttggcgccgttctccaacaggcgacgcaccagatagggcagcagctcctcgtggccgccgacgggcgcataggcccgcacgatcacggtctcgtcggaccatcgctcggcggcggcgtcgtacagggcctcgcccatgccgtgcaggcgctggtgctccaccgtgacgccgcggtcgcgcgccatgcggcgcacggcggccagggtgtgggcgttgtggctggcgaattgcgaatagatcgccggcgaggcctggatcatggcgcgggcgcagaccagatagttcaggtcggtcgccgccttggtcgtgaacactggatagtcggtgcggccgaacacctgggcgcgcttgatctcggtgtcccaataggcgcccttgaccaggcgcaccatcagccggcggcccgagcggcgggccaggtcggcgacccgctggatcgtctccagcccgcgcttctgataggcctgaaccgccagacccaggccggtccagccgcccagatcggcctcatgcgccagacggtccagaagcttcagcgacagggccagccggtcggcctcctcggcgtccatggtgaagttgatgtcgtgcttggccgcgatccgggccaggcgcagcacgcgcggatacagcgtggcccacacgccgtcctcctgtgtcgcctcatagcggggcgacagggccgacagcttcaccgagacgccgtgcccatgctccggcccctgccccgtggcggtccggcctaccgcctcgatggcgtcggcgtagatctgctcatagcggtcggcgtcggccagggtccgggcgccctcgcccagcatgtcgaaactgcacagccagccctcgcggttcgatcgcttcagcgccgcctggatggtgcggcccaccacgaactgctcgcccatgatcttgacggcggtggccaccgcctggcggatcacaggctcgcccagacgaccggcgatgcgtttcaggaagccgggcaggtcggtcctggcctcgtcgtccacatccaccagcttgccggtcagcatcaggccccaggtcgaggcgttgacgaacaggctgtcggactggcccaggtgcgaggcccagtcggccgagccgatcttctcggcgatcagccgatcccgcgtctcctcgtccggcacgcgcagcagggcctcggccaggcacatcagcgccaggccctcgcgggtgcctaggctgaactgctgcaggaagctctcgaccaccccctgcttcctctggctgcggcgggcgtgttcgaccaggtcgatcgcctcggccacgaccgcttcgcgttcgccggcgtccagcggcgtgagcgccagattgtcggcgacggccgcgcgttcgtcgcggaacttgtgatgatccaggccgtcccagacggccaggctcgacgggttgaaggcgggcgacgtcatcggcggacaaatcctgtggatttccggtatatgccggagttcattgaaggtgcttcgtatgataggctctgtcgccgaagatcgttcggcgtcgccacccgctttccgatgattgacatagactccgtggaccggcgcatcctgcgggtgctccagtccgacgcacgcgtctccaacgccgaactggcccggcgctgcaacctgtcgcccgccgcctgtttcgagcgggtccggcggctgcgcgcaaggaaggtcatcaccggctacgccgccctgatcgacccggcccaggtcggccgcgacctgctgatcttcgtggaggtcctcctggaccggaccaccggcgacgtcttcgaagccttcgcagaggcggtgcggcgccagcccgaggtgctggagtgccacatggtcgccggcggcttcgactatctgatcaaggcgcgcgtcggcgacatggacgcctatcgcgcctttctcggcgacgtgctggtgaagatgcccggcgtgcgggagacccgaacctatgcggtgttggaagaggtcaagtcgacgacggtgctgccgctctagcgatccacgcgcgctaaagagacacacacgaaggttgtggggtgacggcgacggcggccttccgtaagaacggctccaccgcaaagtccgtcgcgagcgatctgtccatgtcagtgatctttcccatcatcatgtgcggcggcgccggaacgcggctttggcccgcctctcgtccgtcgaggccgaaacaattcatacccctggccggcaatcggtcgctcttccaggaaaccgtcgatcgcgtggcgcccctggcgggagaggacggcgcgctcgtggtggtgggcggcgcggcgcatcacaggaccatcctcgaacagttggccgagatcggtcgaacggccgtcgtgctgcttgaacccgaagggcgcgattcggccgccgcgatggcggcggcggcgctttggactaagcagcgccgtgcagacgccgtgaatctgttcgtagcgtccgaccaccacatcccggatcagcaggcgttccgactggcggctgaggcggcctgcgcggccgccaccaagggtcggatcgtcacgctcggcgtcgtccccaccgcaccttcctccgcctatggctacatagaacccgcatcggccgggctggccgaggttcgcgccttcgtcgagaaaccggacgccaagacggcggcgcaatacatcgcgaacggctatctctggaatagcggcaacttcatcgttcgcgcggacgtgctcttcgatgagatcgaggttgcgaccgccggcctgagcgaagctgtctcggccgccttggaggacgccaccgtcgatgggccgtccatcttccttggcgaacgattctcgtccgcgcccaagatctcgatcgactacgctgtcatggagcgcacgcaacgggcgtccgtgctgcccgtggatttcgaatggtccgatctcggcgcctgggactcggtgcatgcttccggggaaggcgatgtcgggctgcacgtcttcgaggacagcgagggctgtctcgttcgcgcctgcgacggcgtgatggtcgccgcgatcggcctttccaacatcggcatcatcgtcgagcaggacgccgtgctggtgaccgacctgaagcgaagccaagacgtcaagaaggtcgtcgaacgcctgaagcagttgtcgccgcgccacctcgatttccagcagccaaaggaagaggacctggcggatggcgccgcacgcttcgccgcctggatgcggcagtcggccttgccgacctggtgcaccctaggccagaattcggccggcgggttcgaggagctgttgggacaggacggtcggcggctggattcggcgcgccgggcgcgcgtccaggcccgccagatccaggtttacgctgaagcggggcgcctggattggtcgggcccgtgggatacggcagtgcgggcgggcctggaatggctggacgcgaagttcctgaatccggacggtcaggtccgcacgcggctgtcgtccgatggcgcgcctttggacgagaccgtcaccctctacgaccaagccttctacatcttcgccctggcgtcggcgcatcgcctggcgccggaactcgcgagcgagagcacggcccgcgccgtccgcgatggattgctggcccaagcccctgcgcaaggcggcctggtcgaggccggcgcgcatccctatcagtccaacgcccacatgcatctgctcgaagcggccctggcctgggaagaggcgggcggcgacaagggctggagcgacctggcggaccggatcgtcacgctggccctcacccgcttcatcgatcccgagacgggcctgttgcgcgagttcttctctaaggactggtcccccgcccccgggctggacggcagcctgatcgagccgggacatcagttcgaatggtcatggcttctgacccggtatggccgcgcccgttccgacgccgcgagcctggaagcggcctggcggctgttcgagggcgggctgaaaggcgtcgacgccaagcgcggcgtggccgtggacgcatgcgacatcgccggcggcgttcgcagcgccagggcgcggctgtggccgcagaccgaatggctgaaggccgccatgatcctggctgcgaccaccgacgacgcccgaagggacctctgcctgacccaggccgcccgggcacagcgcgcgctgtggcgttatctgacgccgccgggtctatggcgcgacaagatgctggagaacggcaagttcatcgacgaaccggcgccggcgagttccttctatcacatcatggcggccttcgcgcaggtccagacctcgttgggagcgctgaagccgtccatgaagggcgcgctggagcttcgttgagatgaagacggcatgtctcgccttcgtcatccgaaccgtctagaagttccgcccttcgtccacggctcagggtccgcccgcctacatgcgcatcgttctggccaccgacgcctgggagccgcaggtcaacggcgtcgtccgcaccctgacccgcacggtcgcggaatgccgcgccatgggccatgaggtcgaggtcatcgagcccagcctgttcaagactatcccctgtccgacctatccggaaattcggctggcgctgggggcggaagaagagatccgcgagatgctgcgcgccttcgagccggaggcggtgcatatctcgaccgagggtcccatcggcatcgccacgcgccgcatctgcgtggaatggaagctgcccttcaccaccagctaccacaccaagttcccggaatatgtgtcggcgcgattcccgatcccggtgcaggtcggctacgcctatatgaagtggttccacaagccgtccggtcggctgatggtggccacgcccaccctgcgtgacgagcttcaggaacacggcttcaagaatgtctcgccctggtcgcgcggcgttgataccgagcagttcaatcccgacctgccgcgcatctatgaagagctcggcggcgccgattggccacgccccttcttcctgaacgtcggacgggtcgccgtcgaaaagaacatcgaggccttcctccagctggaccttccgggcaccaagatcgtcgtcggggacgggcccgcccgcgccgagcttcaggagaagtatccggaggcgaagttcctcggcgcccggttcggcgaagacctggcccgctgcttccgcgacgccgatgtcttcgtcttccccagctggacggacacctttggcctggtgatcctggaggccatggcgactggcacccccgtcgccgcctaccccgcccacggcccaatcgacatcatccccggatcgaacgccggcgccatcgacgacgacttgcgcacggcctgcctgcagtgcctcgaactcgatcgcaaacaggtccgcgcctacgccgaaaagttcagctggcgcgcctccgccgaacagttcgtcgagaacctccagccctaccccgaacccgaacgcggccgcttctggcgccgcctccgccgcatcgcccgcgtccgcaagcgcgcggcggcttaagctctcactccaccgtcaccgacttcgccaagttcctcggctgatccacgtccgtgcccttctggacggcggtgtagtaggccaacaactgcacgggcacggcgtagaccagcggcgcgatcaacgggtggcagttcggggcgtcgatgcggcggatgcccgcgccatgcggggctggggcggcttcgggggcgatcatgatgacggggccgccgcgggcggagacttcctgcaggttggaggcggtcttttcgaacacgtcgtccagtggcgcgagcgcaaccgtcggcgtttcctcgtcgatcagggcgatcgggccgtgcttcaactcgccggcggcgtagccctcggcgtggatgtagctgatctccttcagcttcaacgcgccctccatggccagcgggaacatggccccgcgtcccaggaacagcacgtcgtcggccttggccagatcatgggcgacggccttgatgctgttgtccatccgcagagcttcagcgatcaggcgcgggctctcgaacagcgccttgaccagttcggcttccttgtccgcatcaacacggccgcgctgaacgccggcggcgacggccagcgccagcagcgccgcgacctgggcggtgaaggccttggtggaggccacgccgatctccggccccgcatgcgtcggccacagcacctcggcctcgcgcgccatcgacgaggaatggacgttgaccaccgccgccgtgcgcaatccctggcgcttgcaccacgtcaggccggccagggtgtcggcggtctcgcccgactggctgacggcgatcgccagggtgctcttgctcagagccggcgatcggtagcggaactccgacgcgatctcgacgtcgcacggcaggccggcgatgcgctcaaacgcatagcggccgatctggccggcgtagaaggcggtgccgcaggcgatgatctggatgcgatcgacagcggcgaagtcgatcgccccggtcttggccttgccggtcaccaggtcgagatattccgacagggtgtgctggacgctgtcgggctgttcgtggatctccttttccatgaagtggcggtattcgcccttctcgaccatggccgaggaggccgagacctgaaccaccgcccgctcgacgggcgcgccgctcgcatcgaacatgcgcgcgccagaacggtcgacggcgacataatcgccctcctccagataggagatcttctgggtgaagggaccgacggccagggcgtccgagcccaggtacatctcgccctcgccccagccgaccaccagagggctgccgcgccgggcgcccaggatcaggccatcctcaccctcgatcagcaccgccagcgcataggcgccggtcagccggtccaaggtcgccttgaaggcgtcgagcggcgccaggccttccgacagcgtctgatccagcagatgggccaccacctcggtgtcagtctggctttcgaacacatggccctgagccgtcagttcggctttcagctcggcgaagttctcgatgatgccgttgtggaccaaggtcacgcgcccggcctggtgcgggtgggcgttgggcacgttcggcgccccgtgggtcgcccagcgggtgtgtccaatgccgacggtggccttcagcggctcatcggcgagcacctcttccagcgcgcggatcttgcccttggctctgcggcgctcgatccggccgtcgaccacggcggcgacgccggcggaatcatagccccggtattccagccgcttcagactgtcgagcaggcgcggaacgacctggccctcgccggtgacgccgatgatgccgcacatggggttcgctcctgcaaggacctgaggtgaaaaggccggctttgcagcggcggcgggatcggactatgccgtcggcatcatgcccggactttcggataggcgatcttaagcccgatcgcatctgaatccgggtttcggaaggtttcctcgaaagcgggacggcatcttgagccagagaaaatacttcggcaccgacggcatccggggacgggccaacacccatcctatgacagccgaggtcgccctacgggtgggcctggccgccggcaagctgttccgcacggaggcggatcgtcgccatctggtggtgatcggcaaggacacgcgtctgtccggctacactatcgagccggcgctggtggcgggtttcgcctcggtcggcatggacgtgcgcacctttgggcccgtgcccacgccgggcgtggccatgctgacgcgctcgatgcgggcggacctgggggtgatgatctcggcctcgcacaacaactatgcggacaacggcatcaagctgttcggcccggacggctacaagctctcggacgagatcgagctgaagatcgaggcgatgatggacgagggactgggtgagggcttggcggccgccggcaagcttggccgcgtcaagcgcatcgacgacgcccagggccgctatatcgagatcgccaaacaggccttccccaagcgccttagcctgaagggtctgcgcgtctgcatcgattgcgccaacggcgccggataccgcgttgcgcccaccaccctgttcgaattgggcgcagaggtgtgcgcggtgggcgtggagcccaacggcgtcaacatcaacgcggattgcggctcgacccacccggcgacactggcggaggcggtgaagcgctaccgcgccgacatcggcatcgcgctggacggcgacgccgaccggctgatcgtctgcgacgaaaagggccaggtggtggatggcgaccagatcatggccctggtcggtctggactgggcgagacgcggcctgctgaccggcggcggcgtggtggcgaccgtgatgtcgaacctcggtctcgagcgtcggttggaggccgggggcctgacgctgcagcgcaccaaggtgggcgaccgctatgtgatggagcggatgcgcgagggcggcttcaacgtcgggggcgaacaatcgggccacatcatcctgcacgacttcgccacgaccggcgacggcctgatggcggcgctgcaggtgctggcggttctggttgaatccggaaagccgatgagcgagctggcgcgccagttcgatcccgtgccccagcggctggagaacgtgcgcttcacctcgtcggcgccgctcgagaccgccggcgtcagggcggccatcgccgaggccgaaggcgcactgaacggctcgggccggctgctggtgcgcccgtcaggcacggaaaagctgatccgcgtgatggccgaaggcgacgacgaatccttggtcaggcgggtggtgagcgacgtctccgcagcggtgcgcgcggccggctagagggcgcggttgcgctccacgatgttgccgacggcgttgtccccgtcgtcggcgctggagccgaacggccagccggcgtccgcccggcaatagggccgccgtccctcccgcgagcccaccacgaccagccgaggcctgaaccacgcggcgccgcgaaagacgttgtcggtgatccggttccacgacggcgtctggtggcggatgaccccgtcctcgccgcagttgcgataaagaaagacgccgccctgcccctgcaggttgaagcgattgccgactatgcggttggcgcccgatccgtccacggcgatcacctcccgcccggttcggacccggaactcgttgttctcgatcaccgcattggcgctttcggcgtccagatagaccgccgtcgataccgagcgcccggcgaaggtcgagttgcggacggtcgtccttgtcacgcccggcccgacatagagcgggatcgatccgccggcttcgatccgcaccgcatcaagcgtcacgccgcggggcgccgccgcctgcgccgcgcgggtgaagcccgcccgccgggatgcgtcgcgcaggtcgctcatagacccgcccgcgcccatgccccatatccgcacattgccgaggatgacgcagcggcgaaggacaacgctcttgggcgcgctccagccatccccctccggacgtgaccagatcgccacggtaggcagccgggtcgtgccgggtcgatccgacatcccgatccggccgcctttacagtccagagcggcgccggaagcttctgcgccttcgatgagcaccggccgctgcacatgagcgcgggcgttaagcaccgcacggcaggccagccgatagggcgtcgacgagggcgcgagcaggtccgcgacctcggctgcggtgcagtctcgcgcggcaggcggcgtcaacgccagggcgagggccagtccgatcacagcgcaggctcgctcaacgccagccgctcggcggcgcagcccggatgcgtcaggcctgaccgccgcagcgcctgcacctcacgccgcaggtcgggcaggtcggactgaaacgccgccgtcgccacgatctccaggcccagccggcgccccagccgctcgccttgcataacctcatccggcgccgcgacgccgcagatcgcctgactgaccccgatctcgtgcccgacgcgccggatcgccggcgccgcatcaggcgcggccgccgccaggagttcggcataggcggcgcccaccagggtctcgcgcggagggcgggagcgggtctcgccggtgtccatcgtgcggcgtctgcaggcgcgcccatcggcggcggcggtcgccggcgccgcagccttcaggcggtcggcgacctgtcctgcgtcgccgaaagcacgggacagcgctctctccagcgactgcgtctgtcccgaggttgagcgcacgccaagggcgcagtcgaagtgttgaagggcatagcgcggccgcagctcggcgtgggccgtcgccagcaaccagcggtccccgccctcgaccacgtcgggcatccggcgcgccgggtcctgcggcaccatgtcgccggccagcacgtccgcccgggatacggcgaggtagccggtctcccttgatgactccggcacggcggcgcaccccgccaatgtggcgaatgcgcaggcgatgacgagaagagagcttaccggccggcgttccatgtcaactgaaccgaggtgcggtccgtctctccgggagaggcgacgacctgcagactggcgccgttcggctgggcgccggacgcgccgtaggcccgcgcgtcgccctggttcatgcccataaccgaggtcaggcccgcggcctccgcatgctggcgatagaaggcgaccaccgcatccggctcggcgtcggtgtcgaaggtgacaagcccgccctcgccatcaggcccgaccgccgtggtcgccggctcttccaccaccgcgtccggatagagcaccgcaaaggccggcgcatcgggcgcagctagggaaagctgcgcgctcgttccctgaagggcaggcgccgcggccgccgatcccgctggtccggcagacgccggcgcaggccccggatccgccggggcgtgttccgccgcgggatcgcatgcggccagtcccaacgtggaaaaggcggcaagcgccgcccagtggcgaatcatcgaaatgtgcgtccctgaacccgagaggtcttaggtttcaccgtggcgcctcgctgtggcgcccgcaaggcggtcagcccgaggcggcgtccgcatcgtctccgcgcccgccttccgccggatcgccggcgggaccggtgaaaccgtcgccggcattcttgatgggatcggggtcggcgttggaaggcgactcgggatcggccgacgccatgccttccgtcgccaacgtttcattgatggcgtcctgatccggatccgcttcggaccctgacgccacgccgccgcgcagcgagcctgcacgcgtgtccgagcccatgtccgttccgctcaaggcctcggacagagtgtcggcctgatgacccagatccggcttctcgcccatgtcagcggcttcagtggcgtcgcagttctcgggtgcggaatcagtcatcgggcgctccttggatgtcgcctcatcaaagcgcaggcgttgtgaccggttccccttgatcggcgggatcggcccccgatctagcagtcatgatcccattctccgttcttgacctgtcgcccgtcgtcgaaggcggcgatctccgtcgcgcgatggacgagacgctggccttcgcccaggccgccgaccgtctcggctaccagcggttctggctggccgagcaccacaacatgccgggcatcgccagcgccgccacctcgatcgtcatcgggcatgtggccgcaggcacacaacgcattcgcgtcggctcgggcggggtgatgctgcccaaccatgcgccgctggtgatcgccgagcagttcggcacgctggagacgctgcacccgggccgcattgacctgggtcttggtcgggcgcccggaaccgacggggccacagcacgcgccctgcggcgctatttcgaggccgcggaccagttccctcgcgacgtggccgagctgatccactatttcgagccggcgatcaagaatcaggcagtgcgcgccgtaccgggcgccggtttgcacgtgccgatctggctcctgggctccagcctgttcagcgcacagctggccgggcaaatgggcctgccctatgccttcgccagccatttcgctcccgagatgctgaaggaggcgctggccatctaccggcgcgagttccgtgcgtcggagcggctggacaggccgtacgcgatggccgccatcaacgtcttcgccgccgacaccgacgaggagggtagacgcctgtccacctccatgcagcagagcttcgcccgcctgcaacgcggccgccccggcctgctgcctccgccggtcgacgacatcggagcggtgctctcgccgggtgaactcatgggcgcccagagccgcctgctctactccgcggtcggcggccccgagaccgtccgcgatcagatccggtcgtttatcgacatgaccaaggtggacgaattgatgatcacgggcatgatgcacgacaatcgggcccgcatccgcagcctggagatcgtggcgcgggtgcgggaggcgctctgagcgtcttgacatggaagcttatagtgacgcccttcccgctaccagctaggtaagggttcatgacgaacttctaccctgtgatcatgtgcggcggagctggaacccgactttggccggcctcccgtccatcccggcctaagcagtttctgcccttgtccggcaatcgatcgcttttccaggaaactgcattgcgggtcgcgccgctcgtcagcggagatgccgtgatgctcgtcatcggaggcgtttcgcaccgcgacttcatcctgaaccagcttgaggaaatcagcctcgctgctcaggtgattctcgaacccgaagcgcgagactcagccgcagcgatggccgcggcggccgcttggacggcgcgagaagacccttcgggagtgaacgtctttgtggcttcggatcaccacataccggatgcggaagccttccagtccgcggtgcgccgagcaggttcagccgcagttgaggggagaatcgtcacccttggcgttaaaccgcgatcgccgacatcggcctatggctacatcgcaccctctggcgcgggcctctccaacgtgaaggcttttgtcgaaaaaccggatgcggagaccgcacgccactacgtggaagaaggctatctttggaacagcggcaactttgtcgtttccgcgaagacgatgcttaaagagttacgcagctcagcctcagccgtggaggcggcggttcaggccgccttgccgacccaaacagggcgcgcggttgcaacgctcggtgcgtctttcaggtcagccccgaagatttccatcgactatgctgttatggagaagaccaagctcgcgtccgttctgcctgtcgacttcgactggtcggatttgggagcatgggactctgtagcggcgactggcgaaggcgatgtcggaacccacgtgttcgaagatgcggaaaattgtctcgtccgcgcaccagatggcgtcatggtcgcagcagttggcgtacggaacctggctgtggttatcgaagacgatgctgttcttgtttgcgatcttgctcgaagccaggacgtcaaaaaggttgttgagcggctaaaggttacgtctcctcagcaccttgatttcgccgccgccgcagcagaaagcctgcccgatagtgcgcgacgaatggcgcattggctacgacaagcagcgctcccgctttggggcacgttgggccaagatgaggatggcggctttcgtgagctgatcggcttcgacggactgccggtggcctccgtgcgtcgcgcccgagtgcagccgcggcagattcacgtgttcagcgaagccggtcgactcgggtggcgcggcccttggaagcgggcggtcgcgctgggtctccaacgcttgaacgaaggctatgttcgtgatgacggtcgcctacgcgccaccctctccgaggaggggcagcctctggatgatcgtgcgaaaatctacgatcaggcttttcttctcttcgcgctcgctgcgtgtgcggacatggaagcttgcgaacagcgcgccattgacctgcgtgataagctgctgagcgaagtcgacgccgtcggcggtttcatcgagcaggacgagcgtccctatcaatccaatccacacatgcatttgctggaagcctgcttggcttgggaggcggctggcgccgatgagggttgggctttgctggccgaccgtctggtcgacctagcgagccgatgcttcatcgatgctgatggcggctttgttagagagttcttcgacgcgaactggtcgccggccgaaggcgacgatgggagcttggcggagcccgggcatcagttcgagtgggcatggttgctggcccgttacgcatccgcccgccaagatgacgctgcgatgcacatggcgcggcgcctttatgactttggattgaagggcgtcgagccgcgtcgccaagtagccgttgacgctctcaacgctgacggttccattcgcagcttacgcgcacgcctctggccgcaaacggagtggttaaaggccgccctcattctcgccgaacatgccgaggatggagagcgcgcccgttacctgcgggacgcggctcgcgcccaacgtgcgacttggctctacctgacgcctgaaggcttgtggcacgacaagtgcttggccaacggcgagttcatcgatgagcctgctccggcaagttccttctaccacatcatgggcgccttctctcagctgagaagctccttgccggtattgtaccccaacgatcagcttgatcttcgccttggctgaggccgatcagcgccgccacgcattgatgaccgtatgacccgcctcgtcaccttctccgacggcaccaccgtcccggttctcggccagggcacctgggagatcggggatgatccggcatggcgggacgaggagcaggcggcgctgtctcgcgggatcgacctggggctgacggtgatcgacaccgccgagctgtacggcgacggtcggtcggagcggctggtgggcgaggtgatcgcaggccggcgggacgaggtctttctggtctcgaaggtgcggccggagaacgcctccgagatgaagatgatgctggcttgcgagaagtcgctggagcggctgggcgtggaccgaatcgatctctacctgttgcattgggaaggccgcgttccgctggaggagacggtggacgcctttcaggagctggtggatgagggcatgatcgcgcgctggggcgtgtccaacctggatcttcgcgccatggagcggctggtcgatattgacggcggcgccgactgcgcggccaaccagctactgtacaatctcggttcgcgcggggtggagttcgacctgctgccgtggatgcaggcgcgcgacatgccgatgatggcttattcgccgcttgggcgcggggggctgctcgagcatccgctgatcaccgacatcgccgatcgccatgacgcctcgccggcgcaggtggcgcttgcggccgtgctgcgtcaggacggggtgatcgccattcccaaggccagcacggtcgagcacgtcgaggccaacgccgaggcgctggaaatccgcttcgacgccgaggacctggacaggctggaccgcgtcttttcaccgccgaccaaggcgacgccgctggacatcatctgaattggaaaaggccgggatcgctcccggcctttttgcttacgcagtcggaccttgctcaggccgccgccttggtctccggcgcgaagcggccgtagaaggtctcgttcttcgccgccatgtcgcgcagcagctgcgggaccttgaagcggtcgccgtaggtctccgccagacgatccgccgtctcgacgaacttggccaagccgatgccgtcgatgaagctcgccggaccgccggtccatggggcgaagccccagcccaagatggctccgaggtcggcctcgcgcgggtcgtcgatcacaccctcttcccagcaccgcgccacttccacagcctggcgatacagcaggcgggtcttcagctcgtcaatctgggcaaaggccgaggcgccttccggctggtcgatgcccttggtgatcggggccagttccccaagacccgcccagagcgtcttgggcttctgatcgtagtcgtagaagcccttgccgttcttgcggccgaaccgtccgccctcgaccatggtggcgacgatctgctcgccctcgttggggacgtacttgtcgccgaggtcttcgcgcgtctgtttggcgatcttgtaggacaggtccagcgccacgtcgtcgtgcatctccagcgggccgcgcggcatgccggtcatgcggccgacgttgtcgatcagcgcagggccgtagccttcctccagcatcgccatgccttccatcaggaaggtcgagaagcagcgcgaggtgtagaagccgcgactgtcgttgaccacgatcggcgtctttttgatcttcaggacgtaatcgatcgccttggccagagcggcgtcacccgtcttttcgcccatgatgatctcgaccagcatcatcttgtcgaccggcgagaagaagtgaatgccgatgaagtccgccggccgcacgctggcctcggccaggccggtgatcggcagggtcgaggtgttggagccgaacacggcgccgtccgccagctgcgcctcggcgcgcttggtcacgtcggccttgatctcgcggctttcgaacaccgcctcgaccaccaggtccgagcccttgatcaggtcgtagtcggtggtggcggtgaccagggccagggtcgcgtcgtgcttgtcctgggtcatctggccgcgcgacaggcgcttcttcagcaggtcggcgacatgctgcttgcccttgtcggcggcttcctgcgtctggtcgatcagcaccgtctcgataccggccatgacctgcacataggcgatgcctgcgcccatcatgccagcgcccagcaccgcgaccttcttgggatcggacttctcgacgccggccgggcgcaccgcgcccttgtccagctcctgcttggacaggaacagcgagcggatcatggcctgcgcctgcggcgtcatcagcgtcttgatgaagtagcgcgtctcgatccggaggccggcgtcgatcggcacctgaaggccttcatagaccgccttcatcaggttcagcacggccggatagttgccgtaggactgcttgcgcagcatggcgttgccgaccatgaagttctggatgccgaccggatggtaggggccgccgcccggcagcttgaacgacttgtcgtcccagggctgctgggccttgccgccattcctgatccaggtcttggccgcctcgaccgcctgacccttttccaccacctcgtgcaccacgcccgcgcccttcgcgtcgttcgggcgccacgacttgccttcgctcatctgcatcagcgcggcctgcacgccgatcaggcgcgtcaaacgttgggtgccgccgccgccggggaacaggccgaccttgatctcgggcaggccgagttgaatcttgttgtcgttttcgaccacgcgatagtgacaggccagcgtcagctccagtccgccgcccagcgccaggccgttaatggccgccgcgaccggtttgccgcaggtttccagcgcccgcagcgcgccgttcagcttccatcccgcatcaaacgcggcctgcaggtcgcccgcgcccgacagcatgcccgaggccatgtcgccgagatcggcgccggcgcagaagccgctcggcttgccactggtcagcaccgcgcctttgatggcttcgtccgacttgatgcgttcgacgacctgcgggatctcggccatgacctggccggtcagggtgttcatcgaacggccggccacgtcgaaggtgacaagggcgatgccgtcggcgtcgacgtcgatcttgaagttttccatgatgatgatctccgaaatcagacgcgttcgatgacggtggcggtgcccatgccgccgccgatgcacagggtcaccagcgcggtcgacttgtccgagcgctccagctcgtccagcaccaccgaggtgatcatggcgccggtggcgcccagcgggtgacccatggcgatggcgccgccgcagacgttgatcttgtcgtgcgggatgtccatcgcctgcatgtagcgcagcaccaccgccgcgaaggcctcgttcagctcccacagatcgatgtcggcggtggtcatgccgaggcggttcaacaatttgcgcgacacatactcgggcccggtcagcatgatcgacggctctgaaccaatggaggccgcacccttgatccgcgcccgcggcttcagccccagcgcctgcccggcttccagcgagccgatcagcacgccggccgccccgtcgacgatgccggacgagttgccgggcgtatggacgtgcttgacccgctccacctctgggtagcgctggttgatcacggcatcgaacgccatctcgcccatcatggcgaaggacgggttcaggccgcccagcgtctgcatgtccgtgttcggacgaatggtctcgtcgtggtcgaggcgcaccagaccaagctggtccttgaccggcaccaccgacttgctgaaccggccctcggcccacgacttggccgaacgcttatggctttcgacggcgtaggcgtccacgtcgtcgcggctgaacccgtatttggtggcgatcatgtcggccgacacgccctgcggcacgaagtaggtcggaaaggccgaggacgggtccgtcggccaggcgcccatgtccgagcccatgggcacgcggctcatcacctcgacgccgccgccgacggcgaagtccgcctcgccggccttcacctttgccgcggccatgttcacagcctccaggccggaggcgcagaagcggttgatctgcacgcccgccgtttcctgcgaccagccggccgccagcaccgcggtgcgcgcgatgtcggcgccgagttcgcccaccggcgtcacgcagcccagcaccacatcgtcgaccttgcccgtgtccagagcgttgcggtcgcgcagcgcctccagcacctggctcgccagcgacaggccggtgatctcgtgcagagagccgtccttcttgcccttgccgcgcggcgtgcggacggcgtcgtagatgtaggcgtcagccatggtgcgtctttccttgtctgcctccgcctcgccgcacggcaagaaggagggtccggagtcgaaacctggccgccaagaaccctacgtttacgtcaacgtcaagtaagaaggcgcgtgatcggatgcgccgcctgatcagcgatccgtcaggcggctggctccgccggtgatgcggcacacatagtcgcgcgccggattggcggactgcgaacccgtcggctgcagaataccgtcgcgagcgcggcagtccgcgtcgagcctgtccagttcggcctgatagcgaccggtcccgccggtgcttgcgcagcccgcaagcaggaccagaccggccaacgcggcggaactgagtgcggacttcttcatgacgacctccatcgatcctgcgaaacgcgggggacgcccggacgatccgcagtcaagaggcgaccgacagtcgaaccagcttgccgtcgtcctcgtcggtgatgacccacacggcgccgtcgggcgccacggccacatcgcgaacgcgctcgccaagatcggtgagcagccgctcttcacccacgactcgatcgttctctatcaccagccgcgccaactgcttgtcccgcaggcccgccaccagcaggtcgccgtcccagccggggaacatggcgccctgatagaagacggcgccgcccggcgcgatcaccggatcccagtaatagaccggctgctccgtgccctcgcgcgcggtgacccagggaccgggctggccattgtactcgatgccgtacgatacctcgggccagccatagttggcgccgggcttctccaggttgatttcgtcgccgccgcgcgtgccgtgctcgatggtccagaccgcgccgttcggctgcaccgccacgccctgcacattgcggtggccatagctgaagatctccggccgcgcgccgtcgcgcccgacgaacggattgtcctgagggatggttccatccgcattgatgcggatggtcttgcccatgtgggagttcaggtcctgcgcctgcggccgcatcggcttgtccgaacgctcgcccagggtgatgaacagatgaccttgttgatcgaacgccagcgacgagccgaaatgcttgtcgccgtcataggtcggctgcgcgcggaagatcacctgaacgctttcgacgcgcgcgccgtcgtccgacagccgcccgcgcgccaccgaggtggcgttgccgccctcgcgtggttcggcatagctccagtagatcatgcggtcacgggcgaaatccgggctgatcgcaacgtccagcaaaccgccttggccgcgcgcatcgacgcgcggcaggccctgcaccggctcgctgatccgcccctcgcccgtgacgatccgcagccgaccccgcttttccgtcaccagccagcggccgtccggcatcatcgccaggccccacgggtgctccaggcccgaggcgaccacccggtacatcagcgcctggtcggtgcgcaccgccggcgcccgggtttgcccctcaaaggcgggccgctgatccggcgcattcgccgcccgcgtctcaagcgccgcgccacgcggcgcggcggcgtcggactggccgggcgcctctccgctcgccccgcaggcggcggccagaacgatcagcgaagtcgaagcggcggcggcgatcaggcgcatggcgaggttcccgatgagcacgttcggccaacaacgagcacaagcacgacggtgttccaagtcccaagcgtcgcgcgcaaacgccgcagccgctaggatcgccgccgatgctcaccacccgcttcgccccctcgccgaccggccggctgcacaagggtcacgccttttcggccctgaccgcccggcgcgcggcgcgcgcgagcggcggacgcttcctgctgcgcatcgaggacatcgacccgacccgctgtcggcccgagtacgaagccgccattcttgaggacctgcgttggctgggtctcgacggggatggcccggtccgccgccaatccgagcatctcgacgactacgcccacgccctgtcccaccttgaggcgcgcggcctgctctatcgctgctttcgcacccgcaaggagatactcgacacgatcggcgacgcgccgcacggaagggtggaggccgttcgtccgggtccgcacgccgccgacgaggagacccgcctgctgggagaaggccgccccttcgcttggcggctgtcgcttgagcgcgcccgcgccgttatcggcgaggacgcctggcgcgacttgtcctttatcgaagagggcgcaggaccgaatggagagaccggccgcatccccgcccggccggagaccgccggcgacgtcgtgctgggccgcaaggacaccggggtcgcctaccatcttgcggtcacgcatgacgacgccctgcaaggcgtcaccgatgtcgtccgcggccgcgacctgttcgaggccacgcacatccagcgccttatccagaccctgatgggctggcccgcgccgcgataccgccaccacgccttgctcaccgacacagccggccgccgctacgccaagcgcgaccgctccgtgacgctggccgagctgcgcgcgggcggcatgagcgcggccgatctcagagccgaactgggcttcagctcctgcggctgaacacgcgcgaggcgccgtagccggtcagggcggcgaggaggacgcaaagcacgccgtaggtccagggctggcggtgggcgaagtcgtagatgtcgcgctccagccccaccttctcgacggtcagggtcaggttggagaccgacgccggctcgccgtcctggaacagccagacctcggcgtgatagcggccgaccggcgccacggccggcagttcgacctcggcgcggaacaggccgcgatcgacgaaactgacgccctcgggatcggtgttgtagagggcggccgcctcgcgcaggcggatcacggcgcgacgccactcgaggtagtcctcgcccaggcggctgaccaccacgtcgcgaacgccgtagcgggtgacggtgcgactttcctccggcgcctggatgcgcaggtgatcgacgccgacgcccaggcggcggagctggccgaagtcggcgatgtccgacaggggccgcgtcgaggccgtcatgtagaatccgggcgccccttcgaacagcaccggccggctgttcagccacacgcccagggtgcggacctttcgaacaaggcgcaccggcgcgtcgggcccgcgcaccaccaccaccacgtccgccggtcggtcgctcgggttgaacaccgctccgtagagaacgatcgaagcgccacggaaaccggagtccacatgcacgcgcgcctcagtgagggcggcggccacgcgcaggtccctggtggtggcgaccgagcgctcgggcggcggcgcctcgacaaccgggggcggcaaggcctgcatcatcagtccgacacccccggcgcgaacaggaacacgtccgacggctccacgaacaggccgaggcccatctgcagtccgaccagcagcacgatcaggcccagcagggcgcgcagttcctcgccccggaaccggcccgagaagcgtgcgcccgcctgcgcgcccaccacgccgcccaggagcagaatggtggccagcacgatgtccacggtctggttgcggccggcctggagcacggtggttatggcggtggtgatgatgatctggaacaggctggtgcccaccaccacgcccgcacgcatgcgcagcacatagagcatggccggcaccaggatgaagcccccgcccacccccatgatggcggacagcacgcccgccaacacgcccaggccgaacggcggaatggcgctgatgtagaggcccgagcgaggaaacttcatccgcaggggcaggccatacagccacaaggggcggcgacgctccttgcgcggcgcggtgattccgcgtcgcctgcggatgatctccgtcaggctttcgcgcagcatcagcgaaccgatcacgcccaggaacagcagataggagatcgccaccaccaggtcagcctgacccagcaggcgcagatagcggaacagctccacgcccaagagagcgcccgtcgcgccgcccgcggccatgacgccgccgatccggtagtccaccgcgccctggcccgaatagcggatcacgccggaggtggaggaggcgaccacgtggctggcctggctggccaccgccaccgtgggcgggatgccgaagaagaccaggatcggcgccatcaggaagccgccgccgatgccgaacagcccggacacgaagccgaccaccgcccccaggatcaccaggagcggccagttcaccgaaacctcggcgatcggcaggtagatatccaaagcgcgcgccttcggctggagcggaagcgaacaccgccgaacggcgaacggaccctgtctagcggtccgagcgccgccccgccacccgccgccgtgcgatcagccggcggcgtccgcggcctggaaactgtcggcggcccggcgcgcgatctggcgcgcggcgggactggcggaagcgttcagccggtcataggccgcgcgcgcctcggcgtcgccggagcgagccgcgatggcgtaccaggtcaacgcctggctggtgttcggagccaacccctgcgcgccgttctcgtaaagacgggcgacgttgtactggctgtcggtgagaccgcgctcggcggcgcgcgtcagccacttcagcgcctccgcccggttctgcccgccacccacgccgtcgtacagatacatggcgtaggcgtgcatgcccttgggatcgccgccctcggccgcgcggcgcgcccagcgccgactctcggccagatcgacgtccacgccgcgctctccggcctggtagaggccggccagatgcagttgcgccgaggtgtcgcccaggttcgccgcggcccgcagcgtctcgacgccagccggatcatcggcgtccaactgctcaacggcgcgcgcataaacctcggcgccgcgacccgcgttcgctggagaaactgcgcccgtcggcgtcagagccacggccgcaagcggagccgccgcgttcgccgacggtccgtcgcccggtcgagacaggccgaagctcaagccattgtcctccgccaggccgttcagcccgaacaggcccccggtcaccgccaccgccgtcaccgacgccagcaaggccttcttggcggttgatccatcctgcgccgcctgcttatccagccgctcctgcagcttggacttgccgccgcgccggaggttcaggccgaagcccttgcgggcgggcggctccgcgaccgccggcgtcatggcggcgcgggcggcgtcgatggtggtgcggggggaggcggcgcggccttcggcggcggcggcgctcatgctggcgcgaagacgacggggatccacgaagtcggtgtcggccgagaagtcgtcctcgacatcgtcgagggtctgaacggcgggtcgggcttcggaccgggcgggtgcgaggggggcggcttgcgcctcggccgtggcgtcaagcgcgtcggaaacatcggccccgccgaaagaggcgaagcttgttgcgccgaagggtccggcgggggtcggcgccgcgtcctgatcgagctcgggcgccggctcggcctcggcgtgcagatcgccccagtcgtcgtcggcgtcaaacgaggcgtcgggaaaggcggcggcgcgccagtcggcctgggccgtgtcgggcgccgtctcaggggagaggtcttcggcctcgagcggcatgtcccggacagcgacgggagcggcggcggcgaccggagccgcagcggctgtcggcgtcggcgcccgctgatcgatgctttcgcgggcttcggccagaaggcgggcggtgcgctcctcgctcagccgcatgcgctcggccagttcgcccgaggcgcgatcgtagcgctgctcgatccgggtggagctttcggccaggcgctgaccgatgtcgtccagcgcctgctgcgagcgacgctcggtctgggcgatgcgctccgacagccgttcggagatgcgagtgatctcgtcgcccaaccgctccagggcgacagcgtggcgatcgtcggcagccgtcaagcgctgctcgattcgctcggcctggcgcgtgaactggccatcaatgtgggcggacttgccggcgaagtccgcctcagccttggcgaggcgacaagctatgtcggcttcgatccgcgacgacagctgcgcggtcttgtgggccaggtcgccatcgaccttttcagccagggcgcgagccatggcctccatctgggtcgcgggcgaggcgccttccgctcgggtcagccgatcgcccagattctgggcgatgcgcaccacctcgcgccccatggcctcgatgccttcggcagacttcgcttcggacgcccggacctgttcgccgaccgacgacagcgtccgctcgatgcggtccatccggtcctcggcctttgtgtcctccagccggcgcatcatctcgacgcgattgctttcaacttggcgcgccagggtctcggccagcttttcgaagcgaagcgcctcgcgcgcgccctccggctcgatccgagcctcggccgcatgcaggcgcttgtccagatcggcgaacgagcgttccaggttccgcaaggcgtcggtggtgcggccctgggcctgatccagccgctggccgacctgggccagcgcgtcggcgctcagcatccccgccggggcgcgggcggcggccttctccaccgcctccatccgcgtgcgcagctcgttcactccgccgcgctgccgttcctcgatctcgtacaaacgaccggccagagcgccgatggaggtctcgatcttgccgaagctttccagcgtgcggggaccgtgctcctgctcgaacttgcgcaggcgcttctggccctcgcgcacttcttcggcgagttcgtcggcgcgaagggcctgggccttgccggccttgtcctgggcctccagccggcgcagcagtccggccacggcctgatccacgccctggatcgccacggtggaccggcgctcagccgcctcgagccgcgaggcaatcgcatcgaccgaggcgcctagtcgcagccagtgctcgtcggaactgtcgtaggcgtcgtccagccgacgcgagcggcctcggcgctcgaacacctcggcgacatgggggcggcgcggcagggtggcgtaggcctcgtcttcctcgccgtcctccatgatcatggagttcagccactcgcccaaggtcatgcccgagcgccgcgccagatccttggcgatctcgcgggccttagggtcaatgccctttacgctccaaggcgccgccgctgcgctcactgattcgcctcccgacccattcagcgaacgctaaccgcccagatgctgggtgtaaacgcgccgttaaccgcaatatctggaggcggcctgtcgcgtctgtggacagcctctcccgaacgcagggttgtgacgcccacatggttaatgcgggatgaagattaacctgctggaaagactcgagctcttgccgaacggcgcatcctcggccacgcctgcggcgatgactctctcgacgacgctgatcctgctcgccgcatcgctggggctgacgctgctggccggatggcggggcgcgaggccgcccgatccgcgcaagggaccgcgcatgatcccgtggcggttcatcatgctggccggcgcggcgctggcgctgctgctgctgatccacctgacgacgctgttcggcgccgaacgcgccccttgggtctagccggcggcctccgagagaggaacccgaccgcccagccgggggtttgcctgtgcacttcccacgaacgacgcaggagatgcgaacatggccggcaaggacctgacccctcaagaggccgaaaccgaattctggaagagcctgaaggagtccaacaccggcatgctccgcgtcgaccggccgggcgagcacgcccagccgatgacgggatatggagagcccgagaccggcacgatctggttcttctcccgcgacgacaccgacttcgccaaggaagtcgccggcggcgggcagatgggcatgttcacctaccaggccgaggatgaagaggtttacgcctgcattcacggccagctgtcgatcgatcaggatcggtcgaaaattgacaaatactggaacccggtcgtcgccgcctggtatccggagggcaaggacgatccgcacctgaccctggtccgtttcgacgggcaggacggccgcgtctgggtgaccaaggaaggcggcctcggcttcggcttcaaggttcttaaggccaatgtcaccaagaccgaaccggatgtcggcggcgtgtcggacgtgaacctgggctaagcagctccagcgccagaaaaaggggcggtcgcacgtgcgaccgccccttttcgattcagccgccgaagcaccaggccagcaccgccttctgggcgtggatgcggttctccgcctcgtcccacaccagcgagcgcgcgccgtcgatgacggcgtccgtcacctcctcgccccggtgggccggcaggcagtgcaggaagacggcgtccggcgaagcgaggtccatcagcgcctcgtcgacctgataagcctcaaaggcgtgcagccgcgcctcatagtccttgtcgcccatggacacccaggtgtccgtgaccaccacgtcggcgccttccgccgcctcgcgcgggtcggaggtcaggctgaccgcctccccgcccttggccaggtcgcgcaggtccggatgatattccgcggggcaggccacgttcaggtggaagccgaacttggcggctgcgtgcatgaagctgtggcagacattgttgccgtcgccgatccaggcgatcgtctggccggctaccggcccgcgatgctcctcgatcgtcagcaggtcggccaggatctggcacgggtgcgagcggtcggtcaggccgttgacgaccggaaccgtggcgacgcgggcgaaccgctctacgtcctcgtggtcgttggcgcggatcatcaccgcatccaccatgcgcgacagcacccgcgcggtgtcctccaccggctcgccgcggcccagttgcatgtccgaagcggtggcgatgatggaggagccgcccaactggcggatggcggcgtcgaagctgaagcgggtgcgggtcgagttcttctcgaagatcatcgccagcacacggtcgcgcccgggggcgtcggcgtcggcgcggccctgcggccaacccctgcgcgcctgcttgcgggcatgggcgtcgtccaggatggcgcgcagctcggacgcttccagccggtggatgtcgaggaagtgcctgaccatcacgccgccagcttttcgcgcgccgctgcgcacgcgccttcgaaacgcgtgatcgcctcgcgggcctcttccaacgtcaggttcagcggcggcaagaggcgcacgcagttgtcgccgccgccggccaccagcagttgctgcgtgtcgcgcgccagggccatgaactcgcggttgttggggtgcagcttgaccccgatcagcaggcccttgccccgaacgtccacgatcacgtcgggatagcgttcctgaaggcccgccagctgctgcttcagatagccggcgatctcggccacattgttcagggtctcgggcgtgttgatggtcgacagggccgcctgaccgacggccatggccagcggattgccgccgaaggtcgagccgtggacgcccacggtcatgcccttggccgccttggccgacgcgaggcaggccccgatgggaaagccgccgcccagcgccttggccaccgccatgatgtcgggcgccatgccggcccactcgtgggcccacagcttgccggtccggcccatgccgcactggacctcgtcgaagatcagcagcatgccatgttcgtcggccatctggcgcatccagcgcaggtcttcctcgggcgtggcgcggcatccgccctcgccctgaaccggctccaggatgatcgcggcggtggtcggggcggcgaaggcggcctcgagcgcgtcccggtcaccccacgtcagctggtgaaagccctgcatcggcgggccgaagccctcggtgtagctggggttcgccgccgcgttgatcgcgccataggtgcggccgtggaacgagccgtcgaaaccgtagatgtcgatccgctccggctggccgttggcggagtgatacttgcgcgccgtcttcagcgcgcactcgaccgcctcggtgcccgagttggtgaagaagaccacgtcggcgaagctggattcgcacagctggtccgccagggcttcctgccccgggatgcggaagatgttggacacgtgccacagcttctcggcctgatccttgaccgcctgcaccagcaccggatgcgcatgccccaggccgttggtcgagatgcccgccacgcaatccagatactcggtcccgtccgtcgaccacaggcgcgcgcctcgcccgcgctccacctccagcggcgcgcgattgtagacacccatcagatggttcgtggacacgggacctgcacctccaaaagcgagacggccccgacgcgggcgcgacggagccggacttcaatgaggcctgacttgtcggaccgcgcggcggcttagtcaacaccgggcgcggcgcggggaaccggccggcgcccgcccggttagattcgggatgcggctgagggcgcctaactcttcagccgccagcccgaacggaagaccgaccagcacgctgcggccatgacgaccatcagcaccgcgccgcccacggcgccgaccgcgaggttgctttcggcgtggccgatgaagccgtagcggaagccgtcgatcagatagaagaacgggttgaagtggctgaccgtggcgaacggctccggcaggttctcgaccagatagaaggcgcccgacaggaaggtcatcggcatgaccacgaagttctgcaccgccgacaggtggtcgaacttctcgctccacaggccggccagcacgcccaacatgcccatgatgaagctggccgccacggcgaaccagatgatggcgaagatgttggcgacgcccagccgtgcgaacggcagcacgcacaccgccgtgactagacccaccagggcgccgcgcgtggccgagcccagggtgaagcccagcgtcagctccagcgggctgagcggcggcgtcaggaagtcggtcgccgtgcccatgatcttggcctggatcaggctggaggatgagttggcgaaggcgttgttcaggatcgccatcatgatcaggccgggcgccacgaactcggcgaacggcgtgccgtgcagcggcggtcgcgcgccctgcagcgccaccacgaacaccagcatgtaaagaagggtcgtcaccaccggcgcggccaccgtctgggcgcctaccttccagaaccggcgcacctcgcgttgatagagggtgatcaccccgacccaattgacccccggatagcggcggggctgcggcagcccggccgggcgcgtggacaggagatcgggcgtgctcatggccgcgcagatgcgcccgccggctcgctaccgcaaggctgagcggtctcgcagaacaacgattcaatatctggtttctgtggacagcctgattcgcacatgttgcgtcgcttaacaggaggtttacaactgattgtaggtctggagcccggaggggcccccagccactacatattgaatcctgaacgccggagggtggcatgaccgcaggctggaccgacgatcgcgtaggcgcgctgaagaagctgtggctggagggtcagtcggccagccagatcgccaagcagctgggcggcggcgtgacccgcaacgccgtgatcggcaaggtgcaccgcctcggcctgtcgggtcgggccgcgccgtcgcaaccggtgcgcgcccccgccccggccttccgcaccagccgcccacgcaccgcggcgtccaccgtggtggaaacagtggcagaggccgcttcggcgccgatcgttcgtcgccttgaggtggttcaggcgccgaagcccgtcgagtcggtcgccgcgccttcgcccgcccaggtcccggacctgccaggcaccgccacggtgctgacgctgggcgcccacatgtgcaaatggccgatcggcgatccgtcctcgcgcgagttcagcttctgcggccgtcgcgcctcagaaggcgtctactgcatcgagcacgcgcgcgtcgcctatcagccgcaggtccgccgcggcggcaaggacggcgcgtccgacctggcccgctcgctgcgccgctacatctgaccgcacgaccacccggcaatggacaaggcctcgccgatcgccggcggggcctttctagttgaggctgcgtctggcctcaggcgtatccagcgagaaggccggtatcgccgcctcgaatgaacggccttccgcatcggtgaaatagtaggccccgaccatcgtgcccgtgggcgtgctcaagggacagccggacgcataggcgtacgcgtcgccgggctggatcttcggctgctcgcccaccacgcctgcgccacgcacctcttcggttcgtcccagcccatcggtgatcgtccagcgccgagccatcagctgcacggccgcgcccgttaggttcaccacctccacctgataggcccagacccagcgcccgccctccggattcgactgaccggccaggtagctcggccgaacccggaccagaatgccgttggtttcggcgctataggcaggggcgtcgtgcatgggctatatgctcgccccgccacgcggcgggtgcaagcgtggcctgtgcgggatcgatcggcacgggctccctcggcccagaacaggacgacatgagcgcctattcccccacccgccccggcattctgcccgcccagggcatcgaggccctgatcgccggcggcgccatcgctgccgatacgccgttcgacgtcgatcaggtccagcccgccagcctggaccttcgcctgtcggaccaggcctggcgcgtgcgcgcctcctttctgcctggccggcgcaaggtcgaggaccgcatccgcgacgtggccatgcacgcggtccaggtcaccgacgccggcgtggtgctggaaaagggctgcgtgtacatcgcgcgcctgcaggagcggctgaagctgcccaagggtctgatcgcccgcgccaatcctaaaagctccaccggccgggtcgatgtgttcgtgcgcctgctgaccgaccagggcgcatccttcgacgacgtggccgagggctacgagggtgcgctctacatggagatcgcgcctcagaccttttccatcctggtgcggcccggaacccggctgaaccagttgcggctgaaggcgggcgagccgcccaagctcgaaacccgcagcgtcggtgtggacctgcgcggcggcgacgtcgtgggttttcgcggccgccgtcatgcgggggtggtcgatctcgaccacatcgacggccacgatccgcgcgacttctgggagccgctgagcttgcgtcgcggcgagctgctgctcgatccgggcgagttctacatcctggcctcctcggacgatgtggagatccccgtcgatcaggccgccgagatgacgccgatcgatccctccgtgggcgagttccgcgtccactacgccggcttcttcgatcccggcttcggcacggacgaggcgcacggcgcgggctccaaaggcgtgctggaggtccgcacccacgacaccccgttcctgctcgaacatgggcagatcgtggcgcgcctggtgtacgaaccgctgacggaacgccccagccgcctctatggcgagagcggcagccattatcagagccagggcctgaagctttccaagcacttccgcccctggggttgaggcgaggcgtcgcgccgcccgccctttgccgcgccgcccgcatggtctagtcaggcgccatgaccatggaggcgaccatgaagcgtgtgatcgttctgggcggagacggcttttgcggctggcccaccgccctgcatctgtcggcgcgcggctgggacgtgacgatcgtcgacaacctgtcgcgccgcaacatcgacaatgagctggaagtccagtcgctgacgcccatccgcaccatgggcgagcgcatccgagcctggaaggagatatccggccgcgacatcggcttcgtcaacctgacggtcggaaaggagttcgaccggctggtcgccctggtccgcgacctgcgtccggacagcatcgtccacttcgccgaacagcgcgccgcgccctattcgatgaagtcggcgcgccacaagctctacaccgtcgacaacaacctgaacgccaccaaccacctgctcgccgccattgtcgaaagcgggctggacgtgcacctggcgcacctgggcaccatgggggtttacggctacggcaccgccggcctgcgcatcccggaaggctatctgaaggtcacggtggacaccgacaacggcccggccgagcaggagatcctgttcccgccgaaccccggctccatctaccacatgaccaagacgcaggacgccctgctgtttcagttctacgccaggaacgacaagctcaggatcaccgacctgcaccagggcatcgtctggggcgcgcagaccgaggagacccgtcaggatgagcgtctgatcaaccgcttcgactatgacggcgactacggcacggttctgaaccggttcctgatgcaggcggcggtgggctatccgctgacggtgcatggctcgggcggccagacgcgggcttttatccatatccaggacacggtgcgctgcgtcgagctggcgctggagaacccgccgaagcgcggcgagcgcgtgcgcatcctgaaccagatgaccgaaagccgccgcgtgcgcgatctcgccagcattgtttcgcgcctaacgggggccgaagttcaccacgtcgccaacccccgccaggaagcggacgaaaacgagctggtcgtcgccaacgacggcttccgcgaactgggcttgaagccgatcacgctggccgaggggctgatgcaggacgtgacggagaacgcccgccgctatgccgaccgggtcgacctgtcgcgcatcccatgcgtgtccgcctggaacccggatcgtgcggaggcgctggagcacgagcaagctcggccgtatgtcgagccccggtccgccctcagcgcctgacggtcaggagttctgatgccgcaagcctcgtccgccccctcgcttctggtctttggaggaggctatctggggcgggcggcggcgctcgaggcgatccggcgcggccgcgcggcgaccgccacgtcacgtgatccggcgcgacgagcgatgcttcaggccgacgggatcaaggccgtggatccggcagaccgagaggcgctcggccgcgccgtggcccgacattcggccattctcgtcaccgcgccgcccgacgcgcgcggctgtccggcccagcgggtgctggcggaggtcgcgggagacgcctggcccgactggatcggctatgtctcctccacttcggtctatggagatcggtccggcggctgggtgttcgaggacgggccgctgaacgccgccagcctggaaggcgcccgccgcgtcaacgccgagcgcgactggctggacggcgcgcgcggcatgggcctgacggtgcaggtcttccgccttcccggcttctacggtcccggccgcagcgtcgtcgatcggctgcgcgacggctcggcccgactggtcagaaagcccggccagatcttcaaccgcatccacgtggacgacgtggtctcggccctgttcacctccatggaccggccgcatcctggcgcggcctacaacctcaccgacgatgagcccgcgcccgccgacgtggtgctggagtgggcggccgaacgcctgggcctgccccgtccgcccgaggtggactggatggacgacagcgtgggtccggtgatgcggcgcttctatctggactccaagcgagtctccaacgcccgcgccaaggccgaactggactggcgccccgcctatcccagctggcgagagggtctacaggcggtccttgaacagaccgcctgatctctggccctagaaggggatcaggttgcgctggcggctgtagctcatggtgccgacattggcgccgaggcgcaggccgacgccggtgcggatgggcgcaagcgtgatgccgtccgcgcgctgatagttcacgcccagtcccgccaccagataggccgttccctccacgcccgggaagcggcggtagatcatgtccggatggaacaggccgtagaccagggtgaacacccggctggcgttgccgccccagtcccaacccaccgacgcgccctgccagaacacctcctgcggggcgaacatctccttcatgtgcagggcgccgcggccgtagcgcgcaccgaccacgaaggcgcctgcgccctcctcgcccgcgatataggcggtggggcggtcgccctgttcggcgaagatccgctcgaccgcgctgcccacgacctcggcggcgatgcccagttcgcgcgatccggccgagaccacctcttcaaaggtgtaggccggcgcggtgttgtcggtggcgatcggatagttcggatcggacggcgcggtggcgcacgcgctcatggacgaagcgccggcggcggtggcgagccccgacaggatcagttgacgacgatgcaggggcaaaacggggccccggcagccgcgcccgccgatggcggggccgcgagggccggaccgtcgccgggctttgaggcagccttgcggcctgatggttaaccgcaccttacaggagtggcgcttgtccacgcctgcggaggcctcaggcccgcagccgcgcgccttgcttctcggcggccgcgacgatgcgggcgctcagggcctcgatctcggcctcggtcagcgtcgcctcgcgcggctggatggccacttccagcgccacggacttgaagccgtcctcgacgcccttgccgcgataaacgtcgaacacccgaacctcggtgatcagcgtcttgtcggcgccggccgcagcccggaccagatcgcccgccggcttggcctcctccaccacaaaggcgaagtcgcgcgtcagcggcgtcagcttggcgagatcggccgccccgcgcgtctttcccgccttgccgcgcggttccggcacggcgtccagcacgatctcgaacgccagcatcggcccatcggcgtccaggctcttcaacacgcgcggatggagcgcgccgaactccgcgatcagggtcttcggtcccaactgcaagcgcgccgagcgtcccggatgccaccaggggcggttctgcccctgccccagctgcagcgaggcgaccggcgcgccgatctcctccagcaggctcatcagatcgcccttcaggccgaacaggggatcctcacccgctcctccccagtgccgggccgcgtacggcgcgatcagcccggcgatgacggtgcgctggtcgcccggttggtcgcccagatagatgggcccgatctcgaacagggcggcgtcggcgtgcccccgcgcggcgttgcgcgccgtcgcctcgatcaggttcggcaggatcgacggccgcatgcagtcgaggtcggccgcgatgggattctccagcaccagacgcgcgtcgccgccgccgaacagggtcgccgtcgactgcttggtgaaggaccaggtgaccgcttctgaatagcccagggccgccagcgcccggcgcgcggtccgcacccgcgcctgacgggggctcagcactccgccggccggccgcgcgaccgggggcagcggcgtctccggcaggcgatcgaagccctcgatccgcgcgacctcctccaccagatcggccggcccttccacgtcgcgacgccaggacggcggcgtgacggtccaggccgcgccccgctcgatcgcaaagccgagcgcctgcaggatttccgcgatccgatcctccgacacgtccagccccgacagacggtgcacatgggccgaatcaaaggcgaaacccgttgggctcgccggggcttggccggcgaccgtgatctccgacggctcgccgccacacaggtccaggatcagccgggtcgccagctccagtcccgggaccaccgaggcgggatcaacgccgcgcgcgaaacgatactgcgcatccgaatgaatgccgtgcgcccgtcccgtctgggcgatggcgatcggttcgaaccaggcgctttcgataaagacgtcggtggtctcgtccgagcagcccgtgctgaccccgcccatgacgccgcccaggccgatcggacgctcacctcccgcatcggcgatgacgcagtcggcctccgacaccgaataggtcttgccgtccagtgcgatcagttgctcgtgcacgccagccgcgatgtgctcggcgcccgcggagacctgccccgcccgcaccacgatctcggtcccgaccagcttgcccgcatcataaacatgcaggggccgcgcctggtcgtaggcgatcaggttggttacatcgaccagccggttgatcgaccgcaggccgatggccgcaagccgccgctgcagccactcgggcgacggcccgttcttcacgccacggatcagccgcccggcgaagacggggcagagttccggcgcctcgatgcgcaccgcgatcggcgacgggaagccgccgcgcaccggcgcgatctcccaagtcttcagcacgcccgcgccggcggccgccaggtcgcgtgcgatgcccgccaccccgagccagtcgggccggttcggggtgacctcgaagtcgatcaccggctcggcgccgaacacgccggcggcgggcgcgccgacctgcagcgtctccggcagctccaggatgccgtcgctctcgtccgcgagctccagctccgaggccgagcatagcatgccgttcgacaccacgccgcgcaccggcttctcgaccagcgtcacgccgagacccggcacataggcgccgatcggcgcatagatggtcgtcagccccgcccgcgcgttcggcgcgccgcagacgatctccttcatcccgtcgaccgtctcgacctggcagacctgcaggcgatcggcgttggggtgccgctcggccgagacgatccgcgccacggtgaacggagccagcttcgccgccggatcgacgacctcctcgacctccagccccgccatggtcatggcgtcggcgatctgatgaacgtccgccccggtctcgaggtggttcttcagccaggaaagcgtgaacttcatcgcgccggctctccgctgaccgccaacagcatgtcgatcacctgatgcgatccggtgaagcccacgttgaagaactcgcagccctcgaaacggcagtcgcgcatgggcacagtgcccaaggcgcgcggtccggccggccgcagcaccaggttgcgcatgtcgccgtctcggtcgccaaagttgcagccgtcaaaggtcacgcccgcggacaccagcatgatggcgggtccctggatgcgacatcggacgaagttgcgacccgtgatcagaccggtgcgctccgcacaggcggcgtagagctcgaacagattgacgtccacatcctcgaatctctcggcgtgcagattaccggcgacgcggaccgagcgggtgatcggctgataattcattgtccggaggcctttctggccgactgcagggtctcggacagttccgtcagaaactcgggggagccggtaaagccgacctgcacgaaacggcagcggacaaagcggcaatcctgcagcccgatcacgccgatgagcttgggacccctgggctggaagagaagcgagttgacgtcttcggcaaggcccatgttgcagccgtcgaaggttgtgccgaccatggcggcgaccaccgccggcccttcgatgacgcattcggtgaaggtcttgcccctcaccacgccttcaccggcgttcaggctgtgcattgcgaggagcggcagccacactccctgcttgttgaactcggtctgcgccaccagttcgcgcccaaaagcctcggacatcatatcggtcatgtgagcgaactccggatcagctgaggccagaggccgggtttggcgaggcgaaggcggagaagccgtagtgcttcagccagcgcgtgtcggcttcgaacatggagcgcaggtctgggacgccgtatttcagcatggccaggcgatcgacgcccatgccgaaggcgaagccctgccattcgtcaggatcgagcccgcaggccttgagcacgttcgggtgcaccatgccgcagcccaggatctcaagccaatcgtcgccggtgttgaagacaagcttgccgcccgaacggtcgcagcggatgtccatctcggcggacggctctgtgaaggggaagtggtgcgggcggaaccgcgcctccacgccatccagctcaaagaagcgggcgataaaggtctgaagcgtggtcttcagatgccccatgtggatgtcgcggtcgatcaccagaccctcgatctggtggaacatcggcgtgtgggtggcgtccgagtccttccggaaggtgcggccgggcgcgatgatgcggatcggcggcttctggctcatcatggtgcgcacctgcaccggagaggtgtgggtcctcagcaccttgcgctcgcccgtttccggatcgggcttcagaaagaatgtgtcgtgcatctcccgcgccggatgcttgggcgggaagttcagggcggtgaagttgtggaagtcgtcttcgatgtcgggaccttcggccacggcgaagcccatctcggcgaagatggcgatcatctcgtccatcacctgcatggtcgggtgcaccgcaccgcggcgacgcgggcgcgacggcaatgtcagatcgacgtgctcggatagaaggcgcgcatccaactcggccgcttccagctcgctcttgcgcgccgcgagggctgcggacaccctgtcacgcagaccattcagctgggggccgcgttctcgccgctcgtccgggctcatcgcccccatgcccttcaacaggccggagatcgagccgctcttgccgagcgcccccacccgcacctcttccggggcggccgcgctttcggccgagccgatggcgttgatgagttcgagttcgagttgggccagggccggatcaggatgtgacatcgcgcggatcgtctagcgcctgaaccgccgttcgtcaccctttgcactcgcgggagcgaggcgagttgcaccgcacacggacgggttttcccaaaggcgccgcgaaaggttcatttacggcaaagctggcgttagatttctggacctaaaccggccccgttaaagaccatcttgggggacgggatgccgctgatcggggactatgtggagcggatcgcgccggtgtcgcccgccacgccctgcgcccttgtcctggaccggttcaccgacgagccgaacaccatggcgatcgcggtcgtcggcgacgacggccggccgctgggattgatcgagcgcaacgccttcaccctgcgcatggcggccgagttcgggcgcgccctctacgcccgtcgcccggccgaaagcctgatggatcgcaatgcgccggtggccgaggcctcgctgggcgccgagacctttttcgagacctacgaccaggccgagctgggcgcgctgctgagcggcttcatcgtggtgtcgggcgggctctatgtcggggtgggctcggcccttcaggtgatccaggcgggcgccgccctgcaccgacagagggccgagaccatggcggccctggcgcgggacctctccgcggcggaagccgaggccagcgcctccagccgcgccaagtccgagttcctggcggtgatgagccacgagatccgcacgcccttgaacggcgtcctgggcgtcgccgccctgatggagcgtcaactggagcaggcggagatgcgcccctatgtgcgcaccatcatcgactccggcgaaagcctgctgcgcctcctgaccgacgccctggacatgtctcgcgcctcggccggcatggtggtgctggacgaggcgcccacggatctgcagcggatcgccgccgatatcgacgccctgtggcggccccgtgcggaggagtcctctctcgagctgcggatcgagacgcacctggaggccggcgcctgggcgctggccgacggcatgcgcctgaagcaggtgctcaacaacctgatcggcaacgccctgaagttcacccgcgcgggcggcgtccacgtcacggtcgccacgcgcgaggacggcgatcgcatgacgctggacctcattgtggacgacagcgggccgggcgtgtcgccggcggccgcagctcgcatctttgagccgttcaacacgggcgaagccggccgcgagggcgcgggcgccggcctcgggctggcgatctgtcgccagatcgcagagcagatgcgcggccggatccgactggagacctcgccgcaggacggcgcgcgtttccatgtgcaggtgtcgctggcgccctgcgcggcggcggacggtcccccccggatcgcggcggctgaacccacgccgcacgagacgctgcatgtgctggtcgccgacgacaacgccaccaaccgctttgtggccggcaagctgatggagatgttcggctgcaccttcgagatggccgagaacggccggcaggccgtcgaggcggcgaccctgcgtcggttcgacctgatcctgatggacataaagatgccggtgatggacggcgtccaggccacgcgcgccatccgggccctgccgggaccggcggccggcacgccgatcctagccctgacggccaacgccgacgagcgggacgaggcgatctacgtcgccgcaggcatgaacggggtggcgcaaaagccgatccagcccgacgcccttctgaacgccatccgcttgacgctcagcgaggcgtcccgcggcatgatcgccgaagcggcctgacaccgaacagcgaaacgcccgccccggcgaaccggagcgggcgttgatcgatcgatcaggcgggcggctttacgccagcgcggcgcggaccttatcggccacggccttgaagcccgtcgcgtcggcggcgatcgaagccagcaccttgcggtccagttcgatgccggccttgttcaggccgttgatgaactggctgtaggtgaagccttccagacgcgcggcggcgttgatgcgctggatccacagggcgcggaaattgcgcttcttggtccggcggtcgcggtacgcatactgaccggcgcggtccacggcggccttggccgtgcggatggtgttcttgcggcgaccggagaagcccttggcctgctccagtacctttttgtgcttggcgtgggacgtgacgccccgtttcacgcgagccatgatttagtccttcaaattcttttcggtaagatcagtcgagctgcgtgcgccgatcaggcgtacggcatgtaggacttgatcttgcgggtgtcggcgtcggacatggtttccgtgccgcggcgctggcggatgtacttggagttgtggctgatcaagcggtgacgcttgcccgcgactccggccttcaccttgccgctcgccgtgaatttgaagcgcttcttggcgcccgacttcgtcttcagtttcggcatttcagtctccttgttggagggcggtcgtcctttgggctgcttgagcccgccgggtgaacaccttccagagtttaagagccgcccaggcatgcctgttcgcccgacggctcggtacgcgaaggcgcggcttctacgccaagcaaagcctcgacgcaagacgccccggcctttcgaccggggcgtctcttcaaccgcgctggaaaacctcagcggggcgccaggatcatgatcatctggcggccttccatcttgggcgagaactcgaccttggccacttcgtcgaagtcggtctgcaccttgttcagcagcttcatgccgagttccgggtgggccatctcgcgaccccgaaagcgaagggttaccttgaccttgtcgccctcctcgaagaagcggtgcatggccttggtcttcacctcatagtcgtgggtgtcgatgttcggccgcagcttgatttccttcagctcgacgaccttctggcgcttgcgctgctcggccttctttttctgctcctggaaacggaacttgccgtaatcgaggatcttggccaccggcggatcggccgtggcgacgatctcgaccaggtccagcccggcttcctcggcggcttccagcgcggcggaggtcggcatcacgccctgcttttcaccgttctggtcgatgagcagcacgcgcggcgagcggatttcctggttcatacgcggcccgtccttcacgggcggcgcttgcatgggacggcgaatgggcgtcgtttccttatgtgatcagagaaggcgtattctgacgagacggagcgcgtggcggatcgccacgttcctcccgatgggccaatatggccgtgaaagccccgtttttcaagccgagcccctccccatgatccagaccctgatccgtcccgacggcgagacgctggcctttcgctccgtcgggggctcaggcccgaccgccgtgtggatcggcggcttccgctcggacatggaggggaccaaggcgctggcgctggacgcggccgcgcgagaacggggctggaacttcgtccgctatgaccacttcgcgcacggcgcctcttccggcgactggaggcaggcgacgatcgggcgctggcgcgaggacgcaatcgccctgatcgaccgtctggaggggccggtgatcccggtcggatcgtccatgggcggctgggtggccctgctgctggcgctggttcggcctgagcgcgtgcgcggtctggttctggtcaatccggcgcaggacttcaccgagcggctgatgtggccgggcctggccgaccacgaacgccaggccatcctgcgcgacggcgagaccacggtgatcgaggatggtctaggcgcctatgtcctgacccgcgccatgtttgaggaggcgaagggctggatgctgctggacggccccatcgacatcaccgcgcccactcacatccttcagggccgcgcggacgacgtggtgccgtggcgtcatcaggtcgaactgatcgagcgccttcgcggcggcgacgttcggctcgatctgatcgagagcggcgaccatcggctttcgacgcctaacgacctcgaccggctgatcgcagcggttgaaggaatgcgagcctagcgcggtcccagcagcgagccgtacaggtccgtgcgccggtcgcggaagaagccccaagccgcccggtgccggtccaggtagtcgaggtcgaaggcgtgcaccaccacaccctcctcgtcgcgtcccaggctttcgaccagatcgccgcggtggtcggcgatgaaggacgagccgtagaagacctgtccggcctccgtcacctgctcgtgcccggtccggttggcgcccaccacaggcacgacgttggacaccgcgtggccctgcatcgcgcgccgccagggttcggcggtgtccaattccttgtcgtgcggctccgagccgatggcggtgggatacatcagcacctcggcgccctgcagcatcatggcgcgcgcggtctcggggtaccattggtcccagcagatgccgacgccgacccgcccgaagcgcgtgttccacaccttgaaccccgtgtcgcccggtcggaagtagtacttctcctggtagcctgggccgtcgggaatatggctcttgcgatagaggcccaacgcctcgccgtccgcgtccagcatcaccagcgagttgtaatactgcggcccgtcgcgctcgaagatggacaccggaatggctacgcccagttcccgcgccaccggcgaaagcgccgtcacgcacgggtgctcgcgccaggcgtaggcttcgccaaaccagcgctcttcctgcgagacgcagaagtacggcccttggaacagctcggacggcaggatcacctgcgcgccccgccccgccgcctcgcgaacgaagtcgaccgtcttcttgatgttggcctgcatgtcctcgccataggacgtctggatcgcggcgacggagatcgtgcggggcatcaggccggctcctgctgagagatgcagtgaaaggatccgccgccggacaggacggccagtgacggcagcggaatgatctcgcgatcggggaagacggtctgaagcgcctgacacgccaggtccgccgcccgctcgtcgccataggtcggcacgatcaccgcgccgttggcgatcaggaagttcatgtggctggcggggatgacctcgtcctcgtcctcgatccggcccggcgacgggatccgcagcacccggatcgcgcgtccctccgcatcggtcatggccaggagatcgcgcgccacggcgtcatagacctcggcgttcggatcgttctcgccccaggcgatcgggcaggcgaccacccccggcgccacgaaccgcgccagattgtccacgtggccgtccgtatggtcgttcaggaggccgtcgcccagccacagcaccttgcgcgcgcccagcgcctgggcgagcgccgcctcggccttggcttcggtccagtcgccgttgcggttggggttcagcaggcactggcgcgtggtcagcaccgtccccgccccgtcgtgatccagcgccccgccttccagcacgacgtcgtggcggtccaaggtcacgcccgccgcccgcccgatctggtcggcgacttcgtcgtcgtgcggcaggtcgtacttgccgccccacccgttgaaccggaacgcggccgcccgagccgagcccgcaccgaagatcggcccggtatccctcagccagatgtcgccgaaacgaccgcccacgacctggacggccggcgcatcggcgaagcgcgcccgcgcctcctccagcgcttcggcgttgccgaccatcagcttgacccgctcgtcccccggccccgccagcgcacgcaccagcgcctcgacttcggcttgcgccggctccaggttctcctcccacagctccgcatgcgacggccagccgacccacatcgcgcgatgcggcgaccattcggcggggatgggcgggctcatggcgctctccggggatcaggacgacagccgcgccatatggcgtccaccgctccctacttcaacagccaagaaaaaaggcggcccgcgaacggaccgcctctctcccgccttgacgcttgcgctgtcgcttagaagcggtagcgcacgccgaacttcatctgccacaccgaggcgttggtcaccgttgacggcgtccgctgcgtgaagccggtgtaggtgtactgggtattggcagcatcgcgcgtagcggcgacattgttcgagatgtacgggaagtcgatctgctgcagcgtgccccactcgtcgttcagcagattgccgaagttctcgatatccagataggcgctgatgcgcgatccgcccgggaagaaggccggcagttcctgctcgatgtgcaggtccaccgtggtgagatacggcgagttgaaggcgttacgcggcgagatgctgccggcgtagtcgatcaggcccgtctgcttcaggaagtcgttgaacgccgccacgttgaaggtggagctgtaggtcacgatcgggtcgctggtcgccgtcacgttgcccgagctgtccacctgcggcacgtacagcaggttgcgattggtcgaggtgtagtcgccgaacaggttgcccgagctgaaggtgtagctgaagggcaggcccgagcgacgctgcgcaaacagggcgaagcgggtgcgatagtcgccgaagaaggcgcgctgatagctgacgctcagcttcaaggcgtgctcgatctcatagttcgagctcgacagcggcggcatgttggggtccgacacggcgatgttgccgaagttcgagcttgccgtcgatgacgtgccggccgacgggtcggtcgcgtccaggtaggtgtagctgaagttgaaaccagcgccattcagccagccatcaaaccaatccttggacacgcccaccgcaaactggtccgcctcgccgcccttgaagttggtcagcatgagaacctgctggcccgtgcgggtcgggttgggtccgaacaccggacgaccatccggagcggtcgcattctgggtctgcagcaggctgaggtcgacccagcctacggtgttctccagctccgagtggacgtactcagccgtcatgttccaggcgtcgcccataccgaaccggctgagatcgaagcgcttgttcacacccagcgacgtcttccagatcgacggcgtctcgaaggacggatcgatcaggttgatgttgcccgtaccgcggttggcgctgtcggtgacttgggcttgaccaatcgggctgacgttgaagccatcgacgttgcttaacactgcggcgttagcatcgcatggtgcgaagttgcctgcgaagttcgagctgtaatctctcgagatgcggcactggaacgagccagtgagattgcccgggttcgtgtagctgttagaaatccagacgttcggcgaaccaccctggaaacgaccaaagccgccgtaaatcgtcaggtcctccgaggcgcgccagttgaagccgaagcgcggctgcagaacgaagatgccgtcgaggttggtcgtgttggagaagccgtagcggcgctcgaacgcctcattgtactgcggctcatcgtccgaggtgtagtagtcgaagcgtaggccggcggtgaccgtcaggtcgtcggtcgcctgccactcgtcctgcacgaacagggtgttcaaggcatagctgaaggcggctgcgccgtcgttcttgttgttcgacgctgcgttggtatagccgaacgaagaggcttgacggttgcggaaggcctcaatggaggcgaattcatattcgccgttcgccacctgaacgaacaggttgaagatgtcctgttcttcgcgctcgaagccgccggtcaggcggtgcccgaagcccacgtcccagttggcgaccgcgcggtaaagagtcgtatccaccgtaagggcgttggcgtgacgcgagcggtccggtccaaggcggatcgacgcctccggccctcgcgaggggccggtgggatcgaccaggtagatctgcatggaggcgaagtcgttgccggccaacgactcggagatgttctccacttccttgcgcgacaccgacagttcggtcgagaaggtgtcggtccagtccgagaacagctggcccttgtagaccttcaggttgctgaccagcgtataggcctgcgacagcagccccaagctcgggtagttgccgcccgtcgtcgtgccgccaagacgaagatcgccgccctcagtctgctggtaagaggcgaccgcgcgatggcgatcgttgatgttccagtcaagcttggcgaagtacttctcgtcggtaacctccaaggcgtcggcttgccagtccagcggatcatagccgtacacttcacgcgcaatctgacgaacggtgtccacgtccgcttgggtcacgcccggcacctggttcgcagcgcccgatccggtcggaccggtgaagaccggctgcgtcgattcatagttctcgtagttcaggaagaagaatagacgatccttgatgatcgggccgcccaggctggcgccccaggtcgtttcttcgaactgcccgctgaggctgcggttctgacgttggccggtgacgaaatcctcgtatgagaaggagttgccctgcaggccttcgttggtggtttcccagaacgcggtgccgctgaactcattgccgccggacttggtgaccgagttgatcacgccgcccgtgaagctgccgtactgcacgccatagggcgcgacatcgacgctgaccgcttcgagcgcgtcgatcgagataggcgaacgctgggtcggatagccgttgccgttcagaccaaagtcgtcgctctgacgcagaccgtcgacgaggatcgcgttggagcgggtgttctggccgccgatcgacagggcgtcgttgttcgacggatcaaccgtggcgaagggcgaggtgcggacgaaatccttgatgtcgcggctgatcgagggaagggtctcgatgtcgttcaggccgatgttggtgcgcggggaggtgcgcagaccgccggcccgctgaccagtcacgacaacgtcgcccagatcggcggcctcatcagaaagggcgccgccgccgacgatgatgtcgatgctggctggggtgccgataccgatggagccggcttctgtggtcgaggaaccggcggtcgagttgaccgtcacgatataggggccgccgacgcgcaggttgcgggcgctgtaggcgccgacctggtcggtcgcggtgatggaagacgtgcccgacggaacgtgggtgaccgtgacttcggcgttcgccaccggcgcaccggccgcatccgtcaccacgccgcggatgccgccggttgtttcctgcgcgaaaacggcggtggacgccgacagcatgatggccacggtcgaggcgccgtaggcgagattgcggaacttcatgaactatccccagagagcaggctaagcctggacagaccggcgggccggccgtgatggcgccccattaggccgggtgtccgaacgctggacgacagttgcatgacagagtcatgacatggaaggagggtgacgcatgcgccacacccggtgggtcagctgacggcgcgctcgaacatgtccgccaggccttccgccgccaggggctgggtgcgcggctcgtgatagttgccgttgatctggcttgcggcgatgacatgggcgcggaagcggtggaacagcgcctcgtcgggaggcgtcggctcggaccagaagcggtcaagcggcttctggtccgtcaggccttcgaagtcgaagaaggcgtccccgaggaccttgaccggcgtatggaagcccaaggcggacagagccgcgctggagttgttgacgaccatgccccgagatgcgcggcacaattcgttgagatggccgccgtcgatgaaatccacccggtcggccacgccgcgctccatcgccagccagcgcgtgatgcgacgcaggctgacgacgcccggatccagcggatggttcttgaccactaggcggcaatccccgggcgcatgacgagcgaagctgtccagagtcgcggccataaaggcgctgttgtccgcatactgcgaatagcgcagcagttgcatgtcgccttcgcgctgcagacagacgatgaagaacggtccgcgcgccgcgatctgctccgcatcgcgcgtgcgccggggtcggaaagcgaggccgagatagcgtcgaacatggccgatgcactgcttcaacggtgaatgcgggtaatgaacaacgaagttcggaaagaccgccgaccccatagcttccgctatgtggtacaggctgatgttggccacatggtgcggcaggatgcgcccgacaggctgcaccgcaggcggcggcagggccggcgcggcgtaggcgccgcgaaatcgcggcagtccgcttgagccgttcactccattgcgttcaacggtgatccagtctgggcggaagtagccgttttcgagcacccagacgcgcgcggcgagcgcctcgacctgggacagcacggcccggttatagggaccgccttcgccaaagacgatcaggtcggtgacgccaccggcgatgccggcgagatccgccgcccattgctctggacccggcttgtagatcagcccccccgcgcggcgccaggacgcagcgtccgcggcgttgaagatcatgcgctgaaccgacgcccccctcgcctcgagcgttctggccaggatgcgggcgaacccgccaaatggcgcggtgacgatcaggaagcgtcggccgccgaggccttgggcgccgaccgcctcgcgcggagcgcttcggtgctgagccgatggccaatgcgcctccctcgcgtgcattgccaccccgggctggcgacgcgatctgctccggtacatctggcgttcggacaagcgtcgccggaacgaggggagatcaaccacgcgcggcgctctccagacggcgtcggactttcagcccaagcccctcgcccgatccgatttcgcacacgccgcacatgacacgtcttttgagccgcagagcgggatcgatcaagagagtgatccgcaacaagccgagggtgttgtctgtgcaccaaccattcacgccaggttacgcaaaaggccgccgctcttttggagcgacggcctgatgttcgtcatcggttttcttggtccggctcgggagcgagagggccggcgggccggctctctcgtccttggctcgggtcttagaagttgatgtcgacggtggcgcgacggttcagcggttcgcgcacgccgtcggcggtggcgcgggccagctgggtttcgccgcggccgtccagcgacaccacgccgcccgacacgccctgggcgaccatggcgtcagccacggtgcgggcgcggcggttcgacagacccacgttgtaggcggccgagccggaggtgtcggcgtggccgaccaccagcacgcgggtcggacggcccgacttggcgtagttggcggcctgcgtcaccaccgagcgggcttccgccgtcaggtccgagcgatcccagtcgaagtagaccacgaactgacgggcctgcggggtcgccggaggcccgtcagttcgtgggctacttcgactgggatcgctcggacctgacggcgggaggccgctcgggggggacgcg

SEQ ID NO: 5 - DNA, 262282 bp, brevundimonas massiliensis
  source 1..262282: mol_type = genomic DNA
caatccccatcgcctgcactcagcactgggctatatcagccccgctgaggccgagcgcaaagcggcttaaccccgtccacttttacgggggaagatcaaacccgcagcgaggtcctatggcgaggggattgtctttctgacctcccgaccgtcaagcgggctcgtggaatagcaatctgggtggagccggcaaggccgggggagggggcggctggagttcagtgccgggacgaaccgccgcgaggatcaagcgctccaggcattcgatcgcctcccgcttctcctcaagatagtcgtgctggacatagaccgacatggtgatggacgatccgccgcctagctcgttcgcatggttgagaagcttggacagaatgaaggggcttgtcctggctcgcgccagcctggtcgctccgctgcggcgcaggtcgtggaccgtgatgtccggaatatcgatcgcggccctgatgtcgcgcatggcgtggctgatcgccgagggatgaatggcgcccggcgcctcgccgcgcccgacgaagacaaacggcgacggctccgcgccctccgacggctttggccgaagcgccagggcttccttgatcaggacgatcgaaaacgcgcccaagggaacgacggtggtgcgtccggccttggtgcggccggcggggatcgtccatgtcttctcggcgaaatcgagttcggcgactcgcatctccgcgacctccgcgcgtcgctgcagaagtagggccgccagctggatcgcgatccggatcggacgccccaccattagcgcctcgtcccggcctttcggcagcggacgtcggtagccggacgtgtcttcgagggcccgccagagcgctcgcaactcgacatcgttgaggacgcgcgtccgcggggtttcctccgcgagatcgtcgagctgctgggcggggttcctgagaacccgatcttcggagattccccacgcgaaaatctggctgatcaggctccgggcgcgattggacgtaactcccttgccctcttgcaggatctcccgaaggcgtttgcgcaccacgtccttggtcaccgcttcgatgcgcaaacccgcgatctggcggagatgcttccggtagaggttccgttcggaaaggatggtgggcgcgcgcttgcgctttttgctcgggcgatactctccggtctcggtggccctgaagtagccctcggccatgtcgtcgaacgtcctcagcgtctgagccttggcttcggccttgatgacctgaatttcggtcgctggatcgcggccggcgtcgatctcggtttgaagtttcctcgccttcgcgcgggcccccgcgaccgtcagcgcggcggcgtcgcccagggcttgatccggcggaacatagcgaccgagccgaactctcggctgacttccatccagacgccgataacgaaagccccagactttcgagtgccccgaaacccgcaggtagagacccttcaggtccgcatcccagagctcgagacgatgttcgtcagtcggtctgagcgccgcgacgctccggtctgtcagtcgtgtcgcgcccatctgaatcctcgtccgaagcgccccgattttggggagcaaatggggagcaaattgcagcaactcgaagcatagcgacgaagaggggtgaattcaaaaactttctaaaaacagtgcattagcacagtcctgaacagtcctgaaaaggcattggaggccgctgggggtcaaggggtcgcaggttcgaatcctgtcgctccgaccattgaaagaaagcccgcgatctcggtcgcgggcttttctgtttccgtcagccccgctcggcccacttcagcagcgggatcaggggcaggccccaggccgtgccgccgatggcgaagaacaggaagtcgagcagcgccgaggcggggaacaggccgcgcagcgcgatcagcgcccagacccagaaggcgagaaagatcagaactcccatcgccgcgacgaaccggcgggcgcgagcgcccatcagcgcttgctccggaacaggaaaaaggcgagcaggcagaacatcgccccgcccatcgcccagggaacccaagtccagctgtcggtgatcgccaaggcgaagacgcgcacggccaggaaccagccgcagaccgcccccgtcgcggacaccagcgatgtggccagcagtccgcgccgccccgtcagcagatcggcggccgccgccagcaacaaggcgccgacggcggcggtgatgatctcggcgtactccaagtccggcctctcattgcgcaagcgcgacgttaacttaaagcgactcgccctcgccgcctgagccgggcataccgccagggtcgcatccaaggacggcgacagcatagtcgggtcagcagcaggcgtcgaatgaaccgtttcgggacctatgatcgcagccgcatcgtggccgcgtggctgttcgccaccgccgccctggtgttcgtgatggtggtgatcggcggggtgacgcggctgaccgggtcggggctgtccatcaccgaatggaagccgatcatgggggcgatcccgcccttgaacaccgccgactggctggaggccttcgaaaagtacaagcagatcccgcagtacgcccaggtcaacgccggcatgagcctggccgagttccagggcatcttctggtgggaatggctgcaccggctggtcggacgcggcatcggactggtgttcggcctgccgctggtcgtatttctgctgttccggttcgccccgccgcgttcgcgtctgcgccgatgggcgatgccggatcggctgatctggcgctgcgtgctgctgctggcgctgggcggcctccagggtctgatcggctggtggatggtgtccagcgggctgtccgaacgggtcagcgtcgcgccggagcggctggcggtccacctcggcctcgcctttgtgctgttcgccgccctgatctggacgggcctggaggcctggttcggagagaaccacgtccgcccgcccgcgggatgggcgaggggggcggggctgctgttcggcctggtgtttctgcagtgcctgctgggcgcgctggtggcgggcggcaaggccgggctcgtctacacggactggcccctgatgaacggtcaggtcctgccgccggccgactggagcctgggcgcgggcgccttcctgcacgaccaggcgctgacgcagttcaatcaccgtttaggcggctatgttctgctgatcggggcttccatctacgcctttcaggcctggcgctggcgcgtcgccgaagggatgggggcgggcgccttcgccgtcgccggggcggtatggctgcaggcgctgctgggcgtcttcaccttgatccacgccgtgcctcttgtgctgggcgtcctgcatcaggcgggtgcggccctggtgctggcggcggtgacggcgaacctgtggatcgcgttgcgcgcccaggcgcgcatcttcatgagcggcccccgcgccgtgcggcgttagatgcggtattttaataccgtacagattttacgttgtcatatcaatgcggtagcgcgagatgtcctgagcgaactgcattgacgtagacggacgcctcctgtactagcgcgccttccttcggttccccagcggggccggacccgatttcgtcttccaggaacaacctcatgctgaagagcaccacggcttcgttgaagccggccgaggtcgagaagaagtggatccatatcgacgccgaaggcgtcgtggtgggccgcctcgcgacctttatcgccaaccgcctgcgcggcaagcaccgcggcgactacaccccgcacgtcgattgcggcgactatgtcgtcgtgaccaacgtcgacaaggtggtgttcaccggcaagaagtcgaccgacaaggtctattatcgtcacaccggccaccctggcggcgtcaaggagaccaccccggccaaggtgctgggcggccgtttccccgagcgcgtgcttgaaaaggctgtcgagcgcatgctgcccaaggagagcccgctggcccgcaagcagatgacgcacctgcgtctgttcgccggctccgagcacagccacgaagcccaacagccggaaaccgtcgacttcaagtcgatgtcggccaagaacgtccggagcgcctgagcatgactgacgcgacgcaaacgaccgcgaccggctttgacgccctgcgcggcctgaccgcttcggccgagtccgaagcccccgtctatgagcagaagctggactcgctgggccgcgcctattcgaccggcaagcgcaagaacgccatcgcccgcgtgtgggtgaagcccggcaccggcaagatcaccatcaacggcaaggaccaggagcagtatttcgctcgtcccgtgctgcgcatgatgatcgcccagccgctgacggtctcggaccgcgcgacccagtacgacgtgatctgcacggtcgagggctcgggcctgtcgggccaggccggcgccatccgccacggcctgtcgcacgccctgacacactatgagccggaactgcgcaaggtcctgaagccgcacggcttcctgacccgcgacgcccgcgtcgtcgagcgcaagaagtacggtcgcgccaaggctcgccgcagcttccagttctcgaagcgctaagtccggtcgcaagcgcgacaggcgaaaacgaacaaggcgcttcggggaccacccgaagcgccttttttctgtccgcagatgcggccaaggcggaacgcatgacccataccctcttcatcgacggcgaggccggcaccacgggactggagatccgcgagcggctggaggcgcgcggcgatctggagttgatcctgctgggtgaacggcgccgcgacgtggaggcgcgacgcgaggcgctgaacgcggccgatgcggtgatcctgtgcctgcccgacgacgcggcgcgggaggccgtcggtctgatcgaaaatccggccgtgagggtgatcgacgcctcgaccgcctatcgcgtcgcaccgggctggacctacggcttccccgagatggacgaggaccagcgcgcggccgtggcgggggccacgcgcgtgtccaatcccggctgctatccgaccggctttatcggtctgatgcgtcccctggtgcgggcggggatcgtgccggcggatcggccgatcaccgtgaacgccgtgtccggctattccggcggcggcaaggccatgatcgccgagttcgaagagaagcggggcgcgccgccctttcgcgcttacggcctctccctccagcacaagcacgtgccggagatgacgcgccattcgggcctgaccacgcccgtgctgttcgcgccggcggtgggcgcctatcgccagggcatgctggtggaagtcccgctgcatctgtccagcctgccggaaacgccgtcggtggagcggatccacggggcgctggtcgaacactatgaaggcgcgcggttcgtcgaggtcgccgacctggacgagacggaggcgatcacgggcatcgatccgcaggggctgaacgggaccaaccgcatgcggctgcatgtgttcggcgaccgggcaggcgagcaggtcaggctggtcgcgctgctggacaacctgggcaagggcgcctcgggcgcggcggtgcagaacctcaatctgatgctgggtctggacgaggcgacgggcctgagctgaccccgcttcagtcgtcggcgcgcgccttcagggccgagtcgatcgtcaggccgaaccagatcgaggcgatgataatcagcaggccgtaatcccgtcccggcgcgaacaccggcgcggacgccgcggcgatcaccagcaacgggaacagcccggcgaaggcggcggtcgccggagcgtcgcggcgaatcagcggtcgtgcgtcccgcttcatgaacctggacacagggccgttcgcgaccacgaacacgagggcgcagatcgccgccagcagggcgtagcgcagctgtgatcccggtacgccgtagagccccgcggtcatgaccagcaggatcagggcgacgccggtgctgacggccaaaagcaggttgggttcgaaacggctcaatatccggcgcccttatccgcgaggtacgcccaagatggggatcgccgcgtcgattgcttgccacgggagcctactcctgtgacgaacacccatactagtgcggccgacggtcccgggcgcgctcgggcttccgccggttggggcgatggcctatgtcctgtttgatcatgatccacctttcgacaacaaccgttctcgtcgccgttgcgggactggcgacctgcggctgcaccacggccctggaccgcagccaggcggcggtcggcccgatgtcggagcgtgtcgacgcgctggtggcggccaatcggacctatccgcgctgggccgacttccccgccgcgcccgccgatctcccgacatctcaggtgttggcggggcgggtgagcgatctgcagggatcgagcctgcgtctggccggtgaaacctccaggatcgactggaccctcggcgacccggaggccctggccgccgaaactcgccgggccgtgggcgcggtgccggcgtcgccggacgcgatacgtacggaggccgaagtcgaagccttcgcccgccggctgcgggaacgcgcaaaggcgccgccgcctatcgatcgccagccttgaggcgtccgggccatggctgatggtggagccggtgcgggcggccggcccgcctttctgggcgtcgagcgatctttgtcgggccgcacctggcgacagcggccggccgacgcgtcgcttgttcggcatcatatgcaggccttggggctggacgagccgctggcgcgcgccatggcgtcgcgcgaggtcggggccgacgaaggcgcgcactatctgaagccgacgctgcgcgcgctgttcccggacccctcatgcttcgccgatatggatgcggctgcggcggcgatcgtcgacgcggtgaagcgcaaggccggcatccatgtcttcgccgactacgatgtcgacggcgccgccagcgctgcgctgctgatccgctggttcagggcggcgggtacggaggcgtcgatctatgtgccggaccgcctgaccgaaggctatggtccgagcgcacgcgctttcgacacgctgaaggcctcgggcgccgatcttgtgatcaccgtggactgcggcgccgcggcgaacgaggctctggcgcatgccgccgcgatcgacctgccggtcgtggtcgtcgatcaccacttgatgcgggccgagccgcccagggcgctggccgtggtcaatccgaaccgcagcgactgcgggtcaggccagggcgtgctggctgcggccggagtggtcttcgtgctgctggcggcgttgaaccgggagggccgcaagcagggtctcttcgcagagcgggcggagcccgacatccgccgctggatggacctggcggcgctgggtgcgatctgcgacgtgacgcgcctctccggctttaaccgcgcgctgacgggcctgggcctgaaggtcatgagcgattggagcaatcccggcctgcacgccttgctgaaggcggcgggcgtggagccgagcgaggccaaggtcagccacgccggctttatcctgggacctaggatcaatgcgggcgggcgcatcgggcgttcggacctgggcgcgagactgctgtccaccgatgacgcgaccgaggccgcccggcttgcggccgaactggacgccctcaacgtccagcggcgcgaggtcgagcgcgaggtcaccgaaaccgccatccggcgcgtcgaggcgaccggcgtgcacgccgacaattcgcccgtcgtggtcgtcgccggggaggactggcatccgggcgtggtcggcatcgtagccgggcgcttgcgtgaacgctggcgcaagccggtgatcgtgatcgggatcgacccggtgaccggcgtcggcaaggggtcgggccggtcgcagccgggcatgaacctgggacgcgccgttcaggcggcatgggaggagggcgtcctgctcgccgggggcggccacgccatggcggcgggcctgactatgcatcgggcgcgtctcaacgatctggtggccttcctgcacgcgagacttgcggctgagcgcgtcgaggctctggccgacgacgtcctggacatcgacgccctgatcgagcctggcggcgccagtcgcgacctattcgaggcttttgagcagctggcgccctttggccccggcaacccggagccggtctttgcgctgagcggcgtccaggcgcgcgagcccatgcagatgaacggcggccacatccgttgccgccttgtcgcgcccgatggcggcggcctgcgagcggtcgcctggcgatgcgccgacctgcctcagggacgcgctctgctgtcgggccaaggcggtctcagcgtcgtcgggcggctgaaggcggacgactggaacggccgccgcggcgttcagttcgagatcgaggatgtcgccgatccacgcatggcctgaggccaagcttgacctttcggcgttcgttcattttcctcatttttctcgcttgcacagccgaaaaggcccggctatatcgccggctctcccgcgcagcggtcccttcgtctatcggttaggacgtcaggttttcaacctgaaaagaggggttcgattcccctagggactgccacgcgggtcaaaatcttctagcctttcatgctgttagaagcgcctttggctaaccgggcgaccgggttagccaaatctcgttccccatccgtatcgatccgtgccatcgcggccttggcggcgagggtctgatctcgacggcggatgtagatttccagttccttcaggctggcgtgtccggtgatcgactggatctccaggattgtgcagccagcgtcagcgaggcggacggcaatgcacttgcgcaggccgtgggcggagcattcaggaacgcccgcttgtcggcaggcttccttgatccagttgccaaagcccccggccgtgtagccctcgccatactgggtcagcaggagctgcatctggtccgccggaacggtagcgatggatgcagccagacgtgggtggatcgggatcgtcagccaagcgccggtcttcgactgtcgaaccgacacgccggccgccgacaggtgctgccgccccatcatccgcacgtctttcgaccgctggccggtgtacagcagcaggtccatccccagccgctgtttcgtcccgacgggccaccgggcctcgaacgcggccacctccgcctcggtccaggtgtgatagccgtccgtccgatacgcgatcttcttgatcgccatggccggattgtcggttcgcaggccacggctgacggcgaacgccaggaaccaccgcagggccttgatgaagttgttgcgggcggcgttgccctccatcttgtcgcgcaggctcagcaggttcgccgacgtaagcgcgcggactgtcttgtcgccgtggtcgcgcctgaagcgctccatgacgccgcgatagttggcgcgggtggtctcggccaggttcgaccattccgccgacgcgtaggccgctaccgccagggcgttgatgctgcccggctgagtacggccttggccgggaacgatggcctgcgcacccgccgccgcctgataggcttcagcgaactcaggtgagcccggcaggcccggcagataaacggtcggcagtcccttcttgcggaaccggtaacgcaccttcccatggcggtcgcgcatgggcgtgacgttcaggaagcctagctgccgcaggccgcgtcccatgccgcgcgctccctttccatagcctcagtgtcgttgctggcgaccggggagggggccttcaggtagatgcgcgccacgccgccgggcaggaggtcgaggcactcaggcgacttgccctcggccgccaggaccgcgagggcgcgtttcagctcatgttgcttgaaggtgcgggcggtcactgagcgacctccacaccgaacaccaggggggtgccaacggcctgagccaaatggacccccagcgcctgcgcatccaagacgatccaagggactgccgccccgtcaacagcgttggcgagtgagcgataggccagaaagggagcgctgtccttggacacgacaaagcggcccaccttttcggtgagctcatccattttcccggggatggcgctggagatcgcgaaggcccagaccaagccgtccacaccctgattgccagccgccgcgatcatggttgccgcctgtgctgggccgaccagtcgcgaaacgcggtcgaggaccaggaggcgcgccaactccttcggggtccagcgggtccagcccggattgtccttgggctccagcgggccgcccgccgaacgccacttccgttgcagagcggtcgagacaccggtgatcgcggcggcctcagcgggggagaaagtcggctctctaaccataccgtcccatatgtcacgattttaccgccgtcgcaataccgttctgcatttcacggttcagcgcccactcgatctcacagggcagcggccgaacgttgatcaggtcgcattggtggaacagctcctccaatgcctcctcctgggcgggtgtgagggcgtcggggatcattcgaagtcctccggctcatagtcgcccgagggtgcgccctcgtcctcgcagtgacgtgatggtgtggacgacctccgcctgacgggctgttctgggtgtgtcgtcatcagggacgtcacgtctaggagcggtatcatgcagaccatcgctgtcgtcgggctcgatctggcgaagactgttttccaggttcacggtgtagccacagacggcacggtcgtcgtgagacggcaactgcggcgcggccaggtgctggccttcttccagtcgattgggccgtgcctgatcgggatcgaggcgtgcgcctcagcccaccactgggcgcgtgaactgatggcgatcggccacgatgttcggctcatgccgccggcgtacgtgaaggcctatgtgaagcgcggcaagaccgacgccgccgacgctgaagcgattgccgaggctgtcacccggccgaccatgcggttcgtggctgtgaagtcgaaggcccagcaggcggtgttgatgctgcacaagacccgggatctcctggttcgtcagcgaacgatgctgatcaacgcactgcggggccacctcggggagttcggcatcgtcgcgcctcaaggtccagctggggtgcgggcagcgctgaagagtctgcgtgaagagggtcaggccctgccggatctggcgcatgccgcgcttggcgggctggcagaacagctcgaacaccttggcgcagagatcagccgtatggagcgtcggattctcgattggcatcggcaggatgagacgagccggcgactggcgaccatcccaggcatcgggccgatcactgccagcgccatggcggccagcgcgccagatccgagtctcttccgttccggtcggcagtttgcagcctggctgggactcacgccgcgggccaatagcagtggcggcaaggaacgccagggcggcatcagcaagatgggtgacagctaccttcgacgtctcctggtcgtcggggccacggcggtcctgcgaatggcccggcagcgaggacgcgagggctgggtcggcaatctcctcgaacgcaagaagccgaaggtcgccgccgtggccttggccaataagacggcgcgcatcgcctggaccctgatggcgggacaggaggactacaagcccacagcggcatagagatcgggccgggcttcacccaggaccggcgccgtagacgaaggagtggtgagacgtgatgacgaaccggccgcagccggggatcggtgaaacccagggggtcagagcgcctcgagcgcgttgacgtgattagggagccggtccgcggacttcatcagggccagcagcgcaaacagctgcatcaacaggccgaacacatgactgcactcgaccgagcgccaacgtcgtttccactcttgcgtcttggaggtcgtccacacatgacgtccctgatgacgacacacccagaacagcccgtcaggcggaggtcgtccacaccatcacgtcatggggcatgtcgaagacgggcacatatcttggcgggagcaccatcctcggctggtccggtgcgccccgctcggcagcgagaaagcgaagcggcggaaagggcctactggctcgggaagttgaagcgcacggaccgacgctccagcggtctgagcacatgccgccgctgggaccggctcctgttcaggctcgcaagccgtctgctccgaagcctgcacggaagaagaagccgatctccgcagccgaactcgtccacttcagcttcggcggccgttccaaggatcgcgtgctggacgatctcgaacccatcgtctggaagctggcccagaatggattccgcaaaccggccgacgtcgcccgcctcctcaacaagcaaggggtgaagacggcttgcggcgaacagtggagcacccaactcgcgtggcccctgctcgccctcttgttcgagcggcgccgacagcagagagccgcccgcccctcgaaggcgcccgccgctcctcgcgtccattcgacatcgaaggcgccgctatcgagcgaagagatcgcacgccgactatctgcgctggggcgagtagcccgatctcattgacgccccgacgatccgcagcctctacgtcagccgccgactgactggtgcctgaccgcgcggcttgcgccccatcaaccgggcaaagacgctgatcagccaagcccaccaagactgccgacgcttgccctcgctgttgaaggcataggggtaggcgtgcgcgtcgctgtcgatgtcgccggtcggctgggccacgcgagcctgatagtcggctttgaacgccttgaagtccttgtagacgacgtaggagaggtagcccgccacgcccagcgcgatcagagccggtgccagtttggaaacggtcacggcgaagcctttggctccagccgatccgacccctgccgcgctcaacatctcaacgaccggcgccggaatgccgtggaaatagcagtaggctccagccgccacgaccgcgaccgtagcggctcctgcgaggatgggcatggtggcaggagcagaggccacggacactgctgtcgccgacatctgcgacagaacgccagcggccgtggtgaaggccgatacgacgttcgctccgacataggtgccgcccagataagacccgccataagacaggatcgcgccgcccgccgcatgctggaccaaggcgagaccgcccaccgtcagaatcgccatttggcctcgttgtgaaaactgccgacatgagtttgcaggggcggtgtcataacagctatttcggaaggctcgggaatgccggaaagtctatcaggtccatcgcggccttgagcgtcgccaaatccaccccgcgtccatagcctcgcgccaccgagtttccgtccttgtggccggagatcaggtcgtgaacttcttccttcgcgttcgacatgcgagcggctcgcttccaactatgccggaacgagtggaagactttttgggggtcatccagcccttcgcccttcactttagcgacggcctcacaccagcgcccccaccacttgccgaactggtccgacattttcaccgcatcgccatcgagttcggggaacaacgatccggctttgaccccggcgacatactcaaggaagccgagggcgatcagtcggtcgtggatcgggatgatccgccgggccgagcggttcttcacccgacgcattcccttaagcggacgcgctgtcaggtcgatgaagctgatcccgttctcggtcttgatctccgacacgtccagcgacgccagttcctcgatccgcccgccggtccagagcgcgatgatcggaagccaatatttgtgatctttggtcactagagagccgggagcattccgatagccaaaggccgaggctgcaccttggaacatcggcgccttgaagatggccgctaagtcctcggcttcgtaaggatcgcgttcttcgctctcttccgccgatggcttcttcatcatgttggcggcggggttcttccgcatgaggtcgcgatccacggcaaactcgaagagggccttgtagacgacggtccagttccagacggtcttgatgtgaagcactcgatagtcgtcgcgcttctcggcttcggcgatggcccttacgaatggcgttttcgagatgtcccgtttggtgttcgggaatcgcttcaactcgatcaagaacgaatccatctggagcgccgtgatctgagacacgtcggggtcgccgaggaattccgacagacgggtcacatagccacggtgacgcttttcgctctttcccttcgccgcctcccaacggtcgaacaggtccaagagcttcatcccggcaacgggaccgagcggcagcgcaactggcggctccaccgtcaccggcaacacaggcgcgggattgggggcttccggtgcatccctcaggttgcccttccgatattccatgaccgtttgttcgacgctggccaaagcttcggcaaaccatccgcgtatgtttgggatcgctgggtgagccggatcgcacatgatcccttgaccgttcagagcgtccgacagacgagcgtcgaaatctgcgatcttcgaccagtctccggcccggaggtcaccgaccatctgaacgtgatcgcgcatcgtgtccgagaagccgaccggtgccggttctagttcgccgttgaaggccgcgtttagagccgtcttgatccgggccgaacgccagcgctggatagcggtaaaagcccggtcccgatcaatactttgacgctggaggggagccatggcctgcttcgcacgatcttgagccttggcgatctggtcggcccagtcggcaagaatgggagcgccaacccgaacagcttcgttttcgtccttggtgctgagggcgaccttaaattcgctctttccgaacaccgcccgtaggtccgtcggaatcaccttccgggcctcccaaagacccgaaacaccgctacggcgtagacctttcaccttggacgaagcgtgaatgcgttttcttcccattttggaccgaccttttggaccgaggtcgtcgtggaaatccttgcggagtaaggacttccaatgatttcaatgggattaaggcggatggctggggaactaggactcgaacctagaatgacggtaccaaaaaccggagtgttaccattacaccattccccagcaggtccggtgttccgccggcgcgtcagcgccggggagcggtcgaatacgccaagctatcggcggatgcaacaccctctgtgacgacaatttcaggcaatgcggggtctatttcattggtggcggaataggcgcttgcgggcgtttggcggcgtcgctataagccgcctcctcgatacggaagccgcccgcgggcgggccgatccggtgtcggagtgtggctcagtctggtagagcaccgcgttcgggacgcgggggtcgcaggttcgaatcctgccactccgaccatcttcctcccgacctaagtccttgtcgcgctgaacggcccggaacccgacggcgggtttgcgcgtctactgctccgctaagggcggagggattgatgaggattttggcgatcgccgcgtccgcggcgatgctgttgagcggcgttgcgtcgccggctcgcgcggacatgtctcaggccttcggcaacacggtcgtgtcgcactatccggacggcggctgggtgaagcatttcttcgagccggatgggcgctattcggcggtgtggtcggacggccgcaaggtcagtgcgcgctggcgccaggaaggcgagcgggtgtgcctgaacgaaatccgaccgcgcatgctgatcggccggttttgcacctccatggtcgcggccggcgtcggctccacctggcgatcgcgcgatcccatcggccgaaccgtgcgcaacgtcctggtggccggccgctgacggcttgtggcgatcgaacaggccgagaaccttttgtgccgtaggtgtgccgcgccatcttcggaaaggctcggatgttctcggtcaatgtcggaatggacgcccttgccggacagctccgatccccctagaacgcccgttctgcctgcatgcggatgtggcggaactggtagacgcactggatttaggttccagcgccgcaaggcgtggaggttcgagtcctctcatccgcaccaaggtcggcagacgtgaaaaaggccccggatcgctccggggccttttcttcgcttagaggccgatcagccgttgtcctgacccggcgtcggcgcgccgggcattggcggcaccggcacctgcggcgcgttcggatccagttccggcacttcgaccaggccgtgacgcatgtggctgtgccagaagccgtacccgaaatagagcaccaggccgatcgccgaccagatcggcagcaccagcttggcgtccaggggcaggttgaagaacagatacaggcaacccgccacagtcaggggcgcgatgagccacagcgccggggtgcggaacggacgacgacgatgcggatccttcttgcgcaggatcatgacgccgatagccaccatgaagaaggcgaacaaggtgcccgagttcgcgatgtcggccagcttgcccacggggaagaaggcggcggcgatcgtcaccagcacgccggtgatgatcgtgacgacgtgaggcgtcttgtacttgtggtggaccttggacaaggcgttgggcagcaggccgtcgcgcgccatcacaaagaagatgcgggtctggccgtagatcatcatcaggatgaccgaaggcagcgccagcatggcggcgagaccgatcaggttgccgatgttcggatgccccatctcgcggagcacgtgggccaaggcctccttggagcagctgaccggctcctggccgatggccgcgaggctggcgcagcgatccgccagagcctgcgagcccggcgccagaaccgcaccggcggcgtccgtcacaggctgggcgccgagcggagagccgatcacgcccgcggccaccagcatgtagaagacggtgcagatcagaagcgagccgatcaggccgatcggcacgttgcgctgcgggttcttggtctcctcggccgcggtcgaaacggcgtcgaagccgacataggcgaaaaagatggaggccgccgcgcccgcgacgccgagaccgcccgccgccgagacgcccgtcggcagaaagggctcgaaattgtccatgttcatggccggaatggcgagaatgacgaacaggctcagggcggcgaccttgatggccaccagcacggcgttgacccgcgcgctttcggtggtccccaggatcagcagtcccgtgaccgcgatggcgataagcgtcgccggcaggttgatgattcccccgccgccgaagaagccgcccgaggcccatgcgggcaggccgatgcccaaccagccctgcagttgcccttggaagtagccggaccagcccaccgacacggcggcccccgcaatggcgtattccagcaccagggcccagcccaccaaccaggccaggaactcgcccatgaccgagtaggtgtaggtgtaggccgagcccgacaccggcgccatcgccgcgaactcggagtagcaaagcgccgcgaccgcgcagaccgcccccgccaggacgaacgacagcatcatgcccggtcccgccttctgagccgcctcggcggtcagaacgaagatgccggtgccgatgatggcccccacgcccagcaacgtcagctgaacggctcccagcgaccggtgaagcgacttcttctcggccgtggccagaatcgcatcgagcgacttaacgcgccacatgaactatcccctcaggatgatggcggctccccggccgcgttggcgggacgctagacacggttgaggcggcgcgcaacgcgaatgacacgcggacgacgcggccgagacgctttcttgatgccgccaagccacgctatgggcgagcgatgttgccgatccacgacgttctccaaccgctgaaggccgcgcttgaggtcgggaacacggccgtgcttgcggcgccgccgggcgcgggcaagaccacggtcgtgccgctggcgctactggacgcaggctggctggacgagggcaagatcctggtgctcgagccccggcgcatcgccgcccgcgccgccgcggaccgcatggcggacatgctgggccagcaacccggcgccacggtcggctatcgcacgcgcctgcagagccgcaccggcccggagactcggatcgaggtcatcaccgagggggtcttcacccgcatgatcctcgacgacccggggctggacggcgtaggggcggtgctgttcgacgagttccacgagcgaagcctggacgccgatctgggtctggcgctggcgcgggaaagccaagggctgctgcggcccgaccttcgcatccttgtgatgtcggcgacgctggatacggcgggcgtgtcgcgcctgctgcccgacgccgtcggtcggcctgcgccggtgattgaagcgcagggccgggcctttccggtcgagacgcgccacctcgggcgcaatccggccgagcggttcgaggacgcggtcacgcgcgcctgcctgacagccttgcaggaggaaggcggctcggtgctcgtgtttctgcccgggcagggggaaatccaccggacggcgcgcctgctggccgatcggttgcgggatccgtcggtggatgtgacgccgctctacggcggacttgaccgagccgagcaggaccgcgccatcgagccctcgccggccggtcgtcgcaaggtggtgctggccacctccgtcgcggagaccagcctgaccatcgcaggggtgcgggtggtgatcgacgccggactgtcgcgcgtgccccggttcgatccggccagcgggctgacgcgcctggcgaccgttcgcgtcagtcggtcctcggccgagcagaggcgaggacgggcggggcggaccgagcccggcgtctgctaccggctgtgggacgaggcgcagacacgggggctggtggtcgatcagcgaccagaaatcctggaagcggacctgacgggtttcgcgctggacctcgccaggtggggcgcgcgatccacggacggcatggcgttccttgatgcgccccctgccggctcgctggccgaggcgcgggcgatcctgacgcggctcggcgccttgaacgccgagggcgtcctgacggagcatggtcggcggctgacccggattccgttgtcgccgcgtctggcgcacatggcggcggcggcgtcggacgcaggcgacgcgttgctgggcgcgcggatcgccgccgtcctcagcgagccgggcctcggcggttccgccgtcgatctgagcgaacgcctgtcgggcttcgagagggaccgttcggcgcgcgcgcaggacgcccgaaagctggccgagcgctgggcgcgcgcggccgggggcgggaagggcggcgaggtcgatcccgccgtgctgctggcgcaggccttcccggaacggatcgcgcgagcaaagggcaagccgggggagctgctgctggcgagcggccgcggggtcatggtcgatccggccgagcggctgtcggccgaaccctggctggcggtggcggacctcggcggcggcgatgtgcgcgatcgggttcgcctggccgccgggctcgatcctgagcgcatcgaaaccgatttccgccacctgatcaccgttgaggaccggctgacccgcgaaccctccggccgcgccagcctgcgccgtacccgccgcctgggcgccatcgttctggacgacgagatcatcggcccaccggatcgcgcggagctgaccagagcgctgcagcgggatttcgaaacgcgcggacttggcgccctgcgttggggcgaggcgagtacggcgttgcgggcgcggctgcggtttctgcatgacctttcgcctgagtggccggacgtgtcggatgatgcgctgacccaggcgcgtgagacctggctctggccgatgctggaagacgcgcaggggctggacagcgtgtcggatgcgaaactggccgaagggcttcgggcgttgatcccatgggatctgcagcggcggctggatgaactggcgccgatgcggctggcgacgccgctgggatcggccgccatcgactatgcggcggagggcgggccgcgcgtggacatccgggtgcaggaactgttcggaacgacccgacatccgacggtcgggggcgggaggacacccctgacgctggctctgctgtcgccggcgcggcggccggtgcaggtcacgcgcgacctgccgggtttctgggcggggtcgtgggcggcggtgcgcgccgagatgcgcgggcgctatcccagacatccttggccggaggatcccgctgcggcggccccgaccacgcgagccaagccgcgagggacgtgacggtcagccgatcagggcgtccgtgaccgcataggccatgacgcccgtcgccacggccaggttcaggctgtcggcccgcccgcgcatcggaatcttgacgttgacgtcgcaggcggacgccaggcgatcggtcagacccgcctgttcattgcccatcaggatcagcgccggggctttcaactcgcacgagcggtaaccggcggtcgcatccaggcgggggccgatcacgctgccgccccactgttcgcgccacgaaagaaaagcgtccggcgtggtccgggtgatcgagacggcgaacaccgatcccatggtggcgcgcacggcctcgaccgagaacggatcgacgcagtcgccgatcaggatcacgcccccgcagccggccgaatcggccgtgcggatgatggtgccgagattgccggggtcgcgaacctgctccagcgcgacccagcacggagagcgcgaggcgtccacctggtccagcggcgtataggtctgccggaacacgcccagcacggtctgagggttctcgcgtcggctgatcttttccaggatcggatgggtgaccagcaccacctcgccgccggccttggcggtctctgcacgggcgcggtccagcagcgggtggggccgcgcgtcctgtcccaccagcagcaaccgcggtgcatgaccctgatccagcgcctcgccgatgaacttcagcccctcggcgagaaacgtcccggtcgcgtcccgctgcttgcgcatgtgcagggcgcgcaccgccttgaccgtgtcgttggtcagggaggtgatcagccgatcttcgcccatcacgcgctccagcgcgcgaaaaaggacaggccgatggcgcgcggatcagggccgtcctccgacagcgccagctcgccccagtcgatccgacccgcgcgctccggcatcgcagccttcatcaggtgcgccagcgacaggccggaaatcctggccgcataggcgttcagcagcaggaaatcggcgtcgttcgccagaagggccgcgcagtcggcgagcaggctcggaatgtcgtcgaacagccgccacacctcgcccgtcgggccgcgcccgtacttgggcggatccaaaacgatcccatgatacttcgagccgcgcttgacctcccgcgcgacgtatttgcgggcgtcctcgacaatccagcggatcggacgatccgacagatcggactgctcggcgttctcgcgcgcccaggccacggacttcttggaggcgtcgacgtgcgtcacctccgcgcccgcggccgcaagcgccagggtcgccacgccggtgtagccgaacaggttgaggatgcgcggtcgctccagcttgcggacccgcgcgtccatccactcccaattcgccgcctgttcggggaaaaaggccaggtgccggaacggcgtgaaccgaccggtgaatcgcgcctccttccagctcaacgggaaggtctcgatcttggcggcgtccgggcggaagcgccagcgcccagcctcgtcctcgtcctcgggatcgaacacggcgtcggcttgcccccaggcggcgggctcacgcggcgaccacaggcattggggttcgggccggacaacggtgaagcggccgtaccgctccagcttctttccgtctccggaatccagcagggcgtagtccttccaccctcgggtgatgagcgtttccggcgtgggcgacaggacaggcatggccgccccataggcgttcaggcggcctgtcgtccagcgtcggcgcggttgatcggctcggcctcgtccgccatggcctcatcgttgtcttcgcgcctatggggcgtcttgtcccagacaaacggttcggagatcagccgccatgcggcatgaccgaacgccagggtcagcatggaccagtagacaggcgcggcggccatgtccttcagcgtgaatgacagtccagcccgccgggccccgacagcgcaggacagccaggcggacgcgacgccgccgaacatgacgacaagcgcgctgatgggcgtcaccggctgcatcccggcgatcgccgccatcaagaccgcggcggcgagccatccaagagccatcgcatgcgcggccgccgagatcagcgccgctcccagcgtcatcgcgagcgccagaacgcccttgaagcccagtccgtccaacgagcgcgtatgtaccccaagggtctgcatgtaccccttcagccagcgtgtgcgttgaggcagccagacctcaaggtcgccgggaggcgtctcgtacgttggacgccgggtgacgcccagccgccagccctcgcgccagaggcggaagcccaggtcggcgtcttcggtgacgttgtaggcgtcccagcctcccagcgaacgcagaacatccgtgcggatgtgattgcttgtgccgcccagcgggaagggcaggccgagccgcgccatgcccgggagcgtcacttcaaaaagcgaggcgtactccagcgcaaactggcggtcgaacatcggcgcccgttcacgcctcggatgccgacgaatgcgcaagggcgcttgaacgcagccgaggccgggctcggcgacgaagcgggccgcggcttcgcgcagctgcaggggatgcggttcgtcctcggcgtcatagatggtgacgacgtcgccggtcgcgaactgcagcgcatggttgagcgcgcgaggtttggtgcggggatcgccgggcggaacgatcagtatctcgagccaggccggccgtttcgccgcctcggccgcagcgatggtcgcctgatcatgcgcctcaaggaccagaaagccctgcaaccgatcttccggatagtcgatcgcggcgagccgtcgggccagctgctgaacgatgtcggcctcgtcatgcagggccgccagaacagtgtagcgcggccaggacagtggctcgtgaggcggctgctccggtctggcgctcgccagcgtcaggatgatacgccacacggcgcagatgatgaacaggctctgtccgaccaacaccagcaccagcccggtgaggtcgggatcgaggtagaagccggcgaccagcagggtcagcagcgccgtgaccatcaccgcctgcatgcgactcagaccaagacgccgcgcgccctccgcaaccgtcggcatcgcgtccccacccatttccaagctaacggctaggctgaagcggcggatcaagcaagccggattgcgggcgccacggccttgccgctattgcacgagctgatctgcatcggagctcgcccgcttgtccgacaccacccctcccgcaacgcgatcggcccgaaagccgaagggggaggggcattcccgccgggccgagatcctggaggcggccgagcgcatctttgtcgagcatggttatgaaggggcgacgatccgcaagatcgccgatgaggtgggcctgtcctcgaccgccctctacatgcatttcgccgacaagggcgaaatcctgctccaaatctgccgcgacgcgttcgacatgctgctggccagtgttcgcgaactggcggcgctggatgcgccgcccgaggtgcgcctgcgccggatgatcgaggcctatatcgacttcggcttcgcacagccgaacgcctatcgcctgatctatctgacgcggccgcttgaggcgcgcgacggcgcccagagcgcggctcaggaactgggcggcgagttgttcgcggccttcgaggaggtggtgcgcgaaacggtggaggccgggcgaatgagcggcgacgcctccacgacagctcaggcgatctgggcgtccgggcacggcgtggtgtcgctgatgatcaccaagccgtactttccctgggccgagcgagagcggcttatcggcgtgttgctggatgcgctgttcgccgggatgcagcggcggtgaaggcgccggccgtggcggtgctcggcgcgatctggcttctgccggcgtcagccgacgcgcgcccgctgcgtgtcctgtcgctggatcagtgcgccgaccagtacgcgctggcgcttgcgcctgacgccgagctcgccttgtcgccccgcgccgacgatcctgattcgcacctgcgcgccttggcgaaggggaggcgccaggtccggcccacgctggaagccgccacgacctttcagcccgacgtggtgatccgatactggggcggagagcccaggctgcttgcggcgctggagcgtcgcggcgtcaagacggccagtgttgaggacgtggcggacttcgacggcgtccgcatgaacattcgccgcgtggccgaggcgctggatcgtcgcgaagccggcgaggcgctgatcggcgacatggatgcaaagctggcgcgcggccgttcggaaatcggcggatcggcgctgtacctgaccgcgggtggcttcacggcgggttccggcacgcttatcgacgcggtgttcaaggcggccggcctccgcaatctggcgcccggcgccggatatcagcccttcagtgtcgagcgggtggtgctggagccgccttttcgattcgtcctggcctttttcgagcaggcgcgggccgactggcgcggcgccggccgtcatccgtccgtgcgcaaagcggcgcggacccggatcgtcgccagcctgccggcttcggtgctgacgtgtcccgcttggttcaccgccgacgccgtggtgcggttgagcgctggaagatgaggcctgcgcgtctgtctctgtgcctgggtctgggctgcctgatcgcgctcgccgcagcgatcgccttcggggagagcgctcttgatttgacccagtactcagcggccgtcggtgatcctgcatcgccccctggcgaagtcttgtggcaggtgcgcgcgccaagggcggtctgcgccatgctggtcggagcggcgctgggcttgtccggcgcggtgatgcaggggctgctgcgcaaccctctggccgatccgggggtgctgggcgtctcggccgtatcggcgctggcggcggcttgcgccattgtcgcgggcggcgcggcctgggccggcgttgtggagggctcggccctgatcgggaccctgctggcgggcgccgccctggcgattgcggcgagccgtctaagatccccggaggcgctgatcctcttcggggtggcgctgtccagtttcgcgggcgccctgaccgcgctgattttcaacctttctccgtcgccgatcgcaacggccgaggtgatgagctggctgctgggctcggtgcagaaccgcagctggatcgacgtggcctgggtggcgccggcgctggcggtcgcaagcgtgctggccgcacggacgtcgccgggcttgaggatgctgtcgttgggcgaagaggcggcggcgacgtccggcctgtccatgcggcgcttcaaggtcttggcgctgctggcgacggcgcttgcgaccggcgccgcggtggcggtggccggcgtgatcggcttcgtggggttggccgcgcctcatctggtccgaggcgtggtgcgcggcgatcccgggcgggttctgcttccctcggcgctggccggcgggctgatgctggtcgccgccgacctcctggcgcggatgatcccgacggaccaggagctgaagctcggcgtgttcaccgccctgatcggcgcgccgctgttcgctctggtggcgtggcgggcggcgcgagagtggcggctgtgagcgccgtcgaactgaggagcgtctcggcgcgggtgggcggcgcaagggtgctggaggcggtcagcttgtcggcggcgcccggagaggtcgtcgccctgtgcgggcccaacggcgccggcaagtccagcgtccttcgcgcagcccttgggctcctcgcggtgcaggagggcgaggtcattcttggcggcgcgccgttgaacaccctgtcggcgcgccgtcgcgccgaatgcgcggcctatctgccgcaggacggccgcatcggctggaacatgccggcgatcgaagtcgcagcgcttggggcgccctttctggacgcagagaccgccgtcacccgcgcgcggcaggcgctggaccgcgtaggcgtcgcccatctggcggatcgcggcgtggccgacatgtcgggcggcgaacgggcccgggttctgctggcgcgcgccctgacgacgggcgcagcgacgctgctggccgatgagcccttggcgggcctggatccagaggctcagttgctggtcgccgccgtgctccgccaggaggcggacaggggcgcggccgtgctgaccagcctgcacgacctcggtctggccgcccgtctcgccgacagggtcgtggtgataaacgggggacgcgtcatcgcggacggcccgccgctcgaggcgctgcggcccgaagtgctgcgcgaggttttcggcctcgatgcgcggtggatcgaggccgacggcgcccccctactggcgatgcgccgggccgtctagtcgtgtcctactggtaggcgcgaggaccgttggagccccgcgccaggtcggcagatggcgtcagcggtgccgagccgccgttcagccgagcgcggtagacctgaagattctccatcacccgcatcatgtagttgcgcgtctcggtgaagggcgcgcactcgatgaagtcgacgggatcgacctgggcgccgcgcggatcaccgcaccgcacgatccactgcggcggacgcgcgggaccggcgttgtagccgacggtggtcagcagcatcgagcccgagaactggttcatcagttcgcccaggtgatagctgcccagcgtcatgttgtagtccgggtcccacagctgctcggccgagaagctcatgccgagccggcgcgccacgcccgaggcggtggaaggcaggaactgcatcatgccgcgcgcgtcggcggaggagcgggcgcgcgggtcgaagctcgattcctggcgcgtgatggcctgggtgaactccagcggggcggcgcccgcgacctgcggcggcacgcgcaccggatacatgcgctcgggcatgacgatgccgcgttggctggccgcgcggcccaccatcatggaggtgaactgttcgccgtagccgcgcgtcaggtccatcagcaacgctaggtcgccggcgttcggcaggtcgtcgtcgagttggtaggcgaagacgcgcagcaggctggtttcgcccgtctcgccgagaatacgggccgcgcgcaccacctcattggcctcgaaccgcgcgacctcttccggcgacgggtcgggatcgccgggcagggtcagggtcgagacgcccgccttctcggccgccaactggccatagaaggtctgccagtgctgggcgccggcctggtagaactgcatggcgcgagcctggtcgcgctgagcctcggcggtccgccccagccagtagagggcgcggccctgcgtgatcggcgtggacgaggctgtgcggagcgtctcgaagtggcgcgccgccgtcgccggatcgttcagcttggtcagggccccccagccggcgaagaactcggcgtccaccatccggtcccccgagatgaagccgtgcccgttcatggagtcataggccgcccgccagttccgcgcttgaagggcgtcgaggaagtagttgcgccgctcgctccatagcgtcgactggccttcggcgtggctgggcgccgggggcagggcggccagaaggctgaagccctcggactgccggctctgagagcgcaggatgcgcgcgcgctccagcgccacggccggatgggcggcctgggccggcgtcagggtggcgaccacggcgtcgggactataggccgtgcgcaggctcaacaccgcattggctatgttggcgcgctctggcgaaacaagcgggatcatggcgcgtgtggccgggccgtgtggaccgctgagcagcatgttcagacgcgcttcgtggtccgcctgcgtcagccagccgccccagcggccctggatgcggctctgctgcgcctcttcgaaggaccgggtccgccaccaatcgcggatcagagcctgcgcctccatcgagcggttccgctgctccagcgcggaggccagggcgatggcgccctgcgctgtctggggttcgccgccgtcgaagaaggccagcgtctcgtcggcgcccgcaccggcgagatcaagcgcacgctcgcccgccgcctgccgcgactcgccgcggggccaggccgccatgtcgcgtttcgcccgcactagttcgacataggacagctgctgcgccgaagtgtcgatcagcgcccattccaccagcttgcgggccgtgggatcgccgatctgctgcagggtcgagcgggtgcccgccacgtctcgcgcccgagccgatgcgagaccctggcggaacagcgccgtgtcctgatcgttcagcacgcggccctgataggtcgcgccgggcgcctggctgctgtaggccacgggcccgcccgacggcagaacgtcctggggcgtgggcgcaaggatggccaaggcggccgcaaggctggtcgcgatcatgaagtgtcctgttcccattcatcccggttgcggcggggccgccggcaacctaccctccggcgctccgaaagcggcgcgtgacgccaaccccctcgcaggcaagaagtttcaatgaccgcccccttgttcaagggcgtgatcaccgccctgatcacaccacttcgtgacggaaacgtggacgaggacgccttcgtcggactgctggagcgccagatcgccgcaggcgtccacggcgtcgtcccgatgggcaccacgggcgaaagcgcgaccctgtcggcggaagagcacaagcgtgtggtcgagctgtgcgtaaagacgtcggccggacgggtgcgcgtggtcgcgggagcgggcgcctctgcgacggacaaggcgatcgacctagcgcgtcacgccaagagcgtcggcgcggacggcgcgcttgtggtcacgccctattacaacaggccctcgcaggcgggcatggtcgcgcatttccgcgccgtcgccgatgcggtgcagctgccgatcctgctctacaacgtgcccggccgcaccggcgtggatctgtccgacgacagcgtcatcgcattgtcggagcatccgaacatcgtggggatcaaggacgccaccggcgacctgtcgcggatcagcgtgatgcgcgcggctattcacggccagttcgactatctgtccggcgacgacccgtcgtggctggggtacgccgcgcacggcggccacggcgtgatctcggtgacgtccaacgtggcgccggagggcatggtcgccttgcacaacgcgatcacagccggcgacttcgccacggcccggacctggcaggaccggctgatcggcctgcacaaggggctgttcctcgacaactcgccgtcgccgacgaagtacgcgctgtcgcggctgggcctgtgctcggaggaggtgcggtcgccgcttgcgccgacggccgaggcggtgcggccggccatcgaccgggccatggccgatgcgggcgtcgcctgatggccgcgtctcaacccaaatccaaaaccatcgccgagaaccggcgcgcccgcttcgactacttccttgaggataacaccgaggcggggctggtgctgaccggcaccgaaatcaaggcgctgcgcgacggccgggccaacatcgccgagagctatgcggcggtggaagggcgcgagatcgtgctgatcaacgccgacatcccgccgtacaagcaggccaaccgcttcaaccacgagccgcgccgcccgcgtaagctgctgctgcacagaaagcagatcgaccgcctgatcggcgcggtccagcgtgacggccagaccatcattcccctacgcctctatctgaacgaagacggcaaggccaagctcgagatcgcgctggccaagggcaagaagctgcacgacaagcgtgaagcctccgccgagcgcgactggcagcgcgacaaggcgcggctgctgaaagagcggggctaggaggtcaggcctccagcagtatcctagccctgcggaacaccgcctcgaacatctcgggcgtcagacggccggtgttcgtgttgaggcgcgagcagtgatagctgttcaggatgacatagccgccggcctcgccctccgcgccatggccagccggcatggccgtgccgggtcgtccgaaagccttcaggatgttacggcgcgaaacatcgcccagcgtcacgatcaccctgaggcggggcagggcggccaaccggtcgataaggaacggcctgcaagtcgtctcctcgatcggcagcggcttgttgcctggcggggcgcagcgcaccgcgttggtcaccatgcagtccaccagttgcagcgtgtcatccagacgcgcctcgtagtcgccccgcgcgaagccggtcttcttcagcgtctcatacagcagccagccggcatgatcgccggtgaaggggcgccccgtccggttggcgcccatgcggccgggggcaagtcccgccaccagcagccgcgcatccgggtcgccgaaggagggagccgggccgttgaaccagtcggggttctggcgggcgttctcctgccgataggcgaccaagcgcggacagcggggacaatcgcgaggcggctcgggggtcaggctcatgctcaggcgctctttatccggccgaactcggccgtgaggtcggcgagatcgaggtagtggtcggcctggcggcgcaattcgtcggcgatctgcggcggctgggtcttcagggtcgagacgacggtgacgcggacgccgcgccgctgcaccgcctccaccaggcgtcggaagtcgccgtcgccggagaacagcaccgcgtggtcgatgtgcggagccagctccagcatgtccactgcaatctcgatgtccatgttccccttcagccggctgtggccctgtgcgtccgtgacgcgcttcgtcggcttggtgacaacggaaaagccgttgtagccgagccagtccaccagcggccgcaccgccgagaactcttcgccctcgaccacggccgtgtaataactggctctcaccagccgcgaacgggcgttgaaccagtccagcatgcgccggaagtccagctcctgatgcagggcgcgggctgcggaatagaggttggcgccgtcgatgaagaccgcgagccggtcgttggagtggaagggcatggcgatgtccggcgaagcgaaaggtcccgatccgacgacggccgctgtcgcgttcgacgattcggatctggagaaggcagtcatcgtggcgctcggctgcaatgacaagggggcgtggtcgtcctgccatgaggcgctggaggccgcgctggcgcggttccgtccggaggggctggacgtgacggcgcgttcgtcgtggtggacgtctcaggcctggcccgacccttccgacccgcccttcctcaacggggtagccatcgtgcagaccgatctggacgcgccgggggtcatgtctgtgctgggtcggatagaggatgcgttcggccgccggcgcggcgcacgcaatgcgcctcgcacgctggacctcgatctcgtcgcctatgcacgtttgagcggggatttcggcgggctgatcctgccgcacccgcgcgcggccgaacggctgttcgtcatgggacccctggcggagatcgccccggcctggcgtcatccggttttgaactcgcgctccggcgacctggcgcggcaggctttggtgggccgtgacgcccgcgcggtctgaaagccgcacttccgccgccttgacgttgcaaaaacagggctctgtctgtatttgacgcgactcttcacccgcgtccgaaggattgtcatggcccgcgtcaccgtcgaagactgcatcgagaaggtcccgaaccgcttcggcctggttctgctggccggtcaccgcgcccgcagcatcgccaacggcgcggccctgacgctcgaccgcgacaacgacaagaacccggtcgtggcgctgcgcgaagtggccgaggacaccgtgcgtcccgacgaactgcgcgaaaccatcatcaccaacctgcagcgcgtcgacgagcgcaccgaggccgaggacgaggccgagacagtggctctgctggccgagccgcagcacatgaacatgtccgaggccgaattgatccgcgcgctgcaaagcgacaaggaaggcggccaggaggagcgctactgacccccgacgggtcaaccggcgtcaccattctgccggcgcggaccgacgcggccccgccggcgccctctcttgcgaacacgatccgaccggccgacggcggcgcgcccgccaagcgcgcgccggtcctgcgtcagttcgagttgatcgaggccgtcaaggcctatgaccccaccgcagacgaggctgcgctgaaccgcgcctatgtttatgcgatgaagatgcacggctcgcagctgcgggcctccggcgatccctatttcgcccatccgatccaggtggccggcatcctgaccgactatcggctggacaccgccacaatcatcaccgccctgcttcacgacgtggtcgaggacacctccgccacccgcgacgatatcgccggcatgttcggcgaggagatcgccggcctggtcgagggggtgaccaagctcagtcggctggagcttcaggccgagcggacgcgccaggccgagaacctgcgcaagttcatcctagccatcagccgcgacgtgcgcgtgctgctggtgaagctggccgaccgcctgcacaacatgcgcacgctccatttcgtcaagccggagaagcgcgagcgaatcagccgcgagacgctggaggtctatgcgccgctcggccgatcgatcggcatccactccatcgcctccgagctggaggagctggcgttcgagcacctgaaccctacggcccgcaccgccatcgagcgcaggctggaggccttgaagcttgagcacggccgcgccatcgagggcgtgtcctcagaggtcgagcgggtgctggccgaaggcggcatccccgcgcaggtgaagggccggcagaagacgccgtattccatctggagaaagctgcagaggaagtcggtcggcttttcgtccctgtccgacatctacggcttccgcgtgctggtggatgccgaggacgactgctaccgggcgctgggtatcattcaccgcgcctggccgatggtgccggagcggttcaaggacttcatctcgacacccaagtcgaacaactaccgctcgctgcacacgactgtggtgggtccgtcgggcctgcgcatcgaaatgcagatccgcaccgacgccatgaaccgcgtggccgaggacggggtggcggcgcactggtcctacaagaaccagtcctacggcttggaccgcgaagccatgcaggccgacggcggacgcgatccgctgcagaacctgcgccatctggtgcaggtgatcgagcacggcgagggcggcgaggactgggtcgagcacgccaagctggagatgtatctcgaccaggtcttcgtgttcacgcccaagggcgcgctgatcaccctgccgcgcggcggcatgccgctggatttcgcctatgcggtgcacaccgaggtcggtgacacggccgtgggggtgaagatcaacggcgaactgaagcccatgcgaacgccgctgcagaacggcgacgtggtcgagatcatccgtggagcgaagcgcgaggccccggccgactggcgcaacctgacggtgaccgggcgcgcgcggtccgccatccgccggcatatccgcaccaacgaacgcggcgagttcatccgcctgggtcgcgcggcgctggagcagacgctgagccgggtggacaaggcgctggccgacctgtcgctgaagccggttctcgagacgctggccgttgcaagcgaggacgacctgttcgaggggttggggcgaggccgcctgtcgccagcggcggtggcggagaccctctttccggccctcgctccccgtctgcgcggcgggcccgagaagcagcggatcgaaagctccaaggctcggctgttcgtgcggggcggcggcctgacgcccggcgtcaccatgcatttcggccagtgctgcacgcctgtgccgggagaccgaattgtaggcatcctggagccggacgcgggcctcacggttcacaccatcgactgccagaccctggcgagcttcgccgacgacgactcggtctggcatgatctgcagtggacgccgcaggcggagaccgaggcggtcgccgctgtgcggcttcaagccaccatgcgcaacgcgccgggggtgctgggcgaggtggcgaccctgatcgggcaggcgggcggcaacatcatcaacctgtcgctggcgcaccgacagcaggacttcttcgacgtcatggtcgatgtagaggtagaggacgccaagcacgcgacgaccatcgtcgccgccctgcgcgccaacccttccgtggacgccgtggaccgggttcggggctgaacgggcttcaacgccgcgcgcgaaggcgctagagcggagccatgaacaccgaagacgtcctgaacgagttccgccaggccaacgcgctgcgcgagggtcatttcgtcctgtcctccggcctgcacagccccgtctttctgcagaagaacctcgtcttcatggacgcgcgccgctgcgaacggctgtgcaaggcgctggcggacaagatcacggcggctgcgggcgcggtggacgtggtcatctccccggcgggcggcggcatcattcccggctacgagacggcgcggcatctgggcgtcccgtccatgtacgtcgagcgggaagggggcgtgttcaagctgcgccgcggcttctcggtcgagcccgggcagaaggtcgtgatggtcgaagacatcgtcacgacgggcctgtcctcgcgcgagtgcatcgcggccatccaggccgtgggcggagaggtcgtcgcagcggcgtgcatcgtcgatcggtctgggggcaaggccgatgtcggcgtgcctttgatcgcgctggccgcgctggaagtgccggcctatgcggccgacgccctgccggctgaactcgcggcgctgccggtcgaggatccgggcagccgccgtctggcgaaaaccgcctgatgcgcgagcgggtccgcctgggggtcaacatcgaccatgtggcgaccgtgcggaacgcgcgcggcggcgcccaccccgacccggctcgcgcggcggaggcggcgctggtggcgggggcggacgggatcacggcccacctgcgcgaggatcggcgccacatcacggatgcggacatcaatgtgctgagcgccctgtgcgcccgcgctgaccgcccgctgaacttcgaaatggcggtgacggacgagatgctgtccatcgccctgcgtcatctcccgcatgcggcctgtctggtgccagaacgccgtgaggaggtcacgaccgagggcggcctggcgggttcgggacacgaagcccggattgagcccgtcgtccgggcgctgagcgcggccggcgtgcgggtgtccttgttcatcgaaccggccgaggatcaggtcgaggcggccaaggccgtcggagcgcaggtggtggagtttcacaccggccgctactgccacctttccggcggcgagcgcgaggtcgagttcgagcgcctggccgccgccgccgcgcaggccgacatcctgggcctggaggtccacgccgggcacggcctggactacgacaccgccccgcgcatgctcgcgatccccgaagtgcgcgagctgaacatcgggcacttcctgatcggcgaatcgatcttcgtcgggctggacgccgccatccggcggatgcgggccgccatggacgcggcggcatgatcatcggcgtcggcgcggacctgtcggacattcgccgcatccaggcgtcgctggatcgcttcggcgaccgcttcaagcagcgatgcttcaccgagctggagcgcacgcgctcggaccgcaagccggatccggcttggagctacgccaagcgattcgccgccaaggaggcctgcgccaaggcgctgggcaccggcatgcgcgccaacgtctattggcgcgacatgggggtggtgaacctgcgctcgggccagccgacgcttgcgctgaccggacatgcggccgagcatctggcgcgactgacgccgaccggccaccatccgcgcatccacctgacgctgtccgacgaacatccctacgccctggccttcgtagtgatcgaagccttgccggtgtcgtaatcccgctataggcgtcgcacacgaccgtcgttcaaggcggcgaaggatttcaagaaccgcatgagcgacgaccgcaagccccacggggcggcctccgacccgaccccggaacaggcgttcgccgcatccgaggccgacatgccggcgagcgccgctcgcgccgatcgcgaccagccggtgttcgaccgcaaggcgcgccgccgcgaggtcgcgggcaaggccggcagcgagaccgccgaggtcgtcaagaccatcgtcttcgccctgttgatcgccatggtgctgcggatcttcctgttccagcccttcaccattccgtcggcctcgatggagccgaacctctacgagggcgactatatcgtcgtgtccaagtggtcgtacggctattcgcgccattccatcccgttcagcccgccgatcttcgacggccgcatcatgggcaaggccccgcagcgcggcgacatcgtggtgttcaagctgccgcgcgacaacaagaccgacttcatcaagcgcgtgatcggcctgccgggcgaccgcatccagatgatcgccaacaagctgcacatcaacggccagccggttgacgacgtggtggtgcgtcagggcgagatcaacgacatcttcggcccgcgccccgtggtgcaggcgcgcgagaccctgccgggcggccgcaccttcatgacgcaggacttcggccccggcggcgatttggacgacacgcccgtgtacgaggtgccggccggtcagtacttcatgatgggggacaaccgcgacaactcgatcgacagccgcgtcgagcagtccagcggcgtaggcctggtgccggaagagaacctcgtcggcaaggcgcaggtgatcctgttctcttggaagcctggcgcgtcgctgtggaaccccggcacctggttcaacgtgcggctggatcgcttcttcaacgtcctgcactgatggccaacatcagggcagaggcggtcgaggcgctgcaacgccggatcggctacgtctttcgcgaccgcgcgctgctggaccgcgccctgacccacgccagcgtgggggagggcgccgcgcccggcgcgcatggctcgcgcgacaacgagcgactggagttcctgggcgaccgggtgctgggcctgctgaccgccgagcggctttcggcggactatccgctggccgatgaaggtcagttgtcggcgcggcttcacgcccttgtcgacaaggccgcctgcgcccgcgtcggcgaggcctggggcgtggggcccgcgctgcgtctttccgccggagagaccaagacgggcgggcggcgcaaggccggagtgatcgccgacgcggtcgaggcgatcctggccgccgtctttctggacgcggggctggacgccgcgcgttccgtgttcgccgccgcctgggccgaggagttggctgcgccgtcgtcgcgcgaactcaccaaccccaagtccgccttgcaggaatgggcgcaggggcaggggcggccgctgcccagctatcgggtgaccgagcgcgccggctcggatcatgccccgacattcacggtggaagtcggggttcagggcgtggagcccttgaccgcaaagggccgttcgcgtcaggacgcggaaaaggcggccgccgtcgccatgctgcagagagaaggcgtgatttgaccgacacccaccctgagacccagcgcgccggcttcgccgccatcatcggcgcgcccaacgccggcaagtcgacgctggtcaaccggctgacggggtccaaggtctcgatcgtcacgcagaaggtgcagaccacgcgctttccggttcgcggcatcgccatcgagggcgacgcccagatcgtgctggtggacacgcccggcatcttcacgccgcgccgccgtctggatcgcgccatggtggcctccgcctggggcggggcggaagacgccgatgtggtggtccacctgatcgacgcccagtcgcacatcgacgccgagggtcgcgacggcacggctgccgaccgccgctcggccgaggacaccgagaccatcatcgccaacctgaaggcgaccggaaccaaggtcatcctggccttgaacaagatcgacgggatgcgccgcgacaccctcttggcgctgtcgcagcggatgttcgaaaccggcgtctacgaagaggtctatatgatctccgccttgagcggcgacggcgtggatgatctcaaggcgcgcctcgcccgatcgatgccggaggggccctggctctatccggaagatcaatccgccgacgtgccgatccgggtgctggcggccgagatcacgcgcgaaaaggtctacctgcgcgtccatgaggaattgccttattcggcggcggtggagaccaccagcttcgaggaaaagcccgacggctccgcccggatcgagcagaccatctatgtcgagcgcgagagccagcgtccgatcgtgctgggcaagggcggccagactgtgaagtggatcgggcaaaaggcccgcgaggaactgaccgagctgctggaccgacccgtgcacctgttcctgaccgtcaaggtcgatccgaaatggcaggacagccgcgccctctacgcccagttcggcctcgattacgacgtctgagttcccgtgtttcacgttccccgctatgccggcggtcacccgcgtcttgtgctcgtcctgatcttcggcggccttctgatgctcgccggcgcggtgggctggtggtcggccaagaccccgatgcacgacgccgctctggccgcgagccgtcgcggcgagctcgcgcctcggccgccgctggtcgtcgtcgaagaccttccgcaactaaccgagcggctgaaccgcgaagccgcggccggtcgcttcatgggcggcgtccttgtcgccaaaggcgaccaagtgctgtttcgccaggtctacggcatggcgaaccgggagcaggggcgggcgatgcagctgaactcgcgcttccgcctggcctcggtgtccaagcagttcacggccgccgccattctgaagctgcaggaccaaggcaagctgcggatcgacgatccggtgtgcaagtggatccagccgtgcccggccgcctgggcgccgatccgcatccaccatctgctgtcgcacacctccggcattcccgacctgatggcgcgtccggcatggggattggggcgtgtgactccgatcacgctggagaagctgaccgaagattcaaagctttacgggcttcagttcacgccaggatccaaggtgcgctacaacaatgcggccttcaatctcgccgccgcggtcgtcgaaaaggccagcggtcagccgttcgctgattatctcgaaaccgccttcttcacaccgctgggcatgaaggacacgggcgtcgatctggacgggggcgaccatgggatcatcatgggctacgccaactttcccggcggtctgacgccccagccgaacgccaacgtctccgtggtggcgggggcgggggcggtttattcgacgctggacgacctgctggtctggaaccgcgccctgcatggcggccggctgctgacgccctacagttatgcgcagatgatcgccgaccacgcgcccgccgacacgcccagcgagcgcggtcgcccgcaccgtgactatggatacggcgtcttctcgagccgccttggccagcaggtcacgcccgcctttgaagaccgccagatttaccatacgggcagctggggcggcttccgcaatctgatcagctatcagccggatcaggccgtgacggtgatcgttctgtccaacaactaccatctgcgcgaccaggtgtttctgctcacccagcagggcatggccgaggcgctggggcggccgtttccgacagggctgcaccgctaggatcgctggatggatttccacgaagacgcctttgttctgtcggcccgagcgcatggcgacaccggcgtcgtcgtggacctgctcagcgagacgcacggacgacgcgccgcctatgtggccggcggcgcatcgcgcaagatgaaacctttcctgcaggctggggcgcgggtgcaggcggactaccgcgcccgcacctccgatcatctgggatcggcccggctggaggcggtgggcgagggtccaagcggactgttcgacgacccgctggcgctgatcggcctctcggccgccgcggccgtggtccagggcgcgctgccggagcgagagccgcacccgggggcttttcttgcgttcgaggccttgatgaccgcttttcaggcgccggatctctggccggcgatctttgttcggttcgagatggggctgctcgaggatctcggctttggactggatctgacgcgctgcgcctcgacgggctccgtcgatgacctggtctatgtcagccccaggaccggacgcgccgtgagccgggaggccggccagccgtacgccgaccgcttgctgcgtcttccgccattcctgctgggcgctcaggctgggctgcgcgcgggcgatgtcggcaccggcttcgacctgaccggacacttcctggaagccttcgtgttcaacccgcagaaccggccgctgccgccggcgcgcgtgtggatgctggacaagctcagggacgctgaccgactttaggcgaatagtcgatttcgcataatatatcttaggcgcttcgcagcaggatgagtcagcgttcccgcgccgccgccaacttctccttcagcttggtcctcttcaggtcatgttccgtggtgagcgcgaggcgttgctgctccagggcgttcatctgctcgtcgatctcgcgcaaggcgtcgtcgtgcttcttgtccaatgcatcaagtttcgccttcagcgccttgatgagccttgcgttagtatccgcaggcgccttcgacttcggtttggctggagcgatccgcccgacgtcgatggcttcgcctcgctgtacgacctcgccgggcctggccatggcagcgtcgtagtcaggtccggcctcgacctcatgagccagtcccgccttgaacaggtcctgtccgacgccccatgcctccagcgccttgggccgagacgtcgtggcgacgctgaaggcgtgaaagccgtctgaccaggaaaagaccttcaaacgcgccaccgtcacctccaggaccgctgaaccatacttccttaaacgcaccggcctatccaatgggggcaatggccgtcgttcatccatcgcgatccggcgagatcgccgatccgccagcctgggaacggctggcggcgggcttcgtgctgttcatgctcacgggcgcgctgctggctccggtgctggcgccggaccagtcggagacgccgatcctgcgcctcacctggttgccggtctatgcgctgaccgccggccttatggccctccggttcgaacggatcatcaaggcctggccggcctggctgctggcgggactgctgctggcgctcgccttcgcctccaaatactggtcgatcgacccggaggtgacccagcggcgcgtcatcgccatggccatcaaccccagcttcgcgctctatctgggtgcggtgttccgggacagcgccctgccccgcctgttgatgcagacctgcctcgtcatggcggtcggcagcctgatcatggtcttcgcctatcctcagatcggcgtccaccaggccgacaacgccggcatgtggcgcggcctgtggtacgagaagaaccagatgggcctggtgatggtggtcggcgcagtgtcggccgcggcctgcctggccgccggcgatcgtcgaccttggacggcgctgatcgcgttgggactgtgctctcttttggtcctggccagccagtccaagacctcgctgttgtgtctgctgctgggggcgggccttgtgggcggcctgtggagcctgcgacgcggcggtgcggtgctgacggtggcggggctgtggggcggcgtgctgctggcgggcggcgcggcctggatctggttcgtggattcggcggcggtgctgacggcgctgggcaaggacccatcgctgaccggccgcaccctgatctgggaaagtctgatgcgtcgcgtggccgagcggccttggaccggctacggcttcagcgccttctggggccgcgactcggtgcccgccgcattcgtgcgtcaggagacggcctggccggtgccttcggcccacaacggctggatcgatctgctggtgcaactgggatggccgggcgcagtggccgtgggcgtggtgatcgccgtggccgtggtgctggtcgtcttgcgcctggacgggatgggcgcgcgcgagggctattggagcggcgcctacctggcggtgttcctgctgttgagcctttcagagagtgtgttgctcaaccacgccagcctgccctggacgctgatgctggcgatactttcccgcgcggtgatctttgacgccccacagaaaagcgcggcgcttgcccgcgcgccgtccgaggcttacgggaaccggctccgaatcgcctcagactatgtgaatggcccatcccgccgacgacctgttcgcctcctttgatccgccctccccgcccgccaaggcgcctgcgcctcagccggtgaagcccacggccgccatcgccgcggcggccgaagccgtgacgcccgtcgccgctcagccctccgccacggcaggcgccgccggcgcctactccgcctcctccatcgaggtgctggaagggctggagccggtgcgcaagcgtccgggcatgtacattggcggcacggatgaacgcgccctgcatcacctgttcgccgaggtgctggacaacgcgatggacgaagcggtcgcccgtcacgccaagctgatcaccgtcgacctggacgccgacggctacctgtcggtccgcgacgatggccgcggcattccggtcgatccgcaccccaagcaccccggcaagtcggcgttggaggtggtgatgaccgtgctccactcgggcggcaagttctccggcaaggcctacgagacttcgggcgggctgcatggcgtcggcgtgtccgtggtcaatgcgctgagcgagcatctggacgtcaccgtttggcgcgacggctttgaatggaggcagtcgttcagccgcggtcacgtgctggcccccatccagcaggtccagccgtccaaaaagcgcggcaccctgatccgcttcaagccggacgaagagatcttcggcgtgggcgcggcgttcaagccggcgcgcctgttccgcatggcccgttcgaaggcctatctgttccggggcgtggaaatcaaatggtcctgcgcgcccgagcgcatcaccgaccagacgccgccgcaggccgttctgcactttcccggcggcctggccgatgcgctggccgaccgcatcggggagctggagacggtgacgcccaccttcgccgggcggatggagcgcaagggcgaggcgggcgcggtggaatgggcggtgacctggtcgccgatcggctttggagaggccgacggcttcgtcagctcctactgcaacaccgtctcgacgcccgacggcggcacgcatgaagccggattccgcgccgccctggtcaagggcctcaaggcctatggcgaactgatcaaggaaaagcgggccgaggtcatcacggccgaggacgtgatcgccaacgccggcgccctgatcagcgtcttcatccgcaaccccgagttccaggggcagaccaaggatcgcctgtcctcgccagagggcgcgcgcatcgtcgagcagctgctgcgcgatccgttggaccactggcttaccgagagccccaaacaggccaacgccctgctcggcttcgtcatcgaccgggccgaggatcgcctgcgccgtcgcaaggacaaggaggttcagcgcgccgcggcgaccaggaagctccgcctgccaggcaagctgtcggactgcagccgccaggccgccgagggcacggagttgttcatcgtcgaaggcgattcggcgggcggctcggcccagcaggggcgtgaccgcacgacccaggcgatcctgccgctgcgcggcaagatcctgaacgtcgcctcggccaccgtcgacaagctgcgccagaacgtggagctgtccgatctcgcgctggccatgggggtgcagcccggcgcgcgcttcaacatcgacgacctgcgctacgagcggatcgtcatcatgacggacgccgacgtggacggcgcccacatcgcggcgctgctcatcaccttcttctatcgggtcatgcccgagacgatccgtcagggccgtgtgttcatggcgctgccgccgctgtatcggatcagcgcgggccctctgagcgagtatgctcgcgacgacgcacaccgcgaagagctgctgaagaccgtcttcaagggcaagaaggtcgagatcggtcggttcaagggtctcggcgagatgatggcgtcacagctcaaggagaccaccatggatccgaagaagcggaccctggcgcgcatcaccgtgcctgacgcagaaagcagcatcgaggatctggtcgagcggctgatgggcaaacgggccgaggcgcgcttccagttcatccaggagaacgcccgattcgccgttgaggacctggacgtctagccggcgtttcgatccagccaggccccgacccgcgcctgggcgtccagctccagatcgccgtagaacaggctgtagggcggcgtcttgcggcggtcggcccagttgccgggcgtacgggacgattcctggctgggccgctcaaagcgcagcagtccgtcgcggcactgcgtggcgacggcgcgggcgatcaacgcaggccgcgcctcccactccagccccgtggcgttggtggcgccgtgatgcaggcggctaggaacaggcgccgtgtcgcttgagccggtcaccggattgacgcacaggggcgcacggcccgcgcgctcctccaactggccccgcccatcgaacaccagcgcgctctccagcctgcgcctcgcggcagcatcgtcatcctccggaacctgggcccagccaacgacgcagccggcttgatcccgacggctgcaggccggcacgtcggccggcagggcgtcggcggcgacaagcgtatcaatcagataggcggcggcgacgcgcctgcgcagagccgcgtccggcgcgatacgttcgcgcagcagacgatcgatcaattcgccgccctgctccacccccgccaggatgatggggccgtccgggtgtcgtcccagccaggcgtcgaacgcccgctccacgtcctcataggcgaagctgcgggcctcgcgggcgtcgtctcgcggcgtcagccgtgcgtagaggctggcctggcggtacaggggcgcgctgacgtcgcccgcgcgcgcaaagggcgcggcgtagttcggcaacacgacccggcgcagataggccagggcctcttcatcgtccgtgacgccgttccaaccctcgccgccgtcgtaggtggtggaatgcacaaagaagaccgacgcggggccggcgcctcggctccgcacgtcgcgcatggcccatgcgccggcttgcgcatagtcgggcgcggccggcggctcataggtctggaaggggatgcgagggttcaggcttgatcgcacgatggctccgccgaacaccgccaccagaatggtgaacagcgccaccagcgccaagccgatgtagccggcccattgcgccaaggtcagccgaggtcgcgtcaccggatcaggcggcccgccgctgcggcgcctttgcgcccacttcgcgcgccaggtcgtcaaaggcgatcagttgccgcgccaaggcttcaaactggccgagcggcaccatgttggggccgtccgacggcgcatggtcggggtccggatgcgtctcgatgaagacggcgtccacgccgaccgaaacggcggcgcgcgccagcaccggcacgaactcgcgttggccgccggaggaggtcccctgcccgcccggctgctgcacactgtgggtcgcgtcgaacaccacggggcagccgatgtcgcgcagcaccggcagggcgcgcatgtcgctgaccagggtgttgtagccgaagctcgcgccgcgttcgcaggccatgacattgggattgcccgcgccgaccaccttggcgatgacgttcttcatgtcccagggcgccaggaactggcccttcttgatgttgatggcacgcccggtggccgccgccgcgagcagcaggtcggtctggcgcgacagaaaggccgggatctgcagcacgtccaccgcttcggccaccggcgcgcactgcgcctccgagtggacgtcggtcagggtcggcaggccggtgaccgttttgatctcggcgaagatcggcagggcgtcggccaggccgatgccgcgcgcggccgtggccgaggtgcggttcgccttgtcaaagctggtcttgtagatgatgccgacgtccagccgctcgccgatctccttcagggcgtgggccgtctccagcgcatggtggcggctctccatctggcagggaccggcgatgaaggcgatgcgggcgccgcctccgatcacgaccgggcgctgcacgccttcagacagggtgatgacggcgttgggctggctcacggctgggctttctgtgcgttcgggcgttgaaacaggcgacatatagcgcaggcctgcggcgatcaggtggcgcgaaacgtcgccgaccgcaatagcatggacccgcacgcccgcatgaccgcacgcccgatcctgatgtggcttcgccgcgacctgcggctccgggacaatccggcgctggaggcggctcgaaccagcggccggcccattgtgcctgtctacatccgcgatacgcatctggaggggcgtgcgatcggcgccgcatccgagtggtggctcgacaagtcgctccgcgcgctttcgtccgacatcgccgagcgcggcggacgcctgatcctgcgccacggcgacagcgaggccgaactgcatcggctggtcgaggagaccgacgcggaggcgctggtcttcaaccgcctgtacgagcccgacgcgcggacccgggaccgcgatgtcgctcatgcgctgagctgcgcaggggtcgaggtcacaagcttcaacggatcactgctggcggagccggaggcggtgaagaccggaggcggcggcccgtaccgggggttcacgccgttccgccgcgcgctgatggcgcagatacagacgccgccgccatcccccgctccggagcggttcgcgcccgcagaaatcgggagcgacgacctggcggattggcggctccatccctccgctccggactggtcgcagggcttcgactggcggccgggcgaggctgcggcgttggccgagctcgacggatgggcggcggacgcctttgcggactaccagcacggacgcgacaagccctcgggctccgccagcagccgcctgtcgccccggcttcactggggagagctggcgccctggcgggtgctccagacggtggaagcggccgcgcgaaacggggcggcgccgttcgaagcggccgagaagttcacgtccgaggtcgcctggcgcgacttctcgactcatctgctgcaccattttccctcgatcgagcacagcgccttccgccccgcctatgacgacatgccatggcgcgacgatcccgaagggctcgacgcgtggaagacaggccggaccggctatccgctggtggacgccggcatgcggcagctgtggaccacaggctggatgcacaaccgcgtgcggatggtcacggcctcctttctgatcaagcatctgctgatcgactggcgagagggcgagcgctggttctgggacacgctggtcgacgccgaccgcgccagcaacctgatcaactggcagtgggtggccggatccggaccggacgccacccccttcttccgcatctacaatcccgtggcgcagggcgagaagttcgatgcggagggccgctatgtgcgcatgtggcttcccgaactcgcggggcttccgaaccgctggctgcatgcgccttggaccgcgccggaggctgtgctggccggggccggcgtgcgcctcggcgtcgactaccctgcgcccatcgtcgatcatgcgcaggcgcgcgcccgcgccctggcggcgctgaagagcctgcccaaggcgcactcggacgactaggcggagcgcacgaccgcgcccaactctcgccggcaggcctcggcctcttcgacgtgcgcacggcgacgctcttcgccctgtttgtccaacgtgttgtagggcatggcgaggcggcggttgtcacgcagacgaccgcggttccgctccaggaagccccagtagagccggttgaacggacaggcgtcagggcccgacttcgccttcacgtcatagcggcatccgccgcagtagtcgctcatccggttgatgtaggcccccgacgccgcatagggcttggtgcccatgatcccgccgtcggcgaacagggccatgccgcgcgtattgggcatctccacccattcataggcgtcggcgtagaccaccagataccactcatcgacctcgtccgggtgcacgcccagcagcagcgcgaggttgccggtgatcatcagccgctggatatgatgagcgtaggcgtgggcgcgcgtgccggccacgacatcggcgacacaggccatctcggtctcgcccgaccagtagaaccacggcaggactcggtcggcgtccagtgcgttgcgcaggcggtactctgggaccttgagccagtagatcccccgcacgaactcacgccagcccaggatctggcggatgaagccttcgacggcgttcaggggcgcacggcccgccagatgctcggcctcggccgcgcggcagacctccatcggatccagcaacccgaggttcagcgaggtggagatcatcgcgtgccacatccatggctcgcccgtcgccatgtcgtcctgccatcggccgaagcccggcaggatgcggccgacgaagtccccgagcacctccagcgcctcctcccgcgtcaccggccagccgaaggcgtccaggtcgccgaaatgctccgggaaaaggcgagccacgtcgtcgagggcgccgcgcgtgaccgcatcgggcgggatgcgcagccgctcgggcggttggacccggccgctcagcggcccgcggttgtcggcgtcgaagttccaccgttcgcccgccggacgtgcgccctgcatcagcaggcccgtctcgcgtcgcatctcgcgatagaagaactccatcgtcagttcggccttgccggccgcccagtgtcggaaccgcgcatgcgagcagatgaagcggtcgtcctcccggatagcgacggctgcggaggccccctcggcgaaggcggccagcgcctgcgccagccgccactctccgcattcggtcaggaacacccggtcgatcggctggtcggccagcgcccgctccagctcgccgacaatggagccgctgttgtcgggatcgtcgatccggacgtagcgcaccgtgacgccttgtccctccagcctcgccgcgaagtggcgcatggccgagaacaccagtgcgatcttctgcttgtggtgccggacataggtggcctcgtcccgcacctcggccatcagcaccacgtcgcggccgggatccaggtcccgcagggcgctgaggctgtccgacagttgatcgccgagcaccagccgcagggcgcccgtcgtgctaggctggggcatgaacgcttctccgctgatctccatcgaagaactcgcggcgacgctcggtgatccgaagctgcggctggtggacgccagttggcggctggacggccatgacacccgcgccgatcacgcgcaggagcggctgcccggcgctgtcttctttgacctcgaagccgtgtcggacacatccaaccccctgccccacatgatcccgcgtcccgaggtcttcgggcgggcggcaggggcgcttggcgtcgctgaagacgaccgcatcgtcgtctacgacagcgcgggtctgttctcggcggcgcgtgtgtggtggctgttccggatcatgggcgcgtcggatgtccgcgtgctggacgggggtctgcccaagtggcggcgagagggacggccgctggacagcggcgcggccgcggaggtgcggcccgcaacctttcatccgtgcatgaaaacggcggcggtcgcggactggagcgaagtgcgcgaggccttgaccgggcgggtccaggttctcgacgcccgcggcgcggcccgcttccggggcgatgcgcccgagccgcggcctgggctgcgcgccggccacatgccgggcgcgatcaacctgccccacggcgatctgctgcggccggacggaaccctgaagcgcggctccgagctgcgcgagacgttcgagggaaatggcgtcgatctgagccggccggcgatcaccagctgcggctccggcgtcaccgccgcgatcctgacgctggccttggccgacctgggccttccgtcgcgtctctacgacggctcgtgggctgaatggggcggacggccggacctgccggtggagaccggctgagatcagccggtggtgtccggaaccgggctgcgacgttcggaccccggcagtacgtcggactgagggtcggcggcttcgaccgcctcgtccttttcgccccgcgacacgatggtggccagcgcgaggtcgccggtgacgttcagcgtggtgcggcacatgtccaggaagcgatcgacccccaggatcaggccgatgccttctgccggcacgccgaccatgaccaggatcatcgccaccaccggcagcgatccggccggcacgcccgccgtgccgacgccgcccaggatgcagaccagcatgaccacgatctgctgcgtcaaagtcagctcgatgttgaagaactgggccaggaacaggaccgtgacgccttcaaacaaggcggtgccgttctggttggccgtcgccccgacggtcaggacgaagcgggcgatctttcgcggcagctgcagctgctcctccgccgcgcgaagggcgaatgtcagcgaggcgttggacgaggcggtcgagaaggccacgatcatgggctcgcgcacgccccggaagaacctggccggcgacatgccgcccagcagccagacgaccagcggatagaccacgaacatgtggatcgccatggcgcccacggccactccgacaaaggcggccaggcgcaccagcaattccagtccgaacagcgccgtcaggttgaacatcaggcaggcgatggccagcggcgccagcttgatgaacaggttgatcagcttcatcgtgacttcgaaaaggccttggatcacctcctgcagcccatccgtcgccgggctcttggccatgaccaggccgatgccgaagaacagggcgaacaccatcaccggcaggatcgcgttctcggcggcggccgtgaatacgttggacggcaccagatccaggaagaagtcgcccagcgagatgctggtaggggcgttctccacgatgttggcggctccggcgcgaccctgatcgagcagcgcctgcgccagcgccggatcgaccccgcgccccggctggaagacgttgaccatgcccaggccgatggccaccgctatgcctgaaaccaccaccgtcagcagcagcgtcttcagccccgtccgcccaagcgaagcgagatcgcccatctcggccacgccgatcaccagcgccgagaacagcagcgggatcaccatcatgaacaggagccgcaggaagatctgtccgatcggtcccgtgacgttggacgtcagccacaccacccatggcgcgtcgccgccgacgcccagattgacaatgaggcccgcgcccagacccaccacgaagccgataagcatcagccagtgcagggcgaggccgcgcgtcttcgtttcggtcatgagttcctcaaggatcaggcgcgggcgtcagcgaatcggcaggccgtagatcaggccagccggctgagcgttccattgtgcgttcaagccgcgttccaggtcgagcgccgattgcgatccgagattgcgctcgaagatttcgccgtagttgccggtcgcggcgatggcctgcgccgcccaacgcctgtccagctccagcatggcgccgaagtcggcgtccaggcccaggagccgccggatgcgtggatcgcgcgcctgctgggtctggtcctggaccgtggacgccgtgactcccagctcttcagcgagaatgagggcgttcaacgtccatcgcaccagcgaagcccagcgctcgtcgcccgacgcgaccgccggccccaacggctccttcgacaccacgtcggaaaggatcacgtgactggacgggttcggcagaaccgttcgtgcggcggccagcgccgagatgtcgccgctgaaggcgtcgcagtcttcgcggccgtaggcgtcgcgcgccgcctcctcgctgggcaggaccacgggccgatactccaccccgttcaggcggaagaagtcgtcggcgttctgctgggaggttgagccgccctgcacgcagatgcgcgcgccgttcagctcggcggcgctgttcaggttcagcgcccgacggaccaggaagccttgtccgtcgtagtagttggcgccggcgaaaacgacgccctcccccgcctcgcgcgtcagcgtccaggaggagttgcgccagaggacatcgatccggccctcctgcagcgccacgaaccgctgctccgtcgtcacgggcacgaaacgcaccgcgttcggatcgttgaagatcgcggcggccatcgctcggcagaagtcggcgtcgaagccgcgccactcgccgcgattgtcggtataggcgaacccgaccagacccgaatgcacgccgcagttcagtcgaccgcgtcgcttcaccgccgccagcacccgactgggcgcacgctcggcggcgaccggcgcggcggcgacggtcgtcggctccgcctcgggcgcgggcgcgtcgcgtcgaccgcacgaggcggccaacaggctggtcagggcgaccaaaagcgccgcttttcgcatcgagtcgtgacctccgccgcttgcgccccgcttcggtttagaggcctttggcgccgcatcgcaacccgcagggaccttccccatgcctccgctctccccgcgcacccggctgatctccgcagcgacaagacgcggaaaaggacgtcgtcctgtgaacccgccgctggagcgcgcgtcgacgatgctcagcgactcactgggatccatgctcgatccagcctccggtcccgtctatggcctggacgggttgagcgcggcctcggcgctgaaagccgccctggctgatctggaaggcggcgaccacgcctttctggcgccctcggggttagcggcggtgacgattccgctgctcgccttgctggggcccggcgacgaggtggtggcgtccgacgccgtctatggccccagccgccgattcatcacccgctacctaggcgcacgcggagtcgccagtcgcttccacccggccgacgcctccaccgaggccgttgtcggcatgctgtcgtctcggacgcgcgtcttgctgatggagtcgcctgcgtccctgaccttcgagatcgccgatgttccggcgctcgcacgcgcctgccgggaacggggcgtgatcagcgtgctggacaacacctgggccgccggcctcgccttccgacctctggaccatggggtcgacgtcagccttcaggccctgacgaaatacgcctccggccattccgacgttctgatgggatcggtggtcgtcagggatcagaccctggcgagcgccttggccggcgtgatcgaggacatgggctggcacgtctcgcccgacgacgcctggctggcgctgcgcggcctgcgcaccctgccgctgcgctatgccgagcaggcgcgttcggccctggtcgtcgccgaatggctgcagcagcggccggaaacggcgaatgtgctctatccgcccctgcccggctcggcctcgcatgaaaggtggcggcgcgacttcatcggggcggcttcgttgatgggcgtggtgctgaagagagaccccgccttcgccgagaggctcctcgacgcgctgacgctgttcggcctcggctattcctggggcggcttcgagagcctggccacctttgaaagcccgcagctcgcctttcgccggcattcaccggagcttcccggcgccctgatccgcctgcacgtcggattggaagacccggccgatctcatcgccgaccttgatcaggccttcgcccgggccgccggctgaaacccgcagtttggcgcgccctgcaggactcgaacctgcaaccgtccgcttagaaggcgggtgctctatccggttgagctaagggcgcgtggaggcggaagtgcccgccccgtaaggggttttatcgtaccgggcaagagaacgatcagcgaccgtcagactcgccagtcggacggtcgtcagactcttgtgctgcggacgttcccgacgtggcctcgatagcgtcgattgatcttcccccgtaaaagtggacggggttaagccgctttgcgctcggcctcagcggggctgatatagcccagtgctgagtgcaggcgatggggattgtagaagccctcgatgtatccgaacaggtctcgccgcgcctggtctcgggtggcgtagacgcggtgatgaacgcgttcggtcttgagggtgtggaagaagctctccatcggggcattgtcccagcagtcgccctttcggctcatcgacggggtgatgccggatcgggccagggctgatcgataggcttcggctgcgtattggatgccccggtccgaatgatggatcaggccgggcgcggggcgctgacgttcgacggccatgttgagggcgtcgagggcgatctcggtgtgcagggtctggcgcatggaccagcccacgatcttgcgggtgtgcaggtcgaggatggcggcgagatagagccagccttcgccggtcgggatgtaggtgaggtcggcgagccagacctggttgggcgccgccgcctcgaagttccgggccagcctgttgggcgcgatgggataaccgtggcggctgttcgtcgtccgggcgcgacgcggcaaggccgccaagccccgcaggccggcgcggcgcatcagccgctccacgcgggatcgaccgacccgacgcccatgccgccgcagggtggcgtgaacgcgcggcgagccgtaacagccgctgctctccgcatggatcagccggatatcctcggtcagctcgcgattggcgacagaccgctggctctcggggcgaccgcgccaggcgtagtaaccgctggccgacaagcccaggaccgcgcacatcacgcgaaccggccagacctgacgatgctcatcgacgaacccgaacttcatcgggaggccgctccgaagatgagcgcggctttttttaggatgtcccgctccatccgcagctgaccgttctctcgccgcaaccgggccacctccgccgccagatccgacggcgacggggacgacgcctgcgttgtggggcgccgcgacgcccccgtcgcctgcaccccgaactgcgtcatccatcgacgaagcaccgtctcgtgcagcccaagctcgcgggccaccgccccgacgctcaggccgccgttggcgacgcggtcaacggcctcgcgcttgaaagaatccggaaagttccggcgttgaacactcatcagacactcctctccagctccgaaaagctagcatgggtgtccaccaaaccgagggaggatcagcgcgtcgttcctgggcggtgtctcgaccctcgctggcgggttcgcgtccaaacgcgcgaaagcagccaaggcgcaggcagccgagatcgaagccagcatggcgcggcttcagggccttcagatcggcgagcagtcgcgcgaggcgctggcgggggcgctgggcaacattcaggtgatcacgtccgcgcgcggcgtcagcaatgacgatccaaccggccgggtgatcgaacgccgcacgatccaagatgcctaccgcgacgaagccgtagcggtgctggcggcgcggaatcgtgcgtcgaacgcgcagcttgaggcgcgcggctaccggtcggcttcccgctggtccgtgcctctcgccgtcctgaacagcgccagcagcttcgccaacgcctacagctacggctccatggggatgaagggctgatggctctcggaaccggactcaatgtcgcccgcggacagggcacgactccgctgacggacatgtccggctttgcggccggtgacatggcggcagcggagggattcgagcgtgcggcgcagggactcggccggctggtcgatgcgatagagccggtcgcgcagcaggccgccgcgcgtatcgccgagcaggaagtcgccgccggccgattccaggaacgcgcgactatcaccggcgccgacgtggcgttcaaccgcgcgatgacggcgggcacgatggcccggctggagaaccagcgcgacgccgatctcgacgctctgcgcctccagcacgccttcgatccggaaggcttccgcaccgcagcagccgaataccggacaaacgcgctcggcggtgcggttcctggcgcgctcgccatggaatggggcgcaggattcgaccgacgcgcgggcaacgtcttcggcaccatcgcagcggccaaggccgagctggatctgcgcgaggccaagggcgcgaccgaggcgcggatcgagcgcctgacctccgagacgatcggcatggcgcaaggtcgcgcgctcggggatgtgctgggcgccgacgacgtgcagggcaacctgctgcaaatccggctaatgtttgagggtcttgcgggcaatcccgcattcggcatgtcatctgaggaagccgcgctcaagggtaacgaggtggtggcccgcatcaaggccggcgccgtgtccgcccaagcgacgaacatcctgcgcgccgagggcgcggacgccgcctatggcttccttcagcagcttcagaccgggaccgatccgctgctcgatgcggacgaacgcaccctcgccttcaaccaggcccgcgatgccgtgcagcaggaagttggcctggccaaccaacgccgaaaccaagccgaggccgagcaggcggcgatcgagcgcgaggctcagcgcctgatcgacgaggacgtggcgcagctcgaactgacgggcgaaagctcgggactgaccgaggatcaggttcgggcggcgggcgggctgacggcggtcgcgcgctggtacaaggcgcggtcggaagcgctggagtttcaccagcttgtgggcgatctctcaggccttgggccagaagaggcggcggcgcggatcgcggagcgaacggccgcccgcagcgtatccgccctgcccgccattcaggatgctggcgacctcaacagcgtcgtggcggccatcgttcaggtcgagagcggcggcgtaagcgggctcgtcagcgacgacccggatggcgctggcccagccggcggcggcgcgtacggcgtcatgcaggtgctgccggagacggcgcgtcgcatcgccgggcaactcggccttcccttcgacgccaaccgcctgcgcaacgatcccgcctataatcagcgcattggcacggcgtacctccagcagcttctgaaccgctacaacggcgacaccttcctggccgtcaccgcctaccacgccggcgagggcaacgtggacggctggctgcgatccgtcggcgacccccgcagcggccagatcacgcgggaggcatggctggccggtgtggagtcgcgcggcaatccgcgctcggctgcttatcctcgcaaggtcatggccgcgatgggcgccggtcgagcatcggctgcgtgggacgcctaccaaggccagcgggcgcagcgtgacgccgatccggccaccgccatccaacgcgagttcccagtgcgcgccgcacgggaggcctggcaggcgaacccaacccgaacgcctgctgccgagggctatgtccaggcgaacctcgacgcccagtcccgcgctaacatcagcgacggccgccggcgcaccctgccgatgcagtcgctggtgatctatgccggcgacatcgaggccatagccaagcggggcgacacggcggcgtacaacgcctacacgcagcgcctcgtccgtaccttcggccgacatgggcagcgggtccttcaggacgtgctggaggtgcgcggcaacaccgcgttcgccgcccaaatcgcagcgcgcgccacgcagcaggcgtccaccggccagagaccgacccgcacgcagcaggcgcaagccaacaccgccgcgcgtgggcagcggatgacgcaggcggcgaccggacgcggtggcggcaacgtgcgagccatgtccgatgatgccgtgctcgccgccgcagggctgaactgatgagcgaccgcgaagccgccctggccgaggcctatcgccgggggatcatgaagcccgagcagaaggccgcctatgaggaggcgctgcgccgagggctggtgaagcagggaccggatcgcacgctgggacagcggttcctcgacaatctcggggacgcctgggaacggtcgggtgccggtcagctgaaccgacaggcgtcggagggcgtgtgggctgcacctcggctgcgtgagggcgggctggtggatcgcggcctggacgccgtgttcgggcaggatcgtggcttcgtgcgcggcacgtcggcactgacaccggcgcagcagcgagagcgggaccgtcgcgcccggtatgacgccctcgccaaagccgacccgatcgagaacgtcggtgacttcgcggcatttattggcggccagattgcgggcggcgcggcctcgccggagaactgggtggcacccggtcgttccgtcgccacacgcgcggcagggaacgcggccgtggccggcggtgctgacgtgctgctgcaaggcaacgacgtgatgtcaggcgtgcaggacgactacagcgtggttcagacgctgggcgcggcggcgctgggcgctggtctgtcggcggcgaccgatgcggtgcggccggtcagcgacatggttcgccgggcgttcaccgacaaggtggagccgcgcacgcgacccgctgcgccagagcaagccagcaccgacggggctgcggccgacgcgtctccgacggcgcgcgagggcatcaccgtcgaaggccccgatggcgtggtagtggacgtgccggccgcgcccgcgcagcccgagttcggaatcgttcagcgcgtcgatcgcaggacgccgctacgggatgcgctggcccgcgcccgcgaaggcgaactgccgcagcaggtgggggccttcatgggccgcgcctacaccgccatcgtcagcgaccagcatccgctcgcgcgggtggtggaggacctgcgcagcgcgacggagggggtgaccggcgcgcccgtcgacattcgaccgagcgaggatccgcgcaagctggcgcgcgggcggttcgattgggccgccatcgggcaccaggatttgctgcacggcgtccatgcctatcgcgggatggagccgacgacgcccgctctggcggacgtggtatcggcggtcgaggtgcgcgcgcgccgcatggaagaaaagccggccgaggccatccagcgattcaatgaatacatggtcgcccggcgtgcgagcctggaatgggaccggttcaaccgtggcgaactggagaacgcgcccgtcgcgcgtacgaaggaagaggccgacgcctatgtggcgcatgtggagtccaccgatccggagttccgcgagctgtcggactcggtgaacgcctattcgagcggcctgctgaagaaggcgctggacggcgggctgatcgaccaggcgacctatgacgcgtcgctcgccggccgagacttctatgtcccgctgcgccgcgtgcaggacgaaggcgcgaagccgggtggcaataagggcggcggcagcaacgcgggttcggaggtgaagcgcttccggggcagcgagcgcgatgtggtcgacccggtgtctgtgctgatccagcgcacgtaccggctgaaccagcggatccggcagaacgagctgaacttggcgctgatccgcatgggcgaacggctggaggcggcgcgccgtgccgccggagacgcagaggcgacgaacggctggctgaagaagctggacacgccgatgcgcccggtgaaggtcgggctggacgaactgcaggcgaacgcgcgggaaggcgccaacgtcgaagacatgttcgacgccgatggcgccgagttctggcgaccggggcaactgaacgagggtggccggcccatcctctacgcctggcgcgacggcaagcgcgaggcgtgggaggtcatcgacaccgagtggggccgcgacgtgttcgaggccatggccggcatgtcgaaggggatggaggacacgttcctgaacgcggtggcggcgcccacagcggtgctggcgcagaccatcacccgcgacccggcgttcctgctgtcgaacttcatccgcgaccaggtgtcttcgtggatcgtgaccgacgtgggcttcgtgccgggcgaaggcgccttgggtgtccgcgccgagctgggccaggaggacgtgacgcgcgtctatggtctgtccggcggcatcagcggcggtgccgcaacggccatgctgggcgaggcgctgcaccgggccgacactctgtcgctggcgaagaagggtatccgcgcgcgctacttctccagcctgggcggactgctggccaccagcgagatcactgagaccgggacgcgcctgcgcgtgttccagcgggccttcgatcgcgcgcgcaaggcggggttcagcgagtacgattcgctgatcgaagcgtcattcaccgcgcgcgacatgatggacttcggccgcgcggggtccaagatgcacatgacgcgcaggctggtgacgttcctgaacgcctatgtgcaaggcctggacaagacgctgcgcactctgggcgccgacggtgcgacgaggcgcgtgccgctgaaggaggcgatccgcccgctgttcggcatgcaggtgcagccgggcacgatgcgcgcggaggaccgagcggccctgcaactggccggccgggcctggacgaaggtcgcggcagtggccaccttcggcgccgcgatcaccgccctcttccacgacgacccggactggcagcaggccaacgagaaaacgcgggccacgcactggacgatcccctggggcggctatctggtgaagatccccaaaccgttcgagctggccttcctgtcgaacgtcgtcgagcgtggcatcgaggcgacctacggccaggacgaagaggcgtgggagcgtatgtggaaggggctcggcatgctgttcgccccgccggccgacatccccgttgcggccgtggtgggtgggctgaaatccaacaccaacgcgctgacgaaccgccctatcgtgccggatcacctgcagaacctgccgcccgagcagcagtaccagcattggaacagcgggttctcccggtggctgggtgagaagatcaacgtgagcccggcgcagatcgactacgccatccaggggttcgctggccccttcggctcctacctgctgaacggcatggacgccgccgatcccgaccggccgtctggctcatggacggacctgccagtcgtgcggcggttcgtgaacccgtccttccgcggttcgcaggacaagcgcgacttctacgaccgcgccggcgcaaagacctcggagcttcaacgcgccctgaatggcatgcgcgagtatcaggaacagggccgcatggacgcggcgcaggcgatcttcgacgacctggacgatgcgggtaagctgttcgtcacgagccagatgggcgagacgccgactcgtaggctcaatccgctggagcgcgcgcgggtgttcgccacagaagccagccgcctgatcggggaactgaacggcgctttgccgaaggacgagggagcgcccctccccccactcagtcggcagaccaagcagatgatcgaggacgcgctggaacgcgtagccgtggccgagatgcgcaacgccatgatcgtgacgcgccagtccgggttcgtgaaccgcaagcaggaggaccgcgccgggttgtggaaagacctgcgcgacctgtcgccggaggtggccgctgagcttgagcgtcgcctgggcgtgggccgcgacaaggcctacgactacgacaccgtgatggatctgtggccggaggtggaggcgcggctgaaagctgaaggatcggcggcctatctcgacgatctggcatctgacgcgcagggccgcaccccatcctggggcgacagctacgacgacggcgagttgcccgacgcgctggtctacaagccctgacggcggcggtgcattccgcgcgatgcgtgatcgcccgacgctgcgtgcatggcctccaacgtgacgatcccgccgtttgacaccgcgcccgcgaccatcgtgggcgcgacgccgcaggccgtgttccccttcgacttcccgttctgggaggctgccgacatcctggtcttcgtcaacggcgtgcaggtggcgcaaggcgcctatcaggtcgaaggctatgccgtgcagaacggcgagccggtcgagggcggattcgggtccggccgcgtcaccctgaacgtcgccgtagcgaacgccaccgtcgtcatcgatcgattcgtggacggcgcgcgggagagccagttcagccggtcgtcgcccctgccgatgacggcgctgaacgccgacctaaacaagacgaccgcccgacagcaagacgtggcgcgtctcgtccgccggattcagttccaaggcttgacggagcgattggacgccagcggtgcgcgggcggcgattggtctaaatgatccgaccaacctgcccttccaggcggcggccggagggctgctccgttccttgggcgcgaaagctggccaggagcaacgctccatcctagatttctgccgcacggatcgcacggcgacgcagaacacggccggactaaatgcggcgctgtccagcggaaagctggttcattgctacggcgcagaggggcagtcgttccagatcaacggccccgtcgtgttggcggacggtgcacagctaattggtagcccaaactgcaagacggttctggtgccgcaagccggcgactacgacacgttccagcttcagggcaactacgtcacactgcgcggcttcaccgtctacgaggactccaagacggccggcaccggcgccacctttcgccgcttcatctcgggtatcgtagagaagctgctgatcgaggacatcgacatcgaggccagtcctcggttgtgggcagagacgcggacaaccggctactacaagcgctcgaccctgcgcgagatcgtcgccaaacggcatcggggtcccggcttcttgaaagaatgggcctacgcctacgactacattgagccgtcggtgaccatcgacttcaacggctcaaccagcccgaaccacacggcctatcgtcaaatcggcggcaaccttggcatcgccgagggcggaacctattgcggtctgaatgtgctgggtacagcgtccgaagttgggatcacgacgacgcagatcgccttctgggtttccgatgtggccgaagggcatttcgagcacgctcggagcgattcctgcaaaggcggatcgctgttcgacggctgcacgaacctgcatctgaaccacagctacttcggcctgtctgacgacatccaggccacccttattgactgcacctatgtgcgcggcgtcctgcccgtcttcaggggacgcaagctcgtctccggaacggcgaacaaggccggcctggacatccagaacggcaatgccaacgtgatgctcgtgggtgtcgacgcgcacgaaaacacgggcgatggcgtcctgaagagtggcgccaccagcagtcgcatcgtaaccctccggtgggggccgccttgtttcgctgaattctccggcgatgctctgcgcttaagcctggtcttaagaccgggcgttcgagcgagcttaagcgcagatgagccagattaccctgctaacgggaccggaacgccgccgccggtggcgcgacgaggagaggctggccatcctggaagaagcgttttcgccgggggcctgcgtcagtgaggtcgcccgccgtcacgaggtctcttcgagcctgatctacacctggcgtcgtaatgcgcgtacgcagaccggcgacccggctttcgtcgaagccgtcatggcggatgctgggtccagatccgggccgagcggtgatccggtgatccgggttgaactggcggcggcacgagtgagcatcaccggtgccgcctcgccggtgcttgtgggcgcggtgctgcgggcgctgcgatgatacccccaggcggtcgagtctggatctccactggccacacggacatgaggaaggggatgcaggggctggcgctgctggtgcaggagcacctcaagcgcgatccccacggcggcgacctctatgtgttccgcggtcgcggcggctccctgctgaaaatcatctggcatgacgggatcggcatgtcgctctacgccaagcggttggagcggggacggttcatctggccgaaggctgagggtggagctgtcgcgctgacaagcgcccagctgggctaccttctggaaggaatcgactggcgtaatccccagcacagctggcggccgagcagcgccggctgagccgaaaatagttgggcccggctgcattttagggcgccacaagcggcgtgatctgtgattcaattcgggtcatggaagccgcgaccgcgcccagtgcagaggagttcgaagcgctgaaggcggcgctggccagcatgcgcaacgagcgcgatgaggcccgtgccgaggtcgccgtcgccaaggcagagcgctctgaagaccaggcgctgatcgcgcacctgaagctgatgatcgccaagctgaaacgcgagacgttcggcgtctcctcggagcgttccagccggttgctggatcagatggagctgcagctcgaagagctggaggcctcggccaccgaagatgagctggccgccgagaaggcggcccgggcgaccacgacggtcagggcgttcgcccgtaagaagccgtctcgccagcccttccccgaacacctgccacgcgaacgggtggtgctggaaacgccgacggcctgcgcctgctgcggcggtgagcggctgagcaaactgggcgaggacatcaccgagacgctggaggtgattccgcgccagtggaaggtgatccagacggtgcgtgagaagttctcgtgccgggactgcgagaccatcgctcaggcgccggcgccgttccacgttctgccacgcggctgggcggggccaagcctgctggcgatgatcatgttcgagaagttcggccagcatcagccgctgaaccggcaggccgagcgctatgccagagaaggcgtgccactgagcctgtcgacgctcgcggaccaggttggcggcgtcgcttcggtgctggcgccgctgtaccagcgcattgaagcccatgtgctggccgccgagcgactgcatggcgacgacacgaccgtcccggttctggccaagggcaagaccgacatcgcccggctctggacctatgtgcgcgatgacgcaccgttcggcgcgacttcgccgcccgcggcgatcttccactactcccgggatcggcgagggatgcatcctcagacccatctgcagacctggtgcggtgttctgcaggccgacgcctatggcggctacaacgaactctacaaggagggccggccgcccggtccgatcctggaagcagcgtgctgggcgcacggccggcgcaagttcttcgagttggctgaccttgaggccgcccagcgcaagaaggcgcgcggcgagaagcccagagctgtgtatcccaaggcgctggaagccgtgcgcctgatcgacgccctgttcgcgatcgagcggaccatcaacggcgccagcccagccgaacgtcttgccgtccgccagacgcagagcgcgcccatcgtcgccgaactcaaggaatggctggccgcggcacgcgagccgctgaccggcagccacggtatcgtcaaggcgatcaactacctgcagaagcgctggccgtccttcacactcttcctggaggacggccgcgtctgcctgagcaacaacgccgccgaacgtgctctgcgaggcatcgcgctcgggcgcaaatcctggctgttctgcggctcagaccgtggcggccagcgggcggcgaccatgtacagcctgatcgccactgcgaagatgaacgacgtcgatcctcaggcctggctggccgacgtcctggcgcgcatcaatgaccttcccagcaaccgcctcgacgagttgttgccgtggaactggaccagctcatccgtcgtggcgcttccgtgagcgggccgtcacccactgagaaggtgcacatcacgtccacctgcgagcggttcatcgaggatatcttgaagccgcggttcttgccggtcgtacgtccgactgagttcaactatcccgtcaatatccagggcaagtggcacggagcccgctatcggctcatccaacgctaccgctctggcttcgctgacaacctcggttacgagttcgacgcgccgttcgtccgtctcgactggctcgccccggacagcttcaacatccagtggcatcgccacaccggggtctggcactgcctttaccggtccaaaaccctccgccaggccctcagactgatcgagacggacggcattctacagccgaactagccgtcagctcgtcgcggtgctcaccggatgggtacgtcgcatcatcatccccggctacatcaccctcgacaacggcggccgtggcatcaagaccgtgagcggcggcaccttcagcgcctcgggcggcttgatggacgggaatacggccggcaactacgacattggcggcgccattcaccagatactggccagccagaacaacggcggctcctacatcaatgtcagcggagtgggcacaggatgaccgtcagccaagaacagaaatgccaggtgctctatgccgtggccatgtcgctgcgtgacgcgcgcgccgtcgctgcctcatgcgcccgtatcatcgttgaagcgtgggctggagagaccatccagacgctggaggatggagacggcgccaaggtcggaaagcgcatcgaaaatgcggaatccgctctcggcatccgtctattcgacgccacgccaacaggcctcgtgctcactgaggccggccgcgcgtgggtggaaaatcggatcgaagcctacaccctgacggcgtagagactgccggccatggggttgtcggggttcgtccggtcgaagacgaacaggccgctcttgaccatcggccggatgaggtcagcctgggtcttcgccggatcccaccacttgtgccactcgatcatcattacatcgatcgacttgaacagatcggctcgctccaaatcttcgaagatggcgaactccgaaccctcgcaatcgaccttcataaccacgcgctgacccgccgccttggcgttgtcgatgataggtcgcagggtttcggctgccgatgcaatgtggatcgtctcttcggcgccgactgacgtgccggcaatactgacgccgacagtgttggtatcctgaactttgacctgtagggcctctttccgatccgccagcccgaaggggtaggtcgtgattttcggctcaaggctcgggttcatggcgatgtttgcagcagcgcgagcataaggcgtggcgaatggctcgaaagagtggacggccttgatcatagggttgttcgccagaagcagcgatgtcaggcccacgttcatgccgatgtcgatcgcgacacattcgactggagagacgaacgtgtactcgttgatgaaaaacagctcggtgaaaagctgcagttcttcttccgagtgcacgcggcaggtgatcccctggaccgtggcggttatggtatcgtctacatcgaaatcgacgcccaactcggccagacgacggatcgcagaatagttcttgcgcacgaagtccggcacttcgccacgcaatgtcaggaagcgtccagcgtcggccccatcgagcacgaccgacaatgggcgctcgtacgctacgcgaaagggctgtcccaaggcgtgtacgcgaaactcgaccaccgcattccctggaagatcgaagtccaactcggtcaagccgctggagacgaccttttccgcaagcacggtcgtaccgctgtttgtgacgacatctacgcgagcaacatcgttggccacgttctcggcggtgatatcgaaagcgaccttgaatcgaccggtcgctagttcagcgtagggaccatagacgacacaacctctggtgttgtcagcgacatcaacccagccgtcatccgcgatcatcgcattactaatgtgccgcatgagcccctccaacccctgagggaatccatagcgccacttggcctagaagagcaacggtgcattccggctcccgcccgacaaggcaatgctggcagcatgaccaacgccccccttgccgcagagccgatcatcgtcgatcccgatccgaccgcagccatggtttgggtcgctatacggtcgttgctgttcgccgctggcgggttcttcgtcggcaaaggctgggtgacgcaggagaccttggaggcggtcgtcggcgcactgatggtgctgctgccagctgccttcgtgttggtgaaatcgcggcagaacacggcgaagctggcgcgcatggcggctgtggcgccggataatgtggcgcaggtgaagtcgtgagcatcgtcgcagatgacgacttcgtgcgcgagttccagcggcgcgcggggctgcatgacgacggatgggctggtctcgacaccatggccgcgctcgaccgactgctgcccgccccggccgcacccagcaccgccatccccgacgactactggccaatgctgtcgaagatcgagagcggcgaccggccgtatgttcaggcgccgacttccagtgcgtcgggcctctaccagttcatcaagtccacttgggaagctgagggcggcaagtggggaccgacgctgcggccggcgttcggtgggctgaagccttcagaacaggagcaactggcccgggcgaaaaccttcaccgccaagaacgcggcctatctgtccgcgcgaggcatcccgatcaacaaggccagcctctacgccgcgcacttcttcgggccggtgaccgcggcgcgggtgatcgctgccgacgtgaatgcgcgggctgacgagatcgccggcgccgcggcgacgaacgccaacccttcgatcctaaagggcaagaccgtggggcagttcctgacctggctgcacggcaagaccggggaatgggcgcgatgagctggctgatagagcacgtgccgttctgggcgtggatcgtcggcggcgcagcggtcacggccgtcgcgtggcgcctcctcggcatccgcggcgggtttgccgccctcgcctttctcggctcgctcctgctctggcgtgatggccggaaggatggccgacagtcccaagtcacgaaggagcggcacgatgccgatcaagccgttcgccaagcagacgctgcgcgcgtcaatgctgctgtgcgcgatgctgaccctgaccagctgcgagcatctgacgggttccggcgagactgagacgcccatcgctggcgcagacaccttctgtcgcgtcgcccagccgatcacctggtccagccgcgataccgacgagacgattcgtgaggtgaaggcccacaacgctgtcggcgtgcgcctctgcggatggaagggcgtcggctgatgccttcttctgaagagatcatggttccagtgtccaagcccgaggcgatggtgcaggccgagattcacgccatgcgcacgctggcggacgccgtgcaggcacagggaaagtcgatcaccgagcacatgggcgccagtacgcgcgccttggagaagcttggcgagaaggtcgacgacatgaacggtcggctgatccggctggaggagcagaagcacgggcgcgagatcgagcggctggacggtgcgctccagaaggcactgacccgcgtggatagtctggagcagacccgagacaaggccgtgggtgccggcgcgttggtgacttggctgcggcagaccgcaccttggctgatcgcgattctggcttccggcgcggcggtgttcggcgtcaaggcgacgggttcctgaccgtcggactcgctctgcccgccctagacaattcaggcgcttagctgaccggcacagacacggaacagtcagacgctccgacgccgcttcaaccacatgccaccgcttagaaggcgggtgctctatccggttgagctaagggcgcgaaggtgtggaagcgctgacgcgtctcagtgcgtccagggttgcttgcgcgtggcggcgaagttgtcggcgtaggccttgatgatcaccggctgttcattgggcgcgtgcaaacggaaggggatgccgtgccgctcggcgtaggcgaccgcttcttcctgggtgtcgaaagtcagtcgcacctgcccgttcatgtcgccggagctggtccagcccatcagcgggtcgatggtgcgggcggccgcgggctcgaactccagacgccaggagaggctctttccccgtccggactgcatggcggtcttggcggggcgggagatgcgggcgagcatggcgggtctctgcggcggccagtggttcccgcgccggtcggggcggcaggattcgaacctgcgaccctctggtcccaaaccagatgcgctaccaggctgcgctacaccccggaccggcgcgacgccctcttgccatgcgcggcccggctccgcaacgcggatcgtccgtgcggcgtcactgtttgaagtaggggtgctcgatccggtcgccgacgcgcgcttcgatctcttcggttcggccggcgcgcagctccagcacgccgttcgcccgcccgttcgaggggatgaggctttccgacattggcgtcgcatgcggcgcgatggagatgatgcggccatccggcgcgagataaaggatgtccagcgaactcggcgtgttgcgcatccagaaggcctgctcccgagccggctcgcccggccactggaacagcatgccccggtccgccggcagcggttcgcggtacatcaggccctgctggcgctccgcctcttcgtcggcgatctcgaccttgaagtcgtgccgtcccgacgtcgtgacgatcgtcagaggctcaagcacgcgcccttgagcatcgacaggcgggcttgatccgcacgcggagagaatcagcagggcgaccaggcccatcgatctcagcgttcggcccatggctctctccgtcgccctcaagtcggaatcaaatatccgtacggatttcggcgaccacaaggcccttgggaccctgcgcgaaccggacgccgacagaatctccgggggtcagttcgtcgaaaccgcagcgacgaagcgtttcgatatgaacaaagatgtcgccgggagctccgtcgcgcaccacgaacccatagcccttggtgcggttgaaccacttcaccacggccggctccagctttccatcgaccggcccggccggcgggctgacgccgtccgatcggcgcggcgccgccgcaggcttgtcgccgtcgcccagcaggtggatttcgacggcctgccaacccttcggtcgtcgggcgcagtcgcaggtgatcggcgcgccctcctgtgcggtctccaaacccttgtcgcgcaggctggtgacatgcagcagcacgtccctgccgtcggtcgtcgacgggtcgtccggcacgatgaaaccatatcccttgccgatatcgaaccatttcacgcggccgctgacgcggacgcgctctgcggccgcgtcctctccgtccagatagtctgacacttctcaggcccccgcctgcatcctcactccggcgacatgcttaacactgttccgcgagaatttggaaaggccaaatgccagggttgtccgctggtcgcgcgaaagccgctgatcacggcctaaaatgtcggggaaaggctcccgcgtggcagtccctaggggaggctctgggcctcgcctgcaaggcgctgtttcgcttgctttcctcagtcgtggcaggcacttacgaacgcatcgttgaaagattcgtagaaaagttcgtagaaaatggctctgcgtggcagccggacaacgaggaagttgaaccccggcatctatgctcgtccggatggccgttatcaggcccacatcggcattcctaacgacgtgcagttcgcctatggacgcccgaaactcgtgctctctcttaagactgacgacccggaagaagcgaaccggcgtcacgcggacatggtcgcccactacaacgcggctttcgacctactgcgtcgtgggacggcctccacggcgttcgaagcgttcgccgttcggctccatgcctcccaaacccgcgccatcggcatcggcaacgacagggtgatcctccctcggtttggtggacacccatgctagcttttcggagctggagaggagtgtctgatgagtgttcaacgccggaactttccggattctttcaagcgcgaggccgttgaccgcgtcgccaacggcggcctgagcgtcggggcggtggcccgcgagcttgggctgcacgagacggtgcttcgtcgatggatgacgcagttcggggtgcaggcgacgggggcgtcgcggcgccccacaacgcaggcgtcgtccccgtcgccgtcggatctggcggcggaggtggcccggttgcggcgagagaacggtcagctgcggatggagcgggacatcctaaaaaaagccgcgctcatcttcggagcggcctcccgatgaagttcgggttcgtcgatgagcatcgtcaggtctggccggttcgcgtgatgtgcgcggtcctgggcttgtcggccagcggttactacgcctggcgcggtcgccccgagagccagcggtctgtcgccaatcgcgagctgaccgaggatatccggctgatccatgcggagagcagcggctgttacggctcgccgcgcgttcacgccaccctgcggcggcatgggcgtcgggtcggtcgatcccgcgtggagcggctgatgcgccgcgccggcctgcggggcttggcggccttgccgcgtcgcgcccggacgacgaacagccgccacggttatcccatcgcgcccaacaggctggcccggaacttcgaggcggcggcgcccaaccaggtctggctcgccgacctcacctacatcccgaccggcgaaggctggctctatctcgccgccatcctcgacctgcacacccgcaagatcgtgggctggtccatgcgccagaccctgcacaccgagatcgccctcgacgccctcaacatggccgtcgaacgtcagcgccccgcgcccggcctgatccatcattcggaccggggcatccaatacgcagccgaagcctatcgatcagccctggcccgatccggcatcaccccgtcgatgagccgaaagggcgactgctgggacaatgccccgatggagagcttcttccacaccctcaagaccgaacgcgttcatcaccgcgtctacgccacccgagaccaggcgcggcgagacctgttcggatacatcgagggcttctacaatccccatcgcctgcactcagcactgggctatatcagccccgctgaggccgagcgcaaagcggcttaaccccgtccacttttacgggggaagatcatgaggacgacggcgcggccgagcccagcctcgcctttcaggaggcgcgatccttcgacagccaggacgagatcatccggtggtcgccgacgggcgggcctgactacaccgacttggaggaagcctgctgacgtgatggtgtggacgacctccgcctgacgggctgttctgggtgtgtcgtcatcagggacgtcatgtgtggacgacctccaagacgcaagagtggaaacgacgttggcgctcggtcgagtgcagtcatgtgttcggcctgttgatgcagctgtttgcgctgctggccctgatgaagtccgcggaccggctccctaatcacgtcaacgcgctcgaggcgctctgaccccctgggtttcaccgatccccggctgcggccggttcgtcatcacgtctcaccactccttcgtctacggcgccggtcctgggtgaagaccggcccgatctctatgccgctgtgggcttgtagtcctcctgtcgcgccatcagggtccaggcgatgcgagccgtcttattggccaaggccacggcggcgaccttcggcttcttgcgttcgaggagattgccgacccagccctcgcgtcctcgctgccgggccattcgcaggaccgccgtggccccgacgaccaggagacgtcgaaggtagctgtcacccatcttgctgatgccgccctggcgttccttgccgccactgctattggcccgcggcgtgagtcccagccaggctgcaaactgccgaccggaacggaagagactcggatctggcgcgctggccgccatggcgctggcagtgatcggcccgatgcctgggatggtcgccagtcgccggctcgtctcatcctgccgatgccaatcgagaatccgacgctccatacggctgatctctgcgccaaggtgttcgagctgttctgccagcccgccaagcgcggcatgcgccagatccggcagggcctgaccctcttcacgcagactcttcagcgctgcccgcaccccagctggaccttgaggcgcgacgatgccgaactccccgaggtggccccgcagtgcgttgatcagcatcgttcgctgacgaaccaggagatcccgggtcttgtgcagcatcaacaccgcctgctgggccttcgacttcacagccacgaaccgcatggtcggccgggtgacagcctcggcaatcgcttcagcgtcggcggcgtcggtcttgccgcgcttcacataggccttcacgtacgccggcggcatgagccgaacatcgtggccgatcgccatcagttcacgcgcccagtggtgggctgaggcgcacgcctcgatcccgatcaggcacggcccaatcgactggaagaaggccagcacctggccgcgccgcagttgccgtctcacgacgaccgtgccgtctgtggctacaccgtgaacctggaaaacagtcttcgccagatcgagcccgacgacagcgatggtctgcatgataccgctcctagacgtgacgtccctgatgacgacacacccagaacagcccgtcaggcggaggtcgtccacaccatcacgtcacccgcgacatcgttcaggaaacattcaagttcgaagccgtcgatctcgcccgcgccatcgagaacgacgcggacggcgaggcatcgcaacggttgttcgaccggcgccaagcgacctcctttgctgtggaggtttcaggctctcatagaagtcgaatccgtcaaccagatcagaaggcatatgcggcgcccgactgctttctaagcgtcgtgaaacatccgaaagagggcggcgtcttccttccgttcgaaccggaagagatatcgggcgtcgcgaacctccaagccaaccgtgccgtcgtcagcccgatccaagagtcggatgccgtccgtgatggtatcgagtgaccattctcctttggtgcttgtcccgcaccaaaggagaagagggttcagtgggtgcttcgcaaggtcgagagagtcctccgtgacccaagcattgttgtcggcagacgggatcgtgaaaggcacggtgtgctggtgagcagtgacagtaggcatgataaactcaaaaatgaatgcttcgaatatgatgtaaaactaccatgccggaagcactcatgcattattaaaatggttctacatcacggtcgcgccgtgatcttctgaagttagtcgccaagttcaggtttaactcgcgggatcggagcgatgccgaacccggaatccatgatatttgcggccgagagatcgaccgagaggcccaagcgcttgcgctgatccgcatagtgcagccgggcgttttgcgcctcgttgatggctccatcgatccgatgactcagccactcgatatggttcaccaacatcgagatgcatgcctcctgagcattaagacgtgcctgagcgtcgtcgagagccgtggccagcaaatcgttgatctcatgctgggtcatcacgctgccgcctttcgcgcacgatagtcccttgctcgttccgccgccgtcttgggcggcctcttcggatcagctttccgaccgggctttgccttggtgtaagtcagcccgagatcgacgaagttcagcgttgtgcggaacgggaaacccgccgcttggaaatagtccgcgaggaaggtcgcttgctcgcggtcgtagacattgacggtcaccggtcgggggtcgttcggcatacgcaacgacgaccggaacacgatctggatcaggtcttcgaactctcgatcccggcgcacagcctcgtggtcaagcagacctccggtcatggcggcgaacaccttgtgctcggcgtcgcttgccttggccgagtagaggatcgagcactgcgtcagggcgcggtaggcgttcgacccggcgatcttcggcgacacctgcactccgggaagcttcagatcgccccgcttcttgttggccgcccaatagtgctggcgtgcatcgacgttctctctgacccatctgctccatgccttcacagcacgacgaccggattccgttgtctcgaagaatgtggacccagccctgtggtccgtggcgacgtagttgatcgtgagatcacggcccagccagatatcgctttttccgatgcacatgggcttccaaacgatgtcggggcaaagtgccgtggagaggcgataggtgatgaggctgtcgaagctattcgcgaggatgaaggcttggtcgtagacggccagttccgcgacatcccagaggctgaagtaggtcagcctctgtcggtgctggaggtcttcccacgcctccagattgatcaccgccccgcccttctgcacgcggctgtgaagggctgcgacagggcgggtaagatcgtctgccgccagcgcgcgggaagagggggcgtcagtcttcggaagaagcttggaatatcctttggtgaacggctccagattgtaggtggcctcccagaaaggcgcggatgcccccaaatcgaacgatcccgaggaccaaaccttcgggtcttcgtcgatgatgatggaccacccccgacctcggacgaccgagtgatcgaccctcttcatggcttcgtgggtgatgatgaggacgatgtgctcctcgtcgctcagccgctcgatttggagcgggaaatcgcgggacacgacgttgcccgcctcgctcgacatggaccggatggcgacgaagcagcccccctctgccgcagcttcggaaattcgacggtggcggggtgcgaactcagccgtgcggtccacgacatagatgtatcggccgggagtctgcccaatgtgcctaacggcccattctgtcttgccagcaccgcaggccgcgttgctgtagtaaagctcttgaatattcatgaaatgaattaaccagaccagcgcccttatgcgtcaggtcatgatctatttagaacgacattcgtcgttctgcattattattcgcgttctgggttgacaggagttgcggtcacgggcgcaccccgtcacatcattagtctaatatttattagaggattggcgtgacgcgctggggcgacgacccatcctttgttgccgagcactgcgccgcgccgtagcgcgacggctccacgccttcgatcacggcctcccggcagaagaagccgctcggcctatcgaagacctgtcgctgcttttcaaaccagatggcgccgaggagccgggttcttcggacacaccaaacccaaaaggcgcaacgaagagatcggcagcttccgccgatctcgaagttgctggcggcgccgtaaggcgtcggcgtcgcgatcacacccagtccatcgcccgttgaggcctaccccttggcccacttcgtcggctcgacacgcttattgacgtagtagtcgcgaagcgaccgcgaggttgcgcccgtgattgactggtgatggctcgggatagcgacctctcgaaaggtatacttctgagagacatcggatgaggtgtgtgggtatgtcgcgttaatagtcagatttgggtgacagattctccgaataccttatcctacaatctatctccgacaacgcggggctttcaggggttatcggacacgaatgctgatcggatattcgagatgctcggcgcgcgggcagaatcatgagtctcagatcgacgcgctggaacgggcggggtgtgagcgcatcttcattgaaacagcttccggcacgcgatccgacaggcctcagcttgccgaactcctcgacttcgcacgggccggagacaccgtatgcgtggttcgactcgaccgactcgcctgcgatgtccgtcaaatccttgatctcgtcgatcagttcacccgccgcgacatcggcctgaagtcgttgagcgaggccatcgacagcaccacacccagcggaaggctggcggttcacacgctggcggcgctcggccagtatgaagtcgaacagaagcgtctggcctgtgaggcgggccgacgagcggctatcgcgcgcggtcgcatgggcggtcgtccaaaggcgatggacgaaacaaagctcaagattgcgaaggcgctgatggccgacgaacagctttccatggccgagatcgcccggcaggtcggcgtggcaccgagcacgctctatcggacgctgccgggtggacgtggggccttggcggcggcctgactgtccgctcaggccgccctatcgaagtcggtcttgtcgaggtcggcgtcgatcaggaagccgaggtggggtcgctcatgcagtcgcgctgcgatgaacccggtcaggtccgcttcgctggccgccagttgctcggccgtgatcgcgcctcggaagagttcgtagcgcagccacacccggtaggtattcacgacatcggtctcgccatagtcggcgcactcctgaatacgacccgcccggacgtgatcccagaccttggagccgtcgatgccggtgggtttgccgggcaggcccatcatcttgcacagatcgtccagcccgaccttggcgttggactggaagctggccagttcatcacagagatcgacgtgggcggcgtcgtagcgtttgaagtaggaacgggaggtcaggccacgcgccgcgatcccgttgaccatagcccggtagcgcaggaccggcaggtcgaagcctgagccgttgaaggtgaccagcgtcggccgcaacgcatccacgcgggcggcgaaggccgagatcagggcgatctcgctccggtctccgatgtgcggggcgcccagcgatctgatccgccacacgccgtccgtgcgctcggcgacgagcgcggcgagcacagcgactttgtggagcggaagtttggggaatttctcgccgagaatttcggcggcctcatcgtcggtgagggtctcacggccatgcaagcgcgcgagcgtctcagtgcaaggcacggtttcgagatcgaagacgatggtgtgctggctcaagagacctccgggctacgaaggagcattgtctcgcgtttgaatgatttgtcatccaaaccacgacgcggccgcttgttggttttggcgtgcacgttggttgaccgttcggcccaaatcaccggatacaaagtcggtccaaaacggtttcacagcaccgaggttcggcgttgatttgattgggaaaagggcggtctggcgaaaatcctagttccccagccatcctcttcttccgacatcaggcgtcattcgcggcttcggttaccttggccaagtgcgcgcccaccgcctcgatgcggcgctgaccaagcgcacgccggcgggtgagcaggtcgggcgatccggcgtcgtaatccttcatcagccgctcgacaaaggcgccggaacgcacattcgccagcacctcgtccatggcggcgcgcgcgggctcgccgatgatgcaaggccccgtgtcatacgcgcccagttccgccgtgttcgagatgcgcccgaaggcgccggcgacgccacgctcgtgcatcagatcgaccacgagcttcagttcgtagaagcattcgaaccaggcgacctccggcggatagccggcgtccaccagcttcgaaaacgccgcatccaccagttcggcggtcccgccgcacagcaccacctgctcgccgaacaggtcgctttcgcactcgtccttcatggtggtttcgagaatgcccttgcgcccgcaccccagccccgccgcataggataagccgagcgcatgagcctggccgctggcgtcctgatgcacgccgaacaggcaaaagacgccctgcccctcctcatagaggtcgcggatgcgcggcccgatacccttgggcgaggcgaggatgacgtccaggtcggagcgaggctggaccaagccaaatcgcaccgacaggccatgggcgaagatcagggccgcccccggacgcatcgccggctcgagttcgtctcgccagagatcgcggtgtccctcatccgaaaccatgaccgcgacaacgtccgcctgagcggccgcctccgccgccgtcacgacgccaaaaccatcggcggccgccttcgcccgcgtggccgatcccgctttcagtccgataacgatgtcgtcgacgcccgagtcgcgcagattcagcgcatgggtgcggccctggctgccgtagccgatcacggcgacgcgcttgccccggatgatcgacaggtcgcagtcgcggtcatggaagacgggaagcggattgggtagggtctgggtcatgagcacagacatagcgccctccgacgtcatcgccttctggaaagaggcgggagccgacaagtggttcgccaaggacgccgccttcgacgccgatttccgcgagcggtttggacaggcgcacttcgccgccgcccggcgcgagttcgacggctggatgcagtcggcggagggagccctggccctgatgatcctgctggatcagtttcctcgcaacgtctttcgcgggaccggccacgccttcgccaccgatccgctggcgctgagcctggcgcgtcaggccttggcggccggctttgatcaacggacggagatggctctgcgccgcttcttctacctgccgttccagcactcggaagccatggcggatcaggatcgggcgcttgcgctgttccaggcgttggaccgccccgccaacgatcgctgggccgagcatcaccacggggtcatcgcccgcttcggccgttttccgcaccgcaaccgggcgctcggtcgcgagacgacgctggaggagcaggcgttcctggatcaggacggctttacgggctgatagctgtggagcgtgcgaaaccatcagaggcgcacgacccgaatcgctgtcatcctgcggccatgagcgccgtcctcagcatcgccgatcacgttcgcccgcacgctgctgcggatcatccggaatggcagtacctcaatctgctgcgcgacatcctggacaatggctcgcgacgcgatgaccggacgggcaccggcaccctgggcgtgttcggccgtcagatgcggttcgacctgtccaggggctttccgctgctgacgaccaagaagctgcacctgcgatccatcatcgtggaactgctgtggtttctgcgcggcgacaccaacaccggctggctgaaggagaacggctgctcgatctgggacgagtgggctgatgagaatggcgatctgggcccggtctacggcaagcagtggcgctcatgggcgacgccggacggccgatccatcgaccagatcgagcgtttgatcgaaggactgaagaccaaccccaacagccgccgtcacatcgtctccgcctggaacccggccgatgtggaggacatggccctgccgccctgtcactgcctgttccagttcttcgtcgcggacggaaagctgagctgccagctgtatcagcgatcggccgacgtcttcctgggcgtgccgttcaacatcgcctcctatgcgctgctgacgatgatggtggcccaggtcgtggggctcgagcccggagacttcgtccacaccctgggcgacgcccacctgtatctgaaccacctgaagcaggccgaacttcagctgggccgcgagccgcgcgcgctgccggtcatgaccctggcgtccaagtttgacctgttcgccttcgagcccggtgacttcacgctgagcgcctatgagcctcacccgcacatcaaggcggcggtcgcggtctgatggcgtctttgacgctggagcggctgagcgccgacgtcgcgcgaatctccgacatctatgcggccgagcacggcatcgatcgcgatcgtgactgggcgatgctgaagctgcaggaggagcttggcgagctgacggccgagcacctgcgcctgtcgaaccgggctcggggcgagggcgaccctgacgctctcggcgacgaggcggcggacgtgctgggcatgctgctgatctattgcgcacgcgccagcgtcgatctggaggccgccatgcagcgcaaatggctgaactggctggagcccagggcatgagcgccaagattgttctggtggtcgcgcgggcgcgcaacggcgtgatcggccggaatggcgacctgccctggcggctgcgttcggacctgcagcggttcaaggccgtgaccgtgggcaagccctgcatcatgggccggcggacgtgggagagcctgccgctcaagcccctgcccggccgtctgaacattgtcctgaccagggacggctcctacgaaaccgacggcatggccaagggcgcgctggtctgcgccacgcttgaagaggccctggccatcgcgcgcgagacggcggcggaggacggcgtggacgaggtctgcgtcatcggcggcacggccgtattcgaggcggtcctgcctcgcgcgcaccggctttacatcaccgaggtggacgcggctccggaaggcgatgccgtgttcccccccttcgacgaaaccgcttgggccgagacttcagcggaacacgttggggcgggcgacaaggacgaccacgccatgacctttcgcgtgctggagcgccgctagaggcccagcgtcccagccacggcgccggcgacttcggcgaaacgacgcgcgatttcgccatcgggatgtccgacgaccagcggacgccccgcatcccccgcttcgcgcagggcggcgtccagcggcagatcgcccaagaaagggatcgacaaacgcgcggcctcggcctcgccgccgtcccggccgaatacgggtccgctcatgttctcgatcagacccagcgtcggcacgcccacgcgctggaacagggtgtgcgcccggcgggcgtcggccagagccacctcttgaggcgtggtgacgatcaccgcaccatccagcggcgtcttctggatcagcgtcaactgaacgtcgcccgtgcccggcggcagatccaccaccagcacgtcaagcggcgtctcggcctttccccagcgcgtctggcccagcatttgggtgatggcctgcgaggccatgggtccgcgccagatcatggcgtcgtccgccttggtcagcagcccgacggacatcgccttcagtccgtgcgcctcatgcgggacgatggcgccgtcctcgtacgccggttgccccgacaggccgagcatggtcggcagcgaggggccatagacgtccgcatccagaacgccgaccgacaacccctgtgcgctcaaggccgcagcgaggttgaccgcgacggtcgacttgccgaccccccccttgccggacgcgaccgcgagcacgcggcgcacatgggccgggcggttcgtcgccacgggcgcctttgcgcgcccctgatcgacggcggcgggcgacagactggcggcgcggcgtggcgctggcgcggtgggcgtctccgccgtcagcaccaccgaaacgcgcgagacgcccggcatggcacgcagcacggcttcggccgcatcgcgcacgggcgcgtacagcgcggtctgtccggcgggcgcctccagcacgaatccgccccgatcgtcggccacgaccaagccttgcaccagccccgccgacaccagcccctgacccgaactagggtcgatgacgcgttccagcgcagccaggacggcggatcgttcgaccatgacgatttcctttgacgcttgcgggcgggtggggcgcgttctatcgtcggaaccgtttctgttcgagcccggatttgaccactcagccgcgcatcaccctgctggccggccccaccgcctcgggtaagtctcgcctggcgatgagactggcgcgtgagactggcgcgctgatcgtcaacgccgacagccagcagttgtacgccgacctgcgtgtgctgacggcccgcccgtcgccgcaggacgagtccgaggccgagcacgccctctatggcgttgcggacgcggcggacgcctggtcggtgggacgctggagccgtgcggcgttgcagcagatccaggccgccgaagatcgaccggtcgtgctggtcggcggcacgggcctgtacttcatggcgctgacgaaggggttggctgagatcccgccggtggcggactccattcgcgccgagctggagtgcgattttgacgttcaaggggaagcggagtttcgcgcgcgtctggctcaggacgaccctgcctccgccggcgccgtcgagcgtggcgaccgccagcgtctcgtccgtgccgccagcgtgctgcgcgccagcggcaagcccctcagcgcctggcgcgccgacacccgcccgctcctgcctgcggcaagctggtccggcctggtgatcgagcctgaccgcccggcgctctacgccgcctgcgacgcgcgcgtggacgtcatgatggccggcggggcggcggcggaggttgaagccctgctcgcccgccgtcttgatccctcgctcccggcgatgaaggccgtgggcgtgcgtgagctcgcggcctggatcgcgggcgaaacgacatgcgaagcggcggtggaggcgctgaagcaggcgacccggaactacgccaaacggcagctgacctggttccgcaatcagacgcccgattggccgcgcaccgccccgtgaggcgtcgttgcccgaatcatgtcagcgctaggggtgtagggagagaacgaccatggcgatgacgcgcggcctgctgctggcgggcttcctgatggcttccaccgccgtgcaggcgcaggagccatggcaggtgaagcaggcgtgggtcagcgcccacgagtccttcctggctggcgaggcgctgcagggacgcggcagcgcgacacgcgacgaggccatcgccgccgcctacatggcgtcccagttcgaaggcttcggcctgacaccgccgccaggcatgacatccttcttccagacgacgggcgtgacacggatcacgcccagcggccaggccgacctgaccgtaggcgacgtcacggtggcggaaggcgcggggctgacgctgctgatgtcgtcgggacagtcggcatcgggcacggcgcagatcgccggagccgatcccgccgccttgccgcaggctgcgatcgtcatggttcccgacatgggcgcggcctcggtcggcgcctggatcggcgcggcggcggccaagggcgtgcaggtcctggtgctgcgcgagaacgaggcgctgacgcagcgcatcagcgcagccggcggcaagacccgcacgcccgttgccctgaccacggaagcggcgacgcggcgcagcccggaggtcgcggtggtctcggccgagatgttcgaccgtcttgccgccttggccgacgctcaggcgaccctggacctcggcgaggtcacgcggacagagagccccaccaccaacgcgatgggctatctgcagggcagcgatccttccgctggcgtgatcctgatcagcgcgcacctggaccacattggcgtgcggccggacggcgtggtgatgtacggggccaacgacgacgcctcgggcgtggcggcggtgctggagctggcgcgcgccatggcggcggccggccagcccaagcgcagcatcctcttcgtcggctacggcagcgaggagatagggcttctcggctccaagtacttcgccgccaacccgccggtgcccctgaccgacatcgtggccaatctcgagatcgagatgatcggtcagcaggatccaaagatgccggccggtgtgatgatgatgacgggctttgatcgttcgaacttcgggtcggagatgaaggcgcgcggcgcgttggtcgcgcccgacccctaccctgagcagaacttctttgaacggtccgacaactaccagctggcgctgcaggggatcgtcgcccacaccatttcgggctgggcggtgacgccgacttaccacacgccggaagacaccatcgccaacctgaacctgcccttcatgacccaggcgatccagtcgctggtcgagccgctgcgctggctggccaacagcgacttccgaccggagtggacggccgaggggcggccgcgtcagcgctaggccttggcatacggccgcacgccactatattggccttgttcgggttcgcccggactatggcgataaacgcgcttgtaataagcggaccggacccgggtgcgattcccggcggctccaccatccttccccgcgttatcggcggagcgagcatggggccgactagcatcgacggacgtgtaaagaagactgctttcgctcgtcctggcccaccgtatcgggcctttttctaactgcgaacgataacttcgctggagaagtccgcctcgccgcgtaatgcggttcggttgatttcgaatcttaagtcctaggggttcagatccctgggcggggcccggagggcgcctggcaacagaagccctccacttttctcaaaaatcccccgcgcgcgcgccctccccgtctttcgtccgggcgcgtgcgcgtctatgggtcgcctcgccagcagccgaggtgacgatgaccgaccagaccccgccggtcgacgagatggactatgagacgatgacgcacgaggccttgcggacggtgatccgcgatggcctgctgcgcgccgcctcccccgccggcctgccgggcgcccaccatttctacatcaccttcaagacccgcgcggccgacgtgtccgtgccgcccgacatcctcgccaaatatccggacgagatgacggtggtgatccagcatcagtacgaggatctggacgtccagaacgaccgcttttcggtcaagctgcgctttggcggcatcccgcgcgtgctggccatgccctacacggccgtgacccgcttctacgatcccagcgtgcagttcatgcttcagtgggacgaccccgaggtgatcgaggagcctgcgccggctccggagccggacgcgccggtgcccgtcgccgacggccccaaggtcgtttcgctggatcagttccgcaagaagtgatgccggcggatcagcggcgcggaaagctccgcaccatgatccgctcgcgctcgccttcgaaccgctccacgatcagccgcgccacttgcgcgtcgtcgtggaacaggtaccccttgatggcgtccaggatggccttggccagattgtcgaggtccatgatcggcggctcgccgacgtgctccatccggatctcgaccacgtggtcgccccaggacggccgcgcgccgcgccactccttgcgcatgaattcatagatcagcggcttgtagtatttcgcctgggtggtcaggccgtcgacagtgatctcgacggcgtcgccgttctcgcgggctcgcaccttgcccgcgccgacccagccggtggtcatcgtgacggcctcgccttgccctgcatggctctcgtgctacacgcctcgtcccatcaccgccacgcctgaagtcgagcccgtacgatgagcaacgtccgcaccgaaaccgacaccttcggcccgatcgaggtcgccgccgaccgttattggggcgcgcaggctcagcgctcgctgggcaacttcaagatcggctgggagaagcagcccctgccgatcgtccgcgcgctgggtgtcgtcaagcgcgcggcggccgagaccaacatggcgctgggcaagctcgacgccggtgtcggcgacgccatcgtcaaggcggccgacgaggtgatcgagggcaagctgaacgaccacttcccgctggtggtctggcagaccggttccggcacccagtcgaacatgaacgccaatgaggtcatctcgaaccgcgccatcgagatgctgggcggcgagatgggctccaagacgcccgtccaccccaacgaccacgtcaacatgagccagtcgtccaacgacacctaccccacggccatgcatgtcgcctgcgccgaggaagtagtgcaccggctgatcccggcgctgcagacgctgcgcaacgccctgaacgacaaggccgcggcgtggaaggacatcatcaagatcggccgcacccacacccaggacgccacgccgctgacgctgggccaggagttttcgggctatgttcagcaggtcgagaacggcatcgagcggatcgagcaaaccctgcccaagctgatgcagctggcgcagggcggcaccgccgtcggcaccgggctgaacgcgcccgtcggcttcgccgaaggggtggcggacaagatcgcctccatcaccggcctgcccttcaccaccgcgcccaacaagttcgaggccctggctgcccacgacgccatggtcttcacccacggcgcgatcaacacggtcgccgccagcctgttcaagatcgccaacgacatccgcttcctgggttcaggcccgcgttccggcctgggagagctggcgctgccggagaacgagccgggcagttccatcatgccgggcaaggtcaaccccacccagtgcgaggccctgacccaggtgtgcgtgcaggtgttcggcaacaacgcggcgatcaccttcgccggctcgcagggccacttcgagctgaacgtcttcaatccggtcatggcctacaacttcctgcagtcggtgcggctgttggccgacgcggcggtcagcttcaccgagaactgcgtggtgggcatagagcctcgcatcgacaatatcgagcggggcttgaacaactcgctgatgctggtgacggcgctgaacggcaagctgggctacgacgcctgcgccaagatcgccaagaccgcgcacaagaacgggaccaccctgcgcgaggaggccgtcggcggcggctatctgacggacgccgaattcgacgaagcggtgcggccggagaagatgatctctccgcagtaaccggctgtaaaacgaaaaaggccccgccggtcgccggcggggccttttgcatttcggagagagagccgcctagtgcttctctgtccagcgttccttggcctcgtccttggtgatcgacaggtggacgtgcttgtcgtccacgcgctggacccaggagaccgggatcaggtggtgcttgaagccgccggcgatatcaagcttggccagttcgatctgatcgcccagcacatgatcgacgcgaccgacgtgaccgccgtccgagcccagcacttccagatgttccttgatgtcggccgagttgatcatgagggttcctcgcgttgatgcgtcatggcagattgcctgcgggggtaacgcgcccgggtctttgcggtttcggacggaggaggacgccgcatgggcgacgtcgtgaacctgaatcaggcccgcaaggccaaggcgcgcgcggaagacaaggcgcgcgccgccgcaaaccgcgccgcccacggccgcagccgcgccgagcgcaagcaggcggaggcggacaaggcgcgactctcctgtcatctggacggcgcaaggctcgacgagtgagaggcgcgtaatgcggttgcttcaggcttggggcgagcggatcagcagcagttggcccgccagcaccagagccagccccaggaacgccgacaaaccgaatcgcgccccttcgaacaggacggagaccagcatggcgatcggcggcgtcagcgccgagatatagctggcggtcgcatatcccttcagccgcgcgatcgaaaaataaagcccgaacgcgatcaccgagccgaacagcgccaggtacagcagggccaacagatagctgaggtctgtctcgatccgccactcaacccccgtgaggaggccgtacagcgccagcatgcccgtgccgtacgccatggcccaggccgtggcggtggcgatcggcgcctgcgcctgctgcccgcgccaggcgaagtagttgccgaccgtggagctgaaggtggcgatcagggcgaaggcgacgcccgccagcgcggtgcggtccatcccggccgccactatctcgccgccggacagcacggccacgcccatgaccccgcacagggcgccgccccaggcggctcgcgacgccttctggccgaccacgatgcggaacatcgccaggttcaggaaggccagcgccgcgaacatgaccgccacgaccgccgaggccaccctctcctccgcggcgtagacgaagccgtaggaggcggcgaagacgaacgccccctgccccagcgcggccagatgctggttccggttcatccgcaccggccgccgcgtaaccaagcagaagccgaacatcaccagcgccgacagcccgaaccgccatacgaccgagacggtgggatcgaccacgcccagttgcagcgtgatcgcataccaggtggtgccccagatcagggcgcagacgaccacgccgccgatggccaagccggcgggcgacaggatgcgggcggggtgggtcatggggcctcgaaagcgtgcgacggcggcggcgcggccaccgatgctcaatgcggcgcttcccttcggccgtccagatgtgtcaccgctcgctgcggaggaacccagcccatgagcggattgaccaagcgttcggtgagcctgtccggccatgcgacctccgtggcgctggagccggagttctgggcgatcctggatgcagtggccgaagccatgcagctgtcacgcgcggcgcttctgatccggatcgacgaaagacgcgggcgtcggcccctggcctcggcctgccgtcttctggcgctggcctgggcgagcggcgatcgctccttcgcggccgatccgggctgacttccgccgatgtgctacttatgttctcacctcgattcagccgtcttgtgaagtcccccgcccgccgtgaccgacctgccttttccccgtatctccgatctggcgcgcgcgcggccgcccgcgggacttgcgccgacgcacgactatctcgccggcctgaaccctgagcaacgggaggctgtggagacgaccgaggggccggttctggtgctggcgggcgcgggcaccggcaagacccgcgtgctgacgacccggctggcgcacatcctggcgacgggccgcgcacggccttgggagctcctggccgtcaccttcaccaacaaggccgcacgcgagatgcgcgagcggatcacccatctgatcggccccgacgcggagggtttgcgctggctcggcacctttcactccatcgccgcccagatcctgcgccgccacgccgaactggtcgggctgaagtcgaccttcaccatcctggataccgacgaccaggagcggttgctgaagcagctgctggaagcggccaacatcgacacaaagcggtggacgccgcgttcgctgtcgggcctgatcgatcactggaagaaccgggggtggaccccggacaagctgccgccggccgaggatttcgccaacggcaagggccagggcctctacgcggcctatcaggcgcgactgcgcacgctgaacgcctgcgacttcggcgacctgctgctgcacaacatcacgatcctgtcgcagcatgcggatctggcggaggaatatcgccgccgcttccgctacatcctggtggacgaataccaggacaccaatgtcgctcagtacctgtggctgcggctgctgaccgcctcgaccggcaacgtctgctgcgtcggcgacgacgaccagtcgatctatggctggcgcggcgcggaggtggacaacatcctgcggttcgagcgcgactttcccggcgccaagatcgtcaagctggagcgcaactaccgctcgaccacccacatcctgggcgctgcctccggcctgatcgcggccaaccgcgaccggctcggcaagaccctgtggaccgaagcggatggcggcgacaaggtgcgggtgcgtggggtctgggacggcgaggccgaggcccggctgatcgccgacgagatcgagaccgcccgccgcacgggctgcaaatacaaggacatggccgttcttgttcgcgcatcgtttcagatgcgggcgtttgaagagcggttcgtcatgctggcgatcccctacaccgtcatcggcgggccgcgcttcttcgaacgcgccgaaatccgcgacgcccacgcctatctgcggctgatcctgtccgaagacgacgatctggcgttcgagcgcatcgtcaacacgcccaagcgcggcgtcggcgacaccagcgtccagaagatcctgcacatcgcccgccagcacggcctgtcggccatgacggcggtgcgcggcctgatcaacaccgacgaactgcaggcccgcacccgcaccgccctgtccaacttcgtgcgcgacctggatcgctggcgcgcgctgtccgagaccacgccgcactggcaggtcatggagacggtgctggaggagagcggttacaccgacatgcagaaggccgaccgcacgtccggccagacgcggttggagaacctcaaggagctggtgcagtcgatgcagcagttcgacacgctgcaggcctacctcgagcacgtttcgctggtgatggacctggatcgcggcgccggagacgacgccgtgcagatcatgacgctgcacggcgccaaggggctggagttcccgctggtcttcctgcccggctgggaggaaggcgtatttcccagccaacgctccatcgatgaaaagggcgaaaaggggttggaggaggaacgccgcctcgcctacgtcggcgtcacccgcgccaagcaggacgcccgcatatccttcgccgccaaccgacaggtgtacggccgctggacatcgcagctgcccagccgctttgtcgacgaactgccgatcgcccacgtcgaggcgcagtccgacaccggctactacggcgcatccagcggcatgaaggaggccaagagccggtgggacgacgttcccagcttcggcaacagctactcctctcccggctggaagcgggctcagaccttcaccgccgcccagcctccccgcccaacccacgctcgccgagccgtcatcgagggcgagggtcgactggtcgccacggccgaccccaaggcgagctcgggctggaccaagggccagcgggtgtttcaccagaagttcggctacggcgacgtgcgcgtggttgagggcaacaagctgctggtcgacttcgaaaaggccggcgagaagcgcgtcatcgacacctttgtcgaaaaggcctgagccgcccagcgcatgaaagagagcgcgccccgcgaggagcgcgcccttttacttgtcggatcgccctagtggctgacgacgacggccgcgccgtcgaccggcggttggggcgcaggcaacggctcggccgcctcgtcccattccgttggcgtcagagcgcccgtcagggcccagctcaaggcttcgtccgccgtggagatcggcacgatctcaagcgccgacttcacattgtccggcacgtcggcgagatctttttcgttctcctgcgggatcagcaccgtcttgatgcccgagcgcagcgccgccagcagcttctccttcagcccgccgatggcggtcacccggccacggagggtgatctcgccggtcatggcgatgtccttgcggatcgggatgccggtcaggacggaaaccatcgcgacggtcatggcgacgccggcggacgggccgtccttgggcgtggcgccgtccggcacgtggacgtggacgtcggtcttctcgaacaccggcggcttgacgccgaagctgagcgagcgagcgcggacataggaggccgcggcggacaccgactccttcatgacctccttgaggttgcccgtcacggtcatgcggccgcgaccgggcatcttgatcgcctcaatggtcaagatgtcgccgccgaactcggtccaggccaggccggtgacgatgccgacctgatcgttctcgtcggtctcgccatagcggaacttcttcacgcccgcatactcggccagcttgtccgcatcgacggtgatggacgccgcgttggtcttggccatctcgcgcacggccttgcgcgccagtccgcccagagcgcgctcgagcgagcgcacaccggcctcacgggtgtagtagcggatcaagtcgcggatcgtgtcttccggcacgatcagttcgccgtccttgagcccgtgatcgaccagttgcttgggcagcacatggcgcttggcgatctcgaccttttcgtcctcggtgtagccggacacccggatgatctccatccggtccatcagcggctgcggcatgttcagactgttggcggtcgtcacgaacatcacctgcgaaaggtcgtagtccacctccagatagtggtcgccgaaggtcgaattctgcgccgggtccagaacctccagcagagccgaggacgggtctccgcgccagtcggcgcccagcttgtcgatctcgtccagcagcacaaaggcgttggtggtcttcgccttcttcatcgactggatgatcttgccgggcatggagccgatgtaggtccgacggtggccgcggatctccgattcgtcgcgcacgccgcccagcgacatgcggacgtattcacgtccggtcgccttggcgatggacttggccagcgaggtcttgccgacgcccggaggtccgaccaggcacaggatcggtcccttcaggctgccggtgcgcgcctgcacggccagatactcgatgatccgctccttgaccttctccaggccgaagtgatcctcctcgaggatgtcctcggcgcgggcgagatcgatcggcttctgcttggccttgccccacggcacggacaacagccagtcgagatagttccgcacgaccgtcgactcggccgacatcgggctcatgttgcgcagcttcttgacctcggcctcggccttggtgcgcgcctccttggatagctttgtcttccggatgcgcttttcgagctccatgatctcgtcgcgctgatcgtcggtctcgcccagctcacgctggatcgccttcatctgctcgttgagatagtactcgcgctgcgtcttctccatctgccgcttcacgcggctgcggatcttcttttcgacctgcaggacgctgatctcgccctccatcaggccgtagaccttctccaggcgctgcggtacgtcgatggtctcgagcaggccctgcttgtcgctgattttcacggacagatgcgcggccacgctgtcggccagcttggaggcgtcggtgatctgcgggatggagctgagcgcctccggcggcaccttcttgttcagcttcacatagttctcgaactgctcgaccacggcgcgcagcatcgcctcggcctgtgacggctcgcccggctcgtcggcgatctcgacggcttcggcttcgaaatattcggtgcggtcggtgaagcgcgtcagccgcgccctgcccttgccctcgaccagaaccttgaccgtgccatccggcagcttcagcagttgcagcacgctggccagcacgccgattgggtagatggcgtcgggtgatgggtcgtcatcgacggagttcttctgggtggcgagcaggatctgcttttcgcccttcatgatctcgtccagcgccttcaccgacttttcgcggccgacgaacagcggcacgaccatgtgcgggaagacgacaatgtcccgcaggggcaggacgggaaggatcttggtctcggacatatgcacactcctgggcccttgatgatctccggcccgccgccgcgtccgcctcggcgtcatgctctggcggatcgaagcggcccgtcgattccgacggcgttcggctgagtatgtggcctctgggcggcagggttcaagcgtggcggaaagagcgccggccacatcgtgcggccaagccacgcgcaaagaaaaaggcgagcccgccggctcgccttatccggttccaatcgaccgcctggatcaggcggctccgtcggccttcttcttggaggcttcggagtagatcagcagcggctgggccttgccgtcgatcacctcggcgttgaccaccacttcctcgacgccctcgaacgtaggcagttcgaacatggtctcgagcaggatgccctctagaatggagcgcaggccgcgcgcgccggtcttgcgggtgatggccttcttggccaccgccatcagcgcgtcctcggtgaaagtcaggcctacgttctccatctcgaacaggcgcttatactgcttgaccagtgcgttcttgggctctgtcaggatggtgaccagagccttctcgtccaggtcctccagcgtggccagaaccggcaggcggccgatgaactccgggatcaggccgaaccgcatcaggtcgtccggctcgacgcccttcaggatgtcgcccgtgcggcgttcatcaatctccttgaccttggcgccgaagccgatcgaagccccctcgccccgcgccgaaatcaccttctcgaggccggcgaaggcgccgccgacgatgaacaggatgttggcggtgtcgacctgcaggaattcctgctgcgggtgcttgcgtccgccctgcggcggcacggaggcgacggtgccttccatgatcttcagcaaggcctgctgcacgccctcgcccgagacgtcgcgagtgatggacggattgtcggacttgcggctgatcttgtcgatttcgtcgatgtagacgatgccgcgctgggcccgctcgacattgtagtcggacgcctgaagcagcttcaggatgatgttctcgacgtcctcgccgacgtaaccggcctcggtcagagtcgtggcgtcggccatggtgaagggcacgtcgatgatgcgcgccagcgtctgggccagcagcgtcttgcccgagcctgtcggtccgatcagcatgatgttggacttggccagttcgacgtcgttgttcttcgtcgcgtggttcaggcgcttgtagtggttgtgaaccgcgaccgacagcaccttcttggcgtgcgcctgaccaatcacgtaatcgtccaggacctcgcggatttccttcggggtcggaacgccgtccttggacttcacgaagccgatcttgtgctcttcgcggatgatgtccatgcacagttcgacgcattcatcgcagatgaacacggtcgggcccgcaatcagcttgcggacttcatgctggctcttgccgcagaaggagcagtacagggtgctcttggcgtcggcgccggctgctttggtcatggacccttcttttcactcccgcgatgcgcctcgacatgaggcgaaacgcgcttactccgcgttgattccgtaatcctggtcgcgaaggtcttcaaaaaatgacaatcacctatcgttcgtcccgccacaaccccgaaggcgacagggggatgctgcgaggcgacaatgggtcagactcaacgaggatcacggcgaatgtctgacatggggaggaccgagccgcttcgccacttcccgtcgttcgatcccgcgggccgtcccatcgtggcgttcgactttgacgggacgctgacgatccgggacagtttcaccgagttccttcggtggcgtgcggggccgggcggttgggcgctaggcctggtgaagctcgcgccggccctggcgcactatgcgcgcgatcgggatcgtggacggatcaaggcggcctcggtgaaggaattcctcagcggcgtctcgcgagcggaactcgacgccgacgccgagagattcgccgctgactcatggtcgcgcttcatgcgtccggacgctctcgcctgctggaacagctggggagaacgcggcgcttatcgcgtgatcgtcacagcctcgccggaggataccgtggcgccgttcgctcgccggctgggcgccgacgcgctgctgggcactcagatcgcctttgacgaacgagatcgggtcacgggcgccttcgccggcgagaactgccgcggcgcggaaaaggtcaaccgcctgcgcgccgccttcgggcccgacgtccgcttgcgcgccgcttacggcgacacatccggagacacggagatgctggccatcgccgaggaacccggcttccgagcgttcacacagaggccctgacggtcagcgcccatcggcgtccacgtcaaacaccatcgccttgccgcgcgaagtgggagaccagcccgcctcaatcaccgacgcaacggcgtttcggacggcgtcgacgttgacgcgctgcttttccacgtccgggtgcccgttcgcgcgcatgggcatgggaaactggacgatagcttcgcgcttgaaacccttaaggcgcagcgatagtgccaggccgtcccacttacccccacctttcggctggggctgacggcggatttcccactcataggtctcgccatcgacttcgacgacgccgcttgggtctcgcgtgtgttgcatccggcactgatagcacaaaagaaaaaggcgcaccggtgagggtgcgcctttccgtgctcaaccgcagccggatcaggcgccgggcgtctttactccatcggcgtcagcctgttcgcgacgatcgtagacgtggtccacgataccccaagccttggcttcctcggccgacatgaaatggtcgcggtccagcgtgttctcgacctcctccagcgtccggccggtgtggtggacgtagatctcgttcagccggcgcttggtgtaccgaatgtcctcggcgtgacgctcgatgtccgaggcctgaccgcggaagccgccggacggctggtgcaccatgacgcgcgcgttcggcagagcgattcgctggccggcctcgccagccgtcaggatcagagagccggccgaggccgccatgcccatcacgaccgtcgaaacggggctcttgatgtactgcatggtgtcgtagatcgcgagcgccgaggtcacctgaccgccggggctgttaatgtacatgctgatttcctttttcgggttctccgattccagaaacagcagctgggcgcagatcagagacgccatgccgtcctcaaacggcccggtgaggaagatgattcgctcgcgcagaaggcgcgagaagatgtcgaacgaccgctccccacggctcgactgctcgaccaccatgggcacgaggttggattgcagatagtcgatcggatcgcgcatgaaggccttctcggatgcgttgaacaggcgcgactcgcttggtcgcccgcccttgctctgcatatcgcgttccgaaggctgcgccgcaaggtcggacaacgcacgtgaaaaagggcggagccgccgactccgccctttcgatcgaccaggatcggaggagatcagccctcttcgtcttccttcagcagctcttccttggtgatcggcttgtccgtgacgtcggcgacgccgacgatcaagtcgaccaccttctcctcatagatcggcgcacgcatctgcgcggcggcgttggggttctggcggtagaagttcagcacctgctgctcctgccccggatagttgcgggcttcctgcaggatggcggcgttcagctcctggtcggtgacctggacgttgttggcgcgaccgatctcggccagcaccagacccaggcgcacacgacgctcggcgatggtgcggtactcggccttcaggtcctcatcggacttggcggcgtcttcctcaggcaggcggccggccgacttgtcggcttcgacctgctgccagatgccgtcgaactcggcttcgaccatcttcggcggcagcgggaagtcatgcgcttcatccagctggtccagcagggcgcgcttcagcttgaagcgtatctggcggctgtactgctggtcgaggttcgacttcagcagttccttcagcttgtccagcgactccaagccaatgcgggtggcgaactcgtcgtcgatcttcgactcggcctcggccttgatcgccttgaccttgacgtcgaaggtcgcagccttaccggccaggtgcttggcctggtaatcctcggggaaggttacctcgatcgtcttgtcttcgccaacctttgcgcccgtcagctgctcttcgaagccggggatgaaacggcctgagccgatcaccaggtcggcgtcctcggccgagccgccttcgaacgcctcgccgtcgatcttgccgacgaagtcgatggtcagttggtcgccgtcggccgccttgaccgacttgcccttcttgtcttcgtagatcttggcttggccggccagttcggtcagcgcctcgtccaggtcggcgtcggaggcctcataggtcggacgctccagcttcagcgtcttgggatcgacgggcgtgaagtcgggcatcacctccagcgccatctcgtaggacaggtcttcctggcccgcgacgaccttgtccatgtccgaaaccagcttcatctcggccagggcggcggggcgcagcttggcctcgtccagcgccttttggctggtctcgttcagctgggcgttgatgatctcgcccatgaagtcgcggccgaaggtcttgcgcacgtgcgaggccggcaccttgcccggacggaagcccttcagcttcatctggggggcgacttccttgatgcgctggtcgagcttggcgttcagctccgccaccgggatggtcaccgcgatcacgcggctgaggccttcgttcgacttttcgacgacttgcatggtcgggattctgacgctctggggcgccggggccatgaacggccggcgcggagtggataaagcaagagagccgcccccgtcaggagcggcgcctcgaagcccgcccttatgtcgaggcggagttcaaaggtcaacgcggcgatggttttgcgcgcgcctccgccttgctagacaggcggcatgacccagaccggctctcccatcggcgtcttcatcacgccggtcactccgctgcagcagaactgcaccgtcgtctggtgcacgcacacccggaaagcggcggtgatcgatcctggcggctcggtcgatgcggtgctgggcgaggtcgcccggcggggggtggcgctggaccagatttggatcacgcacggacatctggatcacgccggcggcgcggccgagatgaaggagaaatccggcgtccccatcataggacctcacccggacgacctgttctggatcgagggcatcccggcgcaagggcagatgtttgggctgcccgaggcgcgcaccttcacgccggatcgatggctccaaggcggcgacacgctgacgctgggcgagacgagctgggaggtgcggcactgccccggccacacccccggtcacgtgatcctgttcaatcgcgccgcaaggttcgcccaggtcggcgacgtgctgttcaagggatcggtcggccgcaccgactttccgcaaagcgatcccgccgcgctcgtccgctcggtggtcgagcaactctggccgctgggcgacgacgtgacctttgtgccggggcacgggccgcattccacattcggcgaggagcggcgcagcaatccgttcgtatcggacgcggcgctgcgccggacgccggtcgagcgccccgcgaccggccccgcctgaagcgttggtcagcggctgatcagcacgcccagcagcacgcccgcgatcaaagcatagaaggtggccttcagcggctcctcgacgatgcggtcgcgcgtgtcggcggccgtggtctgagccagggccttcaccttgccggcgtcttcgcgcaccgcctgccgcagcgaggcgacgccttccccgatcgcggtcgtaccttcggttcccgtggaggaaccggccagcaaagcgtcggcgtcgcgctccagtcggcgcgacatgtcgtcgccctcggtgatgatgtcgtcgggcgtggtcgagggatagctgtcggtcattgccgtctccgttgaaaggcttgtcctttgtcgggcgaacaacccgccagcacatcggcggttcctgtgtctgcccttgtgaacggcggcgtcacgcgtgcgttggctaaggacaggagacaaccatgacatacatcgaacccacccccactggcgttccgggcccggagatcgacccgagcccctcgccgcagccggaactcgacccttccgacacccctgaagaggcgccgccgctggagtcgggcggcggtgatcctggcgattctcggccctacgggtaggcgccagtcaaggtcgaaaatccttcaagatcagcggaccacgaaaactgaaatccggccggaaccgctccgattcaaccgggttcactttggtaagcgccacaacaatcaggaaaggacctcagatggcggaaggacagaccacacgcggctctggtgtttccaaacggggcttcgcctccatggacccggagcggcagcgcgagatcgcccgcaagggcggcgccagcgttcccagcgagaagcgcagtttctcgcaggaccggggtctcgcggcgcaagccggccgcaagggcggcgaagcgtcccacggttcgcgcaaggatgaagcgccaccgcccgccgagtaatcggcgcgcagggcgatagaagaagaggcggcgagctcaggttcgccgcctctcttgcatggatggtcgactgatcgtcagtcagttcgcggtgagcgtggccaaagccacggctggatcatcggagacgtcgaagcggcgtatcgaccaaccggcggcctcacccatggtctccaccatctcgcgcgtgaacttgcgcgagctttcggtgtgcagcgtctcgccggcctgaaacaggaacctccggccggccacatcgacgctggtcgccctcgtggcgcgcagatgcatctccatccgtgattggtccggtctccagaccgcgcgatgctcaaaggcgtccaggtcgaagtcggcgccgagttcccggttcgcccgcaccagcaggtttcgattgaacgccgctgtcaccccctggccgtcgtcataggcggctgtgagcacgcccggatccttgaccaggtcgacgcccaggatgaacagcgcctcgtcgcccagcatgcgacgcgcctcgcgcagaaagcgtatcgcctgctcgggctccaggttgccgatcgtggatcctgggaagaagccgatcttgcgccctttcccgagttcttccgggagggccgccaaggtttcgaagtcgcccagcacgggcgcgaccggcagggcgggatagtcctgcctcaaggccgtggccgcggcgtccagcgccgccttgctgatgtcgagcggcacataggccgccaggtccggtgcggcgtccagcaggatgcgggtcttctcgctcgcgcccgagccgaactccaccagcacagcttgcggtccgaacatggccgcgaggtcgccagccgtacgacgcagcaacgtcgtctcctggcgcgtcggataatactcgggaaggcgggtgatctcctcgaacagccgcgagccttccgcgtcgtagaaccacttcggcggcacggccttttgcgtgcgggacaatccctggatcagatcacgacgaaaggcctcgtgcgcatcctcgtctgtgtcgctttgcgtcgcagcggcgtcggcggccattcgcagtcccatgaaggcccacctttgctggggataaaagaagttgcggtaggtggttcgggcatgccccggaggcgtggcgaaggatccgccccgcagcaccatctggttggccatgaacttgccgttgtactcggcggccgtgccttccgtcggcttgaacccggggtacggctgataggcgctggacgtccactgccagacctcgccggccagattggtgaaggcgtcgggggtggtcgccgccgcgtgctcccattcggcctcagtcggcagacgcttgcccgcgaaccgagcataggcgtcggcctcgtagaagctgatgtggcgcacgggcgcgccggaatcgacgggcgcgcggccggtcagcgacatcgtcgtccagccgccgtccggcgtctgtctccagtacgccggggcggtccacccttccgccttcaccgtcgcccagccgtccgacagccacaggtccgatctcgcatagccgccagcgtcgatgaagccgatccaatcgccgttggtgactagatcgtggtccaacgcaaacggctcgagaaagaccttgtgcctcggcccctcgttgtcgaaggcaaatcccgcctcgtcggcgccgatctcgatcaggccgccgtcaaagacagtcgagccgccacgaggacgctccgcctcggtgtcgcggggctcggccgcataggccgcaggatcgagcggggagcgcgacatcaggtgcagcagatccatcaggaacaactcctggtgctgctggtcatggtgcaggccgagctcgagcagatagcgggtgaggccgtcggtgggcgcatcgctctaagaaggcggccatgcgcctgtcgatctcccggcgataggccatcacctcgtccagcgaagggcgcgtcatcagcccccgctccggccgcgccacccgctcgcccagcgcctcgtagtaggagttgaacagaacctgataacgctcatcgaccggtcgatagccaggctcgctcgccagcagcatggcttcgaagaaccagctggtatgcgccaggtgccacttgcccggactgcagtccggcatggattgagcggccagatcctcggccgagagcccctgcgccaactcggtcatacgagcgcgaatccggcggaagcggctgatctcggcggccgcgcggggatcgggctctaggcgtacgttcatggcgctgcctccgactgctccatgaacggctgcttatggtcaaggttccgcgttcccgcagcctttatccttgaagcggccatactccagccgggcgatggtgcggttatgcacctcgtccgggccgtcggcgatccgcagggtccgcaccgaagcgtaaagctccgccagcggcgtgtcggccgagacgccggcgccgccgaacgcctgaatggcgtcgtcgatgacctgcagcgccatgcgcggcgcagccaccttgatctgggcgatctcggagcgcgcgcccttcgcgcccacctcatccatcatccaggcggccttgagcaccagaaggcggcacatctcgatgttggtgcgcgcctcgccgatgcgctgctcccacaccgaatgctcggccagacgctttctgaaggcggtgcgcgacagcagccgctcgcacatcagctccagcgcccgttccgccgcgccgaccacccgcatgcagtggtggatccggccgggacccaggcgcccctgcgcgatctcgaaccccctgccctcgcccgcaatcaggttggcgaccggcacgcggacgttgtccagcaccacctcggcgtggccgatcggccgctcgtcatagccgaacaccgacagcatgcgttcgatgcgaaagccgggcgtgtccgtgggcacgatgatctgcgattgttgcgcgtgcgtcggcgcgtccgggtccgtcttgcccatgacgatggcgagcctgacgtttgggtgcgccatgttggtcgaccaccacttgcggccgttgatgacatagtggtcgccgtcgcgctcgatgcgcgtctggatgttggtggcgtccgaggaggccacctccggctcggtcatcagaaaggccgagcggatctcgccgtttatcagcggacgcagccaacggcttttctgcgcctcgtcgccatagaggtgcagcacctccatgttgccggtgtccggcgcattgcagttgaacacctcggccgaccacagatgccgccccatcatctcggcgagcggcgcatattcgagattgctgaggccggcgccggtctcgcccggcaggaacaggttccacagcccctcggctcgcgccgcggccttcatcgtctccatgacaggcgcctgacgcgacgggtcggcggcgacctgggcgcgatactcggcttcgcgagggatcaccttctgctcgaggaagtcgcgcaagcgcgcctgccactctagagcgcgatcgccgtgtcggaattccatgggcagtccccgatgcagaaacggcgcgggccccagggcgccgcgccgtcgatccgtttcgctagtcgtcgcgcatcagcgcttcagcagcggcgccagcttctgggcgatcatcatgtcgccggcaatcttcagcttgccctgcataaaggccatcatcggatcgaggcggccctcggaaagggcgatgaagtcgtcccacttcatcgacacggtggcgtctgcgggcttgtcttcgttcgtgacggtgttcgggaccgacgcgccgtcgatgaagatcttgtcctgaccgtcgagatcgagcttcacggtcttgccgaggccggagttgtcgccgacggcggcgcggattttttcggtgacttgagccagatcggccatgttgatcgtctccttgggacggtgggtggataaggcctagcgcgctccgcagagggcgccaagatcacgtcgggtaagcctcaggcggcggcttccttggggtctccgtcgcggaagcgccacttcatcaccagcacccaggcggacatgcagagggccacggcgttggagacggtgaccggccacgcctcggtcatcgcgccgtaaatcacccacaggatgaaacaactgaccgtcagcgagtaggtccggaggctaacggcggatgcgtcgcgcgtcttccagatcttgagcgcctgcgggatgaagctggtgatcgagcacagcgcggcggccgagccgatcacgttggccagggtctggtgatccatggccgggctaaagacccttcgccgggccgtccggctcatccggttcgccgtccgcatccttgtcgacaaagtgcgtcggtccgcgcctcatgggagacagggcgaacagagcgcccgcgagcaccacggcgccgattagcagaaggatcagttccatgaatgcccaacgcgccagcgctccggccgttcgcttatgtcagcgatacggcgcgcggggcgtggagggccttacgcgctcgtaggcgtagccgagcgagagaatccgcgcgtcctcccacttgccgccgatgaagctgagccccaccggcatgccgcggtccagccccatgggcacggtcagatgcggatagccggcgacggccgccagccggctggccgagccctgcatctcgtcctcatcctccggatcgttggtccaggcgcgcgaggtggtgggcgcgatcagagcgatcagcccgtgatctcgcatcatcctatcgatgccgtcctcgcccgccgccttcagagaacgcgcgcgcgcctcgacataggcgggatcgcccaggccgcccgtcttctcggcgcgctcgaacagatcctgcccgaacaacaccgtctcgcgcggttcggcggcgttgaaggcgatcacgtcagccggggtgcgggtgcggccctgcgccgggtgggggggggccagataggcgttgagatcgtgcttcagccccgtcagcaggacagtcagcccccccccgccgatccgccgatagtcggcgggcgcctcggtcacctcgaccacctcggcgccggccgcgcgcaaggcggtcagcgactgctcgaacgccgcacgcgtctctgccgaatagccgtccagcaggaagcgcatcacgccgatgcgcgcgccccgcagcgagccggcgtccagcgccgcgcgataatcgaccttgcgtgcgtcggcctccgcggtcgccacatcggccggatcggacccggcgatggcgctcagcacgatcgccgcatcctccacagttcgcgtgatcgggccggcggtgtcttgggaatggctgatcggcacgatatgggtgcgcgagacgaggcccaccgtcggcttgaagccgaccacgccgttcaccgacgccgggcaggtgatggagccgtccgtctccgttccgatggcggcgggcgccaggccgatggcgacggccaccgcgctgccggaggacgacccgcagggcgtccgctccaggtcgtaggggttgcgggtctgccctcccacggcgctccagccgctgattgactctgacgagcggatgttcgcccattccgacagattggtcttgccgaggatcaaggcgcccgcttcgcgcagccgcgtcaccaacggagcatcgcgtccgggcgcattgctcgccagcgccagtgatccggccgtggtcggcatgtcgcgcgtctcgatgttgtccttcaacagcaccggcatgcccgccagcggcccgcgcgcgatcgacgccggcgcgtcggcgaaccggatcacgctggcgtaggcggcgtcacgctgttgcagggcggcgacatcaatcgacggcgtcgaggcgcaagcggcgagcgacagcgccgccaacgccccgccgatcagtcctgcgcgtcgtgcgagcgcgtgccgatggtgcggtcgaggaagtccagataggtgcgccattgctgcagttgcctcggatcgccgcggacgccgtgccgctggccgggataaagcatcatctcgaacggcaggctctgctcctgcagcttgtcgatgacgcgggtggcgttgggcaggatgacgttgtcgtcggccattccgtgcaggatcaacagccgcccggtcatgtcgcccaggcgcggcaggacgtcggtgcgcgcatagccctccggattgtcctgcggcgtcgacatatagcgttcggtgtagtgggtgtcgtagagcgcccagtccgtgggcgccgcccccgccatcgccccggccaggcccgcctcgggctcggtcagggtcatcaggctcatgaagccgccgtagctccaccccatgatggcgatgcgctcgggatcgacaaacggctgacgcttcagccattgcgccgccatggtctggtcctgggtctcgacaacgccgagctggcgatagttgctggtctcgaacgcctgcgagcggtcgccctcgccccgattgtccaggcggaagacgatatagccggcctcggtcagcagctggctcgtcgccggctgccagctcttttgcacgcccgcgccggtgcccggccccccatagacctgcatcacgaccggatacttcttggacggatcgaagtcaggcggcgtctgcatgcgccagaccagcgtctcgccgtggctctgcagggttccgaactcaggctcgcgcagacgcgagacgtagggcgcgaacggatggtcggcgtccagccggttctcctcgatccagcgcacgcgcgtgccgtccatccgatagagcgccgattgcggcggcgtcttcgggtcggaatagttgccgacataggccgtgccgggcgcgttcaccgaggcgttccaccagccgccggccggagtgatcgcaaccggcgcctcggtgcggttcaggctggcgcggaacagctgctgctcgatcggcagctccttgccgtcgcgcatggaggcggtgaagaagacttcgcccgtctgttcgttgacgccgtttaggcccttcaccggccagacgccgcgcgtgatcggacgcaccactcggccgttgcggtcatacagatagagatgacgccagcccgagtcctcgttggaccagatgaagcggccgtccgccagcacatggaagtcgtcgttcagatcgacccaggcgtccgcccgctggctgacgatcacgcgcgagcggcccgtcgctggatcgacgctgagcagatcgagccgcttctggtcccgcgactggcgctggacgtacagcgtgcggccgtcgttcgaccaatcgacccgcgccagatagatgtcggtgttgtcgcccaggtcgacctttatgcggtcgccgctctggagatcgcgcacatacagctcgaccacggcgttcggccgcccggccttggggtagcgctgttccaccacggtcgtgcccgcgccggtgatctcgaagcgcggcacgatgtcgaccgggctctcgtccacccgcgtcaaggcgatgtagcgctcgtcgggactccaccagtagccggtgaaccgcttcatttcctcctgggcgatgaactcggcggtggcccaggtgaccaggtcgcgcccgtcgtcggtgatcggcgtctcctgacccgtcgccaggtcctgcacataaaggttctggtcgcgcacgaaggagacgtaggagccccggggcgagaccttggcgtcgatctcgtccgcctcggtctccgtcaggcggcgcaccgatccgtccgcccgcgtcgccaggaacaggtcgccctccaggggcgccaggatgtagcgtccctgctgatcccaggcgtaatccaccacgccccgcgcgctgatccgcaggcgctcacgccgggctttttccgcctccgacagctcgccggcctcgggcgccagcgcgcgggcgtcgatcagcttgtagggttcgccctctccggtcggggcggcccagagatcctgcacgttcgaatcgtcctcacgtccccgcagaaacgcgaccagctgaccgtccggcgacaggctgacgccgcgtgcgacggggccggcgaggctggggctcgagaacacccgttcgggcgtcagcacggccgggtcggcgggcgcctgcgcgatcgcggcgcttgcagagagcaggatggaggaggcgagaagaagggtgcgcatccggcgaagctatccggcgattccgcagccgtcatcagggaaaatccgccccgcctttcctgcaacaggttcgcagcctagataggcgcgatgaccgacgccgccgtctcctccccgcccgtcaaggccagcccgttccatcagttggaggtgctgtgggtccgccactggaccgacagcctgttcagcttcggcgtggcccggcccgatgacttccgcttccgctcgggcgagttcgtgatgatcggcctgccgggcgaagacggcgccaagccggtgctgcgcgcctattcgatcgccagcccctgctgggacgagcagctggagttcttctccatcaaggtgccggacggccccttgacctctcgcctgcagaagatcgaggggggcgacaccgtgctgatgggcaagaagccgacgggcacccttgtgctggatgcgctgaccggcggcgaacggctcttcctgatcggcaccggcacgggcctggcgccctggctcagcgtcgcgcgcgatccggagacctattcccgcttcggccacatctatgtggttcacaccgtgcggggcgtggcggacctcgcctaccgcgacttcttcaccagcggcatccacgacgatccgctgatcggcgacgaggcgcgggctcagctgacctactatccgaccgtcacgcgcgaagcgttcgacacgcccggccggatcaccgaccggattaagtccggcggcttcttccgcgacctgggcctgcccgaaggctttgatcccgccaaggaccgcgtcatgctgtgcggctccatggccatgatcaaggaagtgggcgaactgctggagaccttcggcctgaaggaaggctccaacgccgaaccggccgactatgtgctggaacgcgccttcgtcggttgaggcgcggcggcttagccgctaacccacggccatgagcaagcccgcccttgtcgccgtcgacccccgcgtcgatcccgccgcctgccagaccatgagcgaggtccgacagggcgtcgatgctttggaccgcgccctggtggccctgctggccgaacgtcagcgctacatggacgccgcggcccgcatcaagccggatcgagacgccgtccacgacgacgctcgcatcgaggacgtggtcgccaaggtcctgaccgccgcacaggcgcaggggctgtcgccggacatcgccgagccggtttggcgtttgctgattgaccgctgcatcgcgcacgagttcgcggcctatgaccgcacgcgcggttagcgcctgaggcttctcagcatcagctcatggcgataggcggcgacgtcggcgagcgccgcgtccagggccgagcgcacccgctccagcgccggcgacgcggtcttggcctccagcgcctcggccgccgtgcactcggcggcgagttcatgggcgccgatgccggccgccgcgccccgcagggtgtgcaccgcatcgcgccagccttcgaccccggggttcagaaggccggaccatagagcggcttgttcggcgaacagacccagcacctcttcggacacctccggatcgtcgccggtcgtgcggtccagcaccgagaagtcgaccgcccccgaaaggtcccgtcgcgccatcaggcggcggcctcttcgcccttggccagacgcgagtgccgcgacgaccaggcgaagtagatggcgacgccgatgacgttccagatcaggaagccgatctgggtcgtgccgcgcaggctgagaaagaagacgatgcagccgatcaccgtcagaccgccgaccagcggccacagcggcgccttgaacacgcgccgtctccccggctcgcgcagcctcagtacgatcaggctgacccccacagcgcagaaggccgccagcgtccctgcgttagccagcgacgccagctcgtccagcggcagcagccccgccaggatcgccaccaccacggcggtgaacaccgtcaccacagccggcacgccccggctggacacccgcgcgaggcgcctcggcagcagaccgtcacgagccatgcccagaaagatgcggctttgtccgaacaggaaggccagcagcactgtcggcaaggcgatcaccgccgccgccgcgatccactgcgccgccgtgccctgccccagctcgcgcatgatcagcgacagcggctcggcgctgtcggcgaagctggcgaccggccgcgcgccgatcgccgccgccgccaccagcagatacagcgccgtgcacaccagcatggaccccacgatgccgatggcgagatcccgctccggccgcttggtctcctccgccgccgtcgagatggcgtcgaagccgtagaaggcgaagaagatgatggccgccgccgccatcacaccggtctgcacgaacggtgcgccgaagccgttcggcatgaatggggtgaagttgtcggcgtcgaacgccggcagggcgaccgcaacgaacactgcgagcgcggcgatcttcaccagcaccagcacggcgttcagggtggcgctctccttcgtgcccagcagcagcaggcccgtgaccacgccgatgatcgccacggccggcagattgatgatcccgcccgcatgtggccccgccgtcagcgccgccggcagatcgacgcccagcccgcttaggaaggcgaccgcatagccgctccaccccacggccacggccgagaccaccagcgaatactcaaggatcaggctccagcccaccgcccaggcgatcagctcgcccagcaccgcgtacgagtaggtgtaggcgctgcccgccgtcggcatcatggtggacaactcggcgtaggccagcgccgcgcacgcgcacaccagcccagccagagcaaagctgatcagcaccgccgggccggccagccctgccccaaccccgatcagggtcaggatcccggtgccgacgatggcgccgacgcccagcgccagcaggtgcggccagctcagcgtcgccttcagccgtggcccctcgtgcgagtgcgccagcatggcgtcgatcgagcgacgccggttccagaaggccatgaccgtttccccccgccgcctgtgcctgcggctgattccgccgcgaccttagcgcgcttcagaaagtttccgaaaccgcttgccaagccgccgccctctgggtagtaggagcgcccttcgggacggccacaccgcttccgaagacaagacgaccggtcgggtgattagctcagttggtagagcagctgactcttaatcagcgggtccacagttcgaacctgtgatcacccaccattcgtcttcttgattccaaacaactttccggttgagccgtcagacacctaactagcagttgggagtctggttgggcgtttttgttctcttttcgagcttctgtatagccgatgcggcgagcgccggatcacgcttgaggtagtgcgaatcaaggattgcgccgacgtctctcaggctgtgcccggtgatcgtggcgatctcagcctcattgcatccggcgagcgccaggcgggtgactgcggtccctctcaagtcgtggaacgtcacatccttcacgccggacttttcgcaggcctttcgccacgacgcccggaagccggactcggtccaagtgtgaccgcgctcggttcgaaggatcgtcagagcctccaccttggcggactcgccgttcgcctttgcggcgtcgcgagcggccttcgccgcgtccagcgccagccgtagcggctcgccggccgggatgacgacgcgggcgccggtcttactctggcgcaagcggatggtgcgcccgtcgtatgcgctccacgttaggcgcagcaggtcgccttgccgctggccggtccagagggccaggacaagcgcgaggtgaaggtgtgccggcgccttggcgaggaacgcggcttcgtcggcgtcgctccacacggagtcgttgcggtcggcgcgatacaggcgaccgatccgctccagtgggttcagcggcgtcagaccgcgatccgcagcccaggccagcgcacgggcgaaaacggcgaagcggtagtcagcgttgcggcgagaggtgacggccagtcggtcacgccaagcaaggaactcgccgcgcgtgcgtcggtcgtgaaggcctttcagggggaagtcgccaaactcggcagcgatcgcgcgaaggtgcttcttgtagtcggcgcgggatcgttcggcgagcgagaggaagtcggatgacgactcgaacgagtccaggatcgtcgccagcgtgtcggacggctgggctttgcgtgtctccaccgccgcgttgtaactggcgatgaactcaggcgagcccggcttgccatcaaggcgcgggccgcccttccacgcgtagaagtagacaaccgtggagccatcggcgagccgcttgttgacgcgattaacgcccttgagtcgcacgcgcatccctcttggccttccactggtcgaacgggtcgtccgaagaattgtccgccgctttccccggcggttcaatgcggatctcgccatcggccaggattctgaccgcgcccacttccatgccggcggcgagaacgcctttcagcgccctcgcaacgtcggcttgtttgaagcgggtcgcggccatcggacttcttagaagctgccgttcagacggacattgacgctcgccgacgggttcgccgccgccgtggtcgccacgccgatcttcgtattgccgcttgccgtcttcgacacagccttgtcagcagcaacccagtaaacgaggtcaccagggttaatggcgagcgcgctgatcttgggcagcataaaaacgccctcgacgtcgaggtccacgtcgtcaccaggagccgcatcgccgttggccacgccgaagatgctgccgatgatgacgccttctccagacttcacgtcggcaggggccggaagggtcagggtgcgacccggttgcacatgattacgcatgatcagaatcctttcgaggtatggaatcggatggttttgaccgccggccggccgccgatctggcgccgcagttcagcgcagtaggtcgccaactggcgagccgacgcggcgttgtatcggacccgctcgccgttctgatcctgcacctcgaccacggcggcgccggtcatcaggcgatcgtaagccgcttcggcagaggcgagacgttcggcgagcgagcccatcatggtcaggcgcccgcgttgcggaagacgccacgatgatcgacgacgccaacgccgaagtcatagatgacgcgataggtgcgccccaggacggcggcatgttcgccgaacggaatgaccttcgggccaggtgcgccggcgtagttggcgatctccagaaccggggcgctcgcgttggaaccgaagaggtaccaggacgagtcttcgatgcggggttccaccagcaactcaagcttgccgctgaacacgttgacatcttcggccttggtcgcagccagcgttgcaaggatctgctcgccgtcggtctccagttcaggaccgacgacaaggtaacgcggggtcactccaaccggagtcacaccatcgatgtccttttgcgaccgcagcgccaggcggccggccttcaggttcgggagggtcagagcgccgcctgcggcggcaaggttgccatgatcggcatggaacagacgcttaccgtcggacatgaccgggccggcgccattggcctgctgcagaagcgcaaccagagctttcgcctctgttttcgcggccgtccggccgatattctgcatcgcagcgccgaacacgttcagcgaatcgttgatcagcagcttgcgcgacagggtccagtcgcggccgaaggtaaggataggataggattccgagccttcgccgatgacgccggacttcacttcaccgccttccgtcacctccagaaggtccgaagcttcgcccatcttgagcacgcttacgtcacgaaggtcagacacttcccgccgcgtggccagttgcttcaacggcgactctgctgccgcataggcattcatcacgacgcggttgctgctctgttccaggattgtcgggaagtcggacgtcgtcatcatcgcgcgctgcatcaggctttccgacgtcatccgttcggtgcgctcgccggcgcgctgcagggcgtcgcgagcgaaatcaacgaagccgaagccaacaaactggcgcgccgcatcggacgccgcagggccgcccatgcgctgcgccagggcttcggcttgccgctgcacgatcacagtcgggtcagtgttgtcgtgcagcacatgcgcgcggatagaggtcacgcccgattgctgctgacgctgctgcatggcttcgaaggcggcggcgcgggcggcgtgaatgtccgcttcggcgtcgatctgggcattcgcccaggccgcatccaagttggccgtttcggcgaggctgcggatctgggcattgacggccgcgcgggtctcgatctgcggctgttgctgctgttgcgtgtcttcggccgccgccacttgtgcaggcatggtcgcctcgctccttatgaaagccgacgggtcggcggggatcgggaccagcgacgcctcgaggaggtgccatttggtcgccgtacgggtccgcgtggagccggaagacggggcggcgtccgtccacttctccacgcggtagccgatggaaatcccggtcaggtcgccgcgctcaatggcgtccaaggtggccgggttagagatgcgaagggtcgcgtcgatgcggccggtctcgaaccggacgtcgaccacgcggcccagcacgtcagcgatgctgccctgccgatgcgagtccagaaccgggatgcggtcggccaaggtgacgttctcacgtcccacggcgagccgttcgataaagccgctgcgttgaaccggggcgcccgtcgaaagcgtggcgtcaaccgtgcccgtctcgcggttcaggctctccggcgcgaacgccagtgccgcacgcgtaagggtctcgtgttcaagaacatcggtcatcggggggcgctccgcttcaccggtcggccaaggtcatccaggatcggccgcgtcatgcctgtcagcagcgcatttcgatgctgcagcgcctcgagcggcgtagccgggacttcgcgcacgatggggcgcaccaaagggtcaaacatcgccctgcccttcctcttcttcgtcgggttgaggttgcgacggcggggcggcgccgaagttcaggccaagggcggactcgcgcgcacggtcggcggcgatctcagcgtccagagcttcgacgctccagccgcgttcggcgactacctggcgacgcgaggtcaggccggcgtcgatcaactcacgataggccttcgcgtccttggccggatcaacccacggcatcgccgggaacaggtactcggctgcggtccaggcggccgggtcggcttcaaagccgtcggcgatcaggttgcccgtcagcaccagggacgtgaccgcgcgagcgtgaaccctgcgcagcagctgcggcgcgagggttccgtattgaacctgctcgactcgctggcggaagctcaccaaatcggcgcgtaggctcgagtagttggctttggagagatcaccgctcaccaggtgcgccggcacgcccatcccgacggcgaccgcgcgaagctcggcggacaagaactccggcgcctgttgcgcctgctgtggcgaggcgaacgacagttcatagccgctcggcagaaccttgaccgaacccggctcaaggccctcggtcataatgctcccgcgttgatcgccagcgaagggggactcgccggagagatcattcgcgttctttaggaacccggcgaaacatgcgctgaccttgaagccgaccagcagcgcgtcgttcagctcgtccaggtcacgcagcttcgtgaccacgggggccagccacgacacgccgcggacctgccctgcgcccagcggtcggaagaggtgaatgacatcctgcgccgcgacacggcgggccggctgccatgcgagggcgaacgcggtcggcgcttctggccggatccagtaggcgacacggcgaccaaaggagtcgaactccacaccgccgacgatctgggcgccgtcgccgagatcgcgcgtttcggattcatccagtagctcggccggcaagtggcgtaagcgcaggccttccggcgtatcgaccagcaccactagggcttcaccgtcgatcaccagggcgcgggcgatggcggcctgcagtccataccagtcgctcccgccatcaatgtcggcaacgtcgctccagcggtcgattgcggcgcttacggccgcccgcgcgtccgcgtcaggatgcgaggggttggcgcgtgcgccggtcccgacaagcgccgtaacccacgcttcaacggcggcgcgggcatgcgggttgttcgcgtaaaggtgccgcgcccgctgccgcagtggagcaaccgcgttcagggtctcagttgccgtgcgaccaaaggcgggtgtgccatgccaggggcggccgtgagcgccctcgaactggcggcgtgcgggcgccggcgagatcatgcgggcaagggccgtgcgggtgcgatcgatcacgttcatcccagctgcgccttaatcgctccggcgttgcggccgatgaagttgaagaaggatcgctcgccggactcggtctcgagtccctgcgcaaccatgtcgccgggatcgatgacgttgacgctcttgagcgttatgggcgcccgtccagccaatccgccgttattgcgatggcgtgggtcatcctcagtcagcacttcctcgttgcgctgcaggatcgccggcacttcgtccggccgcagcccggcaaggccaccgctgtggtagcgcatcgctccggcaaagacggcagggttcacgggtcgccagccgccgcccgatccaaccaggccgccatcgtgacggaacaggccgttgatcatgctcgacaggaagccgccggttccgctgccgttcgacgtaccagcccccgcgcccagtgcgttgaggatggcctgttgcgcgatcatttgggcgatctgcgtcaggaaatcggcggcgaagttcaggaaggagtcgcgcatggcgtcgaacacgccggccccctcgcctagcgcgtcggtgaaatcgcccagcgcgttcacgccgccgcccaccagcatttgatcgatgtcggcggccgtgagcaccgtcgtctggcccacgcgctccatctcgccgttcagccggccggcgccgctgatcagttcctcgagccccatgcgcgccgcttcggcttcagggccggagaggctttgcagcagggcaagcgtgttagtcgcggcggcgacgatctgggcgttcagcgcgacgatctgatctcgcagtatgatcgcgcccgccacgtcgccagcgtcgctcgcctcgcccagtcgctgtagaaggatgctgcgctgctgcaccagggcgttggtgtcacgctcggctgcctgctggcgccgcgctgcttcggcgatgtcgtacgccgcgcccatgatctgggcgtaagcggccttcgtttcggccgtggcgttggccatgccggtcgcggtcgtgcgggcgatgaaggccgcgcggctttccacctcccctcgctctcgtgcgaggtcgagacgcgcttgctcgagcgtcttcgctgcctcttgctccgctcgggcgtcgtacagggcgccgacagaactgcggattgcagcctcttgttcgcccgtgagtgtcgtctgcgcctcggcagcctgcagccgcgcccgctcgatttcactcaggatctgcgcttcgcgttcggctgtgccgatcagcttcagttcaaactcacgctggcggttcgcggcctcgaggttggcgacgtactctgcctgcttttcggctaggcgctcgccctcggtgtcgcgcttcggcctatcaggcgtgctctggttcgccacggggggcgggtcaaaggtggtgtccggggcagtcgcggcggccgtttggctggttcgccgtatgccggcgatctgacggttcacttcgtcacggcggcgatgcaggatcgccaagcccgcatccgcctcccgctcattgagcatgttcccgcgcgcacgccggttcaggcggatgtcccggtcaagctgccgatgttcggctgacagggtttcaagccgcgtctgttgcacgcccggcaagcgggcgatcacgcgatcgatcaaaccgagaatgctgcccagttcgtcgcggatggcgtcccattgaatgccgtccagcatcgacttgccaaaggcgccccacgcctcgccgaagttatctaggatgcgagcccaggtgccgtccatcttggcagagatcgccccatagcgaccttcaaaaatggcgaaggcttgggtgcgggcctcaacgtcccgcttttgctcccgcagcgcctcaatgtgcttccgctcgctctgggtcaggaagcctagcttgtcatctagggcgagcacttcgtcggcgttaccggtgaaggcttgggttacgctgttgatcgactcggccaggtcgtcgcccgtcaccttcgccaggccgcgcgccgactgggcgaatcggtcaaaatactccggccgcaggccttctctcagcgccgtgctgacgatgccgcgaacgtcttccgccttaacgccgatggcgctcaacgcttcagcgtactccgccagatccttcttgctgtagcgggcggcattgccggacacggccagctgatcattcacaagcgagacgcgcttcgcctcatcgctcatctgcttcagcgccacaatcagcggcgaaacaacaatggctgctgccgcgaccgccggggcaaaccggaggatggcggacgtggccgcgggaaaaatctgggcaatctgcccgccctgctgcgcaaaggcctgcatcggcgaggtgccggacgcgatctgtgtgatcaggtcattgacctgatagcccaggttctgcagctcatggggccgcaggcccaaggcccgaccgcgctgctgcacctgcgttacggccatcttctgggcggcttgcccatacgcgcggccggcctcttgcgcggcacgctctgagcgacggaactgggcgactagcgaacccgacgccgacaaaccggcggctcgcaccttcgtttccagggcgtcggcctgcgcagcggcggccttgaatgacacttccagcttgcgtgtgctggcgacagcggcactgtagttttctcgcccgatgcgaccttgcgccagggcgaccttgtttaggttcgcctgcgccgatcgaacgcctgcggccgtggcgtcttcggcccggatgcgcaggttcatatcgcgcgtgttgctgcccttagccatgcgcgggcgcccccgtcaggctcttgatcagcgatctgaaggcgccgaacgccttccgagtggtcgcgggcttcacgcccatgttcggcactgtggccaaggctgcttggaacgcgatggcctgcgcagcgaggcgttggttctcgcgtcgcatgatcgaatccgccacgtcggcgagcgtacccagtggataggactccgggtcgcggtgaccgtgcgccgtggcgatgagcgccagttctgtcaggctccagcggtaggtcgcgaagtcggcgggcgcctcgctcttgcgaccggctgcggcgcgctgcggctcaaccggcgcggggcgctcacgtcggaaggtcaggtccgcgaccattgcgagcgcggcgtagatgtctgccgggtcgtaaatctcgccgatcgactcggcttcatcaggcacgtccatcgccgtcgctagggcgcgagccgcaaggtcagcatgatcaaggatcagcggctccagggcgccgtcatgggcgaacgcggcataagcggcttcacagccgtccgggtccgcgtatgcgagcgcatacagatcggcgagggttaggccgcgaagggcgactgtcgcgccgttgatctccatgtccgcccgcaccgcgatcatgtcaggcccgcccggcagtcggagcggcagcgaggctgtagggcaggatcgcccgcaccacatttcgccacgtcatgtcgtcaaggcgacggtcatcgctgacgcaccacatggcgttcgccaggttcatcaggtcgcccgcgctgaactcttcacgcatggcgtgaagccgcatcaccagcgcagcgcggaagtcgccttggcgagcccaaggcacgcaaggcgctgcggggtcagtcaggtcgaggtgagcgtccagcacctcgccaagggccgaaccagcgcggcagactatgttcgcgatgatggcgttcgctgcgagaacgtccatcggctcaggcgtccgatgcgcgatcaagggcggacgcaagccgcagcagcatcggcgtaatctcaatctgcaggcgggcgaagaagacgtgatcaccggggacgcgccagcgtgtcacgctcccatccggttcaactcgggccagggtcggtatcgactgaaccgcccccgtgtcgtcgcggaagcgcagcaactccacgatccagttttcgccctgtgcgatccgccgcagggttgcatcaaggctgatctcgaaagtgccgaacggcgccatggtgaccacgtttcgaccgtggcgcaggcacgactccaggctgcggagttcgatgccgccgacgccgttatcaacggcctccactaggacagcgcaaaccgctgcggatagccgatccatgtagcgcagcccgttgtcgccgctttccccaacgcccactcgcgttgctagattgcgcacctgcgaaagcatacggctgcgatcacttcggtcggaggcttcacagattgccgtgctgacttgttgaagcgtgaacatgagaaggtaatccctcggaggaggcctcaacatgccactgcgccagtggactcgcaaatggttatttttgtccaatattttttgacaaacccgttctattgctcctccgtgggattactgatatgacgacttcgcttccgcgaggctggccggcctgagaagacgcgggagcgccgggcgtagggtgatgctgcgttccggtcgcccactcgaggggtagacaggcgagggccgtcacggcggaccatcgtctaggccagggtttaagagttctccttttacagcggagcccgccgttcagcgtgatgcgatcggcgggcttctttgtattcgcaccacgtttgttgggggcaaatgtcagacaacgcgacagattttctctgacaaaggtcagtaatcaattgtcttgcgtttagtcaccacagcctcttaactttggatcgtcgcaaacgactgcggtcatctcaaacagaggtagacatcatgattattgaaagcacttggggcgcggactgcgaggccggacgggccgaagccggacgtctgctgacagaggctcgacttaccggctgcccagtcagtttgttcaacagatgcgctgctatcgcagagcgggatggtcagccgaccggctttgatgtcggcttctatagcgcactcactcttgcggcgatcggctaatggagcccgacaacttcccacgggtcaaagacgtggcggcgcggatcggacggagtccgcggatacgacaacgccagttcataagataaccctgcgatgcgaatgtggcgagcgtcaccacctcgaccgccgccctccatcgatccagcctgacctaatgacggccggcatggtcggcttcatcgccacgaccgacgctagttcctcggcgcgctgttcaagattgacgttcaccagctgccgcgccgcccaggcgtagaccgtcgagtccaacgtctcggcacgacggcccttgatccgctcgaaccggacttcggatcggccgcgcgacatgcgcacgacgcggcgctcgcttaccagctgttcaaagaacaccggcgacaggctttcgctgaaccgaaccccctgccctcgcgccagtcggtcaaatagccgcgacttcacagcgtcaacgccgatcagccaaagaggtgcgccgctggattggcttttttgcaggaacgggcgtgtgaagccggcgacgcccttgccgctcacgacacggcgtttttggcgcggccgagtaaatgcgtgaacaatctcgacatggccgccagagccggaatcgaccacagccgcgtcaactttgatcgtgccgcctttcggatgtggccaggtcatccgcagcagagcgtccagttccgcccagaccgagtcgccgtcgacggcgccccagaatacttcgtgcgacaggatgaagatgtcgctttcgctgtgtccaagcaccacggcttcgaggcgatcattctgcacgtccacgccgacagtgataatcagcacctccggcgggatggcggcgagactgaacggctcgcgccggtcacacagcgcaccatcatccaggtcgtcaccctcgaggcgccacggctcgcctagaacgatattggtgaaggcctgcagcgtctcaggtgactttttcgcctctaggaactcagcgaccaacacgctccaacggtgcgcaaaatgcgggctgcaaagagcgttgatccggaagcccgcatggcctttcacctctggcgccgtcgctcgccaacggccggcctcgaccatggcgggtttggccgactcctcgaccacacaaccgttcgcggggcacgtccaggtgacgggttcgggtaggtgcttgccgtcctcatcctgccgccaggtcagatcagaccaccgaatctcggataactcgccgcacgatgggcacggcacctcaaagatgcgcttatcactcgccgcgtaggcacggctgatcggtccagtttcgaaaacgggcgtcgaaccggagacgatcttacgattgcggccgaacgtccgcgtgcgttccgttgccagcgctacagggtcgccctcttcggtcgcctcgtacccgtccacctcatccatcagcaggatgcgcaccgtgtgaccgcgaaggttgcgaggcgcacgggcgccaacaaacttgagcgatccgccggcaaagcgccggtcgtacatcgtgctccggtcgccttccccttgcgtcagcaggccccgaagtgtcggcgaggcgtcaaacacttcctccaggtcgaccgcgaaccgccgcgcgtcgtcagtggtcggctgcagcgccatgatcggcgcggggtggttggcgacgaaggaaccgatgatgccttgaacgagggcggaatagccgatgcgcgcggacttgagcacgctcacccgctcaatcgccggatcgtccaaggcgtcgcaaatgccgcgctgatacgcccagagacgcatacggccgggaagcgccgacgcggcgtccggcagatagacgttttgctcaatccattccgccgttgagaggctgggcggcggtcgcagcagcgccagggcgtcgcgtcgcaggatctggagcgcgtcagtcatcggccaaggcctccagtgcgcgccgcacctcggcttcgatctgggcaatgtcgtgtgacgacaggtgcggaagcaccgcgccgacgcgggccggaaccgctagcatccccgcccgcacgtcacgcatgacgccgccccatgccgctcgcacgtccgctgttgcaaccaggtcgccgcgggacgccgcattgtgcagctcgagcttttccgcagccgccttggcctgacggatcttctccagcttcagcgggtcatcgtcgctgtggcgtgtcgcccggtcggcgatccaacgcgagtaaccgcggatggattgttccaggtcgtacgccgccgggccgctgcgggttcccttgatcgccttcaccaccacgccgttcgcgccgtgcttccgaacggtgcgcgcatccagccccaaaaggtcggcgagatcaggttctgaaatcaggccgtaggagcccgtttgcatcatctccgctgtcgcggggcgggccggctctttgatgccgcccagcgggccggaatcggggcgcagcagccattccacgtcttcatcaagcgtcatcgcgtggattcctgatctgattttttctgcagcgcgtgaaaaaccgcgagtcgccgaccccccgaggggcgcccgccggggaaggacccaccctcgcccgccgacccgcccggcagaccgtcgcccgcctgccctgtcatcctgccgacgcgcaccaccgcagcgcggtcgcaccacggcgccgaccgggtttgcgtcggttgcgtcagttgttccgtattgccctcacatgtgtgcgtgcgcgcgtatgtgggagagatctggaaaaaccgacgcaaccgacgcaaccgacgcaaaccggggccgaacgtcgatttagatgcacgtttgctgcgcgacatcgatttagatgcaagttcgtggcgcatcagagcgactccagtccgccaaggtcggcgatcacccgcacgcccttgaagccgcgccctcggatgccgcccacgtcccgaacactggcgaaacctgcctgacgcatccgatcggggaaggtcttgttcttcgatccgggatcctcgccgccttgccgggcgaaccatgaccacgaatcccagagggtggccgccgtgtcagcttcgttcggccccacggcgcagcactcgtccagccaagcggcgaacgagtcctgcatgtcgaagtacgcggccgttgccgttcgcacgatctcaggccgttgcaatccacgctgctgccagtcgaggcacccggccacgcaccaggccaggatgccgggaaactctcgcgccaaggcttccttcaaaccgtgatcgacacgcgccggccggtgctcgaacggcaggacgttgaagcggcgacgtattgcatcgtccacgttctgcagcgccggcgcgtgattgccgacgatcgtgagcttgaactcgggcgtgaactcgaaatcgtcctgacgcatgaagcgcgccgtcaccttgtcgccgcctgtgagcgccttgatccgctgttctgcccaggcgcggccttgctcggtctctgacgcccgcgcgaaccgggcgcccttcagccgtgcgatctcggtgctgtggcggtcgtatttcgacgccgtaagcgtctcggtcgccacgttggtcgcgtagtcgccgaagaggtcgcccagcgtattgatggccgtggatttgccggacccgcccggtccatagacgaacaagagcgcctcttcgcgcgtgtcgcccgtcaggctgtaccctgcccattgctgcaggaagcggatcgcgtcagcgtcgccgccggtcgcctgatcaaggaaggccagccatcgggggcagtcccgcaccggatcgaagcgcccccttgggacgggcgccgacgccgtgagtcgggtcatgccatcggcagggcgggaaggccgaaggtcgccggtgcgcaggtcgatcgtgccgcccggcgtcgccacaagccaaggatcggcgtcccatgcgtccgcggtgacggcaaaggtcgggtcggcgcgggcgaaccgctccacggctgatgcggcgttcgccttggcgagagccttggccgcagccgagtcggggttggcgctggccagttcgcggcagatgtcccgcgcccagttgaacgcaagctgcgtctcttcacgtcgccagtgagtgccggtccagatgaaccagcgccccgtcgaatgacagaacctcagcttgccggcatgacgcgccgcaaaggccaacgccacgccatcctcagaaagcgcaaagccgtcgatcgtgacgggcgccgcgctccagccgtgcgccttggcgaggtcgtacagcgagccgatacccactgccctgccccgatcatcggcgaaggatcgccagacgcgggcctgatctcgagcgtcgaacttgtcggactggcgcgaccattcacgccagacgacttcggcctcatcgcccccgcgcccttcggcgtgaagggccatgccgacccgcaaccaatcgtcgcggtcgtcggcgggaatgaaggtcagcgcctctttgatccgcgcccagtccggtgcgatcagcgacatcaggtcgtcgtcatcgtcagcgagcaatgccgcgacttcggcgtctaggttcggcgcggcttcgtcacgatccggccgccggccgatgctcggcagtccgtccagcgtgtccagcgccgcaccttccactaggcgcacttcatgggccgcgccgtcgcccagtgcgccgaagtaataggactgagatgcaacgaagctttccggctccagtacgccgccaaggacgccgttcagcttggccgtcagcgccgcgcgctcgccgggcgcaacggtcgccgacaagggcgccagcacgcgccagcgaggagcgtcagggcgatgtctgggcgatgtataaagcagggcggcgacacccgccgccttcagccgtgcgtccgcttcgtccagcgtgacggcacctttgtcatagtcgccttcgataccctcaaccgccagcaagttggcgtcattccgcaatgcgcgggctgcggtggccacgtcgccgaaggtcgccaacttcagccacggcaaccggcccttggcgatcttggctgcttcctcgctttcgtcggtcggcgcgggtcggcgcgtggaacggatgacatcggcgaactggcgcagcgtggtggcctcgcgcgtctggcgcgttgcgcgcgcagacgtgaagcgggtgatggtgatcggtcgatctaacggtgaattgtgtgggcttgaggcgaggccgaggaggtcgtatatttccgcctgaagctgcccggcttcctctgcctttgcgacgccgttccgtgatccagacggagcggcgtttcgcgtttctggtggtccgccgggcgggtgatccaagcccagaaggtcggcgagatcagttggcacttcggccataagccattgattcagcattgaaggattcacctccggttgggaggaaagtcctatggaatcagcagaagacggcgactcttaatcagcgggtccacagttcgaacctgtgatcacccaccattcgtcttcttcatttccgcaaccgacgaaaatgatggccctcggcgcgaggcaggatcaacgcgtgctcgcgctcccttgcggcgggacggtagggcgcgagtaacgcgcccttgttgatccgtcacccaatcgccccaacgcagccctccgcctcgcctggcgacagtcgggcgtccgtcagggccagggtccacccatgatgcgtgttcaggccccagcgccgggcgccgccgccgtcgcccgcgtccccgccagcggtgaccaccacgcgacggccctttggcagggccggcggatcgatcttgccgacggccagcgaggtgggcgtgtcgccgccgtagccgtcgaagacgctgagcatcgaccactcacgacgcagccccatccaccaggcatcctcggtgttgacggccagcacggcgacgccgcgcccctcggcggcgaaggccagcgccttttgcggatcgcgcaccatgcggatgtccgccgccgcgccgaaccgcagacgcgcgccgtcgaaggcgcgcgtgggctcgatcggcgcccagacctgcacctgaaggcggccttggcgcgccagcccccagccgacgatctcgcgccacagatgctcgaccgcctcggcgttctcgggcgcgcatctgtcgagcatccgcgcctggaccgtctgctcacggtcgggccgcagcttggtgtgggcgccgcttggggcgtccttggcccgcccgacgacggaggccacggccaggcgctgttcgaacagggcgaggatctggtcgtctatgcggtcgatctcggcgcgcagcgccgccagcgcctgctgttccggcgtcaggtgcggggcggcttcaggccacgcctgtttcagagaggatgcggtcaaggggtgcggctttcggcatggtgtttcgatgtgcaggggcgtgctgccgctcgacaaaggagcggtcgccggagagacggtcaggagcggaaaacgcccgacgcctcagccggcgtatcgaaagccgaaataatagccggccaccgcgcgcgaacggtcaaaggaacgggaaaggtcgcgcgagaaggacatgggtccgcagggttccggcagggcggatcgttttcgatcctcgcgcctgttcaacacgcaacaggcgtgcgccgtcaacccttgttcaggcttagcaggacaaagcgcgtgcggttgtcgcctgaatcctgaagatcgttgcggaggatcgacaggccgtaggcctcggcggcgccggcgggcgccagggccgcgcgcgtcggatccccggccttggccacggctcgcgcggcgcccgcggtgtcgaaagcctcgacagtcctcaagttcatggcgctcaaggtcgccgcgcactgcctcagggcgacggggtgactctccacgctgcggatgtccgacagccgcgccccctctacggccatcagcgcatggcggatcggccgccagacctccgcgatcggctcagcccccagcgcggcgaccaggctcgccgccggctccaccacgccgacggacgagttctcgaccggaatcagggcgcacccgcatgcgcccgtcttcagcgcgttgatggccgcctcgaagctgtcgtagccgaccgcctcgtcccaaggccgcagcgcgagacaggcttcatgactgaacgatcccggcgcgccctgataggcgacgcggccgtgctcttcgcttgggccgctcgcggtcatgtcaggccgcccgcgcctggtcggtgcggacagccttcagccgttcagccaccaggaacgccagttccagcgcctgatcggcgttcaggcgcggatcgcagtgcgtgtggtagcggctggacagatcgtcctcggtcaccgcttgcgctccgcccaggcattcggtgacgttctgaccggtcatctccaggtggacgccgcccgggtgcacgccctcggcctcggccacatcgatgaaggtgcggacttcgcccaggatgcggtcgaagggtcgggtcttgtagccgttgccggccttcagcgtgttgccgtgcatggggtcgatcgaccacaccaccttgcggcccgccgccttcaccgcgcgcatcaggccaggcaggcgcgcgccgaccttgtcgtggccgaaccggccgatcagcgtcagccggcccgacacgttgtccgggttcaaggcgtcgatcagcggcaggaggtcgtccgcctccatggtcgggccgcacttgacgccgatgggattgcggatgcccttcatgaactcgacgtgggcgccgtcgagctgccgggtgcgctcgccgatccacagcatgtgggccgaggtgtcgaaccattcgcccgtcgcgccgtccagccgcgtcagcgccgattcgacgttcagcagcagcgcctcgtggctggtgaagacctcgacccggctgaggtccgggtgggtctccggcgtgacgcccacggcctccatgaaggccagggcctcggtgatcttgtcggccagctcccggtactgggcgcccgccgcattgtcgccggcgaagcccagagtccagcggtggatgttgtacaggtccgcatagccgccgccggcgaaggcccgcagcaggttcagcgtcgaggcggactgattgtaggcccggatcagccgctgcggatcgggtacgcgctcttcgggcgtgaaacccatgccgttgatgatgtcgccgcggtagctgggcagttcgacgtcgccgatctgctccacgcccgacgagcgaggcttggcgaactgtccggcgatgcgcccgaccttcaccacgggcttcctgcccgcaaaggtcagcaccaccgccatctggaggatcagacggaaggtgtcgcggatgttgtcggtcgaaaactccttgaagctctcggcgcaatcgccgccctggagcaggaaggcctcgccccgctccacctgggacagccgctcggtcagcctccgagcctcgccggcgaacaccaggggcggcagcgcccgcagctcatcctcgacggcggccagggcgcgcgcgtccggatagtccgtcggcatctgcaggacgggcttcgatctccagctttcaggggtccagcgcatggtcatgcctgtgaggataggacctcgcgccgccgctcacaatcgcgacggcgcagggcaaggaggatcagctgccgtcggcgccgagatcctcgggcgtgggggattgttcgccggccgcaccggccttgcgttcggccttggcggccgccttcgccgcggccttctgggcggcggcgcgctcacgttcctggcgttcgaagttgtagttgggcttccgggccatgatcggtcttgctcctgctcagtctcaaagtcggcccatcaacatggcgccgaaaccgggagacgcaaatcgccgtcgccctgctcgcccgaccgtcagatgcccgacgccttcaccgcgtcggtcgagacggcgtccggatcgcccggcagccaggcgacatggccattgtagacgccctcgttcaggatgccctcctcgcgcgcgaccagcaccggcaccagcatctggccggtgacgttggtggcggtccgcatcatgtcgatgatccggtcgatggcgacgatatagccgatcccctccagcggcaggccggcggtggacagcgtcagggtcagcatgacgatggaggttcccggcaccccggccgtgcccagcgaccccagcaccgccgtcaggccgatcaggacgtactgggtcagcgtcagatcaatgctgaaatactgggcgatgaagatcgacgcgatggccggatagatggcgccgcagccgtccatcttgacgtttgcgcccagcggcacggcgaaggcggcgtaggcctggggcacgcctagcctctccaccgtttggcgcagggtgatcggcagggtgcccagcgacgaagaggtggcgaacgccgtctgctgcgccgcgaacgcaccccggaaaaagctgaccaccttcaggccgtgcagcttcagcaggccggaatagaccacgaagatgtggaacaggcacgcggcgtaaatggcgaagatgaatttgccgagcggcagcagcgcctcccagccatagccgccgaccaccgagccgatcaggccgaacacaccgataggcgtcagctggatcacccatcgcgtgatgcggaagatcacggccgccccctcgtccaccagccgccgcacgccctgcgcgcggtcgcccagcgccaccagcgccgatcccaccagcgccgagaagaagatgatctgcagcacccgaccttcgctcagcgccgcgaacgggttggtcggcacgacgccgatcagcacctccagcggcgttgggatctcacgcgccctgacctcgcccagcggcagatcggccaggcccagccccggattgatcaggtggccaaacgcgatccccaccagcaccgccagcagagaggtgaccgcaaaccagacgatggtgcgcacgcccagccgcacggcgccggcgccctcccccagcttggcgatggagctggcgatggtgaacagcaccaagggcgccaccaccatccggatcaggttcaggtaaacgtcgccgatcggctgcagccagacctcggcctgctcgcgcaggatcagccccgtgacgatgcccagcacgaagcctgcggctgtccgctgccagagtggaatggcgaagaaacgggaaatcatgaacggcggccttggggagacgagtgcgtcaaggtgtccacacaggccgcgatccgcaaccgcatgcgcgacggccgtttgcgagttcttctgtcagcgaccatcagccctgctgtcagccgacacccatcgcccggcgcacatagaagccggcgatgagcgcgtccacggcctcctccacatcctcgaaggcgtcgatcagcacgtccgcgccgagttgctccaccggcacgggcgtgtagccgaatgtggtgaggatgcagggcaggcccgcatcgcgcgcggcgtcggcgtccggtgctgcgtctccgatcatgatggcgcgcgcgggatccccgcccgcgatccgcaccgcctcgatcggatgcgcaccgctgggctttctggcgctgacccgctccggccccacaatcgcggcgaagcgatcggccagccccagccggtccatcagcaactcggagaggtcggtccgcttgttggtggccgtgaccagcaccgcgccgcgcttcgctagtcgatccagcgtttcttcgacgccttcgaaggcgcgcgtgccatcgacgatgtgcgcgcggtagtcggcgaggaagcgctcgaacagcgcctccgagcgggccctctccccatccgcccccacggcttcaaagccatgcgccagcagagcccgcgcgcccgagccgatcagggtcttggccgaatccatcgacactgtcggcaggccctcctcaaccagcaggcggttcagcgttccaatcaggtctggcgccgaatcgacgagcgtgccgtccagatcgaagacgagggtccagccctccaggtcgcggtcggtcatgatgtcggtctcggaggttctaaagcacgcctgcgcattgtagacggcgcggaacgcctagacgccgggacgatccatgaccagccaaacccgctcacgcgccgccgtcatcctggccgcaggccagggcacgcggatgaagtcgccgctgcccaaggtgctgcaccgcgtcggccatcgcgccatgctggatcacgccatcgatgcggccgaggcgctgggctgcgagcgcatcgtggtggtggtgggcgaccactccccagaggtccgggcccatgtcgaggcgcggctgggcccatccagcatcgcggtccaggacccgccgctgggcaccggccacgccgtgcgggcggccgaggcggcgctttccgggttcgacggggacgtggtggtcacctacggcgatgttcccctgctgaaggcgtcagacatcgaaccggtcttcggcggcgagggcgtgacggtggtcgggtttcatgcgcgcgatcccggcgcctatggccgcctgatcctggaaggcgacaccctgcgcgcaatcaccgaggccaaggaggcgtcggcggcggttctggcgctcaccgcctgcaactcgggtgtcatggccgcgccctcggccctgctgttccaactgctggctgacgtcaccaacgacaacgccaagggcgagtactatctgaccgacgtggttgaacttgcgcgcaaggcgaaccatccgacccgcgccgtcttcgccgaggaagacgccgtcatgggcgtcaactcgcaggccgaactggcccaggccgaagccctgttccagacagtccagcgcgacacctttctggccgccggcgtcaccatgccggcccccgagacggtccacttcgcgtgggacacacaggtcggaggcggtgcggtgatcgagccgtttgtggtcttcgggcccggcgccgtggtcgaaggcggggcgcgcatccgcagcttcagccacatcgagggcgcccgcgtcgcgtccggagccgaggtcggcccctacgcccgcctgcgccctggggccgacctggccgagggcgtgcgcgtcggcaacttcgtcgaggtcaagaacgtcaccatggccaggggctccaaggccaatcacctggcctatctcggcgacggcaccgtgggcgagaaggccaacgtcggcgcgggcgtgatcttctgcaactacgacggcttcaacaaggcgcgcaccgaggtcggcgccggcgcctttgtcgggtccaacagttcgctggtcgcgcccgtcagcatcggcgcgggcgcggtggtcggttccggctcggtggtgacggaggacgcgcccgccgacgccctggtgttcggccgcgcccgccaggtcaacaaaccgggggccggcctcgccttccgcgacaaggccaagagtaaaaaggacgcgaaatgagcgacctccagaagaggaacgccggagaggcggcggcgcaatgcgtcgaggccggcatggtcgtggggctgggcaccggctccaccgccgcctggttcgtcaaggcgttggcggcgcgcggcctgtccggcctgcgctgcgtgcccacctccgacaggaccgccgacctagcgcgcgacctgggtctgaccctgtcgacgctggaggacacgccgcgcatcgacctgacggtggacggggccgacgagattgggcccggtctggccctgatcaagggcggcggggccgcgctgctgcgcgaaaagttggtgtgggaggcgtccgaccgctgcatcgtcatcgccgatcaggcgaaagtcgtgccggtgctgggcgccttccccctgccgatcgaagtcgtcgcgttcggccacaagaccacggccaatcgcctggccgacgtgctgatcgatcacgatatcagccagcccgcccgtgtgcgccaggccgaccgtggtcttgtccgcaccgacggcggcaatctgatctacgacgccgcctgccgcgccatccacgatcccgcgcgtctggccgacgacctgaagctgatcaccggcgtggtcgagcacggcctgttcctggacctggcggacgaggccatcataggcggcgacgccgggaccgaacggctgcgcccctgaggcgcccacttcccgcacaagcttttcgccacaagcgtgcctatattgcggccatgacctttcgacccaccaccatcgaacgcgcctaccagctggcggagagcggcgtctgccgcaccgtcggcgacgtcaagaagcagctcgcggccgaaggcttcgtcggcatccaggaccagctctacggcgcgaccatcaccgcggcgctgcgtcagcgctgcctgaagttctacaaggcgcaagagcctgcggaaggctgatcgtccttcgttcttgcattccggggctgaagcggccatcttgcggcctgtcgatctctctgcgtaacgcattcgttctccgcgcctcgccctgggatctgttgccgctcctttcagaccgacccccgccaggcgcgctgttgcgtctggccgtttccgatggaggtcctgaaatggcgaccggaactgtcaagtggtacaacccgaccaagggttatggcttcatccagccggacgacggcggcaaggacgtgttcgtgcacgtttccgctgtcgaaggcgccggcctgcgcggcctggatgagaaccagaagatctcctacgagatcgagcgcgaccgtcgctcgggcaaggaatcggccggtcaactgaagaccgtctgagacctggcctctcgctagtctgactttgagacggcggtcctttgcggggccgccgttttcgtttgtgcgttgccgccgcgctccccggcgcctaagtcggctcgacccaagacacgccggagccggacatgagccattcctacgactacgacctgttcgtcatcggcgcgggatccggaggcgtgcgcgccgcccggctgacggccctggacggcaagaaggtcgcggtcgccgaagagcaccgcgtcggcggcacctgcgtgatccgcggctgcgtgcccaagaagttcatggtcatggcgtccgaggtcagccacgccctggagatcgccgaaggctacggctggtcgttcgacaacgcccgcttcgactggccgaccttccggcaggccaaggacgtggagatcgcgcggctgtccggcatctacaccgccaacctcggcaaggccggcgtggatctgatccacggccgcgccgtgctgaaggacgcacatacggtcgaaatcttgggcaagaaccagacgatcaccgccgaacgcattctgatcgccacgggcggccgcccgtggaagcccgaggccctgccgggcattgagcacgccatcacctccgaagaagcctttcagcttcccgaactgcccaagcgcatcctgatcgccggcggcggctacatcgcggtcgagttcgccggcatcttcgccgggctgggagtcgacaccaccctgatctaccgcgggcccaacgtcctgcgcggcttcgacgacgacgtgcgcgcgcatctggccggcgagatcgagaagcggggcgtcaaggtcatcctgggctgccagcacgcctccatcgaaaagactgaggccggtctggtcaaccatctcgagaacggcatgcgcatcgagacggacgtggtgatgttcgccaccggccgcgtgccgcacgtggtcgatctggggctggagacggccggggtggaactgaacgaggcaggcgcgatcaaggtggacgccttctcccgcacctcggccgagaacatctgggccatcggcgacgtgaccgaccgcatgaacctgacgccggtcgcgattcgcgaggcggtggcgttccaccagacggtctatcgcgacaaccctcagcacttcgactacgaggccgtggcgaccgccgtgttcagccagcctccggtcggcgtggtcggcatgacggaggcggaggcgcgccacagctgcgccgccggcgtcgatgtctatgtcacccgtttccggcccatgaagtacgccttcaccggctcggacgagcgcgtgctgatgaagctggtggtggacgcagacacccagcgcgtcgtgggcgtccatatcgtcggccccgacagccccgaaatgatccaattggccgccatcgcggtcaaggccggcctgaccaaggcccagtgggacgcgacttgcgcggtccatccgaccatggccgaggaactggtgacgctgaaggacaagcagacggcgtcgagcggcgccgcctgaggaccggctcagcgtgtccgttcgcggtagcgctccagcacgtccagcctgatccggtccggcaccatctgcgcggacgggccgctgttgccgaagagcagcagccgcgtgtcgccctcggcggccctcggccacgtcgggcgcccccggccattcggatcgcccgaccgcgcaaacgcggtccagtaggccatcatcgttcgcgaggcggcacggtctcggtcctcgaccggatagggcaaggtgttcagcgtgccgaacacataggggcgctcgatcgcgtgggtcgcgccgccatgcggctcaggattctgggccgagctgacgtcgaagcggtaaagccacgccggatgtcccgcccgcgcatgcaggcgggccaggtggcgcgccggttcggcgaagatcaggtccgtcaccgcctgagcgtcgaagccctccaacccgccataggcctgcgccgcttccgcacgctcgagccacgtcatttcatcgtcggccgtcccgtagccgttggggtcggtgggacgcatccaccagaactcgcggctgttggtgccgatgatcagcggaacgccggactgcccgccggctcgaaacgccgcctccacctggtcgggcacgatccgcccgtcgatgatcgacaggtcgccgttggcgaatgtgggggcgggcgtcagaaacaactcggccggcgcgcccctcagatccgcggccgtgcgcaggccggcgccatgggcgaacacctcgccgcgttcgcgcgccgacggctcgccctttgggccgcgccggtccagccaggcgacccgttcgcggcccagcccagattgcacgacggcgcggtggaacagcccctgcgcgggcggcgagatcatcagccgcgtgacgatcgcgcctccagccgattcgccaaacacggtcaccttctccgcgtccccgccgaacgccccgatgttggcgcgcacccagcgcaacgccgcgatcacgtccatcagaccgtagttgccggccgcctcacccggcggccgctcggccgccagagccggatggtcaaagaagcccagccggcccaacctatagttcagcgtcaccacgaccacgccctgctcggccaaggctgagccgtcgtacagacccgcagttcccgagccgttgttcagcgccccgccgtggatccacaccatgaccggagccggccttggcccccgtccggtcggcgcccagacgttcaggttgaggcagtcctcgctcatcggtccggcgcccaccccgggatcacccggcgccggcgcttggatgcagatcgcgccataagaggtcgcgtcccgttctccttgccacgacatcggctcggagggcggccgccagcgacgctcgccagtcgggggcgcggcatacggaatgttcttgaaagccgaaaccgtccgaccgccttggccgacgagcacaccttgttccaccttaacgataggcgcggcttgggtcatggagggcgaggccagaaagaggacaaaggcgagagaagcgaagacggcggcgaaagtcatgcgcccctaaaagcaaaaagccgcgccgggttgaagggttcgaaaaacctggcggccgtcctgaaccttcgctgtagataggcgttcaagccggagtttgggtggggtggtctttgagacttttcgcgacgggcgacaacgccggagatctgggcgctgcgtttgacgcgtcgccgaacgcctatgtgctcttgcggccggcggacctgacgatcgtcgccgccaaccaggcctatctcgacgcagtcagcgtgacccgcgaccagatcgtcggaaagcccatgttcgaatcgttcgactccggatcgggcagcgacgctccggagaacgtacgccaggtccgcacatcgctggagcgggcccgcgacctgcgccagcgggatcatctggcggcggtgcgattctcgctgctgcgccctggcgcggatgggcggccagtctatgaagaacgtctgtggagcgccacccatacgccggtgctcaaccgggacggcgaagtcgtgctgctgcttcagcacacgaccgacgtcaccgatctggaggccgcgcgcgacgagacgaacggccaccccggaccttcgcgcacggccgtcggcggccaggttctgaagcgcgcgcagcaggtccaggaaagcaaccgacgtctggaggccgaacgtaaccgcattgtcgagatgatcatgcaggcgccgggcttcatggcgcttctgaccggtcccgaacatcgcttcgaaatcctgaacgccgcctatcatcggcttgttggcgggcgggacatcgtgggcaagccgatcagtcaggctctgcccgagcttggcgaccagggcttcttcgacatcctggacaccgtgttcagcaccggcgagccgttcgagggccggcaaagtcgggtgcagcttcagaccgggcccaatcggctcatggagaatctgtacctcaacttcgtctatcagccgatccgggacagttcaggggcggtggcgggcatcctggttcagggctacgacgtgaccgacagcgtccgcgccgccgagcgccagaagctgatgatcgacgaactcaaccaccgggtgaagaatacgctcgcgaccgttcagtcgatcgcggttcagaccgcacgttcgcacggggaccccgccaccttcgccgaggcgtttcagtcgcgcatactttcgctgtctcatacccatgaccttctgacccgcagccactgggaaggcgccgacctgcgggccatcctgaaccacgagatcgaggcccacggcatcgcacgcgtcagcctcaacggaccgccggtcgcgctggagcccgccatggcgctctcgctgggcatgatctttcacgaactcgccaccaacgccgccaagtacggcgcgctgtcgcacgcggacggtcgcgtgctcgtcgactggaacgtgaccaaccagcgcgatcggatcctgcacatttcctggcgcgaggcgggcgggccgccggtcatcgaaccggatcgccgaggattcggaagtcgattgatccagcgcaatgttcgtcacgatctggcgggcgagatcgatctggtctacgccccctccggactaacggcggagctgacggttcccctcgacggaaggcagacaggatgagcggcgagttgcagggtcgacgcgtgctggtggtcgaggacgagtccctggtcgccatgcttctggagaccattctcgaggacatgggctgcacgccggtcggaccggcgtccaacatcgacgaaggcgaggcgctggcccgcgacgaagcggcgctggacgcggccctgctggacgtcaatgtcgcgggacgtcaggtgtttcccgtcgccgcggctctcaaggcgcgcggcgtgccgttcgtcttctcgaccggctacggcgaaggcggcctgccggatgaatggcgcggcaaccccacgatccagaagcccttcaccgaggccgccatccgcgacgccctgatgaaggccatgaacatcgtcaccgtctgaaccgtcgttcagggctgagccggcgcctgcctctgcaggggcgcccgcttcagcgcctgcagattggatgagcccgtgcagaagcacgctgttctgagttggcgcaccaccagctgaaagtggctgatcacggcctcggtcgagatcgtggcggctgggagcacgcccgccgcctgtcccacgatgtcggcgcccagccggatcgccttggcggcgtccagaccgtgccgcaccccgcccgagccgatcaacaacagatcgggcgccgcccttcggacctccacaagcgcctgcgcggtgggcgcgccccagtcggcgaacgctgcggcgtgcgcccgatcctcggcgttctgtgagcgctcgccctctatcaacgcccagttcgagcctccagcccccgccacgtccagcgccgccacgcccatgtccgccaggcggcgggccgtggacgccgatatccccgcccctgtctccttgaccacgacaggtgcgtccaggcggcgaaccagagcttccagcgcggcccccacgccccaccagtcccgatcgccttcaggctggcaggcctcctgaagggggttgaggtgaacgatcagggcgtcggcgccgatcgtttccatgatgcgccgagcctcgtccagcccgaagccgcgggtcagctgggccgcgccgatattcgccagaatgggcgtatccggcgccctgcgcctcagcccgccgtccagcccgtcggcggctccccgcgccaaggccgcgcgttgcgagcccaccgccagggcgatgcccagatgctgggccgcttcggcgagacgcgcgttgatctcgccggcgcgcgccgggcctcctgtcatggagctgatgagcaggggcgccttcagccgtcgccccaggaagtccgcgcccaagtcgatcttggcgtgatccaggtccggcagcgcctcgtgaacaaagcgcacggcgtcgaaaccggcgtcccgagcatgacgaccgcgtccctgcaacacgacgtccaggtgctggtccttgcggacgattatgggatcttcgctcatgacgccttgcacgaagcttgggtgatcaaggcttgcgttcgatggtcagggcgtaggcgccggtcgcattcggaccgaacgaccgcgcccgcaccacatagtctccgtcctccggagccgtccaggacagccgcgcgtgagtatccgacaagccgtcgtcgtctgtcgccaggctttcgaacggctcgccctccgcgtgccggccgacatcaatgaaggcgtcaaaggcgttggagaccagcgtcagctgcaacttctcgtccttcttcgcctggaaccggtaggcgtcgaacgcggcgccctcctctgtgacggcgtcagactccgacagggcgccgcgagcggtttcgccgacgacaaggacgcccggctccggctcggggccccggtctgtcagctccagcgagtagagcccccgctcctcgggccccaagggcagcgcgcgaaccacatagtccccgtcggacggcaaggtcaggttcagccgcgcatccgtgccctcccccaggccgtcgtcgtccgacgccagaacctcaaagggcccgtccgccgatccgatctccagataggcgtcgaagtcgccggatctcagcaccgcctgcacgcgctgtccctcgcgcccgttgaagcggtaggcgtcatagcgcgcgccgttgtcggcctgggcgtcggtgtccgcgatctctccctcgaccgttcggccaaagctggcttccacgggcgcggggggcggcggcgtctcctccacccgcaggcgatatcggccgacctcttcagccgtcagggcgcgcgcttcgatcacatagtcgccgtcggccgctagagcgtgcgagatgcgcgcgtttgtgccgtcgcccgcgccgtcgtcgtcctcgtcgagcgcgtccggcccgccagccgagcgcaggaccagataggcgtcgaaatccgacgactccagcgtgatcgagacgtgctgccccgcgcgtccggagaagcggtaaaacgcggccggcgcgccgtcgtcgttgaccgccgccccctcttgcagttcgcccgtctcgttggcgggcaaggtcagcggcgtggcggccggtgcggccggggcggcggtcaggccgagccggtaggcgccgagcgactcgtccagcgatgtcgcacggatcgcgtatgcgccggtctccggcgccgtgaagaccagccgcgaattcaggcctcggccgggcgcatcgtcgttgcgcgccagttcctcgaagctccgccggttctgccggccgacgatcaggacagggtcgaagctgtcggattcaagcgagatcgccactcgttcacccgcccgagcctgaaagcggtagccgtcgtagtgcgagccgtcgtcagttgtcgggtcccggccggtcagctcgccctcgagggaagcgcccacggaaatccgcccaccctcctgggccaaggcggagcccgccatcgccagggcgatgacgcctgcgagcggcaggacggacgaatggcgcatggtcggtctccaaaaagcggcgcgatcatagacgccgatccagcggaactgtaaatcgcgggcctgccccgatgtccgacccggagacgccagatgacggctgaacctgcacgcgcagccctgatcgacggcaaggcgttctcggccgcgctggtggagcgcgtcgccgccgccgccggtcgcctgcgccaggcgcatggcgtccaggcgggcctcgccgtcgtcatcgtcggagaggacccggccagtcagatctacgtgcgcaacaagggcgagcgcaccctgggggcgggcatgcggtcggacacccacaggctggcggagacgacgacgcaggccgagctgctggcgctgatcgcccggctcaacgccgacggaggcgtgcacggcatactggtgcagctgcccctgcctgcgcacatcgattcgtcggcggtgctggcggccattgatccggacaaggacgtggacggcttccacatcgtcaacgccggacgcctggccgtcggactgccgggcctggttccctgtacgccgctgggatgcctgctgatgctgaaggaccagctgggggacctttccggtctgcatgcggtggtggtggggcgctcgaacattgtcggcaagccgatggcgcaactgctgctgggcgaaagctgcaccgtcaccatcgcccattcccgcacgcgcgacctgcccgccctgtgccgcaccgccgacatcttgatcgcggcggtgggtcgccccgagatgatccgtggcgactggatcaagccgggagctacggtgatcgacgttggcatcaaccgcgtgccctcgcttgatccggccaaggcggccgagggcaagacgcgcgtggtcggcgacgtggccttttccgaggcggagcaggtcgccggccgcatcacgcctgtgccgggcggcgtcgggccgatgaccatcgcctgcctgctcgccaacacctacgtcgccgcctgccgccagaacggcgtcgcgcccgagccgttggacgcctgaccctcagccttcacacttgtggcgcggcgggcgagcgggaatactccgactcgttgttcgtcgagcgctgtccggagcccgccatgtccacgaccaagcccgccgccgccctggcgctgtccatgctcgcggcgtccgtctcgggctgcggctacaacaccattccgaccaagcaggaacgggccgaggcggcctgggccgacgtgcagaacgattatcagcggcgcgccgatctgatcccgaacctggttgcgaccgtgcagggcgcggcgatccaggaacggaccacgcttacggatgtgatcaacgcccgcgcccgcgcgacagccgtcacggtctcggccgaagacctcgacgatcccgccgcctttcagcagttccagcaggcgcaagggcagctcagcagcgcgctgtcgcgtctgctggtgtcggtggaggcctatccgcagcttcaggcgaatcagaacttcctgaccctgcaggaccagatcgaaggcgcggagaaccggatcgccatcgcccggcgcgactacaacgaggcggtgcgcgactacaacaccagcctgcgcaccttcccgaacgtgatctgggccaagaccgtgcacgcaggatcgcagccgatgcagctgttcactgcgaccgccgaagcccaggccgcgccgcaggtgaacttcaacctcggcgggccctccgccgctccggccgcccagccgggcggtcaggccgcgcccgtggcgccgggatcgccgccgccggcgcgctaagagcgccagcgtggctgctccctcattcctgagacgcatggcacggcggctgtcggtgctgatgctggggctcttgatccttgcatcgacgacgcccgcgctggcgcaagccgccccgcagtttccgccgctgaccggacggatcgtcgacgaggcgcggctgctctcaccggccaaggaggccgagatcgacgccaagttggccgcgctggaggccgacaccagcgaccagctcgtcgtggtgactctaaatagcttgaatggcttcgagatcgaggactacggctacagactcggccgccactggggcatcgggcgcggccagaaggacaacggagtcctgctgatcgtcgcgcccaacgaacgcaaggcgcggatcgaggtcggctacgggctggagccgatcctgacggacgccttctcctcgcgcgtgatccagacgctcatgctgcccgcctttcgaaccgggggatacgagcgcggaatcaccgagggggtcgacgccctgatcgcccagatgcgtctcgatccggccgaggcccaggcgcgggcgcagggcgtggagcccgaacgcgctcaggcgcccatcggccctatgatcctgatcgcactggtgtttctgttcatgttcatgggcgccatggggtccgccagccggcgcgggcgtcgctatcgtcgtcggggcgtctcgccggtcctggtctgggcggcgtccgaagcctttcgggcgagcgccagcagccgacgcggcggttttggttcaggaggcatcggcggcggctttcgagggggcggcggaagttttggcggcgggggagcctccggcggatggtgacgaccttttcggccgaggacagcgcgcgcgtggcggccgcgatccgcaaggcggaggcgcggacctccggcgagatcttctgcgtcgtcacccagcaggtctcgagctaccgcgacatcagcctgggttgggcggcggcggcggccctgatcctgccgctggcgctgctgccgctcggcttcgactccgcctggtttccgggcattggcgacagctgggaggcggcgcatctggcctcgagggacatcaccgtggccaaggcgatcggcgcctacgccgtcctgcaggccgccttgttcatctcggtcttccttctcacgcgcatcccggtggtgctgcggctggtgacgccgccgaacgtcaggcgcattcgcgtccgccgcgccgccgtggcccagttcctggcgcatggcatccacgaaaccgaggcccggacaggcgttctgatcttcgccgccctctatgaccatcgggtggaggtggtcgccgacgagggcgtgcaccgcaaggcgccggcggaggtgtggggcaatgccgcgctcgccatcaccaaggccatgcaggacggccggccggccacggggttcgaagcggccatcagcctgtgcggagacgttctggccgagcacttcccgcccagcccaagcgacgtgaacgaactgcccgaccggctggtcgtgatctgaaccgcgcgccgcatcggggtcgcaatccgccgacaaaaggcctagccaaggcacagccgccgctatccaccgggattcatgccccgtcttctcacctacaatgtgcaccgctgcgtgggcggcgatcgccggctcgacgtggaccggatcgccgccgtgatcgatgagcaggagcccgacatcgtctgccttcaggaactggatgtaggccgcgcgcgcaccgggatggtggatcaggcgcgctccatcgccgaccgcctggaaatgacctctcgcttccacccggccatgcgggtcgaggccgagctttacggcgacgccatcctgaccccgcacccggagcggctgatccgcgccgacgccctgccctccgttcccggaatcccgggcctcgaaccgcgcggcgccatctggtcggcgatcgacatcgacggcgtcacgctgaacgtcatcaacacgcatctgggtcttgttccgcgcgaacagcgcgcccaggctcgcgcccttgtgcaggacggctggaccgacgcctgcacgggccccacgctgctggccggcgacttcaacgcgacctccatcacacgcccctaccagatcctgtgcggccggcttgaggacgctcagcgccaactgggccttcgcccctcggtcaagactttcccgtcaggcttccccgccatccggatcgaccactgctttgtcagcccgcatatcgagatcaccggcgtgaagacggttttctcgccgctggcgcgcaccgcgtccgaccacctgccgctgatcgtcgatttcagagtgcgtccggagagctgaacgtcagccgggctcccgcccgccctcggacgccgggcgagtgcgccgcgagcgctccagccgcttccacggcctccaggcgtccgacgacgatcccggatcgccaagctgccactcggcgatcatccgctcgatccgcttcggcgggtccgagccgagcggatcgagcctgcgctctccaaagctgcagatcgcctttccggtggagccgagaaccgcctccatcgctccaaacgtctcgccggacacgccgacgaaatgcccgatcgtgcggtgtcgatgcgcggcgatggcggcgcgcccctccatcgtcgggggctcgaccgacacgtcgcactctgtgtccagccccatagaccggttgttcaggttggtggagccgatccgcagcagcttgtcgtcgatcaccgtcaccttggcgtggactatgatccgctcgccgccttcggttcgggggctgaaggcgaagaagcggttgttccggtccgccgcctccagtcggtacaggacctcggcgcgcgccgtgtccatggtcatgctgtcgaaccagctggggctcttgccggtggagatcagcaccacctccggaccgtccggctcggccagccgctcggccagcgccgccgcgatgaccggcgaggtgaaatactggttctcgaagtagatcagccgcgtggcgcgccggatcgcctccagatgcagcgcctcgttctcgcgcacctccacgcgaccggcccacttcggctcggtgcgcgagacgcccaccggcgcgtcgtgaatggcgaccggaacattgtcgggccaggggtcgccgtccacctcgtccggcagcgtccgctcccacgtggccttgaaccatcgctcgcgagcgagatcgcccagcgcgcgcgccgcaggcccgctgacgaccgccatggtctcgtgccgcggcttgcagatgacgccggacggcaggcatcggcgcgggtcgtgatcaagatgctcggccgtgtcccagcggtcggtggagacgtcgccgccgccgcagaaggccaacttatcgtcgatgatcaccaccttctggtgatgacaggcgccgatgggcccgggcgaatccagccggaactcgaccatgcgcttgcggaaccagcgctgcgccttatgcggatagaagccttgcgacgccgcgatcagcagcggcgacttccagatcagcagcctgacgtccaggtccggcctgcgccgcaccagcattcgcaactggtgcccgatctcggcctgcttgtcccctggccgggtgttggcgtccagatgggtgcgcggatcgaactgccagcctaggatcaccaccgaccgctgcgccttggacaaggaggacgccagggccgtgaaataggcgtcgttctccatcagcacggcgaagcggtccgcctgagcggtgcgccacaggcccggccccggttcgagcagactgcctttgtagccttcgtctgtagccgtcatccgatcagcctgcctgactcgcccgacaacggtatcgaggtctcatgacgcttcagcttgctctccgttccacggttgcggttcgcgggtcaacggccacgctcccagatcattgttgttttcgccgcatgggcgtagaagggacggaactggatgctttgggaggggcggccgtgcagacgttgatcgagctgatcgccggcttcattgtcttcctggctgcggccgccctgtctcagttcggcgtcgatatccacgcccctcgtccggccgaacgcgaagtgcaccgggtcggcgactgtcggtcaagcgccgccgcgcccttgttgaccgccccttcgacaaagccccgctgctgacgggatcgggcggcatccgcctttgacctcgccgcgcgagccgctagggtctcctgcgcccgctggcgtcctgtcagtccttccgtgatcgagatcgacatctgatgaagtcccgcatgcggccgccgctgaagctgaccgaggacgaaccgccggcgtccgcagagctgtcgccgccgatcttcgacagggatgatcaggatgggcccgtgcagcccgcgagtcgggcgcccgccgaccctggcgctcgagccgcgcccatgtcggagcgtcaacgccgacgcctgatggagcagcaggccgcgccgccgccggccgcgcagccgctggcgaccgcggacatcgccctgcccccggacaccgcgcccgccccgtatcagccgcccgtcaccgcgcgcgcgtcgcgcagacgccaggacgctacggtgcgccaggcctatatcatcgcaggcgtggcctcggccctgtggatcggcgggatcgcgtcccccgcggcctatgagttcggttcgaacgggcagcccctcgatccgctgcgcctcgctgtctatctgctgatcgccctggcgcccctcgggctggcgctgatgctggcccacgtcgtgcgtcagggcgccggccttgcggcggaaagccgtcgggctcgcgagctgtccgacgccctggtggctccgacggccctggccgcgcagcagaccggccaggtgctgcagaccctgcgcgccgacatcgacaacgccgccctgacgaccgagcgcgcccgcgccgacatggccctgctgcgcgaggcgctggccgaggagaccctgcgcctgaacgaggcggccgagaccgccggccgcaccgcccgccgactgggcgagaccctaggccgagaacgcgaccagatgcagacgctgtccgttcagctcgattcgcagtccgtcggcgtgctggacgccgtcgagcgccagtcgcgcatggtggtggacgcgtcggacctcgcccagacccagttgcgcgaggcggaggcgcttctggccgcccgcgccgccgatctcgccgccgcggcgggagaggcccaggacgccgcgcgtctggcctcggacgacttggcgcgccagacgctgcggcttgaaaacgccggctccggcgtcgccgaacagatccagctggtggaggaaggcctgggccagcaacgcgcagcgttggtgaccacggcctacgcccttcgaaccgaccaggaagacttctccgcccaggtcgaaagccagcgcgcccaactggtggagcagctgtcggcgtcgcgcgccgcggccggcgagctcggcggcgcggcccaggcctcggccgaatcgatgcgcgagctgatcgaggccgcgtccgaccagctgcgggccttggtggagatgtcgcaacgcgaggccgatgggttcgacagcgccaccaagctggcgctggaccggttcgaatcgctcgccgccgaagcccgcgactcgctggtggaggagacccgtcgatctttggaggcgcttcaggccacggccgaggactcccgcgccgccgccgccgaagccgccgagcaggctcgccaccgtgtcgaccgactgggcgaatgtctgttcgaggcggcccagcgcgccgatcaggcggccgacgcccgcatcgaggaagcccgccgggtcgtcggcgaaacggccggcctggtggatcaggccggcgaacaggcggtggagcgtctggaggtcctgcttgagcgcatgaacgcgacactggagcaggtcgacgccgccttcgccgaaatcgaccagcgcgccgcccgcctgccggaagatgcgcgcgcccacgtcaaggccgtgcgcgcctcggttgaagaaggtctcgcctccctgaccgccgcctcgcgcaaggcggccgaggacaacgaggcgctggaagccggcttccaggagcgggtccggcgcaactacgacatgctgaacgaggcggtgcgcctgatgagcgtcgtctcgggcgacggggcggcccggcggcgcgacccggccgccgccgagcccgagcgcacgccgccgcgtccgcctgcaccagacatcgagcctgtgcaggccgagcgccgcgccggcggattgcgtgggcggctgggccttgcccggccggagccgacggagccgtctgcacccacgcccctgcctccgctgccgccctatgtcgctccgcccaccggcggcgatgatgtcggtttggactggcaggatctgatttcggacggcgagccggagacgccgcgcgcctcgacgcctgccgagccgccggacgccgcactgggtgagcgcatgatcgcctcggttcggcgcatgggcatcgatcccaacgccctgctgccccgctcccgcatcgaggaggccgcgcgtgcgatcggacgcagcgatcccgcagcggctcgccacatcgtccggcgcgtggcgccggcggcggtgcgcagcgtgtcccgcagggtgcttggcgatcccgaactgcgctcggatgccgaacgctatgttcgaggcttcgccggccggctggcggacacggcgcgcggcggggatgtggccgatgtccaggcgcagctgaccacggacgaggggcgcgccttcatgctgctggacgcagcggtcggagacgtcgcgggatgaccgggcgcggcgatgcggcgctccgtcgccccttggccagtgcgggatgacggtcggcgctcgcgggctgatcatcgcgtcgggcctgtgcggcgctctggcggtcggactgggcgccttcgccgcgcatggggtggaagccgacgcgcgcgccttgctgaccacggcaggccactatctgctggtccactctgtgttggcgacggcctgcggcctctggcgcgaccagcgcgcagccacggccggtgccctggcgcttggcggcgcactggtgttcagcctgtcgctttcggccatcgccctgctgggtctcagatggatgggcgcggtggcgccgatcggcggcgtgctgatgatcctgggttggcttctgctcgcccatgcggcatggcgtcagagacgttccggcgatccctcgctttactgaaagatcctgccccagatggcttttccgacgcccgacctcccgcgccgcgacctctatcccgagattgagccgttcgcgtcaggctggatggagacggacggcgttcatcaaatctactatgaggaatgcggcaatccgcaggggctccctgtggtggtcttgcacggcgggccgggcggcgcggtcaaccccggcatgcggcgcttcttcgaccccgccaagtaccgcatcgtcctgttcgaccagcgtgggtgcggacagtcgcggccgaatgcatcgcttgagaacaacacgacctggacgctgatcgaagacatcgagcgcctgcgcgagcgtctgggcgtggatcggtgggtggtgttcggcggctcctggggctcgaccctgtcgctggcctacgccgtcacccaccccgaccgcgtgctgtcgctagtgctgcgcggaatcttcctgctgaccaggaaggagcttcactggttctaccaggacggcgcctccatgatttttcccgacgcctgggagcggtttgtggagcccattcccgaggccgagcgcggcgacctcatgggcgcctactacaagcgtctgatcggcgacaacgtcgacgagcgggaacgctgcgccgtcgcctggtccagctgggagggcgagaccgtcagcgccgcagggcccgacgcccgcccggacaagttcgccgaacccgagttcgccgtcgccttcgcacgcatcgagaactggttcttcaccaacggcggcttcttcgaggaagacggctggctgctgaagcaggtcgatcggatccgccacatcccctgctggatcgcgcagggccgcttcgacgtggtgacgccgatgtccggcgcctgggcgctgcaccgcgcctggcccgaggcgaagctggatgtcgtcggcgacgccggccacgcctcgtccgagccggggatcgtcgacagcctggtgcgcgcgacggattgggccgccggtctctagcggcccgccgacctcagccgcacttcacctcgcggatgacgccgctgctctcgtcgaacaggatgttcaggcgcgccggattatagtccatcgtcaccgggcaggtggtgcaggtcacccgccatgtcgcgcccgcgggctggcccggaagctcggagcggttgcggccgatatagctgcggtaagcgtccgcccggcattgcgacggtccctcgcccgtcgacgaacgatcgggatcaaccccggtgaccggggcgcaggcggcggcgcagagcagcagggcggcggacgacagtcggcggatcatgggacgttctccttcagcatggggcttcagccgcaacggacctgctcgatcacctcggtcttttcgtcatagaagacgttgaggcgatagggtgagaagtcctgggtgaccgggcaggtggtgcaggtcacgcgccggttcacgacatcgaccggcaccgggatttcagcctttgtgcggccgaccagccactgcatttcgccggccttgcacaggtcggcggtcggatttgtcggaacgcggctgccgatcggaggattgagttgcgcttcttcgactgcacggggcgcggacttgtcggacacgggggtcgaacaggccccaaggacagcgagagccgcgatcaggccgccttttcccagcgtccgtcctcggactggcgccagtagctgaggtcggcgccctgccccttcagccgccgccaacgctcgcgcgccgcagccagcgcctgatcgtcgcgtccgtcgaagatgatgaagcaccgctcgataccctccaggccatccaggtccgtgtcgtcgatgacaaacagcgcctgagaacggttaaggttctcggccgcgacgcttagcagcaccggctggcgctcggcgtggggctcgtccgcgcgcccgtgcggcaggaagctatcgtcgcggaaggtccagagacgctcgttcaccggctccagcgcctcgaacgaggcggcgcgcacggtggcgcgccatccccgttgaagcgtcttgtcgagcagcaccggcagcacctgatcgagcgaggaccgctccaggtggtagaaccagatctcggggccgccctccgccgtcatcagccttcgtaggcgtccgccaccatgcgatcgagcgtgcgcacgccgaagcccacggcgccgtccggcacggtcgggttgatgctcttgttggtccaggcggtcggcgcgatgtccaggtgcgcccacggcacgccattggtgaagcgctgcaggaacagggcggcggtgatcgatccgccggcgcggccgttgccgacgttcttcacgtccgcgatctggctgtcgatgtgcttttcgtagatcgacgggatcggcatgcgccagaagttctcgccgaccttgggagctgcggccagcacgttgttcgccacctcgtccgagttggagaagacgcccgcatagtcgaggcccagcgccacgatcatggcgcccgtcagcgtcgccaggtcgatcatgaacttgggcttgaagcgctcctgcgtataccagagcgcgtcggccagcacgaggcggccttcggcgtcggtgttgatcacctccaccgtctggccggacatggacaccaccacgtcgcccggacgctgggcgttgccgtcgggcatgttctcgaccaggcccaaaacgccgaccgcattcaccttggccttgcgaccggcgagcgcatgcatcaggccggacacggcggcagcgccgcccatgtcccacttcatgtcctccatgccttcggacggcttgatggagatgccgccggtgtcgaagcagacgcccttgccgacaaaggcgatgggctgctcgccctcattgccgcctttccattggatcacggcgagttggctctcgcggcggctcccctggcccacggccagcagggtgcgcatacccagcttctccatctcggcttcgccaaggatctcgacctcgagacccaggcgctccagctccttcacgcgacgcgcgaactcggcggggtagaggatgtttgcgggctccgacaccagatcgcgggagaactccacggcctccgccacggccgccagcggctccagcgcgacctgcgccgcacggacgtcggaggcgaccacgcgaaccgaggtgatcgagggcttcttctcgggcttctccgtcgtgcggtaacggtcgaagcggtagctggccagccgcacggcgaaggcgatccgcgccgcctgttccggcgacaggtgcgccgcatcgatggtcaggcagtccgcgcccgacagcttgaccgcgtgataggcgttggcgcccgccgcctcgacggtgaggtcgtcgagcgcgcccgcgtcgcccgcgccgatcagcacgatggtgtctgcgtccgcaccggcggttccggcgacgctcagactctggcccgcggcgcccgtcagtcggctcttgctcatcgcgcgcgtcaaagacccgccggttttgccgtcgatctcggcccccgcacctgcgaactggcgtccctcgtggaccagcagggccaggatttcacaagcgccgggggcggccacaaactcgatcttcatacagaactccggccgggtcgcgccgcccggtcttcttggtaagcgatgaggaagggccgtcggcttgccgccgccgtgccgggatgtgctactagatgcgcctcaacagggccgcctgcaaccgggtggatgcgccacgtctacgatgctgattcaacgctacctttttcgacagatctcgacgcgcgtcgtggcggcgtgcgccgccctggcgggaatcggcgtgctgagccaaagcctggaccagctggaagtcatcgtcgagcgcggccagagcgtctggatcatgatcaagttgacgctgctggcggtgccgcagctgctggctgtgatcctgccgttcggcctgttcgtcggcgccctgatcgccctgacccgcctgcagcgcgagcaggagctgaccgccgcattcgccggcggcatgacgcggtggtcggtgatctcgcccgcgcttcgcctgtccgccaccgtcgctcttctcgccctgttcatcaatctgttcgcccagccctgggcgcagcgcgaggggcgcgcccagaccttcgccatccgaaccgacctggcggcgctgctggtgcaggaggggcagttcgtacaggggccggagggcctcaccgtctatgtgcagcagatcgagcagaacggcttgctgaagaacctgtttatctaccaggaagacgaaggcaaggtgacgacctgggacgccgccgaggccaggttcggccgcgccaacggcgcacccgtgctgaccctgaacgacggctcctggcagcagtattcgtccagcggcgtgctgaactacctctcgttcgacaactatgtgttcgacctgtcgcccttcaccgcgacgaccgagacggtgcgctacaaaccctccgacctgtacctcagccagctgctgcggccgacgccggacctgctggagacggctgggtcgcgcggcgagctgttggccgaggcgcattcccgcatcgcctcgccgctctatgtgctggtcgccatggccatggccatggccgcgatcatgggaggcgcgttcagccgcacgggctactccgcgcgcatcgccaaggcggcggcggccttcctggtcgtgcggatcgtcggtttcgcccttgtcgccgccagcgcctggaacggctggctgaacgtgctgcaatacgtcgtccctgtcgccgccaccgccatcgccctgcgccttctgtttcgcgcgctgaagcccaagcgtcgcaggcgctggcaggtgctggccacgcaaaaagcggggctggcatgaccgaggctccgtcatcgtccgcctcgcccttccgctggcccgcgctgggccgcatcgaacgctacgtgttgggccagcaactgcgtgcgctcgccgtggcgctgggcgtcatctcggcgctggtcatgctgatcgacttcgtcgaagtctctcgcgggcctgggtccagcgcggacctgtccgcgttccagacgctgggtctcgtgctgctgaagtctccggcggtcatcgtcaccctgctgccgttcgtgttcctgttcggcaccctgttcgcctatgtccggctgaatcgacgcagcgagctgatcgcgcttcgggccgcgggggtgtccgcctggcggttcgttctgccggcggccggcatggcggtggtcatgggggtgctcgccgtcgccgtgctcagcccgctggcgtcgaccgccgacggcctctggcgcagcgagcgtgcgcggctgacgggcgccgcgccgggcgtggaggccgccgaagccatctggctgcgcgaaggcgacgctcagcgtcagatggtgatccgcgccgccggccaggatcgcgccaccggcaggctcctgaacacgaccttcttcatctacaccaccgacgacgaggggcggcgcaccttcaacgaacgaatcgacgcccgctccgcgacgctcgccgccggccggtggcggctgacggatgccgtgggggcgcagatcggccagcgggccgtgcgctacaagactctggacctgacgtccaatctggcggatcgggaggcgttcgaccgcttcgcccggccccagtccacgcccttctggtcgctgcccaaccagatccgccgcatcgaggacgccggtttcacctccaccgcctatcggctccagttccagcaggcgctggccacgccgctgatcttcggggccatgtcgatcctggctgccgctttttcgctcaggctgatgcggctgggcgacgtagccaagatgagcgtctcggcggtggtgctgggcttcgccttctttttcgtgacccagttctccgcagccatgggatcggccgaggttgtgccccccgtggtcgcggcgtggttgccgccggttctgacgacgctcgcggcccttaccttgctgttctataccgaagacggctaagccgcgcctgagcccacgggcttgggcgtagagttcggacgggacggatggttcatgcagcttagcgggcggcttcaggtcttgcgaattcgcctcctggccggagcggcgctggcggtgctggcgcccgccggcatggtcgcggcccagacgcaaccaccggtccagcaggcgggccctgacgccctttcgccggacgctgtctatgtcgaggcggacgccgctgtgcgtcagggcgacaccatcacggctacggcaagcgacagcgaacgcgcgctggtgcgcgcgcgcggctacactctacggggcgaaaatctcagctacgatctggcgcagggcgcggcgacggcggaaggccgcgtcgagacagtcgcacccgacggtacggtggtctacgccagtcgggcggaattcggagacgacttcacgaccggcgtagctgtcgatttcgccacgcgaacggccaatggcgccagcctgatggccgcgacagccgtgcgccgcgacgccgggcgtaacgagctgaactacgcgctgttcacgccctgcccgatctgcgacgcaaccggacccaagacccccagcatcgccatccaggccgagaaggtggtccaggacgccgagctgcgagccatcctttatcgcaacgcggtgttccgcatcggcggcgtgcccgtcttctacacgccctttttcgcccacccggacccgactgtggatcgcgcctcgggcttcctgattccggtgctggactacgatgagggccgcggtttctcggtcgaaacgccctatctgcatgtcgtctcgccatccgaggactggctgatcagcccccagttcaacaccgatgtcgcgccgttcctgaacctgcaatggcgccggcgcttcgccaacggcatggtggtggtgcgcgggggctacacctacgagcgcaacttcggcgacttcgacctcgacggcgacggcgactacgaaagcaacgtcagcttcgatgatcgcgagagccgcagctatctgctgtcccacggcgcgttcgacctgcagggaccatggcgcgcgggcttcaccctggagcggacgtcggacaagacgctgttcgaccgctacgacgtcagcgacccttatcaggacaacggcctgtactacggcgaccgccgccgtctgatcacccaggcctatgcggagcggcagacccaacgctcctatttctccattgcggcctttgcgctgcaaagcctgcggcttgatccccgtttcgccgataccgacttccgcgatcccagcggcttccaggtcttcgaggacgaggacaccctgccggtggtcgcccccttgatcgacttccgctgggagccgtattcgccggtcttcggcgggcggctgcggctggaggcgtcggccgtgtcgctgacgcgcgaacgctttgtcggcgcgccgatcctgagccctgaggttcttcccgccgtttccgacggcttgcctggcgtggacacgcgccggatcaccggcgaggcggagtggcgtcgcgtcatcctgacggcgggcggtctgcggtgggagccgttcgtcgatgtgcgaggcgacgcctacgccgtgtcggacctgccggtgatgatgaacgtctcggatgacgagaccgtcacgcgcggccgcgccagcgccgggctggacctcgcctatccgttgatccgacgcaccgccgccgccgacatcattctcgagccgatggcgcaactgtccgcctcgaccacgaccgagttggacccacgcatcccgaacgaggacagccagacgctggagctggacgagacctcgctgttccgcctcgaccgctttcccggttacgacctgctcgagggcggggttcgtttcacccttggcggcagggccacgatccgatgggccgaagaccgacgcgccagtctgtttgtcgggcgcagctatcgcttgaacgccgagaacaacttcctggccgccgtgccggacgcgccggatcagagctatgatccgacggggctggcggccaagcgatcggactgggtggtccagggcgacttctctccgtccgaccggattcgcggctggggccacgccaccatctccgacaacggagacatccgccgggcgcaggcggctgtcgatggtcgttggggcctgcgcaacgtggcgagcctcagctacatcgtggatcgctccaatccggtgctcggtccgttgaatcggaattacgagttcgtccaactggcggcgcagcagctggtgtacggcaactggggcgtcgcgggggccgctatcgccgacctgaaccgcgacgagatcacccgctctgaggtcggcctgctgttcgacgacgactgcttccgcttcgagatcggcttgcggcgtgacaacacccgcgtgcgccccagcggcccgtccgagggactctatgtgcgcctaaacctcgccactttcggcggggcagattacagacgaggcgagatacggtaggtgatcgtgcaggatcgccgaaccgggggacggccgaccgtgaacccgcgccaggacgcgcgagggtcgctttgaggaaccaggacgaacgatgcgtgtgatgcgttacccgatggccgtcgcgatggcggcgatcctcgccggcacggcccatggccagacggcgccgacgcgctcgaccgcgcccgcctccacgcccgcgccttcgtccggacagtcggcggcgggggccttgaaccccgccgccgaggccgctccggcgccggccgccaccgctccccaattcgacttggccgacggcatcgtagcctcggtcaacgaccgcatcatcaccggctatgatctgcgccagcgcatgttgatgctgattctctcgtccgagattcagccgactcaggaaaatctgcccgcgatccagcaggccgccctgaacgccctgatcgaggaacggctcaaggcgcaggagatcaccaactacgaaagcctgcgggtcagcgacgaagaggtcagcgccgagatcgccgaaatggcgcgccgcgcgggcctgacccccgacgcctatctggcgcagctgtcgcaggccggcatacagccccaggctttccgcgagaacctgcgcaccgagatcgggtggagccagctggtcgggggacgcttcaacagccgcgctcgggccagtcgctaccaggtggaggccgaagtgcgtcgcctaaatgaagccgcgtccaaaccgcagtatctggtgggcgaaatctacatcgaggcggcgcgcgtcggcggccagcaggcggcgctggacggcgcccgtcagttggtccagcagatcgtgggcggcgcgcccttccaggccgtggcccagcagttctcggctgcgccgtcggcagcggctcgcaatccgggagacgccggctggatcgtcaaggacacggtgcagcccgccctgcagcaggcgttcgaccagcttcaggtcggccagctgtccaaccccatccccgtcgatggcggagtctacatcatctacatgcgcgacaagcgcgaaggctcctccagcagcctggtatcgctgcgccagctgatggttgaactgccggagaccgccagcgaagccgatgtcgccgctgcgacccgcacgctagaaggcctgcgtcagggcctgacgtgcgacaacatcctgtcccaagccacggcgacccgcggcgtcctgggttcggatctcggcgaatcggacgtgcaaaacctggcgccgcagttccagcaggttgcgcgctcagccgagatcggctcggtcagcacgccgatccgcacgccgctgggccttcaccttctggcggtctgtggtcgtcgcgttggggggctcgaggcgccgtctcaggctgacgccgagcgccggctgcggggtcagaacctggcggtcctggaacgtcgctaccttcgcgacctgcgcaacgacgccctgatcgaggtcaagtgacggctcctctggttctgacgcttggcgaacctgccggcgtcggcccggagatcatcgcggccgcctggcgaaccctgtcaggctcgaacgcgccttttgccgtcatcggcgacgcttcgctgctgagatcacagggtgcgcctgtggcggagatcatggctgtgtcggaggcgccgtcgcgattcgcgtccgccctgcccgtcatccaccatccccttcccgcgccagtcgagccgggcaatcccgatccgcgcaatgcgcccgccgttgcggacggcattgagctggccgtgtctctggcgctctcaggcgaagcatcgggcgtcgtaaccgcgcccatcgctaaagcgccgatgtacgcgtcaggctttcgcttcccaggccataccgagttcatcgccgaactgacagccgatgcgccctatgccggcacgcgtggcccggtgatgatgttgacggcgcgggacctgcgcgcctgtctggtcaccatccatgtcgcactcgatcaggcgtcgcagctggtcacggctgaccgaatcacccgcaccgcgcgcgtggtgcacgagagcctgaagcgggatttcggcatcacgtcgcctcggttggccatggccgcgctgaacccgcatgcgggcgaaggcggggctttggggcttcaggagcttgagacactgatcccgaccgccgagcgcctccgcgcagagggcatcgacatctccgatccccgtcccgccgacacactgttccatgacgaggcgcgacggacctatgatgcggccatctgcatgtatcacgatcaagccctgatccccgtcaagacgctggacttctggggcggcgtcaacgcgacgcttggcctgccgatcatccgcacctcgcccgatcacggcaccggcttcgacatcgccggtcgaggcttggcgcgcgccgacagcatgatcgccgcgattcgacttgcgtcggagatggcggcggcgcgagcggcgcgctaacacccggcgcgtgaccgaccttccttcccttcgcgcgacgctcgacgcccacggccttttggccaagaagagctttggccagcatttcctgctggacctcaacgtcactcgcaagatcgcccgcctggctggcccgttcgacgggcgcggcgtgatcgaggttggcccgggccccggcggcctcacccgcgccctgttggagagcgacgccggcgagatcgtgctggtcgagaaggatccgcgcttcatcccgctgctgtcggagctggacgacggcgccggccgcctgacgatccacgaggcggacgcgctcaaggtccgagaagccgagcttgtggacggccccgcgcaccttgtctccaacctgccctacaacgtcggcacggcgctgctgatcaaatggctgaccggcccttggcttccgcacgccctgaccctgatgttccagaaggaagtggccgagcgcgtggtcgcggcgcctggcgatgaggcctatggccggctggcggtcatcagccaggcggtgtgtgaggcgcgcatcgtcatgcacctgcccgccgccgccttcaccccgccgcccaaggtggcctcggccgtggtccacctgacgccacacgccgaacgccccgcacccgacctcttgaagcggctggagcgggtcacagcctctgcgttcggccagcgtagaaagatgctgcgctctagcctgaaaccgctcggcggcgccgccctttgcgaggcggccggcattgaacccgacgcacgcgccgagaccatagacagcgccggcttcctgcgcctggccgagcaactgccatgaccgttgaaccctttcgcgccatcagcctcagccgcctggctcatcagctgaaaaacgaaggccgctcgatcatccacatggaattcggccagccttccaccggcgcgccggccgccgccctcgcccgcgctcatgaggtgctggaccaggacgccatgggctactgggaaagcgcgccgctgcgcgagcggatcggtcgcctctatcaggatcgctacggcgtcgaggtcgatcccgaccgtattctgctgacctgcggcgcctcgcccgccctagtgctggcgctggccagccgcttccggccgggcgaccgcatcgccttggcgcggccgggctacgtcgcctaccgcaacaccctgcacgcgctgaacctcacgccggtcgagatcgcctgcgggccggagacccggttccagctgacggccgcgcaactcgccgcgctggaccccgcgccggctggcgtagtcatcgccagccccgccaatccgacaggcacgatcatcccggaggccgagctggccgccatcgcctccgtctgccgtgagcgcgggatcgcgatcgtctcggatgagatctaccacggcctgtcctacgtcgggccgacgccgtccatgctgcagttcgagcctgacgctctgatcatcaacagcttctccaaatactggagcatggccggatggcggctcggttggctggtcgcgccggaacatcatgtcgcggcggcccgggcctatatgggcaacctgtttctgacgccgccgtcgctgagccagcacgccgggctcgtcgccatggactgcttggaagaactggaaggccatatccagacctatgctcgcaaccgcgcgctgctgctggacgctctgccgtcgctaggacttcagcggatcgcgccgccggacggggccttctacgtctgggccgacatcggccacctgacgaacgacagcatcggcttctgcgagcagctgctgcgcgacacgggcgtggcgacggcgcccggcgtcgacttcgatcccgtcgatggtcaccgcttcatccgcttcagcttcgccgtctcgacgccggaggtcgaagaggcgctgaaccggatgcgaccctggttcgctgctagaccgcctctctgagcagcgcaccgcgatagtcgccgacccagagattgcggaaccggcgcgaccgctcggcgtgatagatgtgcgccagctcggcgtaggaccggtcgaaatcgtcgttgacgaagacgtagtcgaacgcgtcacagtgctcgatctcgcccttggcgttctggatccggcgctcaatgacgtgttcggcgtcctgtgaacgcgtcaccaggcgccggcgcagctcctccaggctgggcggcaggatgaagacccgcaccgcatcctccgggcatttgcgcgccacttcggccgccccctgccagtcgatgtcgaacagcacgtcgcggccttccgccagcgcccgatcaatcggcgcgcggggcgagccgtagcgctggccgtgcacgtccgcccattccagaaacgcgtcctggtcgatcaggcgctggaactcggcgtggctgacgaagtggtagtcccggccggccacctcgcctggacggggatcgcgggtggtcatggagatcgacagctcaagtccgccatggtcggccatcagccgccggcacaggctggtcttgccggcgcccgacgggctggcgacgatcaggaggacgccccggcggggcgtacggtcattcgacattctgaacctgttcacgcaactgttcgatcacggccttcagctcaaggccgattccggtgagcgcggtggtagcggatttcgagcacaaggtgttcgcctcgcgcatgaactcctgcaggaggaagtcgagtttccgaccggctggcgcctgggccacaagcgccctcgcggaggcgacgtgagccgtcaggcgatccagttcctcgcgcacatcggccttggtcgccaaggcggcggcctcaaggaagatgcggtcgtctaggccgggcgcgtcgggcgcgagttccttgatgcggcgggtgaagcggtcgcggatcgcctcgacctgctcgcccgcttccttttccgctgcgctgatcaggccttcgatgcggccgatgaagtcgatcagcaccggctcaagctgctctccttctcgttcgcgggagaccttcagcgcgtcgagcgcctcttcgattgtccgcgccatggcggcttccagcacgtcccgcgcagtcgcgtgggcgtcttcgtctgcggcttcgatcacgccgcgcaggctcagcaggccgtccgccgacggcggggtcgcaccctcttccgccagctgattcgccagcatcagatagcgggtgagcagcgcctcgttcacggccacgggcgaggcggcggcgccgtcacgcctggcgtgcagaccgacattgatctggccacgggcgaagcgcgcctgccccgccgccttggtcagccgctccagagtgtcgaagccggtcggcccgcgaaaccgcacctccagattgcgaccgttgaccgatcgcgcctcgaccgaccaggtccagccgtcggctgagccatccgcccggccgaagccggtcattccccaaatggacgtcatcgcggtccctggctcgcgcccggcggcagggtgatcgtcgcctgaccgccggcggccggcgcggtctgcggctgctgctcaggcggcgtcatcggtgcgggcgctgcacccggcgcaacgggagcgggcgcatccgggggcaggcgggcgcgctggcgctcgatctgacgccagcgtgccacgttgcgcaggtgctcctcataggtgtttgcgaacacatggccgcccgtcccgtccgcgacgaagaacagggccggatcgctttgcgggttcaacaccgccttcagcgcctccgcaccgggattggcgatcggcgtcggcggcaggccgtcgatcagataggtgttccagggcgtggcggtccgcagttcggacagccggatgccgcgcccaagcggccgacccttggtgatgccgtagacaatggtcggatcactctccagccgcatgccctggcgcagccggttggagaagacggcggccacgcggggccgttcggccgcgatgcccgtctccttttcgacgatggaggccagcaccagcgcctcctgcggcgtgcgcaccaccgtgcccggcgagcgcgccgcccagagttccgcctggttgtcccgcgccgcgcgctgcattcgcgcgatgacggattggcgggtctctccgcgtgcgacctcataggtgtccggccacaacgagccttcctccggcgtctcgcctgcggggccgggcagcacggcctctccgttcaggatgtccaccgcctgcgccgacgaccagccctccggcagggtgacgaagtggcgcacgccgcgcccctccgccagcaagcgaatcacgccgcgcagcgaggtcccggacggtatctcatattcgccggccttcagccgccggtcgtcgccggtcagggccgccgccgccttgaacaggtctgtcgagcggatcacgccactggaccgcaggttcgccgcgatggctgagacgccagcgccgctcggcaggatcacgattgtggagtcgccctggcgcgcgctgggtcccggcccgaaatagatagcccaggccgcgatcagggccacgatcaggaacagcccgaacgtcgccgccccggtcagcagcgcgaccggtcccgaccgtcttgcgacagggcgcttgccgggcgggcgagccacgcggcgcgggcgacgcggcatctcagtcgaccttccggaagatcacggaggcgttggtgccgccgaagccgaagctgttggacatggccacatcgatcttcatcggcttgcccttgtggggaacgaggtcgatcggcgtctcgtgcttgggatcgtcgaggttgatggtgggcggcgcgatctgatcgcggatcgccaggacgcagaaggccgattcgatcgcgccggccgcgcccagcaggtgtccggtcatggacttagtggacgatacggcgaggtccttggcgtggtcgccgaccagccgctccaccgccttcagctcgatccagtcggccatggtcgaggtgccgtgcgcgttgacgtagtcgaggtcggacggctggagccccgcacgcttcagcgccgccttcatggcgcgcagaccgccgtcgccgtcttcggacggggcggtgatgtgataggcgtcgccgctcatgccgtagcccacgacctcgcagtagatcgtcgcgccgcgcgccttggcgtgctcatactcctccagcaccaggacgcccgcgccctcacccatgacaaagccggcgtgctcccggtcgtagggccgcgacgccttctcaggcgtgtcgttgaaggacgtgcacagcgccttgcaggccagaaatcctgctatgccgatcggcacgaccgagctttcggcgccgccgcagaccatgacgtccgcatcgtccagcgcgatcattcgcgccgcgtcgccgatggcgtgggcgccggtcgcgcaggcggtcaccgcggcatggttcggccccttcagcccgtgtctgatcgatatctgcccgccggcgagattgatcagcgcggacgggatgaagaaggggctgacccgccggggtccctgctccttcaggatgatggcggtgtccgcgatgggacccaggccgcctatgccggcgccgaccatcacgcccgtgcgttccttgtcctcgtcgctttcgggtttccagccggcgtcgttcagcgcctcgtccgccgccgcaatagcgtagaggatgaagtcgtcgacccgcttgcgatccttggccgacatgatcttgtcgggatcgaagtcgccctcgcccccgccgccgcgaccgtccacgctcggcacctcgccggcgatggtgcaggcgtaaccttcggtgtcgaaggccgtgatcggaccgatgcccgatcgcccttcgacgatgccttgccaggtcttttcgacgccccagcccaggggggtcagaaggccgatgcccgtgacgacgacgcggcgcatggatggctctccctcttgatctcgatcgtgcgcccgcgaatccctgtcgtgaaatcctcgggtcagaaacagtaaaggccgccgggcgtctccgctaggagcgccgggcggcctttaaccgttcagccgaatggctggatcagcccgccgacttctcgtcgatgaacttgaccgcatcgccgaccgtctggatgtgctcggcggcgtcatccgggatttcgatgtcgaattcttcttcaaaggccatcaccagctcgacgttgtcgagcgagtcggcgcccaggtcgtcgatgaagctggccttttcggtgaccttgtccggatcggcgtccaggtggtcgatgacgatcttgcgaacgcgctcgagggtgtcggacatcggtgtctctctgcctgtttgtgtagtcgccgtagaggcggggtctcatcggtaaatcgccgtctcacggcagcaagggcgacgcaagcccaaaggatgggccgccaaagcattcccgccctttagcacagccggtcgggcgggaaatagtttagatcatcgccatgccgccgttcacgtgcagcgtctgccccgtgacataggccgcctcgtcggacgccagatagacgacggcggcggcgatctcctcgccctgccccaaccgcccggccgggatgcggccaaggatcgcatcacgctgcccctcgttcagcacgtccgtcatcggcgaggcgatgaagccgggcgcgatgcagttgacggtgattccacgcgaaccgacttcctgcgccagcgatttggaaaagccgatcatgcccgccttggaggcggaatagttggtctggcccggattgccggtcacgccgacgaccgaggtcacgccgatgatgcggccctggcgacgcttcatcatgcccttcacggccgcgcgggtcaggcggaaatagctctccagattgacctgcaggaccgaggcgaaatcctcgtccttcatccgcatcaacaggccgtccttggtgatgccggcgttggccaccaggatgtccagcggcgcgccggccgccgcttccgccgccgcaaccagaccgtcgaccgaggacgactccgacaggttggcggtggcgaaataggctcgctcgcccagttcgccggccagatcggccagcaccgcttcgcgcgtgcccgacaggacgacggtcgccccttgcgtgtgcaaggcgcgtgcgatcgcgccgccgatgccgcccgtggcgccggtcaccagcgcggtctttcccgagaggttgaacattccgtctctccctgttccgtcatcctcggacttgatccgaggatcaggcgctgtgccgcgccgatgttgatatggccgcttcgtcgtcggatgcgcagcggcggatgatccgatcctcgggtcaagcccgaggacgacgatggtctcaggcgattgatcgcgcgaacgcttccaagtcctcgggcgtattcagggccaggctctcggcgccgggcgcgatgcgcttggccatgccggtcaggaccttgcccgagccgacctcgacgaagcgggtgacgccgccttcggacgccagccattccatgctctcgcgccagcgcacccgcccggtcacctgctcgaccagcaggcggcggagggtctctggatcggtctcgggccgcgccgtgacgttggccacgaccgggagacgcggcgcggcgatcgcggcggacgagagcgcctgcgccatctcgtcggccgccggctgcatcagggggcagtgaaatggtgcggagacgttcagcggaatggcgcgggcgcccagttccttggccttttcaatggcgcggtccacggcggccttgtcgcccgaaatgacgatgttgccggcgttgttgtcgttggccacgacgcagacgccgagctccgaacccgcctgagccgccgcctcggcaagcgccagatcggtcttgggtccgatcagcgacgccatcgcgccccggccaaccggcacggcgcgctgcatctcctggccgcgcagcttcagcagacgcgcggtgtccgccaaagccagggcgcccgacgccgccaaggcggagtattcgcccaacgagtggccggcgacgaagctcgcccgatcgaccgccacgccgaagtccctgtccagcacccgcacgacggccaacgacaccgccatcagcgccggctgggcgttctccgtcagggtcagctgctcgtcgggcccctcccgcatcagtcccgacaggttctggcccaacgcctgatcgacctcggcgaacacatcgcgagccgaggcgaaggcgtccgccagcgccgcgcccatgccgaccgcctgactgccctgtccggggaaaagaagcgctgtggtcattgtccgtccacgatccgtgattccggcgcgaagcggtaggccgaaccttccgccggggcaagggagcgacggctttccccacgcgcccggctgttgctagggtggaccgatccacaggcggagccgcgcgatgagcctctacggcgactacgatcccgacaacatcttcgcccgcatcctgcgcgacgatatccccagcgtggtggtgtgggaggacgagcacgtgcgcgccttcatggacgtgtttccgcagtcggagggccacgtgctggtcatctccaagacgtcgcgcgcccgcaacatcctggacgtcgaggccgaggtgctggctcgcctgacggcggctgtccagcgcacggcgcgtgcggtcgaggcggcgctgaagccggacgggctcagcctgatgcagttcaacggcgacgccggcgggcaaaccgtgtttcacctgcacttccacatcgtgccgcgctggagcgaccgccccatgaagggccacggccatgcgccgcaggcggacccggaggcgctcaaggcgctggcccaacgcatccgcggcgaactccgctaaggcgcttgcgaaagcgggtcgtgaaaagcataagagccgctgatccgccgggcgcgggccggtttagctcagttggtagagcgccagttttgtaaactggatgtcgcgggttcgattcctgcaaccggcaccacgcgctctgagggaacgatcctcccgcatcgccatttttcacttgccggccgagcgtcgggggttcggtccgccgagcgccttgcagagcctgcgctcgccccgctgaaccctcgcgatcagcggggcttttccgttgaaatctggcgcttctttccgatcggcgctacagtggggcttcatcggggcgcgccttgattcatcctgttcgtcaggtggaatgtccgacaacatcaacaagctgggacacaggatcggcgcgcgcggaggccgcacccggcgctctatcctggacgccgcgcgcggactgctgaacgagcggcatgtgggcgagatccgggtagccgacgtggcgtccgccgccggcgtctcgccgtcgaacttctacacctacttcaagacggtggaggagccggtcctcgccctgtgcgaggaggcgggcgcggactgccggggcctggaaaagcatttccagaccgactgggcgggcgagcgcgcctttgcgtcgtcgcgcgccttcgtcaccgatctgctggcggtgtgggacaagcacgctccggtgctgcgggtcgagcacatgctggccgacaagggtgagccggcgttcgcggaaagccgcatcaaccgcctgcgccggctgcacctggcgatcgaacgccgcatcgcccaggcgcaccacagcggcctgatgcccaagacgctgagcccccgcctcgcctcctaccaggtcgccagcctggtcgaatcgaccgccgccgggttcgagctgctgcgccgcgcggacacggccgaggccatcatcgacaccaccgcgcacctggtggtgaagctgacgaccggccgctgaccgtcgtcagcccgcgcccatcgccactccgatccggtaggtcacaaaggccgccagataggccaagccgaacatgtaggcgatcatgatccaggtccacttgcgcgagttggtctcgcgccggaccacgcccagcgtcggcatgcactgaggcgcaaagacgtaccaggccaggaaggccaggcctgtcgccagcgaccagttggcggccagcgtcgaggccatcatccccgtcgcggtctcggcgtcggccaccgcatagaccgaccccagggcggcgaccgccacttcacgcgcggccatgccggggatcagcgcgatcaccatctgccagttgaagccgatgggcgcgaacagcggctcgagcgcatgacccaggatgcccgccagcgaatagtctatggctggccccgtcgcgccctccggcggataggggaaggtcgaggcggcccacaccaggatcatcagcggcaggatgatgcggccggcgcggttcaggaagatcttggcccgaagccagaggttgaacaggacgcttttcacgtccggcagcttgtaggccggcagctccatcatgaacggctcgaccgccccgcgccagaagacgcgccggatcagaaaggacaccgtcagggcgctggcgatccccgccgcatacagcccgaacatcaccagcccctgcaggttcgcaaatccccacaccgtcctgtcggggatgaatgcggcgatgatcagcgtatagaccggaatgcgcgccgagcaggtcatcagcggcgcgaccagaatggtggtcagtcggtcacgccggctctcgatcacacgcgtcgccatgatgcccggaatggcgcaggcgaaactcgacagcagggggatgaaggcgcggccgtgcagccccgcgccgcccatgatgcggtccatcagaaaggccgcccgcgccatgtagccgaaatcctccaggacgatgatgaacagaaacaggatcaggatctgcggcaggaacaccagcacgctgcccacgccggagatcaacccgtcgacgatcaggctctggagcagaccgtcaggaaccgctgtggcgaccagcccgcccaggcccgccacgcccgcctcgatcccgtccatcagcggaccagcccaggcgaacaccgcctggaacatgacaaacagcaggcccagcaggatcagcagaccggcgacaggatgcagcagcaccgaatcgatccgccccgtcagggtgtcgggccgttcgggcggacgcacgcaggccttcaggatgcgctcggcctcgcggtgcgccgaacggagctgcgccgcgtcgggtgcatgccacccattgtgggtttcgacgcgccacacgccggcctcggcctccaccgccgcgaccaaatcgtcgatcccgcgcttgcgcgtggccaccgtcgtgacgatgggaacgcccagttcatcgcgcagcgcatccagatcgatgcgcaggccctgtcgctgggcgatatcgtacatgttcagcgccagcaccatgggccggccgacctgcttcagctccagcaccagccgcagcaccaggcgcagattggtggcgtcggcgacgcagaccagcacgtccggcgcctcttcgcccgccagcttgccgagcaccgcgtcgcgcgtgacctcttcgtccggactgcgcgccctaagggagtaggttccgggcaggtccagcaccgtcatggtgcgcccgcccgcggagcggatcaggccctccttccgctcgacggtgacgcccgcatagttggcgaccttctggtgcgcgccggtcagggcgttgaacagggccgtcttgccgctgttgggattgccgaccagcgcgatgcgggcgggacgaagggcgatgtccatcaggcggcgtcgcagcggatcagcaggctggcggcctcgcggcgccgcaaggccacacgcatgtcgtcgaccttcatggcgatcggatcgcccccgaacagcccttggtgcagcagttcgacctgagcgccctcgacgaggcccagctccagcagacgtctctccagctcgacctcgtgttcctcgtgccgcgcctggtcgccgacctggacaatgacgccgcgatcgccgcaacgcgcctggctcagcttgatggttttggtcatgaacgctcgccttgacgacgccccccagcgccgcgattacctgacagtgattatcaggcgctacggcaggacgccagcttggcggcggcttggacatcctgcgccattgcgacacgccggcgctgcggtatcaccgtgagacaccgatcggagctctccatgatccgccgcctctccgccgtcgctcttgtcgccgcatcgctgtccgcctgcggcggcggcgagggcgatgcgccggccgcccccaaggcgccgccgctgaccgatgcacagaaggccgtgcggctggcctctctccccgccccctacgaccaagccgatctggagaacggtcgacgcgcatttgcacgctgccggtcgtgccacaccctgaccgaaggcgggccgaacatgacgggcccgaacctgtggagcgtgttcggccgccaggccggctcgcacccacgctacaactactccaacgcgctcagcagcgccggcttcgtctgggacgccgagcgcctggaccattggctggagaacccgcgcaccttccttccgggcaacaagatgagcttccccggacttcccgctgcgacggaccggcgcgaccttgtggcctttttgaaggtggagacgggctatacgccagcgtcgacgccgcccgcctcctgatcctcactcggccggagccagaccttcaggacgcgagccctcctgggcctcccactgctcgatcttgcgggcggtgtattccggcgatcgggtgaagcgcgccagcaggccatagatcaccggcaccacgaacagcgtcagcagggtcgcgaagatcgctccagtgaagatcaccacgccgatggtctggcgactgcctgcccccgctccctgccacagcaccagcggcaaggccccgaaagccgtggcgatggaggtcatgatgatgggccgcagacgcagggtggacgactcgatgatcgcctcgctgatcgatcgcccctgatctcgcagctgattggcgaactccacgatcaggatgccgttcttggccgccaccccgatcaggataatcaggccgatctgcgaatagatgttgaggctcgagcccgccatcagcaggccgaacagacctccagccgccgccaggggcaccgtcagcatgatcaccgccggcgtgatccagctttcgaactgcgccgccagcaccaggaagacgagcagcaacgccaggccgaacgccgccgcgacggcgccgccggcctcctgctgatcgcgcgccgcgccgccccactgaagggtgatcccgctcgtctgctgcttggccgcctccgtctccaggaaggtgaccgcgtcggctatggtggtgccggggttcaggtcggcctgcaaggagatggaacgctgccgatccaggcgtcgccgctccggcgtgtccccggtcgtttcagtggcgaccacggccgatagcggcaccagctgtccgccgccggtcgcgacataaagcgcctccaggtcgccgacctcgcggcgattgttccgctccgtctgcaggatcacatcgtattcctgcccgcccttgatgtaggtcgtggcgcggcgagaaccgaacatggtctccagcgtccgtccgattgtctgcgacgacacgccaagcgccgccgccttttgcggatcaacatcgaccagcaggcgcggcgagttgggctcatagttcagacgcggccgggaaaagccggggttctcctgcgccgccgccagcaccggctgcagccaggcgtagatttggctgtactccgcgcccgtgacgatcatctcgaccgagttggagttgccgcccccgcgctgaaaggcgccgggagtggaggcgttgacctgggcgtccgtctggctccgcagcttgcggttcaattcctgagcgatctcgtcggccgatcggtcacgcgccgaccagtccgcaagggtcagtgttgcgttgccagagttgtagctgccaccgccaaagcccggcgcggacaccagataactgtcggcttcgcccgaggcgcgatagtcctcaaggatcggttccagccccagcatgatccgacgggtgtagtcgaagccggcgccttccggcccctgcacccgcacgctgacgcggccgcggtcctccggcggcaccaactcatccggcagggtgaagaacatggctgcggcgccgccgccgaccagcaggatcagaccggccacgccgaacacggccgcgcgacgcccaagcagggcggacaaggaggcgccgtaggagtttttcagcccgtccatcgcccggtcgacgcgacgcgcgacccagccgccgccatgcgccggcttcaagattttcgacgccagcatcggcgacagcgtcagcgccaggaatgccgagaaggccacggccgccgcgatcgccgccgccagctccacgaacaggcggccgatgtagcccggaaggaacagcagcggcgcaaacaccgacagcagcacgatcgtcgtcgccacgacggcgaagaacacctgccgggccccgcgctcggcggcgaccagcggcggctcaccgaggtccaggcggcgctggatgttctcgaccacaacgatggcgtcgtccaccaccaggccgatcgccagcaccagcgccaggagcgtcagcaggttcagggagaagccgagcggggccagcacgatgaaggtcgcaagcaggcagatcggcgcaacaatcgacgggatcagggcggcgcgcaggctgcccaggaagatgaagttcaccagcgccaccaaggccatggagatgccgatggtgatccagacctcgtcgatggcgtgcgaggtgaagaccgagttgtccgagccgatcgccagctcggttccgggcggaaggctgggctggatctcctccatcatcttcttgacgccgtcggagatggccaggtcgttggactgggcctgacgggtcaccgccagaccgatctgatcaacgccgttgcctcggaacaggcggcgatcctcctcgggcgcctcctcgatgcgggcgatgtcgccgagccgcgtcacataggtcggctgcccctggatgatggcggccgagccgctgcccgtgccggtcgccgtcgcgctcgacacggaggccgagccccgcgtgccgatcggcagctgggcgaagtcctgcggcagcgcatagttgcgggcgacacggaccgtatagtccttggacgtggactccagcgaaccggccggcagctccacgttctgggtggtgagcgccgtctcgacgtcggtgacggtcaggttgcgcgcggccaacgcggctggatccagccagatgcgcatggcgtagcgctgctcgccgtagatgttgacctgggccacgcccggcaccgtcgccagccggtcgacgaggttgcggtccgcatagtccgtcagctgcagcctgttcatgctggtcgagcgcaggaacaggatgataatcggctggctgtcggaatcggccttcgccacttccgggggatcggcctggtcggggaggttgccgatcacgcgcgacacgcggtcgcgtacgtcgttggccgcatcgtcgatgttgcggtccagcgagaactcaatgttgacgttggagcggccgtcgcggctggtggagttcagccgctccacgccctggatgccggcgatctgctgctcgatcggctcggtgatccggctttcgatcacctcggcggaggcgccggcgtagctggtgctgaccgacacgatgggaggatcgacgtccggcagctcacgcaccggcaggaagaagaaggccgcaagcccgatcacgcagagcacgatcgacgccacggccgcaaaaacggggcggcggaccgacagatcggagatcatcatcgcgtggcggctccgccttgcggtgcaggctgggctccaccctgcccgcggcctgaagccgtcgtcaccggcgcgccgggttggatgcggttgaggcccgagccgacgatccggtcaccggcttcaaggccggagatgatctcgacgaagccgttctcgaccgcccctgtctgaacctcgactcgctgggcggtcgagccgttctcaccacgtgcgatacggtacacgaaggcgccttcgccttgatactggaccgcagcctcgggcgcggccggctcctgccgctgtccctgctggacggcgacccgcatcagcatacctgggcggatacgcccgccggggtttgcgaactcggcgcgggcggtggcggcgcgcgtggtctcgttcacgcgcgtgtcgatcagggcgatccggccctgaaacgtctcgtcgccgtatgcgtcggccgtcgccgtgatcaccgcgccggggctcagctggctgaggtagcgctcaggcagcgggaaatcgacgcgcacagaagaggtgtcgtccagcgtcgcgatcaccgcgccgggattgatcaaggtgccggcggtgacggtgctgagccccagagtgccggcgaagggcgcgcggatcaggcgatcgccacgccgcgcctgcgccgccgacagctccgcctgcgcagtctccagcgccgtctccgcatcctcggccgtcacccgggcggcgatgcctcgctcggccagggtctgatagcgttcatactcgcgccgcgcctgggcgacggccgcgcgcgcctgaatgatggcggcgtcctcctcgcgcgcctgcagctccaccagcggtgcgccggcggccacgcgctgaccatcggtgaacaggacccgggtgatcagttccgtggtggaagaggtgatgttaacggaccgcaggcccctcgccacccccagcacccggatttgatcggagaactggcgcggcgcgaccaccgcttcggaaacctgttgcccccgcccggcgccgccggacgcgccgccaggtcctgcggctccgccttccccatcgcctccaaagccgatcttgacgacggcggcgacgaccatggcgaccagaacacaggcggcggcgatgagaaagaagtggcgtttgatcacgctggcggtctcgcgtcggtcagggcgcgaccgacttacccgttcagggcgccggcgcaacattaagtgtctgtaacgcgagcacgcccggtttccgtcgcgtcgcctagaaccttttccagaccgacagaacggggcctccagagaccggcgtttcgcgtccagcaacggtttgccgccagccggcctgcacgctccaggtccccagatgcctcacaacggatgtctccgccgacagccagcgcgatccgccgtccgccgcgccgccgtaggcctgcgccagcaccagccagcgctcgccgaagtgcgcgccggcggtgaagtcgacccgcgtctcgtccggcaggccgtcgcggatgcgccgggccgcctgcagttcgacaaagctccggtcgaagccgaagcgcggacggccgccccccccaaaagaccggccgatcgacgcccgggcctcccagtcgcgctcgccgacgccgagaggcgcataggccgcgttgcgcccatcgcccgcttcggcgaagccgccatagaggctaacggccgtgcgatcgtcgcgccacgcctgccaggtcacgccgatctcgatcggtccgcgcccatcataatcgacaaaggcgtcctcgcccgactgccactcgcccttgagctgcagcgtcaatcggtcggtcaggccgtattcggcgaacacgctcaaggcgtcgtcccgctgcggcgccggcaacggccgctcgtcgccggctggatcaaagccggagtcggcctccatcgcctcggccttgacgatcacctgcgctcgccccttgggctgcacccaggcgcccgccagcgcgggcgtggcggcgaggctcgcccccgccgccacgaccacccatgtcgccgccttcatgcgtcgtagcccggcgacctgcgatccagcatccgcagcgcgcccggccaggccagcgccgagatgaagccgatgccgcgcccctgctcccttgtttcggcctgggccgcgtccggcgccgtcagcaccccgtcggggccggcggagagagccgcgatctgctgggcgcaggcccgctccaagaagaacatgccgacccaggcctgcgccgccgtctcccccaccgccagcgtcccatggttgcgcagcagcatcagtggcttgtcgcccaaatccgccaccagacgctctcgctcctcatggttcagcgccagaccctcgtagccgtggtaggccacctgatgctgaagcaggcaggcgttctggccgagcggcagcagcccttccttctgggcggccaccccgacgccggcgaccgtgtgcaggtgcatcacgaacctggcgtcctcacgcgccgcatgcaccgcggagtggatcgtgaacccggccggattgatgaagctgtcggtctgatcgacgatgtttccatccagatcgaccttgaccagcgccgaggccgtcatctcctcgaaataccagccgtacggattgatcaggaagtggtgctcgggcccgggcacgcgcgcggagatgtgggtgaagatcatgtcgtcccacccgtgcagcgccaccagacggtagagcgcggcgaggtccacgcgtgcgcgccactcctccgctgaaaccctggcttgaactccggttgctccgtccgccatgccgtcttcccccctgcagccttcggcagcgtcgaacgccgcacgcccggcgtcaagcttaggttgctaagcgaaggttcgccgcgcaagctggcggtcgcggatcaacgaggattcggagaagcgccgtgtccagcgtcgtcatgcaagatcagcccgggcatgccggatcagacacgctttcgctgtccgagctggtggaactggcgcacagccgttcgccggaaaaccggcggcgactgctggacggggtgctgacgctgtgcagaacgcagccggacatctgcgcctccccggtcctcggcgacatcttcatgaccttggccaggcaggccgaacgggacatccggatcaccctgtcgcaggccctgggggacgccgactgggcgccgcctgcgctgatccacatcctcgccctcgacgacatcgagatcgcgcgtccggttatcgccgccagccccttgctggccgatgccgacctcctgcgcatcttggtcgaggccacgcttgagcaccagatcgaggtggcgcggcgcccgcgcctttccccggtcgtcgccgacgcaatcatcgaccaggcggaaccggcgccgctgacggcgctcgccggcaacacgtccgcgcgcctcaacgacgatgcaatgcgtcggctggtggagcattctcgccggatcgcggggctgcgctcgcccttgtctcgtcatccacgcctgaccgaagccctggcggcgcaactctacgaatgggtgggtcaggcgctgcgtgaggcgatcaacgaccgcttcaagatcgaggatgcgcggctggctcccgccatcgatcgtgccgtcgaacaggcgcgcggccgcagcggcccccttttcctggaggggaccaactcagccgccgacgccgaggctgaccgtcgcctggtcatgaagctgcaggccggcggtcaactccgtgcgggtctattggtacgagccctgcgggaggatcgcctcagcctgttcgaacacgtgctggccgcactgacgggctttcccttcagccagatccaggcggccttgcgcgcgccgggcccggagatgctgtttctcgcctgcaccgccgccggcgtcgacaaggcggtgttctcacccatgctgcttgaggtgcgcaggctgtgcggcggcctgccgggcggtcctgcggaatggcggccgcccgccgtcacgcgggaaggcgccgcccagctgtttcgaaaattggccacgacgcctaacggctctgcggtttgactcatgggccgtgctgaggcttgcctgcggccgtgaccactgatcttgatccacgtccgggaggcgcaagtccgcgcctggcctttgtcgccagcgaccgaccagaggcgcagtcggcccgccgtgagctgtccgcccgttatggcggcgtcaccgaggacgaggccgacgtcatcgtctcgctgggtggcgacggtcagatgctggagacgctccacgccaaccttcggcgcgggaccccggtgtttggcatgaaccgaggctcggtcggttttctgatgaacgactacgccgaagatggtcttctggagcggatcgcccaggccgaacggacggtgatccatccgttgcagatggacgcctggagcgaaacaggagcggtgcagaccggccttgccctgaacgaggtctcgctgctgcgccagacacgccaaagcgccaagctgcggatcagcatcgacggcaaggtgcgccttgaggaactgatctgcgacggctgcctggtcgccacgccggccgggtccaccgcctacaacctgtccgcccatgggccgatcatccctttggatgcacgcatcctggcgctgacgcccatcagcgcctttcggccgcgtcgctggcgcggcgcgcttctgtcccacggcgcccgggtgcggttcgaggtgcttgagccggacaagcgccctgtcagcgccacagcggacgggttcgaggtgcgaagggtcgcccgcgtcgacgtgttcgagcgccgagacctgcagctgaccatgctgttcgacgcgggccgttctttcgacgagcgggtgctggcggagcagttcgccggatagcggtcaccctatgttaaggccgcggcggcatgctcggcggaaatcgtctgggaagtcgtccatgagcaatccggcccaggtcatccggccgcccaacaccctgcgcgccaaggtcggcggcggcttcggcatcaacgccgacgccatcgccatcgccatcgccaaggccgaagaagcgctgaaggcgatgtccacccagttcgcccagtggctgcaagacgagatcgccaagctggacaaggcgcaggccgacatccgcagcctcggctatacgcccgagacggccgaggctctctactttcgcgcccatgaccttaaagggctcggcaccacctatgagtatccgctggtgacgcggatcgccggatcgctgtgccggatgctcgacgaccccgcgcgtcgcatggacgctcccttgatcatcatcgacgcccacgtcgatgcgattcgagcggtggtccgcgacggcatcaagaccgacgaccatccgaccggccgcgccctggcggagacgctcgaagcgcgcgtcgccgagcacctggcgtaaagctttcaaacccggacaggcccgccgcaccgccggccattatttctgaattcccgatcaggcggcggcgcgatgttgcggccgagcgggcccatccagccgctccatcagataggccaggtcgtcacgagacgtggtcggccgctgcgtcaggaatcgctccagcatcctgctgcggaatacgtcgccactggtgtcagcgccctcggcttgcaaggcgcgccaggtgtccaccccggcccggaaggcttggaacaggcgcggcggcagtcccgcgcggtcatagatcgccttcagccccagcggtccggcgtcgtgcaccatctgccaggcgcgcgcgtgcggcgtgttcgccagttcggccagcccatgctccagcaacgccatctgacctcgcgccaacccacgcagcagcagcgaagcggtcagcgctcgccgcgcgttcagttgggtcacgaacgcgccgatgtcggcgctggccgccgcctggtccaccaggtcgacggtcgcccgctcgcgtgcgaactgcgacaggcggatggccgtctcggccgtgacggcgtggcgcgtgaccaagtgttcgcgcacagcgtcgctggcgcaggcgatcagccgttcggtgatctccagcggcaacgcctggcgataggccacggcggccacgacttccggcgcgccgccgaaccgatcgacgatgacgcccagcgaccgctcggacaggtcggcgttgtcgttcgcggccaaggttcgcacggcggtctccccgccctcggccgccaggacctcggccacgtcgcgcgacacgcgaggacgcgcggccaccgccgtctgacgcgcggccgagccggcccgcacgatctcgatcaggtcgtcgtcgccgaaggccggcgaaaagccgatcagcggcaaggcgatcgagtcgacatccgccgccagtctccgcgccacgtcgttgggaatgaggtccgagctcttcagcgtcacggccatggcgcgcctgacgagctcagccgcgtcctgcgccagaacacgcagtatcttctgcgccgccgcccgatctgtcggatcaagcgaaatccgctccatgcttcggcacagcttatgcgcggcctctgcgcgctcgtcctcgtcctcggccttgaccagccggcggatgtcgacatcggtcaggcgggcgcgaaaggcggtcatcgggggctcgcagcgggatcggatggtcggtcgatcatccatccctgttgcttaacgcgcggtttaccatgcgttgaagactacgccgcatcctctgcgcgcggcgtgaacgcctggccaaagccgccgccgctcgatccatcctgccccagaagaagagccagcagcccctgatcctgtcgaatccgctcaagccgggcggccagcatcatgtcgggattcgatggtttcgaagcaggaacatcggttgggccgcttcccgccgcgggcgcgccgccgccggcggagcgctgcagattggcgtggacctccgcaacggtggccgagcggccgtcccgatagaagatcgaacgattggcggacgccgcctcgggaaacagagccgccgcgctggcgcccggccgcgtctgcatggcctccatcagcttggcggcgccggcgggccccaggaagtgggccgcgtaaagatcgccggcgcccggctcctgacccgtgcggccacgcagataggctgcgttggacgccgtcagctcggccgccatcgaagaggccgcctgggggtcgaagcgcaggtccagcactacgttacgcgcggacccctccacccgccagcgcccgtccccgcccctgtggatcaggtccgcatattggccgtagccatggctcggcccgtgctgcttgaccgtcgccagccaggtctgctcgatgaactggaacagccccgccgccgaagacgtgcgcgccttggcggccgggttcatggcgctctctcgccgggccgtcttcatcaggaagtcgaagtccacgccggtcgcgcgcgaggcgcgtcggatcgccgcctccactccgtttccgcctggaatcgcaccaacagccatagcgcgttaaccatcgacgaacgtggttaaccaaacgctaatatgcattgatcgagcggttcaaccgacagctggatgaaaccgtcctggatccagtcgccgaacgtccgcgtcttccggcttcccgctcacgccgtccgcaatgatccggcccgccagcggccccagcagccaaccattgcggcgcggggccagcgaaagccacaggtcctcgccgtccggcgcgcgaccgatgatcggcagaccgtcggggctggcgccgcgcacgccgaccttccattccacgggcaaatcgaacaggtcgcgccccaataatgcggaggcggcgctcgtcagccgttcgccgtcggcggcgtcaggctccagatcacgccgcccgacatccatggtggctccgaccaccgcacctgtgattccgggcgcgacatagacgccccgcccgcgaacggcgtgatccgccaggcgcgtcccgatccgtccgatctgtccccggatcggctggatcgcgccgatcaggcgggcggcggcctccggcgttcctgctggcggcgacgccgcgcctgtcgccagcacgacgcccttcgccgccgcatcacggccctgacaggtgacagtccaccgcccgtgctcccgccgcatcgtctcgacctcgccggcgacgatccgcacccgtccgcgcatcgcttgcagggcctggccgggatcgacctggaggtcctggatcgccgtcagcacgttttggtcccgccgcgcgtcgaagtcgagcctgcgcatgcggtgctcgatgtcgtcgatgccaggcccacgccactcggcgcccggcgtcagcagggtgacgccagtggcgtccgcgaagtcgggccagaggtcgcgggcgcgtcgcagcaaggccgcatggccggcgtcgacgtcttcgagcgccgcctccatggccggcgcgatcattccggcggccaccgaagaggcgttctccccgcccggatcgatcaccatcaccgaacgcccgcgccgttgaagctccagcgccgcgcagagaccaaacacgccggcgccgatcaccacgatgtcgttgtcggaagtcacgccgggtccatccaccctgccgcgccgcgtggcaagcccttccccacactcggcggagaccgctaagacaagagcgtgcaaagcctcgaaatcctgtcccgaacgcctgacggcgccgtctcctcgcccgccgcgcgccgcaacgccgagccgatcctgcgcgtgctgaaggcgcacctttcggcccacggacgggttctggagatcgcttccgggtccggcgagcatgccgcgaggttcgcctcggccctgcctggcctcctgtggacccccagcgacgtcagcgtcgaggcccgcgacagcatcgatcgctggagagccgccagcggcgcccccaacctcgcggcggcgctggcgctcgactgcctgcagcctgacgcctggcccgacgccgctttcgatgcggtcttctgcgccaacatgatccacatcagcccggtcgaagcgaccgacggtctgatgagactggctgggggcgtcctgccccgccccggggggctgttggtcctgtatgggccctttctggagggtgaccagccgctcgccccctcgaacgccgcgttcgacgcaagcctgagggcgcgcgatcccgcctggggtctgcgggatcgggacgccgtgatcgcgacggctcgcgagcatggcctcgccttcaccctgcgcatcgccatgcccgccaacaacctcgtgctccttttcaggcgcgcctgatgagctttgtccgcaccttcgacggcgccgagccgatgcgcctcaacaagtggctgggccagaccggcgtctgttctcgccgggaagccgaagggctgatcgccgacggccttgtgtcgatcgacggcgagacggtgcgcgatcccggccgcaagatcgagcctggccagacgctgactctcgaccagcgcgcccaggcgaccctggcggccggcgtgaccatcgtgatgaacaagccggtcggctatgtctcgggtcagccggagccgggcaaggttccggccgtgcgccttctgaccgccgccaaccttgtcggagagggacaaacgcccgcccgagacgcgtccctgccgccgattggtcgactggacgaggactctcgcggcctcttgctgctgtcgtcggacggggtggtggccaaggcggtgatcggtccgcagtccgagctggacaaggagtatctcgtccgcgtcgacggccgcgtgaccgaggccgccctgtcgcggctgcggcacgggctcgaactggacggccgccggctgaagcccgcccgcgtcacccagatcgaaccgcaacggctccgcttcatcttgacggagggacgcaatcgccagatccgccgcatgtgcgaactggtcgggctggaggtgatcgatcttcagcgtatccgtatcgggccgctgaagctggacgatctgcgtgaaggtcgctggcgccatcttacgccaagcgagcgcgaatcgctggtcaggcgctgaccgacacgcctgcgaggcccgccagccgggtcagttccgcgacatggccggcgaaggccgctctcccgttcgccgtcaggccgagccaggtgcgttgtcgcccggcgaaggcggccttgcgcaccttgacgtatcccgcctcctccaactgcttgacgtgcttggacaggacggagtccgacacgccgatgccgtcgcgaaccacgccgaactccacctcgtcggcggcggacagcatggcgcagatctgcagccgccccggcgcgtggatcacgccgtcgaagaccggcgcgctcaagaccgcgcctccccttccgcgaggtagagccgcatccacagacgcgacagcgccagggccgccacaaaggccgccgcgccgagcgccagcgcccaatgggcctgatccgttcggccgagataaagcgccccgatcatcatcgcgcccagcagcaggccgaccagaatggcggcccagcgcgcacgcctgggcgacaggccggtgacgctgacgccgttcttttcggaccaccgcttccacagcagcgccaggcaaaccgccccgccgccggacgccagcacattgaacggtatcggcagggcctgacccgccaccatcaccgccgctatggcggagtagctgagatcgtaacgccaggagccccgcgtcatgcgccgccggacgacgtcctgcgagcgacgaatgtccgccaacgcctgatcatggatgttccgctcgtccgacatgaccgtctcctcaccaacttcgcagagaagcgatgaccgagactttccattccgtcaagtcgtgcttttcctgcttggaaagtttagctcagcgcctcaaaccacctctgcagcaggatcgcctcggcgcggatccgacccgtgcgctccgccgcctccgcgtccacaccccattggccttcctgaaacgcttcttccagccgtgacagctcgaacgccatctccgccgccagggcgccgcgctgcagcgccagcgcgagcacggccgatcccagcagcggcgtcgccgtcgcgagaccggtcagggcgaagtcgtccagcgccagggccagcgccctgacccgcgcgacggcctcaggcgactgggccacatggacgatgccggatacggcgaccagccggacgcccagctcgcgttcggcccagtcgcgccaaggcgtccaggcgtcgatctgccgccgctcaagcgccccctcgcccagatagcagatggcgtccgagccggcgtaggcggcgatctcgtccgctaccgcctcgcgcgcctgcccgatccggtcgatggccgtagaagccagccgcgtcgccggcatggtcgccggttccatgaactcgccctgggccgcccattcgtcggcgaccagccgcgcggcggcctcggccggcaggatcatcggcttcttggccggggtcttgggcgtgcggccgtccagtcgcaccgcccagccgccatcgaccggcgccgcgtcggccgtggtccagaagcgccggatgcgctcctcgacctcgctgaaacccttcctcgccgcgagaacgggatcaagattggggatgtggctcatctttgcctccgcacgcctccgaacgagtccgcctccgcctcgtcctcggaaaagccgaagtgggcgaagcccgccgtcatttcgggaccgagcggcgcctctacaaccagcgttccgcccgcggggtgatccagctcgatcctgcgggcgtgcagttgcagccgtagtgagccgctcagttcgacggaggcttcggtcttgtacttgggatcgcccaggatcggatggcccatggccagcatgtgcgcccgcagctggtgcgtccggccggtgaagggcctcagcgccatccaggcggcgcggtgggcggcgcgtgacacggtgacgaacgccgtctcggccggctcggctcccgggtccttgggctcggctggccgcatcatttcgaagtcgttgatgccggatttcttcagcggcaggttgatctggcctgcggccggcttggggttgcccatcaccacggcccagtaggtcttcctggcctgccgccgggcgaaggcgcccgccagccgcttggcggcctccggtcccttgccgagcagcagcacgcccgaggtgtcgcggtccagccggtgcaccaggcgcggccgctccatcccctcgccccaggcggacagcagccggtcgacgtgcctggtcgtcttggccccgccctgcaccgccaggccgtgaggcttgttcagggcgatcaccaaatcatcctcatagatgaccagtgaacgcgcgtagtcgatgtcgcgctggctcagcaggtgcggatcgcccggctggcgctcgaccacctccggcagcggcggcacgcgcacggcggccccggcggtcagccggccttccggcttgatgcgcgcgccgtccaccctgatttggccggaccgcgccatcttctgaacctggatgttggacagatgcggccagcgcctgcggaaccagcggtccagccggatgccgtcctcggcttcggccacgtagagtgtctggacctcacggctcatgcgaacacccgccgcgcgatgaacaggccgacgaacagggcgccgatcgacagcatcaccgatgcgacgacatagccggcggccagcgccaactcgcgcctttcgatcagcagggccgtctcgagcgagaacgccgaaaaggtggtgaagccgccgagaacgcccacggccgcgaacaatcggatcgcttccgcctgcgcgcctcccctgagcgcaagccagcccgcgagcagccccatcagcaacccgccgatcaggttgaccgcaaaggtcccaaggggccaggcggcctgcggcgccagccgcccggccgccaaccccaggccgtagcgcgccgtcgcgcccagaccgccgcccaaggcgacaagcagaaaacgagtcatggtgcgccgctatacagccggcgacggacgaaagcgaagcgcaacccttcagggcgttggccgggcgtttgggacgaccccgctctccgcccggacgcgatcagcgcctcaggctgctctgcactgagcgcgcgtcatagacctgtggacgatcgggacgagcgccgcgcccggtgatgatctccagcgtggtggaggtcggcgacgggccgctgaagttcaggccgaggcccacgcctactcccgatgacgaccagccgccataccgccccgttcccgcgcccaccgacacgctgggacgcacgccacccgctccgtccggccggccgtcgatccagcgctgcgtcacctcgaaccagtcgtagccgttctcggtagtcacctcggccgcgcgcagaagggcgtagtccgccacggggcccggcgcgccgacgccattgtaagtcacgcgaaatcgatcggactcgatccgctgctcgatgaagccctgaccgttcgaaccctgctgaggtccgtagggggcgagggacgcgcaggcggacagcgccaaggcggaggcggcgagggttaggacggcgatgcgcttcacgacttaactccttgagcttcgacggaatagcgccgctgcgggcggcttggttccttaaagaaggcccatgccgtgacgcaggtcggcgaagtcggcgggggacggcgcctcgaccgtggtcgagcccccctcgggatgcgggaacgtcagcctggccgcatgcagcatcaggcgtggcgccgcccggcccgcgactgtcagcgcgccgccataacgcacgtcgccgatcagcggccgtccgatgtgcgccatgtgcacccgcagctggtgcatgcgcccggtcagcggctcgagctcgaccaacgccccgtcctcgctctccgccagggtgcgatagcggctctgcgagccctgcgcgcccggcgcatcaaaggcgaccacccgcatatagctctcgcggccgatctcctgccgggccagaggcgcgtcgatcgttccgcagcgaggctccggcgccgccgcccccggggccagataggtctccctgaaccgccgcatctgcagcgccttgccgaggaaacccgccgccggcttggtcttggccgccaggatcacgccggaggtgtcgcggtccagccgatgcaccaggtcgggccgcttcccgttcgaccgggcaaaggcccacagcaggtcgtcgagcgtgtgcgccttgatccgtccgccctggctgctcagacccgccggcttgttgaaggcgatgacatgggcgtcctcgtggatcacccaggatcgcacggcggcgatctcttcatcggacaaggcgacgggcggggtgaaagtcatcgcggctcttgaaccggcgtcgcccgagcggtcaagcctcgccctccggcgcgtcctgcatgcgggcgcgcatctccgcccagcgctcaagccgcgccttgaccttctcctcgtggccctcgcccttgggcttgtagaagacgcggcgctccatctcgtctgggaagaagtcggcgccggagaagccctccggcgtgtccggatcgtaccggtagccctttccgtatcccagcgaccgcatcagcttggtgggcgcgttgcggatatgggcgggcggcatcagcgacccggtctcgcgcgccgccttctgcgcggccttgtaggcctcatagaccccgacggacttgggcgcggtggccagatggaccacggcctgggccagcgccagtccgccctcgggactccccaggaagtcgtatgtgtccttggcggcgttggcgatcaggatggacagggggtcggcttcgccgatgtcctccaccgccatgcgcacgatgcgacgcgccagatacagcggatcctcgcccccgttcagcatccgcgccagccaatagagcgccgcgtccggatcgctgcctcgcaccgatttatgcagcgctgatatgaggttgtagtgttcttctctggacttgtcgtaagcgggagcgcgccgttgcagcacccccgccagaccctgcacgtccagcgtctcgcccgccggcaggtcgaacagcacctccgacatcgtgagcaggtagcgcccgtcgccgtccgccagcgccagcagcgcctgtcgcgcttcggcgctcagcggcagcacccgctccatgtgcgcctcggcgcgcgccagcagttggtccaaagcgtcatcattcaagcgcttgagcacgaacacctgagatcgtgacagaagggcgccgttcagctcgaagctggggttctcggtcgttgcgccgacaagcgtcaccactccttgctcgacaaagggcaggaaaccatcctgctgggcgcggttgaagcgatgaatctcgtccacgaacaacagggtggactggcccgccgcgcggcggccccgcgcctgctcgaacgccttcttcagatccgcgacgcctgagaagactgcgctgatcgcctggtattcatagccggcggccctggccagcaggcgcgcgatggtggtctttccggtgccgggcggcccccacaggatcatggagccgagccgtcccgcctccaccatccgccggatcggaccgccctcgcccagcaggtgattctgccccaccacctgatccagcgcggtcggccgcagccgatccgccagcggcgcgtcgggcggatggacgccggaggcttcgaacaggtcgctcatgccggcagatgtaggcgctccgccccgaccttgagaagatcagatgcggccggtcagcagacggccgccgcgattgatgacgatctcggatcccggctgcgcccgctgcaggtcgccgacggcggtggcggcgcgtccgttgatcgtctggatcacgtcgccgcgccggatgccgacccgcgccgcatagcctcggcccgagacgcccgtcacgatcacgccgcgcgcgaacggatcgccgcccagcctgtcggcgagggccgggttcagcgccagaacctgcgcgccggaaaaggcgccctgctccaccaccgtggcgcggtcggtgtcggcgtcgcccggcaggacctgcacccgcgcgcgcagcgtctggggccggccgtcgcggaggatggcgatctcgacctcatcgttcggattgcgcgtgccgacgcggtagttcagcccaccttgatcgttgacctcctgcccatcgaccgcggtgaccacgtccccttcccgcaggccggcgcgtgcggcggggccgttggcgtagagcccggtcaccaccacgccccgcggccgccccagccccagactgcgcgcgatgtcgccggagacggtgtcgcccttcacgcccagccagggccgcaccacgctctcggcgccgccgacggccgagtcgaccacccgcttcaccatcgccgccggcacggcgaagccgacgccggctgaggagcccgagcgcgaaaagatcgccgtgttgatgccgatcaggtcgccgtccatgtcgaccagcgctccgcccgagttgccggggttgatcgcagcgtccgtctggatgaacgagccggagtcggaaatgccggtctcggtgcggttcagggccgagatgatgccgttggtgaccgtctggcccacgccgaacggattgccgatggcgaggaccaggtcgccgacctgctgctgctcgctgtcgtcgatcggcagggtcggcaggcgctcgccgacgttctcgagcctcagcaccgcgatgtcggagcgcgcgtccgccagcaccaccgtggcggggaactcgcgccggtcgttcagcacgaccttgatcgcctgggcgccctcgatgacgtggttgttggtcactacgatgccgtcagtgcggacgatcacgcccgagcctacggattccgcgacccgggcctgagggatgccgccgccgaagaactggaagaagggatcggcctgaacacgctgcacggtgcgggccgagatgttgaccaccgccggcgccgccgtgcgcaccacgggcgcgaagctcgacttcatcgcgccggcgctttcgggcgtcacccgattgctctcggcgaacacgccgtcctgcgccttggagctgttcggattgccgcaggccgacagcatcagggccgaggccagcaggatggatcgagtcttcatcgtcgcccgcgaaaggaggatcatcaccgctgcatttctgccgggctttcaggccggatcaaggcgcgggttcggccttgaaacgacccgcgccccctgctcgttccggcgagcggtcagcggccggtgaaccggggcttccgcttgtccacgaaggcggccatgccctccttctgatcctcgaaggcgaacagggagtggaacaggcgccgttcgaaccgaacgccctccgccagcgtcgtctccagcgcgacgttgaccatttccttgttcatcatcaccgccagcgggctctgccccgcgatcttcgccgcggcggcgcaggcctcgtccagcagcgcgtccggggccacgacacggctgaccaatccagcgcgttccgcctccgccgcatcgatcatccgcccggtcaggatcatgtccatggccttggacttgccgaccagccgcgtcagccgctgcgacccgccgatgccgggcgccacgcccaggttgatttccggctggccgaacttggcggtttcggaggcgatgatgaagtcgcacagcatcgccagctcgcacccgccgcccagcgcatagcccgacaccgccgcgatgaccggcttgcggaagcgggtgatccggtcatgcccgagggcgaagaagttgcccttgaacatgtcggcgtaggactggtccgccatctccttgatgtcggcgccggccgcgaacgccttggccgatccggtaagcaccaggcaccggaccgtgtcgtccgtttcgacgctgtcgagaaaggccgccagctcgccgaacagggtggagttcagtgcattcagcgcctcgggccggttcagggtgacgaccgcatagccctcgtcgcggcgttcgatcagcagggtccaataggtgtcgctcacgccgaagtctccagatcagccagtcggccgcgcagcagctgcagcacggccgagaaatcacgcccgccgtggcccaggccggcgaacatcgcataaagggcctccgactgggcgcccagcggcgtggcggcgttggccctagccgccgcctcctgcgccagcttcaggtccttcagcatcatgttggaggcgaagccgccctgatagtcgcggttcgacggcgcggtcggcaccgggcccggccagggatagtagctggtcacgctccagcactggcccgacgatttcgacgcgatctcgaagaagcgttcgggatccagccccaacttctcggccagggcgacggcctcgcaggtccccagcatggagatgcccagcagcatgttgttgcagatcttggccgcctgacccgcgccgtggtcgccggcgcggatggtgatgcggctcatcggctccagcgccgcctcgacgcgggcgaagtcgctgtcgtcacagccgaccatgaaggccagtgtgcccgcatccgccgccgccgtcccgccggacacgggagcgtccgcaaaggcgtagcctgcgtccttggccagggcggccacctggcgcgccgtctccacgtctatggtggagcagtcgagcagcagcgccgacgtcggcgccgcgccgatgatctgctctgcgtagacctggcgcacgtgcgggccggcgggaagcatggtgatgaccacctccgcgtcgcgcaccgcctcggccaccgaggacgcacgcgtgcagccggcgcccgccgcccgctccagcgcggcctccgacagatcaaaggccgagacctgatggccggccttggcctggttggcggccatgccgccgcccatgttgcccaggccgataaaggcgatgcgggtcatgcggctgctctccctttcttttgctttttcggtgcttagctcggcttgcgaaagcgatagacgaactggtcagtccggccgcggatcgcctcgtcgaagacgttcagcgtgcggtcgtccgctggattggccacggccgtgctttcgccgtcgaagacgaagccggcggcctcgatctcgcggcgcagctgcgcgccctcgatccggtgcaggctctggacctggctgatccctgtgcccgccgcgcccgcgtggtcgatgacgacgaacagaccgcccggcttcagggcgtcgaacaccgcccggttcatccgcgccacatccacgccgaagcccgggatgtggaagtcgtgatactcctggctcatgaagacgaggtccagcggctgctcgaaccgcatggcgtccaggtcgccgttcacccggacgacgttcggataggccgcaaccagagcgtcagccggcgcattctcgcgcgccgccgtccggttgggcacaaaggcgtagaccttgccgccggcgcccgccacctcggcgaacaggcgggtgaagtagcccgcgcccggtcggatgtcggctatgcggtcgcccgcctgcacctgagcgaaagccagcatctccatcggatgccgcagcggatcgcgcgcgacctcttcggccggccgccgggtgtcggcgacggcggcggcataggcggcggtcatggccgaggtcggttcggtcatgcttgacgtggcgcagctcgaaagcacggcggcgcaggcggcggcgagaagaagcggcttcagcatcggtgtccctccagacggttcggcctagctacgcgttgaaccggcgtcggacgcaagcggcgtccagacctcggtctccggcagcggcgcgaacagtgcgtccaagtcggcgtcggacacgtcctcgatccggccgggcgaccacctgggggcgttgtccttgtcgacgatgacggcccggacgccttcctggaaatcgtgcgtgcgcaccacgcggccgcccagcgcatattccatcgccatgttgtcggcgaaggtcgcaagcgtcgcgcccgtgcgaagctggcgcagcgtgatcttcagcgactgcggcgacttggtccggagcacggcgagctgcgccgacgcccactcggacccgtccgcctcaagcgcctcgaagatcgcctccaccgtgtcgaaggcgaacagccggtcgatcgtctcgcggtgggcggccaccggcgacggcccggcctgcgttgcgtgcgcatcggcgatcgcccgtggatcgcctggcgctgcggccaggtcacccttgaaaccggccaagccttccgccgtcatgaagtgggtgtgaatccccagcgcgaccgtatccaccgccttcagccgcgcccccgtcagcgccagccacacgccggtctggcccggcaggcgcggcaggaaccatccgccgcccacgtcgggaaacaggccgatgccggtttcgggcatggcgtaggtggtccgctcggtcgcgatccggacgtccgcggactccgagacgccgacccctccgcccatgacgatgccgtccacgatcgccgtgatcggcttcgggtattcgaacagcaggtggttcagccggtactcggccaggaagaaggtcttggcctccgacgcatcccccgctccgctctcggcgatcatgcggatgtcgccgcccgcgcagaagccgcgctcgccggagtggtcgatgagtatggaggagacggagggatcggaacgccacgcaagcagcgcctccgtcatgatctcgcacatcgaccggttcagcgcatggatcgccttgggtcggttcagggtgatgcggccgagcccgttctcgacccgcgtcaggacttccgcttcgctcatcccttggccagctcccgcgccacgatcatgcgcatgacctcgttggtgccttccagaatgcggtggacgcgcagatcgcgcacgatgcgctccagcggataatccttgaggtagccgtaaccgccgtgcaactgcagcgcctcgtcggcgatctggaaacaggcgtcggtggccatgcgcttggccatggcgcaccacttggtcttctccggatgatcgttgtcgatcgcccaggcaccccgcagcaccatcagccgcgccgcctccaggtccgtcgccatgtcggccaggcggaactgcagcgcctggaactcgccgatcggccggccgaactgtttgcgcgtggcgacataggcctgcgccgtctccatcgccagccgcgcaccgcccagcgagcaggcggcgatgttcaaccgtccgccgtccagtccactcatggcgtagcggaagccggcgccctcctcgcccaccagattgccgaccggcacgcggcagtcgtcgaactggacaatggcggtgggctgggcgttccagcccatcttcttttcgttggcgccgaaggacaggccgggcgtgtccttttcgaccaccacggcgctgatccccttggggccctcgccgcccgtgcgcaccatgacgacatagacgtccgatacgcccgcgcccgagatgaaggccttggagccgttcagcacatagtggtcgccgtcgcggaccgccgtggtccgcagcgccgccgcatccgacccggagccgggctcggtcaggcagtaactggcgatcttgtccatggtgaccaaggacggcacgagccgcgtccgcagctcttccgcgccgaagcggtcgatcacccaggtgaccatgttgtggatcgacagaaacgccgccgtagtcacgtcgccgcgcgacagctcctcgaagatcagagccgcctcgactcggcccagcgacatgccgccatgctcttcggcggcgtagatgccgcaaaagcccatctcggcagcgcgccgcatgacgtcgacgggaaagtgcttgtcctcgtcccagcgggccgagttcggcgccaactcagcgtcggaaaaggcgcgcgccgcctcctggatcgcgcgctgatcttcggaaagggcgaagtccatggccgccctcctcagcgcatcgtcggaatgacgaaggagctgtcggcgtgctccagcgcgctgtcgggccagcgggcggtgacggtcttggtcttggtccagaagcggacgccctccatgccgtgctggttgatgtcgccaaaggccgagcgcttccacccgccaaaggtgtgataggcgaccggcaccggaatcggcacgttgatgcccaccatgccgacgttgacgcgggcggcgaagtcgcgggccgcgcggccgttctgggtgaagatggccacgccgttgccgtactggtgcttggaaggcagcgatagcgcctcctcgaacgactgggcgcgcacgatctgcagcaccgggccgaagatctcctcctgatagctgctcatgtccggcgtgacgcggtcgaacagcgaggggccgacgaagtagccgttctcatgcccctgaaggctgaagttgcggccatcgaccaccagttcggcgccttcctcgacgcccttggcgatccagccttcgacgcgggccttgtgctgggcggtgacgacggggccgtagtgcgcctggtcgtcggtcgagacgccgacgcgcagcgtgtcgatctcggcgaccatccgttcacggaggatgtcggcggtcctgtcgccgaccggcaccaccaccggcagggccatgcagcgctcgccggccgaaccaaaggcggcccccgccaggtccttgaccacctgatccatgtcggcgtcgggcaggacgatgccgtggttcttggcgccgcccatggcctgcacgcgcttatggttggccgcgcccgtctgatagacgtagtgggcgatgtcggacgagccgacgaagctgacggcgtgcaccagcggatgggtcaggatggcgcccacggccgtcttgtcgccgtgcaccacgttcagcccgccgttgggcgcgcccgcctccagcatcagttcggccaggcggaccggcacggacggatcgcgctccgacggcttcagcacgaatgtgttgccgaccgcgacggccacgccgaacatccacatcgggatcatggcgggaaagttgaacggggtgatgccggcgaccacgcccagcggctggcgcatggagtagacgtcgatgccgggaccggcgccctgcgtatattcgcccttcagcgcgtgggggatgccgcaggcgaattcgatcacctccagcccccgctggatgtcgcccttcgagtccgcgatgaccttaccgtgctcgcccgacagcaactcggccagctcgttcatgttcgcctcgaccaggcgcttgaactcgaacatgacccgcgcgcggcgctgcggattggtggaggcccaaccttcaaaggcgttctgcgccgcctggaccgcacgatcgacttcgccggcggtcgccagttgcacgcgggcctgaacctcgccgctgttcggatcgaacacgtccgagaaccgaccgcttgagccgtcaaaggccgagccgtcgatgaagtggcggatgtctcgcatgcaggcgtttccttgatcccggttctcggtgattgcggcgaccatagcggcatccgccgccctcgcccatttcaaagacggccccacaatgcgccaaacccgcaagtttcggtcgcgcatgggggctttcaaggtcagccgccttcctggcgggtttatcccggcgcccgctccatcagcaggccctcgcggcgcgccttgcggccgtagacctgctcgaacaggggcgaggccatcaaggtggtcacgatggccatcagcaccaggatggagaagagcgccgggctgatgatgccccgctgaagcccgatgttgatgatgatcagctccatcaggcctcgcgcgttcatgagcgcgccgatgcccatggcggtccggttgtcctgacccgtcagacgggcggccgcccagcaggccccgcccttggcgaggatggagccgacgagaatcagcgcggtcacgccgagcagtccgatgttgtcgaccatggtcagctgggtgttcaggcccgagaaggtgaagaacatcggcagcagcaccagcacggcgaagggctccagttgagcgcggacctgctgggtcagcaggccgcgcggcatggcgacgcccaggatgaagccgccgaacacggcgtgaatgccgacggcgtccatgacccaggcgcaaagcatgaacaggatcaggatgacgccgaggacgcccgcgctgaccttgccttcgcgttcgacccggcgccccagcggcgccagcagccggggtccgaccgtcagcatgaacgccgcgaacgcagccccgccgcagatcgccttgaccgccaccatggcgccgcccccgaagctggccaggacgatcgccagcacgcaccaggcgccggcgtcgtcgatggcgcccgccgacagggacagcgagcccatcggcgtgccgctcagtccccgctcatggatgatccgcgccagcatgggaaaggcggtgatggaaatggccgcgcccatgaacagcatggcctgccaggtgacgatcccctcaccaaacaggcccatatcgatcagccatggcgtcagcgcgacagccaccagaaaaggggcggccattccggccaccgagaccgccgcggcgctgctcgcggcggttctgaaatgatcacgctcaaaaccgagccccaccaggaacatgtacagcccgacgccgagctgggcgccgacgaacagcacagacctcgactcggccggaaacagcgcggcctgaagttcgggcgccatcaggccgaacagcgacggccccaggatgaccccggcgatcatctctcccacgacctgcggctggtcgagccacgccttggccgcccagccgaccacgcggcaagcggcgatgatcaccgccatctgcaggaaaaaagcgacgctgagttcggcgttcgtcatgcccccgcctgcgacgcattggcgttctttgggacgcttaccttatcgacaaggttggccgaggcgatcggagaagacaagccgcctcggcggtcgaacgagggcgatgcggtccacccgccgggctagagaccgctccctggctgcggatcatgcctgcgtggggccgccgcgcccagcatcatcagcccgccggccgccagcgacaacagcgccagcagcagaagaagcggcccgaaccgcccttcggccgcgagcagataggtcagcgccggtccgagcagcgccggcagggtgttggtcaggttcagcagcccgagatcgcgtcccctgtgcgccgacgacagcagcaggcgcatggcgtaggccgactggatcgccagaaatgcagccaggcctatggcgaaaagcgcgtatccggcgaccgccgtcggccactgcggccacagccccatgacggccagacccgtcgcgcaggcgcacgccagcgccgccagactggcccgcgcgccgcggccacgccggtcgatcagccggccgatcgccacggaaaccggggcgctcaccaaggtcacgacgccggtgatccaggccacacgcccggccaaggactcgcccgaggccgcaccgccgggctccgcaacgctttggaagtagaacaggataaaggcgaacagcacattgcccgccacctgcaccagaaggcgcgagagccccaccacacccaatcgccagaaggcgtgaggtccggcttgcgccggcgccgccacgatctcggcggcggccggccggcgtgtggccagcagaaagggcgccgcaagagccgtgaccaaggaaagcgtgcagaacacccgcgccgcccagctccagtccggcgcccaggtgaccatcaccgccgccaccgtgcccagaggataggctgcgccatagacgccgccgagcacgcccttctggtcgtcacccgtttcgtccgccgcgatggcgatcagcggcgagagaaaggtgttcaacgccgcctggaacaaaaccaccgccgccaccagttcgcccgggctggaagcgagatgcagggcgacgtaggacaaggccgtgcccgacaaacccgctgcggcgaccgcgcgcctgccgaacggccgtccggcccaccggtcgctgatcatgccggccaggatgttgctgacgctggccgccaaggcgcccgcgatggaggccaggctcagcagggccaccttgccgtcggcctccgcgatgctttcgaccttcagcggcaacagcagcgtcagcagcggcacataggcgcaaaccgcgccgccataggccaggccgtacagcagcaggtaaccgtgtcgattgttgcggatcatgagggtggacgcgcgatcgaccttctcctggcccaggcgaagggtggctgaggcggctggccgaagcgcacgtgcgggccattgttcatgacgcgtgagacggtctgcgacgggaagtcggctttctcggtgatgaggcggatcatgacctgagcttcatgtcacactcttggcgggggcgacggcgcggcgcaatgggcggtgaaagaggagtgcgaaggcagctcctgcgccgcgtgatccaacggcggcgctgtaagtgctccaccattccagggtggtgacttggtcgaccgcccctcggctccggctgcggccgcgacttggatccttggaaaactctgtagggttccccgtagctcccgtggtatcgacccctaaacactgaggcaggcccgcgtgatcgacaccatctcgaccggaaatccgggccttgatctcatcctgaagggcggactgccggccagccggctttatctcgtcgagggcattcccggctcgggcaagacgacgctggcgcttcagttccttcaggagggcgtccgcaagggcgagcgggttctctacatcaccctgtcggaaacgcgcgaggagctcgaggtggtcgccgcctcccacggctggagcctcgccgaggtcgaaatcttcgagttcaactcggcggccgacgtgctcggacacgggcgcgaccagacggtgctgcattcctgggagatggagctcggcgaaaccgtgcgcctgatccaggaccaggtggacaaggttcagccgaaacggatcgtcttcgacagcctttcggagatgcggctccttgcacaggatccgctacgttaccgtcgacagatcctgggtttgaagcagttcttcagcggtcgcgacatcaccgtcctgctggtcgacgacatgacaggtgccgaagtggggcaggacagcgccatgcacagcctttgtcatggcgtgatcaccctggagcgtttgacgctggacttcggcgccgcccggcgcagggttcaggtgcagaagctgcgaggcgtggacttcatcgccggcttccacgacctggttatccgcaaaggcggcctggacatctatccccgcctgatcgcctccacccaccacagcgagttcacaggcgacgtcacccccagcggcgttcagggcctcgacgacctgcttggaggcggtccgctcaggggaaccagcaccctgatcaccgggccggcgggcagcggaaagaccacgatcgcgcttcagtacctggatgccgcctgccggcgcggcgaacactgcgtggtgtacgagttcgacgagcggatcggcacgcttctggctcgtgcaaaggcgttcgaccttgatctgcaagcgcatatcgacaacggctgcatgacggtcgagcagatcgatcctgccgagatttctcccggtgagttcgcggcccgcgtgcgcgcgcaggtcgagcagaaccaggcgcgaatgatcgtgatcgacagcctgaacggctatatggccgccgtgccgcaggaacagcagctgatcctgcagatgcacgaactgctgtcgtatctcagccagaagggcgtggtcacctttctcatcaatccgcagagtggattggtgggcaccatgcagagcaacctcaacatctcctacgtcgccgacgcggtgatgctgcttcggttcttcgaggcgggaggtcgcatccgcaaagcgatttccgtgctgaagaaccgtggcgggagccacgaggacaccatacgcgagctgaggatcgactccaacggcatccgcatcggcggcgccttgtcggctttccgcggcgtcctgacggggacccccgagtacaccggcgtcgcctcccccttgatggaagaccgtgcccttggcgcataggaccgcgcctctcggatcgagcatccttgttgcagcgccttacggaagagacgccgaaagcctgatgacgctgctggccgacgaaggataccgggccgtcgtgtgcgacagcctgagcgaccttgtcgcccgcatcgacgacgcgacgggcgcccttttgatgaccgaggaagctcttgtcggcggctcgggcgagttgaagacccgcctgggcgagcaggccgcctggtccgacattccgctgatccttctggccgccagccgatccaaacagcccatgcggcgcgaggcgtcgcagcttgaggtgctcgacctcgccagcaacagcgtcatgctcgaacgaccgctgggccggagctccctgatcagcgccgtcgcctcggccctgaagtcgcgccaacgccagttcgagatgcgcgaccgccttctggagttggagaacagccgcaacgccctggccgagagcgaagccgtccttcgcgtcgtgacggattcgctgccgatcctgatcggctttgtcgaccgcgacctggtctaccgcttcgccaacgccgcctatcgcgactggttcggcgtcgatccggaccaggtcgtcggacggtctgtccgagatgtcgtgggcgatgcggcctttgctgtccgacttcaggccatgcaggcggcgctggccggcgaaaccgtgcggttcgaactgccctggacgcatctcgacaaccgtcgccgcgaggcggaaatccgctatcttccccccagggggccggacgggtccgtcaccggcttcgatgtcttcgtcctggacatcaccgatcggaagatgacggaggaagccctttcggcgcgggtcgccgaacgcacggccgctctggagcaggagatggccagccgcaccgaggccgaagaagcgctgaggcaaagccagaagatggaggcggtgggccagctcaccggcggcatcgcacacgacttcaacaacatgctgacgggcgtgatcggaagtctggacatcatccggcgacggcttgagaccggccgcactcaggacatcggcaggttcatggacgcggcgtccgcctccgcccagcgcgcagcatcgctgaccgcgcgcttgctggccttttcccggcgacagtcgctcaactcagcgccgctcgatgtgaatgcgctggcggcctcgctggacgatctgctgcgtcgaacgcttggcgaaaccatcgccctgtccatcgtccccggcagggacgtcaggggcgtcgtggccgacgccaatcagctggagaacgccattctcaacctggcgatcaacgcacgggacgccatgccggacggggggcggctgacgatccgcacctcgctggccgagatcgacgagacgatcgcgccggagacgccgcaggggctgcagtccggcgcctatgtcgtgatctccgtgtcggacaccggcacgggcatcagcgaggccgtgctggacaaggtgttcgaccccttcttcaccaccaagccgatcggccagggcaccggtctggggctttccatggtttacgggttcgcgcgccagtcgagcggccaggtccggattcacagccgggtgacggaaggaaccacggtcgaactctacctgcccgccacggacctcatcagggatgaagcggtttcgccggacgcccagtccgttcaggagggccagggccagacggtgctgcttgtggaggacgaccccgcggtgcgccagctggttcgagaggttctggttgaactgcgatacgaggttctggaggcgggcagcggtgacgaggcgctgcccctgctgtcgcagccccgcgccatcgacctgcttgtttccgatgtgggcctgccgggcatgaacggtcgccagctcgccgagatcgcccgcgccactcgtcccgaccttccgatcctgtttgtgactggatacgccgagaccgccgccgttcgcggcgaatttctcggcccgaacatggacatggtgaccaagcccttcgccctgccgatcctggcgtccaagatcagcgagatgctgaacccggtcaccgcctgagccgccccggggtggcgcacggtgcgcgccgcgggtcgcagaatccacgcgactcgacaatcttgcagccgtcgtagaccacctgagtgagttcgaaggcgtgccccctctaatcgacagccatcatggtccggcgatccgcttcgacggctcaagggataatggcggcgcgacctgaggcggcgcttcagaccgacatgctcgctgcgctgggttgttcggccgatgtaaccgcttacagtgccgtcagagcagcgcaggtgacactcagatggcggacgtccagcttacgggcatcgagaagcgcttcggcgaagcacgggtgctgaaggggctggaccttgcgatcgccgacggcgagttcgtggtgtttgtgggcccatccggctgtggcaagtccaccctcttgcgcaccatcgccgggctggagacagccgacgccggcgagatcgccatcggcggacgccgcgtcaatgacgccgagccggcggagcgcggcgtcgccatggtgttccagtcctatgcgctctatccgcacatgacggtgtacgagaacatggcgttcggcctgacgctggccaaggcggacaagggcgagatcgaccgccgcgttcgcgccgccgccgaggtgctgaacatctcgggcgaactggaccgcaagcccaaggccctttccggcggtcaacgccagcgcgtcgccatcggccgcgccatcgtgcgcgagccggaggtgttcctgtttgacgagcccctgtcgaacttggacgccgccctgcgggtcaagatgcgctacgagttcgcgcgcctgcatcgcacgctgggcacgaccatgatctatgtcacccacgaccaggtcgaggccatgaccctggccgaccgtatcgtggtgctgcgaagcggcgtgatcgagcaggtcggcgcgccgcttgagctgtacgaacaccccgcaaacctgttcgtcgccggcttcatcggcagtccccgcatgaacatcctgtccggcgtgatcgagagcgtatcgacggcgggcaccgctgtgcggctggagggcggagaaagggtgcacgcggccgtggacgccagccgcgccacggccggcgatccggtcagccttggcgtccggcctgagcatctgaccctgtcgggcgacggcgacgccctgtcggtggaggcgctgttcgtggagacgctgggcgcagccacctacgcctacttcagccatcccgccggatcggagacgctgacggtgcagctgccgggcgatgtcaggccgcaggccggcgagcgcctgatgctgcgcatccccaccgaccggacgcacctgttcgacgccgatggagcggcgttcaaacggctgggctgacgcgtctcctcccgccggaggagcccggcctcacctcaagatcacccgtttgctgccggccgggatggtcagtgcgtctccgctccagacggccgcgcgaccatcgatgcggatcgatcccggacggccctcgccttccggccagcgcagcacgaatccgccgggcggcgcggcgtcgccgtcgaggtccagccgatagtcgcgcccggccttgcgaaggcgataggttagcgccccatacggcgtccgcaggcccacgacgcccacaccctcggccgtgtcgaaccagcgcaccggcacgcccgccgccagcaccagcgcgctgtcgtcgcgctcataggcgaacaggtccagagcggagcggatgtagtccgagctgatccaggcgtgcggcatgtcgccgatgaagcgcggctcgcgcaggtcgcgcccgaccacctcggcccagccgttccaggcgcgcgggcgcacgtccgagaagtagaagtccagcgcccgccacgcctcctcgcgccgccccagccgcaccatggcgctgacgtttctcagctcatagggggtgtagtcgcgccagccctgacggttcttctgacgcgcggtgaagttcgcccaccacttgtcgaacgtcccgttcagcaggccttgcggcagctcgtcctgcaagccgcccggcgacaggccgatggtggtggaggtggcgtcgaagtcgccccgatccgccgcgcccgcgatccagtcgatgtggtggaaggccgccgtggcccgggtcgaagccagtatgtccgtcttgaactgctgctcggaggcgcggatacggcctgccgcctcggcgtcgcccagggtctcggcgatgaaaaccgcatcgcggtagccgcgcaggccccagaagtcgtcccagtaggagtaggccgccttgtccgagtagccctcatggctgatcgtcggcggcagcaggccgaagaggtggcgcgtctcggccgtctggaactccgccgtccgcgtagaggcgcgcagctcgtccatgtagcggatggcgccctgcacctgcggccagacctgtcgcagcagcgcggcgtcgccgccgtagcgataggcctcggccgccaggaagacgaactcgccgtggctgtcgttctccggcaccggatcggcgccgcgcgcatcgacgcaacacggcaccttgccgttggcgaacaggtaaggcgcgtaccagcgcagataatcctcggacaggtcggacaggcccagccggttcagcccctcggccatcatggcgccgtcgcggatccaggaccggttgtacgaccgcgtgccgggctgcaggatcggcccctgccggctcatcagcatgtgggccagcgaggatttcagcacgtcctcgatgcgctgcccctccggcggcaggatcagatcgacccggtcgattcgcgcgcgccaggcggcggcgacccgatcctgcaccgtgtcgagcgcggcctcgatgctgcccgtgacgggaggatcggccggcgcctcgcccaaggccgagacccagccgaacgtgcggctttcgcccggcagaagcgcgaccacataggtggcggccgcggcgggcaggcctgtcgcgtcctcgaccgacgctaacgccgagcgggcggcggccagcagcgactgcggatcggcgccagcgtcgaaggtggaggccgtcacctgatcgggtgcgctcagcatccgcacggccgtgtcgtctcccaggctcaagacgccgccgtcccagccgatccgtgacagggggcttgcgccgcccggcaccgccaggaactgcaccgggccgttcacctgcatggcccgtcccatcagcgccagcgtcagctccaaagggcgcgccgaggtgttggtcaggacgtagcggccatacagttgcgccgtctcgggcgcgccgtcggccagggcggtgacgcgcagggtccagtcgtcatgcgtccacgtcacgctggggatcggcaggtcgtcgtcggcgaggaactgttcgatccggacgtcggcccaggtgaccagccgcccgttctcgatcacgaacggctccatgctgggtcccccgcgccgcagctcgatggcgccgtcctcgccgatcaggccgctttcgccgcccccgtccacgccgacgagtgtccagtagggctgttcgccgaagaagccgcgcggatagaggccgcgccggttctccttggccacggcttccagaaaggcggtgtggtcctcgccgaagctcagcggctcgatctcgatctcgttcagcgcataggcggtgggcgaggcgacgcccagccgctggccggcgcccgcctgtcccgtgacgtccgatgcggccacaagggcgcggggttcgagccgcagccaacgggcggagacttccggcgtgcgcagccagtccgttccgccgttgccgccggtgacggagatcagctctcgccaggcctcgccgtccgaggacgcgctgatacggtagtcggaggcggcgccccgctcagcccaacgcaaggtgagaccgccaaactcccgctcatacccgaggtccagcgtcaggatgagcgatcccgccaccggcgcggtccatgctgtcttgggatcgaggtccacggccaaggccgctgtagacggtccggcgccgtcgctcgccgtcggctgcggcggcacggcgggatcgacgggcagcgggcgcagtgtcagctggtcgatttcgagcgcgcccttgccgccgtcggcggccaccaccacgaactcgatccgctcggcacggcgcagcaccgtctcggggctggggccccacgccttggacacctgacggcggcggatggtgaagcgcgtccagccgtccggcgcgtcatagcgcgtcgtctgtttccaccagacgttctcggcctcggcgtcggtaaacttgacctcgaaggtgttggccggcccgtcgccgcgcacccagaagctgatctcgtagttgtcgggcaggtcgaacgccagaggtcggctggccaccgcatagccagccttgccggcgaagtcgtagtcgagccggatggcgcgcccatcctgcccctgcacggacgacacgctcgagacgatgtcggtcgacgcgctggcctcccaccgcccggcgtcgtccatgttgtcgaggacgcggatgtcctgcgcccgagctatggcggggccggtcagcgccgccgacagagacagggacgccgccgtggcgagaagaagggcgcgcatggcggtctccgtgaaggctcagcccttgacgctgcccgcgagcatgccgcggatgtagtagcgttgcagggccagaaagaggatcaggacaggcgcgaccgtgacgaccgccccggccatcatcagctcgacgtcctgcacgtgctcgcgcgacagggcggccagcgccaccggcagggtgtagttcgactgatccgtcagcacgatcagcggccacagaaagtcgttccagctgcccaggaagacgaacaggcccagggtcaccacgatcggctgcagcgtcggcagcaccacgcggcggaagatctgcccttcggaggcgccgtcgacccgcgccgcctccagcatttcgtcggggatgctgagcgcatactggcgcaccaggaacaggccgaagatcgacgcaagccaagggaccagagcccccgcataggtgttcaccagccccatgctcttcagcatcaggaacagcggcagggtgccgatctgcgccggcaccaccagcgcagccaccagaacctggaacagacgctcgcgccccctgaaccgcagcttggcgaaggcgtagccggccggcgccgtgaacaacagcgccaggatcgtcgccagcgtcgccaggatcaggctgttcaggacatagcggcccatgccctggttcaggaacaaatcctgatagtgctccagggtgaagcgcgaggggaccagcggcggcggaaaggtcgccgcctcgcccgtcggcatgaagctgacggacagcatccagagcagcggaaacagcacgatcagggcgatggccgcgacggcgaggttgagcagaacggccttggccttcatcgcccgcgctccacccgccgggcgacggccagctgcaccagcgtcaccgccaggatgcagaggaacagcacgaacgccaccgccgaggctgagcccaggttccaccatttgaagccctcttcgtacatgaagtagagcaccgtcaccgtgctttgcgccggcccgccctgcgtcatcacatagggctcggcgaacagctggaagaagcccgccaccgagatgatcgacaccagcagcatggtcggcgcgatcgccggaagggtgacatgccggaaccgcccccacggacccgcgccgtcgatccttgcggcctcatagaggtcgtcaggcaccgtctgcagcacggccaggaagatcagcatattgtagccgaaaatcttccacaccacgaacatcaggatcgcgggaatggaggtggagggctggcccaaccagtccaccgccggcagtcccaccccgtccagcgcccagttgatcacgccgtaccgcgtgtgcagcagatagcgccacaccacggccgtcgccaccagcgtcgtcacatagggcgcaaagaacatcacccgccagatcggccgccacttcaccatccggtcgttcaggatcacggccgccagcagcgacgcggcgatcgacagcggcacgcccagcacgctgaaccacaccgtgttcctcatcgcgccccagaacaggggattggtcagcagtcgctcatagttttgagcgcccacgaaacgcaggttgccgagatcggccagcgcatagatgtcgaagtcggtcaggctgagcagcagcgccgcaaccaccggcagcgcgaagaacaggccgatggcgatcatggccggcgcgatgaagccccaggccgcgcgctcgcgccgcgatcggcccgcacggctccgacggatcggcttggtgggaacgggcgcggtcagggtcatgccgccctccccgtctccagcatccagcggcgcttctccagcagccggtcggcgcggcggtcgatctcgcggccggcggcttctgggctgtattcgccgcgcaccatgcgctcggccacgatctgcatctctgtgacgatccgctcccactccggcaccttgggcacggccttcgcgcggctgagctggccttggaacggcgtcagcatggcgtcgccggcgatcgcgggcgtgttccaggcgctctggcgcgccggcaggtcgccgaccagggcgttgaaacgctgctgcacctgcggctcggacagatagcgcaccagggaccaggccgcctgttgatgcggagaggaccggaacaccgccaggcttgagccgcccggcgccgaggcgcccagtcccgtcggccccggaacgccggcggtcgcccagttcgcccgaaagctttccggcaggcgcgagcggaagtcgccgacgctccacggaccggagaaatagaagctgaaccagccgcgctcgaactcggtccagacgttggagatctgcgtcgatgacgccagcggcgccagcccttcgtcgaacaggctcttgtagaaggcgagcgccgagacgaacccggggctggaaaagtttccgcgcgtgtcgcggtcgcgcagcatcggctcggcctgctgcaggccgaacgtcagcagttgctcgaactcattcagcggaagcaggatggcgtaggcgtctccgcccgcgacgcgcttgaccgcatgcatggaccgcttccactcggcccaggtctgcggcgctgcctcgaagccggcgcggcgcaagagatccgtgcgatagaagatcagccgcgtatcgacataccagggcgtggtcatcgcccttccgccgacgcggttcgtgtccagcaccgccgggaactggtccgtcagcagatcggcggccgccggcggcgtgggcgacaaggcgccgatcgccgtcagctcggccacccaggtgttgccgatctggctgacgtccggcagcgacgatccggcgtaggcggtcaacagcttttcgtgcgcggcggtccaagggatggcctgcacctcgacccgcacgccgggatggcgacgctcgaactcgggcatcaggttcggaacctgaccgccctcgttgcccatggcccagaagcgaaggcgcgtctcgcccgttggtcgggaggcgcaccccgccgccgcgcccgcagccatcaggccgagcgcatgacgacgatgcgggcgcgcgccgttcgtcacgccgacaaatacccgccggtgaaacccgcgacctcaagcccacgtcggatgttcggctcatcgcgcatatgacgccagacaaggtccgagcgatggttttcggtcatgatgacgatcggcccctggtcaatgccaaggtaatcgccgtcgacccagccgatcccctccacgatcctcccatgctgcaaaggactgtcgcggaccgtcagcgtcgggttgaagctgtcgaggaagccccactgcgtatagagtcccgcgccataacgcgccttgatcgccttgacacagggcaacacgatctcgggggcaaaggcgatggagccggccgccgccgtgggcgccagcgtgccgtcgtcgcgatcgcccggcccgcgcgcggagtatgaaaagaactcgcgctcctctccgtcgatcatctgcttgaaatcgcccggaccgtcgcaggcggtcagtccccagacttccgacgaatagccggcccagcggcccggattgtcgtgggcgtacttctgctgagcgtagacggcgcggcggctgttctcgaagtagtcgagccgctcgtcccgcaaggacgactgaccccgcatccacgcgtcctggatgtcgcggaaatccacaaacatatggctgtactggtggccgaagatcggggcgaactccaggtgccagctgccccatcgttcggtccagctcttgtcgtagccataggcccactcgtgccagacgccggcgtccagcggatgggtcgggctgcccatggccaagagcaggatcagcatgccctcgttatagacgaaccagtctgcggggatgaaaccggtttccggatgccagcccatgctgatgcggttcggccgcaccacggcccagggccactccacccgctcgtagaggaactgcgccttttcccggatttcagcctcgtccggatggcggccatcaaagtagcgcgccgcgaacagcatccccgcgatcagcagcgccgtatcgaccgtagacagctcgttctgcgcgaaccgaaggccggtctccatgtcgaggaaatggtagaagaagcccttgtaccccgccgcgccggacgcttccggtccctgaggcagggcggcgaagaagcgcagggtgttcagcgtgcgctcgcgcgcctcgtcccgatccatccagccgcgctccaccccgaccggccagcaggtcagggcgaacccgaccgccgcgaccgagcagaaggacttggtcggccaacggtccggcgtcagaccgttgcgcttatccgtgacgtgagcgaaccagcgaaaggttcgctcctgcaactcatcgacctcgcggtccagcctcagcggccggcgctgtgtgccattgaccggatccgccgcgaccgcacgcgtcgccgacggcgtggcttgcgccgccgcctcggctgacgaccccacggccaaggccgccgcacccgccgtggtctgcaacagaaggtctcgacggttcatgaaaggcctctcagggtacgcgacagatagaaaaaggccgcctcccgcaggtgcggaaggcggccgggcaggcgtttagaaggagtagcgcagcgtcgcctggaagctccgggtgggcagtgcttggctggtcgggatgccgaaacgcggattcagcgccgcgccggcattgttgttcacacgatacgcctgatcgaagccgttgtagttcttgaagttgaacaggttgatggcgtcaacgatagcctcgatccgctgaccgtaaaccgtgaagcccttgttgaggcgcagatcgatctgacgcgtggcgaagttcaggcccggcagaaaagcgcgcttctcgggataaccttcaaaccacagtggcttggcgccgtcccccgggttgaagatggtgaatgggcggcccgaccccaaggtgatgatggaggaagcacgaacgtcccaaggcaggcgcaatgtgcccgaagcgacaatacgatgcttctccacgccaggcgtgttgaaccagggcgattggtcgatagtggcgtagtcgaaatcgaacgagccgaggctctgatcacggctgccgttctgttcgccgtcagccagagtatacgcaacattgaagccccagccgctcgcatcggtgtacgggcgatccaaggtgacgtacatcgccttgtaccgacgctcacgatcgctgctcgagtagaacaccgagtcattgaacgcataaggctgacccgtgtctgggttagtgaactgcgatgggcgcactgtaacggcgttggcgtcatttacgttgaggcggttccactggaactcgtctttggttcgggcatatgagaaggtgactgccgcttggatgtcaccgaacttctggcgaacaccgaggttgaactgatcggtgtatgggatcttcagatcatttttgatcaggaagatttcgcctcgaccttgcgttccgcccaacaagccgtcgagcccttcggctgtggcgtagctaggatcccaagcgatggtgttcgtccgaccgccgaaggccccgccatcgggcgagaaaaagatctgccgtgacaggttgaacggcgagaatctttccgaaaatgcgaagttaaagccgacgcgatcgtagtagcggccagctccgccgaaaatcaccgtctgctcgtcggcgaacaggtcgtaagagaagccgatgcgaggttggaaggccccggtgaacgcgtcgcgatcgccatcggagatgtagtcgttgacgtcgacacggcgaacataggtcggatcagcggcgatgaggcccaagacctcacggataacctcaggtgtaaccaggtcattgttgaccgcattatcttcataatcccagcggatgccgagattcagttccagcttgtccgtgacctgccaatcatcctggatatagagtcccagctggttgttcgaaacattcgccggatcggttggtagattgaggctcacccgtgtaggaatggcgttcgaaccgagaacggccgggttcgcggtcacgtcataggtgaactgaggattccggttgaagaacttttgcacgtaataatcgcgcatggagtacttcaccccgaccttgatcgtgtgtcgtccagcaagctcgatttcattgaacgtcagatcgttacgcagcgtaatcgagtcgtcctggatgtcctggttattcgtgcctccgcccgtattgaacacgaaatcggactgatcatagttaaactggaatccgggcgcgtcggcattcgcatcccggtaggcgacgtaagcggcgccggccaggtcgaagttctccgcccgaggattgtagttggaatgcaggtaatcgacggtgaagacgttcaggaagctgtcgccctgaaactggtgacgcaagacaatggagcgggtgtcattgttgatcgcgttagctcgcgaccgaccgctctgaccgccgaagtcgcggatatccgtttccgtacggtaagtcgccgtcagatcgacgatctggcggtcgtcaatctgccaagacagcttgccgaagaacaggtcctcttcaaacggcgcttcaaaggtgccgagttcgtccgcaaacagatcattgtattgggtctggttcaggaacacggagttggaacgggtttcgtccttgcgctcatagctcaacaggtagtgcaggcgatcacggatgatcggcccagcgacagtgccgccgtactgcaggcggtcgagttgcggcttaggttcgccacgtctttcggagaacgtctgctgagcgatccagtccgtgtcctgataggtgacaaagaagtcgccggtcagttcgttcgttcctgagcgggtcaccgcgctgatgatcgcggacgaggcttgttcgtattcggccttgaagttctgcgtcaggacacgaaactcctgcaccgcgccttgcgggaagggattgccgcggctgtcgtcctgcccggccacgccgccgtccaggatgttggacttctggctctgaccgtcgatgaaaacattgatggcgttagccgactgggagcccgcatagatggtgcgttcggaaggatcctgctggacgaccacgcccggcgccaaggcggcgaagttcaagaagttgcgatccacctgcggcaggttgttgatctgctgctgcgagacgtttgtcgcgacttccgaggtgcgcacctcaaagatgcgccggccggtcacaacgatgtcgccgaggtcggttgctgcgacctcggaagctgcaccaccgccggctacgccgctgacgtcaaggtcgagggttgcgacctgccccactgtcagcgtcaccagatcagtggcggcttggccatctgcgctggtgacggtgatctcgtacgagccgggacgcaggcctggcaagacatagacgccgtcttcgccgatacgcccgcggctcacgaaaccggtgctcgtgtcccgcgcgatgatcgagcctccagtctcgggcgattgtccgtcataaacggtgccgcgcaaggtcgacgtcgtgacttgcgccatcgcccctccggcgctgagcaggctgacggaaagcgcaagcgccgatgcggcggccagggcgtgattacgggtcttgatgttaggcatggtgagactcccccctgagattttggtcacgcccttcggggcggggcgtgacccgttctggttgatgttgcaaggcgacgctggactgacgcacgaccagtgcgggacggacgatctcgcgcccggattccggccacgcgccggtggcgggcgcctggatcaaggtgatcagccgctcaagagcgcgcgcgccggtgccggcgatgtcgatcctaagcgtggtcagcgccgggcgcaccagttcggcgatcggcacgtcgtcgaagccgaccacggccacatcctccggacagcgcaggcgcgcctcctggatggccagaacggcgcccacggccatcatgtcgttggccgcgaacaccgcgtccggcggcgacggttcggccagcatccgggcgacggcgcgatagcctgacgcctgggtgaagtcgccctgctcgacacggcttccgagccctgcgtcgccgagcgcgcgcaggtagccctggacgcgctcgtccgcctcgagattgccgagggggccccggacatgggcgattcgccgccgcccggtctgcaccagatgggcgaccgcctgggccgcgccgccgtcgttatcgacaacgatgcaggggcgatcggcgcccacggcggcggcgttcatcagcacgaccggcagcgagcccaccagtccctcggccagcctggccgcatcgaggtgcggcgacagcacgatcaggccgtcgacccgcccccgcatcgagcgcatggctagggcgacctcctccgcatcgtcatgggagcttgagacgatcaggtgtttgccgtgagcgcgcgcggcccggtccatgccgcgaatcagttcggaaaagtactcgccgaagaggtccggcaggatgacgcccagggtgtcggtgcggcgggtcgacaggctgcgcgcgccgctgtgggggacgtagtgcaaggtgtcgatggcttccagcacgcgaccgcgcatggcgtccgtcacggtgtcggcgccgttcagcacacgcgacaccgaggccacggatacgccggagcgtttcgccacgtcgcgtatcgtcgccgacctcaccgggcgacccgcccggacgatggcgagccctctcgcaccaacttccgcctccctgcagcgatcgttccagccttcctctcgaaggtccgtcgatcaaatctgtaaccggttacatcgcacgacgaacaggcggtcgcaatagcgagccgagcgccgtcggtgaaaggccctgaaactccttcactcagccggccgccaagcgcctgcggtggaggtgtttccgcccgcccgtcgcccggacctgatcaccttgcggaggaggtgatcccccgccggcgttctcaatctcaagcgccaagcccaacaacacgctcacaggacggcacggtcaaacgatgcgaagtgaccccgctcgggcggtcatccttcggaaaaggagaggcggtaggcgtggcgctggcctccgccccacgaccaagccagcgctggcctttcataaagtccggtgcgggcgacgctctgagccggattgcaggccgcgatccggcaatctccgccgcaggatggcgtcacacaaggggagcgccgccttgcggcaagcctctgccgctgccgctgccgctgccggtgtaaggatgatggcggagacggagggattcgaaccctcggtaccccttacagggtacgacgatttagcaaaccgttgccttcagccactcggccacgtctccagcggctgcgtcgatagcgggtcgcgggcgcgggcgcaatcccgttgccgatcgccatcgtcgccgggccgaccttggggccgttaacgcgaaagagaggccgccgcggcagggtggcggccctgccctgcaccgcggacccgcatgcccgattgcgctttgcttattgacgacgccgccgccgccgagcccgccaaagggccggacacgcctcgacgcgggccgtttcgcccggacgtctggctcaatgcgcgccagagatccgacgtcaggctggcgccgcatgcgtttcgcgccatcgatgtcctggccgtggtcgccgtggccgtgatcgcgctggcgggtgaaggatcggaccggctggcggatctcgcgccggtcattctcggcgtgctggtcttcgtcgcggccacgccgtcgctgggcggatatcgtttcggtcggacgggcggcgtcctggtgcacctggggccgctgctgatcggctggctgctcgcctgtggcgcggcgatggggctggccctgctgctggagcgaggcgcggaggcggcgcaggtctggtccctagccggggcgggcgtgctgttgctccttcatgcgctgtggaccggcatggttctgcgctggagccgcgggggcgtgctgcggcctaatgtggtcgtggtcggggcgacccgctacgctgaggccctgatccgcagcgccatggaacggcgcgacatcaatgtgctgggcgtcttcgacgaccggctggcgcgggcgccggacagcctggtcggcgtgccggtgctgggcgacgccgaggccctgatcgcacaccggatcacgccctacgtggatcacatcgtcctggccatcgacccgcaggccggcgcgcgcgcgcgggagctgacgcgcaagctggagaccctgcccaatccggtcaccgtgctggtggacgacagcggccgcgacgcagcgctggaccgtctggcccgtgcgccgctgtcttcgctgacccaggccggcagcgacgcccgccgcgccttcgccaagcggatgctggacctgaccctgggcgcgctcgccctgctgcttgtggcgccggtcatggcgctgatcgcgctagccatccgtctggacagccccggccccgtcttctttcgccagcgccgtcacggcttcaaccaggaagaaatcgtggtgtggaagtttcgctcgatgcggcgggaggcggcggacgccaccgccagccgccaggtcacggcggacgacgaccgggtcacgcgcgtcggtcgcctcatccgcgccaccagcctggacgagctgccgcaaatcttcaacgtcctgtccggcgagatgtcgctggtcggcccgcgcccccacgccatcggcatgaagaccggcgacaccgaatccgcgcggctggtcgccgactacgcccaccgccaccggatcaagcccggcatgaccggctgggccgccacccagggctctcgcgggccgctgcacagcgaggcggacgtgcgccgccgggtgcagctggacatcgactatgtggagcgccactccgtctggctggacctgtggatcctcctggtcaccgtgcccgtgctgctgggcgaccgggccgcggtgcgatgagcgcggacaaggacgggcgcatgttctggcgcggcgtgtggggctatctgcccgccaacatcgtccagggcgtggtggggttcgccaccatcgtggtcttcacgcgcctgctcagcgccgaggacttcggccactatgcgctggccttttcgatcaccagcctgctgcacctgctggccttcacctggctggaggccgccatggcccggttctgggccggggagcagacgcccgaaggcctcgccagccatttcgccagcctgtaccgcacggcttttctagtgatcgcgatatttgtcccggcggccgctctcggcgtctggctgtggccggccagcctgcctttcaagctggcggtggcggcgggtctggccggcgcgccgctgcggtgcctggccaagctggcgcaggaacggtttcgcgcggcgggcgaggtcgcaaaggccgcgcgcgtcgacatgggcgtggcgatcgtcggcttcgccgtcggcgcggggttcgcgctggcgggcgcgggcgcggcgtctccgctgctgggcctgctggtcgcgcccttgttcgcgctcccgttcgtgcttccgggcgagttgcggcaggccaggcgcggcgtggtcgacagggcgcgcctcaaggcctacgccgccttcggctatcccgtcgccgcgtccctgacgctggcgctggtgctggcctcgaccgaccgcttcctgctggccgccttcatggatgcggcggcggtgggcgcctatcacgccagctattcactggcgaaccgtacgctggacgtgatgttcatctggctgggggccgcaggcgcgccggccatggtgatggcgctggagcgtggcgggcgcgaggcgctgaggcgctcggcgctggagcaggcctcgacgctggtgctgatcaccctgccggcggcggtggggctggccctggtcgcccggcccatggccgagctgatgatcggcgaggacctgcgcgccgcagccgtgatcgtcacgccgtggatcgcgctttcggcctttctgtcgggcatgatcgcctactacttcggcttcggcttcaccctgggcaagcggacggagctgctgctcctgaccaccgccgttccggcggtcgcgaacatcgggctgaacctgttcctgatccctcgcttcggtttggtcggcgccgcctgggccaccgccggcagcttcgccatcggcctggtcgcctgtgtccttctcagccgacgtgcgatcccgcttccggtgccgtgggggacgctcgcacgctgcggccttgcggccggcgccatggcggccgtggtcgggatcttgcccgcgcttggaggcctggccgaactggtgctggacgcggggacaggcgcggtcgtctacgccgtgatggtgctgatgctgaacgcagccggcgtgcgagacgtcgcccgacgcctgctggcccgccggcaggacgcgcccgcatgacctcgccccggatccacgacaacgccgccttcatggcggccaggcccatcgtgtccgtgctgatccccttcctgagggatgatccgtctgacctgctgacgcagctggccgccgaagcgacgcccctggacggcgcggccgaggttatcgtcatggacgacggcacaggcgatccggcgctcacggcacgtctgcgcgccctgatcggcaccctgcccctgccgatccgcctcatcagcctgccgacaaacgaggggcgagcgcaggggcgcaaccgcctgaccgaagccgcgcgcgcggacgcctttctgtttctggacagcgacatgcggccggatacggagacttttctccagaattggaccgagatcgcccgcggccctgcgcccgccgtggcgttcgggggtttctccttggacgcggcgcctcaagagccgcgcttcgccgtgcaccgcgcgctgtcgctgcgctccgaatgcgtcccggcgtccgatcgcgccaagcagccggagaagtacgtctacacctccaacctcctggtccgccgcgacgtgttcgaggccgagcggttcgacccgggcttcaccggctggggctgggaggatgtggagtgggccatgcgggtgtcgcgccgcttccccatcgtccatgtcgacaatccggccacccacatggggctggacacggtggatgcgctggcccgcaagttcgagcaaggcgcgccgaacttcgcccgcgtcgtcgcgctgcaccctcagttcgcgaccgcctatcccagctacaaggtcgcgcggattctgcgcagcctgcccgcgcgcggtctgctgcgcggagttctgaaggccgctgcgaaggcgtcgcccctgcccgtcgccgcacgcgcctttgcgctgcgcctctatcgcaccgccctctacgccgaggcgatctgatgggcgacgtggcggtgatcgtgcccacgctgcggcggcccgacagcctggagcgggcgctgcgctcgctgttcgcccagacaggcgtcgagggccgactgacagccatcgtggtcgccgacaacgatccgcaaggttcggcggcagaggtggtggagcggctaagacgcgctgcgcccgccccgctcgtctatgtccacgcccctgtgcccggcgtcgcgacggcgcgcaacgccggtctggcggctactgaggctcccctgatcgcctttctcgacgacgacgaggcggcctctcccggatggctgttggccttgctcgcgggcatgcaggacacgggcgccgacgtggtcttcggccccattcgaggccgcgtgcccgatgacgccggctgggccgcgctctatctcgagcggttcttcggacgggatgggccggctgagacccgcctgatcgacgagccctacggctgcggcaattcgctgatgcgccgcgctgtcgcccttccgggcccggcgcccttcgacaccgccatggatcagtccggcggcgaggacgacgtgctgttcgccggcgtgcgtgcccgcggcggccgtttcggctgggccgctgaggcgtgggtcgacgaattcgcgccgccgcatcgcgccacactgcgctacgccctgacccgcgccttcgcctatggccagagccccagccaggccgccgccgcgcgtcgggactggcctggcgtcgccaagtggatggcggtcggcgcggttcaggcggttgctcgcggcctcaaactcgcgccgctctggctcatgcgcagcccccgccgcgccgaggcgatggacggggtggccaaaggcttgggcaaggtgttctggaccaggcggttcgaaccccgcctgtacggcgccgccatgctgaaggcggcgccgcccgccgatcagcccagcgcctgatccagatcagcgatcaggtcgtccacgtcctccacgcccacggacaggcggatcagactatcgctgaccccgcccgcctcgcgcacctcacgcggcaccgaggcgtgagtcatgatggccggatggttgaccaggctttcgaccccgcccagcgactccgccagggtgaacacctccaccccctccagaacgcgccgggtgcgctccaggtcgccgtccagcaccaccgtcaccatgcccccgaacccaccgggcatctggcgggccgccagatcgtgctgcgtatgggcgatcaggcccggatagatcacccgcgccacccccgcgcgggtttccagccagcgcgcgacagccatggcgttttcgcaatgcgcccgcatcctcagcgccagcgtcttcaagccgcgattggccagaaaagcgtcgaacggccccatcacgccgccgaccgagttctgcaagaacttgatccgctgtcccagatcggcgtcggcggtcaccaggaccccgccaatgatgtcggaatgtccgttcagatatttggtggccgaatgcatgacaacgtcggcccccaggctcagcggctgctggcagaagggcgtggcgaaggtgttgtccaccaccaggatcagcccgcgcgcccttgcgatctgcgacagcgccgcgatgtcggccagtttcatcatcggattggtcggcgtctccacccacagcatccgtgtcttcggcgtgatcgccgcctcgaccgccgcgatgtcgctcaggtccacataggcgaagtccagccccatcgaacggcgccgcacccgctcgaacagcctccacgagccgccgtacaggtcatcgccggtgaccacatgatcgcccgcgtccagcagctccagcgccgtggacgtcgccgccatgccggaggcgaagccgaagccgtgggttccgccttccaggtccgcgatgcacgcctcgaacgcctctcgcgtcgggttcttgccgcgtgcgtactcgtaccccttgttcacgcccgggctttcctgggcgtaggtcgaggtggcgtagatcggcgtcatcaccgcgcccgtggtcgggtccggacgctgtccggcatggatggcgcgggtggaaaaaccctggttgttcttcttgccggacatcgacttaccggttcaggctgaggtggttgatcagatcggtgcgggtgatcaggcccacgaaccggtcgccgtcctgcaccagcgccacccggtcgcggtcgaacagggggatcagcgcatctagcggctcggacacctgcaccgtgtccagatcgcgcgtcatggccgaggacaccggcttggcgaaccgctccttccgcgtgatctcgtcggtgttcatgatgtggacgatgtcgctctcgtccaggatgccgaccagccgcccctcgtcgatgatcggcaactgcgacacatcggctccgcgcatccgcttgaaggcggtgtccagcgtatcgtccggcccggccacaaccacgtcgcccttttcgtacttgcgcgtgatcaggtcggagaggtcgccgtgcagttcgcggtccgacagaccctgatcggccagccaggcgtcgttgtagaccttggacaggtatttggcgccggtgtcgcaaacgaaggtgacgcaggtcttgggctccgtctgctcgcggcaccaacgcagggcggcggcgatcagcgtgcccgacgatgagcccgccaggatgccctccttcagcagaagctcgcgcgcggtggcaatcgcctccgtgtccgggatcgaataggcgcggtcgatcaggctcatgtcggcggtgtccggcacgaagttctggccgatgccttcgacggtgtagctgccctcagggccaggaacgccctcgttgacgatccccgccagggtcgagccgaccgggtcggccaagatgatctcggcgtccgaacccacgctgttgaggaaccgcgccgtgccggtgatggtgccgcccgagccgatgccggcgaccagcgcgtcgatccgcccgcccgtctgctcccagatctcggggccggtcgtcttcacatgcgcctcggcgttcgcctcgttggcgaactggttgacgtagtagccgccgggaatcccctgcgccaaccgctccgccatgtcggtgtagtattccggatggccgtgcggcacgtccgaacgcgtcaggcggacgtccgcccccatcgccctgagatgctggatcttctccttggacatcttgtcgggaatgaccagcagcaccttgtagccccgcgcccgcccgaccagcgtcagcgccagcccggtgttgccggccgtcgcctccacgatcgtgccgcccggcttcaagaagccctcgcgctcggccgcctcgatcatctccacggcgatgcggtccttgatcgacccgcccgggttctgcgcctccagcttcagcagcaggcgacatcgtccggtgtcgatccgcttgacctccaccatcggcgtcttgccgatcaggtccagcggcgtcgagcccggcgcgctgagggttggggcggacagggacatgcgaaactccacgcgggatcgagcccgaaagctgagggtccagccccttccggtcaacccgcgtcaggtatgaccgccacacacgcccgctcggccgctggcgaacaccaatcagaatggctatatttctggccataatggagatgggtcatggccacctacggcgttgcggaagccaagaacaacttcacccacctgctggatcgggctgaaagcggcgagcagatcaccatcacgcggcacggcaagccggtcgcggagcttcgccccctgcccgcgatgacgccggagcagcgtaaggtccgactgctggagatcgccgagcggcgcctcagtcggccgccgctcggcatgacgtccgtggagttgatcaacggcatgtatgacgagccggtggaatgatcgactacttcgacgccagcgtcgttgtgccgtttctgatgatagagcctcatagccgcgcggtgatcgacctcatggccgaggcgcagagaccacaggtcagcgactttgtcgtggcggaggtttcatcagccgtgtcgcgactggtgcggacacgaacgctgaccttgacggaggcggacgccgccctgcacgacctcgacgactggattgcggcgacggcggcgccgatcccaatcgagggctccgatgttcgcgaagccactgctctggtgcgtcacttcgacctgaagctccgcgcgcccgacgctctgcacatcgcggtctgccggcggatcgacgcccgcttgataaccctggacatcaacatggccgcagccgcccgagcgctcgacctttcctgcatcaatcccgccgaagagtcggcggcgtgaaggactgaatgacgaaatcaaccaagaggccgcccgcaggcctccccgacaaggacacgctgatcgcctccctgcgtgaggcgggatcggccgagaagaccgccaccgcccgccacttcggcctgaagggcggcgaccgacgcgccctgcgcgagatgatccgcgagcttgaggccgagggcaagctcggcaagcgcggccgcaagggcttctccgaagccggcgccctgcccccggtcggcgtggccgacgtggtcgagcgcgacgccgacggcgagatgtacgtgcgcctggtcgaggcctcgcccgatgcgccgcgcgcgctgttgatgcccgaccgcaagacggcggcgcccgcgcccggcatgggcgaccggctgctggtcaagttccagcgcggagaggacggctgggaagcgcgcctggtcaagcggttggacacgtccgccaaccgcgtgctgggcgtcatccgcaagtcgtcgcgcgagacgcgggtggagccggtggaccgccgctccaaggacgtgctggtggtgcccagtattcaggccgacgacctgcgcgacggcgacctggtgctcgccgccatcgagaagggcgaccatcgatacggtcccaagcgcggcaaaatcctggagaccatcggcagagaggacgatccgcgcgtcgcgtcgcttctggccatacacgcgcacagcgtgccgaccggcttctccgagactgtggagcgcgaggccgaggatcaggcgctgccgacgctgaaggggcgcgaggatctgcgtgaggtccccttcatcaccatcgacccggccgacgcgcgcgaccacgacgacgccgtctatgcacagcgcgatgaggatcccaagaacgacggcggctggatcgtctgggtcgccatcgcggatgtcgccgcctacgtccgccccggcgcggcgctggaccgcgaggcgcgggccaagggaaactcgacctacttccccgaccgcgtcgagcccatgctgcccgaggtgctgtccaacggcctgtgcagcctcaaggccggcgagaaccgcgcctgcctggccgtgcgcatggtgttcgacaaggacgggcggaagaccggccaccgcttcgtccgcggcttgatgcgctcacacgccaagctgtcgtatgaacaggcgcaggcggccatcgacggcgaaacggacgatgtgaccggccccatcatggaggcgatcctctacccgctgtggaacgcctaccacgccatgctgaagggccgggagcgtcgcgctccccttgccatcaactcggccgagcggcgcatccgcatgacgcccgagggcgacatcgcctccatcgagccgcgcgccagcctggaggcgcaccggctgatcgaggagatgatgatccaggccaacgtctgcgccgccgagacgctggaggggaagaagacgccgctgatctaccgcgtgcacgaggcgcccagccaggagaagatcttcaacctggccgacttcctgtccaccctgggtctgccgtggaacaagggcgagccgggcacgaccaagcggttcaacaagctgctggaccagatgcgcgacagcccgcacgccgaggtcgtcaacgaggtggtgctgcgcacccagatgcaggcgatctactcgaccgagaacgtcggccacttcgggctgcacctggatcgctacgcccacttcacctcacccatccgtcgctactcggacctgatcgtgcatcgcgggctgatccgcgcgctgaagctgggatcggacggcctgaccgaccgcgaggtcgccgagatgacctccatcgccgaacaggtgaccatgacggagcgccggtccatggccgccgagcgcgacgccatggaccgctacatcgccgccttccttgaggagcgggtcggcgcgacctttggcgggcgcatcaccggcgtcacccgcttcggcctgttcgtcaggctggacgagacgggcgcggacggcctggttccggtttcgtcgcttggaagcgaatacttcacccacgacgatcgagcccacgccctggtcggcgaacgcacgggccagcgttacacgctcgggcggcgcgtcgaggtgaagctggtcgaggcgacgcccgtcaccggcggtctcctgttcgagatgctgagcgatcccgagccgcgcgatccaaacgcgccggcgccccgctatggcctgcgcggacgtggcggcgacggtccgccgtcccgcggcaagggtcggccgggcggccccaagccgcgcaacggctccaagcccgccggcgggctgaagggggtgcgcaagggcaagcggcggtgaccaccccgttcgacgcggcgcaggacctggccgacgctcctcgcgtcgccacaagccggcgcccgcgcgacgccgcgaccctgatcctgctagacggcgaccgggtgctgatgggccgccgcgcacccggccacgtcttcatgccgtcaaaatgggtgtttcccggcggacgactggaccgcgccgacttcaccgcagctgcgacgggacagccggacagccggacagccgctctgctggacgcccagatgcctgcccgccgcgggcgcgccctgatgttgactgcggtgcgcgagacgtttgaggaaacgggccttgcgctcgggacgcccgccccgcccgcgtcggtcgccggtccctggcggacctatcgacaggccggcgccctgcccgacctgtcggccctgacctatgtggcgcgcgcaatcacgccgcccggcagggcgcgtcgcttcgacgcccgcttcttcaccgcccgggcctcaagcctgctgcgtccagaggcgagcgagggctgcggcgaactggacgagatcgcctgggtgtcgctggatgaagccgagcggctggacctgcccgccatcacccgtttcgtgctggccgaggtgcgcgcacgattgacggattccgcccttccgccgcctttcgtgcggatggtgcgcgggcgacacctggtcacccgcgcctgatcccgatcagtagaatatcttgcggaagttgatgcggaaggcgcggcccaccggctccagatagtcctcctgatagttcagcggcgtggtcccgtcgctggaggtcacctcggtgcggctgtcgaacaggttggtgacgccgaagccgaggcgcgatcccttcaggaacgggaaccgctccaccagcgaggtgcgcgagcccaggtcggcgaaggtgaacaggttcaccgtggtccggtccgagaactccaggtctggacttccggccagatcgccgaacacccgcgtcgactcacgccagttggcgttcaaaaaggcgccgaagccgttcttgaaggccccggtctgcagctgcagctcgttccggggctggccgccgctgctgacgatcgagtcgccgtccagcaggtcgagcggctccagaccgtcgcggatcgtcacctcgtcctggattcgcatgatgtgcgtcacggacaggttgaacacgccctgccccggctgcgcgcccgaaccgccacgacgacgtccaccggggccgcccggaccaccgcctggaccgccgaaggtgatcgtggtcccgccgccgggacgtccgcccgggcctcgcgcgcctggccccccagggttgccctgccctggcgcggcctgtggcgtcggctgaccgaacgggcgcgagaagttaaagccccattggacctcctgccgctcgatcttctcgtagttcaacgcccgtgcgtcgatggacagcaggttgccgccggcatcgcgcacaaaccgctccggcagggcggcctcgaggtcagcggtgatggtcggaaacgtggcgatggagtcgtcgatctcggtgcgggtgtaggctgcgttcagccggaaatcgacgctggtccacggcgtgtagttcagccccagcttcagcgtgcgcttgtgctcggcctccaggttcggatcgccgccggtgatgcggatcacgtccaccgtctcgccggtgcggaagtcgaacaccggcgtgttgggcgtcagttcggtggggtcgttcagctgctgcactgacggcgcgttcttttcgtcggtgtagctgacgttgaagttcagcggatcgatcggcgaccagtttacgccgccgccgaccgtcggcaggccgccaaagtccgacacctcctgatacgccacgttgaagttggcgcgcaggtcgcccagcaggctggggttctcctcgtctcgctggaacagcggcacgtcgacattggcctggacgttgccgaggttgcgcgacagcgagcgctcgctgaacacccccgagcgggtgctttccgagtccagcgtcagccgccgatagccgccggtgatcgtggtccggacatcgcccgccggcagggtgaagggcgagccggtgaacaccagttcggtgttcagcgtgcctgcgacggaccgggccgtgtcgaacgggatcgccgtgaccgctccgccgatgtcgccgaacggattggcggtcgagctgttcgcatccagcagcgcctgcagggccgccgcatcgacgcctcggccggtgcgcgactccgtctccacccggtcgtagccgccggtcgccgtccagcgccagtcgccgacgtagccgtccagcaccgtcgccacattggccgtgcgcgcgtcgctttcgcgcctcagcgcctcgggctgatccacatagcgatggaccagcacgtccgtcccgaacggcgagaagggattgtccgcatccaggttcaggctgacgcccggcaggcccaggtagctttcgctgtcgaggtcctccaggttgacgctgacggtcgcgcccacctgctcgttcaggtcgcgcttcagcgtgcccgacagctcgatctgctcgcgctgcggcgtcagggtgcgccaggccgagacgtcgccgttgcggacgatccccgcgccttgcgtgaagtcctgcagcgtcacgccgcccgctcccgccggcacggcggccacggtgacgacgccgcccgccagggccgacagcgccgggtcgatctctgcgtcctgagacaggccggtgacgttgccgacaaggtcgaacggcgcaccgcccagcgtgcggtcgatgtcgcgctcgctttcgaagatggcgctgtcgcgttcgtggttcaggtcgaacgaccagcgtgtgccgccctcgatgcgcagcacattgttctcgaactcggtggacgaacgccccctttgcgtcggcgcgccatattccacctgggtggtcagcgagcggaagttcgccttcagcacgatgttcaccacccgctggtcggcgcggtagccgtaggacagcgcggtctcctccggcaggatgtcgaagcggtcgatggcctctggcggcaggccccggatctcctgaaagcccgagatgcggcgtccgttgaccaggaacacaggcgagccgccccgcgcgctgcgggtctggctctccagcagcgtcaccagttccccgatgctggaggcgccaaaggcctgaagctgggtcgagtcgaacgaggcgatcggctcctgcccgcccagcgccactccgcgcggcgtgggcgcggtgaccagcacctcgcccaggtcatagacctcgtcgtcctgggtcgtcgtggatggctgaggctgagtctgggccagctgcaccacgggcgcgagggcgagcagaagaagggcggcggtcatgaaggcgtccgtctgggggagaaacagatgttcgtgctaacggtgggcggcgggatttccgtcgtgacttctttgtaacctctgcggcctcttgcgggcaggcgggcggccgttgactttgcggcgcgcctgagtatgttccgcgcctctcgtttccagcggctttcgccgtcgcaaaggtaattgtccgatggccaaaccggcttccatcaaaatccgcctgaactcgaccgccgacaccggcttcttctacgtcaccaagaagaacgcccgcaccatgaccgagaagatggtcgtcaagaagtacgaccccgtcgtgcgcaagcacgtcgagttcaaggaaggcaagatcaagtaagacggcgttcgcctctacgatcttttagcgcccggctggatcgccagccgggcgttttgctgtgcgccgatgatcaggcggcgcgcgcgatcaccgtgttccggccagcggccttggcctgatagacgccttcgtcggcgcgtttcagcaagccgtccggcgtatcgccgaacgtcgtcgccgcgacgccgatggagatggtgacggtcagatgctcggcgccgcccatgacgcggaaaggcgccgaggccacgtcgcgacggatgcgttcggccacgcggtgcgcgtcgtccagcgacgcccccggcatcaccaccacgaactcctcgccgcccatacggcacggcaggtcgatggcgcgcacatttgtggccaggcgcaccgcgaactcgcgcagcacctcgtcgcccgcatcgtggccgaaaccgtcgttgacggccttgaagtggtcgatgtccagcaccagcaccgcgaccgacgacccgccgtggctggcccgcccgaccagcgcctgcagctgtccggtcatgtagcggcgattatgcagccctgtcagcgggtcggtgaccgccatctccaggctggaatccagcttttctcgcaggaagtcgctgtagcgcttgcggcggatctgggtgcgggcgcgcgcagccagctcctgcggatctacgggacggggcaggatgtcgtgggcgcccagctccagcgccttcaccatgcgcggccggtcgccgggatcgatcaccgccaggatcggcgcgcgacgcgccgatgcgcccgacttggccttggcgatcacgcgcaggccgtcgaagtcgtgagccgcgacattgacgatgatcaggtcgataggtccggccgccgccagcagcgccgcctccggatcgctctcgatcgtcggtcgatgctcggccgacagctccgccgccatgcggtcggccggcgacggtcgtcgtcgacgatcatcacccgcccgcccgcgccccgcagccgtgccgagccctcgccctgaacgcccagcctgcgtccgctttcctcgcgttcgcgcagttcgtccatgacctgcttcagccgcgtcagcgacttgacgcgcgcgaacaggatcacgtcgtccagcggcttggtgacgaagtcgtcggcgccggcctcgagccccttcagccgatcctcgcgtccgtccagcgcggtgaccagcaccaccggaatatgccgggtggatgcatccgccttcagccgccggcaggtctcgaacccgtccatgcccggcatcatgacgtccagcaggatcaggtccggctggtgttcggccgcgatcgccagcgcggtcatgccgtcgccgcacgtcagtacgtcatagtattccagcgtcagcttggcctcgagcagccggacgttggtgtccaggtcatcgaccaccaggatgcgcgcgctcattgcaggtgcttcctgacggtgtcgaggaagtgcatcaccgagatcggcttggagatgtaggcctcgcacccgccctggcgaattcgctcctcgtcgcccttcatggcgaaggcggtgacggcgatgaccgggatgtggttcagctcgtcgtcgtccttcagccacttggtgacctccagcccggagatctccggcagctggatgtccatcaggatcaggtccgggtgatgctggcgggcgagcgcccgcgcctgcagaccctcgcgggtctgcagcgtccgatagccctgggagtcgagcagatcatgaaagagcttcatgttcagctcgttatcctcgacgatgaggacggtcttggacatcatcaccctgatactggtccaccgcgcgtcgcgtgagaccttgtcgccttcgttgacgccagcatgacggaggggtcttaagctggggtgaagcccgcctgacggagagcaacgacgtggccatcaaggccatctgccgcgactgcctgtggaccggcgcggaccccgcggggccgccggatcgccgctgcccgtcgtgcggctctcgtcgcgtcgtcgcggacgccgagctggatcagctgtccatcgcccacctcgactgcgacgccttctacgcctcggtggagaagcgcgaccgaccggagttgcgcgacaagccggtgatcatcggcggcggcaagcggggcgtggtctccaccgcttgctatgtcgcgcgcctgtacggggtgggctcggccatgccgatgttcaaggcgttgaaggcctgccccgacgccgtggtcatcaagccggacttctccaaatacgttgtggagtcccgccgcatcctgggcgccctcgccgagctgacgcccctgatccagaccctgtcgctggacgaggcctgggtcgatctttcaggcaccgaacggctgaacggcggccctcctgcgcttcagctgatccgtctgcagcagcgcatcgaggcggagaccggcctgaccgtctccatcggcctggcgcccaaccgcttcctggccaagatggcgtccgagatggacaaaccgcgcggcttttccgtcatcggccgcgccaatgcgcaacggttgctcgcgccccggccggtcaccgccctgccgggcgtcggccccgtcttcggcaagagcctgcgcagcgacggctatgcgaccatcggcgacctggcccgcgcggacgtgcgcgaccttgtccgtcgctacggcgaatcgggcctgcgcctgcacgagctgtcgcacgcccgcgacgcccggccggtgaacccggaccgcgaccgcaagggcatgagcgccgaaaccaccttcaacgaggacctgacgagcgccgccgacctggaggccgagctgtggccgctgtgcgagaagctggcgtccaaggcccgccaagacggcgtggccagccgcgtgctggtgctgaagctgcggcgcaccgacttccgcatcgtcacccgccgcatttcgctgccggagccggttcagaccgcccgcgccctgttcgccgccgggcgcgagttgctgaagcccgaactcggccgtccctaccgcctgatcggcatcggcatggccgaggtccaggatgcggaggacgcgcccgccggcctgttcgccacgcccgaggcccgtgcgctgaagaccgagaccgccatcgacgccctgcgcgcccgcttcggcgccgacgctgtggtggccggacgcgtggtggcgccgcgcaaggagaagccctctcgatgaccgacctcgcccgccgcgcctacgaccacgcctggcggctcgatccgatcgtgcgcagcctgctggacaccgacttctacaagctgctgatgcttcagctgatctggcgcgaacaccgcgatgtgcgggtgaagctccaggtcatcaaccgcacccgctccgtccggctggcggacgagatcgacatcggcgcgctgcgcgaacagctggatcacgcccgcacgatcggcctgggcaagcgcgaacacgtctggctcgccggcaacaccttctatggggtcagatcgatcttctcgccggacttcctggcctggctcgccgactaccgcctgcccgactatcggctggaagtccgcgacggacagatcgacctttcgttcgaaggcccttgggccgaggtgacgctgtgggagatcccggccctgtcgatcgtcaacgaactgcgctgccgaaccgcgctcaaccggctgggccggttcgagctggacgtgctctacgcccgcgccaagccccggctgtgggacaaggtcgagcggctgcgcgccctgcccgacctgcggctgtccgactttggcacccgccggcggcacggcttcctttggcaggagtggtgcatttcggcgttgaaggaaggcttgggatcggccttcgtcggctcgtcgaacgtgctgctggcgatgaaccacgacctggaggcgatcggcaccaacggtcatgagctgcccatggtcctggccgcgctcgcgcccgacgacgacgccttgcgcgccgtcccttaccaggtgctggaccagtggcgtcagcactacgccggcaacctcctggtggccctgcccgacgccttcggcaccgaagcctttctggaccaggcgcccgactgggtcgcggactggaccggctttcgccccgactcctcgccgccgctggaggccggcgagcgcctgatccgctggtggaccgagcgtgggcgcgatccgcgagacaagctcctgatcttctccgacggcatggacgtggacagcatcgaaacaacgcacgcgcgcttccacggtcgcgctcgtctcagctacggttggggcaccaatctgaccaacgacttccacggctgctcaccggcgcccgcgcgcgaactcgatcccatctcgcttgtgtgcaaggtcgcctcggcgaatggacgcccggccgtcaagctgtcggacaatccggccaaggccgtcggcgaccccgacgagatcgcccgttatctgcgcgtcttcggccagcgcggccacagccgtcaccccgtcgtggtctgaagcttcagccggccttaacggcggccgtgcaggatggcggcatgagcgcctttatcgacaagatgcgccgccgcgccggccgctacctcgatgtgcggccggtcgccgtccggccttcgcgcggaaccttgagcctgtcgttcgacgacatccccgaaagcgcctggaccgaggccggtccggtgctggacgcccatggggtcaaggcgacctactacgtctgcggcgggctggagcgcgggatcaacctcggccttcggcagttcaccacagaacaccttcaggcgctgttcgccgccgggcacgaggtcggctgccataccttcggccacgtctcgaccctcaccctgtcgcctgccgagctcgaggccgatctcgcccgcaacgccgcctgggtcgccgagcggctggacggccacgtcatgaccaccttcgcctatcccttcggcgactgcgccctgacgtccaagacggtgatcgacggacggttcctgtgcggacgcggcgtacgcgacggggtcaatgtcggccgcgccgatcgcgccctgctgcaggccatcggcctggagtcccgccgcctgcccggctacgatctcgaggcgctggtgcagcaagccgccgaccagaaggggtggctgatcgcctatggccacgacgtcggcgatcgccccacgccctatggctgcacagtcgcggacctggatcgtctgctaaccctggcgaaggcggccgacctggacattcagcccgtcgcacgggcctggagccgcatggcctagaagacgccgactgcgccgtccgcccagatcagcagcaccgccgcgatcaccgcaagcgccagccccgccctgagcgcggcccctcgcgccttccacaggatcagctccagcagtaggcccgcaccgatcagaagcacggcggcaaaggcgaagtcgaatgcggtccagtttacctcgtcggtgaagcgcatggcgatcagaggcgccagcagcaccagcgcgaccccgctccaacccgccgtccggatcaggttggcttttccatgaagtctcgccgcatccgtcatcgcattctccccgtccggagttcagaacaatgatacgccgaagtcatgcgcgtgaggagacgcctcggagttccaaccttcctcgtcatcagaccctatacgtcgcattgctgcttcgcagagccctgtgtttttgctaaacagtcgctaccccctggcttgtgccactcagtcctgcttgcgcagggtgagtcacgcttattccgaagttacgcgtgcaatttgccgagttccttcagcatagttctctcaaacgccttggtatgctctacctgaccacctgtgtcggtttcgggtacggtctctgctggagttatttccagggacaacgcccccgcacgcacaatccaataagtgcgtacgagttatgccatccgtcacttccagctggtgcaggaatatttacctgcttcccatcgactacgcttttcagcctcgccttaggggccgactaaccctgcgcagattagctttacgcaggaacccttggtctttcggcgggagtgtctctcacactcctatcgttactcatgtcagcattctcacttccgatacctccagccaggctcacgcctgaccttcactggcttacggaacgctccgcccttgtggggaggattcagcctcccgaacctcgccggatgagcccgagcggatccaaggcccaaggcctaggatgacgatggaggggaacgtcgcccctccgcccacgcgatcagcggctttctcggccacaccatcagccatgaccgggcgacgtattcgccgctgtcgatcatccgcttgcgcgtcggagaggcggtcgccgcccgctccgtgtggatctcgcccggtccccgatggaccatgaaggccccgccgttcagcggattcagccgcaggtgcgcgaggcgcgggctgatctccgtcagcgggggatcgtagaaccagctggagccgatcatgccgcccagctccggccgcgcctggcagatcgccgccgccgtcgcccaggcccggttccagccgttttcgttgaagtcggcgagccagcgcgcctcggtgtgcgcctccagccaggtcttcctccatccctgtgcggcgacatagcggaccaacgcgcccatcccatgcccctcgcgcgcatgccgcaccacctgtcccggtcccatgggcgaggtcaggtcgatcacctgcgaccgcgcccctggcacgctcagcgccagcgcgaaccgcacatccttggcccagtggtcgcggtcataggcctgaccttccgcaccgaccaggaactcggccagccgctcgagccaccagggatagagcgtcatcacctcgtctggcatccgcaacgccgccgcacgttccggcaagccgagcgcccagaaggcgatcagcccacgcttcatctcgtcggatgcgcctgcgcccaatacggtgtccaccgccttggccggcgcttcgaagtcccagtgcggtgcggcctccgcggcgccttcggcggcgggtcctgcggcggcctcaacgcgcgtccgatcatcgggcgacagccgcgcgagcacggtctgaaaggcggtggcgggcgtgacctggggcatgtccatgaccggcatcctagcttacgccggttggcgaacctttaagcgcgcccccggatgacgccgccgcgcgcccgcgctaaaccccgctcaaacaccgcaagaggaccaatctcatgagcatcgacgcccgcctcgccgaactcggcatcgacctgccgaccccggccgttcccgtcgccaactacgtctcctttgttcagacgggaaacctggtccacatctcgggtcagctgtcgaacgacgcctccggcgggatcaagggcacggtcggcgtggacgtttcgccggaacaggccaacgccgccgcccggctgtgcgccatcaacctgatggcccagatgaaggtcgcctgcgacggcgacctgtcgcgcgtcgtgcgggtggtcaagctgggcggctttgtccaggccgggccggacttcacggccatccccggcgtcatcaacggctgctcggacctgatggtcgaggtgttcggcgacgccggccgccacgcccgctcggccgtcggcgtctacaagctgccgctcggcttcgccgtcgaggtggacgcgatcgtggagatccgttgaccttcaccctgacggtccacgaccggatcgccgacatcggccgggaggcgtgggacgcctgcgcctcccccaccggcgatccgttcgtctccttcgactttctgcacgcctgcgaggcgtcgctgtccgccgcgccgcgccagggttgggccccgcggcacttggcgctgcgcgacgagactgacgccgtcctcggtgtcatgcccctctacctcaagggcaacagccaaggcgaatacgtcttcgatcacagctgggccgacgcctatgagcgcgccggcggccgctactatcccaagctactgggcgcggtgcccttcacgcccgcgaccggcccgcgcttcctgtcgcacgcgtccgccgaccacccgacggtgcgcgaggccctgctgcaaggcgccctcaccctggtgcagcggctcggcgtctcctccctgcacgtcaactttccgacccgcgacgactggaccgcgacgacgcaggccggcctgctgccgcgccaggacatgcagttcatctggcgcaacaacggctaccggaccttcgacgacttcctggccgccctgtcctcgaaccgtcgcaagaccatccgccgcgagcggcgcgacgcccaggccgggctcgacatccgcatcctcaccggcgccgggatcgaagaagcgcactgggacgcctttttcgccttctacatggacacgggctcgcgcaagtggggccgcccctatctgacccgcgacttcttcacccgcgtgggcgccaccatgagcgagcgcatcgcgctggtgatggcgttccgggacgacacgcccatcgcaggcgccctcaacttcatcggccgcgacgccctctacggccgccaatggggcgcgctcgaggacgtgccgttcctgcatttcgagctctgctactatcaggcgatcgacttcgccatcgcgcgcgggctggcccgcgtcgaggcgggagcgcagggcgagcacaagatcgcgcgcggctacctgccctcgtcggtctactccgcccacttcatcgccgacccggcgctgcgcgagcccgtcgcccgctatctggaaggcgaaggcccggcgggggagggcgagatcgccgccctgacccaggctcagtcgccctaccgcccggcctagcagccgatcgccgcgacatggaagcttggccggaaccgacggccggttcgcgcgctgtgagcgcatctccccgcacgcaagcgagcaccgctcgaaaggacatatccatgaccgaccaacgcatcgaaggcacggccaccgagatcggcggcaaggttcaaggcggcctcggcgacctgaccggcgactccaagcttcaggccgaaggcaagttcaacgagatcaagggcaaggccaaggactactacggccaggccgtcgacaagctggagaccctcgtcgacaaggctccggtccagtatcaggacaaggctcgcgccggcgtcgatttcgcccgcaacaagcccctgctgaccaccggcatcgtcgccggcctggccctgatcctgtcgcgcgccggccgtcgccgctaagccgggaatcagtccgatcgttcaagccgccgtcccctccggggcggcggctttttctgtgtgtcgacatcgccggacatgcagcgagtctgcagagttcattgacttgagttcagacgttgatgatccttgagaagggggatcagacatgcttcgcaaggtcttactgtgtgcggcgaccgcaaccgtgtgcgggatttcagcggcgccatctcatgcgcaggacagccaagccagctggcgtgttgttccatcggctcagatgactgactatccggccttcgctcaggagtttgggttctccgggcgaacagcattggaatgcattcacgacccggccggagtcgttcggacgtgcgaggtgctttccgaagttccggaggggctcggtttcggggctgcggctgtgagcgtggtgcggcgaggcagtgtgaatccacccaccgagaatggcgttcccgtgggcgcgaggttcaccgtgcggatacccttcaacatgatgggagaaacgcctgagttcaggccttggcagggtcccgagccagacgccgcgagcatcgccctggcggaacagttcatcgcagcaatgggtcctcttccgcccatgtacgatcctgcagccctggaaagcctgacgccggatcgccgcaaaatcgtccccgggttcgtggaggaggcgtttccgtcacagcaggagatgggccgcatcgcggctcgaggcatggctcgcatctttcccgccacagccctcaagtcgatgatggaaggacgctcgccgtccgaagacgatatccgcgcgatcaacaaggccggccctcaagtcattggcggcttgttcgacgtcgcagccgccaacgccgaggtgcgttcgcgatactgcgcccgcttccactgcggcgacgcaccgcaataagaaaacgccggacccgcttccgggcccggcgttcgaaaacggctgatcaggccgtttcttcttcctcttccttcgccggagcgccgctggcgcccttgatgtcgaagtcgatcttgccgtccttcagctggaccttgacgtgtccgccgccggtcaggcggccgaacaggatgtcgtcggccagcggcttcttgatcgcatcctggatgacccgcgccagcgggcgcgcgccgtacagttcgtcgaagccgttcttggccagccagtcggccgcttcgtccgtcagttcgatggtgatgttacggtccgccagctgggcctccaactgcagcacgaacttggtcaccaccgaacggatggtctcggcgcccagcggcttgaaggccacgatggcgtccaggcggttgcggaactccggcgcgaacaggcgctggatggccttgtcgtcctcgccctcgaccttgccgcggccgaagccgatggaggcgcgtgcgttgtcggcggcgccggcgttggtggtcatgatcaggatgacgttcctgaagtcgaccttcttgcccaccgcatccgtcagcattccgttgtccatgacctggagcaggatgttgtagatgtccgggtgcgccttctcgatctcgtcgagcaggatcaccgcgtgcgggtgctggtccaccgcatcggtcagcaggccgccctggtcatggccgacatagcccggaggcgcgccgatcaggcggctgaccgtgtgacgctccatgtattcggacatgtcgaagcgctgcatctcgatgccgagggtggaagccagctgcttggccacctccgtcttgccgacgccggtcgggcccgagaacaggaacgagccgatcggcttgttcgggtcgcgcaggcccgcccgcgcaagcttcatcgccgccgagacctgctcgatggcctgctcctggccgaagacgacgcggttcaggtcggactgcagctccttcaggctctcagtatcggatttggacaccgacttgggcgggatgcgggccatcttggcgacgacggcctcgacctccttctggccgatgacctttttccgcttggattcgaccaccagcatctgcgaggcgccggcctcgtcgatgacgtcgatcgccttgtccggcagcttgcggtcggacatgtagcgggccgacagctccaccgcagtacggatcgcgctgtcggtgtagcggaccttgtggtgctgctcgtagtaggtcttcagccccttcaggatcttcaccgagtcctcgaccgtcggctcgttgacgtcgatcttctggaaccgccgcaccagggcgcggtccttttcgaagtgctggcggtactccttgtaggtggtcgagcccatgcagcgcagcgaccccgacgccagcgccggcttcagcaggttggaggcgtccatcgccccgccgctggtcgcgcctgcgccgatcaccgtgtggatctcgtcaatgaagagcacggcgttgtcgtggttctccagttccttgaccacctgcttcagccgctcctcgaagtcgccgcgatagcgggtgccggccagcagcgcgcccatgtccagcgagtagatggtggcgtccttgaggacgtccggcacctctccgttgacgatcttgcgggccaggccttccgcgatcgcggtcttgccgacgcccggatcaccgaccagcagcggattgttcttggtgcggcggcacaggatctggatcgagcgttcgacctcagcctggcgaccgatcagaggatcgaccttgccctggcgcgacttctcgttgaggtcgacgcaataggcctccagcgcctctccgcccgacttggcggcggccgcatcctcgacctcttcgggcgaagcgcccttggccggcttggcttccgacgcgcccgccttcttggcgatcccgtgggcgatgtagttcaccgcatcatagcgcgtcatgtcctgctcttgcaggaagtaggccgcgtggctctcccgttcggagaagatggcgaccagcacgttcgcgccggacacctcttcgcggccggaggactggacgtggatcaccgcgcgctggatcacgcgctggaagccggcggtcggcttggcgtcctcgccggccgaggtggccagcgccgccaggtcgttgtcgacataaagcgtcagcgccgtcttcagcgcggcgaggtcgacgttgcaggcgcccatcacgccggacgcgtccggatcgtcgatcagcgccagcagcaggtgttcaagggttgcgtactcatgccggcgctcgttggcgaagccgacggcgcggtgcagggtttcttcgagaggacgcgaaaacgagggcattgggggaggttcctctcagtccttttccatcgtgcattgtagcggatgctggtgacgtctcgccgtctccaccacctgggcgaccttggtttcggccacttcgtaggtgaacacgccgcacaccccgaccccatgctggtgcacatgcagcatgatgcgggtggcgtcctcgcggctcttctggaagaaccgctccagcacatagatgacgaactccatcggcgtgtagtcgtcgttcaggatcagcacccgatacagcgagggcttctgaagtttcggcttggtttcggtgaccgttgcggcgccttggccgccgccgcgctcaccgggcctttggatgggcattcgtgttccgtcgtggggagatcgtcttgaggctcaagatagggattgatgccccgatttgaaggcgcgtccagtcacagcttgcgtgagggccgcaggttccgcgccctctcccaaaaaagccgcacttggcttgaagaagcctgacgacgttctgcgggtaacaactccgttgacggctcgttaaccaccgcgaaacccctgcttctcatggtatgggccagttcagcgtcaggccggggggccccgccgccctcttgtctcagaggttccttgagttcgcccatgatcgccagtcttcgtcgcgctcttgtcttccttctcaccgtgggcctgctcagcgcgggtcccgccagcatcggctcggtggacaccggcttcggcgccgcgccgctgcgggcccaaagctctgaaaacagcaaatacgccgccatcgtcgtggacgcgtccacgggagaggtgctgttcgaccgttttgcggacgcccggcgctacccggcctccaccaccaagatgatgaccctgtacctgacgttcgaggcgctggagcagggcaaggtgcggctggacgacgtgctgaccgtcacctcgcacgcggcctcgcagccgccctccaagctggggctgggcgcaggccagtcgatcaccctagacaacgccatgcgcgccaccgccgttcgttccgccaacgacatggccgtggcgctggccgaacacatcggcgggggctccgagagccgcttcaccgccatgatgacgctgaaggcgcaggagctgggcatgacccagacccgctacgtcaacgccaacggcctgccggacggacgtcaggtcacctcggcccgcgacctgtcgatcctggcgcgcgccatcatgcgcgattatccgcagtactaccgctatttcggcctgcacgactgggcctacaacggccgcgactaccgcaacaccaacgggctgctggccacgggtcgcggctacgacggcatgaagacgggctacatcaacgcctcgggctacaacctggtggcctccgcggtccgcgacgggcgccgcatcatcaccgtggtgcttggcggccgttccagcgccagccgcaacgcacatgtcgcggaactgatggacaccggcttcgagctggagcgccggcgcgaggccggagagcgcatccaaatcgcccagaccttctttgaacagcgcggcttcggcctcggctcggcggccgcggacgacgcgcccatcgcctacgcctcagcgtcggacgaggacggcggcgtcccggcgaacgccgtggcctatacggccgcccccgcgccgacagtgcggccgacgctggtggccgacgccggctcgaccgcccgcgcctggacgccgtccgccccgcgtccggctccggcgccggttcaggcccaatccccggctcagcctcagacccagacggcgcctcgcgtcgcagagacgcgcgctgcatcgacgacgcggacgcccgcgcctcgcgcctcctcttcggctccgcgaaacgtgaccgcgtccctgaacggagcgcctcccggcgccgccgtcgcgccatccaccacgccgcgacgcccgcccgcctccacgacctccgcgcctgcgccccgcgcccccgccggtcgctgggccgtgcaggtcggcgccttcaaggaacaggatgtcgcgcgcgactggctgacggaggtgaaccgccgcttccgcgctcagttcgcctcggctgagcagacggtggacaacgccggcggctggtatcgctcgcgcttcaccaacctgtccgaagccggcgcccagtccgcctgcgccgccctggccgagcgccgcgtcacctgcatggtcatccgtccgagctgagcgcaggcggcttcagggcgccctcaacgaggacaccgcgccgccgcctcgacctgtgggcgcagcacgctcatgaccgccagtggagcgtcggtggcgatgacggacacgccctgctccaccagcgtccggtattccgacacgtcgccgtccgccgcatagacgtcgtccagccgacgaccttcggcgcccagcgtgccgaactgcgcctccacccccgcatccttcaacgcccgccacagcgccgggcgcgcttcgcgtgatccggtccaggccaaaatctgcggggcgtgcagcccgtccagcccagtcagatcgctcagccccgccgacaccatcatttcgggggcaagggtcgagaccgcccgcgcgtcgtccgcggaataggtgatcaggatcccccggccctgtgcgcccgtgcgccgcacctcgtccacaaccgcgcgggccagcgtcagggtgtcggccgggtccgcgggcttcaggtcgatgctggcgatcgcgcccaccgcccccgccgcctccagcgcctcggccagcgtcggcggcgcggcgtccgtcagccggccatcgctgccgcgcaggcgcacggccttgacctgatcaagcgtcaggtcggcgaccttgccgcgcccggtggtggtccgatccagcgtctcgtcgtgcatcagcaccagttcgccgtcccgggtcagcacggcgtccagctccaggatcgcgcccgggatcgcccgtccggtcgcccggatcgccgcgatcgaattctccggctgatccggcgccgacaccgcccgatgcgccgagacggccacgccgcgctcgcgcacgcagtcgaagtatccggccaggatcggaccgtcgcccgcgcccggcgcccccacgcccgcgcaggccgtcagcggcagggccgccgtcaggatcagacccagagtgcgggaaagggtgcgggactgggcccgggactgggcgcgggtcggggtatgaactgggcgcatgaagacctccgtcgtcgcgcccccatatccgtcggcgcgcctggagaacagcccttggggatcggcccttgccgccgggtcgccggcgacgcaccttgcggcccacgacagcgaaaggcgaatcaaggtgcaggatctggcgggaccggccatcgggaccttggcccttgttgcggccgcgggctacctgctgggctccatccccttcggcgtggtgatcacgcgcgccgccggcgccggcgacgtgcgccggatcggctcgggcaacatcggcgcgaccaatgtcctgcgcaccgggcgcaaggacctggcgctggcgaccctgctgctggacgcaggcaagggcgccgtcgccctgctgctcgcccgccaccttctcaacagcgagacggccggggccatcgcgggcggagcggcctttctgggccacctgtttcccgtctggctcggcttcaagggcggcaagggcgtggccaccttctttggcctgctgatcgccgcctgctggccgctgggactgatggcgggcgccgtgtggatcgcgaccgcctttctgttccgcatctcctcgctgggcgcgctggtcgcttcggtggccgcaccgctgatcgcgctggttccctggcccgcggccggcctgcccgcggcgcagcctgtgctggtcctggcgatcgtgaccgccatactgatctggatccgccatcacgagaacatcgaccgcctgctcaagggcaccgaaccccggatcggcggaaacaaggcgtgaggctggcgggcgaggagcgcttcgcccggctgcggctcgctcggaccgaccgcgtcggtcccgtcgccttttcccagctgctggcgcgacacggctcggcgctggccgcgctcgacgccttgccccagatcgtgcgccgctcgggcggctcgctgacgccgcctgcgcccgagcgcatcgagaccgagttgacggcgggcgagcgcatcggcgcgcggcttctggtcctgggcgatcctgactacccggccgccctcgccgcccttgatccgcccccgcctgtcctgtgggcgcgaggcgatgcgacgctgctgaaccggccgtgcatcgccgtggtcggcgcccgcatcgcctcggcgggcggccagcgcctggcgcgcggactggcgcagcaactcggccaggccggccacgtcgtggtctcgggtctcgcccgcggcatcgacggcgccgcgcatgaaggcgccctgcccaccggcacggtcgccgtcctcggcggcggcgtcgacgacatctatccgcccgaccaccgcgatctctacgcccgcatcgccgatcagggctgcatcgtctccgaaagcgcggtcggagcccgcgcccaggcccgcgatttcccgcgccgcaaccgcatcatctccggcctgtcgcgcggggtggtggtggtcgaggccgaggttcgctcgggctcgctgatcacagcgcgcctcgccgccgaacagggacgcgaggttttcgccgtgcccggctcgccgctcgatccccgctcccgcggtcccaatgaactgatccggcagggcgccgtcctgtgcgaaggaatcgaggacatcacgcgcgccttctccggcctgcggaccctggcggagcccgacatgccgccgcctgtcctcgacgaggcgttcgatccggcgctgctggagcgggtcgccgccctgctctcgcccacgcccacgccgcgcgacgaactggcgcgcgctctcggagctccgatcgcacaggtggctggagcgttgctggagctcagcctgaccgggcgagccgaactgcttccgggcggtttggcgtcgctatagccgaggcggctgttccctcgcgccgcgccgggctgactgggccgactcgccagatcggccgccgcttccagcaaacaggccagccgctcgtccccgtcccaccgggccatgcgcgccagttctccagccatcgcgccgacgtattcgcgcactggatagtcctggcttatgggattgggctgactcgtcgctgcgcccgcgtcaggctcgttttcttggtggtggtgcagctgtgaacccatctcgccctctcttcaggagagatcagtggacacaatctaagcgtgctaatcaagcaggttggtaaccggtggttatccgcaacagccggtcattgacttaacgcccgccgccaaccacgttcgcgccccttccagagaccgcgcacatgaacctcgtcatcgtcgaaagccccgccaaggccaagaccatcaacaagtacctcggctccgattacgaggtcctggcctcctacgggcacgtccgcgacctgccgtcgaaggacggctcggtcctgcccgacgacgacttctctatgcactgggaggccgacgccaagggcgccaagcgcctgtccgacatcgccgcggccgccaagcgcgccgaccgcgtcatcctggccaccgaccccgaccgcgaaggcgaggccatcagctggcacgtgctggaggtgctgaacaagaaaaaggcgctcaaggacacgccggtggagcgcgtcacctttaacgccatcaccaagtcggcggttctcgacgccatggccaatccgcgccagctcgacatggagttggtcgaggcctacctcgcccgccgcgcgctggactatctggtcggcttcaacctgtcgccggtgctgtggcgcaagctgccgggcgcccgctcggccggccgcgtgcagtcggtggcgctgcgcatcgtcgtcgaccgcgagatggagatcgagcggttcaagccgcaggaatactggtcgatcgaggccgacctccacgccgacagcccgcctttcaccgcccgcctggtcaagcacgatggcaagcgcatccagcgcctcgacatcaaggatgaggcgaccgcctcggtcgcccgcgccgccatcgacgccggcgacttcaccatccggtcggtcgagaagaagcccgtccgccgcaaccccgccccgcccttcaccacctcgaccctgcagcaggaagcagcccgcaagctcggcttctcggcccagcgcaccatgcaggcggcgcagaagctgtacgagggcgtggacgagaccggcggcctgatcacctacatgcggaccgacggcgtccagaccacgcccgaaggcatcgcccaggcgcgcgaggtgatcagccagcagttcggccccgccttcgtgccgggcgagccccgctactacaagaccaaggccaagaacgcccaggaggcgcacgaggcgatccgcccgaccaacatcgcgcgccaccccgacagcctgcggctggaatccgacctgcagcgcctctacgagctgatctggaagcgcatggtcgcctcccagatggaggccgcgcggctcgaccggaccaccgtcgacatcgagacgtcggacggccgcacaggcctgcgcgccaccggccaggtggtgacctttgacggcttcctcgccgtctatgaggaaggccgcgacgagaagtcccgccagtccgaggacgaggacgacgacaccacccgcctgcccgccctgaaggaaggcgcgcgcgccctggtcgatgcggtgcgcgccgatcagcatttcaccgagccgcccccgcgcttctccgaggccaccttggtcaagaagctggaggagctgggcatcggccgcccctccacctacgcctccaccctgtccaccctgcgcgaccgcgaatacgtgcgcgtcgacaagaaccgcttctaccctgaggacaagggacgcctcgtcaccgccttcttggagcagttcttcaggaagtgggtggagtatgacttcaccgccgcgctggagacccagctggacgaggtgtcagccggcgacctcgactggaaggtgctgttgcgcaacttctggcaggatttccatgccgcgacccaagcggcgggcgagcttcgcaccaccgccatcctggatgcgctgaacgagacgctgggcgctcacatcttcccggacaagggcgacggctccgacccgcgcgaatgcccgctgtgccaccagggccggctgtcgctgaagaccagccgctttggggcctttatcggctgcgaacgctatcccgagtgcaaatacacccgcccggtcgcctcacccgatgcggcggacggcgcggccgacagcggcgaccgcgaattgggcgtcgatccggccaccggccagccggtccacctcaagatcggccgcttcggaccctatgtggaaacgacgccgcccgacgccgagaagccgctgcgctcctccctgcccaagggctggtcgccggcgtcgctgacgctggaaaacgccctgcgccttttgtccctgccgcgcgaggtcgggccgcaccccgaggacggcaagatgatcactgcgggcttgggccgctacgggcccttcatcctgcacgccggcacctacgccaacgtctcggacatcgaggaggtgttcgacgtcggcctgaaccgcgccgtcgccctgctggccgagaagcgtgccggcggcccccgcggccgcggcgcggcccaggcgcctctcaaggacctgggcgtgcatcccgagaccggcgatcccgtccacgtcatggccggccgcttcggtccctacgtgaagtccggcaagatcaacgccaccctgcccaaggacgtaacccccgaggacctgacgctggacgccgccctgccgctcctcgccgcaaaggccgacgccgcgccgaagaagaaggctccagccaagaaggctgcgacgtccaaggccgaaggcaagacaaccgcgcccaagaaaaaggcgccagccaagaagaaggccggcacctgacggcgaccaggcgcgcaccgcacctctccctccctgttcggggagatagctgagccgcaaaggaagccgggtggcggcggccaagcgcccaacggcagtgtggccgagccacgcccgcgccgcgtggccgaggcgcccccagttggccgctgcgcgaccatcctctgcgttcaaaggcccggcgccccgcccgcccatccaaccggatgcatgaacgcaggccggggccttcgcgcgcgttcgaacgcgcggcggacgcttatccagacgggggaagaagcaagaacagcggccgttcgccgctgtggaagatggtaccgcctctcaggcttgaactgaggacctccggctccacaaaccggcgctctaaccaactgagctaaggcggcccgctttcgcgagaggcgttgtctaccggcatgacgcgtccggatcaagcaccgcgcacagggttttgcatcaaaggcgacggcgctcgaaccaaagaaaaaacgccccgcgggctgagcccacgggacgttccatcttgttgacgccagcgcctattggagctggaagcgcacggtgaaccgcgcctgtccgccttgcgccacaccatcgacggtgctcggcgagaagcgcgccgagcgcatcgaccgaagcgcctcctggccgaagccggcgcccgagggcgtctcggagacgacgctgcagttcgacgccgagccgttcgcgccgaccgtgcagagcagggtcaccgatccggcctcgatgccgcggtcctgagcccgttgcgggaactccggagccggacgacgtccccacgacacgttggtcgtgaccgcctggcgcggcggggccgcgggcggagccggaggggccggcggcggcggcggtccggggaccacgaccggagggccggtgtactcctgacgctcgtccttcttcgtcggttcgatatagacc

SEQ ID NO: 6 - DNA, 201526 bp, brevundimonas massiliensis
  source 1..201526: mol_type = genomic DNA
gggttaggcgataagaccgccaccatcctccgccccgagcttgcagcgtaatcatccgcgcggggcgtcagctttcgtcgaaacggtaacctctagtcacactccgggcgaaggcccggcgcccgcccgccctccaaccggatgcgaaagccgcagccggggccttcgcgcgtcaccagtccagccgcgatttgccttccgtcacgacacgccgctaagccagcatcgaacccgtggagagatttcgatggccgcacccgcctccctgctcaagggcctcaccctgccggtgatttcggccccgatgtttctggtctccgggccggatctggtggtcgaggcctgcaacagcgggatcatcggcacctttccctcgctgaaccagcgcaccaccgagggctatcgggagtggctgcgcgacatcaagagccggctgaagcccgaagccgccgcgttcggcgtcaaccacattgttcatccgaccaatccgcgcctgctggcggacctgacggtgtcggtcgaggaacaggttccgctgatcatcacctcgctgggcgcggtgcgcgacgtggtggaggcggtgcacggctacggcggcgtggtgtttcacgacatcgccaacgtgcgtcatgcgcgcaaggcagccgaggccggcgtcgatggcctgatcctggtggcgaacggcgcgggcggccatgccggcgtggtcaacccgttcgccctgatcaacgaggtccgcagcttctatcaggggaccatcatcctgtcgggctgcctgtcgacgggccaggacgtcgccgccgccctgatgatgggcgccgatttcgcctacatgggcacccgcttcatcaacaccgccgaggcgatggcgtcggacggctacaagcagatgatcgtcgattccggtgcaaccgacatcacctacaccccggcggtttcgggcattccggccaacttcatgacccggtcgctgctggaaaacggcatcgaccccaagaccctgcccgagcacaagctggacatgggcgaagaggccaaggcctggaagaccgtctggtcggcgggccagggcgcgggctccatccacgacgtgctgccgacggccgatctcgtgacccgcctgcgacaagaattcgctcaggcgacggaacagttcgcgattcgagcgggcgcgcgttaaaggctccggacatccccatccccgctttcttcgcgagccgtcatgacccgcatcgtccccgccgccctggccctgtctcttcttgcggctccagcctgggcgcaggaggaatcctccagcgactcggcgtcttccgtcggctcgcagggcggctgggccttcagcgtcggtgccggcaccgacaaccggtcgaagaacgcctccaaatccaacggcgatcctttcgtgtcgggcacggcggaatgggaaagccagtccggcttcttctacgccggccccagcttcgagacggtcaagagcaacggcgcggatgtcgagttcaacgccgtggcgggcgcccgcccctattgggccggcttcgatatcgacctcagcgcggtgtacaaggtacgccccggctcggacgacggcgtggacgacgaagagtggcaggtcggcgcaatcgtggaacggtcggttggtcccgcccgggcgctgttgcgcgttgaatatgcgtttgacgccttcggctcgacggactcctacgtctggaccgaggctaaagcgggctgggccttcaccaacagactggaaggcagcgtcgccgtcggcaagcgcgagcagaagggcagtatcgactacgtcggctggaacgtcggcgcgacctacgccctgaccaacgcgctggagcttgatctgcgctactacgacaccgacgccaacagcgaaggcgaacagtacaaggaagccctggtcgccagcgtcaactacgccttctaggcgctgagccgcgaaagaaagcccggcgcgcgataggtcgagcggttcatcaccacgccggggatgcggccgccgaccgcttcgatctcgtcgcgcaggatcgccggaccggacgcggcggtcgtctcggcggcgatcaccagaatgctggcgtccacgaacggggccaggatgatggccatgtcgttgcggtccgccgccggcgtgtcgatcaccaccgtgtccgcgtgcggtctcagggcgtcccagtaatcgggccggccgagcggctcggcccggtgaccggatcgcagcgcctccatgcggaaccgcgtggtccacagccgcccgcccagacacgcccgggcggtcagcagccgatgcgccgggatcgtccgaccctgcgcgtcggtgattcgcggcgtgacggcgaaaaaggtcgaaccgttcggcgaggcctgcaccggcttgctcagggccccgaaccgctccggctcggccgcgatcgcctccagctgcccctgctgggccaggtcgccgtcgatcagccacacgggctttcgcgcccgcaccgccgccagccgcgcatactcccgcgccaccgtggacacgccctcgccggtagaggcgccgacgaactggatgatgcgggcgcggtgcgccggggccggccccagcgccgcccacaaccccgccatctcgcccgtcagatcgaccatgctgctcagtgcgccttggccggcgcgaccgccagcaccggcatgtccagcgtacggctgaccgacccggccgtcgagaagccgcggcgggagaagatgcgcaggaggccggcgcacagggcggtgaaggcggcgaacaggaaggcggcggccagcagcggcgccttcaggctcttgccctgcgccggcggctgggcgcgggcgatcaccgtgacgttgtcggcgcccgcccggaccagggcggtgtcggcgcggctttgcgtctcgcgctgctggaactcacggatcgaggcgctcagcacctcgcggttgccggccagattggcgttctcggactccagcgccgtcagccgcgcctgccttgcccggatgtcgcccagctggcggtccagcaccgccagccgcgcctgcagcgaatcacgctccgcctgggcgttgatccgcgtggtctccagctcgacccagatcggattcggcccggtgcggacctccttggctcccaccgccgtgcccgtgccgacataggcctgaagcccggcgatccgcgcctcaatgtccttcaccggctgggcgtcaggctgatagcgcgccagaagctgctcgcgttcggtgcgcagttgcagaatctggtcctgcgccgagatgttcagatcctgctgcagcgcgatctcggccggcgtggcggcctgctgcgccaccagggtctgcagacgccgcgaggcctgattcgcctgcgcctgcaccgacagccgctcggcgaaggccgtctgataggtcgccgccagcgtcgccttcgccgtggcgaagtcgccgatgtcattggaggcgaggaaatcctcataggccgcgtccgccgagcccagctcgtcctcaaacgccgcccgttgggtgcgaatggccggcgtattgtcgcggaagacttggcggcgataggccagatactgatccaccagggcgttcagcacccgcgccgcccgttgcggatcgccggatttgtaggacacctggatgatcggactgccgaccgagacgccgacgccaagcccgctggagagcgccttcagcgccgccgtctcctgctgagccggagaacccttggcgggttcgcccaggatggtgtcgacgcccagcgcccgcacagtcatcagcttgacttcctgactgttcaggatcgcggcctcggactgcgccacctcgtcggcgttgggcgcctgcccccgctcggccgtgccgacgcggggctgatagacgtactcctgccccacgcctgcgaagacgctggcgttcgccgtataggtcttcttcagcgtcaacaccgccgccgcgcctagcgcgaacaccagcagaaagaccacgatcatcagcagcagttcgcggaacagcagacccacgacatccagcacgccgtagcgtggtcgggctggaacgtaggcagtcgggcgcatgggcgtcgccgaatccgtgaaagcttcaggtcagccacccttggcccagcggcgttaaccagcggttacccataagcctgcagagtccgttcagacacggcttgcacaggcgctgctccacaatgacccttgatcgtcgcctgttgctgctgaccctcggcgcggtcgggctttccggctgcggcgcgaccgccggcggctatcgcggcggtcaggcgcagccatcctccgccgccattcccggcgacatccccttcgccacttggacggacgacgagccggagtatctgctttatccggcggacgaaatcgaggtggccctgccgacggccaatgagctgacgcgcacgctgcgggtcgggccggacggtcgaatcgccctgcccctgatcgggcacgtcatggccgcagaccgcaccctgcctgagctggaggctgctgtttcgcaggcctacgcctcgcaactcgtgcgcccgacggtcgaggtctcgctgcgccaggccggtccgatccgcgtcggggtcgacggcgaggtgcgcacgccgggcgtttacgaggtcaacggcgacatcgacgcctatcaggcggtgatccaggccggcggcttccagcccacggcccgcatgcacgaggtggcgctgatccggcgtggcccgggcggtgggcgcatgctgcgggtcgtggatctacgtccccgccgcgaacaggccgtggccatccggcgcggggacatcgtcttcgtgccgcgctcgactctgggcgagctcgcggccttcttcacccaggtgcgcgccgccctgccgatcggcttcagctattcgatcaacggatcgaacggcaacggctatgcgcagttctgaggtcgctcaggcggccagcgtcaccacgccctgatcgatgtagcggcgggcggccttttgcgcttcggcgatctcctcgcgctccatctccaggctcatctcgcggcgatacacgcgcgcctcgatcgagcctttcatggccgccaggttgaagatcatgtgggccgacacccggtccatcggggctccgcccgagccggccgaatacatcatgcccagcttgaacaggtcgtcgccgctcatgtccggcgtcggcagcggcagaccgccgtcggcggccgggttttcgtgcgcgagttcttgcgcgatcataaccgtctctcctgaacgagagcctttctggcctcgtctcctgagacgccatcaaataccgccggtttgaagttaaagttaatggcgaaaaccgggccgcatcttttcagcgcagcccggtcaagcgcctcaggacggcgtcatcgcccccgctggccgaacagcatcctgcgcgcggcctccgcgtccttgcccgacgccgcgaggtcggcccgcagatcgccgcccagcgcccggcccttctgcaccgccggccgagcgccgacggcctccagccagcgcttgaggttcgggaagtcggccagggtctggccctgcgcttccggcaggatccacggccaggccgccatgtcggcgatggagtaatcgccggcgatgaactcgcggtcggcgagacgccgatccagcacgccatacagccgatgcgtctcgtcggtgtagcgccgcacgccataggcgatctgccgctgatcgcggatcatcgccggggcgtactggcggaaatgatgggtctggccggccacgggccccaggccgccgacctgccagaacagccactggtccacctcggccttgccgcgcgcatccgcgggatagaagcggccagacttggcgcccagatactgcaggatggcgcccgattcgaagatcgacagcggccgcccgtctggaccgtcggggtccacgatcgcgggcatccgcccattcgggctgatcgcctggaactcgcggctgaactgctcgccggccccgatgttcaccggcttcagctcgtagggcaggctcatctcctcaagggcgatggacaccttccagccgtttggcgtcggccagtaccagagttcgattgggcggctcatgtgtgggctcctgcagctctgaccttcagttaggcgctgcggcggtaggggcaatggctgaacaaagctgacgtcggcgttcagcgcgagttcatgcgggacccgccattttgcagcccatggggagcgtccgcctgacgttccggaaccaaggagcaagttcatgaaccgtcttgccaaggccgccgtggtggcgctggccctgacgaccaccggcgcgccgctggtcgcccaggctcaggatcgcggtgatcgtcgcgaatggcgccaggaacgccgcgaagaccggcgtgagaaccgccaggagcggcgcgacgatcgtcgcgaatggcgccaagacaaccgcaacgaccgccgcgagtggcgtcaggatcgccgcgagtaccgccaggatcgtcgcgagtggcgtcaggacaaccgctgggaccgcaacaaccgcaactggtggcggggtcgctcggacttccgcggctataacggcccgcgctccggctactggtatgcgccgtcctacggctactaccgggtcgagccgcgttactccggctatcgctggcggacgggcggctacctgccggcgcagtaccgcagctactacgtccgcgatccctatttctacggactgcgcgaagcgccccgcggctatcgctacgtgcacgccggcagcgacatcctgctgatcgccgtggcctccggcctgatcgccagcgtgctgtcgaacgtctattgagacccggctgaatgaagaagcgggcccggagagcgatctccgggcccgcattcgttctcaggcgatgccgagcttggccttcaggatgttgttgaccgcggccggattggccttgccgcctgtcgccttcatcacctgaccgacgaaccagccgatggcctggggcttgtccgccaccgccgccgccttgtcgggattggcggcgatgatgtcatcgaccgccttttcgatggcgcccgtgtcggtgacctgcttcaggccgtgcttctccaccacttcggacggcgagccctcgccgttccagacgtggtcaaacacctccttggcgatcttggaggagatcacgccctcctcgatcaactggactaactcggccacgtgcgcagccggcagcggattgtccgcaaactcctgcccgcttgccgccagccgcgccgagacctcgttggtgacccagttggcgaccagcttggcgtctcgccgcccattgcccgtatcctgggccgccgcctcgaaatagtccgccttggcctgatccgagatcagcaccaccgcatcgtactgcgacaggccgtattcgctcatcagccgcttgcgcttctcgtccggcagttcgggcagcgacgccttgatctcgtcgatccacgcctgctccagctccagcggcagcaggtccggatcggggaagtagcgatagtcgtgcgcctcttccttggagcgcatcgagcgggtctcgcccttggtcggatcgaacaggcgcgtctcctgaacgattgcgccgccgtcctccaggatctcgatctggcgtcgcgcctcgtactggatcgcctgggaaatgaagcggaagctgttgacgttcttgatctcgcagcgcgtgccgagatggctgaagtcgccggtcgccttgaacttctcgtactggcccgcgcggcagacagagacgttcacgtcggcccgcagattgcccttctccatgtcgccgtcgcaggcgccgagatagatcagaatggtccggatcttcttcacataggcgaccgcctcttccgggctgcgcaggtccggcttggagacgatctccatcagcgccgtgccggcccggttcaggtcgacgtagctttccgtcggcgacaggtcatggatcagcttgccggcgtcctgctccaggtgcagtcgctcgatgccgacgttgaagaagccgccgtcctcgccctcgacctcgaccacgccctcgcccacgatcggatggtacaactggctgatctgatagccggtcggcaaatccggatagaagtagttcttgcggtcgaactggctcttcaggttgatctgcgccttcaggcccagccccgtccgcactgcctgctccacgcaccagcggttcagcgtcggcagcatgccgggaaagcctgcgtccaccagcgacacctgctcgttcggccccgcgccaaagcccacggccgcgcccgagaacagcttggccttcgacgccacctgggcgtggatctccaggcccatgacgatttcccaggcgccggtgcggccttggattagtttggaagtgttggactcagtcatcgtcattcgttgcctgctagccgggcttccaagtcatcaagtgagggacccacactagttccagtcggagaaccctcgtcaccctcccccaagtcccgagactgctctgcgaagagacgatcatcccaagcacggacgagatcagcacgcgtgcgaaggagttcgataggttcccagccacagtattccgcgtacatcaaaaacgaatgatagtcgctgaggtcgcgcatgacatcggcttgcctaccctcgtgagcgagatcgactcgagattcaagcaggtcaagatcggtgtcgaaatatactcgtccgccagaccaaacaaacctgcgatggccaccgaatgccccgaagctgttttttgcattcacctcgccgcatacggttgatcggtaatgcacctccaagttccggaaggttgccgatcccggatcgcggagatcccctctaactgcatccttcgcttgcgctttgaggagcaatgggtagccaagccaagccaccccccccacgaggagcacgcagcccaacaccaagatcaggcggctggtccgcgttttgggaaagcggactctcaccaccacctctccgccctgcccgtgaacccggccgcatcctccagcgccttgccgacccggaagacggtggcttcgtcaagcgctttgccgatgacctgaaggcccagcggcaggccgcccgagtcgacgcccgccggcaccgagatgcccggcagacccgccagattggtggtcacggtgaagacgtcgttcagatacatctgcaccggatcgatctgcttgtcgcccagcgagaaggcggcggacggcgtcgacggcgtcaggatggcgtccacctggccccagacattgtcgaagtcctgggcgatgcggcgacgcaccttcagcgccttgacgtagaaggcgtcatagaagccggccgacagcacataggcgccgatggtcaggcgacgctgcacctccttgccgaagccttccgcacgcgaggtctcgtacaggtccgtgagcgaccgggcttcgctcgcccggtggccgaagcgcatgccgtcatagcgcgccaagttcgatgaggcctcggccggcgccacgatgtaataggtcggcaacgcgtattttgtatgcggcaggctgatgtcgacgatttcgcagccggcggccttcagccactcgacgccctggtcccacagcgcctgaatctcggccggcatcccgtccacgacgtattcgcgcggcacgccgatgcgcaggcccttcaccgactgtccgacggaggcggtccagtccggcgtctccacgtccaggctggtcgagtccctggtgtcgaacgagcacatggagcgtagcagcagggccgcgtcctcgaccgtcttggtgatcggcccggcctggtccagtgacgaggcgaacgccaccatgccgtagcggctggcccggccgtatgtcggcttgattcccaccgtgccggtgaaggcggccggctggcggatcgatccgccggtgtcagacgccgtcgccgccaggcacaggtcggccgccacagccgacgccgatccgcccgaggagccgccgggcgtcagctcggcgttggacgccttggacttccacgggttcttcaccggcccaaacgcgctggtctcgttggacgagcccatggcgaactcgtccatgttcagcttgcccagcattaccgcgccgtcgcgccacaggttggcggtgacggtggattcatagggcggaacaaagtcgcgcagcatgtttgagccggcggtcgtgcgcaccccgtcggtgcagaacaggtccttgatccccaagggcgcgccttccagggtcccgccctcgcccgccgcgatccgggcgtcggacgcccgcgccatctccagcgccttgtcggcggtgacctcggtgtaggcgttcagcgtcgggttcgaggcctcgatgttcgacagaaaggcctgggtaatctccgccgaggagaactccttcgccttcagcccgtccaccgcggccttgagcgtcagcttggtcaggtcggtcatggcttactcgaccaccttgggcacgacaaagaaaccgtccgccgacttgggggcgttcgacagcacgcgatccaccttgccgccgtcggtcaccacatcgtcgcgcaggcgcagcggctggtgcacgttggaggtcatgggctcgacgccctgcacgtccacctcgtcaagctgttcgatccagctcaggatgccgttcagctcgccggccagcgtctccagccgatcctcgggggtcttgatgcgggcgagatgcgcgaccttgcgcaccgtcgcggcgtcgatggccatgcggccctccaaacacacaatgaagttggaaacttccaacatgaagttgattttgccgatgtcgattagccgccaaggccaagattcacaaggacggcggctttgactccggggcgctaggggcctaccgcccgcccgtgcccgtcctcgaccttcttgacctgcccgccgcctgtccgcctgacaccccgtggatggggctggacctgggggagaagaccatcggcgtcgccgtgtcggacgccacgcgcatgatcgcctcgccgctcgagctgatccgcaagaccaagttcagcgtcgaggccgagcagcttttccggctgatggatcaccgcaaggtgtcagctcttgtcatcggcctgccggtcaatatggacgggacggagggcccgcgcgcccagtcgtgccgcgccttcgcccgcaatctggaacggctgcggcccgtcaacgtcgccttctgggacgagcggctctcgaccagcgcggtcgagcggttcctgatcgaggacctggacctgaaccgcaagcggcgcgcgggcgtgatcgaccgcacggccgccgcctggatcctgcagggagcgctggaccgggtgcgcgaccaggccacctggatctgatgaacggactaatcctcggcatcgcgccggtctttgtgctgatcgccatcggctacggccttcggaaatccggcttcctgcccgacgccgcctggcgaccgatcgagaagctgtcgatcaacctgctctaccccggcttcctcgttcccgcgatctggagcgcggacctgtcgggcgccagcgccggtcccgccggcggcgcggcggtcgtgtcggtgatcgtggtggcggctctggcgctgctggccaagccgctgatccaggtggacggccccgcctacaccagcatcttccagggcgtgatccgctggaacagctttgtgttcctgccggtggtgcagagccttttcggcgccgagggtctggcggtcgcggcggtgatgatcgcctgcataatcccggtgaccaacatcgcctgcgtggcggttctggcccgctggggcgccgatcagcgcggcgtgtcgccggtggcgctgctcaaggccatgctgaagaatccgatcctgatggcgtgcctgatcggccttctgctcaacttcgccggggttccgccctttcccgtgctggcgcgcatcctcgacctgctgggcggggcggctctgccgctcggcctgatcgtggccggcgcaggcctcagcttcgccgaggtgatgcgccggcgcgtcaccgtgctctgggtctcgggggtcaagctgatggtgatgccgtttttgatgtggggcgtctgccggctgctgggcggggaccagctggcgcaggcgctcgccctgctgtgcggcgcgacgccgggcgccgcggcctcctacatgctggcgcgccagatgggaggcgacgcgccgcttatggccggggtcatcgccctgaccaccgtcggcggcgcgatcaccatgccgatcctgctgatgctgttccatttcgtctgagcgggccgtatagcgccgtctcgatgacccagccgcacgccgtcgccgaacagaccatccacgagcggctgatcccgttccccgccgcgcacttcctggcggcctcggacctgaacccgttcgtcacgccccagctgctggacctggccgacgcgttcgtcgacttcaaccgacagtcgtcgaaagcgctggacgtgctgcacggccgcacggtggtgaacctgttcttcgagaattcgacgcgcacctcctcctccttcgagatcgccgccaagcggctgggcgccgacgtcgtgaccatgccggtcgcctcgtcatcggtgaagaagggcgagacgctgatcgacacggcggtcaccctgaacgccatgaagccggacatcctggtggtgcgccactcggcctcgggcgccgccgagctgctgagccagaaggtcggctgcgccgtggtgaacgccggcgacggacggcacgagcatccgacgcaggcgcttctggacctgctgtccatgcgtcgcgcctttggcgacgtcaccagcctgaccgtcgccatctgcggcgacatcacccacagccgcgtcgctcgctccaacgtcaccctgcttcagatgatgggcgcccgggtccgcctgatcggcccgccgacgctggtgcccggcgacgccgaccgctggggttgcgacgtgttccacgacatgcgcgagggccttcggggctgcgacgtggtcatgatgctgcggctgcagctggagcggatgaccggcgccctggtcccgtccacgcgcgagtacttccgcttctgggggctggaccgcgagaagctggcctgggccgcgcccggcgtacgcgtcatgcatcccggaccgatgaaccggggggtcgagatcgattcggacgtggctgacgacctctccgtctccctgatccaggatcaggtcgaaatgggggtcgccgcccgcatggccgtgctggcctccctcgcccagcgggagatcgcccgatgacccgcctcgccatcgtcaacgcccgcctgctcgaccccgccggcgactatgacggcccgggcggcgtgctgattgagaacggccgcgtcgcgcgcgtcgtccacggctccgctcccgatctgaccgctgaggagaccgtggacgccgccggcctgtgcctgtcgcccggcctaatcgacattcgcgtgaagaccggcgagcccggcgccgagcccaaggagacgctgaagtccgccagcctggcggccgccgccgggggcgtcaccaccatcgtggtccagccggacaccgatcccgcggtcgacgatccggccatggtcgacttcatccagcgtcgcggcgcggccctgaacctcgtcaatgtgcgggcggccggcgccgccaccaaggcgctggacggccagcgcatggccgagatcggcctgatggacgaggccggcgcgctgtacttcaccgacggcgaccgggtcatcgccaacagccgcaccctgcagcgggtgatgagctacgccgccgccttcaacgccctgatcgcctgccgtcctgcggacccgtggctgacggaaggcgcggtcgccgcctccggcgaactggctacgcgcctgggcctgtccggcagtcccgccatcgccgagcgcatcgggctggagcgcgatcttgcactcgtcgaacagaccggcgcgcgcttcctggtggaccagatttcgaccgagggggcgctggagaccttggcccgcgcccgcgccaaggggctggaggtcgccgtctcggtgtcgatcaaccacctgtgcttcaacgagctggatatcggcgactaccgcaccttctaccggctggatccgccgctgcgcaccgaggcggaccgccaggcgctgatcgaggccgtgcgcgacggcctgatcgacgtgatcacctcggctcatgcccccgccccggccgaggacaagcgccgccccttcgccgaggccgcgccaggggccgtggggctggagacgctgcttcccgccgccctgtcgctgcaccacgaggacggcgtcgatctgctggacgtgctgcgtccgctgacgcacggcccggccgcccttatgggcttgggctgcggcgtgctggccgaggaggcgcccgccgacctgatcctgttcgacccgggcgcaccggtggtggtcgacgcctcgcgcctgcgatccaagtccaagaactcgccgttcgacggccgcaggctgcaggggcgcgtcgccgcgacctttgtcggcggtcgcaaggtgttcgaggcttagccgccgcgcagcagccggtcgcgcgcggcgttgacgcggacggccagaccctgggtgccgccctggtccggatgcacccgcgccatggcccgcttccaggccgcgttgatttcggcggccgaggcgtgctcggcgacgcccagaaccgcgcgcgcctccgcggcgctcagcgtctccgccgggcgtgagaccgtctgcgggcgaagccgcgagctgatggtgagatagagccccgcgcccgccagcccgaccgcgacgatccaggccccacgcgccgccgccaagaccgcccctcccagcagggccgcgctgatcagggtcgcggcgacccgccagtccccccggccgttgcgctccgtctgccggcccagccgcaccaacgcccagaccgctatggcggccagcgccagccagatcagccccaagacgtcaagcccaacggttcagccgccccttcaggccgcagcgtccagcggctgcagcgcctgctccaggcccatggcctgcatcaggttgcgcatctcctggcgtgccgccacgtgggccagcgacaccgccaccggccggatctcgttcgacaggtccgccaccgtcaggccgaagggaaacagttcgcggtagatcacccggtcgcgcaggcccggcccgacgcggaagccgacgcgcttggccagcttggtcatgcgctcctccaggcggcggcggttgcgcgcctcggccaccgccaggcggttggtcaccaccagccagtcgatggaggcgtggcggccttgcgtgatcgcgcgcatcttgcgcgcctcccacacgctttcggagtagatcgagggcttcagcagatccaacgtcaccggatcgacctcgcccagcaggtcgaagtcgacgaagctgtcgttcatgggcgtgacgatctggtccgcgcggccgtgggcggcgctggacacggcggtgtcgccccccggcgtgtcgatcaggatcacgtcgacgccggcggtcctggcctcctcgaaggcgcgctcgaacacggcgatctgctcggcggtgtcggccttggccagcgccttgccgtcgcccatgtccggcatcatcggctggggcagctcatgaccgttcgcggccagccaggcgcggcggttgttgaagaagcgcgccatggaacgctgtcgcaggtccagatcgaggatggccaccgtcttgcccgcatgcagcaggccggtgacgatgtggatggccagggtggacttgccggccccgcccttctcgttgccgaggacgatcacatgaggttgggtcatcgcagggcgatctccgctgcggccggcgcgactcaaggaggcgcacggacctactggaccgcagactccgtccggacgatccaaacgtcaacgacgcgttaacggattactgtggatcagccccgggcgcaccagggatcggccccgacgatcttccggcagagaccgcgcgcgacatcgggcgccagcggcccgaccttcaggcgcaccaagcggcttccgcctcgttcgactggttcgaacacgggctgaacaccctgcaactcgcttcgtcccgacagctgttcccaggcggcttgcgccatcgcctcgctggcgtaggcgcccagctggatcatgcgcggatcaacgtcggtgggcgtaggcgcgactgcggcggcttcaatcaccggtgcggcttccgtggcctggactggggtctcccgcctgcgcgcgacggcttgcacgattgcaggagcgggcgtgggcgcgcccaccgccccgcgcatgccggcggcctcagcatcgcgggcgtcccacatctcgtgcgggtccatcaccgccacgcggaccggcgagaagtcggcgccgcgcagaccgcccgaggccgagccgccgcccgatacgtccaccgccgcgacggcgcgggccatgccttcgaaccgccgcgtctccacggcgtcgccgtcgcacgccgaaaggctcaatgcggcgccggcgctgatcagcgcgagcagtactggacgggtcgcttctgcgggcgtcataagcgcgagcctaccgggcggcttttgagacgtccttagcgaacaggcttaagagaaagagtcaacgccagcatgaccgacgcttccctgcccgtcgcccgcaccgttgctgaactgcgcacagccgtcggggaatggcgccgccaaggcttcaccgtcggcctcgtgcccaccatgggcgccctgcatgaggggcatttgacgctcgtgcgcgaggcgaagcggcgcgcggacaaggttgtcgccagcgtcttcgtcaacccgacccagttcgccgcccacgaggatcttggaacctatccccgccgcgaagccgaggacgccgcgctgctggccgaaaccggctgcgacctgctgttcgcccccacggtcaagcagatgtaccccgagggcttcgcggcgcgcgtcgagatcggcggcccgaccgtaggactggagacggacttccgcccgcacttctttggcggcgtggcgacggtggtgaccaagctgctgaaccaggcccgggccgacgtcgccgtcttcggcgaaaaggactaccagcagctgatggtggtgcggcgtctcgcgcgcgacctcgacatcccgaccgagatcgtgggcgcgccgaccgagcgcgacggctggggcctcgccctgtcttcgcgcaacgcctacctgtccgaagacgacttgcagatcgcgcgccgcctgaacggcgtcctggctgaggccgcactcaaggccgcgtcaggcgagccgtcggcgaatgcggaagcctgggcgtcctccgccctgctgaccgccggtttcgaacgcgtcgattacgtcgccgtccgagccgccgacctgtcctcataccgagccggcgcaccgggccgcatcctggccgccgcatggctcggccggacgcggctgatcgacaacatggccgtctgagctctccttatcgatccagcgagcggtccagcgcgcggaacgccgcgatcgcaagttcggtggagttctggaagacagcgggcgtgatcttttcgaagtcgtccgatggccggtgatagtccggatggtagtcgacgccgagatagaggaacggcacttgcgcctcgtgaaaggcggcatggtctgaggccgtcacccagttgttctcgccggtatcggcgggggggtccttgcccaacgccagcgcgatcgagccttgcgccggcagggcctccaggatcgagcgcagcgtcggatgctgataggtcccggtgacccacaggtggttgtccgtctcggcccgcgccgtcatgtcgaagttgaggttcagcgccatggaggtcagcggcacgggcggcgccttgacgaactcgcgcgcgcccagcagcccgcgctcctccccgtccagcgccacgatcagcacgctgtgctcgggcgcttccgccttcagacgcgctgccagctccagcatggtcgcgacgccagaagcgttgtcgtcggccccgttgtagatctggccgtcgctgacgccgacgtggtcatagtgggcggtgacgacgatgtagcgatccggcgctcgcgtccccgggatcagccccacgatgttgacgccgttgaagaccttcggcccgctgcgggtgcggccggtcgtttcgaaccgctgcagccgtccgaacgaggcgggcgccacgcccagcgcctccatgcgggagacaatgtagtttcgcgcacgctcgcccccggccgcgccggtgtcgcgcccctccatgtcgtcggccgagagggtgcgcagatcggtcatcagctgggcatagtcgcgcgccggcgctgtctcgacggccgtagcggcggcgggttcggcggtcggcgtttggcatgcggccagcgcaaggacggacacggccgaaagagcaaggcgaaggcggatcatgacgactccagcgagaagatccgccagccttagcgagcccctgcgccggcgtcagcataacgatccgtcatgcatgccggaatcgcccttggcggtgtaagaggtcgtcatgagcgccgcgcccttcgccaacatccccgtcgccgagttgacgacgcctcaggccgaggccgagctggcatggctggcggccgagatggcgcgccacgacgccctctactacgccgaagcggccccggagatttcagacgccgactacgacgcgctgaagcgacgcaacgccgagatcgaggcgctgcatccggacctgatccggcccgactccccgtccgaacgtgtcggcgccgccgcctccagccagttcgtcgaggtgcggcacggcgtgcccatgctgtcgctggacaacgccttcgacgaaggcgaggtgcgcgacttcgtggcccgcatcgggcgttttctgaaactacccgacgagcccatcgcctttgtggccgagcccaagatcgacggcttgtccgccaacctcttgtacgtcgatggggcgctgagcgtcggcgcgacgcgcggcgacggccgcacgggcgaggatgtcacggccaatctgaagaccatcgccgacattccccaccgcctgcctggcgacggctggccgtcccgcatcgaaatcaggggcgaggtctatgctccgaacgacgccttcgcgcgcttcaacgccgaggccgaggccgagggtcggcgcacctacgccaatccccgcaacttcgccgcaggatcgctgcgccagaaggatgcgaagatcacggcgcgccgcccgttgaagttcttcgcctacgcctggggcgagcactcgtcggacttcgcgaccacccagggcgaggccttggaccgactgcgcgcctggggttttccggtcaacgcgcgctcggttcgcgtcgagggcgcagaaggactgatcgaggtctatcgggggctggagcgggatcgggccgggctcggctatgacatcgacggggtagtctacaaggtcgaccgcatcgattggcagcatcgcctcggctatgtctcgcgcagcccacgatgggccatcgcccacaaattcccggcccagcaggcgaccacggtgctggagggcatcgacatacaggtgggtcggcaaggctcgctgacgcccgtcgcgcgcctgcatcccgtcaccgtcggcggcgtggtggtccgcaacgccaccctgcacaacgaagacgagatcgcgcggctggatgtgcgcatcggcgacacggtgatgctgcagcgcgccggcgacgtgatcccgcagatcctggggatcgtgcccgagctgcgccctgcggacgccgaactctacgtcttcccgacgcattgtcccgtgtgcggctcggaggccgtgcgcgagggcgacgaggtcaagcgccgctgcaccggcggcctgatctgcgacgcccagatcatcgagcggctgaagcacttcgtctcgcgccgcgccttcgacatcgagggcttgggcgaaaagcagctgaccgcctttcacgcccgcgggtggatcaaggagccggcggacatcttccgtctggcgcgggacgacgaaaagctggcgaccctcgaggccgaggacggttatggcgaaaccagcatacgcaaccttgtcgccggcatagacgcgcgtcggatcatcagcctggaccggttcctgttcggcctgggcgtgcgcgacatcggcgaacagacctcgctggtgctggcgcgcgccttcggaagctggtcggagctgaagaccgcctgcctggaggccgccgccggtctgcccagcccggaatgggagcagctggcctctgcgcccggcgtcaccccgcgcgtcctgtcggctctggcgggcctttcgcccgacgctccagacccgtggcccgacggcggcatggaggccaagctgcagcatgcgctggcgggtctcgccaagcctggtcgcgccgcggtgcaggcgctcgcccccgactggccggcggtgctgagactggcgcggatcgcccgcgaagatgcgcccgccgacaccctgggccgcatcgcaggggtgtctggggtgggtcccgtcgcggcgcgcgccctggccgacttcttccacgagccgcacaatctggcggtcgtgtcggcgcttgaggacgagctgaccacaatcgaggatgtcgaacagcccaaggccgacacacccgtcgccggcaagacggtggtcttcaccggcgcgctggaacgcttcacccgcgacgaggccaaggcgcgcgctgaaggtctcggggccaaagtctcggggtcggtgtccaagaagaccgattatctggtcgccggacccggcgcgggctccaagctgaaggacgccgaaaagcacggcgtgcccgttctcagcgaggacgagtggctggcgctgatcggcgggtgagacccgccttgattccgtcgcggatcggggacaacctccggggcaacaaggcgaaatcgccttacccaagggaaacgaccatgaagatcaaagtcctgctcgccgcttcggccctgatcggcgccctcgcctcgcccgcgctggcggccgatccgatcggcgtttggcagacccccaccaacggcggccaggtccgcatcagccgctgcggcgaagccctttgcggaacgctggtcacctccagccatatccgcgccgacgccaacgcccgcgacgagcacaacaagaacgcctcgctgcgcagccgccccttgcgcaacctgccgatgctgacgggcttcaccggcggcccgaccgagtggcgcggcggctcggtctacaatccggccgacggcggcacctaccggggcaccatcaccatgaccaatgacaacaccctgcgcctgcgcggctgcatcgtcgcgcccctgtgcaagacccagacctggacgcgcgtccagtaaggcttcgccatcatgcatgaagaggcccggccggagcgatccggccgggcctttgtcttgtcagcgcttcaagatcagcggttcagggccgaacgcgccgcctcggcgtagcgatggccggaagccgcgtccttgggaaacaccgcctcgatgcgggagaggtcctcaggcgtcagcgcgatctcggccgccgccacgttctgctccagcgtcgaaatacggcgcgtgccgggaatgggcacgaggtcgtccccttgcgccagcacccacgccagcgccagttgcgccgccgtcacgcccttgtccgcagcgatttcagatacggcggtgaccaggtctaggttcttttggaagttctcacccatgaagcgcgggttggtgcggcggaagtcgtccggcgccaagtcatcaaccgacttgatctcgcccgacaggaaaccgcgcccgagcgggctgtagggcacaaagccgatgccgagctcgcgcaccaccgacaggatttcgtcctcgggctcgcggctccacagagaatactcggtctgcaaggcggtgatgggatgggtcgcgtgcgcccggcggagggtctcgggcgcggcttccgaaagccccagaaagcggaccttcccctccttcaccagctccgccatcgcgcccaccgtctcctcgatcggcgtgtccggatcgacgcggtgcagatagtagagatcgacgtgatccatgccgaggcgcgtcaggctcccttcgatcgcgcgacgcacgttggcgggcgagccgtccaccttcagctgggtgcggtcggcgttatagccgatgccgaacttggtcgcgacaaaggcccggtcgcgacggtccgccagcgcctcgcccagaagcacctcattggtgtgcggaccatacatttcggcggtgtcgaacagggtgacgcccatgtcgagcgcgcggtggatcaccgcgatcgactgcgcgtcgtcgccacccccgtagaaggcgctcatccccatgcaacccaagccgatggccgaaacctcgggtccgccaggacccagcgtgcgcgtcttcatgggcgctctccttcttatggtgaaggactgagatgggctcgagcgcccggatcaacaaccgtcgtccgtccgcttcagccagtcgcctagcggcaggtcggaggtcgcgcgcgtctcggccgacatggcgttgcgcatgatctccagcgcccattcggtgcgctgatcatccgggctcgccaccgcgtcgctgggaacccagatgtcgtactggcgcatgtgggcgtcggcggcggtgaacagcacgcagatgtccgccgccacgcccgtcaggatcacccggctggccttcagctgcggcagcagcaccggcaaattggtggcgtagaagcccgagaactgcggcttgatgacgaagtagtcgttcggtcgcggcccgatgcggtcggccagcgccgccgcgtcaggatcggcctgacgcacatgctcgaccagacgtgacttttccgaaggccactggccgaagttgtcgttgacatagaccgtcggcacgccggcgcgatcggcttcattccgcagccgcaggatggcctcggccgccttcagcaccttgggccgcatggcgtcggcgtccgagaactgcagatcgttgatcatgtcgatgatcaacagggccgtggcgccggccgccggttcgatgatctccgccttgtccacgcgcgtctccatgctaacggccggatcaacgcgcggaagaccgattggccccgtccagtcagccgccgtagccgcgtccgccgccgccgaagccgccgcgcgacaccaccgccgtgcggctctgcacccgggtcggcgcctggcgggccacgtcatagtcgcggccgttggtcagcagccggcccgagcggtagtcgcgataggcgtagccgccgccgaatccattggagtagcggccgctctggtcgcgatacatcgggcgatagcgcccgccgtccagcgcctggccgatgatgaagccggccagcagcggggtgaagaacgagccgcccgaaccattgttggtcggctcgcattgcgacggcccccaggtcccctcgcactccgcgcgcgacatgtagcgcggcccttccgtctgccgggccttctcggcctcggcgtaggcggtccggcactcgctgtcgggcgcgttgttcgcatccaggcattcctggagcgacgtataggcggccgtgggctgaggcggcgcctcgacctgggccggcgcggacggcgcatcgccgcacgccgccagcgagaagctggccgtagccatcaggctggtcacctgcagcgtgcgcgaacgcttcatgcggctgatggcgagagtcttctggtcgtcggacatcaaacaggtcctcaggtggtcatgcaggcggcgttcagcaggccgacgcagatggagacggccgccagatacagcgccgccgccatgtcgcccgcctcaacccgaatggccagattgcggaacgccaggcgactgacgatcacgaaggtggcgatctggataacgcccgctaaggccgcccaggccacgaactcggccaggctgatcgtgtgagacagggccgaggccagcggcagcacatagccgatcagggcgccgcccagcgtcaccgccgcggcctggttgccctgccggatcaaggtgcgctcatgatagggcgtgatccactggtagatcagcttgaaggcgaccgtgaacgcccccgccgtcgcaaaggcgaccaggaacgagatcgcccccgcctgaaacgtcatccagtcgaacatccagtcgctcctccacaaggctcgccgtcaggcggcgaattcggccagctccagcgggatgccgaccatgatctcgtgcgtgacgtcggcggagcggccggtcttccgctcgggctcctgctcgatcgccagcatcagttcgcgcccgccgggcacgtcgcgcgcatacagcatgcaggtctggaagatgcgtgcatagggggtgaccgccttgcggtcgtcgtgaatctcttcccagaagctgaccggcggctgacgcgcctcgctttcggcgaaccagaagcgcggccactggcccacctcctccgccgtgccgtcgaacaccggctcgctcagccgatccttccagcgcctgcgcgccgcctcgttcggcggataggcggacgaccagggtatgtagagcgtgaaatcgtaggacaccgcccccgtcgcatcgtcgctcatgccctgcagcatgacgtggtcgtcggtgtagaagcgatgcacgaactgcccgccatccagctcgaccgacccttgcgcggtgatctccagcgcatcgcggtcgagggtgaacaggctttccccctccatccgccgccacgccaacgggtcgagccgcaccgtgcggcccactgtgatgttgcgcaccaccgccaggcggtcaggcgtttcaggcgtggattgactaaacagacgtttgaacatggtgacaccatagctggccgaggccgccgacgcaccagccttgtcaacgcccttggcgaagatcaagcgttcatgttacgcgttgcatgtaacatgcctcgtctcgcacccgtctcctcgaacgccgcctcggaccgcatccgggcctggcgccgcgcgcgccgcgaggccgggatggtgaagctggagttctgggtgcccgaagtcgcccgtgccgacgtcaaggcggcggtgcacgccatcgtgacggattcgacgcgcggccccttgctccagtccttcatgcgtccgaccttcaacgcctcagccttgtcaggagccgaacgaccgatggattccgtgatcgaaaccccgtggaccgtgcccacgatcaaggaggcgctggaaggctcctcgcttgttcgcgagggggaaatgaccctgcgcgtgctggagggttcggacgccgtgctgctggcgaccatgcatgaatatggcgaccttccgatctatctgagcgtcggccgcgcccagatcgtctgctcggtgttgctctggcccgcgtcggagcagcaggatcggcccgccttcaacgagttcctgctcaaggcccagcgtgtcgtgcccctgtccaacttcgccatcaccaatgtaggcgaggaggaatactatgagctgatgggcgagctttcgtgcaagacgacgctgcagaccatcctgatcgaactgcgcaccctggcggagaacgccattgatgcgaccgagctgcgcgagaccttcggctcgcaggccgcctgaggaagaggagacagatccatgtccatgctcagcaaactgtccgccctgttccgcggcaccgcccatgaagccggccaggccgtggtcgacaagaacgccctgcgcatcctcgaccaggagatccgagacgccgacaacgcgcagagcaaggcgcgcgacgacctcgccggtctggtcgcccgtcgccgctcggccgagaacgagctccagagcctgggcgaccagatcgccaaatacgaaagctctgcccgcgcggctctgggtcgcggcaacagcgacctggcgcgtgaggtggcccagcgcatcgccgagctggagagcgaaatcaccacccgcgcccctcaggtcgaggacatgaagacggccgagacccgccttcgccagaccatcggcgccaccgaccagaagatccagacgctgaagcgcgagatcgacatcgtaaaggtgaacgactcggtgcagcgcgcccagtcggccgtggcgctgcagtcgcagggcgctcactcccgcatcggctcggccgcggacagcctgcaacgcatcaagcagcgccaagccgttcacgaggagcgtctgcgcgtcggccaggagttcgaggatcgccgcaccggcgccgacctggacgccaagctgcgcgacgccggcatcctgccgggcgcttccaatgccgacgacgtcctggcccgcctcacccagcaggaagtcaaggtggtcaccccgcagatcacccagcagggcgaaaagtccccggtcgagcgcgactgatcatggaacggacgcgaccgaccccccggccaggctggcaggcgctggctgagcaggtgggcttcacctggcaccacgacagcggcaaaccctactgggacgagtcggtcgcctaccgtttcaccctgcccgagatcgaggacggcatcgaagcgccgaccgccgaactgcacgccatgtgcctcgatctcgtggccgaagcggtcgaaagcgagcggctgatgaccctgctcgacatccccgaggcgtcgcgggattatgtggcggatagctggaagcgcggcgatccgtccctctacggccgcttcgacttcgcctacgacggccagggtccggccaagctgtacgagtacaacgccgacacgccgaccagcgtctatgaaaccgccgtcttccagtggctatggctggaggagcagatggcgacgggcgccctgcccgccaacgccgaccagttcaacagcctgcacgagaagctggtcgaacggttccgcacgatcttcccgaacggcggctttgtgcatttctcgtctgacgccgacttcgtcgaagatcgccaaacggttcgcttcttggaggacctggccaaacaggcggggcttgatccggagttcgtgcccatcgaccaaatcggcctgaacgccgatggtaggttcgtcgaccagaacaactacctgatccaggcgatgttcaagctctatccgtgggagcagatgctgcgcgacgactacgctgagcccctgcctcgcgccgaaatgacggtgctggagccggcctggaaggcgatcctgtcgaacaagggcattctgccgctgctgtgggagcgccacgccggccatcccaatctgctcgaagcctatttcgagagcgatccccagcatgaggcgctgggctcctcctacgtccgcaagccgctgttctcgcgcgagggcgccaacgtggctctggtggacaagggacggaaggccaaggtgctggaaggcggctacggcgaccagccgcacatccgccaggcgctgcacgcaccgccgcgtttcgacgcctcctacgtcatcgtcggcagctggctggtgggcgaccagcccgccggcatcgggctgcgcgaggatcgcggacggatcacgcgcaacacctcccgcttcgtgccgcactacatcgtctgatccaaccttggccttcgcgcgttccgtgactcctcaaagggagcggggcggccatgcgcggcgaactggacacctacaaggccaagcggaacttttcggccacgcccgagccggaagggcgcaagggttcgtccaagtcggcgacccgtcgctacctgatccagcggcacgccgcaacgcgcctgcactacgacttccgcatcgagcacgacggcgtgctgaagtcctgggccgtcaccaaggcgccgtcccgcgacctcaaggtcaagcgcttggcggtggaggtcgaggatcatccgctggattacggatcgttcgaggggaccatccccaagggcaactacggcgccggcacggttcagatgtgggacatgggctcatgggagccgcaggagccggacctcgacgccgccttcgccaagggccagatcaaaatggtgctgcacggcgagcggctgcagggcaaatgggccctgatccgcatgaagaccgatcgcggcaagccgtccaaacgcaacaactggctgctgatcaaggagcgcgacgacttcaccgtcgaaggcgaaggcgacgccctgatggagatcgacgcgtcggtcaccaccggccgcaccctggccgagatcaccgcaggcgcgccgccgcatacgctcaccgcttcaacaaagcccgccgccaggccgaagaggaaacgcgcggcgaaggcccctccgtcctcatcggggccgcccgacttcgtgcccatccagttcgcaaaggtcgtggaccatccgccgcccgccaaggggtgggcgcatgagatcaagttcgacggatatcgcatccaggtcggcgtaggcggaggccgcgcggccctgcggacccgaaagggcctggactggagcgacaagttccaggttttagccgcccaggcggcttcctggccggagggggtcgtcgacggggaactctgcgccctgggccaggacggcacgcccgacttctcggcgcttcaggccgccatctcggacggcgagacggacaagctcatctacttcgccttcgacctgctgttcgacgcagacgaggacctgcgcaatctgccgttggcgcaccgaaaggcgcggttgcaggcctatgtcgatcgtgtgggcgccgccgggccccacctgcgctttgtcgaacacttcgcctcgtccggcgaggcggtgctgaaaagcgcctgccgtatggatctcgaaggcgtcatctccaagaagctggacgatccctatcgcgccggccgcaccgcatcctgggtcaagtccaagtgccgaggccgcgacgaggtggtgatcggcggctggtcctcggaaggcggcgcgcggctgcgttcgctgctggtcggcgtgcgggagggccagggcttgcgctacatgggccgggtcggcaccggcttctcggccgaactgtccaaaaccctgctgccagccttgaaggcgcaggcgtcggacgacaatcccttcaccggcaagaccgccccccggcggggtcgggacatccactggctgaagccggtgctggtggccgagatcgaacacggcggcatcaccgaaggcggcaatgtgcgccaggccgcctacaagggtctgcgtgaggacaagacggcgttcgaggtcacggccgaaccgcaggcccctgccatcgcgccgaagacggcgacgccggcatccaagccgcgcggcagagagaaggtggtggtggccggcgtcaccctgaccaatcccgacaaggtgctgtggcccgagcatgacggccagcgcgcgatcaccaaggccgatctcgcgcgctatgtcgaggcggcggccgagcgcatcctgccccacgtcgccgaccggcccgtctccatcatccgcgcgccggagggcgtgggcggcgagaccttcttccagcgtcacgccatgccgggccacaatccccgcctgaagctgatcgacgtgaaggaacgcaagccctatgtcgccgtggccgatgtcggcggcctggtcgcggtcgcgcagtccggggggctcgaactgcacccctggggctgcaagcccggcgatcccgaaacgcccgaacagatcacctttgatcttgatccagacgagggattgaacttcgacgatgtgatcgcggccgcgctgctgctgaaaccgcgcctggaggcgctgggcttctcacccttcgtcaagaccaccggcggcaagggcctgcacgtcgtggtctccatcaggacagacgcgcgcagccgcattgagtgggaccggtgcaaggccctcgccaaggccgtctccgaggccatgcgcaaggaccatcccgagcgtttcaccaccaccctggccaagaaggcgcgtggcggaaagatcttcctcgactatctgcgcaacggccgcatggccaccgccgtcgccccctggtcgcctcgggcccgaccgggcgccggcatcgcctttccgctatcatggagccaggtgaagccaggcctggatccccgcgcctacaccctgctgaccgcccccgccctgctgaagaaggccgatccatgggcggacttccgcgcctccgccgcctccgcgcggcctgcgatgaagacgctgggcgtctgatccgctaggctgatccatctcaggagacgatcatggcgggcttgaaggacaaacgcggcttcatcgacaaggaccgcctggacctgtccgagcggcaggccgtcgaatactggatgaagcgctggggcgtcacgcgcgaccagatcaccgccgcccaccgcaaggtcggccgcatgaccaaggacatcgcggccgaactgggcaagaagcgctagaggtcaatcaggccgacgtcttgcccttcggctcattgatccagggtggcgcacaggtgtcgcaatgagatttttgcttgggttgctgctgctgctggctgggggatgcatgtccattcccggcgttcattacacgcccaggcagtgctcggttcagggccacggtgttcggattgccggaccgacggaccagcacatgctggcgtgtctgcgccggatgccgccgtcctccgtcgtgaccatcacctccgagggaggatcggtcagcgcggccctggacatcgccgacatcttggcgacctggaaggccgaactgatagtcgagcgctactgcgagtcctcgtgcgcgaactacctgatcccggtttcgcattcggtggtcatccgtccgggggctcgcgtcgtgcttcatggcagcgtggacggtcacatggtggcgcagggcgcgcctctgtcgctcttcatgcgccaaaagtccttcgcgcaggatcatgacgtccatcccggctggctgctgatgcggactgatgaggattttaaggcgcgtcggaacggcgcctcggtggcgggtgctgtggatgcggtctcggcatccccgcgccgcttcattgtcgtggagcctgccttcgccgccacatgcctgccagacgtgccggtccggtgggagccgcaaacctatgccgacaagatgcgaggcgacgccgacctgcgtcgccgaaaagaggccgacggcttcgttctcagcggtagcctaagctgttccgaggcaaggacctatcccgccctgtagcgtcaggccgccttcttccccgccgttgtctttttcgcgggcgccttcttggccgcgggtttcttgggttctgccttttcagaggtcgagctctttgtggcggtcttcttggcaggcttctttgcagcgccgctgctggccgagccctgcaggctggcgcgcagggccgccatcaggtcgatgacgttggtgtcgtcgggttcaggcgcctcgaccacgttcttaccgcccttctgcttggccttgatcatctcgcgcagggcgtcgtcatagcggtcggtgaagtcggccggatcgaaatcgccttccttttggccgatgatgcgggcggcgatctcgaccatgtccttgtcggccttcaccgcagggatgtcgtcgaaatagtcgtcggcggcccgcacctcgtcgtgcgccctcagggtgtaggcgatcagccccttgtcgcgaacctccagcgccagttggcgctcgcgcccacgcagcaccagacagcccagggcgatcttgcccgccgacttcatcgcctcccggatcacggcgaaggcctcggcccccacgcccttttccggcacgatgtagaaggggtcgtcccagtagagccggtcgatctcgtgctcgtcgacgaatttgtcgatcgagatggtgcgggtgctttccagtttcaccttgtcgaagtcggcgtcgtcgaacaggacgtattcgtccttggacacctcatagcccttgaccaggtccctgcgctcgaccggtcccgtgtccgggtcggtcggcaccatgcggatgcggttgttggtctcggggttgatcaggtgaaagctgatgtcgttggttttggtcgtggccgtgtacatcgcgaccggacaggtcacgagcgacagcttcagatgcccttgccaggtgggacgcgcggccatggtgtgtctccgttcaaccgctcaacgtgagtcctccgtcgccggtttcgcgctcagtggaaatcgcgcgagccgggcaggatacggacatcgcgcggatgcttgccggtgggcgagcgcggcgcctgcgggtgtttgacgacgtcggcgcgcgacagctgcacctccaggtcgtagtcctccgacagccggcgcagctcggccgagcggtcgatgacgcggcgcaccatgacgtgcatgacgccctcgatgctcttctccaccgtgccctccacctccatcaggcgcgccgccatgacctcgcggcgataggtctcgaacagccgcgcccacaacagcacgttcacgacgcccgtttcgtcctccagggtgacgaagatggcgttgcccgatcccggccgctggcgcaccagcaccacgccggcggtgcggatcagggctccgtgctttctggcctccgcctccgccgcgctcagcacgccctcgccccggaacacgggccgcaggatctgcatgggatggcccttcagcgacaggcgcgtggtctggtagtcggtggcgatgtgctcgcgcagcggcatgggcggcagctcggccgccgcctcctcgcccagctcccgcgcgccgcgggcggcggccgcctggaacagcggcaggggggcatcgtccggcaggcgccgcacggcccagagcccctcgcgtcgatccaggcccagcgagcgaaaggcgtccgcgtcggcgagcttgcgcatggcgccggccggcagccccgcccgtcgcgccatctcctccacatcacgataaggccgatcccgcgcggtcgtcagggcgccggcccaatcctccctgaagccgtcgatctgccgaaatccgagccgcagcgtcagatcgctcgcgacgggttccaggctgttgtcccaaccgctgtggttcacatcgataggccgcacctcgacgccgtgctcctgcgcgtcgcgcaccagctgggccggcgcatagaagcccatcggctggctgttcagcagggcgcagcagaacaccgccggctcgtgacatttgatccaggccgagatgtagacgagccgggcgaacgacaccgcgtggctttccggaaaaccgtaggagccgaagcccttgatctgatcaaagcagcgctgggcgaaaccacgttcgtagccgcgcgccaccatcttctcgaccatcaggccctcgaagcggtccagcttcccttcgcccttgaacgtgcccatcgcctttcgcaggccattggcttggacggaggtgaagtccgccgcgaccatggcgatcttcatggcctgctcctggaacagcggcacgcccagggtgtccttcaggatgtgcctcagctcgtcgggatcgtgcggcgccgcggggctcggatagtccggctcctccagcccgttccgccgccgcagatagggatggaccatatcgccctggatcggaccgggacgcacaatggcgacctgcaccgccagatcgtagaacttctcaggcttcagccggggcagcatgttgatctgggcccggctctccacctgaaagacgccgatggagtcgccggtctgcagcatcttgtagacgtcggcgcattcgtgcgggacggtgtccagggccatgtcgaggctgcgatgctcggccatcaggtcgaacgccttcttgatgcaggtcagcatgcccagcgccagcacatcgaccttcatcagccgcagctcgtcgatgtcgtccttgtcccattcgatgaaggtccggtcgggcatggcggcgttgccgatggggaccagttcgtccagccgatcctgcgtcagcacaaagccgccgacgtgctgggacaggtggcgcggaaagcccagcaggcgacgggtcatgatcaccgcccgcttcagcatcgggttttcgggatcgagaccggcctggaccacgcgctcgtccggcaggtcgcggccgaagctgccccattccccgccggccagccgcgctgtcacgtcctcggtcaggcccagcgccttgccgacttcgcggatggcgctgcgcgggcgatagcggatcacggtggcggcgatccccgcgcgatgtcggccgtagcgttcgtagatgtgctggatcacctcctcgcgccgttcgtgctcgaaatcgacgtcgatgtcgggcggctccttgcgatcggaggagagaaagcgctcgaacagcagatcgtggtgttccggatcgaccgaggtgatccccagcacgtagcagacggccgagttcgccgccgatcctcgcccctggcacaggatgccttccttgttggcgaaaaggacgatgtcgtgaatggtcagaaaataaggagccagtttctgctcggcgatgaaatcgagctccttgaccaaaagatcgcgaaccttggccggcgctccgtctggatattttcggaccgcatagacggcgactaggtgctccagatgcccttgcgccgttgcccccggaggcacaggctcctcgggatagttgtagctgagttggctcagatcaaaagccacacgcgccaggaaatcctgcgtctcctcaaccgcttccggcgcgtccttgaacaggcgcatcatctcggatgcaggcttcagatgacgctcggcgttgtctttcagccggcggccggcctcgtggatcacggtcttttcgcggatgcaggtcaggacgtcctgcaggtcgcgctcctccgggtcgtgatacagcacgtcgttggtcgccagcaggggaatgtcccatcgctgcgccagcgtcttgagccgcgccagccgacgacggtcgtcgccccgcctgtgcatggcggcgcccagccagaccgcgccgggcgcggcctcagccaaccgttccagcaccgtatccagtccatccagccgacgcggcggcatgaccaccagcagcatcccttcaggcgcggcggtcaggtcgcccagcccgatctcgcattcgcccttctttgcccgccggttgcccagcgtcagcaggcggcacagccggccccagccctggcggtcttcaggataggccaggatgtcgggcgttccgtcgttgaaccgcaggcgcgcgcccaggatcagcttgaacgtcgcggcgcgccgcttgacctcttcgcggtcgacatgggcgaatgtgggattgtcgacccagacgatctcgcccaggccgccggcctcgtgcaccttctcgggcgcccagccttccgcgcgaaagtccttcagcgcgctccaggcccgcaccaccccggccagggtgttgcggtcggccaagcccatgcccgtgtggccgcgcagaagggcgctgagcaccagttcctttggatgcgacgccccttccagaaaggagaagttgctgcgggtcgccagttcggcgtagccgctcatgcgaacacgccatgcagataccagcgcggcggcggctcctcgccgtagaagccggcgcggaacacccagaaccgccgcccctgcccgtcctccacgcgataatagtcgcgcgtccgctccttgggcctatgccaccactcacctgcgatcctctcgggcccctcggcgcgggtcacgacatggtcgatgcggcgccagcggaagcgggcgggcgagccgtccggcagggcggccatggcctctaccggctgcggcgggtcgaacacctgaagcggcctgagcggcggatcggcgggatcgcgctcgccccagtcccccgctgggtcgagggcttcggcggccgcgatgaaccgctcggcgcgctcgggcgcatgagattgcaccggctcgatgcggaccaccgcctgcgggcccagccgcgccgacagccggtcgatcagcggccccaagtcgtcctgcggcgcctcggcctccaacccgctctgcgcataggccagcctctgggcgaccgggatggtcaagcgcaggtgatcaaagccgaagcccggatccagcggccgggccaggctggccagcctttcgcgaaacagccgcagcacggcgggggcggcgcgcgtcggccgacccggccggatcgtgatccgccgcacctcgccgtccacgcggaaaaaggcggcctgaaaggcgcggccgccctgcccccgctggtccagccgatccatgacctccaccagcaggtcgccgaccacggcttcaacatcggcggtttcggtgatcggctcgaccagaatgcgatcggccgcgcagacgcccgccggccgcgagggggtgatgcgcgcatcctcaagccccagcacgcgtcggagccgcgtcggcaggtcggacccgaaccgggcggtcagcggcgcggtcgggcgatcgtcgaggtgcgccagcgtcttcagccccgcgcgagacagggcctgctcctccttttccggcaactccagcgcgttgatgcgcagacgccgccccgccgtgcgcgcctgacctttcgcaaggatcccgcccggtccgaaccgcgcccaggcgcgcgcgctttcggcggtgtcggacatcgccagccgcacctgaagacctatgcccgccgcccgccgcttcacagcgtgcatcagtccggcttcgcccgcgaacaggtgggcgcagccggtcacgtccagcaccaggccgtcatgcccgtccaaggccgccatgggactgaaccggccccagtcctccagcacccgcttcagcagcgcctcgtcgccttccggctggtgcaccaccgatcgcacggcgggcgtgcgcgcctgggcgtcggccagggtcatgccggaagtcaggcccaggctggcggcaagacaatccaccgccgccagccgcaaggcgccgcccaccttgtgcacaaagaccacgggcgtcgcgtcatccgtatcgcctgcgggcgtctcccgcagccgccggtcggccggcagccaagggaaccaggccgccagatagcgacggccggctgaacgatccgcactcacgatcccactccatgatccagggtccggccgacgcgcctccgcgccgccgcatcagttcgacttcaaaggcgggccgaccgggcgcattggcttccagcgcgcgagacggagcggttgtcacgcgccagcggctgtccgcggcgctgggctgcggctcagctcccatccgcaccagaatcgccgtggcccgtcccttggcggccatcagcgacagccgacggctggccgtcagcgtcatggccttggcgtcgccccaggcgctcaacagcaccgcacccacccccgcgctggacagcgcctcttcgcccgccgccaacagagcctgcgtctcgcgcacccgcaccaagacgacccggccgggatcaacgccccactggtgcaggccggggccgtggaggcggccggtctcccgatccgccatctcctgcacgccccagaccagcgcgcccttgtttcccgcccgcaacgccagccccagggcgaacccttgcgcggccgccgcatcgccaagacacgcgggatagacgtcgtgcagcgcgtgactggccagaccctgcagccgcgcatccaccgcatcgacgcccaggccgaagcgttcggccgagctcggcaggctctccgttcccagcgcctccaggcgcgtcttcaggccatcgatttcggggtggacccgcaacttagttctccttttgttcttatatgcctccttccacgaccggtgagtcaatcggagtccgacagggtgttaggaatttcttccggataagtcggcgcgtcttccgccgctcggcgtcagccgaccgccttcaggaacagcacccgcgccgcgccatagtcgcgcgcatccagcctctcatagcccggcgtctcgatttcaggctcgtccgagccgcgctcgaacaccacaagcgcgccaggcttcagccagccgccttcggtcaggcgcagcagcgtctgttcgcccaagcccttgccatagggcggatcaagaaaggccaggtcgaacgcctcgccggccgagccgggccgcacgccaaggtccgtcgcactgcgtcgatgcacccgtgtgcgtccgaacagaccaaagctttccgcattctcgcggatcgcgccgcgcgcgccgtcgtccgtctcgacgaacaggcagaatgcggctccgcgcgacaccgcctcgaaccccagggcgcccgaacctgcataaaggtcgatgactcgcgcctcttggagcggctcggcccaggcggcgtgctccagcacgttgaagatcgcctggcgcgcgcggtcggaggtcgggcgcgtgccctgcccctccggcgcgacgagcgtccggcccttcaggcttccggcgacgatacgcaacggtcagctccggggcgtgcggggctttccgcccggtccacggccgctggtccccgaaggtccggcgggcttgccgccggtccggggcttgaagtcgcgcccgctggtcttgccggtcggccccgcgcggcccgacggcttcgcgcccgccggcttgcggcggtcgtcgatgaactggtcgtcccggggcttgaaggcgcgtttgggtcgatcgacgtccgcgcgcggccgttcgccctcgggggcggtgcgctcgcgcggcttaaaggtcttggaatgttcgaacttgggcttggccttggcccacccgtccttcttggccggacgttcgcggcggtcgaccgcatcggcctgggccgtttcggcggcgcgcacgcggctgggctttctggacgggtccgacatggccgagccagagcgtcccttgacgatgggcgtggaaatgcgacgaccggggatcggcgcgggcgtctccaccgtgttgccggtcggcaggttgtctggacggatgtgttcgcccagcatctcgcggatcacgcgcggcccgacctcctccaccgccccgaccggcaggacgtccagccggaacgggccataggccagccggatcaagcgattgaccgtcaggccgatcgactccagcaccttgcggacctcgcggttcttgccttcggtgatggagacgctgacccacaagttggcgggggccttgccgtcctcggacttgctttccttggccttgtccagcgtcgcttcgatcgggccgtattcgacgccgtcgaccgtcacgccgtccttcagcttgtcgaggtcggcctgggtgacgcgtccgcgcgcccgggcccggtactgacgcaccaaggcggtggacggcagctcaagcgcccggctgagctctccgtcgttggtcagcagcagcagcccctcggtcgccagatcgagccttccgaccgagatcacgcgcggcagaccggccggcagggcgtcgaacaccgtgggccgtcccgccgggtcgttatggctggtcagcaggcccgccggcttgtgatagcgccagacgcgcgtggcctgcgcagccgtgatcggcttgccgtccacggtgatcacgtcctcgcgcgtcaccagggtcgccggcgtatccaggatgcggccgttcaccgccaccttgcccaggccgatcagccgctcgacctctcgacgcgaggctatgccggcgcgcgccatggccttggcgattcgctcgctgcggagcgaggcggcgggcgccttgcttgtctttgcgccatccctgccgccatcccttccgcctgggcgcggacgctctccgcgcggcttgtcgccaaaggatttcgccccgtcttcgctcttgcggaaggcgggcttgcgggggccggaagcgcggtcggcttgacgcgcgaagggcttcttgtcgttgtcgtctgtatggcggaccatgatgagcggttcatgcgcatggcgctggacgaagcgcaagcggcggcggacgcgggcgaggtcccggtgggcgccgtcgtggtcgatccggcgaccggcgatgtggtctcgacaggcgccaacggcccggtcggcgcacacgatccgaccgcccatgccgagatcgtcgccatgcgtcgcgcggcgcaaatgctgggcaattacaggctcaccggcctgacgctctatgtgacgcttgagccttgcgccatgtgcgcgggcgccatcagccacgcgcgcatcggccgggtggtctggggggccgacgatcccaagggcggcgcggtgatccacggcgcgcgcgtgttcgaccagccgacctgccactggcggcccttggcggagggcggcgtcctggcgacggaggcggcggagacgctgcgcgccttcttccgggcgcggcgcggaacacgcacacccagcggacgttaggcggatagccgcccaagcggcgccgttacgcacgagggggcgttgcagccatgaagcctgatctgccgcagttgatgctggtgagcggcctggccgctcttgcgctgttgtccgcctgcggtcctgatccgtccgaggctccggccagcggcgatgcggtcaagcaacgcgccatggaggcccagaccacgcgccgacgcaccggcgcggaaatccaggatcgcgccctgaaccgcgtcatccaggccgtctatctgtgcgagaatggcgagcgcctgtcggtcgacttcgacaatccccgccagatggcgacggtgcgcacctccaacggcgaggcggtcgatctctatcaggagcgtgcggccgacgggctgtggtaccgctccagcaccaccgaactgcgaggtcggggcgccttggccacctggaccagccagggccgtccatcgacagagtgtcgcgcgatcgactaggcctcggcgccttcgtcgatcaggaaggcccggacttcgcctgcgtccacacccttggcgacaaaggcccgccccacgccttgcgccagaatcagggtgagcgccccgccctccgccttcttgtcgcccgccatgcgccccagcagggcatccgccgagaagacgccggcttgaacaagccgtgtcggcagtccggattcggcgaccgcagcctccacccgttccacatgacgcgcttcgcacaggccccgccgagccgagtagcggaaggccatggcgcagcccagcgccaccgcttcgccatgcgccagcgccgcttcttcgaagcccagctcggcctcgatggcgtggccgaaggtgtggccgaggttcagcagcgcccgcttgcctgcttccttctcatcctcgccgacgatggcgctcttgatctccaccgaacgcaccaccgcccgctgcagggccgccggatcgccggccgctcccgccgcgccctcccccgccagccagtcaaagaagccgggatcgcagatcagcccatgcttcaacacttcggcccagccagatcgcaactggcgctcgggcaacgtcgccagcacgtcgatgtccgccagcacaagacgcggctggtgaaaggcgcccaccaggttcttgccctggggcgtgtcgatcgccgtcttgccgccgacggaggaatcgacctgcgcgagcaaagttgtgggaacctgtatgaaatcgatcccccgcatgaacagcgcggccgccaggcctgcgagatcgccgaccacgccgccgcccagggcgataaccagatccttccggtccagaccggcttccagcagccggtccagcacccgctccagctcggcgaaggacttggacgcctcgcccgccggcaccgccaccacgacgctgtcgatgcccgcttcggtcaacgaagcctgcagcgccggcgcatgcagggcggccaccgtctcgtccgtcacgatcaccgtgcgccgctgcggcgcgaagacagcgatgcggcggccggcgtcagccatcaagccgcgccccaccacgacatcgtagggagcaaaggcgccgccgcttacgggaatggcgatcatggctgattttcctgcgctcggcggcttcgccagtggcgacgaagctgtcggtgtatcgcttccaccgcctgtctgtgggagcccagccccacgtccacaatcagatcggcggtggcgtagatcggcgcccgcgcctgagacagcgtggtcagaacctccatcgggtcgcggtctctcagcagcggccgggtgtcgcggcgccccacgcgctcggcgatcaccgaaagctccgcccgcatccacaccgtgtcggcttgggccttcagtaaggcccgggtgtccgggttcagtacggcgccgccgccggtcgccagcaccagcggcggcccctccagcagtcgcttcatcacccgcgcctcgcccgcccggaactcggcttctcccagcgccgaaaagatctcggacaccgtcatgccggccgccgcttcgatctccacgtcgccgtcggcgaagggcatgcccagacgctgcgccagcctgcgtccgaccgaggattttccgacgcccatcagtcccacaagcgctatggtgcgctcgggcgcggagccgcgccgcccgctcatgcagccgatcccggcgcggcgaacgcggcggcttgaagcggaacggggcgaacgcgggcgggcatgatcgggtcatcctctacaccaagcacggcggctcgccagcctcggggcctcggagcgccggcgtgaccccgcagatcgaggcctttcttgagatgatggcggtggagcgcgacgcgtctccgcacacgctgtcggcctacgcccgcgacctcgaggatgcggatacgggcgccgggaacctgttgactgcggatgaagcggcgctcgaggtctggtatgccggcctggcccagcgcggcctgtcggcggcgacccaggcgcgcaggcgatccgcggttcgccagttctatcgcttcgcactgggtgagggctggcgcggggacgatccatcccggcgattggatgcgccgagccggggacgacccctgccccaggtgctgagccgcgaggagatggagcgtctgctggcggccgccggatcggaggacaacgcgcgcgggcagcgcctgctgaccctgatggagctggcctacgcttcgggccttcgggtgtccgagctgctggcgctcaaggtcgaggcggtgcggcgtgatcccgcctatctgctcgtgcggggcaagggcggcaaggagcggctggcgcccctgaacgccagcgcgcgcgaggcggtcaaggcctggcttgccgtgcgcgacgcccgccgcaagccgggtgccccggacagcccatggctgtttccgtcctccggccgcagcggccacctgacgccacgccgcttcgcccagttgctggaccagtcggcgggggcggcggggatcgatcccgcccggatcagcccccacgtcctgcgccacgccttcgccacccacctgttggagggcggggccgacctgcgcgtggtgcagacgctgctgggccacgccgacatttcgaccacccagatctacacccacgtcgcgaccgaccggctggccgaggtggttcgccgcaaccatccgcttgcgcgcgacgactgacggcgcatattcggcaaatggcgaattccttctacgttaaggcgatctgggatcccgaggccggagtctggtgcagcgaatccgacattcctggattggtcttggagacagcgaccttatccgagttcgagtccctggcccgtcatttcgcgccggaactgcttgctgagaacttggatatccacggcccggtgccggtgagattcgaagctgtgggcggcttcgacgtggtcgcggcctgaatatagccctcgctgcaaattcgaatggagacttcaggcgtcactgatcggaagcgcggcgatgcctaaggacttttacttcgaactgacgagcctgctccatgaggcgggatggcgacgcgttctcggagccaagggcagtcacgaaaaatggcgccatcccgatcatccccgggctgtgatcgtgccgcgctcaaaaagccggcacaccgcaaatcaggtcctcaaacaggccggcctgccaaaggcgttctgagccgtcgcttgcccggcggcatcgacgtctttaggttgccccgccttgccttggggcgccttccgccgcccgctgtttccggacgccgtcatggccacgcattatctcgacttcgaaaagccgatcgccgatctggaagccaagatcgaggagctgtcgctgctgtcctcgacggaggatgcgttcgagaccgagatcgcggggctgcgccgcaaggcctcgcagatgcggcagaagacctacgccgcgcttgatccctggatgaagacgcaggtcgcgcgccacccgcagcggccgcacctggtggattacatcgccgggctgttcaccgacttcgtcgagctgcgcggcgaccgccagttcggcgacgaccaggccatcatcggcggcctggcgcgctttcgcggccgccccgtgatcgtcatgggccatgagaagggccacgacaccgcgacccgcctgacccacaacttcggcatggcgcggccggaaggctaccgcaaggcggtgcggctgatggacatggccgaacagttcggcctgccggttctcagcttcgtcgacaccgccggcgcctatccggggctgggcgccgaggagcgcggccaggccgaggccatcgcgcgctcgaccgagcgctgtctgacactgggcacgccgtcgatcgccacgattacgggcgaagggggatcgggcggcgccatcgccatcgccgccgccagccgggtgctgatgctggagcattcgatctattcggttatctcgcccgagggcgccgccggcatcctgtggcgcgacggcgcgcgggccaaggacgcggccatggccatgaagatcacaggctcggacctgatcgggctcaagatcgtcgatcgtctcattcccgaaccgacaggcggggcgcatgccgatccccaggccgccatcgccaacgtcggcgactgcctggccgacgagctgcgcagtttcgacggcctgtcgacggccgaaatccgcaagcgccgcgccgaccgcttctacgccatcggggcgcgctgaaccgcttaactttgcagtagcgttaacgtctcgcacatcgccgtcatccatgatcggacgttcagacgtgcgactcgttgggggcgaagatgcgcaatggaccgccgctcagccgtgagaccacggcatggcgttgatcgcggacgcgctgcgcgacagcgcggtgttcaacttcgcgggcgcggtcacaatgatcgtggacgattcgcgcttctcgctggcgctgaccgccaacgccttgtccggcttcggcatccgcacccgtcatgcctgccacagcgccgccgaagccatccgcatcctgaacgagcgaacggtggacctgctgttcgtggactgcgagatgccggacatggacggctatcagcttgtccgctggctcaggcggtcggggctggagcccaacgcctatgtgccggtggtgatgacggccgggcacgtgcgccgggcgcgagtggcggaatcccgcgattgcggggcgaactttctgatcaccaagccgttcagcgcagcgatgctgcttgagcgcgtgctgtgggtcgcgagagacacccggccgtttctgcaggtcggggactatctcggccccgaccgccggttcaagaccgacccctatgacggccatgagcgtcgcgccgacatgatacgcaaggcgcgcttcgaggccgagcagaacgaagtggaccagcccgcgtgagcgtagtcacccgaatccagaggcgatcccgcctctccaccctggtggaccagcccggcggcatcagcgcgggcgtcggccttgcgcgcgcacgcgccaatctccaggccatggaaggcgaagcccgcgaaatcgtggcccagcggatcgccgatctcgccgccatccccgctccgcaggatggattgctgacggccgaggggctggaggaggtctatcgcggctccgccgccatgatcgacgccgccggcccattcgccttggcggacctgtgcacggcggcctccggcctttgcgacctgacagacggcgcaggagtgtcggactggcgtgtcatcgcggttcacatccaggccctgcggctgctgatcgccctgccggaggaggctgtcgccgagcgcgagcagatactgctgaacctcgacgacgtgcgtcgccggaagctgcctccggtgggtcagtccgccggctgaacctcgcccgcgcgcgtctgcttgcgccacagggcggcgtattccccgcccacacgcgccaccagttcgtggtgagccccgcgctcgatcacccgcccggccttcagcaccagtatctggtcggcgtcggccacggtcgatagtctatgggcgacgatcagcgtcgtgcgcccttgacgcgccttcctcagcgtcttctggatggccgcctcggtgcggctgtcgagtgcgctggtcgcctcgtccaggatcaggatgcagggatcggccagcagggcgcgggcgattccgacccgctggcgctcgccgccagaaagcttcaggccccgctcacccacccgcgtgtccatgccgtcgggaagcgcccggatgaagtcagccagttccgccgcctcggccgcttcccagatttccgcttcgctggcctctggacgggcgaaggcgatgttgtgcccgatgctgtcgttgaacagcgccacgtcctggggcaccagcgccaccgcagaccgcagcgatccttgcgtcacctctcgcacgtcgcgcccgtcgatcagcacgcgtccggcctgggggtcgagcaggcgcagcgccagcttgaccaccgtcgacttgcccgcgcccgaggggcccaccagcgcggtggtcgtgcccggcgcggcgaagaagctgacgtcctccagcccgttcgcgcgcgcgtcatggcggaagccgacaccatcaaatgcgagagaggcgccgcgtgcgtccgccggacgatcgagcgcacgcgcctgggcgctgtccgccacctgaggcgactggcggagcacgcccatcatctcctccatgtcgataaaggactggcggatttcccgataggcgaagcccaggatgttcagcggcgcatacagcgagatcaggatcagcaccgccgcggcgacgtcgcccggtcccatccgcccggccgccgcctcgaacccggccatgaccgccatgacgcccaggcctaggttcatgatcagcccctgcgtcgcgttcagcagcatcagcgagccattggccttcagcgaggcctgctgatactcgcccagcgcacggtcataggcgcccgccgtgcgcgtctcggcgccgaaggccttgaccgtctcgtagttcaagagcgcgtcgacggagacgccggccgcctcggagtccgcggcgttcatcacgcgacgatgccccagccgccagttcgacagggcgaaggtcagggcggcgtagacgccgaccaccgccaccgccaccgcgccgaacctccagtcatagcgcccggcgagcaccgccgcagccagcaccagttcgacgccggtcggaatcaggttgaaggctaggatgcgcagcaggaagtccaccgcccgcgatccgcgatccatcgtgcgcgacagggttcccgatcgcttggtctgatgaaagtcgagcgaaaggttcagggcgtgtgcaaaggtctcggtcgccgccgtccgctgggccgccgcgcggacaggggcgaagatcacgtccgacagctgcggcgccgccgaagacagaaaacgcacgaacgcccagccgatggcgaaggcggcgaagccccagcctaccgctgcggccgcgccttgccccgccgccagccggttgaccgccgcgccaagaaccagcggcgccagcacgcccaacgccttgccccccagcgtcaggccgatcgcggacgccagccgcagggtcagatgcggcgcatgcgagcgccgcaccagaccggccagatcggccagcgccttccaaccatcgacccgggattgctgatcccctgttgttccctgcgcccgcgtcgcggcgtcggaacgccgctggccggggcgttcaccacgcatcgccatggtccttcatatggaagtggttgatcggcgggggaagagcacgcgggcgcccggctcagccgagaccggcgatcgcctcgaccacctcgtcgacggccgccgggtccgtcgcccaggaacagacgaagcgcaccgacccgtcgtcaaagcggtagcaggcccaacccagggcgttcagccgtgcatgcgcctcttcgggcatgcggacgaagacggcgttggcctcgaccggatgcgccagcacgaagggcgatcgcgcggcgataccggcggcgagccgttgcgccattagattggcgtgggcggcgcccgcatcccagtcgccgctttccagaaggcccagcagcggccccgacagcagccgcgccttggacgccgtctgcccggcctgcttcagccgattgtccaaccgccgcgccagcgacttgtcgaacagcacaatggcttcggcgcagggtcccccggctttggcgccgccgaacaccagaacatcgacccccagccgcgcgatctgtgtcaggtcgaacccggccgcggccgcattggcgagccgcgcgccgtccatgtgcacgccgaagccgcgcagcttcgccggctcgatcaggtggcgcagttcctcctcggtgtagaccgcgccgtattcggtggcctgggtgagcgtcagggcggcgggcggctggcgatgtccgacctccggctcgtccagctgggcgtgcagcgccagcgggtcgatcttgcccgagaagcccggcaggccgatcaggcccacgccatggccgaaaaagcccggagcacccgtctcgtcggtgcagacgtgagccgagttgtgcgccagcaccgcttcgaacggctgggccagcatcgacagggcgatggcgtttgcggccgtgccgctgaagacgaagcgcacctcggcgtcggcgtccaggcgcgcgcggatcgcgtcggcggcgcgggccgtgatctcgtcggccccgtaggcccgggcgaaggcttcgttggcgcggaccagcccgtcaacggcggagggcgccatgccggcggtgttgtcggagccgaaatcgtatcgcatcaggcgaccttctccctgtcgtcgatcgtctggacgcgaaccacaggcacgacgttctcgtcgccatagggcaccgcgacctggtgggggaacgggatctcgatgccggcggcgtccagcgcctccttgccgccttgcatcaggtcggcctgggtctgccaccagtcgccgacctcgacccaggcgtgcagcgtcacctccaccgcgctgtccagcagggccgtgacgccagtccacgggtgcggatccgtcagcaccttctcgtgcgacttcgccatttccgccaacacgcttcgcgtccggttcagatcttccccatagccgacggtgaacttgatctcgatccggcgcgtcttctgcccggtcagatttgtcacgacgtcgctgagaaccttggagttcggaataacgatcttgtggttgttggcgttggacagctgtgtcgtgaacagatcgagccgctgcaccgtgccggagacgccgccgatgtcgatcacctcgcccacgcgatagggccgaagaaccagcagcatgaagccggacgccacgttcgacagcgtgccctgcagcgccagcccgaccgccagcgacgcggcccccagcaccgcaatgatcgaggtggtctgcacgcccaaccgctgcagcaccgcgatcaggccgatgatcaacaccagcacccgcaccacctgcaccgagaagctcagcaccgtcgggtcgtgccggaagccgcgcacgcgcgacagcacacgtcgcgccgtcttcgccgcccattttgacaggaacagcgtcgccgcgaggatcagcagcgcgatcgagatgttgatcgcgaaatcgccggccgcgctgaccagcttggcgatcatggcggcgtcggacgcggccgcctgacggcccgactcagccgcttgggtgatgggcgctacgagttcggtcatggaagcggggtctaacgcctggcgcctcgattggaaccccacccggtcattttcaccgctttgacacccggccgccgctgctctcgatggcgtccagcaggtccatgacgctgtctatggtgtccgcctcgcgcgccggcttgtcccagcggatgcggctgacgcgcggaaagcgcatggcgacgccggacttgtgccggggcgagcgctgcagaccctcgaaggcgacctccagaaccagaccgaagtcccgctcggcccgcaccgaccgcaccggcccgaaccgctccaccgtgtgatcccgcacgaacttgtccagttgcttcaactcctcgtcggtgaagccggagtaggccttgcctatgggcgtcagcacgccgtccggcgtccagaccccgaaggtgtagtcggagtagaagctggagcgttttccatgtccgcgctgggcgtacatcatgacggcgtccaccacgtgcggatcgcgcttccacttgaaccacggtcccttgggacggccggccagataggcgctgtcccaccgcttcagcatcaggccctcggcggcggcgcccactggcgggtcgacacgcaaggtcgccagatcgttccaggcttcgtatggcacgacgggcgacagagccagtcgcgcgccgcctccgcgcgtgaccagcgcctccagcctcgcccggcgctcgcgcagcggcagcgatcgaagatcctctccgtcttccgccagcaggtcataggccagcacgccggccgggtgcgccgccatcagcttggcgtccaccgtcttgcggttcagccgctgctgcaggtctccgaacggcgccggtcgtccatcgcggatcaccagcagttcgccgtcgatcgcgccttcaaactccagccccgccatgacatcgggaaaggcgccggagatttcgtcgcccgtccgcgagtacaggcgacagacgccagcctcccgcaccgcctgcaccctgatgccgtcccacttccattcggcggcgtaatcagccggcgacagcttggggaagtccaccgcctcgtctatggcgacggccagcatcaccggccggaaacgcccgggcgcatcggggctgggccgctcggcgcggccttcgagccaggcgaacaggtcggcgtagggcggctcgaccgcgtgccacacctcctccagatcggacacgtcgaccgccggcagcggcgtcccggccggctctccgtcgggatcgggaggtgcgggcgcgacgtccggccggatcatcgccgccgccgtctttgccagcctggctgacaggcccaccctcaacgccccggtcaccagcttcagcagggcccagcggccctgcggctccaaggcgtcgagccaaccttcgatcagagggcgcacctcattgcgaccggccgtgcgcagcgcctccaccacctccgccagctccggctcacgattgggtcgatagtccggatcgcgcggccagatcagcgccgccgtctcagcgaggtcgccgacgtagtcgtaggaccagccgaacagcacgggatcgacccgcgcctcgaccgccttgcggatcatggccggcttggccgcatcaaacgtcaggtcgcccgtcagcgccgccagagcccagcctctgtccgggtcgggcgtcgtcttcagatagtcgcggaccagcaccagcttggcgttgcgcgaggccgtcagcgacaatcgatccagcagttcggcgaagccgcgcatggcgttccatagacaagcgtcgccgtgatcgacgcccggtcagaacgatgcagggggcggcgggttgccggacctcggctcaggccgcgacggcctcgtgcgccagtcccagctgacggacctgttcgcgcccaccgggcacgtgggtcatcagctgcgccaaggcggcgaagtcgatgggcttgttcagataggcgtcggcgccggcgtccaggccggcctggtggtcctccgaccgtgcggaggccgacagcaccaccatcggagtgtcgcggttcacgccctgcccgctgcggatcatgcgcgtcgcggtcagcccgtccatcaccggcatgttcacatccatgatgataagatcgaagggctggtgctgagcgacgtccacggcgatctggccgttctcggccgtcgatgcggcgtggccggccgagcccatccaggcctccaggatcatccgattgaccgggtggtcctcgaccaccagcacgctcagagcctggccttcgcttctctcggcgacgcgggtttcgaccggcgccggcctggcccattccaccacctcggcctccaccgtcatggtgaaggtagagccgcttccgacttccgaactgaccgagatgtcgccgcccatgatgttggtcatgcgccgggcgatcgtcagccccagacccgtgccgccgaagcgacgcgtcgatgaggcgtcgacctgcgtgaacggttcaaacagcagatcgaggtcggccttggcgatgccggaccccgtgtcggtgaccatgaagtcgaagcggacgcgattgggggcgacacgggagccgcgcgtccggaacgtcacgacgccctcgtccgtgaacttgactgcgttagacaggaggttgtgcagcacctggcagacccgcaagggatcaccgcgcacgaccgaagggacatcgccctcggtgatctgctcgaacccgagccccttggcggcggcctgcgcctcgaacgggccggtgatccgcttggcgaggtcgtcgatggaaacatcgacggtctcgaaggtcatcttgccggcctcgatcttggtcatgtcgaggatgtcgttcagcagcgacagcaggttgtcgccagagttgcggatgatcgacagatactcccgctgcgtgccctcgagcctggtcgcgccaagcagttgcgcggcgcccaggacgccgttcatgagcgtgcggagttcgtgcgagatgacgccaaggaagctcgatttcgcctcgttggcggcggccgccttgtcacgagccgtctccaattcctcgatcaggtgcgcctgatgctcctgaaaggcgctgatgcgcccttcgcgcagcatggtcatcatgaccagcacgaacagaccggcggcggtgaagggcacaagcgccagcaacgaccagaactgcggcgttccccaaaggctccccagcatgatcaacgccgccgctgaatagggcgaggagatcaccagcgcctggcgcggcgagctgcgcagctgcgcgaagacaagcacatagccgccgatcagcagggctatggccgcggttgaaccaaacggattgtcgctgaaccacgcaagcaggggcgcgaccgcccaggccgccgtggtgatcgtcgccaccgcaggaaaaatcaggccccaccccttgtcgacgcgtcggctgacccttcgttcaaccacgccgcgcagggcgccggcggccagggtgcctacgaaccagaccaacgcctctatgccgccgatcacgcccagcaatccgacggcccagctggcgatgatgaggtagcgcagatactgcgtctgcaggatcgcctttagggcctgggcggcgtcgccggccttctgatcgccggccctgccgtcgatgctgtccgcttccaccatgcgccccgcccctccaccctctttaactgcggaacgctagggtgaaacggctaagacagtctgaacgaatcttggttaccgatcattggtctgcgagtcttccacaggcgtgagcgcccggacggatagggcatggacgggcccggccagttcagcccgaagcaggtcgttgacggcccgctggcgcgccaggcgcgactggccctcgaaggcgtcggacaccaccacgatgttgaagtggctttcgccgccgggcttggcgtccatgccgccctcgtggtggtggccggcgtgccgccagctgtcgtcgacgatctccagctggctcggggacaggctttgctgcagtttttcgcggataatcgcggcgacggggccttcggacatgatcgcttccttgatggcgtccaattcggccctacacttcggcggatgcccgcttcgtttcaatacaagccgcgcttcaccgacattcgagtgaagccgcccaagcctggcgaaaaggtcgaggacccggatgttctgcacctcaagccgggcgaaaagccgtgccagtggcccgactgccgtcgcgccgcgaccgcgcgcgcgcccaagtcgcgagagcggctgaacgacttctacgagttctgtcaggcgcacgcgggcgagtacaacaagggctggaacttctacgcgggcatgagcgagggcgaggtccgcgccgcgcaggaggacgaggccatgaccggcgggcggcccacctgggagatgaaggccggcaagttcagccgtgaggccgccgccttcgcctccaaaatgggcacgaacaacacgcaagggtcgggctcctggcgcgacagcttcggcctgttcggaagaaagggcgagcagacgccgaacgcgcccggcgaggaccgccgcatcggcaagctggagcgcacggcgctggccgacctcgacctcgagccgggcgccgacaaggctgcggtcaaggcgcagtaccatgccctgctgaagcggttccatcccgacaccaacggcggcgatcgcggcgcggaagccaagcttcagcgggtcatcaaggcctggaagacgctgaagaaggccgggctggcttaaccgctcgcccccgtggaggcggtcaccagcggcgcagaaggctcacggaagtagcggtcgatgccgtcggcgacggcccgcatcatgcggcggcgctggcgctcgtcggccagcaggcgctcgtcttcggggttggtgatgaagcccatctccagcagcacggccggcacgtccggagccaaaagcactgcaaggcccgcgtcgcggtggctgcggcggagcagcggatgctcaaccgcttccaggtgggtcagcaggacccgcgcgaactgggccgaacggttctgtgtcgcgcgctgggtcatgtccagcaggatgcgatccaccgatggatcacggccgggaagccgtagctcgcgatgccagtccgcgccgcgtgtgaactcgcgcaccgcgcgacccgcgccctgttcggacagggtgtagacgctggccccgcgcagagccgggtccgcgccggcgtcggcgtgcagcgagatgaacaggtcggcgtccgcctgccgcgcaattgagacccggcggtagagatcgacataggcgtcacccgagcgggtcaggcgcacgcgatagcggccggtcttctcaagctccgccttcagctgctgggcggcggccaaggtcacggcgctttcccgaagatgagcgccgctggcgcccggatcgcgccctccgtggccggcgtcgatcacgatcataggcttgtcggtccgccgcggcgccggcagcggctgcgaagttgggcgcgtgggctcgacgttcggcacgcccgcgcccttcgccttcacgtcgatgacgtagcggtaatggcccacgccgtcgccgggcggcagcaggaagcgccgttcgatctcgccgttcttggccagatccagctgcacgcgagacgcctcgccctgcgcgccgacccggtagctgcggaccaggcccgagccttcgccggacgctccacgcccggcagccacctccagcagcgaaagtatgacctgcccctgcgttccgtcctcgatcacgcgcccctgcgtcgcgcgctccagatcgatgaccacgcgggtgcgctgtccatcgccgccgaagcggacgcccagcagatcgccctgcgcgcctgacgccagtcctcgcccggccagcatcagcagccccaggcagatgactgcaaaggcgagcgccgtcatcgcccactcccgcaggccccagcgcgacagatccagaaatacgcgaccgttcattctgacggcttcacccaacaccactggccgacataatgcgcgaaccttcttggcggggggttaaggggcaggcggcgggggagcttttaattgcgctccatcgtgcttatgcttggttccgctcgcgaaccgatcgcgccgctccccgttcgggcgatgccggcgcgccctcctcgcggcgctgtgtttcacctcttccgaggaccgacaggcatcgccggcggtccggagaaccggtgccggatcgccgccctcaggccgcgcccggcgccaggacagacgaccttcatgggccttttcggctgcgatccccaacggcttgttcaagccagcgccgcgttccgcggcgggatgacgcgcgccccggccctcttacccattcggcgagccgccgcagcccctgccagatcactggccgggcgggcccgagcgcgccagagagagacccttcatgtcaaagacaatgctgatcgatgcggcgcacgcggaagaaacccgcgtcgccatcgtggacggacgccaggttgaagagttcgacttcgagtcgaaaaccaaacgccagcttcgcggcaacatctatctcgccaaggtcacccgcgtagagcccagcctgcaggcggcctttgttgaatacggcggcaatcgccacggcttcctggcctttaacgaaatccaccccgactactaccagatcccggtcgccgaccgcgaagcgatcatggccgaggcgcacgacgacgccgaccacgccgacgacttgggccgcgaaagcgacgaagagaccgatccggaagccgccctggccgaagaagagcggctgaagcgccggctgatgcgccgctacaagatccaggacgtcatcaagcgccgccagatcctgctggtgcaggttgtcaaggacgagcgcggcggcaagggcgcggccctgaccacctggctgtcgctggcgggtcgctactgcgtgctgatgcccaacacgggcaagggcggcggcatctcgcgcaagatcaccaacacctccgaccgtcgccggctcaaggccgccgccgccgcgctcgaggtgcccaagggcatgggcctgatcatccgcacggccggcgccaagcgaaccaaggccgagatcaagcgcgactaccaatacctgctgcgcctgtgggagacgatccgcgagaccaccctcgcctcccacgcccccgcgatgatctacgaggaggagaacctcgtccgccgcgcggtgcgcgacatgttcgacaaggacttcgacggcattcaggttgagggcgtgcagggcttcaaggaggcgcgcgacttcatgcgggtgctgatgccctctcaggccaagaaggtgcacctgtaccagggctcgcggccgttgttcgcctccaacggcatcgaggacctgctgacgcagatccaccagccgatcgtgccgctgaagtccggcggctatctggtgatcaaccagaccgaggcgctggtcgccatcgacgtcaactcgggccgcgccaccaaggagcgcaacgtcgagcagacggcgttcaagaccaactgcgaggcggcggtcgaggctgcgcgccaactgcgcctgcgcgacctggccggcctggtcgtcatcgacttcatcgacatggacgagggccgcaacaaccgcaccgtcgagaagatcctgaaggacgccttgtcggcggaccgcgcgcgcatccagatgggccgcatctcgcccttcggcctgatggagatcagccgtcagcgtcgccgtctgggcgtcatcgagggcgcgaccgaggcctgcccgcactgccagggcgccggccgcatccgctcggccgaatcggcgtctctggtcgccttgcgcgccgtggacatcgaggccggcaagaacggcgcgggcgcgatcgtgctgcgcctgccgaccgccgtcgccctctacatcctgaaccacaagcgcgagtatctgcagagcctgctggagatgcgcggcctcaacgtcgtaatccagatcgacgacagcctggcccaggccgagcacgccatcgagcgcaccgagaccaacgaggacttcgtcgcaccggaagcggaggtcatcgacctgaacgacggcttcgacgacagcgcctttgaggatgagggtgacgacgaggacgaggagatcgacgaggacgacgacgaggacgacctgtcgctcgatcgcgaagacgaagacgacgacgagccgcgcgagcgcgccgagcgtcaggacgagggtcgcggcggacgccgccggcgccgtcgtcgcggcgggcgtcacgaggtggagactgtcgagagcgaagacgattcggcacccgtcgaggccggcgcggagagcgacggcggcctggcgggcgacgacgaggacgagaacggccgtcgccgcagacgcggccgccgcggcgggcgccgcatccgcgaggacggcgagcgcgatgtcttcgcctgggtgcgcggccgcacgccgtcgctggatgatccctatgtctggttcgatccgctgaaccccggcggcgcttcgtcgtcgaagtctgaagacgagcagccctccttggcggaggttcgtcaggacgaaagcggcgaagagggccggggcggacgccgtcgccgtcgtcgcggccgcggccgcgaccgtggcgaacgctcgggcgcgcccgccttcgaggcggccggtgaaacggagagcctggaggacgccggcgcttcgcaggaggcttcgcccgcgcggagcgatgccgaaccgacacccgtcgcaatcccggccgagccgcaacgtcgccgcgtgcgtcgcaagagcgccgctcaggccgtgttcgaaccggctgtggacgctgaagagacagatgatcagccgatcgccgaggccgcgcctgcgcttgaagcgcccatggctgaagcgtccctgtctgaagcatccggagccgacgcggtcgaagccgatttgatcaaagcggatcaacctgacgcttccgcgcaggtcgagccggccgaaccgggggaccttggcgagcccgtcgtcttggacgtcaccccgcaggaggcggaagccgaacgcatcgaggccgcacaggagccggagccggtgatcctcagccaggctcctcagccccaccggccggaagtcgacgttcaggccctgatctcgcaagatccgaaccagatcgtcgcgccgcctgaaaagcccaagcgcgggtggtggcgccgctgatcgcggatcgctagattgaggaacgacgggcgggggcccaggctttggagcgcgccatgaactggcttccccgccctgcgtcctgccttcgggcgctgcgccgccttgtcggcgcagccggtgtcctggcggtgctggggacggcgggccaggcctcggctcagagcgtgatccgcgacaccgagatcgagggtgtgatccgagagtggtcggacccggtgttcgacgccatgggcctggtgccggcggacgtcgaagtcctgctgataaacgatcccgagctgaacgccttcgccacacgcgggcggatcatggggatcaacacgggcctgatcctgcgcaccaagacgcccggcgaattgctgggggtgatggcgcacgaggcgggccacatcaagaaccgccacaccctgcgcgatggggcgcagaacgcggccaagcagccgttcttcatgaccatggcgctgggggcgctcgccatcgcggcgggccaaccgggcgccggcgccgcgctgatcggctcaagccagtatttcggcacactggacgccctgcgctacatgcagagccaggaaggcgaggccgacctgaccggcgcccgcgcgctggaggccgccggacaatccggacgcgggctggtggagtttttcgagaacttccgctctcaggaggtcttctccgacagccgccgctatccttatttccgcagtcaccccctgtcgtcccagcgcatcgaggcgctgcgccggccggtcgaggccgccgcccactacaatacgccggaaagtcccgagcgcatcgcccagcacaccctgatcctggccaagatgcgcgccttcatggaccagccgaacgccacgctgcgcgcctatcccgagagcgatgcgtccctgcccggccgctacgcccgcgccatcgcctggtatcgcgcgggtcagaccgacaaggcgctctcggcggtggacgccctgatcgccggcgacgtctccaatccctattattgggagctgaagggccagattctgttcgaggaaggccgccccgccgacgccatcgccgcccacgccgagtcggtgcgcctggagccggacgcgcccctgcttcgcgtcaacctggggcatgcgctgatcgagacgggcgaggcgggcaacatcgccgaggccgtcaatcagctgaaacgcgccacggtggccgagcgcgacaacaccatggcctggcgcctgctggctcaggcctacgccgcccagggcaaggagggcgaggcgcgactggcttcggccgaataccacttcgccgccggtcaggaacagcaggccacccagttcgcccttcgcgcccgcagcctgctggaccccggctccatggagtggcgccgcgcggtggatatcgtgctggcgtcgggggccactcaggacgacctcagcgatcttgaccggcgcgaggcgctgcgtcgccccgccaccctgaactagacttgcccgaagaagagacgtgatgaccgacgacgccgcccctccgcccgcacccccaccccccgccgaaagaagacggcgcggctggacgggtccggccgccctggcggtctcgctggcggctctgggtctggcggcctggccctatgtcgcgcccgatgcgttcggatcctgacggtgcatcgctacatggtcagccatcccgaggttctgcaggaagcgagcgccgccctgcagcagcgcgaggagcagggacgcgtcgcctctatcaatcaggcggcggcgaccaatcccagcctgctggcggtcgacgcccgtgaccctgcttttgggcctaccgacgcccgcgtcacggtggtcgagttctttgatttccgctgccccggctgcaaggcggtggcgcacgactatcgcgccctgatggcggcgaatcccgacgtgcggttcgtcttcaaggactggccgatcctggaccgcggagaggacgtcacgtcccagtacgccgcccgcgccgctctggccgcgcaccagcagggcaagtatctggcggtctacgacgccctgatgaacgaacgcgcgctgaacgtagaggcgatcgaccgcatccttcaggcgaacggggtcgatctgccgcgggccaaggccgccatcgcctcacctgagatgacccgccacatcgccgacatccacacggcggcggccgccttgggtcttcagggcacgcccaccttcttcatcaacggcaaggccagcgcaggaatcgacccgcgcgaggtcggccagctgatccaggcggcgaaacgctagatcaggccggccaggggcgaagacggatcggcgtacaggcgcttggccatccgccccgccagataggcttcgcggcccgcgatcaccgcatgtttcatggcgcgcgccatgcggatcgggtccttggcgccggcgatggcggtgttcatgagaaccgcgtcgcagcccagctccatggctcgggtcgcatcggacgccgtgccgacgccggcgtccaccagcaccggcacgcccgcctgctccacgatcaggcggatgttgacctcgttctgaatgccgagccctgagccgatcggggccgcagccggcatgatggccgaggcgcccgcctcctccagccgcttggccatgaccacgtcgtcggtgcagtaaaccatgacgtcgaaaccgtccttgaccagcatgtcgagcgcgcgaagcgtctccaccatatctggatacaggtgggcggtgttcgacagcacctccagcttcaccaggtcccagccacccgcctcgcgcgccaggcgcagggtgcgcacagcgtcctctccggtgaagcagccggcggtgttgggcagataggtgaagcggtccggcttgacgtggtccaccagcatcggctggctcggatcggacaggttcacgcgcctgagcgccaccgtgacgacctcggcccccgccgcctcggccgccgccgcgttctgggcgtagtcggcgtacttgcccgtccccacgatcaaacgtgaggcaaaggtgcggcccgcgacggaccaggtgtcggatgcattctcggtcatggccgtccacctagtcctccgaagcggcgagcggaagtccgagccccgtcacgacgcgttgcgacatcgaccgcactgaactaaactaggtggacttagtccatgaggtccgcgtatgcagacggtcaacattcacgaagccaagacccacctgtcccgccttgtggacaaggccgccaagggggagtccttcatcatcgccaaggccggcaaacctatggtcaaggtgacgccgctggaagactcgccgaagaagccgctccagcgcatcggcttcatggccggcgagttcaccgttccggacgatttcgacaccatgttccaggccgagattgaggccatgttctacggcgacgtcgaggagacgaccaaggcggatcgatgaagcttctgatcgacactcacctgctgctatgggcggcgggcgacccttcgcgtgttccaagccgggcccgcgacctgatcaacgatctcggcaacatccccatgttcagcgtcgtcagcctgatggaggtctccatcaagacggcgcggtctcggccggacttccgtgtcgatgcgcgtcggcttcggtccatgctgctcgcctccggctacgaggagcttgcggtgacaggcgagcacgccgtggcggttggaccgcttgaacccatccacaaggacccgttcgatcgtctccttctggctcaagcgttcgcggaagaggccacccttttgacctcggacgccaccttggctcgctaccagggtccgatcctcaaggtctgacctcaccccccgccgacgaactgaaccagctcgatgcggtcgccctcggccaaagcggtcgtcgcgtgcagcgacttcggcacgatctccaggttccgctccaccgccactttgcgggggtcgagcgacagcgccttcaccaggtccaggatggtggaggccgccacctcacgctgatcgccgttgacttgaatgcgcatgacgttaggtcaacccgttcaaaggcggcgcgctttgatccgcgccgcgccttccgctaaaaggccgctccatcgaagcggttcgacccgcccggagcctatgcccgatcttcccgtcatctatgtgctgaacggccccaatctcaacctccttggcgagagagagccgcacatctatgggcgcgagaccctgacggacgtcgaggcgcgctgcgtcggcgcggccgggtctgaggcgaacatcgtcttccggcagacgaatcacgagggcgtgctggtcgactggatccaggaagcgcgcaccgaggctcaggcgctggtgatcaatccggccgcctatggacacacctccgtcgcgctgcacgacgcgctgaaggcgctgtccattccggtgatcgaactgcacctgtccaatccggcggcgcgagaggcgtttcgccaccactccctggtctcgcccttggcgaccggggtcatcgcgggcctaggcgcgcagggctatgcgctggcggtccaggccgcgctccacatcattcgggaacgcgcctgaggcgctcccgttggcacaacaagaccaaagaaaaggcgaaaccgacatggccgatgaaacgctgaacgccgggggcgagatcgatgcggagctggtgcgccagctggcggacatcctgaacgacacctccctgaccgagatcgaggtggagcgcggcgatctgaagatccgcgtcgcccgcaaggtcagcgccgccgctgcgcccgtgcagtacgccgccatgccggctccggtcgccgcgccggttgcagcccccgccgccgctgccgccatgcccagcgatccggcgaccatcgtcgcccgctccggcgaagaggtgaagtcgccgatggttggcaccgcctatctgcaaccggcgccggaagcgcccgcctttgtgcagcagggcgacaaggtcaagaagggccagaccctgctgatcgtcgaggccatgaagaccatgaacccgatccaggcgccgcgcgacggcgtggtggcggacgtgctggtcggcgacggccagccggtcgagttcggcgagccgctcgtcctgcttgaggcctgatcccgtgttcacaaaggtcctgatcgccaaccgcggcgagatcgcgctgcgcatccaccgcgcatgcaaggagatgggaatctccaccgtcgccgtgcactccgaggccgaccgcggcgccatgtgggtgcgcctggccgatgaaagcgtctgcatcggtccggcccaggccgccaagtcgtacctgaacatcccctcgatcatcgcggcggccgagatcaccggcgcgcaggcggtgcaccccggatacggcttcctgtccgagaacgcgcgcttcgccgagatcgttgaggcccacgggatgagcttcatcgggcccaagcccgagcacatccgcatcatgggcgacaagatcaccgcaaagcagacagccaaggacgcgggaatccccgtcgttcccggctcggacggcgaggtcgagaccgtcgaggccgccatcgaagccgccaagtccatcggcttcccgctgatcgtcaaggcggcggcgggcggcggcgggcgcggcatgaaggtcgcgatgaccgccgacgatctggtcgaggccgtccagaccgcccagtccgaggccaaggccgccttcggcaacggcgccgtctatatggagcgctatctgcagaagccgcgccacatcgaaatccaggtgatcgccgacagccacggcaacgtcgtgcacctgggcgagcgcgactgctcgctgcagcgccgccaccagaaggtgctggaggaggctccctcccccgcgctggacgccgccgggcgcgagcggatcggcaagatcgtggtcgatgcgatcaaggccatcggctatctcggcgtcggcaccatcgagttcctgtgggaagacggcgagttcttctttatcgagatgaacacccgccttcaggtcgagcatccggtgaccgaggccatcaccggcgtcgatctggtgcgcgagcaggtgcggatcgcagcgggtctgccgctgtccttcacccaggacgacatccacttcgaaggccactccatcgaagtgcgcgtcaacgccgagaaccccgagaccttcacgccgtcgccaggcatggtgaacgacttccacgcccccggcggcctgggcgtccgtttggacagcgccatctacgccggctattcgatcccgccctattacgacagcctgatcggcaagctgatcgttcacggccgcgatcgcgaagaggcggtggcgcggctcaagcgggctcttggcgaaatggtcgtgggcggcatcgacaccaccattccgctgttccagcgcctgctggtcgagccggacatcctgtccggcgactacgacatccactggctggagaagtgggccaaggctcagaagggcgcgggcgcctagcgccgttggccgagccggatttcagcgccagcagcccctcctccggcttcgggcccgaggcgctgctggcctgctacgcgcgcggcgtctttcccatggcggaggcgcgcgacgatcctcgcgtcttcatcgtcgagcccgatcagcgaggcgtgattccgctcgacgccttccacatcccgtcgcgcctgcgccgcaccgtgcgcgcagagccgttcgacatccgtgtggacaccgccttcgaggcggtgctggacggctgcgcggcgtcacaggggcccggccgacaggacacctggatcaacggcccgatccgccgcctctatggcgagttgtttgcgcgcggctttgttcattcgctcgagtgctggcgcgaggagcggctggtcggcggcctgtacggcgtgtcgcttggcggcgcttttttcggagaaagcatgttcagccgcgagcgcgacgcctccaaggttgcgctggtgcatctcgtcgcgcggctgaaagccggcggctggaccctgctggacgcgcagttcctgaccgatcacctcagccagttcggcgcggtcgagaccccgcagtcggcctacctccgccgcctgaagccggccctgcatgtgcagccggaccagagtgcgctgacaagacctatgagcggttcagaggctattgagcgggcgatcggataggagccgagttggacggatcaccacgccgccctccgcgcctcaatccttgcagccgaccacccaggcgtcatagttcgggtgctgcaggccgctgacagccggcgacgaggcgaacatccaccctttgaacacctggcgtgtcggcagaggctgggtcgtgccgcgcggctggaccgagacgtcgacataagcgatcgcgtcctccgtcaactcatccggtgtggagacctcgcaggcgctgacgttgaagatcaggttgcgggcgaagcgaacgggtcggcctccgacctgcacctcgaagcgcatcgtttcagccgtgaccttgtcgatggcctggatcaccgcgaccttgcggcgctggcgccggaccggcgcctccggctgttcgatgggcttttcggcggcggcggccttgacgggagttggagcgtccggctccgcctcttcctcgacgatcaccaccggcggcgggacggtgatcggcacgggcgcggccggggcgggctgccccgccggcgcgctctcgaccggcgtagggggcggcgtggcgcgcaggatgtcgccgatgggatcctgggcggggcgggcgtcgcggggcgcgtcctgcaacgcactggcggtcacgccgccggcggtcagcagcgccgccgccgccaggccaatcgccagtcgtccgcccaagcgcgtcattgctcttattccggggtccaggcctggtagtcgccggtggcggccggacgcttgccgtcgttcgcgagggagccgggcgggcgccaggccagcggcgtcccggtcaggttcggcagatggtccttttcccagttgcggcgcggcagcggctgaaccgtcggcggctctgcgaaggtgtagtgcagccagccgtaccagtcgggcgacaccttggacgcctcggcgtagccgttgtaggtcacccaacgcctgcgacgaccatcatagctgacggtgtcgcggctctcgtaatagcgattgccgttttcgtccgtgccgaccagacggccgcgtttggcgatggtgaacagggtgccgatcgtggcgccgttccaccagccgaagatcttgttcaacacgtcaaccaacccacgccaaatcggccgaaccggagggtccggcggctgcgcgatcatagaaacgccggcgcgcttcgtccagcatggagcaggcggtgcaggcttcttaacggagaggcggatacgttggcgcgcggcttgcatgcagcgcgcctcgaaccggagcccacaccgtcatgaaacgcgtccttgtcgccctcgcccttctggccctcgccacgcctgcgctcgcccagaacgcgagtcagatcgccagcgtacggcgcggtgcgaactgcggagggtgcaacctgttccagggcgacttctcggggatggagcgtcgcgggctcaatctatcgggcgcacgcctgcgccaggcggacctcagcctgtcggtcatgaaccgcacccgcttctccaacgccgacctgcgcgacgtggaggcgtatggcggcgtcttctccagctcgaacttctcgcgcgccgacatgaccaacgccagcttcgtcggggcctacctggagggcgcgaacttcgccggcgcccggttgtcggggaccaacctgtccggcgcgaggctgtcgcgcgccacgggcctgacccaagctcagctgaatcgcgcctgcggcgacggttcgacggttctgccgcgcgggctgcgcatccccgcctgctgagcgtctccttcgttacgacgatttaagtaggccgatcaggcgcttcggcgcatgaagcgagtgtggaacagatcagcagctcccttctccgtcgcctcttcgtcgccgtttccgcggccggcctgacgctcgcggccgcacccgccttcgccggcgtcgaactgctgcttcaggatcgcgacgtggcgcggtcggtgtcgctgggcggttcgtgcaatcgttgcgaactgtcggggcgcaatctgaccggcgccaccttcaccggcgcgacctttatcagcgccaccttggtgggttcggacctgcggggcgcggaactggtcggatcgaacttcaccggcagcgacttcacccgggcgaacctacgcggcgtggagatcctgggcgccaacttcgcggaagccgacttcagcaacgcctcgctcgcgggcgccgaggcgcagggttcgtcctttgtgcggtccaacctgtctcgcgccgacctctcgggcgccgagttgcacggcgtgaacttcaacggagccacgctggccggcgccaacctcagcgacagcgagttgttcggcgcgaccctggccaatgtgaaggccgccggcgccaacttcgccaacgcccaggtcaacgcctccaacctcgcgtccggcgatttcaccggcgcctcgttccgcaacgcgcagctgacggccgcgcggctgagcggcggccgcttcgaccgcgccgacttctccgatgcggagatgcgccgcacggacatccggggcgtggacctgtcgggcgctcgtggcctgacgcaggcgcaggtctccctagcgtgcggcgacagctccacccgtctgccgggccggctgacggcccagagctgcagaggcgcagcccgggtcatccgcacgccgcccacgccgccgatcccgccgcgtcagcgcaacctggtgctggtcgccgaataagcggcttcccgccgccgggcggcgggaagatccgtcgtgtcagaccttgatgggcggcgcggtgcggatgtgcagttccttcatctgcttgtcctgcaccggagaaggcgcgctcatcagcagatcctcgccctgctggttcagcgggaaggcgatcacctcgcggatggcctgctggccggccagcagcatgacgatgcggtcgatgccgggcgccagaccgccgtgcggcggcgcgccatagcggaaggcgttcagcatgccgccgaactggtcctcgacaaccgaggcgtcatagccggcgatctcaaaggccttgagcatgatctcggccttgtggttccggatcgcgcccgagcacagctcatagccgttgcagacgatgtcgtactgataggccaggatatccagcggatccttggtgttcagcgcctccagctcgccttgcggcatggagaagggattgtggctgaagtcgaccttcttctcctcgtccgaccactcgaacatcgggaagtcgacgatccagcagaagcggaactgatcctcgtccaggagcttcagctcggtcccgacgcgggtccgggcgctgcctgcgaacttgtagaagctgttcggatcgccggcgacaaagaaggcggcgtcgccctgcccaaggcccagcgccttcatcagcgcgtcggccggctcgcccaggttcttggcgatcggcccgccccaggcgccctgatcgtccgaccagaagatatagccgaggcccggctggccttcgccttgcgcccacgaattcatccgatcgcagaaggcgcgcgatcccccggtcggcgccgggacggcccagacgcggttcttcggatcggcggccagaatcttgttgaacaggccgaatccgccatcgcggaaatgctccgacacatcctgcatctcgatcgggttgcgcaggtccggcttgtccgagccgtatttggcgatcgattcgcggtagggaatgcgctggaacggataggcgtcgacgcgcttgccttcgccgaactcctcgaacacgccgtgcatcaccggctcgatagcggcgaagacgtcttcctgggtgacgaagctcatctcgacgtcgagctggtagaactccagcgaacggtccgcgcgcaggtcctcgtcgcggaagcacggcgcgatctgaaaataacggtcgaagcccgacaccatcagcagctgcttgaactgctggggcgcctgcggcagcgcatagaacttctcgggatgcaggcggctgggcaccaggaagtcgcgcgcgccttcgggcgacgaggccgtcaggatcggcgtctggtactccaggaaaccctgctgaaacatgcgattgcggatcgactggatcacgcgcgaacgcagcacgatgttcttgtgcagggtctcgcgacgcaggtcgagatagcggtgcttgagccggatttcctcgggatactccggctcgccgaagactggcagcggcagttcggcggcttccgacagcacctcgaccgcctgaacccgcacctcgacttctccggtgggcaggttggcgttgacggtcgagccttcgcgcagcaccacctcgccgtcgacacggatcacgctctcggcgcgcacccgctccacccgctcgaagcccggcgtctccgggtgcagcaccagctgggtcaggccgtagtggtcgcgcaggtcgatgaacagcagaccgccgtggtcccgcttcctgtgcacccagccggacaggcggaccgaggagccggcgtcggaagcgcgaagcgcgccgcaggtgtgagagcgataggcgtgcatgaggatcgtcttgtcgggccgcaggggcggcgaaatggaacggcgtagggcgcatcatcgccccggaaagtcaaggttgagggccttgcggccccgtcccgacaggcccggcggattggcgctggacctacgtcctgatgccctgtcagaaacgccttggccttatcatttcacgctcgtgcacctcgggaagccatccatgttcgtcgtcatcctgcgctatttgaaacccatggacgaggtggaggcgcggaccgccgaacaccgggcgtggctggacccgcatgtgcggagcggcctgctgatcgccacgggtccgatggttccgcgaaccggaggcgtgctgctggcgcgcggcggagggacgcgggaggcgctggtcgccctgctccgcgacgatccgttccaggttcacggcgttgccgagtacgaggtcatcgagttcgcgcccggcaaatatcatcccgccatggctgagtttctctgaggttcatccacagtcggcggcgatgctccccattaccaacaggaacctgtgggtcggtcgcggactcggcgcgtgctaagagaaaggcatgcccgccgacggcgccctgaacattccggccggagagcagctgcggctgccgctcgagcgccatggcgcgtccgaggcctttgtggtgtcggccagcaacgaaaacgccatacgcctgctggagcgctggccggacggggccggttcggttctggcgctccacgggccggcgggttcgggcaagagccgcctggcggagatctgggccgagcggctcggcgcggtcgccctgcacggcgccgaggcggggctggttgatctgcgcgagatcgagggtcggccgctgctgcttgaccgcgcccaggacgccgacgacgagagcctgtttcacctgatcaacctggccgtatcgacgggctctccgctgctgctggcctcacgcagcgcgccgcgaggatggtcgaccaccctgcccgacctgcgctcgcgcctggacgccctgcgcacggtggcgctggaggcgccggacgatgcggtgctggcggccattctgcgcgcgcgcttcgccgaacgcagcatcgcgccggcgcccgaggtgatcgactatctggtgcgtcggctggatcgctcggcggaggcggccgaaacggccgtcgagcggctcgacgcgcggcatcgcccggtgacccgcgtcctcgcccgcgaagtcttggacgagttgcaggccgagggcggctgaaggcggcaaatcgcctcgctgcgcttgcgggcgtcacacgagcgcgcgacatacgatccatgaccgacgccgccatccacgacgccacccgaggtcaggaggtgcccgcctcgcgcgcgccgcagctggcgctgagcgaagacctgatggcctcgccagagcggttcttcaatcgcgagacctcgtggctggccttcaacgagcgcgtgctggaggaggccgccaatccccagcacccgctgctggagcggctgcgcttcctgtccatctcggccaacaatctggacgagttcttcatgacgcgcgtggcgggcctgaagggtcaattgcgcgagcgggttcgcgtgctgtcggccgacggcctgtcgccggccgagcagctggagcggatcaacatcgccgccgggcagctgatggccgaacagcaggtgcgctggcgtcagctgcggcgcgaactggcggactgcggcatcgaggtggtcagtggcggacggctgaccaagacggagcgggatcggctggagcccgagttcctgaaccagctgttcgccatcctgacgccgctggccatcgaccccgcgcacccttttccctttctgcccaatctcggcttctcgctggcgctgaagctgcggcgcaagggcgagagccgcaccttctacgccctggttccggtgccgacccaggtgcgacggttctgggctctgccggtggacggccgatcggcgaagggccgccagcgctttgtgtcgctggaggacgtgctggtcctgttcatcgaccacctgtttcccggctgcgaggtgctggaaaggggcgtgctgcgcctgatccgcgactccgacatcgagatcgaggaggaggccgaagacctggtgctggagttcgaggaggcgctgaagcagcgtcggctcggctcggtcgtgcgggtcaagatcgaagcctccatgccgccggacctgcgcgacttcatcgttgaagagctgcaggccgcgccgcaggacgtggtgctggtcgacggcatgctggggctggcgcaactgagcgaactcattccgccagaccggccggagctgaagttcaggggccacgagccccgttaccctgagcgcgtgcgcgacaacggcggcgacattttcgcctcggtgcgtgaaaaggacatgctgatccaccacccgttcgagagcttcgacgtggtggtccagttcctgcgccaggcggcgcgcgaccccaacgtcctggcgatcaagcagacgctgtatcgcacttccaaggacagccccatcgtcgccgccctgatcgaggcggccgagaacggcaagaacgtcaccgccttggtggagctgaaggcgcgcttcgacgaggaggccaatctgcgctgggcccgcgcaatggagcgcgcgggcgtccacgtcgtcttcggcttcgtcgaatacaagacccacgccaagctgagcgtggtggtgcgccgcgagggcgagggcctgaagacctactgccacttcggcacgggcaactaccacccggtgaccgccaaggtttacaccgacctgtcgctgttcagctcggaccccgtgctgggccgcgacgccagccgcgtgttcaactacatcaccgggtacgccacgccggacgagctggaggcgctggtcgtctcgcctctgaacatgaagtccacgctgatcgagctgatcggcaaggagatgtcggcggcggccatgggcaagccggccgccatctgggtcaagctgaactcgctggtcgatcccgaaatcatcgacgcgctttatcgcgccagccaatggggagtgcgcatcgacctggtggtgcgcggcatctgctgcctgcgtcccggggtgcccggcctgtcggagaacatccgggtcaagtccatcgtcgggcgcttcctggagcacagccgcatcgtcgccttcgccaacggccaggacctgcccagcgacaaggccaaggtgttcatctcctcggccgactggatgccgcgcaatctggaccgccgcgtcgagctgatgacgcccatccggaacgcaaccgtgcatgatcaggttctggatcagatcatggtggccaacctcaaggacgatgcgcaaagctgggtgctggacgccgccggacgctacacccgcgtccagccggtcgatcccgaccggcccttctcggcgcacaagtatttcatgaccaatcccagcctgtccggtcgcggccgcaaggtgaagacacggcccgaagagctgcgtctcgagccgcccgtccgctgatgcccgagatgaccacgccgcgtgacatcgcggccatcgatatcggctcgaactcggtccgcctggtgctctaccggctggaaggccgtgcaatctggaccgtgttcaacgaaaaggttctggctggcctaggccgggacctgcccgtgaccgggcggctttcggcggagggactgccgatggcgatgacggcccttcgtcggtttgcggccgtgctggagggcgtgcgccccgagaagaccctgatcgccgccaccgccgccgtgcgggaggccacggacggccctgagttctgccaaagggtcgctgccgaaaccgggctgaacatccgcgtcctgtcgggcgaggaggaggctcggtacgccgcgctgggcgtgctggccggcgcgccgcgcgcgcggggcgtttccgccgacatgggcggcgccagtctggagctgacgcgcctgagcggcgacagcatcgagcgcggcgtgaccctgccgctgggtccctttgctctggcggacggcaaaccgttcgacgccgcgcgcatccgcgcccgcatcaacgaacggctgtccgcggtggccggggatttccgctcggaacgcctttacgccgtcggcggcgcctggcggaccctggcccaggtgcagatgcggatgaaaaactatccgctgcacgtcgtgcaccagtacgagatgacggccgacgacgcgctggaggccgcgcagatggtggctcagcagcccaggcaggcgctggagcgacagccgggcgtgtccaggaagcgggccgagaccctgccctatgcggccctggtgctggaaggtctgatccggcacctgggccttcgcacggtcgaggtctcggcctggggcgtgcgcgaggggctgctgttcgagcagctggatgcgccggaaaaagcggccgatcccctgctggccggttgcgccgcgctgggcggacggcaaggcatctcgcctgctctgccgggagcgctgaatggatggatcgccgacatcgtggcggcgctgccggcggcgttcggcgccgagcgcgaccgggtgctgacggacgccgcctgtcgcctggcggaccttggtgcgcgcctgcatccggaccaccgactggaattggtgttcgaccaggtgctgcgcgcgcccgtgccggggcagagccatgccgagcgcgcctttctggcggttgcggtcaacgcccgctatggcggcccggccaccacgcccgagccgcagaccatcgcgcgcctgctggacgaacggtccgcacggcgcgcccgcgccctggggctggcgatccggctggcatgcgacctgtcgggccgatcgccgcagctgctggcgaacgccagcgcgggtgtgggcgatggagcgctacggctccaggcgcgtcccggctacgccgacgtgctgctgggcgaacagactcgcaagcgggccagggccctggccgaggccatgggcgtggaactcagcatctaaggcgctccccgcctcccgtcgcggtgaacagagttcccgccgtcagccctcgatctcgaccacctcgacgcgtgcgccgttcaggaccagagcgatttcgccgcgcttcagcttcagggcgtcctcgccgaacagttgacggcgccagcccttcatcgcctcgacgtcggccgcgtcgctgagcgcgatcttctccaggtccgagacggtggcgatcagtttggaggcgacgccggcgttgtcgctcttggccttcagcagcaccttcagaagctccaccaccgagggcggcgccggctggttgtgggcggggcggtccatcttcggcgcatgcgcctccggatcggccaggacgcgcttcagctcctcggtcagctccagccccagacgcgagccgccgaagcccttgggaaccgaacgcaggcggttgaaggcgtcgggatcggtcggcgcctgctgggcgatctcgtcgacgccttcgtccttcaggatgcggccgcgaggctggtcgcgctcctgcgccgcccgctcgcgccacacggcgacggccttgaaggcggcgagatacttggccgagaacttcttgggccgcagccgcttccaggcgttttcgggatcggtgtcgtagagcgctgggtccgtcagaccctccatctcggacatcacccagtccagccggccttccttgtgcaggcgatcgcgcagcttcgggtacagcgccgccaagtgcgtcacgtcgcccagcgcataggtcagctgattgtccgacagcggccggcgggcccagtcggtgaagcgactgcccttgtccaagtcgatcttcagcgtctggcgcaccagcgaatcataggccacctgctcgccgaagcccgccgccatggccgcgacctgggtgtcgaacagcggccgcggcatggcgcccagccgcacgaagatctccacgtcctggcgacaggcgtggaagaccttgacgatgttcgggtcgcgcaggatctcgaggaacggctccaggtccagcccgtctgccatcggatcgatgatgccggcgtattcggtcgaagccgcctggatcaggcacagcttgggccagtaggtcgtctcgcgcatgaactcggtgtcgaccgcgatgaaaggcgcgtcggacaggcgggcgcagaactcggccagcgcctcattggtggtgatcggcgtcattccggtgctatagcgcggcgcgaccgcgttgtggcaagacgccgcgacacatttccgccttccgattcaggccgtgacccatgagcgacaccgaccgtccccttgccaacggcctgacctacgccgacgccggcgtggatatcgacgcgggcgaactgctggtcgagcacatcaagccgctggccaaatccacggcgcggccgggatccgagccctcgctcggaggcttcggcgccctgttcgacctcaaggcggcgggcttcgatgatccgctgatcgtgtccaccacggatggcgtgggcaccaagctgaagatcgccatcgagaccggtcgccatgacggcgttgggatcgacctcgtcgccatgtgcgtcaacgatctgttggcccagggcgcggagccgctgctgttcctggactactacgccaccggcaagctggagatcgatgcggcgcgccgggtggtctcgggcatcgccgagggatgccgccaggcgggctgcgcgcttgtcggaggcgagacggccgaaatgcccggcatgtacggcggcggcgattatgatctggcgggcttcagcctgggcgccgtcgagcggggtcaggccctgccctatctggaccgtcagcaggctggcgacatcatcatcggcgtcggatcgtcaggcccgcactccaacggctattcgctgatccgcaaggtggtggagaagtccgggctgacgtggggcgacgacgcgcccttcgccgccgatcgatcgctggcccaagcgttgatggagccgacgcgcatctatgtgaagtcggtgctgccgctgatgaagtccggccggatcaagggcgcggcgcacatcaccggcggcggcctgatcgagaacccgccgcgctgcatcgccgacggcctggaggccacgtttgattgggacgcctggccgctgccccccgtgttccggtggctggcggagacgggcggcatttcggatcacgagatgcgccggaccttcaactgcggcgtgggcttcatcctgatcgcgtcgcccgaagatgcggagggcgtgctggaggcgctgctgacctccggcgaagtcgcctttgtctgcggacagttgcaagccgtcgcatgagaaagcgccgcgtcgccgtcctgatctcgggcgcgggctccaacatggcggccctgatcgacgcagggctggcgcccgacaccgccttcgaggtcgttctggcggtgtccaacatcgcgaacgccggcgggctggcggtggctgaagccaagggcgtcgccgtccagaccatcccccatgcggcgttcggccgggaccgcgcggcgcacgagcgggccatcgacgaggcgctgaaggcgcacggcgtcgagatggtggccctcgccggctacatgcgggtgctgacgccatggctggtaggcggctggcgcgggcgcatgatcaacatccaccccagcctgctgccgctctatcccggcctggacacccacgcacgtgctctggccgccggcgacgcggaggcgggctgcaccgttcacggcgtgaccgagggcgtggacgaaggtccgatcctgggccaggtgcgggtgcccgtccttcacgacgatacgcccgcatcactggccgagcgggtcaagacggccgagcacaggctgtatccgcgcgtgctgcacgccgtctgcaacaccctcgactgacacatacgaaaacggccccggagaaatctccggggccgcttcgtttcagccttgcggccgggagctgggttagcgcggggtcgtcgccgcgccggccacgccgccgatggccgcgccggccacggtcgaaccggtgttgccgcccagcacctggccggccacagcaccgcccagcgcgccgctggcggcgcgttgttccatcgtctggccgcaggcggccagcagggccacgacgccgacgacgggagcgatcttgatcagggtcttcatggttcagtctccttggggaggatgcgttcgatgaagcccaaacaaaacggcccgcccccggttccgaggacgggccatattgtcacggttggtgaaccggtcagccgacgatctggtcgtcggtgaagaactgctcgatctcgatcttggcgttgtccaggctgtcggagccgtggaccgagttctcgccgatcgacagggcgaactgcttgcggatggtgccgtcggcggcctgttccgggttggtcgcccccatcacttcacgatacttggcgacggcgttgtcgccttccagcacctgcaccacgaccggctcggccgtcatctgcgacaccagttcgccgtagaaggggcgctcggcgtgcacttcatagaacttcttggcctgggcgtcggtcagcttgacgcggcgctgggcgacgatgcgcaggccggcgtcctcgatcacggcgttgatcttaccggtcaggttgcgacgcgtcgcgtccggcttgatgatcgaaaatgtgcgttcggtcatgggggtgacttcttgttgggagattgagggtcgcgggcttatagcgacgccctctccgctttccaatcccgccgcaaggccgcgctcgacccatgctccagatttccaacctgacctacaacgcctggggccgccagtttctggacgacgcctccgtcagcctgccgccggggtccaaggtcgggctggtggggcgcaacggcatcggcaagtcgacgctgttcaagctgatcctgggcgaactggccgcgaacggggacgaggtgtcgctgcccaagaccgcgcgcatcggctcggtcgatcaggagcatccggccactcccgtcagcgtgctggacaccatcctggaagccgacgtcgagcgtcattcgctgatgacccggctggacaccgccgagccggaggagatgggcgagatctggatgcggctgatcgagatcgacgccgaatcggctccgtcccgcgcctccgaaatcctggtggggctgggcttcagccaggaggacatccagcggccgatgtcgcacttctccggcggctggcggatgcgggtggcgctggccgccgccctgttcgccgagccggacatgctgctgctggacgaacccaccaactacctcgacttggaaggcgcgctgtggctcgaggcgcggttgaagaagtatccgcatacggccctgatcatctcgcacgaccgcgagatgctgaacgaggtctgcacccacatcctgcacctgtcgaaccgcaagctggagctctacaccggcaactatgacgcgttcgaacagcggcgcgccgagaagctgcggctgctgcaggcgtcgcgcgccaagcaggaggccgaacgggcgcacctgcagtcgttcgtcgaccgcttcaaggcaaaggcgtccaaggccgcgcaggcgcagtcgcgcgtcaagcggctggccaagctgcagcccgtcgagctgccgcccgaggagcgcgtcgcccccttcgtcctgccttcgccgccgcgccccctgccgccgccgttgatccggctggagcgcgcctcggtcggctatgagcccggcaagccgatcctgcgcggcctgaacctgcgcatggacctggatgaccgcatcggcctgttgggcgtcaacggcgccggcaagtccaccttcgccaagatgatcgccaaggccctgcccatcgaggcgggcgagttccaccgcgacgggaagatgcgcgtcggctggttccaccagcatcagatcgaagcgatggatccgacggatacgccgctggagatcatccgccgcgccatgccggaagcttcggaaagcagccgtcgctcccgcctggcccagttcggcctgccattcgagaagcaggagaccaaggtcgaggccctctccgggggcgagcgggcgcgcctgctgctgaacctagtagcgatggacgcaccgcacatcctgatcctcgacgaaccgaccaaccacctggacatcgacagccgccgcgccctgctggatgcgctgaacgagtacagcggcgccgtcgtcctgatcacccacgaccgctcgctgatggagctggtcgccgaccggctgtggctggcggcggacggcactgtgaagccgttcgacggcgacatggacgactacgccaggttcgtgctcgaccgcgccaaacaggccggcatgaagccgagccaggtcaaggccgatcccctgccggaggcggcgcccgcgccgacgcccgtcgccaaggtcgaaaagaagaagggcggcccttccccgtccaccctgcgtcatgcggtcaggaaagcggaggagcgcatgaccgcgctggccgccgatctcgcccgtatcgacgccgacctcgccgaggcggccgcacgcgatcccaaaaagctcgaaggcctgactcgcgcccgcgccaaggcgcaggccgagctggacgccgcagaggccgactgggtcgccgcagaggaagccttggcggaagtagcgtagccgatcattgccgaagcttaatgcggcgcgtgcctgatcggccttgtcgaacgccgatccgacagccaagctcgcctcatgaacagcgacgctccggtcatcgaaactcacggcctgaccaagacctatggctcggtgcgggcgctggacggcctgacgctcagcattcccagaggcggcgtctatggcgtgctggggccgaacggcgcgggcaagtcgaccctgtttcgcacgcttctgggcctgatccggccgacggaaggcggcgccaccatcatgggcagcccgatcggagacgtggccgccatgcggcgcatggggtcgatgatcgagacgccgcgctttccgccctatctgacggcgagacaggtgctgcactggctggggcgcgcacacggcggcgtgtccgaagccgacatccggcactggctggagcgggtcggcctgaccgaggcggccgatcgcaaggtgcgcggtttctccgtcggcatgctgcaacggctgggcgtcgccgccgctttgatgaccaagccggacctcgtcatcctggatgaaccgaccagcggcatggatccgcccggcatccaagagatgcgcgcgctgatccgatcgctcgcggacgacgatggcgtgaccatcatcctcgccagccatcagctgcaagaggtgcaacgggtctgcgaccgcgtcgccatcttcaacaggggcaaggtggtggccgaaggtcgggtgtcggacctgaccgcctcgggcgagcggctgcgcttgtcggccacgccgctggcgcgcgttctggcggttctgggcgaacgcgggagcttggacggcgacgccgtgctggccgccgttcctcgcgccgaggcccccaccctgatccgcgccctggtggaagccggcgtcgagatcgacgaggcgcgatgggtcggtgcggacctggaaagcgtgttcatgaccgaaaccggctggaccggcctgaaggagcccacccatgctggctgacgccgcgcgcgccgaggcctatcggctgtccaagaatcgcgtccagatcgggttggccgtccttgtgacgccgctgctgttcgccgccgggagcttgttcgtgctctggcgcgcccgggtggagggcggcgcggcggcgcttcggatcggcgtgtcaggcgacgcctccgcccccgtgaacctggcgaacgccttcggctttgcagccgacaagggcgccaacggcctgatgctcgtcctgatgctggttgcggccgccaccctgtacgccggcgactatcggtgggagacgtggcgcctgatcactgcgcgcaacggccggccttcgctgctgctgggcaaggtttcggtcatgacgggcctggcgctggccggcatggtcacctttcttgtcgccagcgggatcttcttcctgggccaggccatgatcttcagccgccccttgtctttcgaccttggcgcgggcgaggcgggcgacttcgtgctgctgtggctcgtgtcctggctgcggatcgtgcagttcgcgatgatcggcctgctgacggccgtggtcagtcgatcgctgctggcggcgttgttcgtgccttgggcgctgggctttgttcaaaccatcctgggacagttcggcccggctctgcttggctgggagccgcagggctggaccatgcacctgatgctgccggggtatgcctatgatgcggtcaaggcggtgatcgatccgccggccggtccgactccggggcccgcgcccgcgctgtggccggcgatgaccagcctgatgctgtggaccgtgcttccgctgctgggcgcgctggcctggttcaaacggcaggatctgtcaaaggagtagcggcgggctcaagccgcttctccatgaagacgtcggcgcgcgcatagggcgtcggccgcgcgggcagatgcgtgaagccctcgctctcgtaaagggcgatggccggcttcagggcgctgttggtctccaggtagagccgctcggccccgctgtcgcgcgcagccgcttcgcaggcgcgcagcagacgccgggccaggccccgcccgcgcatcgccggcgtcaccgtcattttggacacctcgaagccgtcctcgatgcggatcagggcgcagcacccgaccggctctccggccgcctccgcgatgaagatgcgtccacctccttccagaaacgcggcctgagggtcgccgatcgccttgtcgtccttggcttcgatcacaaacccgccctcggtcagccaggccttgttcagggccgcccagcccaccgcgtgacgcggttcgtagtcgatgatggtcaagggatcggcgctgctcatcaccgcctcatgccgcaatcgtgggcaaagaaaaagggcggccggatcgcgccggccgcccctcattctgatcgctgaggcgaggctcaggcctcgtcgtcgccctcgtaagccatcaccggaccggagtcctggcccttggcgtcgacgtcgcgatcaacgaactcgatcaccgccatcggggcgttgtcgccgtggcgatagcccgccttcataatgcggatgtagccgccgttgcgctcggcgtagcggctgcccagcgtgtcgaacagcttgccgacctgcgtcacgtcacggacctggctgatggcctgacgacgcgcgtgcagatcacccttcttggccagggtgacgagcttctcgacgaagggacgcagttccttggccttgggcagggtcgtcttgatctgctcgtgcttgatcagcgaggcggccatgttggcgaacatggcggtgcggtggctgctggtgcggccgagcttgcggtgggcggcgccgtggcgcatcggggtctctcctactccggctccggtatcccgcctcttggggaacgcgggacctagaaccgtaatcttctaaccgccccggctttctccttggaggagacgggcggagggttgaacttagatctggtcgtcgaacttcttggccagatcttcgatgttttcgggcggccagttcggcacgtccatgccgagcgacagacccatggaggtcagaacctccttgatctcgttcagcgacttgcggccgaagttcggggtgcgaagcatctcgccctcagtcttctggatcaggtcgccgatgtagacgatgttgtcgttcttcaggcagttggccgaacggaccgacagctccagctcgtccaccttcttcagcagggccgggttgaacggcaggtccggcttgccctcggaggcctccaccgccttcttcggctcgtcaaaggtgatgaatatctgcagctggtcctgcagaatgcgcgaggcgtaggccacggcgtccaccggcgaaaccgcgccgttggtctcaacttccagcagcagcttgtcataatccagcgactgaccctggcgcgtcggctcgacgcgataggcgacgcgcttgaccggcgaatacagggcgtcgaccgcgatcaggccgatgggcgcatcttccggacggttgaactcggccgccacatagcccttgccgttctgcacggtcagttccatgcggatggaggcgccgtcgtccagggtgcagatcacgtggtcggtgttcagcacctcgatgtcggccggggcgtcgatctgaccggccgtcaccgggccggggccggtcgcgcgcagcgtcatgcgcttgggcccttccgcatgcatgcggagcgccagctgcttgatgttcagaacgatgtcgaccacgtcctcgcgtacgccttccagcgacgagaactcatggaccacgccgtcgatctggatggcggtgaccgccgcgccttgcagcgacgacaacagaacgcggcgaagcgcgttgccgagcgtcacgccgaaaccacgttccaggggctcggcgaccaggcgcgccttgcgctgggcgtcggagccgacctcgatctgcggcttctcgggacggatcagctcttgccagtttctttcgatcattttgtccctcgaacgggtttcgccgatctcctgccctgtcgacggggcgcgtggagaccgacgggaatagggggcgacggctggagcggcgtctgcgcttagacgcggcggcgcttcggcggacggcagccgttgtgcggcatcggcgtcacgtcgcggatcgtggtgatcgtcaggccgaccgactgcagggcgcgcagggccgactcacggcccgaacccggacccgagacgttcacttccagcgtcttgacgccgtgctcctgagccttcttgccggcgtcctcggccgccatctgggcggcgtacggcgtcgacttgcgcgagcccttgaagcccatgtgaccggccgacgaccaggaaatcgcatttccctgcgcgtcggtgatggtcaccatggtgttgttgaagctggcgttcacgtgagccacgcccgacgtgatgttcttgcgttcgcggcgcttaacgcgacccggttccttggccatcggtcagctctttctcttacttcttcttgccggcgatcggcttggccggccccttgcgggtgcgggcgttcgtgtgcgtgcgctgaccgcggaccggcaggcccttgcggtgacgcaggccgcggtagcaggccaggtccatcaggcgcttgatgttcatcgatgtttcgcggcgcaggtcgccctcgacggtgtggtcgcggtcgatcgtctcgcggatctgcaggacttcggcgtccgacagctgattgacccggcgggcggactcgatgccgaccttttcggtgatctccttggcggcggcggggccgatgccgtggatgtactgcagcgcgatttcgacgcgcttgttggtcgggatattgacgcctgcgatacgggccacgaaactctccagatgcgcgttagtcagacgcaacaaacgctccggtcaacagaccaggagcgtgggcgcccttcgcggaaggccgtccttatagcggcgattcatcgaacgtcaatggcctgtcgccgcagagccaaatcatcggaagcttacggtcagagtgagcccctcgtcgggcagagcgcgccctccccgcctgggcggatcaaagcggtagaagcccgccgcctgcagcgcggccacgccaaagccgcgaccttccggcgtttcgctgacgatacggcagcgctccagacgctggtccaagccgatccggcagtgaatgacgccttcgccgcccacgcggccgccgaacagaccgcctcgcgcctgtgacggatgcagccgggccagctcggcgttcgaggggccacgcaggaagcgcggtccgctgaagccctctcccggtccgtcgccagggccgactccttcgcccgaacctgacccctcgccgccctgccccagtccgggctgcgccgaggccgcatccgaggcgccgatcaccagcgcgggctcaggcgccggggtgcgcggagcggggatttcaggcgggacgggcgtgggcggcggcgtgtgcacgcgcgagggagcggcgggcgctcctccgccgctgacgggcgtcgggttcggtggaggcggtggtgtgatcggcggtgagggtgggatcagcgccacctcgatcgcaggcgcctcgatttgcggcgccggcgtctcccccacctggcccagcagggtgaacaggccggcgtgcgccagaaccacgccgccggcggccaggaccgagcgcagacggccacggcggggggcgggcgtggcggatggggaatggaggacgacggccgacatctcgggcgatcaacgcccgaaatgggtcaagggtcaggcgcccgcgctttggacgttcagagccgcgtcgatagcggacgccacggcgtcgatggagcccatgccgtccacctcggtcagcttgccctgcgcttcatagtagggaagcaacggcgcggtgttgcggttgtaggcgtccagccggaccttgaaggtctccggattgtcgtcggcgcgaccctggtcggcgtagcgcttggtgatccgctccagcagggcggcgtcatcgaccttgaggcgcacgacgccgtcgatcctggcgccgcgcttttccagcatggcgtccagcgcctcggcctgggcgacggtgcgaggaaagccgtcgaagatggcgccgcctgcggcctcggcctccggcagacgatcctcgatcagggcgatcacgatctcgtccgacaccaggtcgccacgcgccatgatggcctggcactccaggcccagaggcgactcagaagcaatggccgcgcgcaacatgtcgccggtggacagctggaccatgccacgctcctccaccagccgcttggcctgggtgcccttgcccgccgccggcggtccgaacaggatcagattcaaggctcgccctcccccaggctggttcagtctcggatcagcgccgcacgaccgccgggccgcgcccgcgtccccgcagcttggccttcttgatcagaccctcgtactggtgcgccagcagctgggactggatctgcgccaccgtgtccatggtgaccgagaccacgatcaggatcgaggtgccgccgaagtaaaggctgttgcccatctgggcgaccatgaactcgggcagcaggcagacggcggtgatgtaggccgcaccgatcaccgtcagccgggtcagcacataatccagatactcggccgtgcgcttgcccggacgaatgcccggcaggaagccgccatacttgcgcaggttctcggccgtgtcctcggggttgaaggtgatcgaggtgtagaagaagcagaagaagatgatcagggcggcgtacagcgccatgaacagcggctggccatgcgtcagctgggcggtgaccagcggcagccagctcatccagctgggcaggtcggcgttggcggtcatggtggcgacggtcgtcggcagcatcagcagcgaagaggcgaagatcggcggaatgacgcccgcggtgttgaccttcagcggcaggaaagagcgctccccgcccgccatgcgattgccttcctggcgcttcggatactggatcagcagacgacgctgggcgcgctccatgaacacgatgaagaccacggtggcgacggccagcacggcgatgaacagcagagcgaaggccgacatctggccttgctgggccaggcccagcaggcgcgccaccgtgcccggcagcaccgccacgatgcccgcgaagatgatcagggagatgccgttgccgacgccgcgcgccgtcacctgctcgcccagccacatcaggaacatggtgccgcccgtcagcgtcacgacggtggagacgatgaagaagacgcccggctgatcgaccaggccggcctgggcgttcaggcccgccgcgatgccgaacgactgcgccagcgccaggaacaccgtcaggtagcgcgtgtactggttcagctgcttgcggccgctttcgccgccttcctttcgcagcttctcccacggcggatacaccgtgcccatcagttgcacgatgatcgacgccgagatgtagggcatcacgttcagcgcgaagatggccatgcgctcgaccgcgccgcccgagaacatgttgaacatgtccaggatgccgcgcgactgatccgggttctggaagaactgcaggaaagcctgcgagttgatccccgggatcggcacataggtgccgatgcggtagaccagcagcgcgcccagcgtgaacagcaggcgcttgtgcagctcggtcgccttggcgaacgagcccatgttcatatttgcggcgagttgttcagcggccgaagccattatgcgtccccacgactctagagccgtcagataggcggaaagcggcgctcttgcgaggccgctttcgttctttcgtcatcccgatgtcaatatggccacggtcgcggcgaccgggacgacgtatgcggatgtcaggcttgcgcggccgtgcggcgagcgcgggccgagaccttgttctcatcgccgcgcggcgccttgggagccggagccttgcccttggcggcgttgcgcttctcgacgcgggcggcggccttggcttccgcctcgatgcgctgctgggtgaccgagccgccggcggcttcgatcgccttgactgcgccggccgaggccgaccagacgaccaggttcagcttggccgacagctcgccggtgcccagcactcgcacgccgtccttggcgcggcgcagcacgccggcggcgaccagcgcctcgccgttgatctcggccgacgcatccagcttgccgtcgtccacggcttcctgcaggcgccacaggttgacctcagccagcttcagggcgttcggattgttgaagccgcgcttgggcatgcgcatgtacagcggcatctggccgccttcaaagcccagcagcgacacgccggtgcgggacttctggcccttgacgccgcggccggaggtcttgcccttgcccgaacccgggccgcggccgacgcgcatgcgcttcttgtgggcgccttcgttgtcgcggatttcgttcagtttcatgtgcctgatcctttcgggttctagcgcccgctgcagacagcggactcggcgttggaaaaatgaagggccgcttctaggcggccccgcatgggtaggcaagatgtgaaaacgccctcctccgggttggagaagggcgtcgtcgtcgtgttcttacttctcgaccacttccaccaggtggtggaccttggcgatcatgccgcgcaccgacggcgtgtcctccagcgtggactcgcggcccatgcggttcaggcccaggcccaccagggtggcgcgctggtcgttctttcggcggatcggcgaaccggtctgcttgatggtgactgtgttgttctcggccatgtctatcagccctcgatggcttccggcgccgaggcgccgtcgttgcgacgacccatcagatccgcgaccttcttgccgcgcttggacgcgacctggcggggcgaggactggaccttcagcgcttcaaacgtcgcgcggatcatgttgtaggggttcgacgagcccgtcgacttgcccacgacgtcctggacgccgagggtttcgagaaccgcgcgcatcggaccgcccgcgatgacgccggtcccgggaggggccgcacgcatcatgatcttgccggcgccccaacggccgttgccgtcgtggtgcagggtgcggttctcgcgcagcggaacgcgaatcatcgtcttcttggcttcttcggtcgccttgcggatggcttccggcacttcgcgcgccttgccgtgaccgaagccgacgcggcccttgccgtcgccgacgaccatcagggccgcgaacgagaagcgacggccgcccttcacggtggcggcgacgcggttgatgtgcaccagcttctcgacgatgtccgaatccggaccatcgacgggagcgttgcggttgtcacgacggttgcgatcgttgccgccgccgccgcgttggggttgatgcgccatgcttcgcgtcccttagaagttcaggccggcttcgcgcgcggcgtccgccagggccttgacccggccgtgatagatgtagcccccgcggtcgaaaaccacctcggtgacgcccttctcgatggcccgctcggcgatcagcttgccgatggcggcggccgatgcgacgtccgagcccttggagcccttgccgccttccagcgacgaggcggccgcgaccgtcacgccctgggcgtcgtcgatgacctgggccgagatgttcttgtccgagcggtggaccgacagacgcaggcggccgttggcgacggccttcaggcgacggcggttgcgctcggcgcggcgcttggcttgctgttgaagagagagagccatgacttacttcttcttgccttccttgcggcgcaccgtctcgccctggtagcgcacgcccttgcccttgtagggctccggcggacgcagcttgcggatcaccgcggcgatctggcccacggcctgcttgtccgagcccgagatcttgatctcggtctgcttgggcaccgcaaaggtcacgccggccggcggatcgatgtccacctcgtgcgagaagcccagctgcagcgacaaggcctggcccttcatcgcggcgcgatagcccacgccgaccagctccagcgtcttgtcgaagccttcggtcacgccggtcaccatgttggcgaccagggtgcgcgacaggccccacatggcgttggcgcgctggctgtccgaacgcggcgtcagagacagaccctcgccgtcctgcgccacttcgatctcgtcggcgacggtccaggagcgttcgcccttggggcctttcacggtgatggtctggccgtcgagcgtgacgttcacgcccttcggcacagtgatggttttcttgccgatacgggacatcttagtagaccctgcagaggacttcgccgccgacgttcgcgtcgcgagcggcggcgtccgacatgacgcccttggacgtcgaaaggatcgagatgcccaggccgttcttgatcggcttcaggtcgccgatcgccgaatagacgcggcggccgggcttcgacacgcgggcgatctcggcgatcaccggctggccgtcgaaatacttcagctcgatctcgaactgcgggaactcgcccgggttctgaaccaggttgtagccgcggatgtagccttcgtcctgcagcacgtcgaggacgcgctggcgcagacgcgaagccggggtcagcaccttggaacgcttgcgggtcgcggcgttcttgatgcgagcgatcatgtcgctcaggggatcgttgatcatcatgactgtcgtctccccttaccagctggacttcgtcaggccggggatctgccccaggttgccgagctcgcgcagcgcgatccggctcatcttgagcttgcggtagaacgcgcgggggcggccggtcacttcgcagcggttgcgaatgcggttcggcgcggagttccgcggcagttccgccagcttcaggcgcgcgtcgaagcgctcctccagcggcaggctctcgtcgttggcggtcgccttcagggcttcccgcttcgcggcatacttcgcaaccagggccttgacggcttcgttgcggtttacggcgctcttcttagccattgttctcttcccttcccgctcagttcgtcacgaacgggaacttgaactcgctgaggagagccttggcttcctcatcggtcttggccgtggtgcagacaacgatgtccatgccccacatctgatcgatctggtcgtagttgatctcggggaacacgatgtgctccttcagaccggtggcgtagttgccgcgcccgtcgaacgaggtgcccttcaggccgcggaaatccttcacgcgcggcagggcgatcgtgatgaaccggtccaggaactcgtacatctggtcgccgcgcagggtgaccttgccgccgatgaccatgccttcgcgcagcttgaagccggcgatggagttgcgggccttggtcggcaccgccttctggccggcgatggacgacaggtccttgagggcggcgttcgccttcttggagtcggccacggcttcgccgatgcccatgttcaggacgatcttgtccagcttgggcacctgcatctcattggtgtagccgaacttttccttcatcacctggcggatgcgcgcctggtattcgcccttgaggcgaggggtgtacttctcggtagccatcagatgacgtctccggtcgtcttggcgaagcggaccttcttgccgtcttcgtcacggaagccgacgcggctcgccttgccgttggcgtcggcgaccgcgacgttcgacaggtgaagcgaggcttccttgttcttgatgccgccctgcgggtcagcctggctcgggcgcgtgtggcgctggaccatgttgacgccttcaacgacgacgcggttctcggtcggcaggacgcgcagcacgttgcccgtgcggcccttgtccttgccggtcaggacgacgacgcggtcgcccttcttgatcttggcggccatgttacaggacctccggagccagcgagatgatcttcatgtggttcttggcgcgcagttcgcggggaaccgggccgaagatccgcgtgccgaccggctcgttctgcttgttgacgatgacggcggccgacttgtcgaagcggatgaccgaaccgtccttgcgctggatgtccttggcggtgcgcacgacgatggcgcgcacgacgtcacccttcttcacgcggccgcgcggaatggcttccttcaccgaggcgacgatggtgtcgccgatcgaggcgtagcggcgcttggagccgcccaacaccttgatgcacatgacccggcgggcgcccgaattgtcggccacttccaggttagtttgcatctggatcatttgatcagatccttctgattacgaggccgaagccggggaaaggacttcccagcgcttcagcttggacttgggggcgcactcgacgatgcgagcgacgtcgccgaccttgagcgcgttggcttcgtcgtgcgcgtggtacttcttcgaaagacgcacggtcttcttcagaacggggtgcagcagggtgcgctccaccttcacgacgacggtcttctcgcccttgtcggagacgaccacgccttcaagaattcgcttgggcatattcgtttccttaggaagccgaccgcttctcacgcaaaagcgtcgagatgcgggcgatgtctttgcgcacttcgcccacgcggtgggtcttttccatctggccggtggccgcctggaagcgcaggttgaactgttccttcttgagccgcagcagctcgtcggacagctggtccggggtctggccccggaggtcggcgatcttggtcatcaggccgcttcctccgcgagagcgacgccggcgtcgagacgggtcacgaccttggtgcggaccggcagcttggcggcgccgagacgcagcgcctcgcgggcgatgtcgtcggccacgccgtcgatttcaaacaggatgcggccggggtggcagcgcgcggcccagtggtccacggcgcccttgcccttgcccatccgcacttcggccggcttgccggtgaccggcaggtcggggaacacgcggatccacacccggccctggcgcttcatctggcgggtgatcgcgcggcgggccgcctcgatctgacgcgcggtgatgcgttccggctccagcgtcttcaggccgtaggagccgaagttcagcgagaagccgcccttggccgcgccgtggatgcggcccttgaaggccttgcggtacttggtcttcttcggttgcaacatgacttagctctcacgtccccgatcgcgacgcggaccgcggtcgccacgggggccgccgcgttcgcggccttcgttcgacgacggacccgaagcttcctgggcccagcgcttgtcctgagccatcgggtcgtgctccagcacctcgcccttgaacacccaaaccttgacgccgatgatgccgtaggtcgtcttggcttcgtagaagccgtagtcgatgtcggcgcgcagggtgtgcagcggcacgcgcccttcgcggtaccactccatccgggcgatttcggcgccgcccaggcgacccgagacgttcatccggatgcccttggcgcccagacgcatggccgactgcatcgaacgcttcatggcgcggcggaaggccacgcggcgctcgagctgctgggcgatgttctcggccaccagttgcgcatcgacttccggcttgcggacttcgacgatgttcaggtggacttcgccttcggtgcgcgccgagatgtccttgcggagcttctcgatgtcggcgcctttcttgccgatcacgacgcccggacgggcggcgtagatggtgatgcggcacttcttgtgcgggcgctcgatgatgatgcgcgacacgccggcggccgacaggcgctcacgaagccactcgcgcagcttcaggtcctggtgcagcaggcgggcgtagtcggcgccgccggcgaaccagcggctgtcccacgtgcggttcacgccgaggcgcagaccgatcggattgattttctgacccatcaggcggcctcgccggcttcacggaccacgatggtgatctcgctgaacggtttcaggatgcgcgaagagcgaccgcgagcgcggctcgcgaaacgcttcatcaccaggttcttgcccacgaaggcctcggcgacgatcaggttgtcgatgtcgaggttgtggttgttttcggcgttggacacggccgaatacagcaccttgcgcacgtcggtggagatgcgcttgcggctgaactccagctcgttcagcgccttctgcaccggcatgccgcggatcgaggcggccaccaggttcagcttctgagggctgatgcggacgttgaccagcttggcgcgggcttcggtcggggcgacccgacgttcgttcttggactgggccatcggattacttcctcttggccttcttgtccgccgcgtgacccgggaagttccgggtcggggcgaactcgccgaacttcatgccgaccatctcttccgagaccgacacgggaacgtgcttttggccattgtgcacgccgaacgtcagaccgacgaactgcggcaggatggtggagcggcgcgaccaggtcttgatcacgtccttgcggcccgacgtttgaacggcgtcggccttcttgagcagatacccgtcgacaaacgggcctttccaggaggagcgggccattcttagcgagccttcttcacgtggcgggtacggatgatgaacttgtccgtagccttgttcttgcgggtgcgggtgcccttggtgtccttgccccacggcgtgaccggcgtgcggccgcccgaggtccggccttcaccaccaccgtgcgggtggtcgatcgggttcatggcgacgccgcggacgtgcggacggaagcccatgtgacgcttgcggcccgccttgcccaggttctggttcatgtggtcggggttcgaaaccgcgcccaccgtggcgatgcagccgtccaggaccatgcgcagctcgcctgagccgagacggatttgggcgtagccctggtcgcggccgaccagctgggcgtaggcgccggccgaacgggccagctgggcgcctttgcccggcttcatctcgatgttgtggatgatcgtacccacgggcatcgagcgcagcggcatggcgttgcccggcttcacatcgaccttttcgccggcgacgacctggtcgcccgccttcaggcgttgcggcgcgatgatgtaggtcttctcgccgtcctcataggtcaccagcgcgatgaaggcggtgcggttggggtcgtactccagacgctcgaccgtgccgaccgcgtcgaacttgcgacgcttgaagtcgatcttgcggtacagggtcttggcgccgccgccgcggaagcgaacggccacgcgaccgccctgcccgcgtccgcccgacttggtcaggccttcggtcagggacttttccgggcggcccttgtgcagctcggaacggtcgaccagcaccagggcgcgacggcccggggatgtcggattgtaggtcttcaaggccatctgatcagagccccgtggtgacgtcgatcgactggccgtcggccagcgtcacgatcgcttttttgatgtcgacgcggcgacccaggatgccccggaaccgcttggtcttgcccttttgaaccagggtgttgaccttgaggacgttgaccttgaacaggctttcgaccgccgcggcgatctcgtccttggtcgcggtgtcggcgacgcggaagacgaccttgttctgctccgacaggatcgtagccttttcggtgatcaccggggccaggatggtgtcgtagtgcttggcggtgggttgagcgccggccattacgcggcctccttctcaaagaagcgcgcctcgatcgcctcaatggcggccttggtcagcaccagcttgtccgcgcgcaggatgtcatagacgttcaggccggcgttcggcagcacgtcgatgtgcgggatgttgcgcgcggccagaccgaagttcacgtcgacttccggaccggcgatgatcagggccttggcccatcccagcttgccgaaggcctcgcgcagggcggcggtcttggcgttctcgacgttcagggcgtcaacgacgaccaggtcgccggccttggccttggacgacagggcgtgacgcagggccagggcgcggaccttcttgggcaggtcgtagccgtggtcgcggacgaccgggccgaaggcgcgcgagccgccgacgaactgcggcgcgcggcgcgagccgtgacgggcgccgccggtgcccttctgcttgtacatcttcttgcccgtacgagagttctcgttgcgggtctggaccttgtgcgtgccggcgcggcgcttggccagctgccagttcacggtgcgggccagcaggtcgccgcggatgtccgagatgccgaaaacggcgtccgacagttccacgtcgccggctgcgccgccgtcgagcttgatgacagagagtttcattacgcttcaccgccttcggtcgcttcggccggggcttcttcagccggggtcgaggcgggttgagcagcgcccttggacttgaccgagcccgggaacggagcgtccgccggacgggtcttcttgatggcgtcgcgaaccttgacgtagctgccctcgtgacccgggacggcgcccttgatcatgatcaggccgcgctcggcgtccacgcggacgacggtcaggttctgggtggtgacgacttcctggcccaggtggccggccatcttcttgcccgggaaggtgcggcccggatcctgacggttacccgtggagccgtgcgaacggtgcgaaaccgagacgccgtgcgtcgcgcgcagaccgccgaagttccagcgcttcatggcgccggcgaagcccttgccgatggtctcgccctggatgtcgaccttctggccggcgatgaagtggtcggccgacagctcggcgcccacatccagcagaccgtccgcatcgacgcggaactcggtcacataagccttgggctcgacttccgccttggcgaaggtctcgcgttgagccttgttggtgttcttggcctttttcatgccggcgcccagctgaccggcgacgtagccgtcccgctcctgggtacgctggccgacgacttggcagccgtcgagctgaagcacagtgaccggaacgtgcgcgccgtcatcggcgaacacgcgggtcatgcccagcttcttggcgatcacgcccgtgcgcatcggatcccgcctctttcttctttagatcttgatctcgacgtccacaccggcggacaggtcgagcttcatgagcgcgtccacggtctgcggggtggggtcgacgatgtcgagcacgcgcttgtgcgtgcggatttcaaactgctcgcgcgacttcttatcgacgtgcggcgagcggttcacggtgaacttttcgatcagggtcggcagcgggatcggaccacgaacggtcgcgcccgtgcgcttggcggtgttgacgatctcgcgcgtcgaaaagtcgaggacgcggtgatcaaaggccttgagcctgatgcggatgctttgatccatatcggtgcttacttccaatgcggtcggaggaccgcgtccctgtgaaccatttcaaagaccgaagccttcgggcctaggccctcaggtacgcaaatccgcaaaaacgatcggcccacgcagtcccccgcgaaggccgtgaagtcccaagaagctgcaaagaacaggtacttaggtcgtccctgcgaaccgcgtctgcatccggggatgcacagccggtccaacaagagtggcgcttatgccgatcgattccgctttcgtcaagcgcatcctgcagacgggcgtcctcggtggagggcttcggtgaaacgccgatcggcagctgggcggggccacaagcgagtctggggtggcgttaacggcttcgctttcttacgcacacagtagcgacacatatgcgccacatcgcgtgtcggttcggcaacaacgaagcacgtgatgggcaagcggcgcagttttcgtcttccgatctcatgcaatgctggtagcagccgccccccgccccgccggaatggtccgtgggcggagagaagaagaagaacggacacttgagtatgaagacccttttcctcgcctcggccgccgccgccgccctgttcgccgctcccgccgtcgcgcaggacgccatcggatcggtgggcgtgtcctacgcgaacccgtcgatcgacaccgacttcggcgacgccgaagccgacgtctggaccgtggacggcacggtggccctgccgatgaacgactggaccgtcacgctgaacggctcggtcgactacgtcgaggctttcgatgaaagcgacacctccggcgcagccgccgcccacttcacccgcatgttcgcccccgacgtgcgcgccggcgcctttgcgggcgtcagcaacctgggcaacgaagagctgtggaccgcgggcgtcgaagcccagaagtatctggctcaggccaccctgaccggtcagatcgcctacaccaacgccgacgacctgctggaaggcgtggatgccgacatctggacggtgggcgtcgacgccgccttctacctgacgccgcagctgcggctgaacgcgggcgccagctacaacaatgtcgacaccgacttcggcgacggcgacgcctggacctacggcgtgggcggcgagtacgagttcgccaactcgcccttctcgctgactgccggctacacccgcgccgacatcgagtcggtggacctggacgtggacagctggaccatcggcctgcgctacagcttcggcggcggcatccaggcgcgtgaccgcgccggcgcttcgctgggctcgcccgcgatgacgtccattctggccggcttctaagcctcacggcccaacaaaggacgaagccccggcggagcgatccgccggggctttcccatgccgggtgcaaagagagaggccgagggttccacgacccggcccctctccgtcgcgagcgacccggtcagcgcccgatgctgaccgtgcccgaaccgaccaccgaacgggacaccggaccggaggcctcggccaccgacacgtcgccggagccggcgatcgccacctccagatccgccgtgcgaccgccgtaacggacattgcccgagccgccgaccgccacctcgagcctgggcatgtcgccggcgcggatggtgatgtcgcccgagccgccgatggcggcttcgcccggcccgtccacgcgcgccacggtgatggagcccgacccgccgaccgaggcctccagccgtcgggtcgcccccgccatgatggagcccgacccaccgactgcagcctcgagcgcggacgaggttcccgcccggatcgttccggatccgcccagcgccagggacatcttgccccccgtattggcgaccacccaatcgccgcagccgccattgcccagatcgatgtcgctggcgccgcgcccgaccgagccgaacaccgcgccgctcgcgcccacgtccaccgagcggggcgtgcgcagcacgatcagcggggcgtcctccagccgcacgcggccgatgcggcggacctcgaccggcgcgccttccccgggctggcgagcgctcgagggaccgctggagcagttgcggaaagcgttgcgaaggccgccgtcgatgcgcacgtcgccgccccggcgctggacccggggcgccggcaggtcggcgcggccgggcgtgatctccacgccgatgtccgatcggtcctcgacgatcaccacgacgcgggcgatggcgtccttgatctcgacatcggcggcgaaggcgggcgcggcgcagctcgtagcaacggcggccaagagtgcgaacggggcagtcttcatcgggtctcttcctctccagctatgaagaaaagagtgccccccgctcggcctcaagtcattttaactcgaggtcatgacatcgatttaacccgcgggcttcagcgcgcccgcgccgtcggccgcgccgacctcaggctcaaaatcgcgctcgaagctgttcagccggctcttcagcaccccggcctttcgcagagccaccgacgccgcccagcgcgccgccagttcgggtcggctcatcgcgtcggtgaagcggggccgcccgcccgccttgcgcacggccgcattggcgaacagggcgccgttgcggaaccgcgaggtccaggtctggaaatccatcgacaggctgacgcagaagcggccttggttctcaacacggtgcggcgcatagatcggccaggtcagcgcctgccccggttccaggtccatgacctgggcgtcgtcttcgaacgccagcgtgtagggcagttcctcggtcgtctggcgcgccaccacctgctccatctcccgctccggcaggtgcgcctcgtcgcccggatagacgaacacccgcttcttgccgcgcaggtggaacagcaccacgccagcagcatcgaaatggtagggcgcgcccgatcgcggcgaagacaggatcaactggcccgcattgcgcaccgccttcatgcccggataggtcgcctggatgcgacggaagtcctccatcgctgcatcccacaactcgggccagccggtctccacctgccgcagattgacccaaagccgaccctgcttgatcgcctccagtagctccgccccggacagccgcccacgcgcgccggtgcgcaacgagacctggccctccgcgtcgtagtcgtacaggttgatgtcgaacagttccgccggatagcggtccagcagcgcggccagcgcctcatcctctgcgaagccccggtcgttcagcgtgtgcggatggatcttcgcctcagcgatcggtccgggatagcgagtacgacgctggttcatgatgttgctcatcaggcgtgcgccacgcggtggggcgtctttctgcgggccagggccttgttcgcggccgcgcgcgccgcgaccgccgcgccccgcgcccgcgccagcggagtggtctcgcacgcttcgatcgcggcccatcgccggcggatgctggtgcgcagcgcatcgccccgcccgccgccggcccggttcagcaggtccgccgccgcgtcgctgacggtcgcctgcacgcccggcttcagcaccacggcctcccgcacggtctgtcggtcattgcagaagtacttcttgtagtgctcgccctcgaagccgaagtcgaagacgcgaaagccgtcggcgctcgcccgctccatggtgtccatgctcaagagaatgcccggcgagcagcgcgccagactcggctcatagacagggaaccagaaatgatactggtcgccggcgtggagcgagaactccagcgcggtcagctcgccgcctgcgtgcatggtcgctatggacgcgccgaaatcggggtcatccgaggccatcagcgcgtgcagcagccgccgggtccagtcgcaggcgaagatgtcgtgcaggcccgagcgccggtactgcgccgacttcaggtcgatcagccggtccagcagcgccgcgtcgcggacctcgtgccgcacctcgatcgggccaagctccgcgagcaggctgcgccgcgcccgttccttgtccttgaagtatttgccgaatgtcctgcgccgctcggcgtaccagtcgacgtagccgctctccggcagccgcaccatcaccgtctggcgctccccgcccgcctgtccctctccgagccaggccgtgaccgtcagccggctggcgttcagcagctgcgccacctcttccagcgagatgtcgacgccgggcgcggagatcacgccgtggtagtcgttcatcggcgcgcccagcggctgcaccgcccgcccccgcctttgatgcgcaaagaagccgacgacctccccgccgcgccgaaacaccgccactgcggccccggggcatacgcgcgaggcgatctgagcatagcgccaatggaagtacgggctcgccagccttggatcagcggcccgccacagccgccacagcgcgatctgctcgggcgacagcgcctcggcccgggtgatctcgaccgaaacgggtgggttcacgcgccttcatcctctcgtcgacccggcggtcgcctcgcggacttctaagcccgtgcgtctttcaccacggttgaccaccttggtgaacgaagccttttcgggagccgccggccgaaccaagcgttggtgttgctgacgatctttctaggacacgcccccatgaccgacgaacgccccgccccctatccgtcgcagtacgagaaccagcgcaaggacggacctcaaggacagccgccgcgaccggccaccgagcccaagggctcgcaagggtccagcaactccggcgaaaccgccaccgacccggccaccggcgccccaaacgactgacgccgcgctctcgtcccaagttcctgaaccagaaagacctcttcatgattgatcgcctcgcgcgtcgctgcgccctgccggccgtgtccgttctcgccttgcttgtcgctggatgcggggcgccggaaccatccggagccgagcaggcaggcgcgagcggcggcgcggtgggcgcccagggacctctctcggggcagtccatcaacgatgccgcctatcaggcgacgccgcagcccgccccgcccgctcaggagggccagcccgccgcccagcctcagcccagtcctgcgctgatccgcgcccaggtgctgctggcccgcgcccgcttctcccccggcgccatcgacggtttgggcggaacgaacacgcgtcaggctctggccgcctggcaggaggcgcaggggctcgaggccagcggcgatctgacgcctgaaacctaccagcgcctgatccaggcgggcggccaacccgtcacgaccgagtacgagatcacccagcaggacatcgccggcccctatatcggcgtcgttccgaccgaggtcgagccgcaatccaagctgccggccatgggctatggaaacatcgtggaggccctggccgagcgcttccacgtcagcgaggccctgctgcgcgccatgaacccttcggctgactttaaccgcgccggccaaaggctggtggtgccgtcagtgggccagatccagctgcccgccgacgtcgtccgcatcgtcgtcgacaagagccagagcgccgtcatggcctatggcgaaaacgaccagctgatcggcttcttccccgccaccatcggcagcggcgacaatccgaccccgtcgggcacgctcaaggtcaacggcgtcgccaacaatccggactatgtctacgatccggacaagctgtcctacggcaccgccaccgagcggctggtggtcaagccggggccgaacaatcctgtcggcgtggtgtggatcgacctgaacaagccgtcctacggcatccacggcgcgcccgagccagagaccatcggcaagaccgcgtcgcacggctgcgttcgcctgaccaactgggacgtgcaactgctggccgcgcgggtgaagcccggcgttcaggtcgtcttccagggctgacctgagcgatcggagcggcggctagggcgccgccgctccaaaggtcgtgccgtcccacaggtcgcagtggtgacgctcgaagaaggtcgaatcgatccggtcgccttgcgggtggaacacgcggacgggcccgccgccctgcgtcacctggggccacgccggatcgaagcccgtctgcccgaaaccggcccacaggctgcgcatccgcgccgacagagcgcgctgttcgggcgtgaaccgcttcacatccgccaggatccagctggtcccgaacacataggccagttcgccggcgtggtaggcgccaagatccagcccgaccagccgatcgggcaggacaaagggcgcctggcgatcggcgaactcgtacccccataccggcccgtgccgcgcaagcacccgacgcagcgcgtgggacgggcaggcgaaccgctggtcggtgaagttggtggcgatggcgacggcggttccttctttcccgacgggatagcgttccagcacgcgcgccgcctcgtcgccgtacatccaggcggtctccttgacgtagcgatccatgctctggacctcgttggcgaacagacgcccttcgtccaggttggtgccgaccatcaccggcgtgcgcacgtatcgagcctcgtggaaggcgacggcggggttttcgggcgtggtcctgtcgccgtagaccggcccccacgaaccaagaccattgatccccgcccgcagcgacggcgcacgagcaacccgccaggccggcgtcttcctcaaacatccgatctgatcctcgccggcgcaccccagcgcctcggcgaaggccgggccgctcttcgccgcctcttgcgccggaacgagcgacgacggctccaggcatccgccgctctgcaggatcacctggtggaacagtccctccgaacccggcgacgccatcaggtagcaggcgctccacgcccccgcgctttccgcaaacagggtgatattgcctggatcgccgccgaaccctgcgatgttgtcgcgcacccagcgcagcgccgcctgctggtccatcaaaccgaagttgcctccgacgccgtcgccgtccttcgccatctgcggatgcgccagccagccgagcgcgcccaggcgatagttgatggcgaccaccacccgcccctgctcggccgccagccgcgaaggatcgtagttggcgcccgagccgcccgtgaacgcgccccccggtacatagaccatcaccggcatctgggtgtcgcgcgcacccgccggcgcatagatgttcaggtaaaggcagtcctccgaccccacaacgatcccgccgccgccgccgaggatggccttgcgcccaacggcctgggtgcagtcggacccgatgcgcgtcgcgtcccgtcggcccttccagggctccaccggctgcggcgcgcgccagcgcagctcgccgaccggcgggcgggcgtaaggcacgcccaggaaggcgcgaacgcctgcgccctccacgccccgcaccacaccggcctgggtggaagccagcaccgtctcggcatcggaggcgaagcgcacctggtgcacgcggccaggatggatggcgcaggccccgaggccgagcagagcaaggagggcaagccgggtgagtgaccgcatcgtcgaaccttggcggtgggaggaacagccgtaacgcgccgccgccgctcagtttcccggatcaggagccagactgttgaaccagtcggcgtacaccgtgttgcgggccatccggcggttcaggtcgggcgctccgtcgctccaccacaccgggccgcgttcgccaagcgcgcgcttcgccgcatccacccttgctcttgcctttgccacggcctggtcgtcgccggccttcagccccgccccgacctctcgccgtgcggccatgagggctgagacctgcgcgctgcgctcggcgtcgggcaggtgggggttgctcctgcgccacagccggcctcgcaccacaaagtagcggccgtcgggcgtatcgggatagcgatcctggctcatgcgccggtaacgcaaaacccccgccggatggctccgacgggggtgatgttcagcctaaagaccgatcgcgatcaggcgatgatcttggagaccacgccggcgcccacggtgcggccgccttcgcggatggcgaagcgcagcttttcttccatggcgatcggggtgatcagttcgacgttcagctcggcgttgtcgccgggcatgatcatctccacgccttccttcagctgcacgatgccggtcacgtcggtcgtgcggaagtagaactgcgggcggtagttggtgaagaacggggtgtgacggccgccttcttccttggtcaggatgtaggcttcggccacgaacttggtgtgcggggtgatggagcccggcttgcacagcacctggccgcgctcgacgtcttcacgcttggtgccgcgcagcagcacgcccacgttgtcgcccgcctggccctggtccagcagcttgcggaacatctccacgcccgtgcaggtcgtcttctggacggggcggatgccgacgatctcgacttcctcgccgaccttgacgatgccgcgctcgacgcgaccggtcaccacggtgccgcggcccgagatcgagaacacgtcttccaccggcatcaggaacggcaggtccaccggacgctcaggctgcgggatgtagctgtcgaccgtggccatcagctccagcacgcgctgctcgccgatctccgggttcacgccgtcggtcgcggccttggccgagcccttggtgatcggaatgtcgtcgcccgggaactggtaggacgacagcagctcgcgcacttccatctcgacgagctcaagcagctcctcgtcgtcgaccaggtcgaccttgttcatgaacaccaccagcgccggcacgccgacctgacgggccagcaggatgtgctcgcgggtttgcggcatcgggccgtcggccgccgacaccaccaggatcgcgccgtccatctgcgcggcgcccgtgatcatgttcttcacatagtcggcgtggccggggcaatcgacgtgggcgtagtgacggttttccgtctcatattccacgtgcgccgtgttgatcgtgatgccgcgagccttttcttccggcgccgcgtcgatgtcctcgtacttcttcgccgtcgcgccgcccgacttcgccagcgtcatcgtgatcgccgccgtcagcgtcgtcttgccgtggtcaacgtgaccaatcgtgccgatgttgcagtgcggcttcgtgcgttcgaacttttccttggccatcgccaaaactcctgattggcccgggtccgttcagcggatgggcgtcatgctcatcaaaaacctggagcgggtagacgggatcgaaccgacatcctcagcttggaaggctgctgcactaccattgtgctatacccgcgcaaagaatgcgggcgcccacaagggacaaccgcacccggccgccttggttatccaggatcaaccgtctcaagaagcgcgtggtgggggaagcaggactcgaacctgcgaagcttacgcaggggatttacagtcccccccctttgccgctcgggacattcccccgcgcgcgtctcgaaaccgccgaaaccgcttcatccacgaccattcggacgagggtgaaacaaaagccttcggcttgtcccaccgcctagtttagacggtgcgccagacccgaaagcccctggggctccaaatcggagggcgtcttatagtgtcgtcgaaaacagaacgcaacgaccggaaacaggggaaaaacgcgggcgcgaaatcgcgcggcgacggcccgcgtccgcgccctcaaacccccgccccgcaaggacgcggagccgccgagggaccgcgcgggtcgtcacgcggaggcggcgcaggccgtgcggatgcggacaacttcctgtggggtcggcacccggttctggcggcgttggcgaatcccgcccggcgcggcgcgggccggctgctggcgacgccggatcgggccgaggagatcgagcgcgacaacctcgcgcacgggcaccgaatcgaggtggtggacgcgcagggcctgacgcggatgctgccgcagggcgcggtgcaccagggaatggccttcaaggttcagccgctggagggcgtcgcgctggaggcgatcgcggaaccggcggaggggctgatcgtgatgctggaccagctgaccgatccgcagaatgtcggcgcgatcttccgctcggccctggcgttcggcgcgcgcgggatcgtggtgcaggaccggcacgcgccggcgctggccggcgccctggccaaggcggcggtgggggcgaccgaacggctgcctcatgcgcgggtcaccaacctgtcgcgcgcgcttgagcggttggccgacctgggctggcgggcggtgggtctggacggatcgggcgagcagacgctggaagaggcgctggacgcccgaccgaccgtgctggtcatggggtcggaaggcgacggcatccgcaggctggtggccgaacactgcgacgccctggcgcgcatccccatgcccggcggcttcgagagcctgaacgtgtccaacgcggcggcggtggcgttgtacgaagcggcgcgggcgcagcgcggctgacctttttcctcttagcaggcctgccgatgcgcccgagaacaggtgcggcgcttggcgcggcgagaggtcgcggctagagagcggccatggaattcttcgcctcccccgatttcgccagccaggcgtccgccctcggccaggtcctgctgatggacctggtgctggccggcgacaacgccgtggccgtgggcctcgccgccgccgccctgccccaggaccagcgcaagaaggcgatcctgatcggcttggccgccgcggtggtgatgcggatcggcttcgccctgatcaccgtgcagctgctggcgctggtcggcctgctgctggcgggcgggctgctgctgttgtgggtgtgctggaagatgtggcgcgaactgcaggagcagcgcacccacgatcaggccgaggccgaggccgagctggagctggccctgagcatcgagcacggccagggcccctcgcccgaggagctggggctcaagcgcaagacgttcggcgcggccctgctacagatcatggtggccgacatcaccatgtcgctggacaatgtgctggcggtggccggcgccgcgcacgagcacccctggatcatggtgttcggcctggtgctttcgatcgccctgatgggggtggccgcgaccttcatcgccaagctgctgcaccgctatcgctggatcggctacatcggtctggtggtggtgctgtacgtcgcgctgcacatgatctgggacggcgcacgccaggtggtggtccgcacgggcaacttggaacagttcaacgcctccgcccccggtttcctggagatcggcgaagaggaagccgcgcatcatcccggccggcagcggagcgagaccagcgaagtgcctggccccgccgaacccgatccggccgccgcccgatgacgggcgtggccgccgtcgacgtccagcaggcgcacgacctgatcgaggccggcgaggcggtgctggtggacgtgcgcgagccggacgagttcgccgccgcccgcatcgagggcgcgatcctggcgccgctcagccggatgcctcaggcctggcttgggctggaccttccggccgacaagacggtgatcgtcatgtgccgcgtcggcgggcgcagcggccgggtgtgcgaggcctttggtccagagggaccggacggccaggcggtggtcaacatggacggcgggattctggattggcaagcggccggcctgccggttatcacggaaggctgacgaagcggtccatgaagcaggcgaagcctggagttcccagcgtcgtcaggctcgcttccacgtccccactggtcgtcggccctctgttctcgtgcaccatcactttgtgcgcagccaacagttcgtccgagtagacgatcatccctgcacccggaggtgcgcagatctcccgcatctgatcgggcggtaggtcggcgatgcggcccatccatcggaaaaagtcgacatcgacccccgccttgagcagaaacgcgtcttggcgtgcgatctgagcatcgatgtctgcaaggacgctctcgaccgcaccttccaactgatccggaggaacaagctcttccaaaccggcgcggacggcggatcgctcctgagggaagacgccgccgtggaacatcagcaccgcttggtcatcaatgacgcgccggtccgcagccgtgaacagatagttcgcgcatgatgaggcgcagatttggtgcgtgatgacggtggagacgcgcgggatcagggcctcgcccatcgccatgccggcgttcacctctccgcctcccgaccgcaccacgaccaccaaaggagcatcgggatcggttttgttcagcgcctggacgaacgcagccgagctttcggcatcgatcgggccggtgaagcagagaccgtcgtcgcctatggcgtacgtctgcgccggcgcatcatgggcgctcgaactcatccgatcagaacaggctgacagaacctcggcctcccggcccggggccccgatctcggggaaggcgagtaaagcgagcagaagggccaacagcatacgagtgtttctttgctattccgcgccgccgaagcgttccgaccattcggcgacctgggcgtcctcgatcttggcgaagagaacgccttgggcggcgacggcctgacccggggacaggacgttcagcaggtctttgtctgcgtggggccaactgaggtcggctgagccgacggacgccgcgatcttctccgccgagaagggcaggatcggcgccgccagacgcgcgaacagggcgacgaggttcaggccggtgcgcacgcccaccgccgcacggtcgtggtccgtcttcagcgcggtccaaggcgccgcctcctgcaggtactcgttgcccagcacccagcaggcgcggatggccgcggaggctttgcggaactccatggcctcgaaatgctcggtcgcctcggcgatcccggcgcggagatcggccaagagcttcgcctcgatcgggccgggctcgccgccgtcgggcacgacgccgtcgaacttggactccgcgaacttgacgatgcggttgacgaagttgcccaggacgtctgccaggtccttgttggtcgagacctggaagtcctcccaggtgaagggcgaatcggcgtgttcggggccgtaggcggtcaggcgccagcgccagtagtcggcgggcagcagttccagcgcctggtccatgaagacgccgcgcttctgcgaggtcgagaacttgccgccgtaccagttcagccagttgaaggccttgagctgatccaccgtcttccacggttcgcccgagccgatgacggtcgctgggaaggaaaccgtgtgaaaggcgacgttgtccttgcccatgaactggacgtatcgaacgtcttcagcaccctcgtccaggcgccaccagtcgcgccaggttgtgccggtcgcctcggcccactcctgcgtcgcggcgatgtattcgatgggggcgtcgaaccagacatagaagaccttgtcctccatgcccgtccgggggaggccgtccttggtcaccggcacgccccacgccaggtcgcgggtgatgccccggtcgatcaggccttcgtccagatgcttgtaggcgatggacttggcgagttgctgccagccggacttgccgtcgacccaggcgcggatctctggctcgatccgggtctgcagaagatagaggtggcgggtgtcgcgcacctccaggttcttcgatcctgaaaccgccgaataggggtcgatcagatcggtgggatccagcaggcggccgcagttgtcgcactggtcgccgcgcgccttggcgtaggcgcagtgcgggcaggtcccctcgacgtagcggtcgggcaggaagcgggcgtcgtcgatggagtagatcatgcgatccacccgctcctcgatcaggccgttccgctccagtgtctcggcgaaatgctgggtcaggcggtggttctgcgggttggacgagcggccgaaccagtcgtagctgaggccgaacgcctcgcccgcacgcttctggatctcgtgctgttcgtcgcaataggtccgcacgtcctggcccgcagcggcggcggccagttcggccggggtgccatgctcgtcggtggcgcagatataaagcacctcatgaccctgcgcccgcttgaagcgcgcccagacgtccgccggcagcatcgatcccgccaggttccccaggtgcttgatgccgttgatgtagggcagcgccgaggtgatgaggatgcgggccatggtcgtccagacggttcggggaggcgtcggatatagcgagcgccacggcaggcgtcacccttggcgggatcagacccgcagcggccgcctcgccacgcgcaggaagcggccggtcagcagtccgcccgacaccaggctggcgatgatcaccgcccacaccagaccgtcgacgcccatctggtgcgccagcacccagcccagcgggatcatcactagtccatacgagccgaagtgcatgatcgtcggccaccagacgtcgccggcggctcggttcgcctgggccgccacgacctggatgccgtccgcgacgaagaacagcgtcgccagcgccagcgccggtcccgcgatggcgaccaccgccggatcggtgctgtaggcccgcaccagcagcgccgccgtgggccagatcagcagggccacgatcagggccagcaccgtcaccaccgccagccctacgaggccgccgcgcagcacgcccgcccggtcgtgtgcgccatagctctggcccaccacaacggcggtggcggacgacaggcccatgggcatcatgaagacaatggccgacatgttgatgacgatggcccagcccgccgtctcggccgcgcccagcaggcccgcgatcaccgtcatggcggcgaaggccccgacctcgatgaagttggaggcgccggcgcccaggcccaccttgacctgttcgcgctcggtcggacgatcgcgcgcgggcttgcgccagaggttccaggtcttcgcctccggcaggcggacgatgtagatcaccagaaacaccgcaagggcggtgcgcgcgccgaaggtggcccaggccgaggccgccgcgccgtcgacgccgaggttcaggagatccggcaccagcaggaggttcagcgcgacattgacgccgttggccacccacatcgcccacatgcccggcttgggccgcgacagcccttccaggaaaaactgccccgccaccgagatcagataggcgggcatggacaaggcgaagatcaccagcggcagggccgcgccctcgcccaagccgtcctcgaagccggcgttgcgcatgatccagggtccggccaggaccatcagcagcagcgacgccacgccgatctgaagcgaatagacgacgccgcgtcgcagcaccgccccgacttccgcgtgccgcccctcgcccagcatgcgcgcggtcatcacctgcacgcccatcatcaggccgacggcggtggtcaacaccaccgacgacggcgcccaggccagcgagtgaaatgccagctcctgcgacgaataatggccgaccacgatggcgtcggtcaggcccatggtcatgatgccgatgcgcgccagcacgaccggccaggccagggacgacaactggcgcagggtggagcgggtttcggtcgacaggacggacataggaggcggcccagaccacgcgcggccgtccgggtcaactcagcggcctaccaggccccgagttcgcgaagctggcgcaccagttcgtccggcgcctcgcccgcatcgaccgacgacagatcgaccggggcgtccttggcctcgaaatagcgccagccctggaatgggcgtctacccaacggcgcggtgcgcacaaccaccggctccagcgtgatctcacagcggctggccttgccctcgccatgggtgcggatgtccagcaccggctggcggcagacgatcgttcccttgacgacccagaacaacgaaccgccgtcctcgatttcggccgcccgcttcggagtcatgcgggtgtggacgatgtgcggctgtccgctctgggcgcgtcgctccagccattcgacgtcgggcacgccgacgcccagcttgatcatgtgaaggggcatggccgccaagtagggaggcgcggccccggtggctacaatcttaatgaagacggcctatggcgggatggacacggcgcctgtcttccagggccactggatcgcaatgtacggattgatcactcccctcaccgccgcgagcggccggcgtgaggagctggccctgacgctgctggaccccgccgcaaaccggcgcggctgtcaccactatgtggtcgccctcggcgcggacggaccggacagcctgtgggtcaccgagatctgggtcagcgaagaggcccatcgcgcctgggtggcggacatcaaggcttcggaagcgctgagaccggcgctcgcgttgatcgccacctggggcgacacggtgatcacccgccccatggccgggatcgggatctagcgcttcactcggcgacctgcacctgcgccagcacggcgccgtcgacgacctgatcgccgacggcgccgaacaggctgaccacgccgtcgaacggcgccaccagcgcgtgctccatcttcatcgcctccagcaccaccacagtctgacccttggccacggcgtctccgtccgagagcggcgcggcgacgatccggccgggcatgggcgcccgcagggcgccgtcggacgccgcccctgacgccgccgccttgacgcggaaaggctccacgcgcctcgcctctccgtcgacgaacagcacgaagtcgtcgccgtcggcctgaaagccgaaaaggcgctcgccgacctgcacctgatcaaagccgacgtgggacgccgatccgtcctgcagccgccagccgttgggcgacggcgcgacctctccctcgatcgcttcgccgtcgagccgggcgcgggtggtcgcgcgcgccggcgcgttgagtcgaagcccgtaggagagacccggctggccgccccatggcgaaccgccgtcgacaggacgcggagcggcgtccagcgccgcctcggcgatcagtgtcagggcggcctcgcgagccgcgccgtcatcgcgcgccgccagagtcgcctcctccacgccgataaagccggtgtccacgtcgccctcgacgaagcgcccatgctccagacagcgcttcaggaaggcggcgttggtgcggacgggccagacctcgacctcgccgcaggcctgcgccagccgctcggccgccgcctcgcgcgtgtcctcgtgcacgatcagcttggcgatcatgggatcgtagaactggctgacctcgccgccctgctccacgccggtgtcgatgcggacgtcgtccggcaggcggaaatgatccaggcggccgatggagggcaggaaggcgttggccggatcctcggcatagaggcgcgcctccatggcccagccgttcagggcgatctgctcctgcttcagcggcagcggctcgccggcggcgacgcggaactgccattccaccagatcgacgcccgtgacgctttctgtcaccggatgctcgacctgcaggcgggtgttcatctccatgaaccagatgcggtccgccttcagcccttccgacgcatcggcgatgaactcgatggtgccggcgccgacatagttcaccgcgcgcgccgccttgatcgcggcgtcggtgacggcggcgcgggtcgcatcgtccatgccgggcgcgggcgcctcttcgatcaccttctggtggcggcgctgcaaggagcagtcgcgttcgaacaggtggacgacctcgccgtggcggtcgccgaacacctgaacctcgatgtggcgcggacgggtgatgtagcgttcgatcagcacccggtcgtcgccgaacgccgccttgccctcgcgctgcgcgctggccaggccctcggcgaagtcctcggggcggtccacccgcttcatgcccttgccgccgccgccggccacggccttgatcaggacggggtagccgatgcgatcggcctcggccgccaggtgggcggcggactggttctcgccctgatagccaggggtgacgggcacaccggcctcgatcatcagctttttggccgcatccttcaggcccatggcgcggatcgaggcgggatccggcccgatccagacgatccccgccgccatgacggcttccgcgaagtcggcgttctcggaaagaaagccgtagccggggtggatggcctcggcgcccgcggcctttgccgccgccagcaccttggccgcgtcgagataggactcgcgcgccggggccgggccgatcaggatcgcctcgtccgcctcgcgcacatgcaaggcgtggacgtccgcttccgaatagacggcgatcgtgcggatccccatgcggcgcgcggtgcggaatactcggcaggcgatctcgcctcgattggcgaccaggacggaggtgaacatcagggggcttcccggaaggcgttgtgtgcgggcggtcttggcgccgcccttgtcgaagggggtgttactggaaccagctgggctgacgcttttcgagaaaggcgcgcacgccctcctggccttccggcgacactcgggcgcgggcgatgcggcgggcggtatcctcgatcaggctggtgtccagcttgtgctcggcgacgtggtggaccagccgcttggcgtcgcccatggcgcccggcgcattgccggccaggctgtcgctcagcatcgagatgaactcgtccatcgaaccttccggcagcaccatgtcgatcaggcccgcatgcgcggcgtagtcggcgtcgaagatgttgccggtcaggaacagctggcgtgcacgacgcgcgcccaccgcctcgacgacatagggggcgatggtcgccgggataaggcccagcttgacctcggaaaaggcgaagcggctgccttcgatggccaccgccatgtcgcaggccgcgacgatgcctgcgccgccgcccatggccgatccctcaaccagggccaccgtgagggccggcacgtcgtgcaggctcttcagcatcttggccagacccatggcgtcatcgcggttgtcgccctcgctccactcggcggcgtcgcgcatccagcccaggtcggcgccggcgctgaaggtcccgcccgcgccgcgcacaaagacgacccgcacattgtcggcgccgtgcagggtgtcgaacgcctcgtgtagggcggcgacggtcgcagcgtcgaaagcgttcttcttgtgcggccggttgatggtgacgaagaccgcgccgtcctcggtcgagtcgatctgcaccagctcgtcgtcggcgtcgggcgcagcccccggcaccagcggctgggcgatggcgttgatctgcgcctcctcggcgtcggtcacgtccagggcgttgagttcggcgtcggtcggaagttcgcggtcggtcatcataggctcctttgctccgaacaacgcgccggaacaggcttgggtcacatccggaagacgccgaaggtcgtgtccgggatcggggcgttcaggctggcgctgatggcgaggcccagcacgtcgcgggtctgggccgggtcgatgatcccgtcgtcccagaggcgggcggtggcgtagtagggattgccctcgtcctcgtacttctggcggatcggggccttgaaggcctcggcgtcctcggcgctccaggtctcggcgtcgcggtggacggtggcgagcacactggcggcctgctcgccgcccatcacgccgatgcggctgttcggccaggtgaacaggaagcgcggcgaataggcccggccgcacatgccatagttgcccgccccgaaactgccgccgatcaggacggtgaacttgggcacctcggcagaggcgacggccgtcaccagcttggcgccgtccttggcgatgccgccggcctcgtacttgccgccgaccatgaagccggagatgttctgcaagaacagcagcgggatcttgcgcttgcaggccagttcgatgaagtgcgcgcccttttgcgcgctttcgccgaacagcacgccgttgttggccaagatggcgaccggatagccccagatgcgggcgaaaccgcacaccagggtcgagccgtacagggccttgaactcgtcgaactccgagccgtcgacgatgcgggcgatgacctcgtgcacgtcgtagggcgcgcgcacgtcctcggggatcagcccgtagagctcggaggggtcgaaggcgggtgcgcggggctcgcgcacgtccatctccaccgtcttggtggtgttcagattggacacgatcgagcggacgatctcgagcgcgtgctcgtcgttctccgcgacatggtcgaccacgcccgagcggcggccgtgggtctctgcgccgcccagctcctcggcggagatgacctcgccggtggcggccttcaccaggggcgggcctgccaggaagatggcgccctggttcctgacgatcaccgtctcgtccgacatggccggcacataggcgccgccggcggtcgacaggcccatgacgcaggcgatctgcgggatgccttgggcgctcatccgcgcctggttgaagaagatgcggccgaaatggtcgcggtcgggaaacacctcggcctggtgcggcaggttggccccgccggaatccaccagatagacgcacggcaggcggttctgctcggcgatctcctgggcgcgcaggtgcttcttcaccgtcatggggaagtaggcgccgcccttcaccgtgggatcgttggcgacgatcatgacctcgcggcccgatacgcggccgatcccggcgatcacacccgcgcccggcgcctcgtcgtcgtacatgccgttcgccgccagttgcccgacctccaggaagggcgagccggggtccagcagccgctcgacccggtcgcgggggaggagcttgccgcgagatacgtgtcggtccctcgccttgtccgatccgccgcgcgccgcctgcgccacgcgcgcgcgcagatcatcgaccaaggcgctgttgtgcgcgtgaagggctttgtactgggggctgtgcggatcgaccgccgaggtcagctttggcatgcggctggtgtaggcgggcggaggaagggcgacaagcgcgcaggcgacggcgggcttccttgcttgtcgaccgcttttcctctaagagcccgcgctttccggggcttcggtcccgatgcggaacgccaaagggcttgggaaatcgtcccggccgccgcttcgggagccatcgtggacgcgacttgcccggtcgccccgcgccgaggtccagcaagggagaccaccgcatggctctttacgagcacacggtcatgacacgccaggacatctcggcgcagcaggccgaagcgctgaacgacaccatcaaggacctgatcacccaaggcggcggctccgtcgccaagatcgagtactggggtctgcgcaacctgacctatcgcgtgaagaagaaccgcaaggctcactattcgctgctcgccgtcgacgcccctccggccgccatggccgaagtcgagcgccaactgtcgatcaacgaagacgtgctgcgctggctgaccgtccgcgtcgaagagctggacctcgagctgtcgccgctgctggcccgccgcgaacgtgaacgcgatcgcgagcgcgaacgcggcccgcgtgaagacgccgccgccgaagccgccgaataaggaaaccggatcatgactgacgccaccccgaccccgggcgctccggtgggctccggcccggcccgtcgccccttctaccgtcgccgcaaggtctgcccgttctcgggcgccaacgcgccgaagatcgactacaaggacgtgaagctgctgcagcgctacgtctccgaacgcggcaagatcgtgccttcgcgcatcaccgccgtctcccagaagaagcagcgcgagctggccaaggccatcaagcgcgcccgctatctggccctcctgccgtacgtggtgaagtaagatgaaggtcgttctgctcgaacgcgtcgagaatctcggcgccatcggcgacgtcgtgtccgtcaaggacggcttcgcccgcaacttccttctgccgcgcgacaaggctcgccgcgcgacgtccgccaacctgaaggcctttgaactcgaccgcgccgccatcgagcagcgcaacgagaagaacaaggccgacgcgcaaaaggtcgccgacaagatcgacggccagacctatgtcatgatccgccaggccggcgaaaccggccagctgtacggatcggtcgccggtcgcgacgtcgccgaagccatccaggccgaaggcggcaaggtcgagcgttcgcaggtcgtgctgaacaccgcgatcaagaccctgggcgtccacgaagtgctggtccgcctgcacgccgaggtccgcgccacggtcaaggtcaacatcgcgcgttcggccgacgaagccgagcgtcaagccaagggcgaggacgtgatccgcagccagttcgacgacgaacgtcaggccgccgaacagtcggcccaggagctgctggaaggcggcgccggccagcaggaaggcttcggcgaccgggagtaatcccgacttaccgacaaggcttgaagagggcgcgtctccctgaggggcgcgccctttttgctgagccaaagacatccacaggctgtcccctgtcatattcggggcacggccgaatccgtccgcgtccgacgcaggatcacgctagacgcctaaggtcatgaacgccttcgctcccctgcccttcagcgcctctccgatggagccggcgccgtccgtcgcctccatgccgcacaacctggaggccgagcaggcgctgctgggctccctgatgttcgacaatgcggtgttcgagcgactgagcgaccggctgcgcggctcgcacatgtatgagccgttccaccagcggctgtatgaggcgatcgaggaccacatccggcagggcatgctggccgaacccaccatcctgatggagcggttcaagcaggacccggcgttccaggagttcggcggcctgcgctacctcgccgacctggtcgaccgcgccccgccggcggccaatgcgcccgactacgcccgcgtggtctacgacctggcgctgcgccgcgacctgatccgcatcggcggcgacatcatcaaggaagcgcccaatcccgagacgcccgccgacgagcagatcgagcaggccgagcagacgctgtattcactggccgagaccggcaagccgtcgtccggcttcgtcgctttttcgcacgccctgtccggcgccgtgcagatggcggccgaggcctatcagcgggacggcaagctggcgggcctggccacgcacctggacgacctggactccaagctgggggggcttcacccgtccgacctgctgatcctcgccgggcggccgtcgatgggcaagacggcgctggcgaccaacatcgccttcaacgtggcccgcaactatcgttgggagccgaccccggaggggcgcaagaccgtctcgggcggcgtggtcgccttctattcgctggaaatgagcgccgaacagctggccatgcgcatcctggccgacgcctcgggggtgtcttcggacaagctgcgcaagggcgagatcaacgcctccgacttcggaaagattcgcgacgcggcggtcgagatcggcgaaagcccgctctacatcgacgccaccggcggcctgtccatctccaagcttgcggcgcgggcgcggcggctgaagcggatggagcacgggctggacctgatcatcgtcgactacctgcagctggtgaccaccggcgagaacagccagaagaaccgggtgcaggaggtgtcggagatcaccggcggcctgaaggcgctggccaaggagctgtcggtgccgatcatcgccctgtcgcagctgtctcgccaggtcgagcagcgggaagacaagcggccgcagctgtccgacctgcgcgaatccggctcgatcgagcaggacgccgactgcgtcatgttcgtctatcgcgagagctactatctcggccgcgccgagccgcgcgagggcaccgaagagcacctgaagtggcaggaggacatggaccggctggagcatcaggccgaggtcgtgatcggcaagcagcgccacggccccatcggcatcgtcaagctggccttcgacgccgacaccaccaagttcggcaacctggcgcacgacggccgctacgacaacgtcccctacgaatgacgctcgcccggcccgcctcgacgctctagaagcgcggcggggacgcagaggggcggtcatgcaggacgatcacgacatgacgacggtggccgtggtcggcgccggcttcagcggcgtgatgacggcggtgcatctgctggccggagcgaacgcgctgcgggtgatcctgatcgaacggcgggcgcggttcgcgcgcggggcggcctatgacaccgacgatgcggcgcaccggctgaacgtgcgcgccgagggcatgagcgcctttccggaccagccggatcacctgctgcgctggcttgaggcgcaaggcctggatcggggcgacggctttgtcggtcgcggcgattacggacgctatctcgaagacgtgctgcgggacgccgcctccgcccatggcgaccggctggtgcggcgaagcggatgggtggtgcgggcctctcgttcggcttcgggcttcgacctggagctggacgacggacagacacttcgagccggggcgctggtgctggccatcggcaatctggagcccggcgccgtgcccggcttccccccggacgtcctcgcctctccggcctatgtgcagaacccgtggggtcgcgcgctggacgcgccggagggcgcctcggaggtgctgctggtcggctcgggcctgaccatggtcgacgtcgcgatctcgctggaccggccgggacggaccatcaccgccctgtcgcgcaacggccgcctgcccctgccccatttggccgaggccgtgccgccggttccgccgcctccgagcggctcacccctcgccatgttccgccagatccggcgggcgagccgggcgggagagtggcggggcgtcttgaacggactgcgcaccacggcggccgggttctggcgcgaatggtcgccggccgagcggcggatttttgtgcgccgcctgcggacgttgtgggacgtgcaccggcaccgattggcgccctcgatctgggcgcggatccagaccatgatggaccagggtcggctgtcggtgctcggcgggcggattctgggtgcacgaccggagagcggcggagtggaggtcgaatggcgcgcccgggcctcgcaggaggtcattcgccgccgcttcgatctggtggtcaactgcaccggtccgctggcgcaggtggagagaagcgccgacccgctgatttcagggctgctggcgcagggcttggccatgccggagccgctgggcctcggcttcgcggtcgagcccgacgggcggctgctgaaccgcgacggcgtcccgcaggatgacctgatcgccgtgggtccgctggcgcgaggccccttctgggagatgacggctgtgcccgacctgcggcttcaggcgcgggacgccgcacgcgccctgctgtctcggctgggcttggctgatgcatcggacgagaggggcgcggcggccggctgagccgcccgctgctccagacgcgcattcagccgccgtatggtggtgctgcccgtccgctcgaacagaaagggcgccacgccgtggatgatgcaggccagcccggcgccgaccagcgtcacgccggtcctggtggcgaacaggagatgccggccgtagctttctccgaccgagcggggatgttcggtgaacaggcggatggcgagaatccctgacaagtgaccagagacaacctaacagcaaaggcgcggcttggctcccgccctgcgtcgccttgaagcgatcgtgatgcaagccgcgcgggtttgcgccataaggcgaccatgcccgcgcccgccgttctgtccgtcgatcttgacgccctcgcccgcaactaccgcacgctggagcggatcacgggcgtgcccgtgacgccggtcgtcaaggccgacggctatggcctgggcgcggcggccgtggcgcggcggctgatggcggagggcgcgcggacgttctttgtcgcccgcatttcggaaggcgtgctgctgcgccaggccatggggcctgagccggtcatctatgtgctggacggctgtcacggcgaaggcgcggcgggcgagttgcgggcggcggacctgcggcccgtgctgaaccagccggcgcagatcacagagtggctggacagcggcggcggcccctcggccttgcagatcgacaccggcatgaaccgcatcggcgtgcgccccgaggacgcgcccgagccgttcgtgggcctggagctggtgatgagccatctcgcctgcgccgacgagcccgagcagcctatgaaccggcgtcagcgcgacatgttcgccgaagcgacgcagcggtatcccggcgtcacgcggtccttcgccaactccggcgggtgcttcctgggaccggacttcgccttcgaccaggtgcggccgggcatctgcctgtatggcggcgggccgacaggacggccggatgcagggatcgcgccggtcgccgccctgctggtcgacatcctgcaggtgcgcgacgtgccggcgggcgagagcgtcggctactcgcgcggctttgtcgccgaccggccgatgcggatcgcgacctgcgccgcaggctatgcggatgggatcctgcgcagctacagtccggaaggactggtgtgggtcggcggcgagatgcggccgatgctggggcgcgtctccatggatgtcatcgccgtggacgtcaccggcctcgacgtcgcggccggtgaccaggtcgaggtgttcggccccaatcggctgctggacgatgcggcgggcgcggcgggcaccatcgcctatgaactgctgaccggcatcatgccccgcgtgccgaggcgctacgcctaggcgccctgcgtccccagctgacgcaacgccacgccatgtgaggcgtctctccgcctgctaagaaggacgcccatggcccgtgattccgccctttatgtctgccagtcctgcggcacggtccacggcaagtggtcgggccagtgcgggtcgtgcggacagtggaacaccctggccgaggaaagccgcagcgccccgcccggcgcgatcaagcccgccgccgcttcctccgcgcgcgggcgaggcgttcagttcgagacgctgcaatccgacgcacccgagccgccgcgcatcatcaccggcgtggccgagttcgaccgggtgtgcggcggcggcgtggtgcccggatcggccatcctgctgtccggcgacccgggcgtcggcaagtccaccctgctgctggaggtgacggccaaggcggcgatgcggggcgcgcgcgtcgcctacatctccggcgaagaggcggtggagcagatccgcgcgcgggccaagcggatgggtctggcggacgcgccggtgaacctggcggccgcgacggcgctgcgcgagattctgtcgaccctgaagcgcgaaagcttcgacatcgtcatcgtcgattcggtgcaaaccctgtggtcggacgtgcacgacagcggaccaggatcgatcacccaggtccgggcctgcgcaggcgaactggtgcggctggccaagaccggcggcccggccgtggtgctggtcggccacgtcaccaaggacggccaggtcgccggcccccgcgtggtcgagcacatggtcgatgcggtgatgacgttcgagggcgagcgcggctatccgttccgcatcctgcgcgccggcaagaaccgcttcggcgccaccgacgagatcggcgtgttcgagatgggcgacagcggtctgcgcgaggtcgccaacccgtcagccctgttcctgggcgagggcaaggagcgccagccgggcgccgccgtgttcgccggcatcgaggggtcgcgtccggtgctggtcgagatgcaggcgctggtggcgccctcggcctatggcacgccccgccgcgcggtggtcggctgggacaacgggcggctggccatgctgctggcggtgctggaggcgcgctgcggtctcgggttcggcgacaaggacgtctatctgaacgtggcgggtggccttcgtatcaacgagccggccgccgacctcgccgccgccgccgccctgatcagttcggccaccgacatgcccctgccccagggctgcgtggtgttcggcgagatcggcctgtcgggcgaggtgcgcagcgtcggccgcgccgaggcccgtctgcgcgaggcgaccaagctgggcttcgaccaggccctgtgccccgccttgccggcaaaggccaagggggtgaaggcgaccaccctgtcgcggctgacggaagcggtcgaacgaatctcggcgaaccgctattagggtcaggccacagctacaggaccgcagccgaacgtgaccggatacgacgtcttcgccattctggtcatcctcgcctcggcgggcgcgggcttcgtgcgcggaggcgtgcgcgaggtcatcaccctgctgagcgcaatgctggcggcgtttgtggccctgatcgtcctgccgtggacggcgccgatcggccgggcgctggtgaacccagactgggccggatcgatcctggccgccgtgggcggtttccttatcgtctacttcggattgaggacactgggcgcggttctgtccaagggcgcaaaggcccatccggcgctgggcggcgtgaacagcatcctggggctgatcgtcggggccatccgggcgctggtgctgatcggcgcggtgcatctggtgatcgtcgccgccctgccaggcgagcgcacgccgcgctggctgtcacaggccgcgcttcagcctgtcagcgccatggctgcgcgcgccatccaggccggcctgcccggcatcggccggggcgccgatgcgctgtcgccggtgatcgactcttccgtgcgaagaggattctcggacgcagacgccttgtccgcgccccaaactcagcctacctcgccgcctgaagccccctgacatccgtatgcacatcggagcccatacgatgcgccacctgatcgccgatcccgtcgttcaccgcgagcactatcgcgaggccgacgacgaccagctgcggctggagtgcggcgtgtgcggcgtctggggcgcggaggcggacgaaggctcctccatcgtggccctgggcctgcacgccttgcagcatcggggccaggaagcctgcggcatagccagcgtcaaggacagccgcttctacaccgaacgtcaccaggggctggttggcgatgcgttcggcggcgcggacctgtcgcagcgcatgccgggcggcgcggcggtgggccacacccgctattcgacctcgggcggatcgttcctgcgcaacattcagccgatgttcgccgatctggaccagggcggcatcgccatcacccacaacggcaacctgaccaacttcaaatacctgcacagccagctggtcagcgaaggcgccatcttccagtcgacatccgactccgaagtcatcctccacctgatcgcacgcagccggaaggccaagatcgtggaccggttcatcgacgccctggcgcggatcgagggcggctatgccttggtcgcccagacgcgcagcaagatgatcggcgcgcgcgatccgctgggcatccgcccgctggtgctgggcaaggtgggcgacgcctgggtgctggcgtccgagacctgcgccctggacatgatcggggccgccttcgtgcgcgacatcgagcatggcgaagtggtggtcatcgacgaaagcggcctgcagtcgatcaagcccttcccggcccgctcggcccggccctgcctgttcgaatacgtctatttctcccgccccgactcggtcgtgaacggccgctcggtctatgaagtccgtaaggcgatgggccggggcctggcgcgtgaacacgcggtcgaggccgacatcgtggtgccggtgcccgactcgggcgtgccggcggcgctgggttatgcccaggaaagcggcatcccctatgaaatggggatcatccgcagccactatctgggccgtacgttcattcagcccagccaaggcgcgcggcagaagggcgtgcgcatgaagcacagccctaacaaggcggcgctggcgggcaagcgcgtggtgctgatcgacgactccatcgtgcgcggcaccacctcggtcaagctggtccgagcggtgcgggcggcgggggccgccgaggtgcatctgcgttcggccagcccgcagatcctgtatcccgacttctacggcatcgacatgcctgagcgcgcgcagctgatcgccgccaacaagacgctggaggagatgcgcgagatgctggaggtcgattcgctgggcttcctgtcgatcgatggcctctatcgcgccatgggcgaggacggccgcaacaccgccgatccccagttcaccgaccactatttcaccggcgaataccccacccgcctgctggaccgcgagatcgaggaaggcggacgccaagtgacggcgcgccagctgtccctgctggtcagcgcctgatccacaccgccgcccgcgcgcgcgcgcttggacagcgtgtgaggtcccgctaagacacacggcatgtccagcgccgcttcgcccccgtccgctctcctgtccggccgcatcgcgctggtggtcggggcctcgcgcggcatcggctatgagagcgcgctggccctggcgaaggcgggcgcccacgtcgtggcgacggcccggacgcagggcggactggaagagctggacgacgccatcctcgccgcgaccggcgaccgcgccaccctggttccgttcgatctggtggacggcggcggcatcgaccggctgggcggcgccctgttcgagcgtttcggtcgactggacgtctgggtgcaggcggcggcgaccatgggaccgtccggcctgacgcccgtggcccacgccgacccgcgcgagttcgccaaggtcgagaagaccaacttcaccgccgtctatcgcctgatccgctcgctggagcccttgctgcgcgcctcggacgccggtcgcgccattcacctgaccagcagcgtcgcgacgaaaccccgagctttctggggcatgtacgccgcgaccaaggcgggcgccgaagccctgttcaaggcctgggcggacgaggtggagtccacgcccattcgttgcaccatcgtcgatccgggccgcatgcgcacccagatgcgggctcaggccttccccggcgaagatccgacgacgctgccgcatccgtcggagatcggtccgatgatcgtcgagctggcgcgcggcgatcgcacaccgccgctggaactttccttccgcgactggcgctctggtcttcccgccgaggcgcttgtgtgagccacggcggtcgcgcaaccgcttcaactcagtaactctgaacacccgggatgagggctgatcatccgcgggaccgggatcgacgcatgacgacaagcagggacggcacggcgcctggggggcctccccctcacaacgatcagtcgcgcgacaccgcgatgaccgaccagcacaacagcatcttcttcgcggccgtgaagacgacccgcatgccgatgatcgtcaccgatccccgccagcccgacaacccgatcgtgttcgcgaaccccgccttcatcaacatgacgggctacggcgaggacgagctgctggggcgcaactgccgcttccttcagggcccggacaccgatcccgagacggtggccgaggttcggcgtgcgctggagcagaagcgcgaggtgtcggtcgacattctgaactacaagaagaacggcgccagcttctggaacgccctcttcatctcgcctgtctatgatgaggccggcgaggtcatctacttcttcgcctcccagctggacatcagccgtcgccgtgacgccgaggacagcctgcggcaggcgcagaagatggaggccgtgggccagctcaccggcggcatcgcgcacgacttcaacaacctcctgaccgtgatccagggtttcaccgacatcctgcacgcacagcttcgcgaagaggcgggcgtcgacccagccaaggcgagacgcgcggtgaacgccatcagccaggcggcggagcgcggcagcgcgctgacccaacagctgctggccttcgcccgcaagcagaagctgcagagacgcgtagtcaacctgaacgaactggtcaccaaccttgagccgctgatcgagcagacaagcgccggccgcgtccagatcgagacccggctgagccaggacatctgcaacgcccgcgtcgatccggttcaggccgaaatggccttgatgaacctgctgatcaatgcgcgcgacgccatgcccgagggcggcgtcatccacatcgagagccgcatctgcgaggtcggcgaggaggatcagggcgagttgaagccgggctcatacgccgaactggccgtgcgggaccatggcttcggcatgagtccggaggtcctgcagcgcgtcgtcgaacccttcttcaccaccaaggagcaaggcaaggccaccgggctcggcctgtccatggtctatggctttgtgcgccagtcgggtggtgcgttgctgatcgagtcgaagcccgatcaaggcacggtcgcgcggatgctgttcccctgcgacgcggctgacaccgacgccgctaggtcggtcccgcaggttcagggcgcccgggctcgcggcgaaaccgttctggtggtcgaggatcagatcgacgtgggcgactacgcccaggcggttcttgaggagttcggctaccgcgtgctgcgcgccgacgagggccgcggcgccctggacatcctggaccgggaacagtcgatcgacttgctgttcaccgacctgatcatgccgggcgcgatgaacggcgtgctgctggcgcgagaggcgcgccggcgtcggccgcgcatcaaggtgctgctgaccaccggctacgccgaagcctccatcgagcgggtcgatgcgcgcggggccgagttcgagctgatcagcaagccgtaccgccgcaccgaactggccgccaaggtgcgccaggtgatcgaggggccgaccggggtcggctgacgggctctacttcttcggcccgctcttctggccggtgcggatgcgacccgagcggctgacctggcgggcgccgccgcgcgcgcccttgccgatcgccacgctggttcccgccttcttggacgaggacgccttgcccgcgccgatgacacggggcttggcgacgcgcgcctttttctgctccagcgccttgccgggcagattggacagctgctcctgcttctcggccttcagcaccttgcgcggggcggttttggccgcacccttgaaccgctccggcccagacttggcgccgccgccgacataggggttctcgctgccggacttgaccgtcaggcggatgggcgtgcccggcaggtcgaagctctcgcggatcgagttgaccagatagcgcttgtagtggtccggcatggccgaggcgcggctggccatcagcacgaacgttggcggacgggccttggtctgggcgatgtatttgggcttgatgcgcttgccgtccaccgcgggcggcgggtgccgctgggtggccagcgacagccagtcgttgaggtccttggtcttcaccttgacggaccaggtgtcataggcctgcagcaccgccggcatcagccgctcgacgccgcgtccgctgtgcgccgacagggcgacaaagggcgagcccttcagctgcggcagcttgtcctcggccaggcgcttcagctcggccaggcgcgcctgcggctcctcctccaggtcccatttggaggccacatagatcagggcgcggccttcgcgctcgaccagatcggccagctgcaggtcctgggtgtcgaaggcgtcgtccttgtccatcaccaggatcaccacctcggcgaaggtgatggcgcggatggtgtcggcgacggacagcttctccagcttctcctgcacccgcgccttgcgccgcatgccggcggtgtcgaccaggcggatgttcctgtcttcatagacccagtcgaccgagatggagtcgcgggtaatgccggcctccggtccggtcagcaggcggtcttcgcccaggaggcggttgatcagcgtcgacttgccggcgttggggcggccgatcacggcgatgcggatcggcttttccggctcgtcctcttcctcgatgaagatgtcggccgaggcggccaggatcgcctggtagaggtcggccatgccctcgccgtgctcggccgagatggcgacgggctctccgaagcccagggcgtgcgcctcgcccaccccaccgccggaggcctggctttccgacttgttggccaggagaaccaccggcttgtgctgcttgcgcagtcggtcggcgaagatgcggtccagcgaggtcacgccctcgcgcgcgtccatcatgaacaggatcagttcggcgtcttccagcgcggcctcggtctgctcgcgcatgcgggcctcgaggctttcgtcggtgacgtcctcgtagccggccgtgtcgatcagcgtcaggtccatgtcgccgatcacgccatccgcatagcgacggtcgcgggtcacgccggggcgatcgtcgaccagcgccaggcgcttgccgacaaggcgattgaacagggtcgacttgcccacattggggcggccgacgatggcgaccttcagagccatgccggccttctagcttagtttcagccgctcgtcagcgaatgcagacgagttcgccccgatctgtcacgacatagagcgcgccgttgtaggccgacggcgcgatataggcaggcgcgcccaggtccagacgcgcctgctcggcgcccgtcttgggatcaaacgccaccgcctcgccgaacgagttgaccatcaccagacggttggacgccagcatcggcccggaccaggtggggcgcacctggcggtcaaagaagcccaggaagccgccctcgttgcgctcacgcccttcgttcagttcgcgcgtccagtagatctggccagaatcccggttggcgacgatcagctggccgctcttggacacggcgtagaccacatcgcccaccggcagcggcgcgttgacgccggtgaccggcagctgccacttcggctggcccgagcgcaggtccagcgccgacagcacgcccgagtggctgacgccatagatcacgccgcggctgatgaccgggcggccggccacgtcacgcacttcggaaagggcgctggtgcggctggtccgcgacagcacctgctgccacacggcctggccgttggcggcgcgcaccgccaccagctcaccggacgagaagggcgcgatcaccgtgtcgccgctgaccgcaggactggaggcgcgcatgatccgcgccggctcggcgatgccgcgataggcccaggcctgggcgccggtgttcacgtcaaaggcgaacagctggctgtccacgtcgatggcgtagacgcgattaccgacaacggtgggcgcgccgtggatcggcgaatcgaccgtggtgcgccacagcaccgcgccggtgttggcgtccagcgccgtcatgacgcgatagcccgacgagacgaacaccttgccgccggcataggccacgccgccgccgaagccgccgcgcgccaggccttccggcttgatgtcggtgcgccacaggatgtcgccgctgtcggcggacacggccgcaaccgtggagtcgccgtccagggtgaacagcttgccgtcggaggcgacgaccggcgccatcagcgtgccgggcacctgcgatccctcgccgatgctgcggcgccaggccacctggaagttcggcgcggcgatggcgtgctcgaccaggttctccggcgtgccgcccggctgggtccaggcgttcacggcctgcgggcccggcaggaagaagtcacggcccgacagggcggcggacggcgccagctgctgctcgaactccagcaccgagatgcgctggccttcggtggcggtggcggcgggctcgtcgcttcggcccaggccgaacggcaggttgcggcgcaccgtgccgcatgaggccagggtgacggccacgccgcagaccagcgcgaccttgagggctcgggaagtcatcgagggcgtcctgtcggtgatcgtcactgttgcggcgcggcggccggagcgacctgcacgggcgccgccggagcttgagcggcctgaccgggagcggcctgaccctgggtgggctgaccttgggcaccctggggctgcgccgtgggtgcaggcgcggcggcggcggccttgacgatggcgggcagcgcgccggcggttccggcgtcgatcatggcgatggcggcctgggcgcgctggcgcaccggctccggcacgtcctggccgagctgcagctgcacaaaggcggtgcgcgcctcggcggtcttgccgttctggagccgcgccatggccagcgcttcctgggcgaaggcgcgcaaggggcggtcgtcgccggtcagcggctccagccgcccttcgacgtcggccaaggacgccgtgtccatggccaggaaggcggccttgagcgcggcgggatcggacaggatcgggtcgcgcgaggccttggccgcctcgtcgaacagacgaatggcttcgggaatgttgttggcggtgacggcgaggccggcctgctgctgcaaggccagcgacttgtaggcgccgttgccttcgcgcgcggcctcttcgaacgccgtgcgggcgccagccgggttctcggcgcgcagcgcctccatgccgcggtcataggcggccgaggccttgtcggccttgcccgtctggaagctctgccagccccaccaggccagcgccgcgatcagggccagcagcaagagaccggcgacgatcggaccccaggtgcggaacagccgcttgtagcggtcggagcgaagctccccctcgacctgctcgaagacatcaaccacgagaaacgcgccccaaaacctgaaaggatcgaaccggcgcggaccctagagggtcggccccgacgccgcaacgcaagcgctacggcgaagccggctttttggagaagtaggtttcgacttcggcaggaaaacggcggcccttcacatcggccgcatagccggcgacggcgcggtcgatctcgccccgcagatccgcgtatttgcgcacgaacttgggcgtccagtcgaacaggcccagcatgtccggcgtgaccagtatctgtccgtcgcaggcggccgaggcgccgatgccgactgtgggaacggacacggcctcggtgatctcgcgcgccagtccttcggccacgccctcgatgacgatggagaaggcgccggcgtcggcggtcgcctgcgcctcggcgatgaccctctgacgctcctcctcggtgcgccccttggccttgaaggctccgtcggtcagcaccgcctggggtcgcaggccgacgtggcccatcaccggaatgccgcgctggaccagataggcgatggtctcgggcaccgtggggccgctttccagcttcacagcctgggcgccggtctccttcatcatccgggcgcagttctcgtaggcgatctcccgaccgccctcgtaggagccgaagggcatgtcgaccacgaccatggctcgtcgcgcgccgcgcatcaccgcctggccgtgaaggatcatcatctccatggtcacgccgacggtgttgggcaggccgtgcaccaccatgcccacgctgtcgccgaccagcagcaggtcgcaatgcgcgtccagcagggccgccgtcggcgcgtcataggcggtcaggcagacgatgggctcccccccttttcgcgcctggatgtcgggggcggcgatgcgacggaccgtctgctgaacctggctggacacgcgttcactcctggaggcgagccgctcagataggcgggtccgcccccgacgtcacgccccctagaggtcctgagacaggcgaaccgcgccggcggccaggagcgcgaacagagcgccggcggtgatccagaacatctgcatgccgcccgtactcatcagatcgatggacgacaggcccagactgtccaggcccgactgcaccgccccctgagccgtgacgccggccgcctgaaccccttgcgtcagggcggtggtgtcggtctcggcgccgctgaagttcaggttgacgctttcgcgcaccgccacgcacccgcccactatcccggccagggtcagggcgaaggctctcacccgcgaagagcgcgtcagccgcgtctccacctgggcggcgaacagttctgcatccagcatcggggtctgtcgcgcgaacaggcgctcgatggcggggtcgaattcatcagccgacatgcgccgacctcccgactgcgtccggccgcggatcgagccgcgcgcggagtttatccagaccacgtttgacatgagacttcaccgttccgagcggcagattgatggcggaggcgatttccgggtgactgaggcccgcgccatggcacagggagacgcacaggcgttcgacctcgctcagcgccttcaacgcttcgtccaggtccatcaaccccgcggtgtctgaggcaggcgccgcatcctccgtctcgacctcggcgacatagcgcgcctcgtgcgcccgccgcttcaggtaaaggcgcgccgcgatccgcttgacccaacccacgaagggtccctccgcccggaactctccgcacctttgaaaggcctgaagaaaggcgtcctgtgcgatgtcgtcggccacggacgcctcggcccccatccggcgcaagaggccgcgaaccgccgagccgtggcgccgcgccagttctccgaactcgcgcctgccgcccgccgccgcctgggcggcgagctcgttgtcgtgcaggttccgcaacggctgtttcatgacggtcccctcccccggcccgccgctcagtccttgttcttattgaagaagctcaggacgatgaaggcgacaccgatggtgatgggcaggcaggcgatgcccagcaggccgccgtcgaagccgcggttccagccgccattcaggtcgctgaccaaggaaaacgccgcgaggccgacgcccgtcgccagccacagcacgccccggcgcagatcccgcgtccgcgacggcaggctgcgctgaacgtcctttgtcatggcgtcgaccagttcggccggcaggggctggcccttgtcgatcgcggaccgcaccgtcagctgcatctccttcttttcgcggctctttagatagctggggccgacgacgatggcggtgatggtgccgaagacggcgaagatggcgaagatcggaatgaaatcttccacgataataccccttgtgatgccttacggcccagcttgctgccgaggccttctgatcacaagaggcggccaggtgcgcccgtggatgcgtggccggaggtgaaactttcgtaaggcgccgcttgtggcctcagacgccgagcgcctcggcgtagcgctcgggcttgaagccgaccagtcgtcgatcgccgaggtcaagtacaggtcgtttgatcatcgacggctgggccagcatcagggccacagccttgctgggatccaggctggtgcgcgccttctccggcagcttgcgaaaggtcgtgcccgctcggttcagcaccgtctcccatccgtgctcgtccacccaccgccctagcgccgccgggtccacgccctccttcttgtagtcgtggaagacatgggtgacgccgtgctgctcgagccagacacgcgcctttttcaccgtgtcgcagttgggaatgccgtagaggcgcagggtcgtcgtgacggtctggagcatgggcggttctatgccgccggcgcacggcccgcgccagagcccgcagcctggttcgtccacggctcagctggcaacggccccttaaggcttgcgctctaatctcggcgcgaaacgacacgtccggagccgtctgcgaagtaggcctcgccattgggaatgggccatgccgcaccgagttgtccatgcgtaagcgatcaagacagcggatcgccgcttgcgtctctccaaggcgtcgcctcggagacctggttcaggatacccggggcaacatcgccctgaagttcgccctgctcggccccgtggtggccttgatcgccatcggcgccatcgatgtggcgagtgtccattcggcggacagccgcttgcaggatcccgccgatgcgtcggcgctggccggcgctacggagctgtcgctggcgatcgacggcgcggcggccgtgcagcgggcgaacgccatggttgacgccggactcgccgaatggccccaggcgccgcgcgtggagaaggccatcaccgtctccgaggacggggggcagcgcatccttcaggtgcatctgaagggcaaccgcacctcctttttcgtcaacatgctgccgcccggaggatggaacttcgatgcgatggcgcgggggtcgtcggtcagccgcacgcccctgtgcgtgctggggttcaacgagaccgactccgccgtgatccgggtcaaggacagcggccgcatccaggcgccggcctgcctggtgcactccaaccgcgacatcctggtcgagggcggcaacatcaacgcctcggccgtacaggcggtgcgaagcgcgcgcggcagcatctttcccgtcgccggcaccggcgcggcggtcatccccgatccattcgacaagttggatctcaacaagggcaagctctgcagcacccccgtgccccgtctcttcccgttcggctcccacaccctgtcgcccggcgtccactgcggcggcgtgatggttttaggcagcgccaagctgaccttgaagccgggagagcactggttcctgggtgggcacctggaggtgaaagaggacgcacgacttgaggggacggacgtcgtgctgatgttcgacaaggcgtccaagttcgacttcaaggaccgtgcgcaggtcaacctgaacggtcgtcaaagcggaacctgggccggcatggtgatgatcgggatgcgcgacaacacccaggacttcatcatctcggccgacaatgtcgacaccctgcagggcgtcatctacgtgccgcgcgccaagctgatcgtggagggcaagtccgaggtggcaagggacacgccctggaccgtgatcgtggcccgggcgttggagctgaagggatcggcgtcgctgttcatcaacgccaactaccactactcgaacgtgccggtgcctgtcggcgtcggcccctccaccgggccggtccagctggtcgactagcttaaggctacgcgtctagaaccgtcggctgacgcccatcgtcaccacccgtcctcgcgggtcagcgacgacgggatcgtatcccagggcgaattgggcgagcggcggatcgcggtcgatgaggttcaccacgccaagactcaccgtcacgtcggcggaaaggtcgcggctcgcggccacatcgaaggtggtctgggagccgatgcgcgcgtccgtgatcccgctccggtcgttgcggtaggcggaggtgtggtgcgccagtgcgctcgccgaccaaggtccgcgcgtccacgtcgcgacgaactcgccgcgattgcgcggcagcgaccgcccgatggtgttcaggttggtggagcccacgcctgatgtcgccgcagcgccgggcgccagccgaatgtcgtagcggtcgacataggtccagttcgccgagacgcccagccgaccgatgcgggtgtcgcgctcgtagcgagcggcgaaatccagcccatcggtctcgatagaggaggcgttgacgaagttcagggcgacaaaggtcagggttcctgccgtgtcgcgccgcacgcgagtctgggcgtccgtgccgacttggccggcgcggtcgtccgccgccgcctgatcgatcaggctctgcgccgcctccttgaccaccaggttctcgtattcgaaccgccaggcgtccagcgacagctgcagcccgtccagcgggcgccaggccacgcccaggctccagttctcggagtcctccggctcgaggtccggatcgccgtaggtgacagtgttgacgaagacaaagcccccccgatccagaacggacggctgcgacgcctgcgccccctgtcgcacatagacggacggcgagcggaagccctgggcataggcggcgcgcagcgtcagcgcatcgaccggggtccaggccgcggcggccttggggctgaggcgatctgcgccgccctcgctctcgtagcgggcggcgagttgggcctcgaaacgcgcgcccaggcgcaggcgcccttcggcgaacaccgcgccggcgttttcatgccccttgaagtcgggcgacacgccggcggtcagaagttcgccggcgttggccaggtcgctccagtcctgccgatagccgctgcggcgcgcctgagcgcccacggccacctccagcgacccgccgttccaccgggcggcctcgccgctggtcaaggcgtccgccgtccagaggctggccgaacctctcaggccggtatagccggtcagactgtcgatcagcgccccgtcattggccgtgcccgtcccgagataggcgctgccgaaggggttgaagtagcggcaggccccgacgccgggcgcgcctgtggccgcgtcgcatccagccccgcccagcccgttcagcgcgttctgcagcgccgagccgatcacgtccggcttgttgtagaacaccgtctggcggctgaaggtcgaggccaggctccagctccagccgttttcgaaggcgccgtccagagcgcccgcgatgcgacgcgtgtcatagtcgaacaccgcgctggaggcccccgcctccgcgcccagcagccgtccgcggaacagcacgtcttctccgaaggggttgtccggatggctggccggcacgaccagcgatcgcgcgaggatgggaagagacggcgactgccgcacccaggtctggttgcgcgaccaaccggcctcgagcgacaggtccacgtcatcggcgagcggccggcgccaggtcgcgaaaagctgcgttcggtcctcctcgggcgccaggtcgaagaagtccgaatagtcgaggcggcagaaggtgtccgtcgggccggtgcgataggccgagccgaaggccggatcgtcacaatccggatcgggcgcgaaaccgcccgcgttgggccggaagtaggaccccggctggccatagctggtcaccgccgtccatggcgccaggccgtaggtctccgcctgggtgaaatggcgatcgtccgatcctagcgaagagcgatggtagaacgaccccgccagcaccagcggcccgcccagcacctcgcccccgccgatcgcctccagcgccgtctcgtccgatccatcggcggcggcgtagcggacgcggacctccgggcgatccacgctctggcgcgtcacgaagttgaccacgccggccaccgcgtcggagccgtaggtggccgaggcgccgtccttcagcacgtccacccgctgcagggcgatcagcgggaccagcgagttgatgtccacgaacgaggagccgtcggttgccgtcacggcgctggcggtctgacgccgtccgttgagcaggaccagggtcgagccgagccccaggttgcgcaggttgaactgcgccgtgcccgagctctgcggctggttcagctgatcgacctgggcttccgagcccgagttggccgacaccagccgcaccaggcccgatgcgtccaggacgccggccgtctcgaccgtggtacgtcgcaccgtctccaccggcgtggcggcgttgacgcctcggatgagcgagccggtgaccaccacatcgtccagcgccgcggctcggtcctgcgccagcgacacgtcggggaccgccgatagcgaagcggcggctccaagtaggagggcgcgcaaggtcatgttcaggctcgggcgattcaagggacgagccttctagcacccagcttgaaacgtagaaagtcgtttcaaggaggaagcccgggacccttgccgaggttgtgcgttccgcaagactcacccagcccatggacgcctatgccgcaagccgaccaggatgaaccggaaaaccttggatcgctgctggacaagctcgaccgggcggccgagggcaaggacaaggtgcggctgggggacgtgcacgaggcgatcggagagcgcgcctttggtccgatgctactggtcaccggcctcgcggcgctgacgccgctcggcgtcatccccggcttgccgacggccttcgcggtcgtggtggtgctgatcgccggtcagatcgtcatagggcgcgaccggttctggattcctggaaaactgcgcgaccgccggatcggggctgaccgactaaccaaggcggtgcgctgggcccgaaagcccgcgcgcgtcgtcgaccggatcgtgcggcctcggctttcggtcttcaccaaagccggcttcacgcgagcggtcgccttgatctgcgtggtcatcgccttcgccattcctcccctcgagcttctgcccttcgccgtgatcgcgccggcttccgccatcacggccttcggactgggcctgacggcgcgagacgggctgctggtcttgatcgcgctgatcgccagcgccatcagcctcggcctgctgacgctggcgttgtttcactgaatccgctgatcccccaaggagaaccgatcatggccaagccccccaagaccccgccgccggcgccgatccggccgcgagcatccgagatctcgccgacgacggacaaggcgtcctcgccgtcgcccgagacgcaggaggcgagcccgccctctccgctcggcgccgacgccgtgcgggtggaggccaaagccggtcccgcatcgctgaagatcgaggtcaaccacacgccggcggggctgctggctctgagcgcctgcgtcacctccatcctgctgggcgccgccgccattgtctggatctcgacgggtcccgcccgccagcacccgatcgccaccgcctggaccctgcgccgcaagtcctgagcgggcgcggcctggatcaggtcgccggcgcatcgccgcgctggcccggggtgatgacaaaggcgaccaggcgaccgagcccgtcgaccagggcgtgcagcttggtggtcggcccgccgcgcgagcgacctatgccgttggctgaagccccccttttccgcccgtcgccgagcggtgtgccttggcccaggtcgagtccagcatcagctcggcgggcggcccgccggtggccgccagttcctcgaacgcccgccgccagacccccgccttggcccagcggacccagcgattgtagagcgtcttcctgggtccatagaccgccggcgcgtcgatccagcggccgccgctgatcagcacatgaatgatcccgagatcacccgccggtcatccacccgcgccacgcctcgaggcttgttcggcagcagcggtcgcaaccgctcaaactgcgcgtcagtcagccagaactccgaagccatgtcggttctcccgcatccgactgcaggaaatcacgcttcggccaatcagggaatcccgtttatgggtccagaccctagggcgggccctcgaaatccaaccggatcgcgaggacaccaagacgaagcttgccgaactggatggccgcgccgagcagcccgcactgcaaatctccaacatcccgtctgacgcggcagctcagaagagcttccgggtcgtgccgctagacggcagaaatgagcaagatcgggaccgcacgccgatgccgctcatgcttagctattctcgctgaaactggagagcggtcatgactagggcgaggctggagctatgggagaggcggcttggacaggctgcagcgctgctggggcagcgccttgacgatccgccaagcctggccgagctggcgagcgccgccgccgtgtcgccgtttcacttccaccgcgtttggcgcgccatgacgggtgagaccgtgggtcaatccatcgcccggctaaggatggatgcggccaaagaagcactcgcaggcgaagacagaatcacaaaggtcgccatggccaccaggtcagcccgcctgtcagatcacgacgtcagagcttgccttcgcccagcagttcgcgcgtgcgcttgagtgtcgacagaagcgcggccttatatctgatcctccctcggtttggtggacacccatgctagcttttcggagctggagaggagtgtctgatgagtgttcaacgccggaactttccggattctttcaagcgcgaggccgttgaccgcgtcgccaacggcggcctgagcgtcggggcggtggcccgcgagcttgggctgcacgagacggtgcttcgtcgatggatgacgcagttcggggtgcaggcgacgggggcgtcgcggcgccccacaacgcaggcgtcgtccccgtcgccgtcggatctggcggcggaggtggcccggttgcggcgagagaacggtcagctgcggatggagcgggacatcctaaaaaaagccgcgctcatcttcggagcggcctcccgatgaagttcgggttcgtcgatgagcatcgtcaggtctggccggttcgcgtgatgtgcgcggtcctgggcttgtcggccagcggttactacgcctggcgcggtcgccccgagagccagcggtctgtcgccaatcgcgagctgaccgaggatatccggctgatccatgcggagagcagcggctgttacggctcgccgcgcgttcacgccaccctgcggcggcatgggcgtcgggtcggtcgatcccgcgtggagcggctgatgcgccgcgccggcctgcggggcttggcggccttgccgcgtcgcgcccggacgacgaacagccgccacggttatcccatcgcgcccaacaggctggcccggaacttcgaggcggcggcgcccaaccaggtctggctcgccgacctcacctacatcccgaccggcgaaggctggctctatctcgccgccatcctcgacctgcacacccgcaagatcgtgggctggtccatgcgccagaccctgcacaccgagatcgccctcgacgccctcaacatggccgtcgaacgtcagcgccccgcgcccggcctgatccatcattcggaccggggcatccaatacgcagccgaagcctatcgatcagccctggcccgatccggcatcaccccgtcgatgagccgaaagggcgactgctgggacaatgccccgatggagagcttcttccacaccctcaagaccgaacgcgttcatcaccgcgtctacgccacccgagaccaggcgcggcgagacctgttcggatacatcgagggcttctacaatccccatcgcctgcactcagcactgggctatatcagccccgctgaggccgagcgcaaagcggcttaaccccgtccacttttacgggggaagatcaccacgacgagttcgtgctgctcgtaccaaaccagcaggccacatccttacttcttggtgaagccgtcgaccacgccttcccgatgctggcgaccgcgctcatacaggttcgacgtcatgccgatgtagagtacgccgagcgggcggctggcttggatgtaggtcgcgatgaagggccgccgctcgctcatatagccgaggttgatgatggcccgatcctcgggtcaagcccgaggatgacggaagtcaggccttagtcctgatccgctcgcctcttccgtccccacctcgacctgggcgtttcaccattcgccttggccgtgatttccttgagcttgcggccctgcatggccgacaacgcctggccgggtgctcccttttccgggtcgccgaaggcgcggccgtaggtcttcacccgctcctcgaccgaacctaggaactcgccctcccattcggacaaggaaacgcccgccttctcggccgagcggcgggcgcggttcagggcgttgagcgccgaccgctgggcggccttgcgctgggcttcataggggctcggcggcggctttcgcttcaagccgcccgcctcagacctcgccgagggccgacagatagaggtcgaggatcgcctcttcctcctggcgcttggccttgtcctgcttgcggatgcggatgaccttgcgcaggaccttgacgtcgtagccctcgcccttcgcctcggcgaagacctccttcatgtcggtcatgacggcctgcttgtcctcttcgagccgctcaagccgctcgatgatggtgcgcaggcggccctgcgccgtggcggtcaggacgtcaggattggcgtcaaaggcggcgtcgtcagccatggcggtactctcggcaaatcaggggcggacgctaaccatgccggcgggcgttcctcaacctgcgaacacgaaaaaggccgcggacagagtccgcgacctgtggatcgtaaggatcttgggtgcgctatcgcctgtcggctacatgagcgcagcgtccctccggggacgccgatcctcagccctgcttggccttgaagcgcgggtcggtcttgttgatgacatagacccggcccttgcggcgcacgaccttgcagtcgcggtgacgggtcttcagagacttgagcgagctgcggaccttcatggtcggtgtgtcctgaagcgaaaccaatagaaaagccgcaggtccggcaggaccgcggcggaggcggtgcgtatagagacagccgcccgatccgtcaaccgcggcaaggctttttgtccgcccgccgcgtgccgaagagccgctctgttctggaggcctggcctccgagtcgaacggagggtttgcggggttgcacgcccgccgcgtcgccactccgccaccaggccgtgtcagaagcgagtgcggtcatacgtcgcagggcgttaaggaagcaaggtcgcaagagggttaatgcgttcggtcgatcgcggaggaacggcaacggttcggcggctcgcacgcttccttcgcggggttgtgatccccgtagtcgagcccggactgtatcttgcccctcatgcgtttgtcccttcgtcttctgctggtcggcacggtcgcggcgtgcgcgcccatgctgcccgagccgcccctgccgcagattccgccacagaccgcgcctgcggaccagaccccggcgcctgctcccgccccgcaggcgccgccggaccaatcctacgaccagagcggcttcgaaggatggaagcagggcttcctggcgcggcacggcggcgcccggcgcgccgcctatgagcgggaactggcgggcctgtccccggacgcaacggtgatccggctggaccgcaaccagcccgaattctccaagccggcgggcgcctacgtcgccaacgccgtatcggcgacccgcatcgcccaggcgcgccagcgcgtggaccgcgtgccatgggaagtgacccagcgcttcggagtgcccgccgagatcctgatctcgatctgggcgcaggaatcgagcttcgggcaggttcagggcgacaacgacgtgatccgctcgctggccaccctggcctatgagggtcgccggcgcgaatgggccgaagggcagctgaagaacgccctggacatcgtggtggacggcaagcgcgcgcgttcgggcctgaagggcagctgggcgggcgccatgggccagacccagttcatgcccgacaactacctgcgtctgggcgtcgaccagaacggcgacggcaaggtggacatctggggctcggacgccgacgccctcgcctccgccgccaatctcctggcgcaggccggctggaagcgtggccagagctggggctacgaggtcgtgctgccgcagggcttcgactacgccgaggccgagggcccgcgccatccgtggagcttctgggcggcgcgcggcgtggcgttggcggcgggcggcgcgcccaccgaggccgaggcgctggaagaggccgcgatcctgttgccgcaaggcgcgaacggtcccgcgatcctggccctgccgaaccactatgtgatccgccgatacaacaactcggtgtcctacgccctggccatcggcctgacggccgacggggtgtctggtaagccgggactggtcgcccgctggccggacgatccgccgatctcgcgcgagcagcgcatcggggcgcagcgcgcgctgacgcaactgggttatgacacccaaggcgtggacggcgtgatcggagcgaacacccgcgcggcgttgcgccgctggcagctggccaacgggcgcgtcgccgacggctatctcaccgccgccttggccgacgaactggccaggcgcggcggctgaaggcggatcagacctgcggggacgtccagccgccggccagcgccttgaacagcgccacctgataggtggtcaccagggcgtcggattgggccagctgcgcctcggcctggaccagggtgcgctgggcgtcgagcacggtcagaaagctctcggccccggccgtgaagcgcagacgcgacagctcaagcgcgcgattggcctgatcccgcgcctccgtcagcgccgtgcggcgatccagctcgttggcgtagttcgacagcgccgtctccgtctcctgcagcgcctccagcaccgtctggtcgaagtcggcgagcgccgcttgcgtacgggcgtccgccgcctcgatccgcgcacgggcggcgacgatattggggaagctccagctgatcagcggaccaaagccgaagcggaagttccggtcctctcccaggtcgccggcgtccagcgccgtcgagccgaacgaaccgcccaggctgatggtggggtagagcgacgccgtcgccacgttcacccgcgctgcggcggcggccaactgacgttcggcctgacgcacgtcgggccggcgggccagcagcgccgcgccgtcgccgatcgggatcggctgggtcaattgcggcgggcgtccgcaggcggcggcctggctcgcttcggcgggcgtggttccggtcagggtcgacagccggaacagggcctcggaccgggcggcccgcagcgtcggcagggacgcggtcgtctgggccaccgccgcgcgggcgctggcgacatccaggcccgttccggcccccgcgttcagcagcgtctcggtcaggcgcagcgtctcgctctggatctcgaccgagcgttcggccacggcgatctgggcgttggccgagcaggtatcggcataggcgcgcgccgtttcggccgccaccgtgacctgcagcccggccagcgcctcggccgcggcgtccgcatcggcgcgagcggcgcggatcgccgagccgacgcggccgaacaagtcgatctcgtaggaggcgtccagtccgacgtcgtagctggtgatctcaggcgcgtcctcgccgggcggcagtccgatggaggtggcggccgacccgcggctgcgctgcaccgaggcggaggtgttggtggacggcaggcgcgccgatcgcgcctccgacaggctggcccgcaccgcacgcaggttggcggcggccgattccagctggttgttctcggcgaacgcctgggcgacgagtccatccagcgtcggatcggcgtacagccgccaccagtcgtcgcgcgccgggaaggcggacgtgacggccgggtcggccgagccgacgaacgcgcccgtcccctggagggggagagttgggacgggcgcgtcgggccccaccgcgcaagcggcgagaagggcgctggcggatgaggccgccagcaaggtcgaaagcttggaacgaagcatcagaggtcccctccccggccgtgagcgggcgcgggtgcgtcagggtcataaggatcgtgcggattggtgccgtaggtggtgggcagggtgcggctcttgcccggcgtcctgggcagcttgcccgacacccaccgcatgatgacgtagaacaccggcgtgaagatcagaccgaagaaggtcacccccagcatgccggagaacacggccgtgcccagcgactgacgcatctccgcgcccggtccgctcgccagcatcagcggcaccacgccgaggatgaaggcgaaggaggtcatcaggataggccgcagacgggtccgggccgccgaaacggccgcgtcgaaccggttcatgccctcgtcgtcttcggcctgtttggcgaactccacgatcagaatggcgttcttggccgcaagcgcgatcaggaccaccagtccgatctggaccaggatgttgttgtccaggccgcggatgttcaccccgatgagcgccgccaggatgcacatcggcacgatcaggatgaccgcgagcggcagcgtgaaggcctcatactgcgccgccagcaccaggaagacgaacagcaccgcgaccacgaatatcatggaggcgccgccgctggcggccttctgctggtaggccagctcggtccactcgtaggagaagccgtccggcagtgtctgcgacgccatctgctccatgacctgcagggcggttccggacgccacgccctgccccgccgatccctgcagctcggaggccgggaacaggttgaagcggaccacgcgcgcggggccggagtcgtcccgcaacgtcgccaccgagccgatcggcaccatggcgcccgaggccgagcgggtcttcagattggcgatgtccgccaggtcgtcgcgcgccgacggctccgcctgcgccgtcacacggaaggtgcggcccaaaaggttgaagtcgttgatgtaggtcgagccgagataggtgcccagcgtcgagaagacgtcgttcggctgcacgcccatcatcaacgccttgtcacgatcgacgtcggcttcgatgcgcggcgcggaggtgttgtacaggctgaacacctgagccacctgctggttctgggcggcggctcccatcatggcgaaggtcgcctgctccagctcctgatagctctggccgttgcgggcctggatcatcatcttgaagccgccgccattgccgaggccctgcacggccggcggagcgatcagcaggacgttgccttcctcgatgactccggtcgccgcactgagcgcctgagacagggctgcagcctgcaactcgggcgcatcgcgttcggcgaagtcgtccagacggatgaacatggtggccgcattggacgccgccgagaaggacgagccgtcgaggccggcgaaggcggcgacttccagcacgcccgcctgcttgttcacgatctccacggcccggttcatcaccgcggtggtgcggtcaagcgatgcgccggccggcagttgcaccacgccgatcagaacgccttgatcctgctcagggatgaagccgccgggggtgtcgaccagccgccaggcggttaggcccagaagacccgcatagaccaccagcacgatggccacggtgcgcaccagccgcgcggtcaggcggccatagcggtccgacagccagtcgaagccttcattgaacttgcgtccgccccacgccacgccataggcgaccttgccccacggcgtcgcgcgcttgcggcgctgttcttcttcgtccacgtgcttgtggggcttcagcagcagggcggcgagcgccggcgacagcgtcagcgacaccagcagcgagatcagcgcagccgacgcgatcaccacggcgaactggcgatagaagatgcccggaatgccaggcaccaacgccgtcggcacgaacacggccaccagcaccaggccgatggcgatcagcgcgccggacacctcttccatggatcgataggccgcctccttgggcgtcagaccttcggagatggcgcgctcgacgttctccaccaccacgatggcgtcatcgaccacgatgcccacggccaggatcagcgcgaacagggacagggagttgatcgaatatccgagcgccagctgaacggcgaaggtgccgacgatcgacaccgggatggcgatgatcgggatgatggccgcccgccacgtctgcaggaacaccagcaccaccagcgccacgagcaccacggcttccagcagggtgtgctgcacggcctcgaccgacgccgccacatattccgtcggattgtacggaacggtgtaggtcatgccgaccgggaaggtcgccttcagcgcatcgagttcggccagcacagcttcggcggtgcccagcgcattggagccgggttgctggatgacggcgatgccgacgccgcggcgaccgctgaagtagccttgggtgccgtattcctgcgagcccagttcgacccggccgatgtcgcgcacgcgcgtcacgcggccttcggcgtcggtcttgatgacgacgtcggcgaactgctcgggggtctccagtcggccctgcacctggatgggcgtctggaaggcggcggcgttggtcgggaacggcggctgcccgatggagcctgcggcggcctgaatgttctgggactgaagcgcaccggtgatctcggtcgccgtcaggttgcgggcggcggccttggccggatcaatccagatccgcatggcgtagttgccgccgccgaagatgcgcacgtcgcccacgccgtcgatgcgcagcaggcggtcgcggatggtcgagttggcgtagttgccgaggtagtcgacatcgaggctgttgtccggcgacgtcagcgccgccagcatcagaaagcccgacgacgccttctgcaccgtcacgccgacctggcgcacggcggccggcagggccggctcggcgagagccacccggttctgaacaagcacctgcgcggcgtcgaggtccgttccgggctcgaacgtgacggcgacctgcaccgccccatccgaggtcgaggaggactgcatgtagatcatgccctccaccccattgatctgctgttccagcggcgtcgccaccgtctccgccagcgtctcggccgatgccccggaataggcggtggagacggtgatctgcggcggcgcgatctccggatactgcgacaagggcagcagcggataggcgaagatgccgatcagggtgatcacgaccgcgatcacgccggcgaagatcggccggtcgatgaagaagcgcgagatgttcatggacaggtgtcccttgttcgccttggcctgacggctaggggattacaggctgttggcgaagctggcggtggcggcgggcgcggcctggggcgtcggcgcaccggcctgctggccctgagcgggcgcgaccggcgtgatctttccgggctgggccgtgaccttggtcccgggacgcgcgcgttgcaggccgttgatgatgatgcggtcggtgggcgccagaccgctgcggatcacgcgaaggccttgaaccagaggaccggtcacgaccggcttgggcgtcaccgtcccatcctgcgccacgaccatgaccacgcggcggacgccgtcggccgagatcgcggcgtcgggcaccagcatggcgtcataggcggcgttgccggcgacctgcgcgcgaccaaacaggccgggacgcaggaagccgtccgcgttcggcacaatggcgcgcagccggatcacgcccgatccgtcgtccacggcgttgtcgctgaagtccaggcggccggtgcggctgaaggtgctttcatcctgcagcgcgatgcgcaccggagcgccctggttggcgccgccctcacgcagatacttgagaagcaccgcttccgatccgtcgaacacgaagtgcatcgacccgcccgaaacgatggtggtcaggacgtcgccggccgaggtgccgccggcgatgacattgccccggtccacgcggcgatccgacgcccggcccgcgatcggcgcggtgacgcgggtgtagctgaggttctggcgcgcggtgcggaccgccgcgttggccgccgccaggttggcctgcgcgacctgcagctgcgagcggttggtctcgacctccgcctgcgacacggcctgcgacgacagcagggtttcactgcgggtcagattggcgcgcgccagcgtcacctgcgactgggcttgagccacctgggcctgagcggaagccagttgcgcctccgctggagcggaatccagcgtgaacagcaactgaccctgacgcaccatctcgccgtcgcggaagtgcacgccctggatgaagccgccggcgcgggcacggacgtcgacagtttcgatagcctcgaagcggccggtgaactcgtcccagtcggtgacgcgctgcgccagcggctgggccaccgtgaccgggggcgcgcctgctgcgggcgcctgctcgcccttggaacagccataaagcgcggccgtcatcatgacggacacggccgcgatcttaagcgtgcgcatctgcgctctccctgtcggggggtcgtgggtaaggatatgcactcgatatgcgtggggagcgcccgagtcaacgtccggtgacttaatggtgaagccttggccgcttgtcaacacgcgatgacaacgccatatagcgcttaggggttattcaaccctcggaatttccaccttttccgttggaggccgatcgccttgctttgttcttcgcctcgcccgaggaatgcggccgcgactcgcggggccattcttgaggccgcccgtgcgcggtttgcggcggagagctatgatgacgtcggcatgcgcgacatcgcgcgcgatgtaggcgtcgatgcggccctgatcagccgctatttcggttcaaaggaagaactcttcgcgaccgtgctggacaactgtccggacgggggcgagctgatgcagggggaccggtcggatttcggacgacgggtcgcccaccacatagtcttcgagcccaagcgcgcggagaagatgcaggccctgtcgatcatgctgcgctcggtcggctcggcgaaggcgtcggaggctgtccgtcgcagctccagcaagcgcttctatggtccgctcagcgaatggatcggcgggccggatgcggcggtgaaggcgcgcctcgcatctgggatgatcatgggcatggcggtaagccgcgacatcaccggcggctacggcctgacgcccgaagactgcgagacgctgcgcgaccgcctggccgtcattcttcaaggcgtcatcgacgcctgatcccaaagcatgaaggcgcgggccggagcccgcgccttatgatccggaccctttggacgccgcttagtgcggcgacgcaaccggggcggcccgcccctccgcgcctctccagcgcgagcagaccagggcgaaggccgtcagcagcaggtagcccgccagcggcacaaagaaggccaggtgcatgtcgccggaccggtcagccacctgcccggcgatcagcggcaggatcgcgccgccgatgatgccgaacaccagcaggcccgacgtggccgacgccgaggcggtcgaacgctcaagcgtcagggtgaagatggtcgggaacatgatggagttgaagaagccgacggccagcgccgcataggcggccgtgacgccgccggtctgggtcaccacaagacagaggacgaccgcgacggcggtgcagatcgccagcaggatcggcgcccgcacccgcgtgagcagggcggagccgacaaagcggccgatcatggcgccgccccagtagaagggcaccatcttgccggcggcctcgagctcgagccccagcacgcctgggctcgccaggaagttggtcagcatgttgccgatggccacctcggatccgacatagacgaagatcgcaagggctccgaacaccgcccagcgcgacttcagcgccgaaaatatcgagacgttctgcccgggaaccgcgtcccgcgccggcgccgcggcgttgatcgacttgcgagccgagaagatgaacacggcgatgaccgcgaagaaggcgcccatgccgaggaaggcgatgtcgatgctgcgcagcgattcaccgcgtgtcgccgccgtcaccaccgcgcccgccgcgaacacgccgccggtcagcagcacgtgcgcgcccagccacggcccgaccgtcgcgcccagcgagttgaaggcctgcgagaacaccaggcggaagtgagagctcttcttggagccgagttcggccaccagcgggttggccgccacctgcagcagcgtcacgcccgaggcgatcacgaacagcgccaggagaacgcccggataccagtccaccgtggtcgccaccggcacgatcaggcaacccgccaccatggtggccaaggcggcgatgatcgcgcgactgtagcccagcttggaaagcaccgccgccgccggcagcgaggccacgccataggcgatgaaccaggcgaaggtggtcagaaaggcttcggtgaagctgaggtcgaacacccgccgcacggccgcgatcagcgggtcgatcagcgaggtggcgaagccccaggcgaagaacaggctggtgacataggcgaaggccagaccggcgcccttgcgcggcgcggctggcgttgaatcaagactcatcggcggttttcctccggcggccggctctgtcgcggctcaggttctcattgggtgggacaagatcggcgcagcgtccagaccgaaatgcggctcggtaaccaaacgtggccctttgtcccagaaagaaggccgctccggtttcccgaagcggcccgagaggtggcgcgccccatagagggaggcgcgctgctcagaaggatcagaagcgatagttcaggccgaccaggaaggtgcggccatagctctggtggtcgatgatccggcgctcgtcgccgttctcgaaggtgtagaagggctcatccgtcaggttgttgacctgggccaggatcgaaaggccttcggccggacccgactggatctcgtagccgatctgggcgtccaccacggtctcttcgccgacggagcgcagggtgcggccgttgccgaagccggcgacctcgcccaggaagtccgaacggtagcgggccgagacgcgcgcctggaagccgtagcgctcatagtaggccgtggcgttggcgacggtctccgacaggcccggcagggtggtcggtgcctgggtctcgtccggttggacctcgctgtcggtgtaggaggcgctgacgaagaagccgaagccctccagagcgggcgtcacgatctccagcggcatggacagcgagaactcggcgccctggatgtagccgccgttgccgttgtccggcgcgccgacgatgccctggttgatgaccggaacaacgccgccggtcgggtagccggtgaagtcgaagatctggttgcggttaaagacgtagctttccagatgcttgtagaaggccgccagcgagacatagccgcgacgattggcgaagtacttctcgatcgagatatcggccacatcggcgatgtagggcatcaactccggattgccgccgccgccgccccatggcgagttcaggtccggacgcgccaaaggcgtgttgttgttgacgttgaagctgtagttccgcgaggcgcgcatgtcgtccatgcgcggtcgcgccagggtgcgcgacaccgccaggcgggcgaacaggtcgtctcccacttccaggatgaagttggcgctaggcaggatctccagatactcggcgccgccctcaaccgcgatgctttccgatacgccggccccggcctgacgcgctgagaagcctgatgacgattgatcggtgtagacgaactgcatgccgacgttgccggtcagcgggcgccccatgaagtcgtggtcgatgttggccttgatgtatgcggtcgacaccttctcggtcacagtccaattgccagacacaacgtctgcgttcggattgcggaccagatcgtagaagccgctgttgaccaaacccagggcgtcgtagctgagcacctcggagatgccgaggtagcccagatcggtcggggccagcaggaactcggccggaacccggggagagccgcggcccgggatacgcaggtagaactgatcgttgacgaacgacttctcacgctcggagtagttgaagccgaagtcgatggcgttgaacgggctctggtgcagttcgcgacgcgcggtgaggcgcacggccttgatctcgtcctcgatggagggcgtgttcatgtagccgtcctggccgcccgggatcacgtcctggccccagccctgcgagctggtcaggaagatgctgttcggatcggcgtagttcaggcggctggtgaactgcaccacgccgtcctcgttgatccggaagtccagcgtgtcggtggcgccgacggcgttgcggccggtgccggccagggtctccagcacgatgtcgctgcgctcgaccttggagtagttgacgtcgaggccgagggtccaatcttcgttggccacgaactcggtgttccaacccagcgccagcacgttgctatcgcgcgtgttgatgtcgttgcggaccacgcccttcacattgttgaaggtgccggcgacgatcaggccatcttcgattacggtgttgcccggctggagaaccggggccggacggcagacgccggaaacaaagacgttgcccgtgatttcgcaaccgccaatgacggcaggggccgtgtccgtagcaccgcgtcgcaccgggttctcacccagtccgccccactgcagcgggaactcgatgccgcgcagaacctgcgtgttctcgaactcggaatagaaggcgtcgaccaccgtgcggaagcggtcgttggggcgccattccagcacgcccatgtagccgtcgcgcttcagctcgctggacatgacgtagggcttgacgccgccgatcaccaactgaccgatctcttcctcatagcccggacgcacggtgcgtgggccgtcggcgaccagcgcctgaccatagcggtcgtcgccgatctcgatggtcggatagccccagctgttgaagcgctccgactggtacggcgacgacatgtgggcatagcccagcgcgacgccgatggtgtcgtcggcgaactggtcgatgtaggacaggctgtagcgttggccgtggtcggtcgtgcccgagttcagggcgccgatgtcgttccattcatagcgatagttcagcgcgatcgcctgacgaccataggccagcgggcggatggtgcgcagatcgacggtgccgccaaggccctggccgatcagagccgcgtccggggtcttgtagaccacgacgctggacagcagctccgacgggaactgatcaaactcgacgccgcggttgtcgccggtggtgaccagctcgcggccgttcagcagggcggtggtgaagtcgggaccgaggccgcggatcgagatggcctgcgagcggccgtccaggcgctgcgaggtcacgcccggcaggcgggccagcgactcggcgatggacacgtccggcagcttgccgatgtcttcggccgagacgacctcgacgatggaggtgttgttggccttggccgagatcgaggcctcgacggcggcgcggatgccggtgacgacgatctcgtcgacctcggtggcttcgccctcttgctcgacctgcgacggcacggtctggttgggcgaaacgccgggggcggtcgactgggcgtgggcgaccccgcccatgagcgccaggacagcggcggtggacgacagcaggcgcgcacgcccggcgaagcgttgagacattcaatcctccctgtggccgtccgcgtttctgacgctgcgattggcctatcgcaaaagtatgcaaactccagaggctgttgcaagtctgtaatggatgcggcgtttgcgaggcgtggcgaacccagcggccgcgccacactgacgcagtgttgattgggcttgggtctcgacgaaacggcctcgaactgcgagatcaatgcggccattgacagccgccgagacggctgcaaaatcttgcaaacagacccgcaaacataacaagcgggcgcttacagggatggaagatcgaatgctcagcgcttcgcagagagccgccacggctatagccgccgtccttgcggccgccgcatcgtccgcctttgctcagtcgccgaccgatacgttggcgcagttgcggcagcgcccgccgcaggacgaggtgatctacttcgccctgccggaccgcttcgccaacggcgatccgtccaacgaccacggcggctatgcgcccgagaagctggtcagcggctttgaccccgccgatcccgaattctaccacggcggcgacctggcggggctgacgcagaggctcgactacatccagggcctgggcgccaccgccgtctggctggcgccgatcttcaagaacaagccggttcaggtcggcgaccgctacaccggcgcggcgagccacggctactggatcaccgacttcacggcggtcgacccccacttcggcgacgaggcggcgatgcgcgcctttgtggacgcagcgcacgcgaaaggcatgaaggtctatctggacattgtggccaaccacaccgccgacgtgatcaagtatcgcgagtgtccggagaaccgctgcgcctaccgcaaccgggccgactatccctacacccgccagggcggcgtggacggacagccgatcaacgaaggtttcgacggcgcggacttcaccaagctgcagcggccggactgggcctatacgccctacattccggcgggcgaggagaacgccaaggttcccgcctggctgaacgacccgatccgctaccacaaccgcggcgagagcacattcgccggcgagagctcgctggacggcgatttcgcgggcctcgacgatctgctgaccgaggatcccgtcgtggtccagggcatgatcaacatcttcggcggctggatcgacaaatacggcgtcgacggcttccgcatcgacaccgcgcgccatgtgaaccccgagttctggcaggccttcgtgcccgccatgctggagcgggcgcgcgccaatggcattccgaacttccacatcttcggcgaggtctacgatcacgacccagcggtgacggcgcgcttcacccatgtggacggctatccggcggtgctggacttcccgttccagaaggcggcgaccgatgtggcgtcgggcgtggtcggcaccgatgcgctcgccaagattttcgaggccgacccgatctacaggaacggcgcggacaccgccgccattctgccgacgtttctgggcaaccacgacatgggccgcgtcggctatttcgttcagaaggcggctccggaaagctcggacgccgagcagctggcgcgcgtcaagctggcgcatgccctgatgttcttcgcacgcggcgtgccgacgctctattacggcgacgaacagggcttcgccgggcccggtggttacggcgcctcgcgtcaggacatgtgggccagccaggttccggccttccgcgacgagacgccgatcggcggtcgccaggcgccctactccacccaggcgccgctctacacggccatcgccgagatgggccgcatccgccaggctgagccggcgctgcgtcgcggccgtcaggtgatgcgcgcctccggcgacaagccggggttgctggcctggtcgcgcatgggcgaggacggccaagaggtgctggtggtgttcaacagttccaccgctccgatcaacggccaggtcgaggtggaggccgcttcgcaacgctggcagtctgtgcgcggcgactgcgccgcccaggcctcggcgcccgccagctacgccgtcgccgtgcccgccctcgactatctgatctgcaagagcgcttcgtgaacgcccccatcctcgacctgtccctcgccgaggctccagccgctagcgccgccgccgatcaggagtggtggcgcggtgcggtgctgtatcagatctatccgcgcagcttcgccgattcgaacaacgacggcgtgggcgacctcgccggcctcaccgcgcacctggaccacgtggcgtcgctgggcgtggacggtatctggctgtcgcccttcttcaagtcgccgatgaaggatttcggctacgacgtatcggactactgcgacgtcgatccgatcttcggcacgctgtccgacttcgacgccctgatcgcccgggcgcgtgcgctcgggctcaaggtcgtgatcgaccaggtgttcagccacacctccgacgagcatccgtggttcatcgacagccgagccagccggcgagggaagcatgccgactggtacgtctgggccgacgccaagcccgacggatcgccgccatccaattggcagtcggtgttcggcggtccggcctggacttgggacgcccggcgcggccagtactacatgcacaacttcctggcctcgcagcctcagctgaacgtcaggaaccccgaagtgcaggacgcgcttctggccgcggcgcgcttctggctggaccggggcgtggacggcttccggctggatgcgatcaacttcgccatccacaatccggccctgaccgacaacccgccgatcaacgacggcaagaagcgcacgcggccgttcgacttccaggacaagatccacaaccagagccagcccgaaatcatcggcttcctgaaccgggtgcgggcgctgaccgacagctatgaaggccgtttcaccgtggccgaggtcggcggcgactacgccgatcgcgagatgcgcgagttcaccgccggcgacgaccgcctgcacagcgcctacggctttctctatctctacgccgaccacctgtcgtctgatctggtggtgaaggggccggcgatgtggccgggcgatcagggcgagggctggccgtcctggaccttctccaaccacgacgcgccgcgcgccgtgtcgcgctgggcgcaagggcgggacgaggacgccttctcgcgcatggcgatgctcctgctgatgacgctgcgcggcaacgtcttcgtctatcagggcgaggagttgggcctgcctcaggcgcatgtgccgttcgagcggctggtcgatcccgaagccatcgccaactggcccgagaccctgggtcgcgacggcgcccgcacccccatgccttgggcggccgccctgcggaacgccggcttctccacggtcgagccgtggctaccggtcgatccgcgccatgtcgccaaagcggtggatgcgcaggaggcggatgcgggctcggttctgcacgtcgcgcgccggctgatcgcgctgcgcaaacgccacccggcgctgcgggtcggcgccatggagccggtggagaccggcggcgaccttctgatcttcaagcggctggagcgctatgaggaggccgagcgtctgctgtgcgtcttcaatctcggccacgacgtcatcaactggagcccgcccgcaggttggcggctggtcgaggcggtgaactggtcaaaggccgacgccggacgcctgccgccgctcgccggactgctgttcgaggcggaatgaccggttcagccgccacaggtctcgcgaacgatcaggtcggtgggcacgcgctcggaacggccggcggacgcgcccccgtgatccagcagcttggacaccatcagccggccggccttgaccgtgtcctgggcgatggtgctgagcgccgggcggctgtagcggctgaaggggacattgtcgaaaccgatcaccgagacatccttgggcacatccacctcggcatgcagcagggcgcgggcggcgcccagggcgatctggtcggacgccgccacgacgccgtcgaaggcgacgcctcggcgcagcaaggcgtccaccgccgcctcggccgattcgacctcgaagtgcgccgggacgatcagctccggctcgatcggcaggcccgcgccagccaaggcgtcgagatagccgcgatgccgctgcatcgattcggggggctccagatcgcccaggaatacgatgcgcctgcgccccagccgcgccaagtgcgcggtcgcgcgccggccgccctggatgttgtccgatccaaccgagcagtagttctggtccggcagctcggcgccccagaccacgaagcggtggtcgcccgccgccagccggttgaaggcgccgtgcagcgtgctctgccccaaaaagatcaccccgtccgcccggctggtgttgagcgccgccgccaggtcgtcgtaggtcgccggggagatgtggctcatcaacaggtcgcacccgcgctcacgcgccgcctcgcccaccccggccagcagctccagaaagaacgggtcgctgaggcgcccttcccgtccctgcgggcgcggcgtcacgagggcgatggtgccctgcgccccgatcgggccggccggcatgtagcggcgaaaggggtagtcgtgctccttggccaacttccagatcagctgcttggtgcggtcgttcaccgctgggctgtcgttcagcgcccgcgaggcggtggcgatggatacgcccgccagccgggccagatcctcaagtcgcgtggtcttgcggctcacgttgaaaacttttctgcaaatctttcgcttccaatcgccgaaagaacggcggctggcaagtgggtcacggaaggaagcttcacatgatgcaacgtcgatcgtttctggcgcttgggggcgtgtccatgctggcgttcggtgcgccggtcctggcgcaaggcgcgcccaacaccgcccgcgcctcgtcgccaggtggtgtgctgacggtggaggtcagcaccgacaatgacggacgcccgatgtatgcggtcagccgggtgggacagccggtcgtgcgcccctcgcgcatgggctttctgctgacggaccagccgcagatcgagcgcggcctgcgcctgagcgccggccagccggtgacggtggacgacacctgggagcagccctggggcgagcgccgcttcatccgcaaccactacaatgaatggcgcaccaccttcaccgagacgggtggtctgggccgccgcgtcgacgtggtgttccgcatctatgatgacggcgtcggcttccgctacgagttccccgagcaggccgcgctgaccacggtgcgcatcggcaccgaactgacgcagttcaatctggcggagaacggcgaggccttgtggtgcccggcatgggagtggaaccgcgaggagcacctgtatcggcgcacgtccatcgacggcgtcggctcggcccagacgccgatgacggtgcgcggcgatagcggcctgcacgtctcgatccatgaagcggcgctgatcgactacgccggcatgaacctgcggcgcgaaggcggcacggacttccgctgcgcgctgacgccgggcctgaccaatgcggcggtggaacgcaccgcgcccttcaacacgccctggcgcaccctgcagatcagcgacacggccgcaggcctgctcgattccagcctgatcctgaacctgaacgagcccaacaagctgggcgacgtgtcctggttcacgccgatgaagtacgtcggcgtctggtgggaaatgcacctggagctgaagagctggggccagggccccaagcacggcgccaccaccgagaacaccatccgccacatcgacttcgcggccgaacacggcctgggcggcgtgctggtcgaaggctggaacaagggctgggatggtcagtggttcggcaacggctcggacttctccttcaccgagagctatcctgatttcgacatcgagcgggtgacgagctacgcccggtccaagggcgtgcagctgatcggccaccacgagaccggcggcaacgccttccactacgaccagcagcttgagcctgcgatggcgctgtacgagcggctgggcgtgcattcggtcaagaccggctatgtcgccgacgcgggcggcgcgcgcgtcgcggggccggacggccgggccgtgatggcctggcacgagagccagccgatggctcagcaccacctgcgggtggccgaggtcggcgcccggcacaaagtggcgatcaacgcccacgagccgttcaaggatacgggcctgcgccgcacctatcccaacatcatcagccgcgaaggccagcgcgggatggagtacaacgcctggggcaacccctccaatccgcccgagcatgaggccaacctggcgttcacccgcatgctggccgggccgatggacttcacgccgggcatcttcggcatgaagacccgcagcaacgagggcgtggccaccacctgggccaagcagctggcgctgtatgtggtgatctacagcccgatccagatggcggcggacctgctggacaactacgaggcgaaccccgagccgttccagttcatcaaggacgtgccggtggactggtccgacagccggaccctggacgccgcgctgggcgactatgtggtggtggcgcgcaaggagcggaactcggacgtctgggcgctgggggccatcaccgatgagcatccgcgcgtgctgtcggcgccgctgggcttcctggacgccgggcgtcgctaccgcgccgagatctaccgcgacgggccggacgccaactacaccgaccgccgcgaaagcatcgtcatcgagcagcgcgaggtcacctcggccgacatgctgacgctggcgctggcgcccggcggcggtcaggccatccgcttcgttccgctggggcgcagccgtcgccgttgaccgcgatcctcacgccgtcgttctggtcggatcggccgggatgacggcgggggacgtctgaaggaaagatcatgagcagcgccacgcccgaactgatccacgcccaccgcccgcgcctgtccggcctggcgatctggaacatgtgcgtcggcttcttcggcatccagatcggcttcggcctgcagaacgccaataccagccgcatcttccagacgctgggggccgaggtcgacagcctggccatcctgtggatcgccgcgccgctgacgggcctgctggtccagccgatcatcggccacttcagcgaccggacgtggacgcgcttcgggcgcaggcggccctacttcctggtcggcgcgatcctgacgacgctggcgctgatcgccatgcccaacagccccagcctgtggttcgccgcggccatgctgtggatcatggacgcctccatcaacatcaccatggagccgttccgcgcctttgtcggcgacaacctgccggaggagcagcgcaccacgggctatgcgatgcagagcttctttatcggcgcgggcgcggtgttcgcatcggttctgccgtggctcctgtccaacgtcttcgacgtggcctcgacagcgcccgaaggggtggtgcccctgtcggtgcggatcgccttctatgtcggcgccgcggggctgttcggggcggtgctctggacggtgctgagcacccgtgaatactcgcccgagcagatcgccgcctttgagcgcgcgcgaggcctcgagccggtcgcgccgggcgaggagccgccggccaagtcggtgcggggctggctgacgaccggcctggtctgcgcagtgctgggcgcgctggcgctggtgctgatcggcctgctggacctggagaaggagctgctgatcttgggcgggttcgcgctcgggttcggtctgctgctggtcgcggtcggcatgatgcagcggcggcgcatcaccaacgccgccaccgagatcgtcaacgacgtcttccgcatgccggcgaccatgcgcggcctggcggtggtgcagttcttcagctggttcgccctgttcgccatgtggatctacaccaccgcggcggtgaccagcgtccactacggcgcaaccgacacgacctccgccgcctacaacgccggcgccgactgggtgggcgtgctgatgggcgtctacaacggcgtcgcggcgctggcggccttcgccctgccggtgctggcccggcggatcggtcgcaaggcgacccacgccctgatgctgctgttcggcgcggccggcctggcgggaatcttcctgatccgggagcccggcctgctgtggctgccgatggtgggcgtcggcttcgcctgggcgtccatcgtctccatgccctacgccatcctgtcgggcgcggtgccggaccggaaaatgggcgtctacatgggggtgttcaacatcttcatcgtggtgccgcagctgctggccgcgaccgtcctgggcctgatcctgcgcacgatgttcgacggccaggcgatctacgcccttctgctgggcgcggcctccttcgtgctggcggcgatcagcgccctacgggtcaaggagcaccgggcgtgaaccggcgcgcgcttctggccgccggagcggtcctgcccttcgccggcgccgtgcgcgccgaggcgccgtccgccggtcggctggtgacgcacgccggcttcggctcggcccatgtgcaggcgcgcaacgtctcggtctggcttccgcccggctacgacgcgtccgacgcccgccatcccgtcctctacatgcacgacggccagaatctgttcgacgcctcgaccgcgcccttcggcgagtggggcgtggacgagcatctccagcggctgatcgccaccggccaggtgcgcgcccccatcgtggtgggtgtctggaacaccgacctgcgcctgcgtgaatacgtccccgccgacctgatcgcggccctgcccgacgacatgcgcgccgacgtgcaggcggtctatggcggcgagccgctgtcggacggctacatccgttttctgaccgaagagctgaagccgttcatcgaccggacctaccgcaccctgccggacgcgtcggacacgagcatcgccggctccagcatgggcgggctgatctcgatgtatgcggtgatgaagcggccggacgtgttctcggccgccgcctgcctgtccacccactggccgctgaaggtcgaggggctggagcccggcgcggcgctggacgtctggcgcgagcggctagtggacgcctggaccggcgtcatagccgccggtctgccggcgccgggcgcgcaccgcttctacttcgaccggggcgacgagacgctggatcggttctacgccgagttccagacacgcatggacgacgtgttccgcgcccgcggctatggtcccgacgacttccgcagcctggtgttcccgggcgcccagcacaatgaggcgtcttggaacagccgcctggacgtgcccctgacctttctgctttcgcccaaccaccaaaaggaggcgccgcgtgcgtgatctgaagaccctttgcctcgtcaccgccgccggcgtggcgctcgcctccgccgcctcggcccagagcatcgcgccgggcgcgccgggcgacgcccccacctggtccaccgccgccaagaccggcgcgggcgcgtcctacgaagcctatgtcgacggccagtatcgcgacggcggccgcaccggcgccctgtccaaggtttggttttcggtggcggacggcatgctgaccgagaccatgtacggcctaatccacgaagcgcagatcaaggccctgcgcttcgctgtcgcaacgctgtccggcgtggcggtggaaggaacggacacctcgcatcgcaccgaatatctgcatgtggatgcgcaagggcgtccgctgtcgcccgcctacaaggtcaccacgacggacaaggccggtcggttcgagatcgaaaagcgcatcttcaccgaccccgaccgcaacgccctggtgctgcgggtcacgatcaaggcgctgaagggcgacgtcacgccctatctgctgctggagccgcacgtcgccaacacggggatcgacgaccggggcgaggcgaccaacaccgccctctacgcccatgagggcgacacccatctggtcctgcgtcccagccaggtgttcacgcgcgccagcgtcggctttgtcggcgtctccgacggcctgaccgacctcagggatgggcggctggaccgcgcctacgcctcgacaggcgacacggccggcaacatcatgctgacgggcgccctgccgcgcgtgcgtcgcggccagagcctctcccgcgacttcgtgatcggcttcggcgacagccgccaggccgccgaggccgccgccgacggcgccatgtccaccggcctggacgaggttctggcccgctacaacggcgaaggcgagcgcgtgggctgggaggactatctgtccaccctgaccgaactgccgcgcatcgcgcagcaggcgaccgacggcgggaagctggcctacgcctcggccctgatgttgaaggtgcaggaggaccgcacccacgccggcgccttgatcgcgtcgctgtcgaacccgtggggggacaccgtggacgcctccaagccgtcgaccggctacaaggccgtgtggccgcgcgacttctatcaggtggctatggcgatggcggcgctgggtgaccgcgaaacgccgctggccgcgttccactacctgccgcaggtgcaggtcagcgcctccacgcccggcaacacgggcgcgacgggctggttcctgcagaagaccgaggtggacggcacccttgaatgggcggcggtccagtgggaccagaccgccatgccgatcatgctgggctatcgtctgtggaacctgggctggatgtcggacggcgacatggccgacatgtaccgccgcatgatcaagccggccgccgacttcctagtggacggcggcaagatcggcctgttgtggaacgacgctgagatccgcccgcccttcacccagcaggagcggtgggaggagcagcaaggctattcgccttccaccaccgccgccgtcatcgccggcctgaccagcgcggccgagatggcgcgcgaggcgggcgaccgcgcgggcgcggcgcgctaccgcgaaacggccgacgcctacgccaagggcgtcgaaggctcgatgttcaccacgcgcggcgacttcggcgacggccgctactatgtccgcatcacccagaaccaggacccgaacgacaaggcgccgatcggttcgtcgaacggccagatcgcgccggctgaggacagggtcgtggacggcggcttcctggagctggtccgctacggcgtgcgcaaggccgatgacccgtacatcgtcgccaccctgcccgagtacgacgaccagtcactggagcacctttaccgcgtccgctacgacttcggtcccgagggtgacaagacgccgggctggcggcgctacggcgtggacggctacggcgaggatgcggtcacgggcgccaactacggcgtcggcggccagatgagcccgggccagcgcggccgggtgtggcccttcttcaccggcgaacgcggccactacgagctggcgcgcgccagcgtgaacggcacgccctcgcccgccgacatggccgccatccgccagacctatgtgcgcggcatggaacggttcgccaacgacggtctgatgctgtccgaacaggtgtgggacggcgtcggcaacccgaccgagaacaactatgtcctgggccagaacaacgactcggccaccccgctggcctggacccacgccgagtatctgaagctcctgcggtcgctggccgacggcaaggtgtgggatcgctacgagccggtcgagcggcgctacgcccgctaaaaaggaaaagaggcccggcgagcgatcgccgggcctctgtctttcagaacagcaccttgatcgcgcccaccacgcgatcgtcgctgagcggcccgtccacatcggtgtcgaagtaacgtccgtccagcagcaggttctcggtgagcgcgaaggacacgcccacattccaggtcgtatagtcgtcgttcacgtccagccactgacgacccaccgcgccggacaccgtccacctctcggccggggtgaaggcggcgctgacctcgccataggtcgcctgctcgtccacgccgaagaagtccggcgaatagtagacggccgcgccgatcgtggcggggccgatggcgcgggacgccgcggccttgaactcgatcaggttgtagtctgcgccgtccggctcatcgacatagacatagccgatgacgccgaagtcgagcgcatagcccgacgcctcggtgcgccagccgccgtagatgtcgacttccgcatccgtctcgtcgccgaaatcgacgctggaggcccaggcgccggcgtagaagccgctgtccccgaacgtggcgtcgatcccgccctggagagccggatcctgatcggtctggctgacgccccggaagacgtagtcgctgaccaccccgatgttgaaggccacatccacatctgacgactgggcggaggcggcgcctgccgaagcgagcgccgcagtcgaggcaagggcggcgaggcacgcgcgaacgcactgaatgctcattgtcgatctccttgggttggataagggcggcggcgcgcagccgcgcccggtccggccgatcgcgaggatcggccggtgatgatgttcgatccggcgagagccgtcagatcgcttcgagcgcttccccatgcagtgaggtgtcgaggccggcggcctcctcctcttcgctgacgcgcaggccggtggtatatttgcagatcaccaggatcagcagcgtgcccagcgccgaataggcgatggtccaggccagccccagcgcctgggcgccgatgttggcgccctcggacaggctgttgatggcggtggtcgcgaatacccccgtcagcagcgcgccgatcagcccgcccgcgccgtgaatgccgaaggcgtccaggctgtcgtcatagcgcagcagcttcttgatccacaccgaggccgcatagcagaccggcccggcgatcaggccgatgatcaccgcgcccttggggtcgacgaagcccgcagccggcgtgatggcgaccagccctgagaccacgcccgacagcatgccgatcagcgagacctttttcttctcgatgacctcgaccagcttccaggtcagggtgccggcggcggcggcgagtacggtgttcagcagcgccacgcccatcagctcgttggcggcgccggccgagcctgcgttgaagccgatccagccgaccaggagcagggacgcgccgatcatcgtcagaaccggattgtgcgggttgatggggtcgacgccatagccgcggcgccggcccaaaaacagggcgcagaccaggcccgccacgcccgagttgacgtgaaccaccgcgccgccggcgaagtccagcacgccccccgcccaggaagcccccgccccagacccagtggcagatgggcgcatagatgaacagcgaccacaggccggtgaacagcagcagccccgaatacttcatccgctcggcgaaggccccggtgaccagcgccggcgttatgatggcgaaggtcatctggaacgagatgaacaggaactccgggatgcccggcagcaggctgttggccgtctgcaggctgacgccgttcaggaacagcatgtccaggttgccgacatagggctgcagcgcgtccacgccgttggcgccgaaggcgatgctgtagccggcgatgaaccacaccagcgacaccacggcgaacacgcccaccgactgggtgatggtggcgatgacgttcttgcgccgcaccatgccgccgtagaacagcgccagaccggggagggtcatcagcagcaccaaggcggtggagacgccgagccagcctgtgccggcggcgtcgagttcaagcgcggcctggtggccgagcaaggccggcgccggcggcgcggcctcggccgccgccgtcgtggtggccgccgcgcccgatccggacgaggcgaccacgggagcgggttcgaccgaagccgcggcgaaggcggcgcttccccctcctagaagccccgcacctagcaggagcgaggccatgagccccgcccatcgttttctgatctgcgacatcttgcgtgtatccccttctgcagtctcgcagcgggaagtgtttaccgcatatcaacggttcgcaagcggctgagacgtcagaagcgcaacattcgtgcaacaggacggcgacaaagatcattcgccgcataatccatgctggacgatgccccgatcaagcccagtgcatctggacgcgatgcgccgccgcccagtggatcgccctgatcgcgtcgatcaccgcctcggtcgccccccgcgtgcccaatccgccgcccagatcggccgtcaccgcgcccgccgacagcacggccgcaaccgccgcctcgatggagtcggcctcgtcctcgagcttcagactgtggcgcagcagcagcgccgccgacaggatcgcgcccacgggattggccaggtcctgcccggcgatgtcaggcgccgagccgtggatcggctcgaacaggccgggcccgtgcgttcccagcgaagccgacggcaacagtccgattgagccgcccagaaccgatatttcgtccgacagaatgtcgccgaacatgttctcggtcaggatgacgtcgtagtcgcgcggcttcctgatcaggtgcatggccatggagtccaccagggcgtgctccagccggacgtccgggaactcctcggcgccgatgcgggtcacgacctcgcgccacagacggctggtctccatgacgttggccttgtcgaccgaggtcaccttgccgcgacgctggcgggcggtgtgaaaggcggcgcgcgccacccgctcgatctcgaggaccgtgtattcgcacagatcgctggcgcggtcggccgtgcgggtcttttcgccgaaatagacaccgccggtcagttcgcggaagacgatcaggtcgacgccctccacgatctcctttttcaacggcgaacggtgcgccagcacaggcgagacctgcagcggccgcaggttggcgaacaggcccatggccttgcggatggccagcaacccctgctcgggccgcacctcgccgccgtcccactgcggtccgccgaccgcgcccagcaggacggcgtcggcttggaggcaggcctcgcgcgtctccggcggcagggcctcgcccgtcgtgtcgatggccgccccgccgatcagatgttcggtgaagctgaagtggtggccgtagaagtcgccgatgaccgacagcacgtcgcgtgcggcgcgcgtcacctccggccccacgccgtcgcccggcagcagcacgatgttgaaggtctggggtgcggcgttcggcatcagacagtctctctcaggcgctcaaaggcttcgatttcgggcatgttggcctgcagccaccccagggtgtccaccccgttcaaaaggcactgtcgggcgaaggattcgatcacgaaggtgacgggaggcgcatcgccgcgccggatctcgcccgcctgaaggtcgatcgtcacctgctgttccggatgtgtggccagatcgtcccaaacagcctgtgtcaccacgatcggcagaaagccgtttttcagggcgtttgatgtaaaaatgtcggcgatctccgtcgcgatcaccacccgaaagccatagtccagcagcgcccagggcgcatgctcgcgcgaggatccgcaggcgaagttgcgccccgccagcaggatgcggtgctcggccggatcgatgcggttcagcacggcctccggcttctccgatccgtccgcctcgtagcgccagtcgtagaaggcggctcggcccagaccctcgcgcgtggtggtggtcaggaagcgcgcgggaatgatctggtcggtgtcgatgttcgcctggctcagcgtcaccgtgcgggatgtcagcgtcttgaagggctcaggcatgttcctcgaccctcagatagacgcggggatcggtcaggaccccggcgatggcgctggccgcggccgtggccgggctggccaggatggtgcgagcgcccttgccctgccgcccttcgaagttgcgattggaggtggacaccgccagttggccgggcgccacgaaatccccattcatggcgatgcacatcgagcaccccgggatgcgccattccgcgccggcggcgagaaagacctgatccagcccttcggcttcggcgtcgcgccgcacagcttccgagcccggcaccaccagcatgcgcacgcgcggatcgacccggcggccccgcagcacttgcgccgctgcgcgcaggtccggcaggcgcccgttggtgcaggagccgacaaacaccacgtccacggcttgcgaagtggtcagccgccccggatcaaagcccatataggcttgcgccttccggtcggcgtcggaacggggctgcgggaccggcgcgccgacgggcgcgcccgcatccggcgtcgtgccccaggtggccatggggcggatggccgcgccgtccagcaccacctccttgtcgaaccgggcgcccggatcggtcgccaaggcgcgccaacgctcgacggcctcgtcccaggcggcgccatccggcacgtgccggcggcccttcagccaggcgaaggtcgtctcgtccggagcgatcatgcctgcgcgggcgcccgcctcgatggacatgttgcacagggtcatgcgcccttccatgtccaacgcgcgcacggcctcgcccgcatattcgatgacgtgtccggtgccgccgccgaagccgatggcggcgatcacggccagcgccacgtccttgcccgagacgcccggctgcagccgcccgttcaccgtcacgcgcagggtgcgcgcccggcgctgcagcaggcactgggtcgccagcacatggccgacctcggacgtgccgatgccgaaggccaaggcgccgaaggctccatgcgtcgccgtatggctgtcgccgcacaccaccgtcatgcccggttgggtcagacccagctcaggccccatgacgtgcaccacgccgcgatcctcggagtcccagccggccagcggcacgccgtgcgcggcgcagttccgctccagcgcatgcacctgcgcctcggcctcgcgcgtgacataggggcggcgaccatcggcgccgggcggcagggtcggtgtggaatggtccagcgtcgcataggtgcggtcgggccgccggacggccaggcctcggctctcgatctcggcgaaggcctgcgggctggtgacctcgtgaaccagatgcagatcgacgtagaggacgcccggcgtgtcgggggtctcgggccgaaccagatgggcgtcccagaccttgtcgaacagcgtgcgcggcggctcatgcatagcgcagcaccttctggtcggccgtccgctcggcctggtcgatgatggcgatcagttcggcgtcgtcgatctcgccgatctggtcggcgcgctgcttgaacccggtgaccacggcggccaagcgatcgccgtcgatggggcggccgatagtctcggcccgccgggcgatcgcgtggcggcccgaatgcttgcccagcacgaaccaactgccctcgaagcccacgtcctggggccgcatgatttcataggtgcggctgtcggccaacatgccgtgctggtggatgccggcctcgtgggcgaaggcgttgatgccgaccacggccttgttgcgcgccaccgccgtctcggtgacctcgcacagagtgcgcgaggcccgcaccatgtggcgggtctccacaccggtcgagacgccaaaccggtcgccgcgcaccttcagcgccatgaccacctcttccagcgacgcattgccggcgcgttcgccgatgccgttgacggtgacctcgacctgccgagcgcccccttccaccgcagccagcgagttggcgaccgccatgcccagatcgtcgtgattgtgggccgacaggatcacgccgggatgccgggcatggatccgcgccgacagctcgcggaaccgcgccctgacctcgtccggggtggcgtaacccaccgtatccggcgcattcagggtgcgggcgccggcgtccgccgccgcccccagcacatcggccaggaactccggctcggtgcggaaggcgtcctcggccgagaactccacgtcgtcgaacaggctgcgggcgtactccaccgcgcgtacggccgtggccagcacggcgtcggtgctcatcttcagcttggccgaacgatggatcgggctggcgcccagaaagacgtgcacccggcggtgcgaacgcggcgcgggcgccagggcccggcaggcggcgttgatatcggcctcgcttgcgcgggacagcgagcagaaccccggccccccccccccgcccgccacgcggcggatgccctcttcgccgccgggcggggcggcggcgaagcccgcctcgatcacgtccacgcccaggtcgcgcagcacccccgccatccggaccttggcctcggccgacatggaaaagcccggcgcctgctcgccatcgcgcagggtggtgtcgaaaacgatcacacggttcggatcggaggccgcgatctgttcggttcgggttacgcctaagggatcggtcatcatgcggcctgtgcgctgaaggtgtcgggcgagacgcggcggacgccgaacaggcggtcgatctggcgccccagggcgtcggcgcagcgctggtcgtcgcggccgcgcacggtcagggccacggcgcgcgctgcgcccgcatcagccatgctgacgccctcgatgtggaagcccctgcgctccaccaggccgatgaggcgctgaagcgaaccgtccgcgcggtcgatctggatgtggatcgtgctgctcatctcaggagccctccatcatgtcggcgttgctcttgcccggcggcaccagcggccagacgttgtccttgggatcgatgatcacgtgcatcaggcaggggccgtcggcggccagcaggcgggcgatcccgccgtcgatctggtcgcgccgctcgatgcggaaggcctcgatcccgaaggcctcggcgaccctgacgaagtccgggttgtcggacaggtcgatctcggaatagttgccggcgaagaacagctcctgccactggcgcaccaggcccagcgagctgttgtcgatcaggacgatcttcagcggcacgccgtagcggcgcagcgtcgccagctcctggatgttcatcatgaagccgccgtcgcccgcgatggtgaccaccgtgtctcgcggccgcgccagcttcgccccgatccccgccggcaggccgaagcccatggcccccagcccgcccgagctgatgtgcgcctcgggtcgggagaagcggcaatgctgggcggcccacatctggtgctggccgacgtcgcaggcggcgatgaagcgctcgcccgccgcctccgacagccgcttcagcagagcgggggcgtagacgccctcgcccggcgcgtcataccggggggcgtgatccagggcggcgcgggcgcagtccacgatccacggctggatgtccagcgccggcccgccccgcatccgcagggtcaacgcggccagagcagccttcagatcgcccaccaccgccacctcggcggcccgcagctttccgacctccgacgcatcggcgtcgaagtgcaccacgcgagcgtccggcgcgaactcggccagcttgccggtggcccggtcgtcgaagcgggcgccgacgacgagcagcaggtcgcagccctgcaccgcctcgttggccgcgcgggttccgtgcatgcccagcatgcccagcatgcccggcgcatcggtcgggatcgtccccagggcgttcagcgtcgccacctgcgggatggccgtcgcccggacgaacgccctcagcacctccgtggcgcgggcgatcttcaccccgccgccgacatagatcagcggccgcctcgccgcgcggatcgccgcctcggccgccgcgaccgcctcgtcgtccacgccggcggcggtgttgggaacggagaatccgcgcggccttgtggtcgccccgacctgcacatccttgggcagatcaaccagcaccggacccggccggccggaggcggcgatgtgaaaggcctgctccaccgccgccggcacatccgccggatcgcgcaccaagatcgagtgcttcacgatcggcagggtgacgcccaggatgtcgatctcctgaaaggcgtcggtccccatcacgccctgcgcgacattgccggtgatgcagaccatgggcacggagtccatcatggcgttggcgatgccggtcaccagattggtcgcgccgggacctgacgtcgccatgcacacgccgacacggccgctggcccgcgcataggcgtcggcggcgaaagcggcgccctgctcgtgccggaccaggatgtgcttcaggccggatcccgccagggcgtcatagaccggcatgatcgcgccgcccggataaccgaacaccacctcgacccccagccgctccagggtggagatcagcaggcgggcgccgctttgcgcgacggcgggttcgatcttcagggcggcggaggcggtcataacggatcaggcggccttcgccgacgcctcttgagccgatgcgggctcggctgcgttcagccacgccatgcgccggcgcagcgcctgtccgacgatctcgatcggctgttcgttgtcggccttgaccagggcgtcataggccggcttgccggcctcgttttcggcgatccaatcttcggcgaaccggccgctctggatgtcggcaaggatcgccttcatgcgctcgcgcgtgtcggcgttgatcacgcgcgggccggacgaaacagagccccacttggcggtttccgagatgaactcgttcatcttggtgatcccgccctcgtagaacaggtccacgatcagcttcagctcgtgcatgcattcgaagtaggcgatctccggctggtagccggcctcgaccagggtgttgaagccgctcatgaccagctccttggccccgccgcacagcacggcctgctcgccgaacaggtcggtctcggtctcctccctgaagctggtctcgatcagaccgccggtcgcgccgccgatgccgcgtgcatagcccatggcccggtcgcgcgctttgccggtcgcgtcgtgctggatggcgaacagggcgggcacgccgcgcccgcgcgcgaactcgcgccgcaccagatcgcccggccccttgggcgcgaccaggatcacgtccatgtcctcgcgcggcgcgatccggccatagtggatcgaaaagccgtgggcgaacaggatggccgcgcccatcttggcgtggggctcgatcaccgtccggtagatttcggcctgcgccatgtccggcgtcaggatggcgatgatgtcggccccgcgaaccgcctcggccggctccgcggtcggcacgccgtcctcgttcgcgtgacgccagcccttgccgccgtggcgaacgcccgcgaccacgtcatgaccgctgtccttcaggttgcgcgcatgggcccgcccttgcgagccatagccgatcacggcgatgcgctggccggtgatggcgcccggccggatatcgtcgttggtgtagatggtgatggccatggctcaggcgtcctcgtgggcttgggtgaaagccggaacttgcgccggcggggggttggggatggtcaccgcgccctgggcggccgaggccacgctggcgcgatacttggcgaagacgccgcgggccgccttcagggccggcgcgacatgggcggcgcggcgcgccttcaggtcggcggccacgtcgatgcgtcggtcggtgacgtcgatggtgatgcggtcgccgtcgcggatcagggcgatgggcccgcccgccgccgcctccggcgacacatggccggcgacgaagccataggaggcgccggagaaccgcccgtcggtgatcagggccacgttctcgatcccgcgccccttcagcgccgcggtgacctgcagcatctcgcgcatgccggggccgcccttcggcccttcgtagcggatgacgatcacgtcgccctcgcccaccgagccgtcctgcaccgcgtgaaaggcgtcctcctcgccgtcgaagacgcaggccggtccctcgaaccgatcgaccttatgccccgtcagcttgatcaccgcgccctcgggcgccacgtcgccgtggatcacggcgtatgagccgcgcgccatcaccggcccatcaaaggtcgccaccccctgctggcccggcgcctcttccgcttccgaggcttcgacaaacaggctgcggccactgacagtgggcgtgttcacaatcttgcccgccgaggccatgcgctgcgtcaccagccgcgtgccgcccgccgcgaacaggtgcgaggccagaaagcgcccgcccggcttcaggtcgcagatcaccggcgcctcgacgcaggcctggtggcaatcctcgacgccgaacgcgatcccggcctcggccgcgatagccgtcaggtgcatcaccgcattggtcgatccgcccgaggcggagaccgcgacggcggcgttcttcaggctggcgcgggtgatgtatttgcgggccgtgtcgccggcgaacacccgctcgacgatcagccggccgcagcgctcgccctccgccgccttggccggatcgaccgcgggcacgtcgttggcgcccatgggactgatgcccatgaccgatagggccatggccatggtgttggcggtgaactgacccccgcatgcgccggcgcccggacagacggcgctttcgaccgccctcaggccgtcgtcgtccatgcgtcccgccgcatgggcgccgatcgcctcgaacacctcctggaccgagacctcgcgatcgccgatgacccccggcatgatggtgccgccgtagtagaccagccccgggatatccattcgcgccagggccatggcggccgccggaatggtcttgtcgcagccgacgatgcagaccacgccgtccagctggtggccctcgatcgccagctcgatggaatcggccaccacctcgcgtgagatcagcgaggccttcatccccgccgtgcccatggagatgccgtcggtcacgacgacggtgttgaagtcgaccggatagccgcctgcggctgtgatccccgcgcgcacgtccttcgccaaccggtccaggtgcatgttgcacggcgtgaccgacgaccaggtgttgacgacgccgatcatcggcttgtcgaaatcggcgtcttgcatgcccgccgctcgcagatacgagcgcgccgccgcccgggtcgggccgtgcgtcaccgccgcgctgcgcgcgttcggccttcttggctgtgaggtagaatcttgcgtcatgggtctggttcgtcattgaaccgccaagcacgaaaaaccccgcttcctttcgggagcggggtgggtgcggggcgatcctgtgggttgggttcaggtcgcgtgcatccacgccgcttgcgtaagcaggccaagaagtacgagcgaaatgagcgaaaacaggctggcggccgccgaaggcgcacgaacggcgcggaccgccacggcggtcttgcgcttcatcgatgcgattttgcgagcggccacgataggctccctgttctttgcagaggtaaccacagcgccgagagacgcacaagccgccgcgcaataattttgcacatcatgcctcaacatggcctcgaccgcgcatcttcccgccggcgacccggtcgcacgcaaggagagccggcgggctctccgtcttccacgatcacgccttgtaacagcgccgcacttgcaacgggctctcgcgcgttccattgaagccccacacaaaagctcggcttcaggagacaccccatgaccgtccgcgtcgccatcaacggcttcggccgcatcggccgccttgttcttcgctccatcgccgagcatggccgccgcgacatcgaggttgtggcgatcaacgacttggggccggtggcgaccaatgcgcacctgctgcgctacgattcggtccacggccgttttcccggcacggtcgagagcggcgacgactggatcgacgtgggcctgggcaagatcaaggtcacggccgagcgtgatccggcgaacctgccgcacaaggacctgaacgtcgacatcgcctttgaatgcaccggcatcttcacgtccaaggacaaggcctcggcgcacttgaccgccggtgccaagcgcgtgctggtctcggcgcccgccgacggcgccgacaagaccattgtcttcaaggtcaacgacaacacactgagtgcagacgacatcgtcgtttccaacggctcgtgcaccaccaacgccctggcccctgtcgccaaggtgctgcacgacctcttcggcatcgagcgcggctacatgacgacggtgcacagctacactggcgaccagccgacgctggatacgatgcacaaggacctctaccgcgcccgcgccgccgccctgtcgatgatcccgacctccaccggcgccgccaaggcgttgggcctggtgctgccggaactgaagggcaagctggacggatcgtcgatccgcgtgccgacgccaaacgtctccgtcatcgacctcaaggtcgtcgccggtcgcgaaacctcggtggatgagatcaacgccgcgcttcagtccgccgccgacggtccgatgaagggcgtgctggccacgaccacagacccgctggtgtccagcgacctgaaccacatcgccgcctcctccaccgccgccctgccccagacccaggtcgtcgacggcaagctggcgcgcgtgctcagctggtatgacaacgaatggggcttcgccacacgcatgagcgacaccgccctggccatggcgaagctgatctgacccgcctctcctccccgtgcaaatggggatgaggaccatgaagtggcggaggggttcgtcccgcatgcaaacccccccgcctcgccgctgacggcggcgcgccaccccccccatcgctgtgcgaccgggaagagaaggaaagccccatgaccttccgcaccctcgacgacgccacggacctcgccggcaagaccgccctggtccgcgtggacttcaacgtaccgatggagggcggcagggtcaccgacgacactcgtctgcgcgtcgccctgcccacgatccagcgtctgcgcgacgccggcgccaaggtcgcgctgctcgcccacttcgaccggcccaagggcgagcgcgtgccgtccatgagcctcgaacccgtggtggacgatctggagcgactgctcggcgcgccggttcgcttcgccggcgactgcgtgggagaagaagccaaggctgggcttgctgatcttgacgtcggcggcgtggtgctgctggagaacgtgcgcttccacaagggcgaggagaagaacgatcccgccttcgcccggcgactggcggacctgggcgacatctacgtcaacgacgccttttcggccgctcaccgcgcccacgcctcgaccgagggtctggcgcgccttctgcccgcctacgccggcgagtcgatgcgtcgcgagctcgaggcgctggacaaggctcttggcgacccggtcaagcccgtgctgggcatcgtcggcggctcaaaggtctcgaccaagctggacctcctgcagaacctggtcggcaagctggatcagctcgcgatcggcggcggcatggccaacacctttctctacgcgcagggcgtggatatcggcggctcgctggctgaaaaggacatggccgacaccgcccgtgcgatcatggccgaagccgcggcgcggggctgcgaactgctgctgcccatcgacgtggtggtcgcaaccgaggtcaagcccggcgccgccgcgaggaccgtcaaggccggcgacgccctctcggccgacgacaagatcctggacgccggccctgacagcgtggctcgcctcaccgccgcgatggacgccgcccggaccctgatctggaacggccctctgggcgtattcgagatcccgccgttcgacaccgcgaccgtcgcggcggcgcggcacgcggcggaactcgccaaggccggaaagctgacggccgtggccggcggcggcgacacggtggcggcgctgaaccacgcgggcgtgtcggacgacatgacctttgtgtccaccgccggcggcgcctttctggagtggatggagggcaagcccttgcccggcgtcgaggctctgcgagtctgaccgccggctgtaacacggcgtgacttggaagctcggcgggtctagaacaccggccaataaaaagaacctgctcaggagacttccatcatggcgcgcatcacgctgcgacagctgctcgaccacgcagccgagaacgactacggcctgccggcctacaacatcaacaacatggaacagggtctggcgatcatggaggcggcggaagccgtcaatgcgcccgtcatcatccaggcctcgcggggcgcccgctcctacgccaacgacatcgtgctggccaagctgatcgacgccctggccgagctctacccccacatcccggtctgcatgcaccaggatcacggcaacggcccggcgacctgcgccaccgcgatccagtacggcttcacctccgtgatgatggacggctcgctgatggaggacgccaagactccggcctcctacgagtacaacctcgacgtcacccgccgcgtcaccgaaatggcccacgcttgcggcgtctcggtcgagggcgagttgggcgtgctggggtcgctcgagaccggcatgggcgaggccgaggacggtcacggcttcgaaggcaagctggatcactccgaactgctgaccgacccggatcaggcggtggagtttgtggccgccaccaaggtcgatgcgctggccatcgccatgggcacctcgcacggcgcctacaagttcaccaagaagccggacggcgacattctggcgatgcacgtgatcgaggagatccaccgccgcctgcccgacacccaccttgtcatgcacggctcatcgtccgtgccgcaggacctgcaggacatcatcaaccagtatggcggccagatgccccagacttggggcgtgccggtcgaggagatccagcgcggcatcaagcacggcgtgcgcaagatcaacatcgacaccgacaaccgcatggccatcacgggcgcgatccggaaggtgttgatggaaaagccgggcgagttcgacccccgcgcctatctgaagcccgccaaggaagcgatgcgcaaactctgcatcgagcgctaccagcagttcggctgcgaaggcatggccgacaagatcaagccgatgtcgaccgcccagatggccaagcgctacgcctcgggcgaactgaacccgcacttccgcacggcggcgtcgcaggcggcctgaaaccggtccgtcttcgttcgggcgcccgcgcgtgctaagcgcgcgggcgtgaccgacgccttctccgacgacgacgacctcgcccctgatcggctggaggcgagcatcgacgcgcccggcgtgcggctcgacaaggcgctgtccgacgcctttccccagctttccagagcccggcttcagacgctgctggcggacggcgccgtgacgcgcgacggcgtgccggtcgcgagcggatcgggcaaggccctgcccggcctctacgtggtcacgccgccgcccgtcgccccggccgatccccagcccgaagccatcccgctggtggtgctgttcgaggacgccgacctgatcgtgttcgacaagcccgccggcatggccgcccacccggcgcccggctgcgagacgggcaccctggtcaacgccctgctgcaccactgcggcgcgtccttgtcgggcatcggcggcgtggcgcgccccggcatcgttcaccggctggacaaggacacctccggcgtcatggtcgccgccaagtccgaccgggcgcatgcgggcctctcggccctgttcgccgcccacgacatcgagcgcacctacatcgccctgacgcgcggcgcgccttcgccggcgcgcgaccgcatcgtgacgcgcatcggccgctccagcggcgaccgcaagaagatggcggtgctgcggtccggcgggcgcgaggcgatcaccgactatctggtccagcggaccttcggccaacccgccaaggcgtccggcgccccgctcgccgcccgcgtcgcctgcacgcttcagaccggccgcacccaccagattcgcgtgcacctggcttcgaaaggcgcccctctgctgggcgcccccgcctacggctcgggcagccccgccgcaccggtgcgcagcgccgtcgccgaatccggtctgcgccgtcaggccctgcacgcggctgtgctcggcttcgtgcatccggtcacgggcgcacccctgcggttcgagaccgatccgcccgccgacatgatcgatctggagcgtcggctcggcgacctgtgaatacccgaccacagagctaggtcttgaacagcaacagccgctgtgctagaagcggagctcatccggtgcgagtggcgcccgggatacggtcacgctttcgtgtgaccgcccgtccctaaaaaggtcggcaacccatcgctacttgtccggttgaggggagaggcgtcggcgcacattagtggccgaagtcgaagcgcccgctcgtactatcttggtcggagggaccgtcatggccgccaacagctcgctcaccatcatgtcgcccgaacagggcctgtcgcgctatctcacggaaatccgcaagtttccgatgctgaccaaggacgaggagttcatgctggccaagcgctggtccgagcatcaggacccggaggccgcgcaccgtctcgtcacatcgcacctgcgtctcgtggccaagatcgccatgggctatcgcggctacggcctgccgatcggcgaggtcatctccgaaggcaacgtcggcctgatgcaggcggtcaagaagttcgaccctgacaagggcttccgcctggccacttacgccatgtggtggatccgcgcctcgatccaggaatacatcctgcgctcctggtcgctggtgaagatgggcaccaccgccgcccagaagaagctcttcttcaacctgcgtaaggccaagagccagatctcggccttcgaggaaggcgacctgcaccccgaacacctctcagccatcgcgaccaagctgggcgtgtcggaggaagaggtcaccaacatgaaccgccggctgggcggcgacgcctcgctgaacgcgcccctgcgcgccgacggcgaaagcgagtggcaggactggctggccgacgacaccgccgtgtcgcaggagaccaagctggccgaggacgaggagcgcggcctgcgcatgggcctgcttcaggaagccatggaggagctgaccgaccgcgaaaagcacatcctgaccgagcgtcggctcaaggatgatccggtcactctggaggaactggccggccagtacggcgtctcgcgcgagcgcgtgcgccagatcgaggtccgcgccttcgagaagctgcaaaaagccatgcgcgccgccgccgaagagcgcaacctggtcgacgcctgagatcaggcgtgagaccgcgcgcgcggcttcagcccgcgcgcgcctgcgccatgggggcgttcagcgccaggatcgcgccgatcggttgtgccaggccgtccttggtcaccgccgcgccgctgagatagccgtccagggcgttggtcgcgatcgccaaaccgatgtccccgcttttggccgccagcgccttcagcgtctccacctgctgcttggccgcccgcgccgcctgcgccgggtcgtcgttgaactgcgccagggcggccgctaggatgcgcagggcctgcgtcttcgcgtccaccgtcttttcgccggacgccgcatcgcccttgcgcttgcgggatccggcgtactcgcccgagttgaagcggcgtcggtccggtccgacatagccgaccgcctcgatccacgggcgggacttcagggcgacgttctcgatgcgcttgaacaggtcgccggccgtgaaaggcttgcgcaggaactcgtgcacgccggcgtcgcgtgcgcccttgatggagcttgcggtcgcatcgcccgtgaccatgatcaccggcgcggcgcggcacgacatcgatgaccgccgcaaccgccgcgtcaacgtctcgccgttcagcgtctcgccccgccgctcggtgaagatcacgcccggctccacgtcgcgcagcagctccagcgcccgctcttcatcgctttcgatgaagacctcgcgcgagccgatgcccttcatgatgtccatcagcagccgcgcggacgccgggttcggatcggcgatcacgatccgacggatcgacggggcgatccggttcagcgtgcggggatcggcggcgaacaagacgggctccgtggcgacaatcccgtcaagctaggcccgccagggttaagatcgccttgaacccggccgcctcacccctggaagggatcgtgcatcaggatggtgtcgtcgcgctcagggctggtcgacagcagggcaaccggcgcggcgatcagctcctcgatccgccgcacgtatttgatggcgttggccggcaggtccttccacgaacgcgcgccctgcgtgctctcggaccacccctcgatggtctcgtagatcggctcggccgccgcctgatccttcatcccggccggcagatagtcgaactcgcgcccgttgatgcggtagccgacgcagatcttcagctcgtcgaacccgtccagcacatcgagcttggtcagggcgattccgtgaatgccgttgatggcgatcgattgccgcgccagcaccgcatcgaaccagccgcagcgccgcgcccgccccgtcaccgtgccgaattcacgcccgcgctcggcgatccgcttgccggcatcgtcgaatagctccgtcgggaacggcccctcccccacccgcgtggtgtaggccttgacgatccccagcacataaccgaccgaacgcggccccaggcccgatcccgccgccgcctgacccgcgaccgtgttggacgaggtgacatacgggtaggtgccgtggtcgacgtccagcagcgtcccttgcgcgccttcgaacaggatgcgcttgccgtcgcggtacgcctgatccagcatccgccacaccggctggctggcgaacggcagcaccttgggcgcgatgtccagcaactcggcctttaggctggcgacatccacctccggcaggtccaggccgcgccgcagcgcattgtggtgcgccagcagccgctcgatcttggcgtccagcgcctccgggtccgacaggtccccgacgcggattgcgcgacgtcccgccttatcctcataggccgggccgatgccgcggccggtcgtgccgatcttggtcttgcccgcctgcgcctcacgcgcctgatccaggtcgcggtgcagcggcaggatgaggcaggcgttgtccgccagcgtcagcatttcgggagtgatcttcacgccctgcgcctcgatccgcccgatctcgtcgatcagcgcccaaggatcgaccacgaccccgttgccgatcaccgacggcttgccctgcaccacccccgagggcagcaggctcagcttgtaggtgacgtcgcccaccaccagggtgtggcccgcattgtgcccgccctgaaaccgcaccacccagtcggcgcggttggacagccagtccacgatcttgcccttgccctcgtcgccccactgagcgccgaccaccgccacgttcgccaagaccgttatctccgcacttgatgcgggcgcagcctataaccggggaatcaggcgatgtccccccgagcggtcggatttatccgagttcggacgctacggtttggaacgcccactccagccagggcgtggcggcgcgcacgtcggccgtctccaccgtgcaaccgcaccacaggcgcagtcccggcggcgcgttcctgtgcggctccatgtcgaagaccgcgccttcgccttccagtagcgccttgaaccgcacaacgaacgccttctgggcctttgcgtccagcctcaccacgcctgcatccgtgaacttcagacagaccgaagtcgtggatcggatctccggccgctccggcagaaagtcgatccactccatccgctcgacccattcggccagcgcggcatagttggcgtcggtgcgacggatcagctcgcgcaggccgccgatcgacttggcccaatccaaggcgtcgatccagtcctcgatggtcaggaccgagaaggtgttgatcgccacgccgtcggccagcgaccgatcaaagccgtttttgtcggcgatccgcagcaccttggggatcgcccgctcgggccgatagccgtccagccgctccaccgcgcgcggcgacagcgccatgaccccgatgcccgcctcgccgcccaacgccttctggaaactgaacgtcaccacgtccagccggtcccacggcagcggcatggcgaaggcggccgacgtcgcatcgcagatcgccagcccctctcggtcctccgcgatccagtcggcgtccggcacgcgcacgccggacgtcgtgccgttccacggaaacaccacgtccttggaccagtccgcgcgcgacaggtccggcagctcgccccaaggcgcctccagcacctcgggctccagcttcagatgatcgcgcacgtctgacgcccaggtcaggccgaagttctcataggcgatcacctgcacgccgcgggcgcccaacattccccacagcgccgcctccaccgcaccggtgtccgagccgggcgtgtagagcatcacgaaatcgtccggaacctccagcacctcgcgcgtcagccgcaggccatgggcgaaccgctccaccacctccggcgcccggatgccgcggcccagcaggttcgtcagcaggccctccagcgcatagcccggccgcttggccgtgggtccggccgagaaccagggccgttcaggcttgatcggaggctgatccatcaccttcattgccccggctgatagggtcgcttgtcgcgccactcctcggcgaagcgcaccagcgtctcgtccggcgcgtccggcaaggtcaccaccaggcgcgccagcaggtcgccgcgccgtccggcctcgtgtgccccgcggcccttcagcctcagcacccgccccgagttggagcccttggggatcgtcatcgacaccgcgccctccggcgtcggcacccgcaccttgccgcccagcaccgcatcgggcaccgacaccggcaggtccatcaccagatcggagccctcgcggcggaacagcggatgtgccgccagcctcagctcgatcagggcgtctcccgcctctccgccgcgtcccggcccgccctgccccttcaggcggatggtctggccgtcggtcgcgcccttcggaatggttacgtccagcgtccgcccgtccgagaactggatgcggcgcgtggcgccggcgatggcgtcctccaggctgatctccagcgtcgcgcgcacgtcctgcccgcgctggggtccggccggccgccggccgcccccgccgaacatgccgaagatctcgtccagatcgacgccctcgaagttggctcgtccgcccggcccgccttcgcggctgaagccgaagccgctggatccgccctgaccgaacgggctgccgctggcgcgtccgccgccgaagccgcggaactgctcgttgccgtcggcgtcgatggcgccctggtcgtacttggccttcttctcctcgtcgcccaggatgtcgaaggcggcggtgatgcgcttgaaccggtcctcggccgccttgtcgccggggttgcgatcggggtgcaactccttggccagcttccggaacgccttcttgatctcctcgggagaggcggttcgggacacgcccagttccttgtggggatcgctcgccgcgccgtctgtcgctcctcttaggttcgctgataaactacccgtcagttaagccatgccctctgcgcctgaaagccccgcgcggttctatccgccgataaagatgcgcgcctccacgccccagccatagccttcaccccactgcgccacggccagcgcaacgtcggtgacgagcccgtcgggaaaatcctccgccacggctccggccgcataggtgaaggtctcgacggtcgcctccgccaaccgaaccacgcggtttccgtccagcacgcggatgcgatagcgccgcgcgtccagctgcccctccgcgttccagccgacgccgggccgccgcgcacgcggcgtccaccgtaccgtcagggcgccgtccgccgcgtgttccaccgtcagacccgccggcgaccacggccggtggtgaacacccctcggggtgaagacggtctcggcaaagcggtcgccgcccggcggcgcgcctcttggtcctgcccggcagatcagcggcaagcctcgctcgctccgcccgatgtccactcgcggcagtcccgcatccagaaacaccacaagcgcagcctccatcgcgcccgccgccatctcgccgtccgtcccttgctgcgcccgcaacaggccgctcagccgccaggcctctgaaccgatcatctcggcatggcggaactgcatcagctcccagccgccccccgcacactcgaccgcgatctggttgacgccccccagcaccgccgcctccgacgcgctcgccggcgcctcgccctcgacccggacgtccagaacgcttccctcgtcccagccgtcgatcggccccggcgtcaccggcgacaacagcactcccaccgtcgcgggcgtgtccacgaccgcccgcgccgtcaggctgtccgcggtcatgccgacatgcaggctcatcgggcgccacggctcggccgccagcaccacgagcggccggtcgtcctcttccgcccccggcagcggtggcaggtccagcagccgcagcaaaggcgcgcccgccgcctcgaggtccgccgacccgcgccagtcttccgccggatcgagcgccagcgccgttctaagcggccgcaggcgcagcctcggcgtctcgtctatcgccgcctgttcgacccgccagacgcccgcgcggccttccacccgcaccgcatcgcccggttcgacccgcagcgccaggtcgggcccggcggccagcgtcagcgcctcctcgccctcgccgtccagcaggcgcctagccgcccgcgccgccagcccgctgccgcacgccaccggcaggtccagatccagccccccgccgtcttccacctcgtccgaacgcaccgtcaccgccccggtctggtagtccgccgcctcgtcgatgaagcgcacccgcgccgtcgccggccgctgttccagcgaacggtccgccgcctccggcgcgccttcgtcctccagcgccaagtcatcgtgcgcaatatccagcacctcgcccgagcgccccagcacggcgatcccaccgccgcgctcggccgccaccgcatcaaaggccgtcaacagcggcgccagcgcatcgcgcgtccgcatcggccggtcgatcaaatagcccgccgccgcgccctccacgccttccaccacgaaaccgtcgtccgccacgccgccgcgccgcagcaccgccgcgatcaggtcgcgcgcatcgcccgtcagccgcccgttcagccagtgcccgctgcgccaggcgcccgcatccgcccacacgtccgcgcgcgccggaaaggccggatagggccgcgcgtcccagcaccaggcgtccgccccctccagcatccgccccccatagaccgccgacaccggattgttctcgggcgccgcatagtgcgccagtatcgcctccagcgccgcccgctgcaccgcatcgtcgcgcgcgccgctggagtgcggcggcagtctgccttccgagctcttggggtcctggaacagattgggcgcattgccgccccggtccaccgccgcgcagccgaactccgacagccgcaccggcttcatcccaggaacccaggcggtcggcgtcgccctgcgcaccccgcgcggtcgatcatggtgcgcgttcgaccaccagcccttcaggtccttgggccggaacagccagtcctcgccgtgcgccgtgtcgcggatcggcgtgcggacctgcgccgcgcgctcagcatcgccgccgtagaaccagtcgaaattctccccgcccgcgacgttcgccgccagatacgccggatcggcggcgctgtcgtatcgcagcccgtccactccgccgtcgcccacgcgccagtcgctcagcggtggataccagtcgaccgacacatgatcgatgttcggatcggcccacagcggatcgagatggaagatcacgtctcccgtccccggctgatgcccgaaatactcggaccagtccgccgcataggacagcttcacgtccgtcccgaccaccgctctgcactcggccgccaacgtgcggtactgcgccaccgccggatagccgcccgcctgatcccgcgtccacgtcagcccgcgcatctccgagccgatcagcaggccgtcggcgccttcctcccgcacgatccgggcatagtgcagcgccatgcgcctcaggccccacccgttcgcctggccgaacaggctggcgatctgcgccgccgcccctaccccgtcctcgccccgaagacgtccgcgccagggatgcggcgcctgccgcccgccgccatacggatcgggcagagcattgtccgccggcacgtccatgaagatgaagggatacagcgtcacctccagcccacgcgccttcagttcgcggatggcctgccgcacgctgtcgtctgacggcgtgccgccataggcggggcgaccgtcgtcggaaatcagatgggcgtcgccccgctccagccccgccaccgaccaccgcagcggctcggttggcttgtctctgcgctccacccccggcctgacgcggcaatgcccggcccgcagatcgtcgccgaaccagcccaccaccaggctgacacgcttcaggttcggcgcctgcgcctgcagttggtccagcgacacaagcaggtccgcgcgcccctctcccgtgtgcgcattctccggccgggttcgcgtcagcccttcgcgccgcaacaccacgtccgtcgccagggtgaactcgcccgcgccggggatcaggcacacgccctccagcaaatcctcgagccgcccgccgctcccgaccggccggcgaaagacttcaaagctcagctgcggcggccgatcgccataaggcgtcagcggcaggtcctcgaacaccacataggccgtgcctcgatacgcgggagccgtcccttctatggcttcgatcagcgggtccggctgctggtcctccgtcccgcgatgcagccgcatggcgatccccgccgtctccatcggctggccgtcggcccagacgcgcccgatcccgtcgatcggcccctcgcccagcgccacggcgaaactcagcgaataatcatagtcgatggtctttggcccgcccttgccgccgcgctgctcggtgcgtcgttcctgaaaccgcgcggcccagatcacctgccccgtcacccgcgcccgcccgaacacgcaggccatgggtgcgccctccgccgttccctggatcttcagcccgtccagccgagggcccacctgccgcgccggcgacagcgcacccatcagcgccccgtccgccatccgccccagcgtcgcgccgatcacccgcccgacgcctccgccgaccgctccgccgatcccgcccagcaccacctgcgccatgtctcgtcagtcctcgcatccgggccagcggaacaccgccgccagcctccgcttccaccatggccccatccagctttcgaccaccgcccgcccccaataggcgtggatgatgcgcggctccgccccggtcgtgtcgctcaggatggcgcagtgcttgaccatcgccccagggctcatccggaacagcagcacgtcgcccgcccgcatcgtgtcggcgggaacctcgaccagccatcgccgcgccgcctccagcagcctctcctcgccgccgacctcggcccagtccgcgcgatagggctcaggcgtctccggctcctcgcccactatctctcgccacaccccgcgcaccagccccaggcagtccgcgcctgcgcccttcacgctggctccgtgccgatagggcgtccccagccaccctctcgccgcctccaccacggccaatcctcccccatcgggggagggagaccgcgcggagcgcggtggaggggcgcgaccacgccgctcatcgccggctccccccgtcccgccgcccgctcgtcgccgcatgcgccaccaggaagtcgtcgccgggcacgtcgggaaagccgcgatagttcaccccattgccgaacaatccgacacaggtgctccagcgcccgtcgcagctcgcgccagcctcagccgcgaccccgcaccgggcgtcccccagccgcgcgtcgcacatccggccgtaggtccgccccaccacccgctccagcgtgcccagcggcccctgcaaatccgccgtgaaccgcccgccctcgcaccggacccgcgtcagcgtcgccgtccacagccgcacgcgcaggtccggccgctcccagtccacgcgccacaactccaccgccgccccgtcaaaggcgccggccgcgatcgcctcttccgtgatcgtctcgtcgtccagcgccccagcggccgacgccgcgcccgccgccaggccgactgcgctttccgccgcccccgccgtccagccgctcccggcccgacagcgaactccgtccaccgtcaggtcgcgatcatgatcggtgaacccgagccgcactccgtcccgccgcctcagcagccagacatgacacagcgtcgccgccccgctcgccatgcgggcggccatctcttcaggcacgatgcgcatggctcagatcctgatctcgatcagcggcacggccgccattcgcccggcgtcgaagctttccagcgacgcctcgatccggtccgcgtcgaaccgcaccggcgtgtcgaacaggaagccagccgtcaccacagcccccttcgccggcggcgcggccagcgtcaccgcgcccgtcgccacatcgaccgccgcctccaccgcctgcccgttcaccgccgccgtgacggagccctcgaccggcttgcggatcggccggcgcacctcgccataggccttggtcagctcgaacgtccgccgcacgccgtcgccaaccccgatctcctggtccgtggccgcaggcattccgctcggcgcgcatgacttgaagtcggcgaagtcacgaaaccggaacccgtacagccgcccccgccgcgcctcgaagaacgccgtcagcgccgccatgtcgtccagcgaacgcaggttggccccgatcagatagcgcctgcgcccctgcgcccacgggctggagcgccgctcgtatccggacgccagcgtcaccacctccgtccgccgctccactccgccgcttgatccgaacgccagccgagcgggcagccgcacctcatgaaagctcatggcgcttcctgtctccggtttcacttgttcgccttgcgccgttccgtcatgctcaagcttccacgagggggcgaacacgacatgcgcggcgagattctcagctatgacgcggccacgggcggcctgatcagcggcgacgacggccagcgctacggcttcaccgcctcagcgcttcagtcgcccgccgtccccgcccccggcgtgcgcgtcgacttcatcgcccacggcgccgatgcccgcgagatcgtcatcctcgccggcgcccacaccgcatcggcccagactgcgtcggcccagccggccttcgcgaccgcaggctccgccggcctgcccgacatgtccgccgtcgactggaagagcctgatgctttcgttcgagggccgcgtccgccgctcacacttctggatagcctggctgatcctgctgggcgccaatgtagtcgccggctggctgccgctgatcggggtcctgatcagcttggcgctgatctggccaaacctcgccatcaccgtgaagcgcctgcacgacatgggccgcaccggctggctggcgctggtcccctttgtcgtagccattgccatgttcatcgtcggcatcatcttcttcggcctaggcgcggccctcggcggaggatcggacggcgacttcgagaaccctgtggccgccttcgccatgttcggcccggcgatcggcgccttcgccgtcgccgccttgatcggcttcgtcttcctgctctggatcggcctgaccgacagccagcccggcgccaaccgcttcggcccgaatccaaaggggctctaaggcgctcaagcagccccgcgtcgcacgcggggcggtagcgccctcagcatgcccctctcgcgcccaggctgaccgcgcgggccagcatctgggcgatctgcgcctcggacctcagcagggccggggcgccgccgtccacgcgcacattgacggtaacgccggcgccgcccgccggctcgaccacgccgccctgcgccggccggaacacctccggcccgcgctcgcccaccaggtaggcgccgcccgccagtacagcccctccgtccgcgcgcgccccgccgaacatcccgccgacggcctgagcgatcgcgtcccccaggccgcccccgcgccccgcaccggctgcctcttatacacatctgacgctgccgacgaattagacggtgtagatctcggtggtcgccgtatcattattaatatatcttatccacctctgacgctgccgactaagatgatagtgtagatctcggtagttgccgtatcattcaaacaccaagaacatgattgtgtggatacagtggttaatagttgagaaaca

SEQ ID NO: 7 - DNA, 166155 bp, brevundimonas massiliensis
  source 1..166155: mol_type = genomic DNA
cggcgggggcggcggcgggggcgcgaccggctcggcgccgaagctgtagcgcaggcccagcgtcaccgtgtggctctcgtcatagtcgccgtcaaaggtgccaaacgccgtggcgcccgtgccggcggtgaccgaatcgaactccagatcgctggtcaggtagcggtaggtcagatcgatgttggcgcgctcgccgacggcgaaggcgacgcccgcgatcgcctgggcggcaaacttggtggagctgtcgtcggccacgaagctgacgcccggggtggcgcgcatgcggccggcgaagtcggtgttgacgtagttggcgccggcgcccagacccacgaacggacgcagaccccagtattccatgccgaagtcatagatgacgttggccatcagggtggcggactccaggtcgccttccggcgaatagcaggggcccgtcgccggagcgaagttgcacacgccctgggtgcccgacacggcgcgaaccgtgccgatgtcgcccgagcgatagccgccttcaagctcgacgcgccagttcgggttgaaccggtagcccagacgcgcaaacgcggcccagccgtcgttcacgtcgatgttgaagttggcgccgttcgcttccgactcgatgttgatcggctcgatgaactgataacccgcgtcaatcgcgccgtaccagccatccggctccgccgaagccgcgccggccgcgaacagccccgctgccgcgacgcctgcgagaagtttgaccttcatttgcgtcctcactctgaaaaaggaatgccaaaaaatgccggcattgagtccgccgacgtgcccgaaccgaacggcgccgctcgcacagggttccgcaggcaagtggcggaatgtggcgagtgtggcgccatttcaacacaaggaggcggaacccgacctttcgcagaccgactttgcggcggctataccttctcgctgatcttgatcgccacgcggcagccggtcttgatgacggccgacagcagccgatagacgggcgcttcccgactgccgtgcgcaaccgcgtggtcgtggtgctccagttcctccatccggaactgggtcaagtcagcagcgagcgcgggatcgcgttcgccgatctcggcgatctgatcggcgtagtgttcttcgatcacgctctccaccgcctcggtgcaggcgtgcgccgccttctcccccagcagggcggtgcccacccccagcgccgacgccgccacgcgccagaccgggatcatggccgtcggtcgggtgcgacgatcgttcaacaggccctcaaagcgcgcgaggtgcgccgcctcctgcgcctgcatgtgctccaggtccgcggcgacggccgcatgtcccttgcgcccctcgaacacggcgcgttgcgcctggtagatgcgcacggccgcatactcgccggcgtgatcaacccgcaggatctcatccatgcgcgccttgtccgcctcgccgccggggcgcgccagcggaatgcgtctttggctgtggatgtcggtcatcggcttgttcctcttggtgcgcgggcgtccttgggacgcttggccgccagaaggctgaacaccgccagagccaaggagatcaccgcattccacccggccatggagacgcccatccacacccaggccgcctcgtcgcagccgaccacgcggggcgccggtcccgtgcccagcgccagcgccgtcagcccctccagatcaacgccgccgccagccgcgcaggccgccggcaaccgccaccagccgtactcgccgccggcgtgaaaggccgccgcgatcgttccggtcaggaacaccgccgccaggagaaaggacgcgatccggggcgtgcccctccgcccgccgctgatcaacgtccaaccggtcgccagaagtccgatcacggccgctccccagaacacctcccgctgcttcagacaaagattgcagggctccagtccgccgaactgctcgaacgcatgggcgacgcccagcatggcgagcgaggccgccagcgcgaacgcagtccaccatcgggtcagaagtcgataggcgcgggtcatcgccgacctcttagcgcgcggtcatgtctccgtcgaccagcccgcccaaggcgcgctatgtcgatccgtcttctcctggaaactgcctggccatgaccgacattcacgcctccgtccacgaggacgacgtcagccacaacgtcacgcgcctgctgcgcaggctgtccgacgatggtggcgagcacggcctgaccctgcacgaaatccgcgaccggctggacgagcgcgcctacggcctgctgatcctgctgctgtcgataccgtgcctggttccaggtctttacggagtgccgcaggtcgtcggggtggccatactgatcctggcgtttcagcttctgctcgggcgtgaagagccgtggctgccgcgctggttgctgaacctgcgcgccaagggcaagtggctgaaggccatggcggacttcgccgaaagcaagctcagctggatcgaccgcctgtcgcggccgcgaatgcgccgcttcgcctgcggcctgggcgagaagctggcggcggtcttcatgatcctggccaccctgaccatcatcatccccttcaccaacaccgtgccctcggtcgcgctggcgctgctgtcggtggggctgatccagcgcgacggcctgttcgtgctgggcggaaccgcggtggccagcgcctggctgctgttccttggggcgttggcgaccggggctctgatgggggcgggctgggcgacccagctgatccccggcggcgcctgacccctctcgcgggcaggtgatcgcggctcgccttggcgaagcgggcgagcgcgactagtttccgctgcaaccggccggcaaggcctcaccgcattaggcaggacacgctcatgaccgacatcacccagacggacgccgcccgcatcgaccaggagaacccgctcggcgtcgacggcttcgagttcgtggaattcaccggacctgacccgaaggcgatgcaggaccgcctggaggccatgggctttgtcgccacccatgttcatccgaccaccgacgtggtgcggctcaagcagggcgacatctcctttctggtgcaccggtcggcgaagggtcaggcggccgccttcgccggggatcatggcccgtcggccaacggcatggccttccgcgtcgaggacgccaaggccgcctatgaaggcgcgcttcagcggggcgccgtggcggcgccggacgcgcagggcggggcgctgggcgaccacccgtatatccttcagggcatcggcggctcgctgctctatctgatcgaccgatatggcgacgcgggctcgatctacgatggctggaccgagatcgagggatggcgcgagacggcggcgaagaacggcgtgggcctggaggttctcgaccacctgactcacaacgtccgtcgcggccagatgcggacctggtccggcttctacaactcgatcttcaacttcgaggagcagaagtatttcgacatcaagggcaaggcgaccggcctgttctcgcaggccatgatcgcacccgaccgcgccatccgcattccgctcaacgaaagccaggacgacaactcccagatcgaggagttcatccgccgctacaacggcgaaggcatccagcacatcgccctgaccaccgagaacatcttcgagacggtggaggcgatgcgggcgcgcggcgtcgagtttcaagacaccatcgagacctacttcgaactgatcgacaagcgcctgccgaaccatggcgaggacgtggagcggatgcgcaagaaccgcatcctgatcgacggctcggacgaagagggcctcttgctgcagatcttcaccgccgacgtgttcgggccgatcttcttcgagatcatccagcgcaagggcaacgagggcttcggcaatggcaacttccaggccctgttcgactccatcgaactggatcagatccgtcgcggcgtgatcaaggtcgaggcctgatgaaccggcggccgccggcctggctgccctggctcgggccgctgctggcggccggcgccggggggctggcgggcgaatactggctgggcggcggcttctgggtggtgctgatcgccgccctcgtctgcggcttcgcccccattgtcgcctacaaggtgtggaagcggctgcatcatcgttcctgacgcgagacttctcatgcgccctttcctgcccgccgcggccgctctgctgtccgccctctgcacgccggcatggtcacaggatgcgccgcgctggtccctggccatccatggcggcgccggcgtgatcgagcgcggcagcctgacgcccgaacaggacgccgcctatcgcgcggcgttgaacacggcgctgaaggccggatcggctgttctggcgcggggcggctcggccatggacgcggtggaggcggcgatccgcgtcatggaggacgacccgctgttcaacgccgggcgcggcgccgtcttcaccgccgagggtcgcaacgaattggacgccgccgtcatggatggaagcgacctggccgccggagccgtcgccggcctgaccaccacccgtcatccgatcaccgccgcccgcgcggtcaaggagcggtcgccccacgtcatgctggtcggccagagcgccgacgccttcgccgcctctgtgggactcgagcaggtgaatccggccttcttcttcaccgaacgtcgctggcgcggactggtcgagacgctgacggaaagcggtcagcccatcccaccccgtccgacgggcgcgccgtcgcctgagcagaccgctcccaccgcatcccttgcggagccgccgctgaacgaacgcaagttcggcacggtgggggcagtggccctcgacagccaggggcggctggcggccggcacctcgaccggcggcatgacggccaagcgctggggtcgggtcggggacgtgccggtgatcggcgccgggacctacgcctccaacgccgacggctgcgcggtctccgcgaccggctcgggcgaatacttcatccgctccaccgtggcccgcgacatctgccaccgcacggcgggcggcgcctccgtccagtcggcggccgaggccgagatcgcggaggtgggctcgatcggcggggacggcggcgtcatcgtcatgggcgcggacggcgtctcggccttcgccatgaacacgtcgggcatgtaccggggctcggtcgcctcctcgcggccgccggtcgtcgccatctatgcggatgaggcgcggtgagcgacgagctcgagaccatggcggcggaagagctggacgccgcctgcgccatgcccttcgccgacatccgcaagatcacgccttggggcgacagcttcaccggcttcctgccgtccggccgggaggtggaggtggcccgccgttacctctgggcgcatgagccggaaggcggcgtcatcgtggaggtcgaggtccacgacccggagacccgcaccgggcacgaggcgcgcgcgctcctgaccgaacctcgatccgaataggccttgccagcgcaaacggcgggcgtaggctccgccccgtcacgctcttggggggagagaaagccatgacgccgcagcaggtcctgcccgtgctgatcccgatgctggtcgtcgggttgatcgtgctgaaaagccggggcgcgccgcgcaccctgcgcccgcagttcatgtgggtcatgccggctgtggtcctgcctctgatcggcatgggcctgttcttcacgccgcatcagccgttcggcccggtcgcatggctggcgttcgctgcggccctcgcgctaggcgccgccttcggctggtggcgcggcaagacggtgacgatccagaaaacgcccgacggcgtgctgaaggccaaggcttcgccgctcggcgtgatcgtgctggtggccctgctggcgggccgcacggtcttgcggggctttctggaaacccacgccgccggctggcatgtcgatgcggcggtgttcaccgacgcctttcttctgttcgcggtaggcctgatcgtggcccagcgcctggagatgtacattcgcgcccgccgcgtcatggccggcgaacccgacagccacctggccgccgtcgccctacaccgttccgcttgaaaagcggtccgccgcgcgctaggccgtcacctgcctcacggctcgcgggcgtggtggaattggtagacgcgccggactcaaaatccggttccgaaaggagtgtcggttcgaccccgaccgcccgcaccatcggctcggccgcacgccctgaacgcaggaaggcgcgccagtcccagcggccacagcagatcgccccgcttcagcaggacatgacaggccagaggcgccaacacgccggcggtcgtgcccaagacaaggtcggcagggaggggcatccgtacgccggcctgctccagcgcgatccgtaggccgctcgccgccagaatgtgcagcacatagatcgtcatggaggcccggcccaacgccgccgcgccttgaagcaccggacccttcagcacctgaccgagcagcagcacggccgcgccgcctgagagcgcgcatggcaggagccagggcgagcgggcatcgccctgcgccagacccacaagccacagcagcccagccgcgaagacacccgccgccaaggctgcgccgcctgccgcctggccgctgcgccagcgccatgccttgagccccggcccaacagccacgcccgccccatagaacaaggcgccgtgcagcaggccgcgccacaagccctgatggggcgcaaggccgatgctcgccgcgaacgccgccgcgccgaccgtcaagagccatcgcgtccgaccgcccgtcagcacagcgacgccgtgcagcaccgccagcgcatacaggaaccagaactgtccgatcggggcccagccgatgcgcagcagatcgctccatgcccgctcgccgttggtcgcgcccgccgccagcgccgccgccgatccctgaaccaccgaccacagcagatagggccagaccaccgtccacagcttgtcgcccacgaagcctcgtgcgcctcgcgccagcgccgcgcgcacgttcagccccgccagaaagaagaacaggggcatgtggaagctgtagagcgccagatcggccgccccgacccaggccgcgcccaccgcttcaccggcggcctccagcccccgcaggacatggccgaacaccaccacgacgatggccaggccccgcgccgcgtccagccattcgatgcgctgcgcggccggcgtcggcgtcaccggacgcaggcctccggccgcgtctcgcccggtccccacttgtcgcaggcccatgcgatgtgttcgcggatcagggcgcaaggattcgccgcgttgcagggcggatgggtcgcgggactgacgttgcggcagcgctggaccagccgcgtcgccgccgcctctccgatctcgctccggcacggcgtctctccggcggggacgcgcaccggccgcatgtccggcccttcggggatggtcgcctgcggctcagggccggcgttcggctcgccgagctgaggcgcacagccgatcagcatcgccgccagtcccgcgatcaccgctcgccgcatcgtccgccccccagcgtcactcagggccacagtggccgcatcgcccgcgccaggtaaaggggctcagcggccgagcgccgcccgctgcagcgcgaacagttccgcgcagccgctctcggccagggcgaacagccggtcgaactcggtgcgggagaagccgcgcttctcgccggtcgcttggatctccacgatctggcccgctccggtcagcacgaagttgctgtccgcctcggcgttggaatcctcttcgtagtcgagatccagcaccggcttgtcctggaacaccccgcacgacaccgccgccacttggtccaggatcgggtcgctcttcagcacgccctcgtcgcgcaggtagccgagcgccgaggccatggcgacccaggcgccggtgatggccgccgtgcgcgtaccgccgtcggcctggatcacgtcgcagtccagcaccacctgccgttcacccagcgccttcaggtcaaccacagctcgcaaggaacggccgatcagccgctggatttcctgcgtgcggcccgactgctttccgaccgccgcctcgcgccgtccccgcgtgtgggtggctcggggcagcatgccgtactcggcggtgacccagccctggcccttgccgcgcatccatcccgggatgctttcctccaccgaggcggtcaccagcacccgggtgtggccgaacgacaccaggcacgagccctcggcgtagcggttgacgcccagctccagcgtgacggggcgaagctgttcgggcgtgcgttcggacgggcgcatgtggaaatccttggaagcggcggcggcgctgcttatcctgaaagcgtgagcctgtatgccccccagccctcgcctttcgcggacggcgccggtttcgccggcctgaccgggctggacctgcgcgcgcgcgacatctttcgccgcatcgtggaaagctatctggagaccggcgagcccgtgggctccaagaccctgtcgatggggggcgtcgccctgtcgccggcctcgatccgcaacaccatgcaggcgttgacgctggcgggcctgctcgcctcgccgcacacctccgccgggcgcatcccgacgcatgcgggcctgcgcctgttcgtggacggcctgctgcaggtcggcgacctgggcgaggaagagcggcacgagatcgacagccgcctcgccggacgagggcgaagtttcgaggccgccctggacgaggcctccaacctgctgtcgggtctggccggaggcgctggcgtggtgtccagccccgtgcgcgacgcgggcgtcaagcacgtggagttcttggcgttgggccaggaccaggcgctggcggtgatcgtcgccgacgacggcacggtcgagaaccgcatcatgagcctgtcggcgggcgtcacgccgtcgaccttgcaggaagcttcgaacttcctgaacgcccggctgcgcggccgcccgttcgccgacgcccggcgggagatggcgcgtgaactggagatcgcccgctcggaactggaccagaccgccgcccgcctggtggaagacggcctggccgcctggtcaggcggccccgaccgcgagcgcgccctgatcgtgcgcggccgcgccaacctgctgcaggatcgcgaaggcctcgcggacctcgagcgcgtgcgcgtcctgttcgacgacctggagcagaaggagcagttgatcggcctgctcgatggagtcgatgcggcgcagggcgtgcgcatcttcatcggcgcggagacgcggctgttttcgctttcgggttccgccgtgatcgcggcgccctatatgtcgggccgccagcgggtgctgggcgccatcggcgtaatcggccccgcgcgactgaactatgcccgagtgatcccgttggtggactacaccgcccgggtgctggggcgaatgctggacggaaacgacacgtgagcgacacagacttcaacgccaagcccaccgaactggacgccgacgaggctgagatgaacgccgaggccggcctgaacgccgacccgtccgacgccctggcgccgctcgaccaggtcatcgccgagcgcgacgactggaaggaccgcgccctgcgcgtggccgccgagatggagaacctgaagcggcgctccgagacgcagcagaacgacgcccgcgccttcgcgatccagcgcttcgcccgcgacctgctgggcgtggccgacaatcttgagcgcgcgctgcaggcggccccaaaggacgccgagggtcccgccgccggcctggtgaccgggctggagatgacgcagaagtcgctgctgcaggcctttgagagcaatgggctgaagcgcctggcgcccgccgcgggcgatacttttgatcccaacttccaccaggccatgctggagcagccgtcggacaccgtacccggcggctcggtcatccagaccatgcaggcgggcttcgagctgttcggccgcacgatccgtcccgcaatggtggtggtcgccgccaagggatcaggcgccaggccgggcggcgcctatacggctccgcccgcgcaggacggtcaagccttcgacgggaaggcctgacagcagcgcttagaacgcccgccgccaggcgccgatcagggagaaacccggtctggcgccggcgatgtgctggggctcgcggctggcgatcccctgcaccgtcaccgtggatccgtccgccagccgccgctcgcccgccagcgtcagatcgatctgacgaccgctaggcgccgcggaaaagcgtcgctgggaaaaggtcagcgggtcgaagtagtccagcggcacgtcggccagcagcgccgtcagttcgccgtgctcgatccgcagcggctggcccagcgacagggtgacccggtcgcacagcaggctccagcccttgcagccggcagcggcgccgaagcgccaggccaggctggtcgccgccccgtccgtaccgatcaaccgcccctcgatctccgtgcggcccaggctggcctctccgaacagcccgacgcgagggctgaccgcccagtcgccggccagggcgtagaagcgcgtgcgcgacggcagcgccatgtccgaggtcgacggcatccatgcgccgagcggccccagccgttcgtccagcccgccgaggcccaggctgacgccgctggtgcggccacgccacgccagcatggcccgcgaataggaagaggcttcgtcctcgacccgctgcagcggcatgcgacggtcgcccatgccggcttcggccgaaagggacaggccaagccccagccgcacgccgccctgcaccgcgcggtcagcctgcgccagggcggcgaaaccgtcgcccgcgccgtccccaaacggcgaggcggcgccgccttccccctgccagacgttcagttgcaggcgaccggcctcgatcccgaccatggcctcgcgccgcacgtcgtcgtcgcgccagggcgtctcaagcaggttgcgtcgcggcatgatcggttcaggcgtcgggaccggctgggccgccaccaggttcaggcgcaccgatcccggccccacaaggctgacgctcgcctgctgactgggctcataagggcgcggctgcaccgacgggcgcggcgcggtcggatatgccgaacccagctgcacctggaacagccggttataggcgtcataggcgaccgtggtcagcgcgtcctgccggccgaaggcgtcgccgaacgccgcgccgacgaacgatccgggactggcctccgccaccacgcttgcgccgctggcggttggggtggcggtcgcgcccaccggctgaaacgcccgcgtcaggtccagcaggccccggccgtagaccacgtccgtgccgggatcgcccgcgtcccgcgccgtgtcgaacagaatgcgcacggcctgctggccggtcaggttcggaaaggcgtccagcagcagggccacggcccccgacacgtggggcgccgagaacgacgtgccgttggcgcggtagcagatggagccgtcacagccggtgatgatgtcgctgcccggcgctgaaaggtagcccgcggcggccacccccgccttgttggagaagtcggacatcacatcctgcgcagtgtgcgatccgaccgcgatcacccggccgccgtagcgggagtccacggcgtatcgcgccggccagccgggattgtcctcgctgtcgttgccggaggaggcgaccaccacgatccccgcgttggtggcgcgcagcagggccgcctcgaaggccgtccccagccggccgtctccgcccagcgacatgttgatgacgcgcgcgccgttggcgacggcatagtccagcgcccgcaccaggtccgcgctgccgaagcagaactcgttctcgtcgtcctcgcactcgttgatgtctgcgcggatcgacaggatggtcgaccggtaggccacgccgatcgtaccgaaaccgttgaagttggaggcgatgacgcccgacaccagggtgccgtgattgtccggcccctccggctggttgcggccgggaaccacgtcggtcgaggcgctggagatgcgccccaccaggtcggcctgatcgaagtcgatgccgtcgtccacaacggcgacggtgatcccctcgcccgtggcgccaacgttccaagccgcctgagcccggatgttcgccaagccgtaattgcgcccgtactcggccgaactcgtggaaggcggcggaggcggaggcggcggcggagaggcggtggtggaggagggtggtggaaccggtggcgtcagcgcgcccccgcctgatccaccgccgcctccaccccgccgcatgcggccagcggcaggaacagcagcgccgcgcccatcatccaggcggctctcgggcgcgttctcgccagctttgccatcatgtcctcgaaaagcgacttcgcggacacaatgcccgccagaggttgcctcgagatttcaacgtcttggtcaaaagcgcaagcccacgcgcgcactatgccgccgacgacccggcgcgcctcagcgtcaggttcagccgcccgcctccgggcaacaggctggacgaccccgtaagcacgcggtcgatcccgtggcgggccagccgcgccggacccgtcagggcgcagatgtcgccgctttccagcttcagcgaggtggtgcgtcctccctgctctggcccgatgcggaacaccgccgcgtccccgagggagaccgacagcaccggcgccatgaggtccgcttcgtcgcggtcctgatgcagccccatgcgcgcaccctccccgtacagattgaccaggcaggcgtccggcggctccggccagccggtcgccgtgtcccagagctccatcagcatgggcgggatcgccggccagagctcgcccgtgacgggatgatgcggctggtaacgatagccgccgcggtccgacacccaccccagggggccgaagttggtcatctggacagagaaaggccgcccgcccggcgtggtcggccgatacaagggagcccgcgctatcccagcctcgacctgcgccagcagggcgcgctgccgatcctgagacaaggcgtccttccacaggcgaaagccgtccatcgccgtgggcgtctcgtgcaggcaaaggcgttcggatgcgtccaccccgccgatatagcgcgcctgcactccgcatgcgcccgtctcggctcttgcagccccccggcctcttcccatatcggggccaatccggagaaaccccgcaacgcttggggctatccgggaaacaccaaacgccaacccacatgggggcggtcaagcgcggcgcttcttcagcaaggccgccgcatcgcccgccgcaacggagactagaccaagctcatggccaagatcatcggcatcgacctcggcaccaccaactcctgcgtcgccgtcatggacggcaagaatcccaaggtcatcgaaaacgccgaaggcgcccgcaccaccccgtcggtggtcgcccttcaggacggcggcgagaccctggtcggccagccggcgcgtcgccaggcggtgaccaacccggccaacacctttttcgcgatcaagcgcctgatcggccgcaacttcgacgacccgatcgtggccaaggacaagggcatggtgccctatgacatcgtcaagggcccgaacggcgacgcctgggtgcgcgcccacggcaaggactattcgccccaacagatctcggccttcaccctgaccaagatgaaggaagccgccgaagcctacctcggcgaaaaagtcacgcaggcggttatcaccgttccggcctacttcaacgactcccagcgtcaggccactaaggacgccggcaagatcgccggtctggaagttctgcgcatcatcaacgagccgaccgcggccgcgctggcctatggtctcgaaaagaacgacggccagaagatcgcggtctacgatctgggcggcggcacctttgacgtgtcgatcctggagatcggcgacggcgtgttcgaggtgaagtcgaccaacggcgacaccttcctgggcggcgaagacttcgacgtgcgcctggccgactatctggccgacgagttcaagaaggagcagggcgtcgacctgcgccaggacaaactggccctgcagcgtctgcgcgaagaggccgaaaaggcgaagaaggaactgtcctcgaccacccagtacgaggtcaacctgccgttcatcaccatgaacgcctcgggcccgctgcacctgaacatcaagctgtcgcgcgccaagctggaggccttggtcgacgacctggtccagcgcaccatcgagccgtgcaagaaggccctggccgacgccggcctgaaggcttcggacatcgacgaagtggtgctggtcggcggcatgacccgcatgcccaaggtgcaggaggccgtgaaggccttcttcggcaaggagccgcacaagggcgtgaaccccgacgaagtcgtggcgctgggcgctgcggtgcaggccggcgtgctgcagggcgacgtcaaggacgtgctgctgctggacgtgaccccgctgaccctgggcatcgagaccctgggcggcgtcttcaccccgctgatcgagcgcaacaccaccattccgaccaagaagtcccaggtcttctccaccgccgacgacaaccagaacgcggtgacgatccgggtcttccagggcgagcgccccatggcgtcggacaacaagatgctgggccagttcgacctgatgggcatcccgccggcgccgcgcggcatgccgcagatcgaggtcgccttcgacatcgacgccaacggcatcgtcaacgtctcggccaaggacaaggcgaccaacaaggagcagtcgatccgaatccaggcgaacggcggcctgtcggacgccgacatcgacaagatggtcaaggaagccgaggccaacgccgccgccgacaagacccgcaaggacctggtggaggcccagaacggcgccgacagcctgatccactcgaccgagaaggcgctggccgagcacggcgacaaggtctcggccgacgacaagacggcgatcgagaccggcctggccgagctgaagaccgcgcgcgacggcaccgatccggaagacatccgcgccaagaccaacaccctggtccaggcctcgatgaagctgggcgaagccatgtatgcggcccagcagggctcgggcgacgccggtgcggctcaaccggccgacgacggcgtggtcgacgccgagttcgaggaagtgtcggactccgacgacaagaagagcgcctgatccgcaacaggtcgctgaaatgatggggccccgcttgtcacacgataggcggggccctttcatgaaggttgcatcacacgccccggcgcccatctcagccgggacggaaaaacccgtgtcggccggcgctcgatcagaggcgcggccgcgggttcgccgagaaacgaaaagggaccaacgccagatggcgcgtgactattacgaggttctgggcgtcgagcgcacgatcgacgcgcccggtctgaaggccgcctatcgcaagctggccatgacccaccaccccgaccgcaacggcggctcggaagagtcggtgacccgcttcaaggagatatcggaggcttactcggtcctctcggacgaccagaagcgcgcggcctacgaccggttcggccatgcgggcgtgaacggcggcgcgggcggcggcttcggcggcggccagcagggcttttccgacatcaacgacatcttctcccaggtgttcggcgacgccttcggggacgcgttcggcggtcgccagaaccgcagccagggcggtccgcgtcgcggctccgacctgcgctacgacctcgagataaccctggaggaggcgtatcgcggcgccgagcgggaaatctccattccctccaccgcgacctgcgacgtctgcgagggctcaggcgccaagccgggcgccaaggccacgagttgccagacctgccacggcgccggacgcgtgcgccaggccaacggcttcttccaggtcgagcgcacctgtccgtcctgcggcggcgccggtcagaagatcgcccaggccgacgtctgcaccgcctgtcacggccatggccaggtccgcaagacccgcacgctcagcctgaaggtgccggccggcgtcgacgacggctcgcgcatccggctgtcgggcgaaggcgacgccggccagcgcggcggcccgcgcggcgacctgtacgtcttcctgtcagtccagccgcacgagctgtttgaacgcgacaatctggacctgctggtcaccgtgccggtgccgatgacggtggccgcgctgggcggcgagatcgacgccccctgcctggtgtccgaagcgtgtgacggcaactgcaaggcgggcgtaaccgtgccggccggcgcccagaccggcaagaccgtgcgcatcaagggcaagggcatgccgcacctgaacggtcgcgcgcgtggcgatctggtggtcgagctgttcgtggagacgccgaccgagctgaccgcccgccagaaggagctgatgcaggagcttgcgcagtccttcggcgaggcgcagaacccgcgcaactccagctttgctggaaaggccaaacgcttctgggccgacatcctgggcaatcaggacgcggacggatcgagagagaacgcataagcgcatgttccacgccggcatctccggcgcccggggccggatgggccgcgcggtgtcccaggtccttgatgcgcgcagcgacgtggtcgtctcggcgcgcttcgactggggcgagacggcggacctgtcgctgtgcgacgtggtgatcgacttctcgacgcccgaggcgtcggtcgatctggcgcggcgggcggcggaacagggtgcgccggcgctggtgatcggctcgaccggcttttcgcccgagcaggaggccgaactggacagggcggccgagcgcatcgccatcgtcaagagcggcaacttctccctgggcgtgaacatcctgatcggcctggtggagcacgccgccatgcggctggacgccgccgactgggacatcgagatcgccgaggcccatcatcgccgcaaggtcgatgcgccgtccggcaccgcccttatgctgggcgaagccgccgccgcaggccgtggggccgatctggaggacctgcgcaccgctccctacgacggcgtgggcgccgagcgcgaggcgggcaaaatcggcttctccacgacccgtgcgggcgggatcgtgggcgagcacaccgtgctgttcgcctccgaagacgaggtcctgacgctcagccattcggccatcgaccgcagcctgttcgccaagggcgcggtggtcgccgccgcctgggtgcgctcgcgtcgtcccggcctctacgacatgcaggacgtgctgggctttcgtcaggcctgagccttacctcagccgccgacgccggccgggtccccgccccaccggcgcgccggtcagcaccgacttcaacacaaagaagatggcgatcacgatcagatagcccaggaacagcgccgccgcgccgatccagaattcgcccgacagaacgggcggcaaggcgaacgatccgccgcgcgccagcggcagcatggccagaaacagcaggtgcaccaccacggcgcccaccgccgagaccggcagccgccgccacgacgacgtcatcagcgccgcggccagcgcgatcaccaggcccagagcctggttgaccccgtcgaacccggcgcccgccagagagaagacgccgctcagcgcgtcggtgatcccgtccaccagagcctccatcgcctatcgtcccgtcgaaccgaagccgctcgagccgcgcgcagtctgatccagcgcctcgacctcgacccactcggcgcgctcgtgccgggcgatgaccagctgtgcgattcgctcgccacgccggatcacgaagggctccgagccgatgttggccaggatcactccgacttcgccgcgatagtcgctgtccaccgttccgggcgcgttcgggcagatgatcccatgcttcagcgccagcccggatcgcgcccgcacctgcgcctcgaaccccgactgcagcgcgatgcggaagccggtcggaaccagcacccgcccgcccggctccagcaccagcggctgatcgtccgccaccgccgcccgcaggtccatgccggccgagccgtccgtctcataggccggaagcggcagcccctcgccatgcggcaggcgttccagctggacagcggtcatcggtcttccttcagatgttcgacgatgcggccgaccagcgcccgcgcgatctcgaccttggactggcgcggccaggtctccgccccgtccgccgtgaccagcgtcacggcgttgccgtccgagccgaacacgtcttcggacacgtcgttgcccacgatccagtcgcagcccttcctcgacagcttggcgcgcgcgttggcctccaggtcccctgtctcggcggcgaagccgatcaccagcgccggacgccgcggccccggcgccgcgacgcccttcaggatgtcggggttctcgatcagatcaaacgtcggcggcccgcccggtcccttcttgatcttgccgcccgcgatggtgtcctcgcgccagtcggccacggcggcggacagcacggcgacgtcggccggcagcgccgccacaaccgcccccttcatctccagcgccgtttcaacgtcgacacgccgcacgccggcaggcgccgccagcgccgtcggccccgacaccagcgtcacctcgcacccctggtccgccagcgcccgggcgatcgcatagccttgcttgccgctggagcgattggtcaggccgcgcaccggatcgatgggctcgaacgtcggaccggcagtgattaccgcgcgtcgcccctcaagcggccgctcgcccccgatcagatcgacgatggcctgaagtatcgccggcggctcggccagccggccgggcccgtattcgccgcacgccatctcgccctcgtccggcccgacaacggccgcgccgtggaagccgggaaagccgcgcagccgcgccatgttcgcctcaaccgccggatgctcccacatgcgcacgttcatcgccggcgcccacagcacccgcttgtcggtggcgatcagggtggtggaggccaggtcgtccgccaggccattcgccgcacgcgcgatcaggctcgccgtcgccggcgccacgaccaccagatcggcccagcgcgacagttcgatatggcccatggtggattcgtcgtcgggcaggaacaggctctgacgcacaggatggccgctcagcgccgccagcgacagcggcgttacgaactccgcggcggccgctgtcaggatcacccgcaccgctccgcccgccttgcggatcagccgcaccagctccagcgacttgtaggccgcgatcccgccgcccacgatcagcagcaccttgcggtcggaaagcgggagggcggtcatgttctcctctctagacgggccgaccccgccgcgcaaaagaacattgccggaacgcgcaagctgtgcctaacctcgttcggcgggtcaggacagggagagggatcatgaccattcggatcgcggcgctggcgcttgcgggactgggactgctgggtcttgcggcctgcggggaggcctcagcggtggagacgcgggagcgcccgatgcaggccgcatccttggacggcgtctcgggatcgaagcccatggatgcggtcgcggctgccgaaccggccgagaagccggccgtcacctcgacgcgcaacgagaccgccgacgccaaggtgacgcgtctgtacgagcgcaacggctcggccttcggcgccaagtcggccgaggactacgccgacaagatcgaggccttcacccgccgcccgcccaaggacgccgagacggtgaagcgcgccaacggcgacaccctgatctatcaggcgtccaccaacaccttcgccgtggtcgcccgcaacggcacgccgcgcaccatgttcaagccggacgatggtcccgcctactgggcgcagcagaaggagcgggcgcccaccttcggccagcgccggtcctccagccgcgacgagggctgacgcagcctccggcaaggcgtaaagcggcgggatgacgcacgtcccgccctcgcctcgccgcccgctgaagaccgccctgatctatgacttcgacgggacgctggcgcgcggcaacatgcaggaggtcagcttcatcccctcggtcgggatgggcatcggcgacttctggaacgaggccgaacgcctgacccaggccgccgacggcgacggcatcctgatgtacatgcagctgatgctgcaccacgcccgccagaacggcgcgccgatcacacgcgagaccctgcgggaccacggccgcgaggtggcgctgttcgaaggcttgaaggacctttcctggttcgagcggatgaacgccttcggcgcccgctacgatctggacatcgaacattacatcgtctcggccggcctggaggagatgatcgagggcacgccgatccggcccgccctgacccacgtcttcgcctcccactacgtctatgacgacaagggcgaagcggcctggccggcggtgggcgtcaactacaccaccaagacccagtacctgttccgcatcaacaagggggtgcgcaaccactgggagcacgagcgcatcaaccacttcattcccgacgacgagcggccgatcccgttcgaccggatgatcttcatcggcgacggcgacaccgacgtgccgaccatgaagatgatgcacaccaagggcggcttctccatcgccgtctatgatccgcgatccaacgagcgggaccagaaaaaggtctacagcctgatctccgaggaccgggtcaacttcgtcgccgccgccgactaccgcgagggctcggctctggacctgatcgtcaaggggctgatcgggcgcatcgccatcaacgcgggggcgatgccgtcggacgcgcgttgacccgcccggggctttccgctatagccgcgcgctcttgagatttccgcgccgtggacaggtggtctgcggcgtttccgcatcataggtttgacgatggccaacaaccccggcgcccgcaaggcgatccgcaagatcgaagcccggacccaggtgaacaaggcacgccgttcgcgcgtccgcacctacctgcgcaagttccaggaagccgtgacgggcggcgacgccgacaccgccaaggccgccttcatcgaggcccagtcggaactgatgcgcgccgtgtccaagggcgtggtccacaagaacaccggctcgcgcaaggtctcgcgcctggccgcccagctgaagaagatgtcggccgcggcctgacgccttctcggggcgcggtcgcctcaacctgcagacgtttgaaaccggcggtcgcccctgcggccgccggttttcctattgggcggtggttccgccgtcgatcttgaactcggccccggtcacgaagcggctctcgtccgacgccagatagagcacgcaataggccacgtcgtccggctctccgatccgcttcagcggaatgccgcgcgccagccgctcgtgcgccttggcctcatcgccgccggccatggcggtgaagggatcaaggatgggcgttcggatgaacaccggatgcaccgagttgcagcgcacgttccagtcgttcttggccgcctccagcgccaccgtcttggtgtacatccacacacccgccttggtcgcgttgtaggcccccatgccgggcgccgcgaccagtccggccagcgacgagatgttgacgatggaggccggcgccgccgccctcagatgcggcatggcgtgcttgcagcccagcatcactgagcgcaggttgatctcgaactgccgctgccaattctcgaccgtgtcgtcctcggcgaaggccagaggcccgcccacgcccgcattgttgaccagcaccgacaggccgcccagatcgcgcgccgccacctccaccacccgcgcccagtcctcctcacagcgcacgtcgtgggcgtaggcgaccgccgcgtccgcgatctcgtcgttgatcgcctgcgccagtcgttcggccgccgcgccgtcgacgtcgctgatcgccaggcgggtgccctcgcgcgccatcatccaggccatggcctgacccagcccgcccgcgccgccggtgatcaggacgcgcttgccggcgacccggccgctcattcgcgcacgccggcggccagcgcagcctcgtcgatgaagcgggccatgcgaacgtccctgtccgtcaccccgcccgcgtcatgcgtggtcaagagcacctcgacccggttgtagacgttggaccactccggatgatggtccattttctcggccagcagggccacgcggctcatgaagccgaaggccgcgttgaagtcggcgaagcgcagcgaacgcgtgatcgccggacggtcgccatcatgcacgctccaggcgggaagctgcgccagcgcctgctccagctcaattctcgcgtcggtcatggcggttcctcccggcctgtttcgcaaaggcctagcccgcatcgccccaagcgccaagcctgatggcgcatggggccaaacgtccggatgacggcggggcggcgagcggctaaacccctctgcatgagcgacgccgcccctccccctcccggccccgacgccgcgccctcgggcaagacctcgtccttcggcttccgagacgtggatgcgcgcgaaaaggtgcgcatggtgcgcggcgtgttcgattccgtcgcctccaactacgacctgatgaacgacctgatgagcgcaggcgtccaccggttgtggaaggacgccgccgccgccaagctgaacccccgccccggcgagaccatcctggacgtggccggcggcaccggcgacatggcccgccgttactccaggatggcgcgcgcggcgcaggagcggcgcggcggcggcgacgcctccgtgatcgtgctggactacaacgccgaaatgatcctgaacggggtgcagaagggcggcgagcccgagatgcagtggaccgtcggcgacgccatggccctgccgctgcccgacgcgagcgtggacgcctattccatcagcttcggcatccgcaacgtcgccgacatcgaccaggccctgcgcgaggcgcggcgcgtgctgaagcctggcggtcgcttcctgtgcctggagttctcgcgccccacgaccggcgtggtccgccgcgcctatgacgcctggtcgttcaacgccattccgcgcatcggccagtgggtcgccaaggatcgcgacagctaccagtatctggtcgaaagcatccgtcgctttccggatcaggcgaccttcaaggtcatgatcgagcaggccggcttcagccgagtctcggtgaccaacctgtccggcggcgtggcggcgatccatcacggatgggccgtctgaccccgcgcccgccctaccgcaccgcgccggagccgccgccggccatgccggtgaacgatccggtcgggtcgctgctgcggctgatcggctggctgtgggtgctggttcgccatgacgccctgatcccgcgcgaggccacgccgctgctgccccgctgggcgcggccgctcgcccgcttcatccagatgttcgccacgcgcgaaggcaagctgggccgccccggcgagcgcgtcggcaaggcgttcgagcacctggggccggtcgccatcaagctgggtcaggtcctggccacgcgcgccgacatcttcggcatccagttcgctcgcgacctcggccggctcaaggaccgcctgccgcccttcccgctggaggaagcgcggcgagagatcgagcgttcgctgggccgtccggccgaggcgctgttcatcgactttggccagccggtcgccgccgcctcgctggcgcaggctcatccggcgcatctggcggacgggcggcgcgtggcggtcaaggtgctgcgccccggtgtcgagcggcgggtgacccagggactggacgccatgcggctggcggcgcgcctggtgcaccgcctgatccccatggcgcgccgcctcgagcccgaagcctttgtggagaccatcgcccgctcgctggagctcgaactcgacatgcggctggaggccgccgccgcctccgagatggccgaggtcatggccaaggacggctacatgtcggcgcccgccgtggtgtgggacggcgtcggcaagcgcgttctgacgctggagtgggcgcccggtacgcccatgaccgatccggcgctggtggacctgcccgagctcgacaaggatcaactggccgacaatgtggtgcgcgcctttctggtccaggcgctggatcacggcgctttccacgccgacctgcacgagggcaatctgttcgccaatgcgcccgcgcacctgaccgccatcgacttcggcatcgtcgggcggctgggcccggccgagcggcgctaccttgccgaaatcctgtggggcttcatcagccgggactacgaccgtatcgcccgggtgcatttcgaggccggctatgttccgccgcaccactcggtcgaggcgtttgcgcaggcgctgcgcgctgtgggcgagccggtgatcggccgcgcggccagtcaggtgtccatgggccggctgctgggccagttgttcgagatcacagccctgttcgacatgcatctgcggcccgagctgatcctgctgcagaagaccatggtgtctgtcgagggcgtggcgcgccggctgaacccggaccacgacctgtggaaggccgcccagccggtggtcgagcgctggatccgccgggagctgggtccgcaggcacaggcgcgcgatgcgttccaggacgtgctggccgccgcccgcgccctctcgcgccgtatccaggaggagccggaggtccgcaccgtggtcatcgaaaagccccgaaccgcgccttggctggcggcctgcgtgatcgtggcgaccgtcgcctcgctcggcgccttcgccctggccctgtggccgcacctgtcctgaccgccggagccgaaatgaagaccctgctgatcgccgccgccctgctcgccgcgcccctgccggtcctggcccaaagcgtggccgccggaaccgtgcccaacagcttcgacgcgccccgcgccgcccaagccgtcccgacgctcgcggctccagccgcctcacccgctcaggcgccggacacggcccgcgcggagaccgcgctgcgcgacctgatctcggcggcgcagggaacggggttcgactacagcgacttcacggccgatctcgccacgaagatcagggcgcaggaggcgcaggtcacgcccctgatcaagagcttcggcgcgatcaagacggttgaggcgcgcgggcaggagaacggcgccgacctgttccgcgtcaccttcgacaaccaggtcaccgagtggctgatcggcttcgacgccgaagacaagatcgccctgctgctgttccgcccggccgaaagctgaggcctcagtccagccggggctttccgcgcccgctcttgatgctggagcggctggccttggcgacgaggcgtcgctccttggaagctcgcgtcgggcgggtcggcacccggtaggtcggagcgacggccgccttgtcgaccatggcctgcagccgctcgatcgcatcggcgcggttgcgctcctgggtgcgaaagcgcgtggccgttatgacgatcacgccgtccagcgtcagccgactgcccgccagcttcatcagccgcgcgcgctggcctgcgctcagtgaaggcgagttgcggacgtcgaagcgcatctgaacggcggtcgagaccttgttgacgttctggccgcccggcccgccggcgcggaagaagcggaattccagctcctcctcggggatcggcatcatggccgggcgcgcctggctttcaccaccgcctgatccagcgcctgcaggaagcgcgagcggtcggcgggcccgaacggcggcgggccggaggtcgccacgcccatggagcgcagatgctcgcccaccatgcgcccggccagggccgagccgatgctgtcgggggtgaagggctgtccattggccttgagcgcctgcgccccggccttcaggcatcggtcggccagagggatgtcggcggtgatcaccacatcgcccggggacgcccgctcggcgatccagtcgtcggccacgtcaggcccggcgtccaccaccacctgctcgatcagcggctcaccgcgcgggacctgcatccaggcgttggagaccacgaacaccttgaggccgtagcgtcgcgccacgcgatacacctcctccttcaccgggcaggcgtcggcgtcgatgaagagggtggtcatgagaggggcttagcgcagccgcgccgcaaagagaaagggcgggaccgaagtcccgccccttgggtcgtcagttgcgataggccggcggcatgggcgtcgcttgccgatagcgatcgcgcagcaggaggttgcgggcctccagcggctgctccaccccgttcacgaacaccgccgagggctggctcagcggctccagcggatcgccggaccacaccaccacgtcgccggcggcgcccggcgcgatctggccgaactggcccgccatgccgaagatgcgcgccggattgacggtaatcgcggcgatggccgaggcgtagggcaggccgtgcgacaccgcgttgccggcgttgtagcgggtctcgcgcgcgcggtggaccgagccctcgttgcccttgatggcgatcaccaccccggccgcgtccagcgccgccgcattctccatccgcgcggcgcggacctcgaagttggccggcaggttggaaacggggttcagcagcaccggcacgccggccgccgcgatgtccgaggcgaccagccagccctcctcggccccgtcgaggatcagcttgaccccttcctcgcgccccagccttagcacctgctggatgtcggaggcgcggtgcaccgtgacgatcagcggcatgtcgccattggccaccgggatcagcgcctccaggtccgcacgcgacagcatcaggtcgcgcaggcccgcccgctcataggccgacttgttgcgggcgtagagccgcacctcggccagggtttccttgaacagggtgtattccgcgccccgcgcgccacccgccacgccggcgccggcctcgccgaacggcgccgtcatggcgacgcgcggcttgaccaggatgtcggtccctcgaccgaggtggatcacggccgcccgaccggcgaacaggcccggatcatggtagccgccttcgcccgcgccggcggtgtcgtgctcgtgcacatggccccccgatgagcccggatgctggggcaccaccaccgcgcgggtcacgccgcccagccgcgcaaccggcagggtgaaggaccagggatccagcccgtaggacacgtcgaacgcggcgctgagggtgttggaccggttggccaggtcgttggtcccgccgacggagccgacctccgacccggccaatccggagtccaccgcgacgaagcccggcgccaccaccttgccggcggcgtcgatcacgcgggcgccggcgggcgcgccgccgtggcccaccgacaccacgcggccgtccgagatcaccactgtgccgttctcgaccacggaggttccggtcagcacccggccgccgacgatggcgaccgtttcctgagccaacgcgggcatggccagggcgagcgaggccgcggcgcccatgaggatctgcaagatgcgcatcagcgggctcctccacggacgttggcggcggacaggccgtagcccggctggcccagttcaaagtcgctggtcggctggtaggctggattgctgcggtcgaacgccagggcgccgtcgacgaacacctggtcggcgcgggcgtagaccgagaagggatcggcgctccagatcaccacgtcggcgcgcttcccgggctccagcgatccggtttccttgtcgatgccgatggccttggccgcgttcagggtgaaccagctgacggcgtgctcctcggagatgttaaggcccgcacggcgaccggccgacagggcggcggcggcttcctggttcaggcgctgggtcagttcggcgtcgtccgaatggatcaccgcgcatccgccgggcgccgcatccaccagggccgcattctcctcgatgccgtccagcgcctccatcttgaagccccaccagccggtccagatggccgtgcagatgccggcttccgccagttgcggcgccagcttgtaggcctcggtggcgtggtggaaggtggtgatgcggaagtcgaactcccgcgccagatccatcatcagcgccatctcgtcggcgcgatagcagtggttctggatcaggatggagccgtccagcacgcccgccagcgtctcgttctgcaggttgcgggtcggcggcgagccctcgccgtcctcgcgccacttgtcccacttggccttgtagtcgcgtgcggcgatgaaggcggcgcggtagccggccatgttgcccatgccggtggccgggctctggttgcggccgccgtagacgcgcgacgggttctcgccgcaggccatcttcaccgtagagggcgcgccggggaacttcatgccctgcatggtgatggagggcacgttgcggatggtcacgccgcgcccgccgaacaggttggccgagccgggcaggatgtgcatggtcgtgacgccgcccgcgcgggcggtgttgaagccggggtcctgcggccacagcgaatgctcggcccagacctgggcggtgttcgggctggtggcctcgttgccgtcgctcatgccctgcacgccgggcgacggatagacgccgaggtggctgtgcacgtcgatcaccccgggcgtgacgtagcggccgcgcgcatccaccacccggtggccggccggcgtcggcgtggaggcgtcgcccaccgccgccacgcgaccatcggtgacgatcaccacgccgttctcgatccgggcgcccgttccggtcagcacggtggcgccgacgatggccatgttctcgcgtggcaggggccgataggtcgagggataggggtccggattggcagaggcgtccaggccgggagccagggtctcgcgcgccttatccggctccgcctcgcttgagccgcccgtcgaggcgcaggccgatgcgcccagcacggcgcaggccagggccgcaaggctcgcgccccgcagaacatgtccgatcatcaaagcccctctatctccgccagcccggcgggtcactgaacagtgggggcatagaagcggcaacagccgacgccgtcaaagcgtttccggcgccgcctccccgccgggggcggggaggagcaggaaagatcagtccagcgccttcagcagctcgggcacagcagtcttgtagtcggccacccagccgtagtcggcaatctggaagatcggggcgtcggcgtccttgttgatggcgacgatggtcttggagtccttcatccccgccaagtgctggatagcccccgagatgccgaccgcgatgtagagggcgggcgccaccaccttgccggtctggccgacctggtagtcgttgggggcgtagcccgcgtcgaccgccgcacggctggcgcccacagcggctcccagcttgtccgccaggggctcgatcaccgcatggaactcttccgccgagccgagcgcacgaccgccggagacgatgatcttggcggcgcccagttcggggcggtccgactgaaccttttcctcgccgacaaaggtcgtcttgggggcgtcggcgcccgagacgctttcgaccggggccgagccgccctcttccgccgccttgaaggcggtgggacgcacggtgatcaccttcttggcgtccgaggtctggatcgtctccagcgcattgccggcgtagatcgggcgcacgaaggtgtcgaccgacaccacctcgacgatgtccgagatgggcgccatgtccagcttggccgcgatgcgcggggcgaagttcttgccgtcgttggtcgagggcgacaggatcgcatcatagtcgccggccagcggcagcaccgtcgcctcgaccgcttcggccagggtttggcccaggcccgcgctctcggccagcagaaccctgcgcacgcccgagatcttcgccgcggcgtcggcggcggcctgagcgccctgccccaccaccaggatgtcgatgtcgccgcccagcgcttgcgcggccgtcacggtcttgtgggtggtgtcgcggacggccgaaccgtcgtgatcggcgatgacaagaacggccatcttacagaactcccgcttcgttcttgagcttcatgacgaggtcggcggcgtcggtgaccttgacgccggccgagcgcttggccggctcggtgaccttgaggaccgaaagacgcggcgccagatcgacgccgtagtcggcggcggccttggtcgcgatctcctttttcttggccttcatgatgttgggcagggacgcatagcgcggcgtgttcagccgcaggtccaccgtcaccaccgccggcagggccgcggcgatggtctggaggccgccgtccacctcgcgcgtcaccgtggccttgccgtcggcgatctcgatcttcgaggcgaaggtcgcctgcggccagtccagcagggcggccagcatctgacccaccgcattgttgtcgccgtcgatggactgcttgcccatcagcaccaggtccggctgctcttcgtcgaccaccgccttcagcagcttggcgaccgccagcggctccagatcggaatccgcattgatcaggattccacggtccgcgcccatggccagggcggtgcggatcgtctcctgcgcctgggcgacgccgatggagaccaccacgatctccgacgccgtgccggcggcgtgatgctccttgccttccttcaggcgcacggcctcctcgacggcgatttcgtcaaaggggttcatgctcatcttgacgttggccagatcgacgccggtctgatccgccttcacccgcgccttgacgttgtagtcgatcacccgcttgaccgggacgagtaccttcatgggtttatccgtgaaatcgcctgaatatcgtggcagggacatggagcggcccgccgggcctgtcaacgtaacgccgcgtcaagcccggaggctccgtctggactttggaacggcgatgtggatcggaaaatgaagcgcttcctgacctttccccgcctcagcctgctgttcctggccctgttcggcttgtcggtggcgggcgtgttcgtgctgcagacctattggctcgatcccggcaagcgctgtgaggcggccggcagctggtacgacgtcgaaagccgcacctgcgccaagccgatctacatccccgacatccccggccgccccgccggcgtgacgcgcgcggacgcctcgaacgccaagaaccgggagctgatccagctggaggacgaagtcgcccagcagcagcgcgccttgcgcgaacaggtcgcccgcgaaaaggcccagatcgagaaccggcgggcgcagtagcggctagcgcggcgcgcccggcctccacagcacgtcgccggcgccgttggcgttggcgcgccgggcggccacgaacagatggtcggagagacggttcaggtatcgcaccgcctccgggttcaccgcctcgcccgcctccatcaggcgcatggagtcacgctcggcccggcggcagacggtgcgcgccaggtgaagatgcgccgacaggggcgcgccgccgggcaggatgaagctgtcgagcgacttcaggctctcgttcatccagtcgatctcgctttccagccgatctacctgcgacgagacgatccgcagcgcctcccacttgggcggcggctccagcggcgtggccaggtcggcgccgagatcgaacagctcgttctgaatgcggcccagcatggcgtcgatgcggtcgttctggccgctgtgcagccgggccacgccgatcacggcgttcagctcgtccacggttccataggcctcgacgcgcgggtcgctcttggacacggaagcgcctgacgccagccgggtctctccggcgtcgccggtgcgggtgtagatgcggttcagcaccaccatggatcagcctccgcgtgtcgccttccagaggaggccgcccatcagcaacagcaccgccacggcctggaacatgacccgcagccgcatcaaccggttcgagttcgaccgggcgtaggctccgccgcgatagagcgaatacaggccgaaccccagggtgatcgccaccgccgcgaccgcgaccaggatgatgatgtcgaacgcgtccatggcgaaagctgtaggccgacgatccgacgcacgccagcgcccacgtgacggaacacgggtcggctaagcccttggtcacctttgccgttcatcatgccgcgctcttccccgccaggaccatcatgaccgaccgcgccgtccgcaacctggatcacctgcgtcgctccgcgtcgacggcccgggtgctcaacctgctgcgggtgtgggagctgcatggagacagccgcgacgacggcggcgtgcgcacgcaggagtgggccgagcggccgatgttccgctcccaggcgctgaaccgctccctgatcatcaagcatcgtctccggcgcaacgagttcgacctgttcaccggccgccgacaggtggcgaccaaggtggtggtgccgatcgacgaggccgatctgaagacgggcggtcgctatgtcttcgtcaaccagatcggctttgaacgctcgatcgccgaggcctttggtctgcagccggaccaccccgacctggagaccctgcgcctgatcgaccggctgccgtcgctggatccttttctgctgcgcgaacagctgcgtcgcggcggacaggatcccgccgactgctacttctccatctccgacggcgacctgatgcagatgaccgagttcgtgcgacgccagatcgagccgctggtgacgctgagccttgatgaggacaccgtcgccgtggcctcggactcggccgcccggatggcggccaagatcctttccaacgcccccggcaaccagctggaagccctgcgcgacactctgcggctggcgccggagcagtatcaggagggcgtcttctgctggaaggggttcctctattacaaatggagtctggcgcgcctgatgggcgaggtggcgacggtggcggaggcggtgcgcagcgtccagcccgcgggcacgctggaccagccctcccgggagtacctggcccgggggcgcgaggtgctgcgtgggcggatcgtcaagacgtgcgacgaagtggcccgcacgctgcgggtgtatgacgacgcctacgagaacctgacgatccacggccggcccaccgcgttccgggactttctgctggatgcgcccgccatgttcagccggctgggcgaccagctgggcgcgatccaacacatcgtgtcgtattggcgtttccgctttgcgcccggcgcggcccaggtgcaggtggaggagctgatcgacatcttcatggacttcgagacaggcctgctcggccgcgacgagttcgccgagacctcgaggttcatggccgcctgacggaccaacaaaaaaggccggcgtctccgccggccttttgtccgcctgatcatccgatcagtagcggtagtgctcgggcttgaacggcccttcgaccggcaccgagatgtatgacgcctggtccggcttcagctgcgtcagcttggcgcccagcttggccaggtgcaggaaggcgaccttttcatccaggtgcttgggcagggtgtagacctgcttctcgtacttggcggcgttggtccacagctcgatctgggccagcgtctggttggtgaaggacgccgacatgacgaacgacgggtggcccgtggcgttgcccaggttcaccaggcggccttcggacagcaggatgatcttgttgccgtccgggaactcgatgtggtggacctgcggcttgatctcgtcccacttgaagttcttcaggcccgcgacctgaatctcgctgtcgaagtggccgatgttgcagacgatggcgttgttgcgcatccggcgcatgtgatcgacggtgatcacgtccttgttgccggtggcggtgacgaagatgtcggccttgtcgcagacgtcgtccagggtctggacgtcgtatccctccatcgccgcctgcagcgcgcagatcggatcaatctcggtcacgatcacgcgggcgccgccctggcgcagcgaagcggccgagcccttgcccacgtcgccgtagccgcagaccaccgccaccttgcccgacagcatgacgtcggtgccgcggcggatggcgtccaccagcgattcccggcagccgtacaggttgtcgaacttggacttggtgacgctgtcgttaacgttgatggcggggaacggcagctcgccgcgctcggccatctggtacaggcggtgcacgcccgtggtggtctcttccgacacgccgccgatggcgtcgcggatggccgaatagaagccgggcttttccttcaggtagcgcttcatcaccgcgaacagcgcttcctcctcttcgttctgcggggtgtcgagcaccgaggcgtcggcttcggccttgggccccagcacgcacagcagggtggcgtcgccgccgtcgtccaggatcaggttaggatagccgccgtcggcccattcgaagatcttgtgggcatagtcccagtactcctccagcgtctcgcccttgacggcgaacaccggggtgccggcggcggcgatggcggcggcggcgtgatcctgggtcgagaagatgttgcacgaggcccagcgcacctcggcgcccagcgcctccagcgtctggatcagcacggccgtctggatcgtcatgtgcagcgagccggcgatccgcgcgcccttcaacggctggtcgccgccgaactcggtgcgcagcgccatcaggccgggcatctcggtctcggcgatggcgatctccttcttgccccagtcggccagggagatgtcgcggatgatgtagtcggccaaggcaggctcctgcacaggaaaggtttggcgctctatagcggtcggcgcgcgcgccagcaacgcaacatataaggacatccttatacgacgggcgggcggggcggtgtgaggcggttcttaacccgccggcgctaaacgtttccgcatggatcgccgcgctcttcttggtctcgccgccgtcgccgccgcatcggcctcgcccgccgtcgcctcatcgggcaagagcggaggcggcgcgcccgccgacagctacatccgcctgcccgtcgtcaccgccagcgtcatgcgcgccaacggccagcgcggcgtcctctccgtcgagaccggcgtggacgttcaggatgcggccctgcgcctgcgcgccagccagtcggcgccgcgcctgcgcgccgccttcaacacggcggtccagcgcttcgccctgggtctgcgtcccggccaggcgccgaacgtggaccaactgtcgcgcgaccttcaggcggccgcaaacagcgtcatgggccgacccggcgccacggtgctgctgggcacggtgatggcggtctagaggaaggaatagggatccacgtccaccgtcaggcggaccgagcccggacccttcacccgcgccagccacgccctgaggaagccctgcaggtcgacgtcgcggtccgcgcgcaccagcagccgcttgcgccgtcgcccccgcaccagcgccagcggcgcatccgccggtccatagacctctagccgctcggcgttggggatggcctgagccaggtcgctcgccgtcttctccaccgccgtcgcattctcgctggacaggatcagcgccgccagccgtccgtagggcggcagggagccggcctcccgctcggccatctcggcctccacaaaggcgtcgcggtccccggccgccagcgcctgcagcaccggatgctcgggcgtccaggtctgcaggatcgcgcgccccggcctgtcggcccgccccgcccgtcccgtggcctgggccaagagctgataggtgcgctcggccgcccgcaggtcgccgccgcgcaggcccaggtccgcatccaccaccccgaccagggtcaggcgcgggaagttgtggcccttggccgccgcctgggtcgccaccagtatgtcgatctcgccgtccgtcatgcgttggatcagggcgcgggccgagcgggcgtccggcgcggtgtccgagctgaacacggcggtgcgcgcctgcggaaacagctggcgcacctcctcctcgacccgctccacgcccggcccgaccgggaccagcgtgtcctcggccccgcatgagggacagtgcttgggtctggccatcgagaagccggtcaggtggcagaccagccggccggtgtagcgatgctcgaccagccagctgtcggtgtccggcgccgtcagccggtgtccgcaggcgcggcacagcaccaccggcgcatagcctcgccggttcaggaacagcagggtctgctcgcccttcgccagcgtctcgccgatggcttcacgcaagggctgagacagccaggtctgcgggtcgggcggagtttcgcgcaggtccagcagggcgatgtcgggcagcaccgccgtcccgtgccgcgcccccagccgcagccagccgtagcggccgacgcgggcgttccacagcgtctccagcgagggcgtggcggaggccagcaccaccgccgccccctcgatccgggctctcgccaccgccaggtcgcggccgtgataaacgaggccgtcctcctgcttgaacgagctgtcgtgctcctcgtccacgatcagcaggcgaaggttcttgaacggcaggaacagggccgaacgcgcgcccaccacgatgttgcagcgtccagcgaccaccgcctcccacacctggcgacggcgcggcggcgcgacgccggaatgccactcggcggggcgggcgccgaagcgggcggtgatccgctcgatcagcgcctgggtcagggcgatctcgggcaggaggatcagcatctgcgcggcccgatcggcgcgcagtacctgggccaccgcctccagataggcctcggtcttgcccgatcccgtcaccccgtccagcaggaacggcttgaaccccccggcctgaacgcccgccgccatcgcctgggccgccgccgcctggtccgggttcagggtggagggcgcatgatccgggtcggcgcggtcgaaggcggccacggcctcgatctcaacgacctccagcacgccctcgtccagcagtcccttgaccactccggccgacacgcccgccgcgcgcgccagctccgcaggcggcaggctgcgcgcgcccagcgcctccagcaccgccgtccgcgccggcgtcggccgcttcggcgcctggccctcgatccgccgcacgcgtcgttccggacgcggccgcggcgcacgcaagcctttcagcgcggtggccgccatctcgccgggcggcgacagggtccagcgtccggcccactccacgaaatccaccgtgcctgggggaagcgcgggatcatccagccgctgctccaccgccttcagccggcggtttgagccagtggtctcgaacacctcggctacgatcccgcgcaccagccggggaccgagcggcgccgccacatggtccccccgcgccagcgccatgccttccgggacttcgtagtcaaaggcttccggcaccggcagcggcacaagaaccgacgcgaccctcaccgtcgtcctccctgcccggcgcagaaagggagtcgcctcgcgccgggggcggcgctagaaccccgctccatgaaactctttctcgacaccgccgacgtttccgtcatcaaggacatggtccccacgggcctggtggacggcgtcaccaccaatccgtcgctgatcgccaagtcgggccggaacatcgccgaggtcatcgccgagatttgcgccctcgtcgaggggccgatctcggccgaggccgtgtcgctggattgcgacaccatgatccgcgagggcgaaaagctggccggcatcgctcccaacgtcgtcgtcaagcttccgctgacctgggacggcctgcgcgcctgccgccacttcgccgacaagggcatcaagaccaacgtcaccctgtgcttctcctcggcccaggccctgatggcggccaaggcgggcgcgacattcgtgtcgcccttcgtcgggcggctggaggacgtgggcgccgacggcatcgccctgctggaggagatccgggtcatgtacgacgtgcatggcttcgagacccagatcctggccgcctcgctgcgcaacgtcgcccatgtgtcggccgccgccgtggcgggcgccgacgccgcgaccttcccggccgagaccttcaaggcgctggtcaagcacccgttaaccgacaagggtcttgatgcattcgtgtcggactgggccaaaacggggcagtccatcctgtagtatcccgccttcccggagaggttcgttgagcggctcattggacctttccgcgacgccggaaacggacgtggaccagcccctgcactggccgcgcgtgcgcgactggctgcaggcgcatccgcagaccctcctggacgatcgctcgctgctcgaagaggtgggcctgcggccccacgggcgcaatgttgtcgacttcggcgtcgccgccctgacccgcatcgaggctgtggccgagcgcgaggccgatgcgcgccgccagatcgaggccgtcgcgcgcgccaacttcgccgctcagacgcagacccatgtggcgacgctggacctgctggaagcgcgcagccactccgacctggcccggcggctggatgcggcggcgcaggggcgcttcggcctcacgtcggctgcgatcgccctggagaagcccggcggcgtgccgttcggctggcgcgcgctggaggccggcggcgtcgaccgctggctgggcgagcacggcctgacctggctcggccccgcctttccggagctcgacctgttcggcgcggccgccgagggcgtggcgtccgtcgccctggtgcggatgagcctgaacctggatcccgacggcccggcgcgctcggccctggtcgccttcggctcaccggagccggagggctttaccctcaacatgggctgcgaactggccgcctttctggcccgcgtggtcgagcgcatggccgagcgctggccggttctgcaatgacggccgacgaggcgctggccgcctggctggcgcacctggcgcacgaacgccgcctgtcgccgcgcacgctggaggcctatggccacatcggccggctgtacctcgcctttcttcagcgccatcgcggagacccgctgtcggcgcgtgatctgggagccgtcgcggcggccgaggtgcgcgcccacatggccgagcggcgatccggcgacaaaccgctgaacgcccgctcgctgtcccagaccctgtcggccatccgcggccttcatgcctttctggatcgccgcctccacatcgccacgccgcagatcgcgctggtgcgcgggcccaaggtcaagccgtcgctgccccgcccggtgaccgaggatcaggcgcgcggcctgctggccgagccggaaggggatgaggacgccgagccgtgggaggcggcgcgcgaccgggcggttctgacgctgctgtacggctgcggcctgcgcatctcggaggcgctgtcgctgcgccgcttggacgcgcccctgcccgagacgctgcggatcacgggcaagggcggcaagacccggatcgcccccgtcctccccgccgtgcgtgaggcggtggacggctatctggcgctgcagccctttattcttgatcccgagacggcgctgtttcgcgcccggcgcggcgggccgctgagccctcggcatgtgcaggccaccgtgcagcgcctgcgcggccgcctcggcctgcccgagcgcaccaccccccacgccctgcgccacagcttcgccactcatctgctgggcgccggggcggaccttcgcgcgatccaggagcttctgggccacgccagcctgtcgacgacccagaaatacaccggcgtcgacgccgcgcgcctgctgggcgcctatgcctcggcccatccgcgcgcctagaaggggcgcatgagcatcgacatcctggtccttggcgtgccggctttggccgagcggttgctggaacagcgggcggccgatcgcggctggacgctgcatcggccaggatccgacggcctggccccggctgaggtcgcgggtcgcatcgtcgccgtggcggcgtccggtggatggcccgtcgacgcccgattgattgacgccttgccggcgctgaagatcgtggcggttcacgccgtcggctatgatctggtggacgtggcgcacgcccaggcgcgcggggtcgtcgtgacccatacgcccgaggtgctggacgacgacgtggccgacgtggcgctcggactggtgctgtcggtgctgcgaggcctgcctgccgccgacgcctatgttcgggccaggcgctggcccggcgaggggtctctgccgctgaggcgcagcgccagcggtctccgctacggcgtgctgggcctgggccgaatcggaaccgccatcgcgcggcggctggcgcctctggcccgctcgctcgcctatcacacccgccggccggtggaaggcgcgccctggaggcacgagccggaccttctcgcccttgctcgagacgtggacgtgctggtggtcgcggtgcccggaggtgacgccacgcgaggcctggtctcggccgaggtcatcgaggcgctgggcccgcaaggcgtgttgatcaacatcgcgcggggcgaggtcgtggatcaggccgccctgatcgccgcgctgcgggagggtcggcttggcggcgcggggctggacgtcttcgacggcgagccccacgtgccccaggccctgatcgacagcgaccgcacggtgctgacgccgcacatggcctcggccacggtggaggcgcgcacggcgatggcggacctgatgatcgccaaccttgaggccgttctgtccggagacgccgccctgaccccggttccttcagatcagcgctgaggcgaggcggacggcgcctgcgacggttcaggcacgcgaccccactcgcggcccagcgcgcggggctggttcggaacgtcgaagctgatgggcgccgggcatccacggtagcgccgatccagcagcaggtagcgacgcgcctctccgcgatccggcgatcggtccagcaaggaggatcggccctccggggtcggttgcggatccaggccggcctcccgcagcagcgcgtcgcaggcggaggattcaggctggggcgtccgcgaggccatgacgcccgatcggctcggctccgcagcgacgggcgccgcctgcagggcggtcagcaggaacaaagaaacgatcatcgcaccctcctgtcttcgccgaaggatagcagaccgtcgatccggcggcgagccgccctccgctcagatcgccttgatcgcgccgccgtccagccggatcagcgagccggtgatgtaggcgcccagcggactggccagaaaggcggcggtcgcgccgaactcctcggtcgcgccaagacggccggcggggatggtcctgaccgcctcggcgcgcgcctgctcgggcgtcacgcccgtgcgttcggccgccgccctgtccagccgctcgatgcggggggtgtcgatgcggccgggcagcagggtgttgacggtcacgccgtcggccgcgacctcgttcgacagggtcttggcccaggcggcgaccgaggcgcgcagggtgttggacacgcccagcacggccgagggctcgaccaccgtgatggaggccacgttcaggatgcggccccatccggcctgccgcatcgccggcagcacccggtcggtcaggcggaacaccgacagcaccatggattcgaaatgctcgcgccagacggaagggtcgagccccgagacgcctgagggcggcggcccgcccgtgttgttcagcagaatctcgacagatccgcccagctgcctttccgcttcgtccaccgccgcgagaagggcgtcgtgatccgccaagtcggcggcgacaaagccggcgcggcccggcccctcggcgctgagctcgtccgcgacggccttcagcgcgtcggcgttgcgggacagcaggacgacgtgcgccccctcgcccaccaacgctgcggccacggcgcggcccagaccgctggagccgccgcagatcagcgcccgcctgcccgtcagtttcaggtccatgaccgcgcctcccctgtctggccgatcaggcctgcatcatccagtcttcgacatccatggccgcctggcgcacggcctccgagcgcgtcgggtgggcgtggcaggtgcgggcgatgtcttccgaagcgccgccgaaggccatggtgatcgccgcctcgtggatcatctcgccggcctgcggccccatgatgtgcacgcccagcagcttgtcggtttgcgcgtccgccagcaccttcacgaagccgtcggtctcgtggttgatcttggcgcgactgttggcggtgaaggggaacttgcccttcttgtactgcacgccctcggccttgagttggtcctcggtcctgccgacccaggccacctcggggaaggtgtagacgacgctcggcaccaggtcgtagtcgacgtggccgaacttgccggcgatggtgtcgatgcaggcgaccgcatcctcttccgccttgtgcgccagcatcgggccgtgcgtcacgtcgccgatcacccagacaccgtccgcgaccttgaagtggtcatgagcgataaagccgcgcttgtccggcgtgacgccgacgctctccagccccagaccctccgtgtagggacggcggccgatcgcgaccagcaccacatcgcccctgatcgtttcggccgcgccgccggcggccggctccacggtcagctcgacgccgtccttgcccgacctggcgctcgtgaccttggcgcccagcttgaagctcatgccctgcttggtcagggtgcgctggaaggcggtggcgacctcggtgtccatgcccggcgtgatgcggtccaggaactccaccaccgtgacctccgcgcccagacggcgccacaccgatccgagctccagtccgatgatgccggcgccgaccacgatcagcttcttgggcaccgccggcagcgacagcgcgccggtcgagtccaccaccttgcccgcctcaaaggcgacgcccggcagcggcgtgggctccgaccccgtggcgatgacgatgttcttggtctcgagcgtgcgggtcgccccgtcggcgctggtcacctcgaccttgcacggtccggcgatccggcccttgccctgcacccattcggccttgttcttcttgaacaggaactcgatgcccttggtcagggccgtgacgctgtcgtccttggccttgtgcatctgctggaggttcagcttgggctgcacctcgatgccgatcttggcgaactcggtattggcggcctgatacagctccgaggcgtgcagcagggccttggacggcatgcagccgacgttcaggcaggtgccgcccagcgtgccgcgcatctccacgcaggcgaccttgaggcccagctggcccgcgcggatcgcggcgttgtagccgccgggcccgccgccgatgatgacgacgtcatagggagcggaagcttcggccatggggtcctcggaggttcgtctaagcgcagggggaaggcggctcggacactagcgcccgacccgacggaatcaaccgcaagccgcgacttcatccgcctttcgaactggagcggccacagcaaaaaggccgggcgtcgccgcccggcctcttttcgcgtcgaaggcttttcgccttagaacgccatgcgcgccacgacctggaaccagggaccggcttcctcggtttcgagttcatactcgtcgtagtcgcggtcgatctggtcggccaggttgccgaacttgtcgaaggtctcgtccttggaggcgttcagcaggttcgatccggtaaagcgcaccacgatgttgtcggcgaccttcttctcgatgaagacctccaagtcggcgccgtaggaggtgacgacctcttcggcgatcacgcgcgaataggcgtctccctgcttgcggtaggtggcgccgaaggccgcgccccagctggggatgtcgtgggtgaagccggcgttcagcacatagtccgactgcgagttgaagcgacgctcgcccaggaagtcgtccacggcgctgtcgagccaggaatagttcaggaatacgcccgtcgtctccatgccgatgaagtccagcggcgtggacaggtcgaactcgacgccccagacttggccgtcgccgacgttgtcgacgctgtagacaaaggcttcgatctcggaggtgtcctcgtcgtccgcgctgccaggccggccggtgttcacgttctcgatcaggtcggtgatgtcgcgatagaaggcgttgatccccacgacgccccgccgacccagccggcgctccagaccgacgtcaacgccccaggccgtctccggccgcaggttcgggttgccgatgaagtcgctgtcgccgacctcctcctccagcagggcgggtgacaggctgtcgaagtttggacgacgcaccgtgcgggccgccgacacgatcagccggtcgcggtcgttcaggttgtagcgcagactggccgagggcagaaggaagtcatagtcgttgtcgttgacctgatccgccggatccacggtgcggtcggtgatggtggtgtcggtggtctcgtaacgcaggcccgcctcccacttagcggccccctgctcgcccgacagcatgacataggggtcgatgcgagtttcttcgatggtggacacgccgccggccacgccggtgaaggcgccgaaagccggcacggccggacgggctgcgggggcgttgggcacgttgaagcggatgcgcggcgcggccgtgacgtcgctttcgcggtccttgtcggtccactggacgccgaactccagctccaggccggcggcgaggtcgcggctgtgctcgatggcacccgacaattcctcatcctggatgtcgtagcgggtggcgtcggcggtgaagcggtcctcgtctggaaacaccacggcgtcgcgcaggaactcggactcgaattcggtctcttactgctggtcgtcgatggaggcgtagccgagcttgagccgcgtctcgccgcccagcatgccaaaggtgtagcggccgttcagcgacaggttgtcggtgcggatgtccaggtcgttgtcgttgatgacgtcgatgctggccgccgtctgcaagccatcgacgtattcgatcgagtcctcgtcctggtagcggtccgtgcgcacgaacacgcccgagagatccagcacgccgccgccgacctcgacctggtacgagccgttcagcgagtagtcggtgccgtcgcgggtgtcggtctgcgcctccacgttctgcagttcgccgccgggctcgtcgaaccgctggctgaacttctccttggggttgcggcggtcctggacattggcgccgatcagcaggcggccgggcccgacctcgccgccccacacggcgccggcggtgccgccgaactcgccgtattcgctgtcttcccacttcagcgcgcccagacggacgtagccgccgtcgaggctgagcgcatcgcgcagcacgatgttgatggcgcccgcgaccgcatcgccagagcggttagccgaagacgaacggaccacctcgacccgctcgatcagctcggcggggatgcggtcgacaaagaaggagcgatccacgcccgcgcctggcacccgctcgccattgatcaggatctgggggtagccgggatcgagcccgcgcagacgcacgccgtcggactccagcacgtccgacaggaaggcgaccgagggcacgcgcttcagggcgtccccggcggtcagaggctcgaagcgctgaaaatattccaggtcgtaggacagggtggggacgacgtcgtcggtgcgattgcgaacctgcggctcaccagtgacgataacctcatccagcgccgtgacgggaccgcgatcctgcggctgcaccaccggagccacgacgggctcggcggcgaaagccggcatggcgatcgctaggggggcgaaggctgcgcccatcagcaggtgaagtttcatgatccgatccccaaggtcgaggcagctgcgctcgaccgatgctcgcggcgcttagccgcagggcgcgacgcggaagcgacgaacgcgagacgctgaggctgcgtttttccgacccctgcgcgacaatcgctcctgggacggaaaggttgtcatcgtatggcggcggaaacgtcacggcgccgccgttgacgcttggccaagctgtgccgaggaagccgcatcgaacgaaaggaaccgtcatgtcccggacgatcagcctcgcggccccagcctgccttctcgccctgctcggcgcctgcgccacccacgaggtcgactatcaaggcgagggcgagggcgtgatcgggcagggctcgccggtgcaggctgtgctggagacgccgtccgtcggcaccgccggcgaggacgccgccgacgatcccgccatcttcgcctcgacgacgccggtgatggtcaagggcgtgcgcacgccgggctttgtggcgggcacggacaagaaggccggcctctacatctacggactggacggcgaggtgcttcagttcctgcccgagggcttgctgaacaacgtcgatctggtcgaaggcctgagcgtcggcggacgtccgcaggtgctgctgggcgccagcgaccgcacaccgggccgcgaaggcgtttcgctgtatctgttcgatccggcggccggcgacgcggctaacgccgtcaggccttggggccgtatcacctcggacgtggtggagccctacggcttctgcttcgcgcgtcgtggagctgagattcacgccatcctggtcgggcacgagggcgaggtgcggcagttcgtcgtaacggccgatgcgaatggtcagcccgcctcgcgcgaggtgcgccggttcgagatcggcaccatctcggaaggctgcgccgccgacgagccgacaaacgccctgtatcttggggaggagaacgtcggcgtttggcgctatgatctcgacccttccgccggcgctcgccgcaccatggttcagccgatcgcgccgggccgcctggttgcggacgccgagggactgacgatcctgcaggacggctcagcccgctatctgatcggctccagccaaggcgactcgaccttccccgtctggcgcatcgacggcgcgcagcccgactatgtggggcggttcgtggtcacggacggcgcggtcgaccgggtgaccggcactgacgggctggatgcgcagggcgggccggtcggtcccttccccgaaggcctggtggtggttcaggacgacatcaacgacgtcggcacccagaacttcaaatacatcgactggcgcgacatcaagcgcgcgctgggcctctagccggcgactactggtcctcgtcgaaacggcgggcgaccagatcgatcagcgcgtcgatggcctcctgcgcgtccggcccttcggcgaccacgccgacctcgctgccctttccggcgcccaacatcagcaggcccatgatcgaacgggcgtccacggtcaccccgtcgcgggtgacctggatctcgctgtcgaagccggaggccagcttgacgaacttggccgaggcgcgggcgtgcagaccccgcgcattgcagatgcccagggtggcggccgcgcgctcgctcatttctcgcccgccagcacccaggaggcgaccgagatgtatttgcgcccggcgtcctgggcgtgggcgacgcagacctccagcggctcgcgcgtgcgcaccccggccagcttgatcagcatcggcaggttcaggccggcgatcacctcggcccgcgtctgctccatcaccgagatggccaggttcgagggcgtgccgccgaacatgtcggtcagcaggatcacaccgtcgccgtcgtccacggcggcggcggcgtcgacgatgtcgcggcgacggcgctccatgtcgtcttccgggccgatgcagatggcggcgaccccgcgctgcgggccgaccacatgctccatcgccagaaggaactcggacgccagccccccgtgggtgacgatcaccaggccgatcatgaaggcttcactcgcatcccgccccaaccgtccctcggctgcggccgccggaggaggacggacgcgcccgatagggaccgcaagcggaacgtcatagacctatacggcgcagggtcaaagcgtctgaagcgcccgcgccgccagcaccgcggccgaggcggcgaacgggttcagcctgaacaaggggacggcgacaccctccaggacgtgcgtctccggctccggcaggcgctcgatcggctcggcgcaggcgatcacggcggcgatccgagccatgggccgggtggacgctcggatgatcccgagaccccgcgcttcgatgcggccggcgatcgcggaaggcgatgtggcgtagagccgcccgcccgaggcccagaccaggctgtagtcgtccgcaaccagccgccagcccgcgtcgatcaggcgcaaggccaggtcgctctttcccgagcccgacggacccataagcatcagcccccgccactcggccccgcacagcctcgccacggtggtggcgtggatcggctggcgcggcgtctgcggcgcagtcacggccgacggctggcggatgggagaaccacctggaaccgtgcgccctgcacctcgccgtgttcgttcgtcctgttttcggcccacacacggccgccgtgcgcctcgacgatctggcgcacgatcgacaggcccaatccggagttggaaccgaaggccgcgcccttgggccgggacgtgtagaagcgctcgaacaccgtctccaggttctcggacggaacgccggggccgtcgtcctcgatgaggatgcgcgcctcgttgtcggcgccggaaagcacgacccgcactatcccgcccgccggactgaacgagcgggcgttgtcgatcaggttacggaacacctgccccagcggcccgtcgcggccgatcacgcgctgcggctcggccccggcctcgaacaccaccgtcggatcgcccggcttggccgtcgtctcatagacggagacgatgtcgcgcagcagggtattcagctccaccgcgcgcggccgttcgcgcgacagttcggcgtcgagtcgagaggcgttggagatgtcggtgatcaggcgatccagccggcgcacgtcctgctgcagcagattggtcaggcgctcgcgctgctcgtccgtcttgaccagcggcagggtctccaacgccgagcggatggaggtcagcgggttcttgatctcgtggctgacgtcggcggcgaaccgctcaatggcgtccatccgcgccgacagggtctcggtcatggactccagtgatcgcgccagatcaccgatctcgtccttgcggtcttcgaggtccggcaggctgatggcgcgcgccctttgcagccgcacctggtccgccgccgccgacagccgcatcaccggccgcgccacgaacaggtgcagcagcaggctggccagcaggttcacacccagggctacaagggcgaagggcaccagcgcgcggcgctgggcgcccaggatctcgtcgacgtttcccgcctccagcgtcagcacgcccagcacctggctgacatggcgcacggggatggagacggagacgacccggtcgccctcctcattgcggcgcagggtctgctgcgactggcccgccaaggcgtttgcgacctcggcggtcagctcgcggttggcgcgctccagccgctgggcggcaagcgtctcaaggccgacatcccgctcaggctgcggcgtgcctgcgggacgggcgtccggcaggggcgcgccgggaatggcttcggtcacctgatagctgtcggcgaccagcaggccgttgatgtcgtagagtcgaacccgctgtccctgcgggatgaagttgtcgcgcagccaacgggcggccgagatcggatccagctccggcgacggctcgccgcgcgtgatagccagttcgcccaggacgttggacaagagctcggcctgcaccgacaacgattcctggcgcgcctgcaccaggccgcgcgacaactcgttcagcagcaaggccccgccgaagaggatcagcaggctcagcaggttcagcgccaggatgaagccgcccagacgcgaaccgccgaagcggaaggcgcgcctcggcggggtttcgtcgtctccggtcaggccgggatcagctttcgcggtagcggtagccgacgccatacagggtctcgatcgcgtcgaactcgggatccacggcgcggaacttcttgcgcatccgcttgacgtggctgtcgatggtgcggtcgtcgacatagacctggtcgtcgtaggcggcgtccatcagattgtcgcggctcttcacgaagcccgggcgctgggccagggcctgcagcagcaggaactcggtcacagtcagcttgaccgggcggccgtcccacatggactcgtggcgggccgggtccatggtcagcttgccgcgcttgatcgccttgcccgaagcctcggccgagggctccggctccaccccgtcggcgccggtgcggcgcagcagggccttgacccgctcgatcagcagtcgctggctgaacggcttgtggatgtagtcgtcggcgccgaggttgaagcccaggatctcgtcgatctcctcgtccttggacgtcagcatgatcaccggcagctgcgaggtctggcgcaagcgacgcagcacctccatcccgtccatgcgcggcatcttcacgtccaatatggcgaggtcgggcggcgtgctttccagcgcggccaggcccgacgccccgtcatggtaggcggtgatcttgtgtccgtggctttccagcgccagcgaaaccgacgccacgatgttttcgtcgtcgtcgaccagggtgatgttcgccaagggcctgtctcctgccatctgtcgggggcggacgtaggccacgcgggggcgagcccgcgcgcgtccgccgcaaaacgcgttcacactagaaccttggcagatgggccgccaccccgtcggttgcaatcaggtcacacatcgacgtcagcgcaaaccccgtcttaagccgcaggggtgcaggttggcgtcatggccggcccagtccactacgaagtcttcatccgccgcacggcgcccgcgccctggacgctgctgatcgcgacggaggatcgcaagcatgcgatgaccacggccgaagaggtcatggccgacagcggcgcggccgcggtccgcgtcaccaaggagacgctggactccgagaccatggagttcaacagcctcaccatcctgacccgcggcgcgccggagaccaagccgaagccgcgcaacgccgccgccgccggacccgcctgcaccggccccatggacctttatgcgccccaggcccgggcgctgatcgcgcgggtgctggaggactggctggcgcgtcagggcgcgacgacctttgaactgctgcaccggcccgacctcgccgagcggctggaggcgtccggggtcgagttgcagcatgcgatccagaaggtggcggtgcccgaaagccaggcgacggggcagccgatccacgacctgatgcgccattaccagcgcctggccgacgcagccatcgaccggctgatcaagcacgggcggcgcgaaggctttcccgatgcggcgacgcagccgctggccggcatcgccgagcgcctgaaggccggctccgaccgcgcctttgtcatgggcggcgtcctgtccgccgcgctgaaggacctccgcggggctcgggcgcgcctgtcgaagctggcggacctgatcgacgccgccccgcccgaaggcggcccgcgcgccctggtgctggtgggcgccgaacagatcgccagcgagatgctgggggaccgcaaggtcctggccgaggttctcggccccgccctggatcagggcggcagcctggccgccgtgatccgcatggtcgccccgcgcgaggtcgaggccctgacgcggatggacccgcgtctcgccctgttgacgccgacactggatggaccggccgcacggctcggggcgcacttggacgcgggcgagtttccgctgctggcggcgtccttggcccgcatggtggtgcgcgaactgatgagcccgcgccggctgcgcccctccgacgctcgcggcgagatcgacatcctgcgcgcgctggccatgagcctgacggccacggccggtcggctgctgacgctggaggaggtgcagaacgcctttgtggagcggtccaaggcgctggtcgcggccgatttcgtccaggcctatgtggcgccctgcgacaccgtgctgtgcgaggccgagcacctgatgcggctgtgcgagaacgtgaccggcgccgccaacaagcgggccgccgcgcgctggctgcacgcctgcatcacatcgctgcggttcgagaccgagatgcggaagagcgccaaccccatggcggcgctcgccaccctggcccgcctgcagaaggccgctcaaggcctgcagctcaacgagcaggacgaagcccaggtcatcgcggctctgggcgctgtcggcggagcggtcgagaccgaaagccggctgctcgcccagatcgttcgcgccggcgcggcgcccgcgcagaagctgtcggccctgctgcgcctgggtgtcggcgagacggcccctttggggcccgcggccgatcgcgccaaggccgaggccctgcgcctgctgcgcgcgcccgagacccgcaccgccctggcggctgcgccggccgaactgaacgccatgcgcgacctgatgacggccgcaggcctcgccgcctgaacaggtctcgactgcacaagaaaaagggccgggcgtctccgcccggcccccctgagatcgatcgcgatcaggcgatcaccagatgcggacgcgctgatccgccggcaggaagtatttgtcgccttcggtgacgccgaacgcctcgtaccaggcgtcggagttacgcagcgggccgatcacgcggaactcggccgggctgtgcgggtcggtggcgacctgctgcttcagcgcctcctcgcggtacttcgattgccacacctgcgcccagccgtagaagaagcgctggtcgccggtgacgccgtccagcacgggcgccggctggccgttcagcgacaggtggtaggcctccagacccaccgccacacccgcggcgtcgccgatgttctcgcccatggtcaggccgccctgcacgtggaagcccggcagcggctcgtactggtcgtactgggcgcccaggcgggtggtcaggccctcgaagttggccttgtcctcggccgtccaccagtggcgcagcccgccgccgccgtcggacttggacccctgatcgtcgaggccggggccgttctcgtgaccgatccccccgccgatgccgccgtagttgaccgccgcgtcgccgttcggatcaaagaagggcggctgcaggatcgccgccgggaacacgatctcgttgttggccgagttgtagtaggcgttcaccgtctggggcgtcatgccccactcgtccttgtccaccggctcgtcgaggcgggccaggtcggactcccactcgaacaggcccttgcgctcggcgttgccgaccaggtcgtcgccgcggacctcaagcccggagtagtcgcgccacttgttcggatagccgatcttgaccgtgaacttgcgcagcttgtcctgagcttgcgccttggtctcgtcgcccatccaggtcaggttgtcgatgcggtgcgacagggcggtgcgcaggttggcgaccagctcctccatcttggccttggactcggccgggaagtattctgccacatacaggcggcccgtcgactcgcccagctggttctcggcgaacgagatggcgcgcttttcgcgcgtgcgctgctcgggctggccggacaggtcgcgggcgcggaactcccactgcgcgtccgaaaagcgcttggacagcatgggcgccatgtcgtcggcggtgtggaaggcctcccacgcctgcagcagttcgaccggcgtttccgcgtagatggccgcgatcttcggcatggccgtgtcctgacgcacgatcaggcgcggcaccccgcccagttccgcggcgtcatagtaggcctgccaggcgaagcccggcgcctcctgcgtcagctgctggatggtgtattcgttgtaggtctcgtcgcggttgcggttctggatcggggtccagtgggcctcggcgaccttggtctccagcgcgacgatctgggcggccgtctcggcggagttatcccagccgatcatttccagcatccggccgacataggcctgatacttctccttcttgtcggcgtagcgcgcgtccagatagtagtcccggttcggcaggccgatgcccgattggccggtcgagaccacgtagcgggtcggctgcttggaatcgatggtgatgccggtgccgaagaaggacgagccgaagcggccggccgtctggcccatgtagacggccatcttgtcgtggctgtcagcggcgcggatggccgcgaggtatggctgcagcggctgggcgtccagctgctcgatgcgcgcctcgtccatataggcgcggtaggcgtcggcgatcttggcctcgtccgagcccggcgtcaggtcgttgcgagccgcgaggcccgtgaccagcgccttcatgcggttgtccgacagctcgcgcagcagggcgaaggagccgtagctggtgcggtctgagggaatgaccaggtcttccagcgccttgccgttggcgtactggaagaagttgtcgcccggcttcaccgaggtgtcgcggccgttcaggtcgaagccccaagttccgtagcggggcgcctcgacaccctggaagccgctggctccttcggccggagcagtctggaacagcgcctgcaccgtgcagacgtcgtcgacgcattcatgatcgtgcccgtcatgggcgaaggccaggctggccggaagaagaagggcgcccagagcagcgccgacaagcagacgtttcatacgcagggtctcgcaaggccgcctcaccgcgggcgggtcgatcggaccctaggcccctcaggcgcgagtttgtcttaaaaaaagttcatgatccgatttcgggcttcgctagaccgctgtcttttcagcctgatagttcagcgacggggggcaggcgcatgacaggtcacggcggcggcgactacaaggatctggtggtctttctggcggccgcgggcgtggtggtgccgctgttcaaccgattccgcatcagcccggtgctgggattcctggccgccggggtgctgctgggccccgacggcctgggtcgcttcgccggttcgggcgactggctgtcctggttcaccatcagcgatccggcccagctgacgcagctgtcggagctgggcgtcgcctttctgttgttcaccatcggactggagctgtcgtgggaccggctgcgcgccatgcggcggctggtgttcggcctcggcctgatgcaggtcgtcgcctgcagcgcggtgctggcggcgggcttcatgctgctgggccagacgctcgccagcgcggcggtgctggggttggggctcgccctttcctccacggcggtggtgatgccggtgctggccgagcgagggcggctgaaggggacggtcggccgctcgacctttgcggttctgctggcgcaggatctggcggtcgcgcccatcctggtcaccgtcggcgtcatggcggcgctggcgtccggcggcggcgggctcgacccggcggtgctgggccgctcgctgctgacgctggttcccgccgccatcggaatggggctgctggtggtgctgggtcgcgtcgtgctcaggccgatgttccggtcggtggcgcgcgccagaaggggcgatcagggcggcgagctgtttgtcgccgcctgtttgctggtcgtggtcggcgcgggcgtcgcggcccaggcgtcgggcctgtcgatgagcatcggcgcgctggtcgccggcgtgctgctggccgagaccgagttccgccgtcaggtcgaggtgtcgattgagccgttcaagggcctgctgctgggcgtgttctttgtcggcgtcggcatcgggctggacctcgatgcggtggccgccgcgcctcatgtcgtgctggcgctggccgcggggatcatcgcgatcaaggcgaccgtcatcttcggcctggcgcggctgtggggggtgggcggacgatccgcgatcgagaccgccctggtgctcggcccggccggcgagttcgcgttcgtggtcctggcgctgggcatgcgcgagggggtgacctcgcccgacttcaccccgaccgtgcttatcgccgccaccctcagcatgttcgccgtgccgctcatggccatgctcggagagcgtctgtccaagcgctcgtccgccgacgcgcccgccgcgcctgtgccggtcgttccgccgtccggaccggacggggcggtgatgatcgtcggcttcgggcgggtcggccggctgatcggcgagctgctgaccgaacatggccaacccttcatcgcgctggatacggacgccgcggcggtgcagcgcgcgcgggcggacggccaccaggtcttctatggcgacgccggttcggcggagatgctgctgaactgcggggtgcgcaccacgcgcgccctgatcgtcaccatggacgcgcccggcaaggtggacgaggtggtccgcgccgcgcgagccgtgcgcgaggacctgatcctgatcgcccgcgcccgcgacgaccgccatgccgcgcgcctctatgcgctgggcgtcaccgacgccgtgcccgagacgaccgaggccagcctgcagctggcggagaacaccctggttgatctgggcgtgccgatgggcctggtgctggcttccatccacgaacgccgcgaccgctttcgccagctgttccaggaagccgtccccgaagaccgccgcgcccgccccacccgcgccctacgggccgccgcgcagccgagggtgtgagatcacgcaaaagaatgggccgctcgaacgatcgagcggccccatgtctttcaacgaaggacgcctggatcaggcggcggttcgctccgaagcctcttcggccaggatggtaaggccggcgggggttacgtcggcgaagccgccgcgcacctcgaagacccggcgcgcgccgccgtcgatcacggtcaccgcgccttcgcgcagcgccgtcatgaagggcgcatgatccgccagcacgccgaagtcgccctcgacgcccggtgcgtccacctggtccacgaggcccgcgaagacctcgcgttccggcgagacgagggagaagttcagcttgccggccatgatcaggcgctcgcagccatcttggcggccttctcgacggcttcctcgatggcgccgaccatgtagaaggcggcttccggcaggtggtcgtattcgccggccacgatgcccttgaacgagcggatggtgtcggccaattcgacgaacttgcccggcgagttggtgaactgctcggccacgaagaagggctgcgacaggaagcgctggatcttgcgggcgcgcgacacgaccagcttgtcctcttccgacagctcgtccatgcccaggatggcgatgatgtccttcagcgccttgtactgctgcagcacgccctggaccgagcgggcgacgttgtagtgctcctcgccgatgaccagcgggtccatgatccgcgaggtggagtccagcgggtccacggccgggaagatggcctgggcggcgatgtcgcggctcagcgtcgtggtggcgtccaggtgggcgaaggaggtggcgggcgccgggtcggtcaggtcgtcggcgggcacatagatggcctggaccgaggtgatcgagcccttcttggtcgaagtgatgcgctcctgcaggttgcccatctcggtcgccagcgtcggctgatagcccaccgccgacgggatgcggcccagcagcgccgacacttccgagccggcttgagtgaagcggaagatgttgtccacgaacagcagcacgtccttgccttcctcgtcgcggaaatactccgcgatggacaggccggtcagggcgacgcgggcgcgggcgcccggaggctcgttcatctggccatagaccagggcgcacttggagccctcggtcgagccgttgttctccttcgggtccacgttcacgttggactcgatcatctcgtggtacaggtcgttgccttcgcgggtgcgctcgcccaccccggccagaaccgagtaaccgccgtacgccttggcgatgttgttgatcagctcctgcatggtcacggtcttgccgacgccggcgccgccgaacaggccgatcttgccgcccttggtgtaggggcagatcaggtcgatcaccttgatgcccgtgaccaggatttccgacgaggtcgactgctcgtcgaaggtcggggcgtccttgtggatcggacgatattccgaggtcaggatcgggccggcctcgtcgatcggctggccgaccacgttcatgatgcggcccagcgtgcccgggccgaccggcgcctggatcgaggagccggtgtcggtcaccggctgaccgcgcgtcaggccctcggtggtgtccatggagatggcgcggaccatgttctcgccgaggtgctgggcgacttccagcaccagggtgaaggtctcgcccgtcttctggtcgacgttgggtgtgcagggcgttcaggatcgccggcagcgggccggtgaactcgacgtccacgacggcgccgatgacctgggcgacgcggccgccggccgaggcggcgaccggcgcggccgaaaaggcttcggcggcgggcttcggcgcgggggcgcggggcttgggagcggtgggggcgacggtgtcggtcatggctggggtccgtgtcggaatgtcgtggcgtgcgggatcagacggcttccttgccggcgatgatctcgatcagctcggtcgtgatcttggcttggcgggagcggttgtactgcagcgtgagggcgttgatgaggtcgccggcgttgcgcgtggcgttgtccatcgcggtcatctgggcgccgaagaagccggcttggttttcgtacagcgcggccagcacctgggtggtgatgttgcgcggcagaagcgtctcgaggatttcctcctccgacggttcgtactcgtaaaccgcgccgttgaggtcgatgggagcggcgtcgccgtccaccaccgccgggatcagctgcctgcccgtggggacctgcgagatcactgactggaagcggctgtagaacagggtcacgacgtcggcgcggccctgttcgaactcttcggcgatcatttcggcgatcggctgggcggcgggcaggcccaccgtcttgtgctccgacagctcgaaggtgcgcacgatcttgtcgccgtagaggcgcgccagctggtcgcgcgacttgcggcccaccgcgatgatgcggacctgcttgccgttcgccaagaggctgttgatgcgctcgcgcgcggcgcggacgacattggtcgagaagccgccggccaggcccttatcggccgtcgccaccacgatcaggtggcgctggtccgagccggtgccggccagcaggcgcggcgcgccgtcgccggacacgcccgccgccaggttggcgatcaccgcggccatcttgcgggcgtagggacgcgcgctttcggcctggtcctgcgaccgcttcagcttggcggccgcgaccatgttcagggctttcgtgatcttctgcgtggacttcacgcttccgatccgatcgcgcatttccttgaggctggccatccggcgctactctcgcttcggttgggggctcagggtcaggcgaaggtcttggagaagccgtccaggatcgacttcagctcggtttcgagttccggcgtcaggtccttcttggtgcggatgccgtccagcaggccggcgtggttcgcgtggacccgagccaggagctccttttcgaaacggccgacgtcgcccaccgccacattgtcgaggtagccgcgcgtgccggcgtagacggagacgacctgctcctccatcgccagcggcgagtattgcggctgcttcagcagctcggtcaggcgcgcgccgcgggccagcagcttctgggtcgaggcgtccaggtccgagccgaacttggcgaaggcggccatctcgcggtactgcgccagctcgcccttgatggtgccggcgaccttcttcatcgccttggtctgggccgaggagcccacgcgcgacaccgagatgccgacgttcacggccgggcggatgccctggtagaacaggtcggactccaggaagatctggccgtcggtgatggagatgacgttggtcgggatgtaggccgacacgtcgttggcctgggtctcgatcaggggcagggccgtcagcgagccggagccgtagtcggcgttcagcttggccgaacgctccagcaggcgcgagtgcagatagaagacatcgcccggataggcttcgcggcccggcgggcggcgcagcagcagcgacatctggcggtaggcgaccgcctgcttggacaggtcgtcatagacgatcaagccgtgcatgccgttgtcgcggaaatattcgcccatggcggtgccggcgaacggcgccaggaactgcagcggggccggctcggacgcggtcgcggcgaccacgatggtgtagtccagcgcgccggactcctcgagcgtcttgacgatttgggcgacggtggagcgcttctggccgatggcgacatagatgcagtagagcttggcgctctcgtcgtcggtcttgttgacgttcttctggttcaggatggcgtcgatggcgacggcggtcttgcccacctgacggtcgccgatgatcagctcgcgctggccgcggccgacggggatcagggtgtcgatggccttgaggcccgtctgcatcggctcgtgcaccgacttgcgcgggatgatgccgggcgccttgacgtccacgcggcggcgctcggtgaactggatcggacccttgccgtcgatcggctcgcccagcggattgaccacgcggccgagcaggcccttgccgaccggcacgtccacgatctcgcccaggcggcgcacgtcgtcgccctcggcgattgcggcgtcggccccgaagatcacggcgccgacgttgtcgcgctcgaggttcagggccatgcccttcacgccggccttggggaactcgaccatttcaccggcctggacattgtccagaccatggatgcgggcgatgccgtcgccgaccgacagcacctggccgacgtccgagacatcggcttcgacgccgaagttggcgatctgcgacttgaggatggccgagatttcagcggcgcggatgtccatgatgggctctctgtcttcggtctcttcggcgccgatgaggcgcgggcgtcagttgcggggcgcggttcaggcgcgcttgagggcgtatttcatcgagtcgagcttggtcttcagcgaggcgtcgaacagcttcgaccccaccttgaccttgaggccgccgaggatcgacggatcgacccggacggtcagttccggcgcgcggcccagcgtctcgcgcagggcgttgcggatatgcgtgacctggacctcgtccaacggctgggccgacaccacctcggccgcgaccaggccggtgtgacgggcgtacagccgctcgaagccggccagcacgcccggcaggtcacgagcgcggccgttctgagcgagcagacccagaaagttgcgggtggcggtctcgaagcgggcctgggcggcgattcccgtcagacccttgacctggtcgtcggacttcatgaccggcgacgtcgccaggcgacgcaggtcggcgctctcgatccaggcggccttcagcgacttcacatccgcgcgcacggcgtccaggcggcccgtctccagggccagatcgaacagcgcctgtgcgtagcgctcgccgacttccgtcgttctgaaatcgtcagccactaatatggtccgcggtggttgcgtttgggtcgacaccggctgcgaacttccgcgccgatcaagggcctgaaatgcttgtggaaagcacgacaggggccgtctctacggaaacgcccccttcaagccgggcgcctgatagcacggggtttggcggctcgcaaccaaggcgggcggaacgataacgccgcaccggcgctgctgtggattgcgggcgctcgcagccgggcaggctgggtgcgaccacgacgccgccggcttcggcttgatggacgctcacgcccgcgttaccgcttagcctcccagtttcatcggacgccttatgctcgacagcatccttcccctcctctccgaccccgccgcctgggcggccctggtcacccttgtggtcatggaggtcgtgctcggcatcgacaacctgatctttatctcgatcctctcgaacaagctgccgccggagcaccgccagcgcgttcgccgcatcggcatcggcctggccttgatcatgcggctggcgctcctgtcgatcatcgcctggctggtcgggctggttcagccggtcttctccgtgttcggcaacgaattttcctggaaggacctgatcctgatcgcgggcggcctgttcctgatctggaaggccaccaaggagatccaccacaccgtcgaccccacgccttcccacgatgtcctggacaagaaggacgtggtcatctcgaacgccggcgcggcgatctttcagatcatcctgctggacctggtcttctcgatcgactcgatcctgacggccgtcggcatgaccgagcacctgccgatcatggtggtcgcggtcctggccgccgtcaccgtcatgctgctggccgccgatcctctggcggacttcatcaacaagaatcccactgtggtcatgctggccctgggcttcctgctgatgatcggcctggtgctgatcgccgacggcttcggcttccacgtgcccaagggctatatctacgccgccatggcgttttccgccggggtggaggcgctgaacatgctgggccgcagatccgcctccaagaaggagctggcggaagccgcccgcgccgaggccgaccaggccgaggcgcgcgcccggcaggcggaggccgaggccgccgccgatccggccgcccgggcctgacccccatggaccggcgcgcgcttcttctcggcctgattctcgccctcggctcgccgctctgcgcgcaggccgaggttccggttcaggcctatgaggtggtgcgcgcctatccgcatgatccggaggcgttcacacagggcctgatctggcgcgacggccacctgatcgagaccaccggccgccagccctcggtgctccgccgcgtcaggctggaggacggcgagccggtggcgcagcgcaccctggccccgatctacttcggcgaaggcgtgaccgagctgaacggcaagctctacagcctgacttggcgcaacggcgtgggattcgtctggaaggcggacgacttcacgcccttgggcggctttacctaccagggcgagggctgggggctgaccacggacgggcgccggctgatcatgagcgacggcacgccgttcctgcgcttcatcgacccagagaccctggccgagaccggacgcgtgcgggtgaccgccgacggcgcagacctgcccatgctgaatgaactggaatggatcgacggcgaggtctgggccaacctctggcagagcgaccgcatcgcccgcatcgatccgggaacgggcgtcgtcaccgcctttgtcgatctgaagggcctgctgcccaccggcgcgatccgcgacccggccgacgaggtgctgaacggcatcgcctgggacgccgagaacaagcggctgttcgtcaccggcaagcgctggccccgcctgttcgagatccgggtccgtccctgaaagacaaaggcgccgcccgtgagagcgacgccttccctgcttgaagttgaaggagtgatcagcccttcagcgcctcttcggaggcgacgatccggctggcggcgtggaccacggcgccgatccgaagagcggcctggacgtgggtgttgggcacgccgtgcttgcgcagttcgccctcgtgcgcatccaggcaggcgccgcagccgttgatggccgacaccgccgtggaccacagttcgaagtccagcttctccacgcccggattgccgatgatgttcatccgcagcttggccggcagggtggtgtattcgtggttcttcatcaggtgcagcgagcggtagtagatgttgttcatgcccatgatggccgccgccgccttggccgcgttcagcgcctcgggcgacagcttcccgaagcggccgcctcacccgcgcgcaccaccgccggcacgccgatggcgtgggccgaggccaggaagcagccccacttctgctggtcgttcagcagcgtctcgttagcgagcgaagacaggttaagcgagatgtccttgccgtaggccgggatcaggtcgcgcagggcgtcgatcgacatggtcggaatcctttgaatgggtcaggggccggctcgcaccgcgccgcgcgcgggagccgataaagaaaaaggcggcgacggagatccgccgccgccttctcgtgacgttcaggcgaaaactgttacgccgccaggacgtcgccgcccaccgggcggttgcaggcgcacagctcgtcggtctgcagcgcatcgacgacccgcagcgtgtcttccggggcgcggccgacgttgaggttcgtcacatagacgtgctggatgacgttgtgcggatcgaccacaaaggtggcgcgcagggcgacgccctcttcctcgtcaagcacgccaagcgcgcgggccagcttgccgccgttgtcggcgaactgccagatcggcagcttgtcgaggtcggcgtgatcgcggcgccaggccagcttggtgaactcgttatccgtcgagccgccgagcaccacggtgtcgcggtcctcgaaatccttgccgagcttggcgaaggcggcgatttcggtcgggcagacgaaggtgaagtccttgggatagaagaagatgaccttccacttgccctcgaagctgtccttggtgacggtctcgaaggcggaaacgccattctcttcgtggctgttgaagcccggcttcacgccggtgatcttgaagtcaggcagggtttgtccgacgccgagcatcgcgaactccgttcaagttgaagactgaggcggcaaggggaggagcgccgccgacaccgacccatatgtgcccccgcccccttaaagtcaaatggatcatttcgccatccaccatagattttctctatgcagattgaacgaggtggatagattgtcccgttgctgacagcaaggtttatcgattggtttttggcgcggttccgtctcacactctcctctccagtctgctcagggaggtcatcatggacggcgaaagcgcccccaccccgcttcacaacccgcgtaaggagcccgccgcgctgcgctcgctgctgggacgcaccaatcgcgactggtggccgaaccacctctcagtcgacatcctgcatcagcagggcaagaccggcgacccgatgggcgacgacttctcctacgccgaggcctttaagacgctggacctggaggcggtgaagcgcgacctgcacgttctgatgaccgacagccagccctggtggccggcggactacggccactacggcccgtttttcatccgcatggcctggcactcggccggcacctaccgcaccggcgatggtcgcggcggcgcaagcgccggacagcagcggttcgcgccgctgaactcctggccggacaacggcaacctcgacaaggcgcgccgcttgctctggccgatcaagcagaagtacggcgccaagctgtcctgggccgacctgttcatcctggccggcaacgtggcgatcgagtccatgggcgggccggtgttcggctttggcggcgggcgagccgacgtctgggagccggaaaaggacgtttattggggcaccgaggagaactgggtcggcgacgacgccaatgaaacccgcatccagcccgacaaggacatggtgctggaagagccgctggccgcgatccagatgggcctgatctacgtcaacccggaaggcccgggcggtcgtccggaggcgctgcagtccgcgcgtgacatccgcgagacctttgcccgcatgggcatgaacgacgtcgagaccgcggcgctcaccgcaggcgggcacaccttcggcaaggcccacggcgcaggcgacgccaagaaggtgggcgtcagccccgagggcgccgacatcgcccagcagggcctcggctgggtttccggccatgagagcggcgtcggcgaccacaccatcacctcaggcatcgagggcgcctggacgccgacgccgatcacctgggacatgacctacttcgacatgctgctggatcacgaatacgagctggtccgcagcccggccggggccaagcagtggcagcccgtcggcaatcccgaagagacgctggccccggccgcgcacacgccgggcaagaaggtcccgacgatgatgaccaccgccgacatggcgttcaaggtcgaccctgcctaccgcgagatcatggagcggttccgcgccgatccggcgtatttcgccgatcagttcgcgcgcgcctggttcaagctgtgccatcgcgacatggggccgcgcatccgctacctcggaccggacgtgccgagcgaggacctgctctggcaggatcccatcccgcctcatcagggccgcttgatcggggaggccgagatccagcagctgaagcacgcgatcgcggcatcagagctgactgtcgccgatcttgttcgcacggcctgggcctcggccgcgacgtggcgcggatcggatcaccgcggtggcgccaatggcgcgcgcatccgcctggccccgcaaaaggactgggacgtcaacgagccggcaaagctggcgcgcgtgctgaaggtctatgaggacatcaaggccgcgtccgggcttaacgtctcgatcgcggacctgatcgtgctgggtggctcggtgggcgtcgagcaggcggcgaaggccgccggccacgacgtggtcgtgcctttcagcccaggtcgcaccgacgccacggacgagcagaccgatgcggaaggcttcaaggttctggagccccgcgccgacggcttccgcaactatctgcaggtgcagttcaacgtgccgaccgaagagctgctggtggaccgctctcaactgctggggctcacggcgccgcagatgacggttctggtgggcggcctgcgcgtgctgggcgtcaaccatggcgcgtccgagaacggcgtcctgaccgaccggccgggtcagctgaccaacgacttctttgtcaatctgctggatatgcggacgggctggaagcaggtcgacgacagcagcgacgagacctttgtcggctccgatcggctgacgcacgagaagcgctggaccgccacccgcaccgatctggtgttcggctccaactcgcaactgcgggctttggcggaggtctacgcctcggccgacgccggcgagaagttcgtccgggacttcatcaaggcctgggtccaagtgatgaacaacgaccgctacgacctgccgggaccggcgctgcacgccgaaaaggtcggcgcctgacgcggacggacccgcctcgcgcaccggcggggcgggtccgtcgataaaacaaaccgatgatgttttatccggggatagcgagcgcctatgacgcacgcatgctcccccccccgcgtcagctccagtatctgaagcttctggccgagcacggctcgttcagccgcgccgccgaggccgcccacgtcagccagcccgcgctgagcgccggggtgcaggagctggagcgtatcttgggcgcgccggtggtcgagcgcacgcgcggcgcggtgctgctgaccgcggtcggggccgaggcggtcaagcgcgccgaggacgtgctggcccgcaccgaggatctggtggaggcggcgcgcaacgccggccgccccctgtccggccggttccgcctgggcgtgatcccgacggtggcgccctttctcctgccggccaagctgccgggcctgcgcgacgcctatcccaagctcaagctgttcatccgcgaggacctgacgcctcggctgatcgccgcgcttaaggccggtcatgtcgacgccgccgtgatcgccctgccttatgaggcctcggggatcgagcacgcccgcatcggcgacgacgaaatccttgcggcggcgccgacggatcacccgctggcccaagccgccaccgttcgaccgggatcgctgaagtccgacgacctgattctgctggaggacggccactgcctgcgcgatcaggctctggccgcgctcgacatcgacccaccgcgtggagacgacgtcttcgccgccacctccctgcacaccctggtgcagatggtcggatcggggctcggcgtctccttcctgcccagcatggcggtgaaggcggggctggccgacaatccggccgtggcggtgcggcccttcgcccgcgacgacgagccgccgccccgacgagagatcgtggtggcgtggcgatccggctccagccgcgcggccgaggcgcggctgctggccgaagccctgacgctggattgataaagaaaagggccggcggatcgctccgccggccctccttgttccgatcaaccgccgcttattcggccgcttcgctgggggaagccgcttcaacgggagccgcttcgaccggagccgcgacggccgtttccggtccgcgcgccaggttgcgcaggacgtagggcatgacgccgcccgccttgaagtagtccagctcggtctggttatcgatgcggcagcgcacggggaagcgcgccatcttaccgtccgacggacggaacagctcgacccaaagatcctgacgggggcgcagcttgccgatgttcacgtccgacaggccgcggatggtgacgatctcctcgcccgtcaggcccagcttctgccagccgtcctgcttgaactgcagcggcaccacgcccatgcccaccaggttcgagcggtggatgcgctcatagctttcggcgatcacggcgcgaacgcccagcaggcgcgtgcccttggccgcccagtcgcgagacgagcccgtgccgtattccttgccggcgaagaccaccagcggccgcccctcggcctggtagcgcatcgccgcgtcgtaaatcgacatggtgtcggcggacgggaagtgcttggtcacgccgccttcgatgtcgggcgtgatcctgttgcggatgcggatgttggcgaaggtgccgcgcatcatcacttcgtggtggccgcgacgcgcgccgtaggagttgaactcgctggcctccacgccgcggttggtcaggtagacgccggcgggcgaggtcttcttgatcgaaccggccggggaaatgtggtcggtggtgatcgagtcgccgaagatggcgagcacgcgcgcttcgacgatgtcgctgaccggggccggctccatcgacaggccctcgaagtagggcgggttggcgacataggtcgaagagtcgtcccaggcgtaggtctgaccgcccgtgaccttgatgccctgccagtgcttgtcgcccttgaacacgtccttgtagcgtttggcgaacatggacggggtcacggacttgcgctggatctcggcgatttcggccgccgtcggccagatgtcgcgcaggaagacgtcattgcccttcttgtcctgggcgatcggctccttggtgatgtcgatgcgcatcgagccggcgatggcgtaggccaccaccagcggcggcgaggccaggtagttggcctgaacgtccgggttcacgcgaccttcgaaattgcggttgcccgacagcacgctggtcgcgaccaggctgttgtcgttgatcgccttggagatggccgggtccagcgggcccgagttgccgatgcaggtggtgcagccgtagccgaccaggttgaagcccagcgcgtccagatccttctgcaggccggcgtcggtcaggtagtcggtgacgacctgcgagccgggcgccagcgaggtcttgacccacggcttggccttgagccccagcgcattggccttgcgcgccaccagacccgcggcgatcagcaccgatggattggaggtgttggtgcaggaggtgatggccgcgatcaccacgtcgccgtcgccgacggtgaacttctcgccctcgacggccgcgcgcggggcgtcgccgggacgggcgaaggtgccggtcaggtggccgtcgaactcgggcgcggcgttggtcagctcgacccggtcctgcgggcgcttgggtccggccagcgacggcaccacggtggagatgtccagttccagcacgtcggtgaagaccgggtcttccgacgtctcgtcgatccacaggccctgcgccttcgcgtaggcctcgaccagggcgacgcgcgccttgtcgcgtccggtggcggtcagatagtcgatggtagcgcgcgacacagggaagaagccgcaggtggcgccgtattccggggccatgttggcgatggtggcctggtcctcgatggtcatgccgaccagggcgtcgccgaagaactcgacgaacttgccgaccacgcccttcttgcgcagcatctgggtgacggtcagcaccagatcggtggcggtggcgccttccggcagtcggccggtcagcttgaagccgacgacttccgggatcagcattgggatcggctggcccagcatggcggcctcggcttcgatgccgccgacgccccagcccagcacggccaggccgttgatcatggtggtgtggctgtcggtgccgaccacggtgtccggataggcgactgtggtcttgccctcggtcagcgtccagacggtctgggccaggttctccaggttcacctggtggcagatgccggtgccgggcggcaccacgcggaagttgttgaacgccgaagagccccagcgcaggaagttgtagcgctcgatgttgcgctcgtactcgcgctccacgttctgctggaacgagcgcttgtcgccgaagtagtccaccatcaccgagtggtcgatcaccaggtcgaccgggttcagcgggttgatcttggccgggtcggccccgagcttggccatggcgtcgcgcatggcggccaggtccaccacggcgggcacgccggtgaagtcctgcatcagcacccgcgccgggcggaaggcgatctcgtgctcgaccgagcccttgttctcgatccaggcggccagggcgcgcaggtcggcctcggtcaccgagacgccgtcctcgttcctcagcaggttctccagcagcaccttcatggagcgcggcaggcgggaaatcccggccagaccggcttcctcggcggcgggaaggctgtaataggcgtacttcttgcgcccgacggatagatccttgcggacgttcaggctgtcgttcgacggcatagggaggggttcctctgatcagcgccgcccgacaatccggttgcgccttcgcgcgctggacgcaggggcgcacaggtccccggcgcgcgcggcgaaagcctgctgcggcgagcctgcctataatcccgcatgcctcagccgtccatgtatccacgccgcccgcagggacattgagaaccgctcgcatcgcaggcggccggacatgaggctgtcaacactccaggttacggacctgaccctctcgcgcggcgagcgcacgttgttccgcgatctgtcgctccacctccgcgccggagaggccgtggcgctgaccggcgccaacggcgcaggcaagacctcactgttgcgcgcggtggccggcttcatccggccggaccaaggcggcgtgagcttcgaggatgcggcgggcgacatcatcgaaccggacatggcgcgcggtcgcgacctgcaccttctgggtcatctcgacggcttgaaaggccatcggacggcgcgagatgaactggcgtttcagacgcggtggctgggcggcgcggacgcggacgtcgccgaagcggcggatcgcctgggccttgaacccctgctggaccttgaggtgcggcggctgtcggccggacagcggcggcggctggcgctggcccggctgatcgccgcgccccgatcgctgtggcttctggacgagccgctgagcccgctggacgcgcgctggcgacaggcggccggagagctgatgcaggcgcatctcgatcggggcggcataatcctggcggccgtgcacgaccccctgcccgtcgccgcccgcgccgtcgagatcgggagcggacggtgaggcgcgcggtcaccgtgctgtaccggcgcgagctggctctggcctggggcggcggaggcggcgcgctgttggcatgcgcctttctgctgtgcgtgacgacgatgattccgctggccgccggcggcgatccgcgcgtcctgagccccgtcgcctccggcctgacctggacggcgctggcgctggcctccctgctgtcgctggagcggatgttcgaacgcgaccacgaggacggagccctggaccttctgaccaccggccctttgccgctcgaagccgttgtggcggtgaaggcgctggcgcactggagcgcgaccggcctgccgctggcggtcgctgcgcccgtcgcggcgctggcgctcggtcagcccctcgggctggcgccgctcaccttttccacggcgctgatcggagggctgggcttttccttcaccggcgcgctcggggccgcgctggcgctgggcgcgcgtcggggcgggctgctgatcgccgtgatcgtgcttcccctgttcatcccgccggtggtgttcggcgcgggcggcctgcagcgggcggcgctggaccagccggtcgggcctgccctggcgctgctcggcgcctatgtgcttttcgcggcggtgatcgcgccgctggcgggcgcggcggctgtccgcaatgcgcagggctgagacgcttgcccgcaccccggccgccgcgtaagcgctgatcccgatgttcggcctgtcgaaccctgctcgtttcatggccttcacccggccgctgacgccctggctgtggggcgcggcgggcgtgctgctggcctgcggcgcctggctcagcttcaccgcccccgccgactaccagcagggcgacacggtgcggatcatgttcgtgcacgtgccggccgcctccatcggccttatggcctatgcggcgctgggggcagccagcttcttcgccctggtgttcagacatccgctggcggatgcggcggcgcgggcggcggcgctgccgggcgcggcctatacggcgctggccctggtcaccggctcgctgtggggccagccgatgtgggggacttggtgggtgtgggacgcgcgcctgaccagcgtccttgtcctgttcctgttctacctcggctacatggccctgcgcgcctcgatcgacgacgaggcccgcgcggcgagggcggcggcggtgctgggcctggtcggcctgatcaacctgccgatcgtcaagttctcggtggactggtggaacaccctgcatcagccggccagcctgttgcgcgccgggggatcgtcgctggccccgccctatctgcaggcgcttctggtgatgatggcggcctacggcgtgctgttcctggcgctgtggctgacggcgatccgcacggaggtgcgccgacgtcgggtgcagtcgatgcgcgcgcgacgggcgctggaggcgtgatgatcgacctgaacatgagcccctacgccgccttcgtctggccggcctggggaatcagcgcccttgtactggccgcgctggtcgtgcgggccggcctggccgcccggcgttggaaggcggcgctggccgaactggaagccggcgatgaataggtggctggcgctggccccgctggtcgtcctggcggccttggcggccctgttcatcggctggtcgttgaagcgcgatccggtgatcaagccggatgcgatggtcggtcagcccgttcccgcatccagcctgccgcggctggacggcgccgctgcggcggacatccggacgctggcggcgggccgcccggttctggtgaacctgttcgcctcctggtgcgcgccgtgccggatcgaacaccccaggctgatggagctcaaggcgcaaggcgtggtcgtgatcggcgtggcctacaaggatgatccggtcgccacccgcgcctttctggaagagctgggtgacccgttcgatgccgtcctggtcgatcgcgagggtcgcctcggtctcgacctcggcgtctctggcgtgccggagacctttgcggtggacgcctccggccgcatccgcgcgaaacaggccggtcccctgctggacgatcgcgacgtcctgcgcctgacccaggcgctgcaggcggattaacctttttcagacggattgcgttaacactcccgacatgagcgcgattcgtcccggactgccgcagatcgttccgcaaccggcggacgccggacgcgcgcgctcggcccaggctgcggccttcttccgcgccgccgtggatcaggcgcagacgaccaaccctgcggcggctcaggccccagcgcccgccctcgctttggtcgcgacgcgcgcgactggctccgcctcggcgcctgatcctagccggcccctgcggcctggctcgctgctcgacatccggatctagcggtcagctccagccgcggctggcgatgtactgttcaagcgcgttgatgcgcgtgtcgtcggacggatgggtcgaggcgaactgcggaacctgggtctggcgctgcgccgccatcagccgccacagcgccaccgactggctgggccgccagcccgccgcctgcagataatccacgcccagccggtccgcctccagttcgtcacggcgggaatacggaagcagcagaccgtactgcgcgcccagcccgccgatcgcgcccacggcccggccgtagtcgccggcgacgcgcgtgcccagctgcagcgcggcgttggtcagggcgctggaggaggtgcgctcggccgcgtgcggggccacgacgtggccgatctcgtgaccgatcaccgccgccagctggtcgtcgttctgcaccagggccagcaggcccgtggtcacgccgatctggcgggacggcagcacaaaggcgttggggctctggttggtgaagacggcgtagtcccaggtgcgtccgcccaggccggccgcctgcaccaggcgatcgccgatgcggcggatgcggtccacctgggcgcccgtggtcgccgcgttctgggtgcgcacctgctcggcccaggcggcgttcgactgctgcaccagcgagccgttgtcgacgatcagcagctggttgcgccccagcgcctcgttgtaagcgcaggcggccagggcggcgctggccgaggcggcgagcaaggcgatgcggacggcgcggatcatgtcgggctcctgcgggaaagattcagccggagaaaaccggcgatgcgcacagaggttcctgcggccaaacgcgctggcccaaagcaaaaaggcccggtccgaagaccgagccttttgcatttcgactggagcgggcgaggcgattcgaacgcccgaccctcaccttggcaaggtgatgctctacccctgagctacgcccgcactccgttgagagcgatgtgcgctccccgtcgaggagggggcgtatagcggaggggaatgccgtcctgcaagagcaaattcacaaagaatgcgctcaagcagcgagcgaccgcgtcgcaagcgtagcgccccctcgcctcagcgcggcgccaggcgaatggcgccgtcgaggcggatgcattcgccgttgatgtagacgttgcgcgccagctccagcaccagggaggcgtagtcggcgggcgtgcccaggcggctggggaagggaatggcggcggccagggcgtcctggatcttctggtccatgccggccatcatcggcgtccacatgatgccgggcagaatggtgttcacccgcacgccttcctgggcgaggtcgcgggcgaccggcagggtcatggcgtagacgccgccctttgacgccgaataggcggcctggccgatctggccgtcctgggccgcgacggaggcggtattgacgatcaggccgcgctcgccgtcggccatcggctccagcgtcaccatgcccgccgccgattgcgacaggacgcggaaggtgccgaacaggttgacgcgcacggtgcgctcgaacgccgccatgtcgtgggcgcggatctcgccggtgtccttcttgcgcgacacggtcttctggccggtggcgatgccggcgcagttgacggtcagacgctcctggccgtgggcggcgcgagccttgtcgaaggcggcggcgacggaggcgtcgtcggtgacgtcgacctggcagaacacgccgccgatctcggccgcgatcgcctcgcccttttccgcgttcaggtcgaacagggcgaccttggcgcccgtggcggcgatggcgcgcgccgtgccctcgcccaggcccgaggcgccgccggtgaccactgcggcgatgctgctgtcgagtttcatccctggtgttcctatgtttggctgaacctgatgtcttgcgagggatttagcggccatgaccgccaaagccaaaccggacccggccacagcgccgctggacgccatcgacccaaagaaggcgctggttccctccgtgctgcgcctcaacgaaatgcgggtacgaaagggcttctggcccaaggtggtgagcaccgccgcccgcatccccttcgctgatcagctggtcagcgtctggtacgccgcgcgcgatccggagacgcctctgccggccaagggcatgatgctgggcgccctggcctatttcgtgctgccgaccgacgccattccggacatcttcgcgggcatcggcttcaccgacgacgcggccgtgatcgcggccctggtggcgacgctgggcgccaacatcaagcgccgccaccgcgaccaggcgtccgacaccctggagcggctgaagagccgcgagcactgaggccgcgcttggcgaagccctgcgacgcaggctaagccgcacggccatttgcgacaggagaccactttccatgaccgccctgatcctgcacggcggcgccggcgcccggcgcgagcgcaactacgacgccgaggtcgtgcacatgcgcgaggtggtcgaggccatgagggcgcggctggacgccggcgacagcgcgctgaacgtggcggtggaggcggtggcgatgctggaagcgtccggcctctatgtcgccgggcgcggcgcctcgcccaatctggcccaggcctatgagctggacgccagcctgatggacggatcggaccagcgcgcgggcgcggtcgcggccctacagggcttcaagagcccgatccgcacggcgcgcgcggtgatggaccgcaccccccacgtcatgctggccggcgaaggcgcggccctgttcgcccacgatcaggggctggagccgatcggcgatgaggccgcctggttcacccacgccggacagggcgaggacaatcatccgcccaaagggctcagtcacggcacggtcggatgctgcgtgctggatgcgcaagggcggctggcggccgccacctcgactggcggcgtgttcggcaagatgcccgggcgcgtcggggacacgccgatcccggcggccggcacctgggcggacggccgcgtcgccgtgtccggcaccggacagggcgaatacttcatccgcgtcgccgccgccgggcaggtcgcctggcgggtcggctcgggccagtccctctccgaagcggctcagggcgtcatcgaccaaatcggcgagttgggcggcgacggcggcctgatcgcgctcgaccgcgaaggaaacatcgcccatcccttcaacagccagggcatgaagcgggcctggctgacgtcctccggccagatcggcgtggaggtgttcgggcgctgaccgagcgtcgggagccgctgcgggactgggcggacattaccggtctgtaaggtgcgcgccgcgagatcgctggtaaggattcccgcgcgcccggagggacgggcccaagaggaagcccgcctatgaagatccgcctgtccgccaccgtggccgcatcggccctgatgctggggctcgccgcctgcgccaccaccacgccgccgcaggcccccggcgctgatcagcgggtcgagacggccgcgtcgcagccgccttccggcgtggtcgtgccgccgctgggcttcgacaagcgggtgctggcgaacgggctggaggtctatacggcgcgcgacgccgacacctccaacgtcaccgtgcaggtctggtacaaggtcgggtccaaggacgatccggcgggtcgctccggcttcgcccacctgttcgaacacctgatgttcaaggccacccgcaacctgccgcccgagacctttgaccggctgaccgaggacgtgggcggctccaacaacgccttcaccgccgacgacaccaccgcctatttcgagaccgtgcccgccaaccacctggagcggatgctgttcgccgaagccgagcgcatgggctctctggtcgtcgacgagccgaccttcgtgtccgagcgcgatgtggtgaaggaggaataccgccagcgcatcctggccaatccctacggccgtctgttcggcctgttcgtgcccgagaccatctaccaggaaagcccctatcggcggccgggcatcggctcgatcgaggagctggaggcctcgtcccttgaggatgtgctgcgctttcaccgcacctactaccgcccggacaacgcctatctgatcgtcgcgggcaacttcgaccaagcgcaactggatcgctggatcgatcagtatttcgcgccgctgaagaaccccacgaccgccatcccggccaacaacgtcgccgagcccgagccgaccggcccgcgcgaggtcacctactatgcgcccaacgtgccgctgccggcagtggtgatcgcctggccgacggtgaagtacgcggatgcggaccgcgcggccctgacggtgctggacggcgtgctgtccaccggcgaaagcagccggctgtaccgctcgctggtctatgacaagcagatcgccgcccagatcggctccactcccgacttcgcccagcaggccggcaacctcagcgcgctcgccatcatggcgcagggccacactgccgaggaaggcatcgccgccctgaacgccgagatcgcccgcctgcgcgagcagccgatcagcgaggccgagctgaccgaggccaagaacgagctggtggcttccgccctgcgcgggcgcgagacggtggacgaccgcgcaaccgcgctggggttcgccctgatcaacaccggcgacgcttcggccgccgaccgcgagatcgcccagatccaggccgtcaccgccgccgacgtccagcgcgtggccgcccgctatctgacgccgcagcgtcaatcgaccatccgctacctgcccgcagacgccgccaatccgccgtcggttcagaagatgaacgtggatgcgccggtgacggtcgccgccctggctccggcgggcgagccgaccaccctgctgccgcccgaacagcgcgcggccctgccccagcccggcgccgaggtggcgccgtccaccccggcggtggccgaaagccgcctgtccaacggcatgcgggtgctggtcgcgccgacgcaaggcctgccgctggtctccgcccgcctcggcttcgacgccggttcgtcggacgatccggccggcaaggccggcgtggcgtccctgaccgccgccctgctgacgcaaggcacggcgacgcgcaccgcgccgcagatcgccaccgagatcgagcagctgggcgcaagcgtcggggctggcgccggagtcgacttcaccaatgtctacgccaatgcgccggccgacgtgttcccgcaggccatgaccctgatggccgatctggtgcgcacccccgccttcgccgccgaagagctggagcgccagcaggcccagacgctggacgccctgcgcgtcgccctgagccagccgggcgccatcgcctcgcaggtcgcgggccgggtggtgttcggcgacgccccctacggcgcgccgggatcgggcactgtggagacggtgccgaccgtgacgcccgaggacgtgcgcgcctttcacgccgcgcgctatcggccggaagacgccaccctggtcttctccggcgatatcacgcccgaagcggcgcgcgccctggccgagcaggcgttcggcgactggcgcccgagcgccggggcgccttccgccagcgccagccccgccgggcaggttcttccgccccgcatcgtggtgatcgaccagccgggcgccggacaggcggccgtggtggcggcggtgcggggcgtgtcgcgcaccgacgccgactacttccccctgacgctcggcaacaccctgctgggcggcggcttctcctcgcgcctgaaccaggagatccgcatcaagcgcggcctttcctacggcgccggatcgtcgctgggcgtgcgggcggatgcgggcctgttcaccgcccaggcccagacccgcaacgacgccgtgccggaggtggccgaactgatcctgcaggagatcggcaagctgggcgcgaccgagccgaccgaagccgatctggcgccccgacgcgccaccttgatcggcggcttcggacgctcgctggagacggtggacggcctgggcacgctggtggccaacctggccctctacgacctgccgaccagcgaccttcaggcctatgtcggccgggtccgcgcggtcacgcctcagcaggtggaacaggctttcgcccgccatctgccggtcaaccaggccagcctggtgatcgtcggcgacggcaaggtgttcatcgacgccctgcgcgcgcgtcacccgaaccttgaagtggtgaccgtcagcgacttggacctgaacagcggcgccctggagtaggaggccctcagcccgacaggcacacgacctgcgccacgcgaagatcgcggcgcaggtcgtcggccgccttgccgtagttgtcgatggtgaccgcttgcgccagcatcggctcgtccggcgtctgttcaccccggatggccggaagaaaggtgtcgggcgccgtggtgtagatgcggccgcggcgcggcgcctccgccagggtcacgccgacggcgcgtccccgcgcatccagcaccggcgctccggacagaccggagagggtgccgttcaggcccgcggtgcgtccgacctcggcccaggccagcaccggttcgtcgcgcgcgccgcgacctgtcaccttcagcgtctcgcggcccagcagccgcgaggtggcctcgcccggccggccttgcgggaatcctggatggaagccgcgttgccctttgcgcaaaggctccgccgtcgcgatcggcaccgcaggcgggccgccatcggtcagcagcagggcgatgtccgcatggggcgccagccgcacgtcggccgccaccgccttgccggggccaaccacaagggcgggctggcggcagccttcgaccacatggcgagcggtgatccagcgtccgcgctgggcgatggagaaggcggttccggcctgcggcttgaacggagcgtctgggctctgcaccgtcacggtctcatcgaacggcgtcacggggccgagcagaggcccctccccgtccgccggcgtcgcggacggggccggcagcgccggcggggcgtccgcattctcgcgccgcagcagcgacaggcccagcagcacggcggccgtcgccgcatagacggcccagtccggcggacggcgcactgccatcgctcagcccgtcagcgcggcggccaggatcagcgcggtcgcgagcttggcccccaccagcacgatggcggccggcgcctcgccgtgctcgatccgctgcggcaggccggtcaacagcgcatccaccacgcggaacgccagcagctgcagcaccaccgtcgccacgccccagatcaggatgtcccgaacggaggtcgacaccgacagcgacaccgccagcggaatggccaggccgaccagcacgccggcgaacgccaccgccgccgccggattgccctggcggatcagggcgatctccttccacggcgtcagcacggcgtagagggtcgcgcccgccgccagcagcagcagggtcgcgatcaggtgcagcaccatgaccggaaagccggaggcgaaggcctgcaactcggcgctgaagagagcttgggtcagggacgagtccatcagggctcacgctcaagagacccgacgcatgccccattgccgccccaatccgcaagcgcacggcggacacagtgcgttaggatttgtgtcgatgcgcgttctgcccgccgcgtgcgacaaggaggatgagcgtctaagccgccgcctgttcggctcgcctcagggcagaggcgcggaccttttcgctttcggacttcagctgcccgcaggcggccaggatgtcgcggccgcgcggcgtgcggatgggcgaggcgtagcccgcccggttcaggatggccgcgaacgcctcgatggtcttccagtccgagcagccgtagtccgtgcccggccaagggttgaacgggatcaggttgatcttggccgggatgccctgaatcagccgaaccagcgccctcgcctcttccggactgtcgttgacgcccttcagcattacatactcgaacgtcacccgacgcgcattagacaggccgggataggcgcggatggcggccatcagctggtccagctgatatttcttgttcagcggcaccagctggtcgcgcaacggatcgttggtggcgtgcaggctgatcgccagcatggccgcggtgcgttcgcccagcgcctgcagctgcggcaccacgcccgaggtggacacggtgatgcgccgccgcgacagggcgatgccttcgttgtccgagatgatgtcgatggcgtcggcgacgttgtccagattgtacagcggctcgcccatgcccatgaagacgatgttggacaggcggcggtcttccttgggcgacggccattcctccaggtcgtcgcgggcgacttggacctgggccacgatctcggcggcggtcaggttgcggaccagtttctgcgttccggtatggcagaaggtgcagttcagggtgcagccgacctgggacgagacgcacagcgcgccggcgcggccgacgtccgggatatagacggtctcgatctcgatgcccggcgcggtgcggatcagccatttgcgcgtgccgtccctggacacctggcgttcgacgatctctgggcgggcgagggtgaaggccccggccagcgccgcgcgcgtgtccttggcgatgtcgctcatctgggcgaagtcggtgacgccgtagtgatggatccagcgccacacctgcgaggcgcgcatccgcgccttctccggcgggcagacgccggcgtcgatcaacgcctggcgcagcgcctcgcgcgtcaggccggagaggttgacgggcgtcttgagggccgggctggaggcgcgcgaaaggtcgagcgtgacgctcacggacgaagttcccttggagttgagcccgtccttatagcacaaaggcgggcttttgcatggctgtcgatccgccagccatcgtcacccggcgcaactgcggctagggtcgagcgtcttggaagggtcgttcatgccgcctgtgtctgttttcgccgctcgaaacatcctggtcggagctgcggccgcggtcgtgacgctgtcctccgcgggcgcggcgctggcgcagacgcagccggcctatccgccgttcgacgcccgtagaggggtgttcagcttcgcgggcgggctggagaagtcgctgccggcggtggtgcaggtgacgacgctgggccagtcgcgcggacccagctcagccgacgatcccaagccgttctcttccgggtcgggcgtgatcatcgacgcgggccagggcatcgtcgtgaccaacaatcatgtggtggagggcgggcgcaagttcacggtggacctgaccgacggccggttgttcgacgcggtgctggtgggcgccgacaaggccaccgacatcgccgtgctgcgcatcgagccgggcggccgtcctctggacctgacccaggtgcgcaccgtcgattccgacaccctgcgcaccggcgacctggcgttcgcggtcggatacccgctgggactggaccagaccctgaccatgggggtgatctccggtctcaaccgctcgggcctgggcgatgcggtcgaggactacatccagacggacgcggcggtgaactcgggcaactcgggcgggccgctgctggacagccaagggcggctgatcggcatcaacacctccatcctttcgggcggcgccggcggcggcaacgacggcatcgccttcgccgtgccgacgcgcatcctgcagaccgtgaccgagcagctgcgcgaaaccggcaaggtccggcgcggcacggtgggcgccatcttcggctccctgacgccggagcgggcgcgcgagctggatctcggcatcgtgcgcggagcggtggttctggatgtggcgccgggatctccggccgagcgcgcgggcctgcggcgcgaagacgtgctgacgcggatcagcgcccgaccggtggtcaactcaggctcggtgctggcgaccgtgggcctgtcgacgcccgggacggagctggcggtggattacctgcgaggcggccgctcggcctcgacgcggatgttggtggcggaagcgccggccgacgagaatgaagatcggcccacaatcccgacgacctgaaggccagacagcagaacgcccgctctgccgggagggggaggggatggcggagcgggcgtctgcttggaggaagcaccggcccgtcgaagcccttggcggaaacatccagggggctggggggctgttcaggatccggacgcttccgaactccgacaggccgatgatgctggtgtcgcctctcaaccgggcgggcgaaggacggaaacggggccatttcgtgttgcgggccgctgtttgatcgtcggggtggcgtccggaggcggcgcgcctagattgaagccatgagcctgaatgcttcgaccgaccagccgccggccggccccgtctttttcgaccgccgcgaactggacctggtgctgcgggtctatgggcggatggtggcgcagggggaatggcgcgactattccgtagccgggcacaaggatttcgccgagttcgcggtgttccgccgctcgggcgacgcgcctctctaccgcatcgaaaaacggccggcgctccagtccaagcagggacaatgggcggtgatcggcgaaggcggccaaatccttcgtcggggccgcgatctcgcccaggcgctgcgcgtcttcgacgcgcgcaagttcaacgtggtggaataaagaaagggccccttcacaggggccctttccacatcagcctgtcagcggctcttagttccggttgccgcccatgaaggccagcaggaattggaacaggttcacgaagttgatgaacaggctcagcgcgccaaagcccgtcgctacgcccagggcgttctggtcggcgccgatggcgtaataggtcatcttcaggcgctgggtgtcgtaggcgatcagacccgagaagatcagcacgccgatcgccgagatgatcaggtagaaggtccccgactgcaggaagatgttgacgatggaggcgatgatcaggccgatcaggcccatgatcaggaacgtccccatccccgacaggtccttcttggtggtgtagcccaccaggctgagaccgccgaacgccgccgccgtcacgaaaaaggtcgtggccagcgagccgccggtgtagcgcaggaacagcacgccgagccctgcgccgatcgaggcgaccaccgcccagtacagcgtgttcacgccgcgcgcggtggggttcttcatgaagaacatcgaaccgaacaacagaaccagcggcgagaaggccacgatcatgcccagcagggtgtagccgacgcgaccgtccgccgttacctggaacatcagctgctgcacggccggcacattgccggtgacgtaggcgagggcgcccgcgaccaccaggccgatggccagcttgttgtagacgcccagcatgaaggcccgcaggcccgcatcaacggacatgtccgccgtctgcggcagcggccgggcgtagccgttgttgaaatcgctcatcgcgacatgtttctcccaatggcgccggcaagacgtcgccggtcgcatgaagccaatatcggaacctcgcggtcccctcgcaagcagaaccgggcttatcaggcgcggttccggccgctaccaacggtcgcatgccccgcctcttcaccgccctgaccctgccgccggacgtcgccgaggtgctagagcggcgccaatccggcctgcccggcgcgcgctggcgtccactggaggcgctgcacgtcacgctggccttctatggcgaggcgccggaccgccaggccgatgacctcgcctccgagctggcgcgcatcaccggcggtccgttcgagatcgccctgtcgggcgtcggcgcgttcggcgacgcgcatcgcagccacaccctctgggccggcgtggtcatgccgaacgaccccctgtccgtgctggccggtcgttgccggaacgcgggcgagcgcgcgggcctggtgatggaaaggcgcaactatcggccccacgtcaccctcgcctatctgaagccgcaggcgaacccggaccgcatcggcgcctggatggccgggcacaatctgctgagttcgccgccgatccgcatcgaccgcttcggcctgtattccagcgtcctgacgccggacggcagccgctacgagctggagcgtgagtatctgctctagccgctccgcttgcggccggaacggacagcgaacataagacagccatgcccgccgccgccgtgcacctggaactggtcttcagccgccccgaaaccacgctggcggtgacgcgcggcgcggcgcgcgccctggtggacctgggccatgcgccgcttcttgaggtctgtctgccgaacgggcggcgggccgacgtgatggcgctggggcctcggggcgagatcgtcatctgcgaggtcaagtccgggatcgacgacttccgctcggatcggaaatggggggagtacgcgccgttttgcgacgccttctacttcgccgtggcgcccgagtttccgctggaagcgctgccggacgggccggggctgatcgtggccgacggcttcggcggcgcggtggtgcgcaaagcggcgccggttccgctggcgcccgcgcggcgcaaggccctgacgctggcgttcgcgcggctgggcgccatgcgatcgctgcgagagtgaacggaacgtccgctcgccggttgttcaggctcgacacacaccgagaaaggacatccgatggcggacaaggacgaacacccgacgggccccggcgcgggcgaggagaacgacggcctgcacaagccggtcaagccgtctccggagctggccgaggtggtgggcgaaggccccatggggcgcgccgacgtggtcagcgcgctttgggactacatcaagaagaacgatcttcaggacagccaggagatcaaggccgacgacaagctgaaggccgtgtttggaaaagaccgcttcaccatgttcgagatgaacgcgatcctgtcggatcacctcaccgacgcctgatcgcgagcgtcagcgaggcgcccgcttggccagtatgcgctgcagggtgcggcggtgcatgcccagccggcgggcggtctccgagacgttgtggtcgcagagctcatagacgcgctggatgtgctcccatcgcacacgatcggcgctcatggggttttccggcggctcgggcgcctgttcgccgctggccagcaacgccttggccacgtcgtcggcgtccgcgggcttggacagatagtcgacggctccggccttgaccgccgcgacagccgtggcgatcgcgccgtagccggtcagcatgacgatgcgggcgtcggcgcggcgctcgcgcaccgcctccaccaccttcagcccgttgccgtcctccagccgcatgtcgagcacggcgaaggcgggggcgcccatgcgcagctgctcggtcgcctccgccaccgatcccgccgtggtgacctcaaagccccgcgcctccaacgcccggcccagccgggtgcgcagcgcctgatcgtcgtccagcagcagcagcgacttgtcggacagggcttggacgcgggtttccagatcggacatgggggccttcatctttcggtgtcttcaagtggcgttgcaacgcttcgggtcaagccgaactcggctgcgacgtttcgccccgatgccaggcgttcggcgcctcaagcgtcgcgcgcgaccagcggacggcgacccgggcgccgcgcccgccgcgttcggccgccaagccctgccccacgctgacctgtccgccgctgcgctccagaagcgtgcgggcgatgaagaagcccagacccatgccgccctggctgggcgcgacaggcgcgtcggcatcctcgcgcggtcggcgcggacggccggaccgggcggcgtcggcgatctgggcggccagcgcgcgccgggcctttccgtgcggccggctggtgacatagggctcgcccagacgcggcaggatgtcggaggcgaagcccggcccgtcgtccaggatctcgatctcgatccagccggcgtccaccaccgcccgcatgaccaccttggaggcggcgaagtcggcggcgttctcgaccagtgtggacaggccgtggacgatctcgggcatccgcttcacgcgcggcgacgcctggccgggcggggtcttcacctccagatcgaactggaggtcgaagccgcggtgcggggccgccacctcctcgatcagcgcctgcaagcccacgtcggcgtagaggacgcggtcctcctcgggctcggcggacagctgcgccaggatgccgcgacagcgttcggcctgctgcaggatcagggcggcgtcctcggccgccgcgctgtcggccggcgaggcgcgcagaagctccttggccaccacctggatcgtcgccaacggcgtgcccagctcgtgcgccgccgccgccgccagcccgcccagcgccgccaacctctgttcgcgttgcagcacgtcctgggtggtggccagcgccagctccagcttttcggcgtccgtcgccacccgccaggcgtagccggaggtgaacaccacccccgtcaccagcgccgtgcccaggcccagacggtaaagcaacggcagctccagatgctcgtgcagccgccacggcagcggcagcgaccagaagaacagcaccaccaccgccgtcagcgccatcagcccaaggacgcccgcatgtcgcgccgggacggccgccgccgccacagtcactggtgcgaccagcaggacgcagaacggattgtcgaggccgccggtcaggcccagcatgacgctgagctgcaggatgtcgaagccgagctgaaggccggtctggcgaccgtccggcaggctctggtccagccggcgcgcccgcgccatcagtccgaggttcaccgccgccgagaagccgatcacgctcaaacacggccataagggcagcgggaaatgcagggcgaaataggcccacaggatcgccgaggtctggcccagcagcgccagccagcggatcacgatcggggtgcgcagcgacaggccccgacctcgccccgtgatcccgcgcggcgactccgaccagccggacaggtccgcaaagctctgcgacgacggatgggcttctggatggctcaccgagcttctatagaccgacggaccgcaatccggaaaacaacgcccatgccccgccgctccattctgctgttcgccggcgcctgtatcgtcatcgccgtggcgctggctatcgtcaccttggtggtggtgtccgggcgcgagcgggcggcgggcggagagatggcggcgaccggacagccgctggtcggcggcgacttccagctggttgatcaggaagggcggccggtcgaccagacgatcctgaacggcaagtggagcctggtcttcttcggcttcacctattgccccgagttctgccccacgaccctggccgagatggccgcggtgcagcagcagctgggcgagcaggcgcgcgacctgcagatggtgttcatcagcatcgatcccgagcgtgacacgccgcaggcgctgaaggactatctgtcctctgatggttttcccaaaggaacggtcggcctgaccggcacgcctgagcaggtggcgcaggccgcccgcgcctatcgcgccttctaccagaaggtcggcgagggcgagggctatacgatgaaccacgccctgaccgtctatgtgatgggtccggacgggaagttccgcaccactctgggctatggcctcggcccccagaaggcgacgcagatcgtgcgcgacgccatggcgcggggctgagaggcgcgcggctgaggcggcggtcggcttcgtcagtggtccaccgggacggagatcggctgcggctaggccctgacgggccgatcgtgcggctgtcgatcaacccgcgagccaaacgtctgtcgatccgcatcgacgcccgcgcgggcgaggcggtggtggtcgcgccgcgcgagcggctgctggcgcaaggcctggccttcgcccgcaccaagaccgactggatcgcggaacggctggaggcgcggccggtcgggacgccgctggcgcccggcggcgtggtgatgttgaagggagaggctgtgacgctggtcgccaccggcggcgcgggcgcggcccagctcggccggacggcggaggggccggccattctgtcgggcggagagggcgaggccttcgcccgccgcgtcgagaacctgctgaagcgtcacgcccgcgacatcctgaccgcccgcaccgccgtgcacctgcgcactctgggcgaggcggcggggtcggggccggctcgggtgtccatcgtcgacacccggtcgcgctggggctcgtgcagccctcacaaccgctcgatccgctactcctggcgggtggtgatggcgccggagccggtcatcgactacctggctgcgcacgaggtcgcacacctggtccacgccgaccacagccccgcctactggagcgtggtcgaaagtctgatcggcgaccaccggccgcaccggcgctggctgcgcgagcacggcgcggcgctgcacgccgtcggcggctgagcggcccctagaagaacagggtgccggggcggcgctcaggctccgggcggttcggcggcgggacctcggcgccgccgcgcgacggacccggctgcggcgaggtcgggcgcaccaccggcgggccgtaacccggctgcggctgaggttgcggctggggcctggacggttcggcgtagggatcgccctcgtaaggatcgacgggctcggacggctgaccgcccggatcgccgcccatatccggatccatgccgcccagcccgctcagcaggtcgccgaccggatcgggcgcctgccagccctcgggcatcggcgggccgccggggatcggctgaaccgccaggcgcggcagggccgcctccatgaagccccgccagatggcggcgggcgccgcgcccccggtcacgccgcgcatggcggtgttgtcgtccttgcccacccagacggccgccacgaagccgccggtgtagccgacgaaccaggcgtccttgtagtcggaggtggtgccggtcttgccggcgatgtcgcgcccgccgatggcggccgagcggcccgtgccgccggtgacgactcctctcagcatctggttcagataggtcagcggcggattgttgatcgactggccgcctccggcttcggagcgctgatagatcgcccgcccctgcggcgtgcggatccggctgacgccatagggctcgaccctccggccgccgttggcgaaggcgtcataggcggcggccatgtcgatgggcgacacctcgaccgcgcccagcgccatggcgggctccagcccgatgcggctctggacgcccaggcgccgcgcgacgcgcgccacgctgtcgcgcccgatctggtcggcgatggaggccgcgacggtgttggtcgattgcgccacggcctgcgccagcgtcatctgtcccgcatagccgccggagtagttgcggggcgaccagttgccgatcgtcaccggctggtccaccacctgggtcgagggggtgtagcccgcctccagcgccgccagatacacgaacggcttgaacgccgagccggcctgacgacgggcatccaccgcgcggttgaattggctgtcggcataggaggcgccgccgatcatggcgcggacccggccgtcgccgtccaaggccaccagcgccgcctgttcgacccccttggagccgtcgcggtccaggatgcggcgcaccgagcgctcggcggcggtctgcagcgtcaggtccagcgtcgtctcgaccaccatgtcctcggtcggctcgcccaccagcccgcggatcgacttgtccagccagtcgatgaaatactgggcgtgctgggtggccagggtgcgcgacacgatcaccggctgggtcaccgcctgctcgcgctgggccggagtgatgacgccggcctcctccatctcgttcaggaccacggtggcgcgggccgccgcgcgctcgctctcggacaccggcgaatagcgcgacggcgccttgagcaggcccgccagcagcgccgcctcgcccaccgtcagctggcgcgcgctcttgtcgaagtaacgctgcgacgccgcctcgatgccgtatgcgcctgcgccgaagtagactcggttcaggtacagagcgaggatctcgtccttggagaacttcatctccagccagacagccagcatcagctcctgcaccttgcgccgcatgttctggtcgggcgtcaggaacaggttcttggccagctgctgcgtcagggtcgagccgccctgcaccacccgcccggcgcgcatgttggtgacgatcgcacgcgacatgccgatggggtcaaagcccggatggtggtagaagcgccggtcctcgatagcgatgaacgcggccggcacatagtcgggcagggcgtcgaggtcggccggcggcgcctgctgggtgccccgcgtggcgatcagggcgccgttgcggtccagataggtgatggagggctggcgatcgacctcatacaggctggaggtgtccggcaggccgcgcgcgaagacggcgaagaagacgaccagaaagatcaggccccagaccgccaggaccgcgccccagtagagcagtcgctgaaaaggcgtgcgccggggccggcgcccgccgtcgcccgcctgtcctcccccgtagactggacccgccatccaaacctctcatgctcgcgcgccgcagccatcggccccgccggatgtctatcccggatgaaccgacgccgatacggccgcactcgccaagcgcggccgttcacgggagcgtgagcatctattccgccgaaagaaaggcgtcacgccctggggcgcgaccccgatcaggcgttggtccgcacgccgctcaacagcagttcaacctgacgctgagcctgctccgccaaaacgccggcgttccattcgtcatatgccgcgcggcggtagttcgacagataaacgtcccacaccagggcgccgagcagctgaaggtcggcgtcctgacgcagttcgccgcgccccaggccgtcctgcagcacgcgggtgaaaacggcgaccaggggctcggccgccttacgcgcgcggatttcggcctcctgcggctggaaccaggagcgggcgacgatggcctgcatcagcggcaggtggtcgagcgaagcgtggtagacggcggccatcaccgccgtcaggcgctggtcgaccgaggcgtcgccgccgctggcgtccgccgcgacctgagccagccggtccatctcgtcgaccaggaccgcctcgaacagctcggccttgtcctggaaattggcgaacacggcgcccgtggacatgcccgcgcccttggcgatgtcgcggatcgtggccggctcataaccccgctcggcgaagagaccgcgcgcggcgtccagaaccttctggcgtgtgcgctgcttggcggcctggcggcggttcagccgctggcctgcgtccgtttcagcggcggtgagggtctcggtcatgcggaaaactctacgcttgcgcttcctgatcaaggcggaagccggatactcagcctgggtgatgatgggctcggagccccgtgggacgctccgtcgaaccgcccgcagatcaccgatcagcggcgccttccaccatcgaaccgtgacgaaaatgggtcgtggagcccctcaaaattgtggaccaacgtcaggcggcgcccgcgtggagcatgcaggcggggggggcggctccgcctgaggccgggatgagggcgcatgaccgatgcgaccatgatccagggcgtctgccccgaccgcttcgccgccgtgcgcgacgcctttcaggccaacttcgacgacgctccggagggtctcaacgaactggccgcacgcttcagcgtctgcatcgacggcgaggtagtcgtcgatctctggggcggccactcggacacgggccgcacccaggcgttcggcgccgacaccctggttccggtgttctcgaccggcaaggcggtcatggccctgctgatggcgcgggcggtggacgccggcgccctgcgctacgatcagccggtcgccgacctgtggccggacttcgcgcaggccggcaaggcgggggtcaccgtcgcccagctgatgagccatcaggccgggctgccgggcttctcggaggcggtcgagccgtcgctgtggttcgagccggaggcggtcacggcgcggctcgcggcccaggcgccgatgtggccgcctggcacggcctccggctatcatccggtgacggtgggctacctcgccaatcacctgttccagcgggcgaccggccgcaccatgggacaagccttgcgcgaggatttccccgagctggatctctggataggcctgccggagagcgagcacggccgcgtcgctcagatgcgcaagcccaccgcggcgccgagccttggaaccattgatccgatcaagcaggcggcctttctggatcgcggctcggcgccgggcgggcgcggctcgacggagtggcgcaagatggaaatcccgtcggccaatctgcatgggaccgccgccgggctggcgcggatgctgggcgtcgtagcgaccggaggtcggctggacggcgagaccgtcgtttcgactgaggctctggagcagctgacgcgcgagcgcatccacggtccggacaaggtgctgccctacgacatcagctgggcagccggcctgatgcgcaacaccggcctccatgtctttgggccgggcgaacaggcgctcggccactacggctggggcgggtcgatggccatggccgatccggagcgcggtctgtcggccgcctatgtgatgacccgccagtcaccgcaccttatcggcgacctgcggcccaagcggctgttggaggcgctctacgccgcgctttagatcggctcggcggcgggacggggggcccggctccggcgccatgccgccagggcgaacaccgccgccccggaccagatgaagacaaacgacagggctctcagcggcgtgaacggctcgccggccatcaccccgatgccgaactgaagcgtcggcgccaggaactggatgaatcccagggtggacagcggcagccgtcgcgcggaccaggcgaacaccgccagcggcagcaccgtcgcgggcccgctggacagagcccacaaccattgctccggggactgaaagcccgccgcctgtccgtgagcgcccagccacgtcagcagcagcaggccgaacggcagcatcagcaggcattcgatgaacagacccgtctgggcgtcggccgcgacccgctttcggatcacgccatagcctgcgaagctgaaggccaggatcagcgacagccagggcgggcggcccagcgccgccgtctggatcagcacgccgccggccgccagcgcgatggcgatcttgccccagcggtcgatccgctcgcgaaacagcaccgccccggccgccatgttgagcagcggattgatgtagtagccgaggctcgcctccagcgtcgcatggtgggtcgtggcccacacatagacgctccagttggcggcgatcagcagtgtcgaaagcgccagccaacccaaggtcttcggcgtcgccagagcccggcgcgcctgcatcgcctgaccggccaacagcaccagcgcgccggcgaacagcaccgaccagaccgcccggtgcgccaggatcgggcgcggcgaagccgtgcgcggccatggccatgaacagcaggggcatgaagccccacagcccgtagcaggccacggccgccgcgagggcgcgcccgttcggcgccgccgcgccggcgtccgccaccggttcagaccgtgatggagcgatagcccgacgacgacttgatcacgccggtctcatccagcagctgggcgatctgcaccgcgttcagcgccgcgcccttgcgcaggttgtccgacaccacccagaagctgaggccgttctcgaccgtgtggtccttgcggatgcgcgacacatagacggcgaactcgccggcggcgtccaccggggtgacgtagccgtcgtgctcctgcttatcgaccaccaggacgccgggagcatcgcgcaggatctcgcgcgcctcgtccggctcgatggggcggtcgaactcgaccgtcacggcctcggaatggccgacgaacaccggcacgcgcacgcaggtgacggtcagcttgatggagggatccagcatcttgtgcgtctccttccacatcttggcctcctcgtcggtgtagccgtcgtcctggaaggcgccgatgaaggggatgacgttgaaggcgatctgcttggggaaggtcttgggcgtggcgtcgcccaggccgtagatggccttagtctggttccacagctcgtccatgccgtccttgccggcgccggacaccgactgataggtcgacaccaccacacgcttgatccgggccgcgtcatgcagcggcttcagcgccaccaccagttgggcggtggagcagttcggattggcgatgatgttcttctttttcgcatccttgaccgcgtccgggttcacctccggcacgatcagcggcacctcgggatcgccgcggaaggcggaggagttgtcgatcacgatcggtccggccttgccgatcttctccgaccattcgcgcgacaccgcgccgcccgccgacatcagcacgatgtcgaccttggagaagtcgaactgctcgatgtcctggcacttcaccgtgcggtcgccgaacgagacctcgacgcccttggacttgcgcgacgcgatggcgtgcagttcgtccacgggaaagctgacctcctccaggatgttcagcatctcgcggcccacgttgccggtggcgccgacgacggcgactttatagcccatgtttgttggtccttcggacgcgctaccgctcgccgcgcggcggcttgctgcttgagcgcgaggggagttgtgggtctgcatttaggccgtcgcgggcgcgaagcaatcgcttttcggcgcccggccccttaagtggccgcccatgacctcccacatccgccgcgcctacgacatccgcatcgaggaaggggtgatcgcgcccgatccggcgcagcgccaggctctgacggcgctggagcggctggaggaggacctggggcggcgcggcctgttcggctcggtcccggaggtgcacggcgtctatctgtgggggccgcccggtcgcggcaaatccatgctgatggacctattctatgcggccagccctgagcctcgaaagcgccgcgcccactttcacgctttcatggcgcgcatccatgacctggtccgacagtggcgcgaaggcgatgcgaagaccagaaggcgcgtgttcgacacgcacaggggagatgacccgatcccgccggtcgccggcttgatcgcatccgaggcgcggctgctgtgctttgacgagcttcaggtcaccgacatcgccgacgccatgatcctgggccggctgttcgaagcgttgttcgagcgaaaggtggtggtggccatcacctccaaccgagccccggaagatctctacaagaacggcatcaaccgtcagctgttcacgccctttatcgacatcttggaaacgcgctgccaggtggtggagacggctggcgcgcgcgactggcgccgcgaccgcatgtcgggatcgcccgtctggttccagccgctggacgcctccgcgcgaggcggttttgaggtcctatggtcagacctcaagggtggagagccggaggcgccggcgcacctcgcggtgctgggccgcgaggtggtggtggagcgcacggccggatctctagcccgcgcgacgttcgaggagttgtgcggccgtccgctggggccgcaagactacctggcagtggccgagcgcttccacaccctgttcctggccgaggtaccgacgctgggccccggcaatcaccatgaggcgcgccgcttggtgacgctgatcgacgccctatacgaggcgaagacgcggctggtcgttctggcggacgcagcgcccgaagctctctatccggagggcgtcggcgcctttgagttcgagcgcaccgtgtcgcgcctcaacgagatgcaaagccagagctggctcacgcacgagcgcggctaggacacatcggcgtctgttctcggatgcacaaagggccgcggatcgctccgcggcccttcgtgcattcgatggaaggcggcttaagccagcgagccgtcgatgtccttgcaggcctggatcaggccctgcaccgactccaccgacttggccagcatggccttttcgtcgtcgttggtggtgaactgaacgatcttctccacgccgtccgcgccgatcatggcgggcacgccgacgtaaaggtccgacaggccgtattcgcccgacagccacacggcgcagggcaggacgcgcttttcatccttgaggtaggacttggccatggcgatggcgctttcggccggggcgtagaaggccgagccggtcttcagcagggccacgatctcgccgccgcccttgcgggtgcgctcgacaatggcgtccaggtcgccctggctgaggaagccggcctcgaccgcgtccggcagcggcaggccgccgatggtggagtggcgcaccatcggcaccatgtcgtcgccgtggccgcccagcgtccaggcgtggatgtcctgcaccgacacgccggtcttttccgccaggaagtaggcgaagcgggcgctatccagcacgccggccatgccgacgaccttttccttcggcaggcctgagaacttctgcagcgcccacaccatggcgtcgagcgggttggtgatgcagatcacgaacgcgttcggcgcatgcgccttgatgccctcgcccacggccttcatgaccttgaggttgatgccgatcaggtcgtcgcggctcatgccgggcttccgcggcacgccggcggtgacgatgcagacgtccgcgcccgcgatgtcggcgtagtcgttggctcccttcagcgacacgtccgagccgaaaacggcggtggcctcggcgatgtccagcgccttgccctggggcgtgccttcggcgatgtcgaacaggatcacgtcgcccagcgcctcacgcgccgccacgtgggccagggtgccgccgatcattccggcgccgataagggcgatcttcgcgcgagccatggggaggtctccggataggaaaaagaatgggtggcgggcggtctagcccccgcgcggcgcggctgcaagaaccgggctttacggccacgctcgcgcctgcgactagttcgggatccaacaggagtccgccatgcgcatcgccctgctgacaacgtcgctgctcgtcctcgccgccgcttcgcccgcgcttgcacaaacgcccgtgcagcggggcgagacctatgtgtccgcgccctggtggatgcgggcgccggtgatcgcctcgaccggcctggttcaggtcgatctgaccgcgaaccgcgcctatgtgtccgccggcttccgctcggtggatcgcagcgtggccgaggcgtcccgcgccgccgccgaccaggtgcgcgccgtcagccgcacgctgggcgcctatggcgaggacaaggtgcgggtccagacctctctgaccacccagccgctctatgatcagtaccgggacgaggacggcgtgctgcgtgagaaccgccgcgcggaccgcatcgagcgctatgaggcggtggccacggtgacggtgtacgtggacgacgtgtcgctgatcgagcgcatctacgccacgctgctggccgcgcgccccgcctcgctaggtcaggtcagcttcagcctggagccggaaaacgcctggaaggccaatctggcggccgaggcggtcaaggacgcgcgccggcgggcccagaccgccgcgcagtccgcgggcgcgaccctgggcgccgtcaagctgatcgatcccaccggccgagcttgccagacggacgtgctggtgggctggcctgcctatggcggctcggacgatgcggcctattcggtggatgcgtccgacatcgtggtgacggggagccgggtcggcgcgcctccgcctcccccgcctccgccggcgccgcctcctccgcccggcgaagccgacatcgacatggcccagttgacgctccagccgcccaaacagcggatgagcgacagcgcctgcgtcatcttcgagctgaactagaacgtggccttcgctccggatccggccttcgccaacggctccatcgccgtcacggactggccgatatgccatgtgcggcttcaggatgacgggcgtttcccctggatcatcctgatcccccgcgtggagggcgccgtcgagctggaggacctgtccgcagaacagcgcgcgcttttgacggaggagacggtgcgggggggccggatcgtgcgtcgcatcggcgagcggctgggccggccgatcgacaagctgaacacggccgccatcggcaacgtgacggcgcagctccacgtccatatcttgggccggcggcgcgacgatccgctgtggcccgatccggtctgggggcgcggccctgcccttccctacagctcggtcgccatggtcgaggcgatggacgagatcgccgcgggctgaacgcgcgtcagactgcgggcggcggtccgaagcggccggcctgatagtcgtggatcgcctgcacgatctcctcgcgcgtgttcatgacgaaggggccgtggctgaacaccggttcgccgatcggctgggcgtggcccagcagcacgaccgcttcatccccggcggtgatctcgacggcgtcgccgtcatcgtccatctggacgagactccagggttcgacaggcgtcgcgccgacagagacacggccgcgcacgacatagaggaagacgttgcggcctctcgccaccgggctctcgaagcgcgcgccgggctccatgcgcagcaccgccagatgaatgtcgatcagcgactggatcggcgcatcgacgcccagccatgagcccgagacgggctccaccgtcacgcccgtatcggtgcggaaggtcgggagatcggacgcctgcagaccgacgtagttcggcgccgtcatcttcagccgaccgggcagattgacccacagctgcaggatctccatcggcccgcccgcccgcttgaagctctcgggcgacagttcggcgtggatcaggcctgaccccgccgtcatccattgcaccccgcccgcgcggatgatgctctcgccaccgccggagtcgttgtgggcgagttcgccctccaggatgaaggtcacggtctcgaagccgcgatgcggatgcggtccgaacggcaggccgcggttgttcggcggataggtctgcggcccgtgatggttcaggaataggaagggatcgatctgctcgatccccggcccgggcaccggccggcgcgtcaccaagtcgccgatgtcgacgcggtgggccgggtgctggcgcaggacggaacgaggctgaagggcgtctgtcatgcgtcgcatatagggtggaagaggcgccggaccagcgcgatggcgacccctctgcgttgaccctccggccccgcgacactaaagccttccccaccctcccggcgattgaattcactcgcttttgagaactattcgcatgaccgactccagcccggtgtccggcgaccatcccaaggatgcgcgcgacgaccagaccggccgtttcatccagcagccgaacggacgcatccggccgctgtcgccgcacctgcaggtctggcgctttcacctgaccatgctcggatcgatcctgaaccggggggcggcgatcgccctgtcggtcggcgccctgttcgtggcggcctggatcgcggcggcggcgttcgggcctgacgcctacgccggtttcgtcgcggtcatgggctcgcctctggggcttctgatctggttcggcctgacgcttgcggcggcctatcacctgacggccggcgtccggcatctgatctgggacgcgggctccggcctgacgcccaagtcggcgaccaatctgacgctggtcagcatgatcgccgccatcgtgatcgccctgggcttctgggcctatctgttcgcttccggaaaggtgacgctgtgagccgccagcagaaggcccttgtgaagggcgtcaaggtttccgagcgccacggcgcgggcgagtggacggccgagcgcctgtcctcgctgatccttatccccctggtgctgtggggcctgtggagcgcggcggtgctgtcgggcgcaggctacgacggcgtgacggcgtggttcgccagcccggtgaacgccgtgctgttggccgcgaccctgctgatctccatctggcacatgaacatgggcttgaaggtggtgatcgacgactacatccatcggcccggtccacgcggaacccttctggggctgatcgccgtgatctgcgtcttgctggcggtcgccagcgtcttcttcatcgtgcggctggcgctgggttccgcgccgctgcccgccggcttcggagcctgatttcggcatggctgcttacgagttcatcgaccacgaatacgacgtcgtcgtcgtcggcgccggcggatcgggcctgcgcgccgcgctgggcgccgcccagcagggcctgaaggtcgcctgcgtcaccaaggtcttccctacccgctcccacaccgtggcggcccaaggcggcatctccgcctcgctcggcaacatgggcgaggacagctggcagtggcacatgtacgacaccgtcaaggggtcggactggctaggcgaccaggacgccatcgaatatcttgtccgtaacgcccctaaggcggtctatgagctggagcactggggcgtgccgttcagccggacggacgagggcaagatctatcaacgcgcctttggcggcatgacgcgcaatttcggcgagggcccggtgcagcgcacctgcgccgccgccgaccgcaccggccacgccatcctgcacaccctgtacggtcagtcggtgcgccgcgaggtgaagttctttatcgagtatttcgctctggacctgatcatgcaggacggcgcctgcacgggcgtgacggcgcttcagctcgacacgggcgcgcttcaccagttccgcgccaagatggtggtgctggccaccggcggctacggccgcgcctatttctcggccacatcggctcacacctgcaccggcgacggcaacgccatggtgctgcgcgccggcctgccgctgcaggacatggagttcgtgcagttccacccgaccggcatctacggcgccggctgcctgatcaccgagggtgcgcgcggcgaaggcggctacctgaccaactcggagggcgagcgcttcatggagcgctatgcgccgaccgtgaaggacctggccccacgcgacatggtttcgcgctccatgaccatcgagattcgcgaaggtcggggcgtgggtccgaacaaggaccacatcttcctgcacctggaccacctggatcccaagatcctgcaccagcgcctgccgggcatctcggaatcggccaaaatcttcgccggcgtggacgtgaccaaggagccgatcccggtcctgccgaccgtccactacaacatgggcggcatcccgacgaactatcacggcgaggtgttgaccctgcgtgacggaaaccccgacagcgtggtgcccggcctgatggccgtgggcgaagcggcctgcgtgtcggtgcacggcgccaatcgcctgggctccaactcgctgaccgacctggtggtgttcggccgcgccgtcggcctgcgctgcggcgaggtggtggacaggacatcgagcgtgccgtccgcctccaaggcccagaccgacgcccacatcgcgcgtctggaccgcttccgccatgcggacggctcgaccccgacggccgagttgcgcatccagatgcagcgcgccatgcaggccgacgcggcggtgttccgcaccggagagaccctgcaggggggcgtcgacaagctgcgcgccatcgacgcggccggcgccgacatcaagaccaccgatcgcgggctgatctggaacaccgatctggtcgagacgatggagtacgacaacctgatcgcccaggcgctggtcaccatcgagggcggcctgaaccggacggaatcgcgcggcgcccacgctcgcgaggactatcccgaccgcgacgacgtcaactggatgaagcacaccctggcctggaaacgtcccggcgaaggcgtccagatcgactaccgtccggtgcacaactacaccatgtccgacgaggtctcgtacatcgagcccaaggcccgggtttactgatcaatggtccagctctccctccccaaaggctccaagccctccaccggcaaggtccacaaggctccggccggcgccaagaacgtcaagacctacaaggtctaccgctatgatcccgaggtggacgccgatccgcgctgggacgtctatgaggtgtcgtcggacgaccacggcccgatgctgctggacgccctgatccacatcaagaacagcatcgatccgacgctggccttccgccggtcatgccgcgagggcatctgcggctcctgctcgatgaacatcgacgggcgcaacaccctggcctgcaccaagggctgggacgaatgccggtcgcacaacatctccatcgcccccctgccccatcagccggtggtcaaggacctggtgacggacctgtcgctgttctacgcccaatacgactccatccagccctatctgcagtcggacgtggccgatccggaaaccgagcggctgcagacgccggccgagcgcgagaagctggacgggctgtacgagtgcatcctgtgcgcctgctgctcgacctcctgcccgtcctactggtggaaccaggaagagtatctcggcccggcggcgctgctgcagtcctaccgttggatatccgacagccgcgacgacgccacgcagaagcggctggacgacctcgaggacccgttcaagctgtatcgctgccacaccatcatgaactgcgcccaggtctgccccaaggggctgaacccggccaaggccatcgccgagaccaagaagctgatggtcgcgccgggccgcaggaagcaggcggcctgacgcgctgtttcgggagtcggagggaaccccctccgcgaacaaaggttcttggggcgcaatcctgcgcgcgctccaaggacacctcgatgaagaccgctattatcgccgcggccgcagccgccgctcttctttccgcctgcagctccatgcccaccggcgccgccgcccccatcgcagccgccgccgtcgatcaggccgcccccgccgcgatggactatgtccgcatggccggcgcgagcgacctctacgaaatcaactccagccaggtgcttctgcaaacgtcgcagaacgaagagcttcgccgcttcgcccagatgatgatcgatcatcacacccagaccaccgccaccgtcaagcgcgcggcggagaccgccggcatgaccccgccgccgccggcgctggacgcccgcaaggccgacatgatccgacaactgcagcaggcgcagggccaggcccgcgacaccctgtacatccagcaacaggtcatggcgcaccaggaagccctgaccctgcacgccagctacgcccgcaacggcgacgagcccgcgctgaaggccgccgccaccagcgccgtgccgatcgtctcgcagcactacaacgagatcagcgccatgcagggcggcgcttccatgtaagcggcctcagggcggaggatgggcggcgcgtcggctccgatgcgccgcccgtcttttcagtccgtccccgcagccgccctcagttccggattgcgatgcgtgcgatccgcgctatgacccgaccatggccaagatcacctatatcgagcacgatggaaccgagcacgcggtcgaggtgaagcccggcctctcggtcatggaaggcgccatccgcaacaatgtgcccggcatcgacgcggattgcggcggcgcctgcgcctgcgcgacctgccacgtctatgtcgacgaggcctggcgcgaggcgacgggcaagccctcggccatggaggagtcgatgctcgacttcgccgaggaggtcgagccgaactcgcgtctgtcctgccagatccgggtatcggacgccctggacggcctgatcgtccgcctgccggaaaaccagcactagggcgtcaaacaagctccggcgtggcgcgctcgatctcggcggcgtgccagcgccaggcggtgcgcacgatgtcgtccagcgttcgcgtcggggtccagcccagcacctcgcgcgcccgggtgttgttggccaccaggcatggagcgtcccccggcctgcgctccaccacctcgaccgggaagggccggttggtcgtgcggcggatggtttcaaccaactccttcaccgtggtgcccgtgccggtgccgaggttgatcgccgtggtctcgccgccgtccagcaggtagcgcagcgcccgcacatgggcgtcggccaggtccatgacgtggatgtagtcgcgcaccgccgtgccgtcgcgggtgtcataatcgtcgccgaacagcttgaagccctgcctcacacccagcgcggtctgcaccgccagcgggatggcgtgggtctccggatgatggcgctcgccgatccgcccctcctcgtccgcgcccgccgcattgaaatagcgcagggacaccgagcggaagccggcataggttgaatagtccgccagcgcctgctcgatcatcagcttggagcggccatagggattcagcggcgcctgcgggtgcgtctcgtccatcggcagccgcacgggatcgccataggtggcgcaggtcgaggagaacaccagggcctcgacgccgccgcgccgcgccgcctctatcagggtgatcgcccccgccacgttgttctggtagaaccgacccggcgccttgacggactcgcccacttcgatcagggccgcgaagtgcagcacggcgacgggctgatggcgcgcgatcacctgatccagccgcgccgcatcgccgatgtcgccttcctccaacggcccccactgcacgaacgccgcatggccgttcgacagattgtcgtagacgaccggccggaatccggcctgcgacaacgccaggcacacgtgcgagccgacataaccggcgccgcccgccaccagaaccgtctgcgtcatccttgatcccctctccccaggcgacaccaacccttgacccagccagcagttgcggcggcggacgatctttgtcgaggcgccgtcgctgaaccacctcgcacgtcatcttccggcttgaccgggcgagatgatatttcgtaacgctttcgcgcgttctcacgaggtctcgatgcacgttcgatccccatcccgccatgtcctgctcaccgccgccgcctggtctgtcctatccgcgccggctttggcccagactgttcagccctcggcctccccgtccgacagcacgacgctggaggacgtgattgtgaccggcgcgccctatggcgtcagccagcgcgccgcggtgatcgcgacggacgtgctggatgagcagacgctggcgacagcgccgtccgcatcgttgggcgatctgctgaacggccggccgggcgtgcgctccaccgacttcgcgccgggcgccagccggccggtgatccgggggctcagcggcccgcgcgtgcaggtgctgaccaacggcatcggtctgatcgacgcctcctcggtgtcgccggaccacgccgtcgcgaccgacccggccgaggccaatcgcatcgagatcattcgcgggccctccaccctggtgtatggcggctcggccatcggcggcgtcgtcaatgtgctggacggccgtatcccgaccgaaatccccgaaggcgggatcgacggcgtgatctcgggccaggtgtccagtgtcgatgacggacgcggcggcttcggccgcgtcacggtgggcggcgggaacttcgccttcaacgtcgacgccgtgaaacgccgcaccgacgactatgaaattccctccccctccatctcccagcgcctggcggacgtcgaaggcgtcgagcgagaaggcggagacgtccagcccaacagctacaccgacctcgaagcgtggggagtcggcggcgcctacatcggcgacaagggcttcgcgggcctgtcctacaaggagaccgacagcgaatacggcgtggtcgccgaggacagcgtcttcatcaagctgaaccaggagcgatgggacgcgcgcggcgaataccgcttcgaccggggtccgttctcggccctgcgcggctcctacggtcacgccgactacacccacaccgagttcgaggacgtgggcgagcccggcaccgtgttcaactcggacggctgggaaggccgcgccgacctggtgcaacgcgcgcgcggcggatggaacggcgccgtcggcgtccaggccctgtcgcgcgacttcgaggccatcggcgaggaggccttcgtgcccaccgtcggcatcgaggagatcggcgtctacaccgttcagcggctggatctgggcgaccacggcttcgagggcggcctgcgctacgaccgccgcacgctggacgccacgccgcttggcgaggacgccgaggtcgagcgcgagtttgacaactggtccgggtcggtcgccggcttcctgcgccccgcgcccggcctgttccttggactcagcctcgcgcacaaccagcgcgcgcccagcgaggtcgagctgttcgccgacggcgtccacatcgccaccgccgcctatgagaccggcgacatcgacctcgacaccgaaaaggtgaccacgctggagggcacggcccactacgacaggggccgcctctcgggcgacctgcacctctaccactcctggtacgacggcttcatcgacgagcgtgcgaccggcgaggagttcctgttcgaagaggaggacgagctcttccccgtctaccagttcgtgcagaccgacgcgcgtttctacggcttcgaggtcgagggtgcctacgccctgtgggaggacggcgaccgcaagctgtcgctggaaggcgccgccgactacgtccgcgccgagaccgacctgggtccggccgcccgcatcccgccgtggtcggcgaccggccggctggcctggaccaccgcccgctatgacgccagcgtcgaggtgcgccatgtgggcgagcaggaccgggtcgccaacgacttcgaactgccgaccgacagctacactctgctgaacctcgcagccgccgtgcgcccgttctcggaccgcaacgtcaccgtcttcgccgaggcccgcaacctgacggacgaagaggcgcgcgaacacgcctccttcctcaaggacatcgcgcccctgcccggccgcaacctgcgcgtcggcgtcgcctaccgcttctagcgggcgagacgacagtgttcgcaaactctcgcgagacaatcccgggagcctgtcgatcggactgaggctctcgtgatcacaagcaccagtgcgggatcaaggccatagaagcgctgaagtacacgatctcgttcgtgaggcttcgctccaacgaacatcatcgtatcgagatagcgatagaagccgcgattccgccacgtctgctcactgtgctcacttgcgctacatggatcgacgaacggtccagcgcggcgatgatgtcggctggtcgcacggcgtcaggaagccgtatccggtcgcgggatggaaaagccctgacgccagccccgacaaggttacgacttgcggcgcggccgtccaccagtccgcggcttccttccaaccgcgttgtcaaagtcgccgaacggccgctccaggatcatgccgcttgctcggacgtccggctcatctcaaccagcctccgcgtgacgacggcgcatagatcgggattcatctggcctggtattgctgtcagaaaccacagcccgtccgccgccagccgtgcgatgaaggcgtcgagtgcgcgaggatcgccgccgcgcggcatcggcggcgcccatcgttcgatcagccgccgccaggacgcctccagttccggatcatcgacgctttccatcatcagcagaagctcggcacggcgcgtggactgcgcacacatcgtgatgtaggccgcagagcgttcttccggggtcgcttcttcacagctcttgcccgccaccgcagcgagccccgcctcccaactgtcgatcagatgctggtgcgtggcccgtacaagcgcttcacgggacgggtaatggtaaagcaatcccgggcgtgtcagcccggtttgcgcggcgacggcgtcaagcgtcacggcggtgagaccgtggcgctcgacgatcgcgaccaccgcatccacgatctcgacgcgtttgctgccgcgggccatttcatcctcctcagtgtgagccggaatgggccgaggaggccgatccggcgccgtaccgtctgagcagcagacccgtccagacagcccccacggccagcgcggcggcggcgacatgaagaacggtcgcataggcgccgtcaaaggcggcgctcgccgcattgaccagagccgcaccgccagtcggatcctgtgcggcgacgccaagagccgcgatcatgctcgccgtcgcctcctcgggcgcaccggcgggcagcaccacgttcaccgtataaagataggccatcaggctgccgataatggtgacggcgaagagactgccgaactcataggacacctcctccaccgaggaggccatgccggctctggaggcggggacgttgccgacgatggctgtggaggcgaccgacatggccgcgcccagacctgcgccggtcaggagcagtccacccacgatccagccgagaccatgggtgacgccaaccgaaaccatcagaacggacgcggccccgaccgccagtccgccggcgatcaagttccgcaggccgatccggtgaagaaaggcgcctccgataagggccgtgggcaaggcgccgacggcgacccctgttacgagcaggccggcttggagcggtgtgaagccgacaacgagctggaaacgctgcgtagcggcgagctgtatgcccccaatggcgaaggtgatgaaggccgccgccagcacgcccgccatgaaggccggattgcggaagatggaaaattcgataagcggaaacgccagccgccgctgacggcgcacgaagaggacgctggcgccgattgcgaccaggagcgccagggcgggcactgtccagctttgtcccacatgcgccgcttccttgatggccaacacaagggcggacagggcgaccagcgcctggagcgaggagacgacatcccaaggcttggtgggatcgcccgccactttcggcgcgaagatcggcgttccgatcaaggccagcgcgaccactggcacgttgatgaggaacaccgagccccaccagaaacggctgagcagaagcccgctcaccaccggtccgagggccgcgcccaccagggagagggccccccagacgccgatcgcgagattgcgttcgcgctcgaccacgaaggtgacgcggatcagcgccagcgtggcgggcatcatcgccgccgccccgacggcgaggaatgcgcgggccccgatcagcatttctgcggtcggcgagaaggccgcgatcagcgaggcgaggccgaacaggaccaagccgacgacgaacatgcgccggtggccgatacggtcgcctagcgtgcccgcgccgagcagcaggccggccatgaccagcggataggcgttgatgatccacagggcctgggtcgcggatgcgccgagatcccgggtcagggtgggaagcgccgtataaaggacggagttatcaagagtgatcaggatcaccccggccccgacgatagtcaaaagcgcccatcggttgcggatctgcgtcgtcatcgtaggcacctgcgcgagctcaccagctttagtttacaaacatgtctgtaaagttcaagggcgggcgtcagcgcgttttatggtcttctgcgagaagatgcgcccggtgaggaagatcatatcggaaccgaaccactccgaccgcagctcacaaacacccatggtcggtgtcctcggcgttcaacttgcggggacgctccacagccgctcccgcggcttgcccgcgacgccgacaaggggctacagccaagaccttgcgaaggatcgcacggctccgacttgctgcagaagcccaagaccgccggaagatctcgccgaggtgctgcggccagcgatggtgagatgatccggaagtgggcaagcgacatggatgatctggaagcacggcggcttgctgctctcgcacgctacgaggtgatggacacgcccgccgagccagcttttgacgagattgcggccctcgcggccaagctctgcgacgcgccaatggcgatggtgaacctgattggacaggatcgacagttctccaaggcgaaattcggccccgtcacgagcggaccgacgctggagagttcgttttgcgccaaggcgatcctcgagaacgactttctcatcataccggatgctgcgcaggatccgcggttcaaccgcgatccgctggtggtgaccgcaccgcatctgcgattctacgccggctcagcgctcaagaccgaagaggggctgccgatcggcgccctgtgtgtggtggacacgcgacccaggcggcttagccagcttcagcaggaaacgcttagcgtgcttgcgcggcaggtgatggcccaactggacctgcgccgcgcgcgtttggagcgaagcgcgcagctcgccttgacgaagactgacgaacagaacctcggggtgatcctccctcggtttggtggacacccatgctagcttttcggagctggagaggagtgtctgatgagtgttcaacgccggaactttccggattctttcaagcgcgaggccgttgaccgcgtcgccaacggcggcctgagcgtcggggcggtggcccgcgagcttgggctgcacgagacggtgcttcgtcgatggatgacgcagttcggggtgcaggcgacgggggcgtcgcggcgccccacaacgcaggcgtcgtccccgtcgccgtcggatctggcggcggaggtggcccggttgcggcgagagaacggtcagctgcggatggagcgggacatcctaaaaaaagccgcgctcatcttcggagcggcctcccgatgaagttcgggttcgtcgatgagcatcgtcaggtctggccggttcgcgtgatgtgcgcggtcctgggcttgtcggccagcggttactacgcctggcgcggtcgccccgagagccagcggtctgtcgccaatcgcgagctgaccgaggatatccggctgatccatgcggagagcagcggctgttacggctcgccgcgcgttcacgccaccctgcggcggcatgggcgtcgggtcggtcgatcccgcgtggagcggctgatgcgccgcgccggcctgcggggcttggcggccttgccgcgtcgcgcccggacgacgaacagccgccacggttatcccatcgcgcccaacaggctggcccggaacttcgaggcggcggcgcccaaccaggtctggctcgccgacctcacctacatcccgaccggcgaaggctggctctatctcgccgccatcctcgacctgcacacccgcaagatcgtgggctggtccatgcgccagaccctgcacaccgagatcgccctcgacgccctcaacattgccgtcgaacgtcagcgccccgcgcccggcctgatccatcattcggaccggggcatccaatacgcagccgaagcctatcgatcagccctggcccgatccggcatcaccccgtcgatgagccgaaagggcgactgctgggacaatgccccgatggagagcttcttccacaccctcaagaccgaacgcgttcatcaccgcgtctacgccacccgagaccaggcgcggcgagacctgttcggatacatcgagggcttctacaatccccatcgcctgcactcagcactgggctatatcagccccgctgaggccgagcgcaaagcggcttaaccccgtccacttttacgggggaagatcaagaccgttcggccagccccttgcttaaacttccgctgctcgggcttgcgtttcggcgcgaggcttagctcatgggtaaacggattgaatgtctgtccgatcggctttcgcacatcatagacggctgcgaagtgcgccagcttcagcatgtccgcgtcgtcgttgatcgcctccgcggcagcggcctcgatgtagaacttgaggtgaccgatgttgcctttcgtcgcccagtgaagccgggccgcaacatcggtcttgccaagccccgcctggactgagaacggcatgccccggtcgaacgcgtcgcacaccagccggaacgtcggccattcctctgaaccatgacctccgtacgggcggagctgttggaacggcaagccgccgcggcccaccaactgactatcggctttgatcaggtcataggcacccggcagtccgatgcagacgacggacaaagtgttcagatcgacgatcttgcgaaggagcccgcgtccggctcccaggagccgcttgtcgttctcgcgaaagacctgatcgaactcgtcaagcaagacgagttcgaccttctgaacaaccaacgccctcatgaccatggaggcgagcatgggattggtcatccgcagggtgacctggaggcccaggctattggcgaaggcttccaggatgccgcgcataccgcccccaccgtccggcggcatatcgacataggccacgggacgaatgaggcctgtctgtccgacagacgtcgcgaagcgcgaagcgtagtgcttggtcgcgaaagtcttgccggtgcggctgtcaccgatcaccgccgcaatggtgccccgggcaggaaggccgcctttcaccgggaagtggaagcgttccaaagctgcgacggtatcggtgaactgcgggtgctcgacaacgagatcgcggaccgcgcgctgtttgtcggaaggagtcatgcgagtggccctccctcaacggtgcgcacagcaaagccgcgcgtgcgccgaagaaactcaagatcatcgacttcctggcacggcttatcggtgggaggctgttcgccaaacgccggaagcggctccgcagcaaggaggtcacgcagcgaagcgacctgatccttcggcttctcgacatcgaccgcgctgcggtaccggcgcatttcgtcggccccgatgaagcgagcaaccgccttctcgacactgcggcgtccgggatgacgaagaaaccgcatcgcgagctccgccagcgccgctttcgcttccacaagatcgtcgaaggccacgttgcggttggcggccttgacgttcgccagcacaacctggtgctggtgcaacgtcagcccgtccgcgtatttgcggtggcccaatgtcgcaggaacgtggatcggaatgttgcgatacggatcgaccacgacgatctcgccgaggttctggggatcgcggagaaccttatagcggctggacgaaccctcactgctgcgacggcggtgctgcgggtgctgaagcagcgccgacaggtctgggctttcgtagtttatgtggtcccagacgatgccgcccttctggatcgtgcggtgatcgacctggccagcaagggcgatgaagatgtcgcgtgacggcaaaggcggcgtgacaaacttcgccgccttctcctgccaagtcgccagcggctgagcgcccatgccgcggatggggccaagcgccttggtgacatcgacgtggtagatttcacaaatccacttcgtgaggatgtgtcgaaactgttccagcgtgagggccggctggccgagatgctcgtgctgactgcggtcaacgacgttgctcagcgttgtgccgggcaggcggtgaaccagacccacgcccagggtgcggaagaaccgttccagagagcccttcatccacggttggcgcggcgggcaaacctgatggctgaacccgagctcacggccagcgttggaaatgctgtcgccgaggaagtgcagggcaccgtcgacgatcagagtttcgatgcgtccgaagcagggccaaggcgtggtgatctcctccgataagtccttcggatagatcgtgtgcctcaggccctccagaaatgacgcgtagctgggcgcatccagtccgacgccgaaccccaaaaccatcgccgtcgcgcggtcgcggaagcagacgaggtcaggacggccgacgacaagaccgccggcgtcgactagagtgatgtctagcgtgcaatggtcgacctcgacctcctggtacgggcgatccggaatgtcgcgcgtcgcccaggtgcgattatgcttgcgggcgtggccctcgccgaaatgggcgagatcgaccaccagccggttttcattccggcagcgacgctgaaaggtgcgaagagaaggcggcagcaggcgaccgtgagggtcgatgtagcactcaggcaaggagagcctgtcaatcgcatccccttcttcttcatcgatccggctgacttccttgcagacaacggcataggcgaggtcgcagttctgaagatgcagccaagcctccactcccaggtcgatcgcgcggtcgagatgggcgggcagacgactgccgcgtgtgcccttcaggtcgtgacgattggagtatgcggccgttcctaggatttcaccccaagcttcgaactcatccatccagccgaggaccgaagtgaagcctggcggtggttcattatgcttctgggcgatcgaggcgattacccccagcaaccgcttgcgcgaccgtggcaggccctgacaggcctgtacgtactcgtgcttgcgcaggttagccgcgcgtgccttttcgccgatgaccaccggagagagcggagcgggcgccggggcgaccttcgacgatgcctgatgaaggtggaaacgtccctcgcgctgcaaccgagcaatcttgtcgtcacaaacgaggttcgactcgccggtttccatgtgcatcaacaaccactggccggtcgaaagccgcttttcgacaagccaattcgcgccgtccatcaccactacgctgttctggcggaaggcgaagcgcggggtcgaagaggtgggagcgatgaccatcagagcccccacacctgactagacggggaaaacggttcgcctgaatctaccttcgccttgcccgagaacgcgcacttcatcaccgtagtgaaggtctgctcataagtgatgccgagctgagccatcacttcactcaggccgcggatcgagatcggcccgtgctcggcgtcgagagcttgaagtacggccatctcggccttcgggtccggcgcgccgcaatgggccagcatgacctgggcattcgaaagctgaggctgacggcggatgtgccgctcggtgatcagccggaaatgcgcttcgtgatcttcttcatacgcgcgacggatgtgcggttcgagcttcgtccagtcgggtccctcagccagcgcgccagctttcacctcaacgacgatccggcggccgtcgcgcattctcagaacgaggtctggaacgtaatggcgccgctcgatcccattcgccgacgggacaaaataggttaggcggtgacattgaaccgcgtaggcttccacttgcgggtcggcgctgatgagcgcctgggcgtcacgctccaggaggctctcgaacggagcaggtccgagggccttcggggacgcgaaccagccgcggatcgacgagggaggcgagctccgccgagaagctaaccgaaggggcttggcgcccgcgacgagtcccagactctcgtcggacaaggaagagcgtagcggcatctgaaagccacgctgagtagccaaccccgtcattggctggcccccgtgcggcggcgcgtcgtcaactcttcatcagcgcgagactgttccacacggatgatctcaagatgacgagcgcaggctgcgcgaacgctggacatcatcgcgtcgtaccgcgcccactgcgctcgacgagcttcggccgcctggccctcccctgcctgcgtcggcagaaactcaccgtgaatctcgttcttctcggaacgcatcttagtcctccatgtagcgacctccgggtctaatcattcggaaatattcttgatggcaaaaaatgtcaatgatcatttcgaatttttctgctaagtggggttcatggcgacagcaggtgaaatgattggcgtcatcgcgagcgcgattgcgcgcccccaagcgacggtgacatcgttctatggggtgctcagaaaggggggcctcatctccaccaccggccgaggtcggagcgctcagcacctttcttcgttagatgtcgcgcgcattctgatcgtggtgctgtccgccgacgccctccaggaaggcgaggcggtcacccgcttggtgggcgatctttggcacgtccgcggcggcgatgatgatccggagccgcctcaagaactccagttcgaggctgcgctctcgcggttgattgcgttcctggcggatgttcaacacggccgcgcagcccaggacgatggcttcttgggcgacttgcgcagtggtggaatcggagttcgggttacagctacccacctgaccgccgaaatcatcgtaggctcccaggtcaccgagttctcgtccttcgaggagcccccgccggtctcgcatccggacgattgggaaggcctgcaggtgtgcgaccgactccttctacgtgccatgatggagggcatgtcggtcacgcgggggatagaccaaacagtgcttaagctggtggccgccgcaatgccttagcgctgctctggctaagcagacagatttcgtggtccaagtcgatcggtcggatcacgtttaggtagagctcaccgtacagctcggcccacactgttatgtctacggagcgctgctattgtggtctccagggaggctggagtggacgattccgccatacacgagtgggatgatagtggcgttgccgaagccgtggcggcctcggccgcggttgatacacgcaccgacaaccccgaagccgacctcgttcgctccgacttggtcgaacgcgtttttagtaccctcgccgccgacgcggagcgcggtgagggccatctgcagcgcaccgacatcaaccgaatttacctgaggaagcggctgtcgattgcagaatgtatcgaagtcgagagccgcctcaacgcagcgggatacgcgctcatcgatgatgacgaggaccctgttgacgatgagcaagcttctggaagccctggatcagggcgaaagccgaaatatctttcggctgcggaagagcgcgaactcggccgacgtattcagcttgcagcaaatctctctaacgatgcctcacacctagacagcgcctacgtgagtcgagttcggcaggatgctggggcggcccgcgagatgttcgtcgtcacgaacttgcgttgggtggagaagctagcgtggcggcgcggcgagcgccgctacatcaccttagaagacttaaagcaggagggcctcatcggcctgttgagagcagtagaactctacgaccccgagaggggctttcgctttaagacgtacgctacctggtggatcgagcagcgcatggaccgcgcaatcgccgacgaaaaccgcatagtgcgcctacctgttcatctccaagagaagcttgtgaaggtcagaagggctaaggccaaactgacgctcaccaatgggcggcaccccacagaggacgaactcgccgaagcgcttggcctcgatccggaacggctaatgaagctgctctggcgggtgcatgcgactgaagtggccgaaggcgactccctcattggggaagacacaacgctcatgtcggtagtggcagatgatgcggcaacgccgttcgaggttgtatctcagcgcgaactcgaggaatgctttgcgaatcttctcggggagctctcaccccgcgaagaacgcatcctgcggatgcgtttcggcatcggtatggatcgcgattacacgttggaaagcatcggacaagaatacggagtgactcgagaacgcatccgacagattgaggccaaggcacttggaaagctaaagcacccgagtaggagccgccgactgcgtggcttcttggacgcctgaaatggcgcggtatattgggttgggtgaggatgagccgtcagaggattccgagcgtcgggtagccaacgcactccgtgagcttccggacgactggatcgttatacatcatgtaagttggcaatcgcgacgaggcggtcgccaaggtgacggcgaagccgatttcgttgtgcttcatccaaaacgaggcttgctagtaattgaggtgaagggcggcggaatcgaaattcacgacggtcgatggtcaacgatcgacaggcgtggggatcggcacccgatcaagaacccctacgaacaggctaccgactcaaagcatgctctgctgggctgggtgaaagagcacgggctggcaggacgcgtgcgtatcggccatgcggtcgcgtttccacacatgtccaatttgccgaacgttggccccgcgggggcgactgcgattagcttcgccaggccggatttggacacgatcatctccacgatcgaccgatgctttgatcattgggagcttgaggccaagctcgccgtcaacgatacggcgaagctgatcggcctacttgctccgacggtctcgctcactcccaacctagccgggaagacagccgaggccgagcaagacctactcctgttcaccgcggaccaggtggaggcgttcgccggccttcgggcaaatcgtggcgggctcatcctcggcggagccggcaccggcaagaccatcctagccatagctcgcgcgcaacagctaacgaaggacggcttccgcaccctattggtttgctacaatgaactacttggcgcagacctgacgcggcgcaccgcgaacccgcccgcactcaccgccggcactttccattcgatctgtctggctgaagccgccaaagccggcctgcctgtgccaggccagaaggatgcggagtggtgggaacgccaggctcctgaactcctaatcgaagcgtgcgccaccacggaaacctcgttcgacgccgtcgtggtcgacgaggcacaagacttctcgcccctatggctggacgcgctgcgctgcctcatagctaacgacaaggacgctccattcttcgagttcgcggacccccgacaggacatctgggcacgggaatggtcgacagacccgcggcatccattcgtctacgaactcacccgcaatatgcggaacacgcgaccgatcgcggagcgggtggccgcgacgatcgccgtgacttgcaaggaccgcggcgtggctggacccacgccgatctggcgcaccaccgatggtgcaccccgcgaatctgatgtcgtcgccgcggtcgagcccttgctagaccaaggcctcacgcccgccagcatcgtggtcctctgcgaggatgcagccttagcgaatcgactgcgggagaggtcaatcggcgcctactccttcggccgctgggggagcagaggcctcccggttgaaagcgtttcaaggttcaagggtttggacgccgccgcagtcgttctagtcttggcggagaacaagggcccagcccaccaagcgcaggcctacgtgggtatgagccgcgcacgatcgctcctcgttgttgtggggtccggagcaaccaagaaggccgtcaactggccgtagctgtgatgtcgaaatagccggcgccgccggccagcgctttgcgcgacagcgccgtattgaacatccgacaggatggttcaccgagatgcaggcacacagcacatgccgccccagtgtcctcgcacccaggatccaacgcgcagcggtgctcgtcctctaccagcccgtccaacagatgatggagttccgactcgaacagcgcctgtaggccgccaagcacgaagtcgcctcgcgcggcggcgtacacgaagaacgatagggcagtcggcaggacgacctcggaaagggcgctacgttcgatacccgcgaaaaccgcggcgcgcttgatgaaggcgtgcgaataggagtgcaccagttcggtcacccgcacactcgtatccgtaggggcctccggggggcccatcgccgagacgatcgctgatgcagcggtccggccatcctcagccggggcgacgggtaggccgagctccaccagccatgcgtgcaccttgagcggatcaaggcggagtagcatcgcctcggtctgggctagttcgccgtagaccgtgtagtcgccgttcggatcgcgataggtcctgagccggccttcccccgccgccgagggcccccgtgtgtagccgaactgcgccgtgagcaccgggaacttgtcgatcagttcgacgcgctccagcccccctcgtgcgagcgctacaggatagacagtctcgtacaacgaccgcacgaaggccgtctccgcacgcgccagcaggtcggggatcgtgatgcgactttcgaaggtcgcaagtgcgatctgccgtgcttcgcgttcggccacggcccggatcgatgccggcagagccggcattgccgcccgagtgcccggcccagacggcatcacagcaaccatcgcgtcgatcgtggcagcgtcgaacccgcggtcctctagcaggcgccggaccgactccggattgtgagctggcgcggcgtcggtcaaccgccggccggccattcccgacagcacccattcgagggcccgttctccgccgccagcctgctcgatttgcgccaggatttcacgcttcggcgggttaatcatactgatcccgcgcggtttgaagaccgtgccagatcggtggaccgtgaacgacagcgccccaccttggtcgcagtcgcacgcggccccgaagccccgatggatcacgtcgttgcagaccgggcagtagaagatcaactccgcggcggacgcggtacctgggaaccggactgcacgctgctggtgcttcgggcacttgcggacatacggcgtctttatggacccgcaagcatcgtgataaccgacgaacggaagctggcccctccggcgccgcgagccgcactcgcaacggcctatagggtcgtcgtgcaggcgcttgcacgcctggcacaggtagagacgggggaacggctcgcaccaaattccctcatctttgttgagtgaccgaacgcgaactggacgctgctgatagaggtcatcgacgaatccgccgtcctgggcgttgtcgcgccatggcagccccgcgcggatcaactcctcccggagagcgccggtgtcgatggtcgactctaccttgggatcattccaccgcttgactttccaaatgccgccagcggcgtccactgtctgctcaggcaggtgtccgaagaggatttgagacccgctgcgatactccctcatcgggtactatccccctttaccggcgcctgttcttccacatcgcgcaatgacgtcatcggatgacctgtgggcgataggtcagaagggaaccgggaatcggcgggaggctccctcaagttgcgatcaaacatcatgaaccacctatgtagctggtcccgcatgaactcgtcttcttccgtcaacccaagcaccgacgcgatagccgactcatcctgctgcaggagatcaggattttgccggaccgcgttgttgagcgccttgatggtagtaatccggtctccggtggcgggctcgtggaccaaggtgaggcgcgcgagctccaagcccgaaattgtccgctccagaacgcggcggctcttgcgggtgattgggattggctcgacgaaccgatctccgtgcgacacgaattgcgggaacgcgcgatagacgctggcgtcccgctcgcgcgtcatcttcggcacgacgatcactattgccggccatttgcggccgacccgcgccgtcgcctgaatgaactcggccacacctaatgggaaggctaacatgatcatcacgttgagccggtcgatatcgacgccgtgggacatcatcgaggaggcggcgatcaggtggagccgctggtcgaactcggcttccgggtgttctagccggtcgagcgtcttgcgcacttcctcaaaatcggtgcgaccagtcagggtcgcaacgttgggcggcggcgtgagctcagcgtactgggtctcggacgagcggacgacagcatcaatgtcttggagagtattgccgtaaacgacgttggttccgtacaggtcgactaggaagttggcgtagctgggatcgacccgcaattcctcgcatatccgatcgggctgctggacgaggcgccggatggccgattggagggccacgacgagccggtcgacaacaaactccaccgtgagccggcgaggcgcgaacgccacataccggcgcatcagcctatcagagtcagcggcccagaagcctgcgccatcagtaggcggcggttgtgggaaaacacgcgccgcgcggcggtacagtacatcaacctgcttcaggtaccctgacaacgtcgcggaggaggccagaattttcggcttctgtccggaaagctcctcctggatgccgtccatggcgcactcgtaatgcgcatcaaccgcgccaaggctgtcgcgcaggaggtgcagttcgtcctgcagccggaagcttgctgggaagagctcggctgccatcgggagcgtagttgtaggtcccttgcagtcgggcacaaggcacccggtcgggaactcggtccgcttggcgtaagtgtagccgtgtcctggccttgaacatcttcccatcggcgcgccgagcaggccgcgcatgccggtatggcgggagatgtttgctgctttatcgagcgtgccgatgacgatagtaggaaggaaccgccaaatctcgtcatcgaccacgtggatcggcagagcttcgccagccactggacattcggtattgccgcactggtggtcgagcttccatagtactcgatcgaagctggtggtgaccgtgcgctcccgacaaaatggacaggcgtctaggagcaggaacgggttctgcatctcctcgatcttgtcagcgtcctcagtcgcccgctggctctccttcctgatgcggttcggagtggcgccgccgcccactaggaagccaagtgagaaagggtccccgtggatgccgacctcacggcgcaccagctcagccgccgccaaggcattggcaaaacgctgagtctgctggagggacagcatccgcaaagggaagcgagaccatgcggtgacgccggactgcttcccgcgcatacggtccagaaacgcagcagtgagcagcagtcccaggtaggtctcggtcttgccgcctcctgtggcgaaccacacaatgtcgacaatgtcgctctcgtcggccctctccacgaggcaacgaatgttcgctagcagaaaggcaaactggaagggcctccacttcgtgtagcggccgcgcgcagagatcgccatggcgcgattcatgagctggaaggcggtccgcaactgctcatcggcggccaacaaatcggcaccctgccttatgcgttcgacttcggattcaaactcacccttcgccttgcttgcctcggcacgcatcccgtcggaccagccatccacggaggcgcgcgcggtcagggcagcctcgctccacacctcgttgccccatccccggagaacctccagcaagtgttgggcgctggtcaccggattccccgcgagcacatcgaaatctaatgccggctcgggctcggccgacggccagaactcgggccgcgcgcggtcacttgccggtccgtcggatgttcgaacgacgccgtcgagatcaacgacaaaaccgcaattgatcccgtaagcttcaacgttgcggttaaaccggaagctgtcgggtagcgtctcaagttcgaacgcgaggcgtggcaagctctcgacagaaagctccgcttcgaagaagcggccctcagctagttcctcatcctcgggactcgtgtttacgaatgtaacttcaagagagggatggccgccgcggtatgaaacccgcgtcctgatctcggccgatagcgacggtgcgccagccgcggccaaggccgccgcgaaggtgtccgtgccggctcgttcgtccccggccgtacccggcacgtcgaggtcgatcgatacctcgatgcgttcggacttgtcccatgcccaccggaagccgctgccctcgtcggctcggcggcgccgccaaagtgcgaagcccacatgcacggtaaagcgccatgggccggtggtttccggcctcaacttcagcccaatcgcacatggctcaagccgatcctgtcgctcgtcggccaaggtgacgaagtccttgggaccaagacggccaagccagaaacgaccggtcggatcaacgggcgagaatgaggcctcgtcgccccgggcctccacctcgacccgacgctcgagccagcgcacaaagcgctccgcgactcggtagcgggcggcgtcatcttccgccgccgcgatgaatgacttcgccaagcctgcccccttctgcgccctaacttgctgccaccgatatcagctttgggtgccgctcgcccaattcggagtaaggtattcaccaagcttgtgcggctcgtgagctaccaagctgtgtccactgcgatcctcactcatcaatagtcagcggcacttccgcgcatcgcgtccctggcaatacgatcggccgtcgtgctgtgggtggtctgcagcttcgcattcgccgtcgatccgataagcaggccagccgcgaccaatggtgcgtggcgacggagtttggccagcccgacggccggcctgttgtgaccgaataccgcttcgatcgctgcatcgacgagcgccaccgacacctcgacctcgggctggaggatttgggtcagttcctgcccagcttggtccagttcatcgagcagcatgaaaggccgcgttcctccgacgccggcgtgggcccagacgcgctgcatgttcgggatgtccgcttgttcaacgtaggtagagacggcagagacgacggcttcgattctgggctggagctccgctggaatctcattcgagagtcgatcgcccaactctgcattcatttcgagggcgagtatttccttcgaactgccgaaataaaagtcaacagaccaataggcatgaccgtcgacaaaccggtttctaagttcgaagcgcacgccgctctttagctgcagactctgtattgcgaagcgaaaagtccggttaggacgaaaggccgagcccggtcggtctggcggcgtctcggcgggagcaggtactggcgcggtaagctgatcagaatggcttgagagtgccggcaactcatcaggcggcgtccctcggaaagcgtgacctatcaggtaactgaagtggggcggaacagcgttgcccaccattctcagtttctgggcataggtggcgccatagaactggaaggtgatcggaaacccttgcaggctggcacgctcgcggatcgtcagccggcggacggcctcaggtgcctctggagggttgatcacgatgctctcccgcgacacgcgagtgcaggtggctgtgatcgttcggacggccctctccaacggatcggggaaggccatcgaattatacacggtgtgggtggtcttgttggcgcgattgatccgaagttcttctgagttaagcggaacctcaggggcgtggtcgatgagctgcgcgcggggagtggtaatcccgtaaaatggatcgcgcaccggattctgcgctagcgcccggaccacgtccccgagggtagagcggccgaggccatggccgtaggcctgcaatagattcatatcaaagttgccggctacgcagcgttttcgacgttgcggaagcccaaactcttccatgttcacgacgtgaatctggacgccgaggtgggaaaagcactgaagccgtccgccgtccttgagctccttagcgatgattggagcgacgcgggggacgttctccatcgcccaagccttcggctttaggtgatccacgatcctcagaaaggtaatgatgtcttcaagaccatcctccaagtcgccgttgccacctcggttggagaaggagaactgtgtgcagggcggacttccaacaaccaagtcaatatcttgaggcaagtccgcaaacgacagccgacggatatccaccgtttgagcctggtggcggttgttcttgaaattggtttcattggctggcccccaccgttcgtaggaggcaacgacctcgactccggccagccgcaggcccagcgaccaaccgcctacgccagaatagagatcaatcgcccgcaatccgcatccagccgacatctgcccccctgtcgcgtgcaagatgaaagcctactcgcaacgaagtacaagatccagtgcgccgaagtgccgaattggtcagaaatttctgcgccctttaggtcggtatccgttttgagggccgtcgctcgagaggtccagcctgcaggagagctcgtcgtaaaaggagtatcttcggcgcatgcgccgtccaatcatctctgacggagtccaacctgttgtgacatccgacataaatggcgcacccgaagagattcgaactcctgacccccagattcgtagtctggtgctctatccagctgagctacgggtgcgcatgccttggcggcgagggcgggtctttagcggctggcggggcgaggcgcaagcgggcggcgaagattatctggcgttcggcggcggttgacgcttggcgggtgggcgcccgggggctaggtcccgggtctccccgtctgtccgcccaagggttcgccatgggaccgtttcgccgcctcctcgccgttctgctgacgcccgtcgtgctggccgcctgccagacgccggcgccgccggccacagcgtttgccgcgaccggcgcggctgaagcacagccagcgcgcgggccgttcgtcgcggccgccaatccgctggcggcggaggcgggtatggcggtgctgcggcgcggcgggtcggccgtggatgcggccgtcgcggtgcaggccgtgctgggactggtcgagccgcagtcctcaggcctcggcggcggcgccttcatgatggtctatgacgcacggaccggggcggtggaggcctatgacggccgcgagacggcgccggcggccgcgacgccggacctgttccaggagaacgggcgggcgctgcccttccgggacgccgtgctgtcgggtcgctcgaccggcgcgccgggcgtggtcgccatgctggcgatggcccagggcgagcacggcaggctggcctggcgcgacctgttcggcgatgcgcgcgcactggccgacgacggctttttggtcagcccgcgtctggcgggcatgatcgcctcatcgtcggcgcaggttccggaagcgggcgcggccgacgtgatccgctacttcacccggccggacggggagcggtatcgggcgggagaccgcctgcgcaatccggactacgccgcgacgctggaccggatcgccgtcgagggtccctcggccttttatcagggcgagatcgcccgcgacatcgccgccaagacgcgcgaggcgccgcgtccgggcgcgctgacggctgaggacatcgccgcctatcgccctctgaagcgcgacgccgtgtgtcgaccgtaccgactgtacgtcgtctgcgttccgccaccgccatcgagcggggtgtcgatcctgcagatgctggccatggccgagcagacgccggacctggcccaggggccgcagagccccgaggcgtgggtggcgttcgggcggctgcagcgactgatgtacgccgatcgcgaccgctacatcggcgacggcgcctttatgggcgtgccgctggccggattgctggccgaggactacgtcgcggcgcgcgcggccctggtctcccagatcgacggcccggtcgaggctggtcggccgaccggcagcggccccgtcggcgccgcccggacgcgcgagcccgccggcacttcccactttgtgatcgtcgacgccgaaggcaacgccgtcagcatgaccaccacggtcgagagcgtgttcggatcgggccggatgacgcacggcttcttcctgaacaaccagctgaccgacttctcgttttcgccgaccgaggcggacggcgcgccggcggccaatgcggtggcggcgggcaagcggccgcgctcgtccatgagccccctgctgatcctggaccgacagggtcggctggtcggcgcgttgggatcgcccggcggatccagcattctggcctataatctcaaggcgctgatcggggtgctggactggggactgaccatgcaggaggccatcgacctgccgaacctagtggtgcgcggcgacacgatcggggcggacacggcggggttcgatgcggcgacgcgcgaggctctggcgggggccggcatgcccctgaggccgaatgcgtcggagacctccggcctgcatggggcgatctggcgggacgggtcttgggacggcggcgcagaccggcggcgcgagggcgtggccctgaccgcgccctgatccatccggcctgatcagttcggcctgatggagaactgaaaggcgatcaggccctcatcgacgtcggtgtcgacgtcgggtccgaaattgacgccctcggtctcgatctcgcggtagaccacgccgagcgagccctgcatggcgccccggcgataggccacgcctatggaggcgtcgcccaaaaaggcgccctcgtcgcggctgtagccggagcgggcgtagtccccgtcgcgcgtccgggcgaagttgtagccgaccgcccggcctgaaccggcggcgtagacgaaccagcgcgagcgctcgccgaacaccttgtcgccgtccggcatcagcttcttcaggccggagccgacccgcagggtggcgcccgcctcggccgagccgccccggctgcccagcccgatgccggcgtggggggtcaggctgacctccaggccggaggcggtgcgggtccgcgcgcccgaccagccgcgcacatagcggacatcataggcggtgcggtccagttcggcctcgtcgatcggcgtcaccggcaggggtgcgccgtcggcgcggcgcagacgcccgcgggtactgaggctgacccggtcggtgaagccctcatgctccagccacaggtcacgccgatcggtcgccgcagcggcgcctgcaggcctgaagtccgccgtcagttcgaccgccggtccgaaggccgcgtccgcccgcgccgtgaacggcgcctgggcgtccagcttcaaggtttcggaagcggcgtcgcgccatgcgtcgggcgcccaggtctgggcctgggccggcgacaggccggccgccgcgccgcacagcacgcccccgcaacccgcgatccaagccctcagacgcatacgaccccctcaagtcggcgacgagccaccctgcaccacaagccggcccgcgccaatcgccaagttggcgacacattcgagaagcgaacgctgacgcttggcggagagttcctgcgtcagctgatcactgccaccggatcattggcaggcgaggcactcgtcgtagtcggtcttgggcatggagaagaggtccggctggttcggatcgatctcgtcttcggccttgtcctcggcgccggcgaaggcggcgcgctgcaccgacttggagcgcagatagtagagcgacttcacgccgcgttcccaagccgaccagtgcagcatgtgcaggtcccacttgttgacgtcgccggggatgaacaggttcagcgactgcgcctggcagatttccggcgcccggtcggcggccagctcgatcagccagcgctggtccagctcgaaggcggtcttgaacacgcccttctcgtcctcatcgagttcgtcgatgtgctggaccgagccttccttctccagaatggtgttccagacggcctcggtgttgatacccttctgctcgagaaggcgctccagataggggttcttgaccgcaaacgagcccgacagggtcttgtgggtatagatgttggcggggatcggctcgatgcccgccgacgtgccgccgcagatgatcgagatggaggcggtcggggcgatcgccagcttgtggctgaaccgctccatcacgccctgatcggcggcgtcgaggcacggccccttttcctcggccagcaggcggctggccttgtcggcttcgcggcgcaggtgcttgaacagccgcatgttccacgacttggccatggcgctttcgaacgccacgccctgcgcctgcaggaaggagtggaaacccatcaggccaaggcccaccgagcgctcgcgcttggccgaatagacggcgtcggccatggccggcggcgcgcgctggatgaagtcctccagcacattgtcgaggaagcgcatcacgtcctcgatgaagcgcggctcctcgcgccattccagaaaggtctcggcgttgaccgacgacaggcagcagacggcggtgcggtccacgcccaggtggtccttgcccgtgtgcagcatgatctcggcgcacaggttggactgcttgaccttcaggcccagcgccttctggtgcggcgccatctggcggttcaccgtgtcggagaagatcagatagggctcgcccgtctgcatccggatctcgaggatcttggtccacaggctgcgggcgtcgatggttttcctgacctcgccactcttcggcgactttagatcaaaggtcgcgccggccttcaccgcctccatgaactcgtcggtgatgttgatgccgtggtgcaggttcagcgacttcctgttgaagtcgcccgacggcttgcggatctccaggaactcctcgatctccgggtggaagacgtccaggtagacggccgccgatccgcggcggagcgacccctggctgatcgccagcgtcagagagtccatcacgcggataaaggggatgatgccggaggtcttgcccgcgcccttgaccttttcgccgatggatcggacgccgccccagtaggtgccgatgccgccgccgttggaggccagcgccacgttctcgttccagacgttctggatgccgtccaggctgtcgcccaccgcgttcaggaagcaggagatcggcaggccgcgatcggcgccgccgttcgacagcacgggcgtcgccggcatgaaccacagccggctcatgtagtcatagacccgctgggcgtggccggcgtcgtcggaaaaggcggtggcgacgcgcgcgaacatgtcctggtagctttcgccggccaggaggtagcggtcctccagcgtcttctttccgaaatcggtcagcagcgcgtcgcgcgagcggtcgattcggacgccggtctccacgaccttcagctgcggacgaagcggcgtcttcatccgctccgagcctgcgaagttggccgccatcagtgcttcgccgtcagccatatcgatccccatcgcgtgcctgagccaccagatgttgtgtctggtttgcttaagagagactaaatcaccttgttcaggggcactcaacatccactttccaaaaaggatgcctcgacaaacgcaccaaggctctgtcgcgctcgattcgcagtcgatcgcaggctggaatcgctggcctttgtccgctttgcacaggaccgcccacaggcggcttttttcccgtggaggaacgatgccccgagcgtggccgttcgcccatccatgacttcgtccgccctcaaactctttttcgcacgcgccgggcggctagcgcacgccgagttcgccgcactgggcgccatggcggtgatcgcgctgggcgtaatggcctttgtggagctggccgacgacatgaccgaggccgacggccaggcatgggacgcgcgcattctcgcgatgatgcgtccctatgcggatgatccctcgcgcccatggggtccgtggtggctgaaagaggcggcggcggacatcacgtcgttgggcggcatctcggtgcttgggctgttcgccacgatcgccgtggtctttctgctgacccaacgcaaatggctgtcctcgacgctgctggtcgtcggcttggccggaggcgtcgccctttcggagggtctgaaggcggtgttcgagcgcgagcgtccccccgcgatcgcccaggcggtcgagacgatcaacgccagcttcccgtccggccatgcgcttctgtccaccgtcttctatctcagcctcggtgtgatgctgacgcgggcctttccgcgccgccgcttcaagatcttcgtgctttgcgtgtcgatgatcatggcgctgctggtgggcgccacgcgggtctatctgggggcgcactgggcctccgacgtgctggcggggtggagcgtcggcgcggcctgggccatggcgctgtggctcgtcgcctatgcggtcgagcgcttccagcaggcgcgccgcgccccgcttcaggatgcgcccacccccccccccatctgagcacccgcgagtcgtttccgcttgcgccccggcgaccgccgggcgtaaagcgccgctcgtcatcggggagtagccgcccgcgccgatcatgcggggctcgcgtcaacacactttcccttcgcccggagggaatggcgcaagacgccggaaggaccagcagggtcgatccggcacggcaagaccgctggctttcgcagggtgcatccacgcggggcccggctgcgaacgccacaggtccgtccgccgaggatccccgcgcaaacgagaacggcttttggaggcctttctgatctcgaccggcctggtctccatcgcggagatcggggacaagaccatgttgctgtccatcgtcatggcggcgacctggcgcaggcccgcgcccatcattctcggcatcctggcggcgacgctgctgaaccacgcctttgcggcgctggccggcacggtgctggcgcaatttatccagagcgaatggatgcgctggatcgtcgggatcgctttcctcggcttcgccggctgggcgctgatccccgacacgctggaagaccagtcggccgaggttcagcgcggcttctgggccatcttctggaccaccgcctcggcctttttcctgatcgagatgggcgacaagacccaggtggccaccgccctgctggccgcacggttcgagagcctgcccgcggtggtggcgggatcaacgctgggcatgatgctggtcaatgggccggccgtgttgctgggcgaaacggcggcccggcgcctgccgctgaagtggatacggatcgcggcggcggcgggtttcgccgccaccggtctgtggatcctgttcgccggctagatctcgaacacccgatagggcgtgtcgcccagcgtccgcagcacaggcagggcgacgttgtagaccggcacgcccttgttggtgcgcccctcgtgcgcgccgcggtgggcgtggccgtggaccaccagcttgacgttgtcatagcggtcgatggtctcggccagacgcgacgagccgagaaaggcgtggatttccggcggctcgcccatcaccgtctcgacgatcggcgcatagtgcagcatcaccaccgagcgttcggtccgcagcgtgcggatcgaggtgtcaatggcgttggcgtcctcgatcgcctcgcctacgaaggtcttgatcgactgctcgccgaacgggctcagcatatagcggccgaagccgccgacaaagcccttgccgccggcgaatcccacgccctcgatctcataggcgcgtccctcgcccagcatcttcacgcccgcatcgcacagcatcctgaacacgtgatcgggctggccgcactcgtgctcgtggttgcccagcacgcccaccatggggatgcggcacgccttgaggtcctccagcaggatctcgacctcgcgcgtcttgccgtagttcaccaggtcgccgcacaggcacagcacatcggcctcgtcgccgacccgctcgaacaggtcgcggtaggcccgttccgacgtctcgcccacatgcaggtcgcccaccgccgccacccgcaacttgcgcgccggcccctggtccatgccgggctggggcgtctgcgggtcggtcgccggcgcgtcgtttgcggcgtccgacaggctcacgggatcagtggacggggtcatggcgctcctccaggccctttccgaccacatcgccgaaaccccattcggagatatcggccacatagtcgcgcgggctgaacagacggccgcggcacaccttcacgcgcggggccggcaggtcgatctgggcctccagccgctcgctgagctcctccatcagccagcgcggcacccggtcgcgctcggtcggataggcgaagcgaaagttcagcaggtgcgacatcagcacctcccagtagaggtccatctgatccagcaggctcttccagtcgatggcttccgattgcttcaggatcacgtggttcacatccgcgccgtcgtagcgatagcgatcctggatgaagaccttggacaggatcagggccgtcggcggcgtgatcttcacctcgtgtccgtagaccttgatgacgtcgccgccgaaccaggcgtccgacaccgcgatggtgccgttggacatggcgaagatgacgtcgaagaagtgcttgtcgtccttccagaccttggcgatccagcgctcgtcctcgacgtcggtgcgataacccttggcctggaagaaggcgaggatgcgggggtagtcgccgggcttacagaacacgtccagatccttggtgggccgccggatgccggtataggccgttaccgcataggttccggacagcaggaacggcacgcccgactccttcagcagccgcaggctctcctcgtagaacgccagcgcatcaggcggcggctcgaaggtcggttcgaggatcacatcggacatgtcgcggcccttgatttggtcagtgtaggcaaacggcggcggaagcggcgcggttccgcttgcgccgtcgggcttcgaccctcgagcgtcgccgtccgtgcggattcatcaacaggctcatccccatctgattgaagtgccgacaccacatttggtgttcatgacgaaagttgatcgcaacatctgcgaaacaacacttggcgccgggcgcatgcggccgcatggtgaagcgatcctttccgaatccgccaggcctcttttcgatgaacgctcacagcccgatcatccgcccggaaggcgcgcaagccgccggcctcctgaccccctcgctcgcctacaagccgttccgctatccgtgggcgttcgacatgtggaagaagcagcagcaggtccactggatgcccgaggaggtgccgctgggcgaggattgcaaggactgggcgaccagcctgacggagggcgagcgcaacctgctgacccagatcttccgcttcttcacccaggcggacatcgaggtccaggacaactacatggagcgctacggccgggtgttcaaaccgaccgaggtcaagatgatgctggccgccttcgccaatatggagaccatccatatcgcggcctacgccctgctgctcgagaccatcggcatgcccgagagcgagttcggcgccttcatggaatatgaggccatgcgggacaagcacgactacatgggccagttcggcgtggacaccgacgccgacatcgcccggacgctggcgatgttcgggggcttctcggaaggggttcagctgttcgcgtcgttcgccatgctgatgaacttcccgcgccagaacaagatgaagggcatgggccagatcgtgtcctggtcggtgcgcgacgagagcctgcactgcgaaggcgtcatcaagctgtaccacgccttcaacaaggagaccggcgccgtcaccaagaccgtcgccgacgacatcgtcgactgctgcaagaccgtggtggacatggaggacaagttcatcgacctggcctttgaaatgggttccgtcgacggcatgaccccgcacgacatcaagcagtacatccgcttcatcgccgactggcgcctgcgccagctgaagctgccggaggtgtacggggtgacggagaacccgctgccgtggctgcaggcgctgctgagcggggtcgagcacgccaacttcttcgaggcgcgcgccaccgaatactccaaggcggcgacccagggctcctggcacggcgccgacggtgtctggaccgagttcgaccgcatgatggctcgccgcgacatgagcctggtgatcggctgaacccaagccctccggcgacgacaaaaaaggcccggcgacgccgggcctttttcgtttcgatcggtggggcgctcagcgcgcggcggcgatcatccggtcgacctcggccaagtggcgctggacgatcggcacggtggccgtcgcggccgccttcagcgccggcgacgttccagcttccgaataggtcttctgcacgcccagcgcctctttgtgcgccatctgctgctgcgtcaggtacaggcggtcgcgctcgacgccctggaacatcttcagcgcattgaccatggcggcctgatgctgggccagcatcgccggcggcggggtcacgccgtcacggcgcgcggcggccatcgcgtcggtggtcgttttggtgtggtggtcgatcatcatctgggcgaagcggcggacctccgggttctgggtcgtctccagaaccgcctggctcgactggatctcgtacagatcaccaccgccggccagcatcaggaaatccatgggcgacggggcgggcgtcagggtgccggccggggtccagttgtaacgataggattgcggcgtggcctgagcggcggcggcgccggcggagagcagggcggcggcgcagacggcgccggcgatgagcttttgcatggatatcctcgttgttccggcagcagaacctcgccaaacgccgatagttccgcaggatggggcgtttggcctgcgccgtccgcgcgtctagggtccgctggtgaccgcacctaatcctatccccgtcgccttggtcggcttcggctacgccggagagacctttcacgctccgctgatcgccgcctgccccggcctgcgcctgcatacggttgtgtccagccgacccgagcaggtgcgggagagatggccgcaggtccgcgtcgtcgccgatctggacgaggcgctcgccgatgtgggggtcgaactggtggtgatcgccgcgcccaacgccgagcacgcgccgctcgcccgtcgcgcgctgaacgccggtcgggccgtggtggtcgacaagcccttcaccctgaccctggcggaggccaaggcgttggcgcagctgggcgagacgcgcggccgcctgttgtcggtgttccataatcgacgttgggacgccgacttcctgacgctgcagggattgatcgaggcgaaccggctgggccgcatcgtgcggttcgagagccgcttcaaccgctacaggccggaggtccgcgaccgctggcgcgaagcggacacgcccggcgcaggcgtgtggcacgacctaggtccgcacctgatcgaccaggcgctggcgctgtttggtgaacctctgggcgtgacggccgacctggcgatcctgcgccccggcggcaaggcctgcgactacgcccatgcggtcctccgctatccggacaagcgcgtcatccttcatgccgacatgctgagcgccgatcccgatccgcgcttcgtggttcagggaagccgcgcggcgttcgtcacccacgggctcgacccgcaggaagaccagctgaaggcgacgggtggagccggcggcgagggctggggcgtcgatcctcggccgggcgagatcatcgacggcgcgagcggcgagcgggaaccggccatgggcgtccccggcgactaccgccgctactacgacgggatcgccgccgccctgcgcggcgaggggcccaaccccgttccgccgctcgaggccgtggcggtgatgacggtgctggaggcggcgcggctcagcgcggagcgcggatgcgaagtgcgtctggacgcattgcacagccaagccggcgcggcgtaggcttcggtcatgatccttgcgacctcgtccggcgactatccgatcccaccggaggtggcgcgcgtcttgcccgacgtgcccagcccgccgcagcccggcgcgcccgacgcccgcgagcagatggaaagattccaggactggctggacgcctcgccgcagcacgccatcgattatgagcgcgtgcggcgctggcacctcgtgcaggacgaattggccgcagcggccaaggccgaacagcgtcccttcgtggtgacagcggacggcctggagtagccgggccatcggaacgagcgacggtttcccgcgattagaccgctgacctctttcagcgaaagtccgaactcatgatccagtccgtcggctacggcgccaaggccgcgcaagccaagctcgagcgcatcgaattcgaacgcgacgatcccaggcccaacgaggtggtgatcgaggtcctctacaccggcgtctgccactccgacattcaccaggtgaagaacgagtggaagaacaccgtctatcctgcatcccgggccacgagatcgtcggccgcatcaaatccgtgggttccgaggccggccgcttcaaagaaggcgacgtggtcggtgtgggctgcatgatcgacagctgccgtcagtgcgagccctgccagtcaggcgaccagaactactgcgccggccccaacagctggctggccacctacaatggtccgatgacccccaagggcatgacggaggacggctccaacatgtacggccgcgacaacaccttcggcggctattccgacgtggtggtggtgcccgaggacttcgtgctgcgcatccccgagggtctcgatcccaaggcggcggcgccgatcctgtgcgcgggcgtgaccaccttctcgccgatgaagcactggggcgtgaaggcgggcgacaaggtggcgatcctgggctttggcggcttgggccacatggcgctgaagctcgccaaggggctcggcgcggaggtgacggttctcacctccacgcccgagaagatcgagctggccaggtcgctgggcgcggacgccgcctatgtcgagaccgacaagacgtcgctgaccccgctcgccgcctcgttcgacatgatcctgtccaccgtgccggagaagcacgaggtgggtccgttgctggacctcctgaaacgcgacgccacctttgtggtggtcggcaacctcgacgtcatcgacggcgtggacaacatgaagctggccggctcacgccagagcgtggcgggctccctgatcggcaacctcaaggaaacgcaggacgtgctcgatttctgcgccgaaaagggcatcgcgcccgaggtcgaggtcatcgacatcaaggacatcaacgacgcctacaccaaggtcgagaacggcgaggtgcgcttccgctacgtcatcgacatggcgacgctggaggccgcctgatcccaggcgtcaccccggcagacgcagctcgaacaccgcgcccgccgggccgctctcgaccagcctgaggtcgccgccgtgcagggccgccagctcgcgcgagatggtcaggccgagccccgtgccctccgaggcgcgtccgctgacgaagggttcgaacagccgctcggccaggcgctgcgggatgcccggtccgtcgtcggcgatgcgcacgacgcagaagccttcctcgccgcgagcggtgaccgtgatgacgccgcgtccccgctgctcgggcgctcgggcggcatcgccttcgatggcctggcgggcgttgcgcatcagattgaccaggatgcggtgcagctggtcgccgtccgccatgaggccgaagcgggccggaacctcggcctccagccgcaccccgtcgggggtgagacccgcatcctcggccgcgccggcgagcgctgcgtccagcgccagccgcgtcttctgcggcggcggctcctcgctttttccgtactgcagcacattggccgtcagggccgcggctcggcccagcgcccgctccagccgaggcagcaccttggccacctgcgggtccggggatgcggccaggcgctcggacgtcatctgggccgaagccagcatgttgccgaggtcgtggttgatctttgccacggcctcgcccagcgcgacgaggcgcgcgcgcgagcgcagggattggcgcacctcctcctgcatccgcgccagctctcgctcgacccggccgatctcgtcatgccgatcggacggtgcgtccggctggctctcgggatcggccgcgaaatgctcgatggagcgggtcacgcgccggagggggcgcagcaccagcaacgccagacccaggtagagcagcgcccccgccgtcacggagatcagcagcgacaccaacaagctgttcagcagaaaggcgcgcagttcctgcttcagcggctcggccggcgtcacgatctcgatgaagtcgcccgaacgatagcgcggccgcgcctgcacccgcagcgaccgatcggggtgccccacgagcgtccgccacggatcggccagccgcgccaccgtgtcctggcggcgtagatcgatcagttcgggcgcgcgcggcagattgggggcttggagcaggaggcggcgccccccctcctccgtcagggccaccgcctgacccccgccgatccgcatcagctcggccgccgtgtcgtcctccacggcgctgtagggcagggcctcgacgcccacggacgccagctccgccgcctgcagccgatcctgcagccaccgctcatggaaggccgacgcgttgggcgcgacgatcagcacctccaccgccagggtgaagaacaccgtcagcagcagcagccgcgccgacagcccgtccggcttcagcccggcggcgacgcgctggaacagcgccctcacgccggctgcaccccacgccggccgcgcgccatctgcaccaggcggatgcccagcggcagcagcagcgacaggaacaccacccccatcagcggccagaagaactgatgcaacagcagatcgagatccggccgcacgccgcgtcgcaacagttcgcccaactccgagccgatccaggtgtagatggtggtggacggcaggaggcccacgaaggtggcgatcacatagggacgtatcggcacggccatcatgccggcggtggcgttgatcagcacgaacggcacgctggggatcagccgcagcgtcaacagggtggtgaaggcgttgcggtccagtcccttcgccagccggtccatcagcccggcgtccctggcgaacttggccctcagccatgtgccgatggaggtgcggtacacatagtagatgacgaccgagccgatggtggcgccggtcgcctgcgccagcgctccgacccacggcccgaacatcagcccgccgagcagggtcaggaacaccggccccggaatggtggaggcggtggccagtgcataaacgccgacaaaggccagaagcgcgatccacatgtgctcgcgcgcataggcctggagccccagcccatgctcgcggatcatgtccatcgacagccagcggttcaggcccagggcgaagaaggcgacgaccagcccggccacggcgatcagcggcaagagccgcagtccccattccctggccgatcgctgcatcataggatgttccgctcccccgaagattcccgcgcggcgttgactcgcgccgtcatgcgacttatacgcccgcccttcccgcgacggagcctttttgcccgccgctcaaccttttaacgtcaggagccgaccgtgaagcggacctatcagccgtcccgactcgtgcgcaagcgccgtcacggtttccgcgcgcggatggccaccaagaacggccagaagatcgttgcgcgccgccgcgccaagggccgcaagcgcctgacggcgtaagcgcccccgcgtccagatcaggacgcgcgtgagcgagaccctacagatcaagcgtctgctgcggcggccccagttcctggcggccgccaaaggcgtttccgacgcgcgtggcggcgtggtgatccagcgcctggaccgccgagacggccaggcgcacgtcggcctgggcttcaccgccacccgcaaaatcggcggcgccgtggtccgcaaccgctgcaaacgccgcttgcgcgaggccgcccgcgccctgttgcccctccacggcaaggcggggtgcgactatgtgttcatcgcgcgtatgggcacggcggagcgtgactgggaccgtttgcttgacgatgtgaaaaccgtccttacaaggctggcgagccccaaggacccggccgctcggccgcatggccgcccctccagcggcccggatgcccgaccccgatgaaaaacgagaactcgcgcaacacgatcatcttcatcgtggcgtcggccctgatcctgggcctgtactggttcaccgtcctgcgcccgcaggccgaggtgcgccgcgccaaccagctggccgccgccgaacagcagagcgaggcggccgccgatgcgcccaacaccgcgcttcggcccgagagcgccatcttcgtcaccgaccggacggaggcgctgggcgcaggcgcgcgcgtgccgatccagacgccgacgctgcgcggctccctgtcgctgcagggcggccgcatcgacgatctgttcctggtccgctaccgcgagacgctggacgccgacagccaaccggtcgagctgttccgtccgcagggcatggaacacgcctatttcgcccagttcggctggaccggccccaatgtcgcgggcggcgtgccggggccgaacaccccctggagcctgaccgccggctcgacgctgaccccgacctcgcccgtcaccctgacctgggacaacggccagggcctgcgcttcacccgcgtgatctccatcgacgaccagtacatgttcacggtcgccgacacggtgcagaacctggggacccagccgatcaccatcgcgccctacggctcggtccagcgccagggcgtgcccgccgatctcggcaagcagatgatcctgcacgagggcgccatcggcgtcttcggccagcccggccgctacgccaccgaccagtacaagtacaaggactggcagggcaaagcccgcatccaggagacctccaccggcggctggctgggcatcaccgacaaatactggatggccgcgctgatcccgccgcagaccgagcaggtctcggccgagttccgcgtccgtgatcccgaaggcgccaaccagcacgaggccaatgtgctgggcgccagccgcaccatccagccgggcgccagcgtcaccgagacccagcgcctgttcgccggggccaagcgcaacgagatcctgaagggctatgagcaggacctgaacctgccgcgcttcgtctacgccatcgactggggcatgttctggttcctgacccggcccatcttcatggtggtggagttcttcttccagctgctgggcaacttcggcctggccatcttggcgctgaccgtgctggtcaagctgctgctcttcccgctcgccaacaagagctacgagagcatgtccaagatgcgcaacctccagcccaagatggaggagatcaagaagaagttcggctccgacccgcagaagcagcagcaggagaccatggccctgtaccagcgcgagaagatcaatccggtcgccggctgcctgccgatcctgatccagatcccgatcttcttcgccctctacaaggtgctgttcgtcaccatcgagatgcgccaccagcccttcttcggctggatccgcgacctgtcggcgcgcgaccactcgaccatctggaacctgttcggcctcttgccgtacgacccggccgccgtgccgctgatcggcgccttcctgaacggcccggcgcatatcggccttctgccgatcctgtacgggatcaccatgtggctgcagcaggcgatgaacccggccgtgcccgatcccatgcagcgacgcatcttcgcgctgatgccggtggtgctggcttttgtgctggcgccctcgccggccggcgtcctgatctactgggtgtggagcaccatcctgtcgatcctgcagcagtacatcatcatgcatcgcttcggcgccgagaacccgatcgacagcttcatcgcccgcgtgaagtcgcccaagacgaaggccgcgtgaccgacttctccgaagacgagctggagcaggcccgcgtcctgttccagcgcccggcgacattcgtcatgggggccgccaagatcgagcaactgcccgatccggacctgcccgaggtcgccttcgccggccgttccaacgtcggcaagtccagcctgatcaacggcctggtcggcatgcacaagctggcgcgcgcctccaacgagccggggcgcacgcgagaggtcaacttcttcgacctggacggccgcatgcggctggtcgatcttcccggctacggcttcgccaaggcgtccaaggccgcgacgcgcaagttccaggacctggggcgcgactatctgcgcgggcgtgtgacgctgaagcgggtgtatctgctgatcgacagccgccatgggctgaagtcggtggacggcgaagcgctggacgcgctggatctcgccgccgtctcctatcagatcatcctgaccaaggccgacaagctcaagaagggcgagggcgaagcggtggcggcggcgacactgaaggccatcgctaagcgcccggcggcctttcccgccgttatcctgacctcgtccgaaaagggcgaaggcctgcccgagctgcgcgcggagatcatgcgcaccaccggggcgaccctgaactgaccccacagccgccccgaacaagaaaaaaggcccggagatcgctctccgggccttttctcatggtgtcggcggaccggccttattgggctccggcctgacgcacctcgaccggcaggcccagggcgtccagctgcggcttgaccacggaggcgtcgcccaccacgacccagacgaactgatcgggtttgatgacctcgcgggcggcggcatccatctcggccgccgtcagcgcgcgggtgcggctggccagcgtggcctgatagtcgtcgggacggcgatagagggcgttcgagcgtagcgcccccaggatctgcccggccgtctcatagctgccggccagcgaacgggtgttgccgttcagcgtccgctccagctcctgaggcgtcacgccgtcggtctgcaggaagcggtcgtactggctgatcagggcggcgatcgactcgccggtgcggttggcctgcaccggcgcgttgacgatgtagggcacgcgatgctccagcgcgttcaccccgccgcgcacgccgtaggaccagcccttggtctcgcgaaggtccgagttgatccgcgacaggaagtcggagcccagcgtcacattggccgcgttcagcgccaggaggtcgtccgtccccgacaccggcagcaccgcgccgccgtagatcagcgactgcggcgactgaggccggtcgatcaggacgatccggttggtcgacgccgggatcgtcgcggcgaagctcttggttcccttgggggtggacggcgcgcgccagtcgccgaaggcggtctccagctgcggcgtgatggtgctcagcggctggtcggacaccacgaagatggtggcgttgtccggccgcacccaggcgtcgtgctcggccaccagatcggcgcgggtcagggccttcagggtggcgtcgtcgcccgatcccgtaaacgagcgtccataggggctgtcggcgccgtacagcagcggcggcagggcgcgggcggcgatggcgccggggttggtccgctcgctggccagggccgacaggcgggcggcgcggatgcgctcgacctccgacggcgcgaacgccgggttgcggacgacgtccgacagcagcgcgagcgccggcgtcagattggcggacagggtcgacaggtcggcgctggtgcggtccatcgaggcgctgacgctgacggaggcgcctaggcgctcctcttcctcggccagctggttggcgttgcgggtggtggtgccttcgtccaggaggtccagcatcatggcgtgggcgccgagacggtcagcccggtcggcggcgtagccggcgtcgaactccaccgccatgcgcgtcaccggcacggtgtccacctgggcgtagaccacttgaacgccgttcgacagggtcgtgcgctcgaccgcggggaacttcaggtccggcacctcgccgatggtcggcatggggtcgcgagccacgcgctggatctcggcggccgggaccggggtcgcgcccgacggagccgcggcggcctcgacataggcctcgcgctcgcccggagcgatggtcatgtcgaacaccgggcgggtcagccagcgctgcatggcgtcgcggacctgcgccggggtcactgacgcatactgggccagctccttcttgtagtgctcggggtcgccggcgtacagctggccctcggccaggacgttggccttgccgttgacctgctccaggctctggatgcggccggagacgtagcgggtggcgacgcgggcgacttcttcctcggtcgggccgttcttgatgaagtcggcgaccagggtgtccagacggcggccgacggcggcggcgtcctcgcccggcttcacatcgaccgagatgtcgaagatgccgacgcggtggaactccgacagggaggacgacacgctcacggcgctctgctcgtcacgcaccagggtgttgtccagccgcgaggaggccagcccgcccaggacggcggcgccgaccgacagcggcacggcgtcgtcgctgagcatgccgggaaccgcccagctgcgcgtcagccgggtgttggcgacgcggtcgtgcatggttttgacgatgggcgccgacagggtcgggacgtcggcctgcgccggcgtgttcaccgggccgcgcgggatggcgccgaagtatttctgcatcagcggacgggcggtcgcctcgtcgatgtcgccggacagcaccacgatggcgttgttcgggccgtagttgtcacggaaccagttccgcaccgtctccaggctggcggcgtccagatcggccatcgagccgatggtggagtggcggtatgggtggccttcggggaacagcgcctcgagctgggcgtactcgaacaggccgtagggctggttgtcgccctggcgcttttcgttctgcaccacgccgcgctgcagatcgagcacctcctgcccgacctcgccgagcagatagcccatgcggtcgctttccaggaacagcgcctgctccagcgccggggtcggcacggtctggaagtagttggtgcggtcgaaccaagtggtgccgttcaggttggacgggcccaggttgcgcatgcggccgaggtaggagcccggcgcattctccgatccgccgaacatgagatgctcgaacaggtgggcgaagccggtggagccggcgggctcgtccttggagccgacattgtaccagaccgacaccgcgaccaccggggccttgcggtcctcgtgcacgatcacggtcaggccgttgtccaaggtgaacttggagtaggggatgtccacctggccgaccagcgccgagatcggagcggcggcctgcgccggcgcggcggggctggaggcctggacgggcgcggccgggctgaaggcccagactggcgtggtgggggccagcagggcggccagggcgacaaggggcgcgacgcgacgcatggggcgggttcctccggaaaacgttggagcgaaccttaaccgggcgacacacgcgcgcaacgccgtcgccacaaacatgaccaaagcttcatgttccacgatgtcgcagccgctaagagccgcggcgcgtccgcccgcgtcactctccctaatcaagtccctggtcgagcccgacggtgaccagcgcccctcccgcgctcaagccgcgagcgaccgcgtcgcgagcatagcgcccctaaatgtggatggcgtgtccgagcgcgcgcaggctggcctcatggaaggcttcgcccagcgtcgggtggacgtggatggttccggccacgtcctccagcaccgcgcccatctccagcatctgggcgaagctgttggacagttcggacacatgctgccccaccgcctgaatccccaacaggcggtgatcggtcttggatgcgatcacccgcacgaagccgccgtcctccccggcctcgatagccagggcccggccgatggcggcgaaggggaacaccgcggtgatcacatcgtcgcgcccttcgacatcggtcggcagcagcccggcggcggcgatctccggctcggtgaaacagacggcggcgatcgtggtcggatcgaacacgcggtcattgccggagatgatctcggccaccacctcgccctgggccgagcccttgtgggccagcatcggttcgccggtcaggtcgccgacggcccagacgttcttcatgctggtggcgcagcggttgtcgatcttcacgaacggcccggccatggccacgcccatgttttccagaccccagccctgggtgcgcggcctgcggccgacggtgaccagaaccttgtcggcgtccagttgcagcggctcgccgtccctggtcgtgatcgacaacttgccgtcgccgaagccgccggcgcgcgcgcccaggtgcagttcgacgccgtggctcgtcagccacctcgccaccggatcggtcagggccttgtcgtagagcggcaggatgcggtcggccatctcgacgatggcgacctccgcgccgagcttgcggaaggcgatgcccagctccagtccgatgtagccgccgccgacgacgaccagcttcttcggaacctccggcaggctcagcgcctcagtcgaggagatgacgtccccgccaaacggcaggaagggcagttcgaccggctccgaccccgtggccagaatgacgtgttcggcggtgatcctgatgtcgccgtcgtcgctcttgaccatgcaggtcttggcgtcttcgaaattcgcccagcccctgatcaccttgaccttggccttcttcagcagggccgcgacgccggcgttcagcttacggacgatcccgtccttccactccaccgtctgtttcaggtcgatggccggcttggccgccgtgatccccagcgttccgccgcccgccgccttggccaccgtctcgaacttgcccgccgcgtggatgatggccttggacggaatgcagccgacgttcaaacaggtgccgcccagcccgtccgagccatccaccagcaccgtctccagccccagctggccgcagcggatgccggcgacatagccgccggtgccggcgccgatgatcaggactttggtcttcaggatctgggtcatctcaatccgtcttttcttccctctcccgatgggagagggcttgagcgcgcggcggcgaagccgtcgttctggcgcgaaagggtgagggccgtgcgtctccggtaagacccgaccctcatccgcccgcttcgcggccaccttctcccagcgggagaaggaagagttctacatccacaacgtcgcgggatgctccagcaagcccttgatccgctgcacgaagaccgccgcatcatggccgtcgacgatgcggtggtcgaagctggaggacaggttcatcatcttgcgcacgaccatctgaccgtcgcggaccacgacccgttcggcgatcttgttggggccgacgatggcgacctcggggtggttgatgatcggggtgtggaccacaccgccgagcgtgcccagcgaggttatggtgatggtcgagccggacagttcctcgcgcttggccgagccgtccttggccgcgcccgagacgcgggcgatctcctgcgccgtatcatagggatcgcgcgcctcggcgtggcggacgaccggcaccatcaggccgttcggcgtctgggcggcgatgcccagatgcacggcgttgtgggtggtcaggacgccggcctcgtcgtcataggtcgcgttgatctgcggctggtcgcgcagggccaccacgatggcgcgcgccatgaagggcaggacgttgagcttgggctggtccttcgacttggtcgcgttcaggtgggcgcggagctcctccagcgcggtgacgtcgatctcctccacataggtgatgtgagggatgcgccggacgctttcggccatcttttccgcgatcttgcggcgcagtccgatgatgcggacctcggtggtcccctccgcgcgagcgtaggtcgagctcccgctcggagacggggcggcggacgccgccgctccacgcgacaggaagccgtccaggtcctcgtgggtgatgcggccggcggcgccggttccgggcacgaacaccagatcgacgcccaggtcgcgcgcccgattgcgcaccgcaggcgaggccagcggccgttctccggcggtgcggccggtgagggcgggagcggacttgcccccctcccccgctgcgcgggtactcccccccatgaggggagagctgacgcccgccttgaggtcgggggcgaccagcggaacgggagccggagcctgatcctgagcttgggtgggaggggccgcctggaccgacgccgccgccacgttgccggcgcctttcaccgcaaaggtgaccagcgggcctccgacgggcgaggccttgcccgcttcgccgtgcagggcgacgacgcggccggcgacgggcgaggtgatctccaccgtcgccttgtcggtcatgacgtccgccaggatctggtcctcctcgacgttgtcgccgacctggacgtgccaggccaccagctcggcctcggccgtgccttcgccgacgtcaggcagcttgaagacgtaggttccggcggcggctggggcgggctcaggggcggcgctcgacatcggcgccgctgacggggcctcttgcgcagggggaggcgcggacggggtggacaccgccggcgcggcgggcgcctcggcttcggcgttgcccgcaccctcgacctcgaactcgaccagcggtcctcgcacggggaccatcgcgcccggctcgccgtgcagggccgtgaccttgccggacacgggggcggtgatctccaccgtcgccttgtcggtcatgacgtcggcgacgatctggtcctcggacaccacgtcgccgaccttgacgtgccatcccaccagctcagcctcggccgtaccctcgcccacgtcgggcagcttgaagacgaaacgacccatctcagcgtcctccgctcatgacggatttcagggcgtcggccacgcgctgcggaccggggaaatactcccactcaaaggcgtgcgggtagggcgtgtcccagcccgtcacccgcgcgatcggcgcctccaggtggtagaagcagcgctcctgcaccagcgccgacagctcggcgccgaagccggaggtgcgcggcgcctcgtgcacgatgacgcagcggcccgtcttcttcaccgacgcttcaatggtctcgatgtccaacggcacaagcgtgcgtaggtcgatcacgtcggcgtcgacgccggcgtgctcggccccggccagcgacacccacaccatggtgccgtaagcgaggatggtgacgtcgccgccttccttcatcacccgcgccttgccgatcggctcgaggtgtttggcggtcggcacctgcgccagctcctgcgccttccacggcgagaccggcttctcgtgccagccgtcgaatgggccgttgtagaggcgcttgggctcgaagaagatcaccggatcgtcgtcctcgatcgccgaggtcaacaggcccttggcgtccagcggattggacgggatcaccaccttcaggcccgagatgtgggtgaacaggctctcagggctctggctatgcgtctggccgccgaagatgccgccgccatagggactgcggatggtcagcggcgaggtgaactgcccgcctgagcgatagcgcatcttggccgcttccgacacgatctggtcgtaggccggatagatgtagtcggcgaactggatctcgaccacgggacgcaggccgtaggcggccatgccgatggccgcgccgacgatgccggtctcggagatcggcgcatcgaagctgcgggtcaggccgtgcttctgctgcagcttgtcggtgacgcggaacacgccgccgaagtagccggcgtcctcgccgaagctgagaaccgtcggatcctcggccatcttgatgtccagggccgagttcagcgcctggatcatgttcatggcctgaacggcaggcgcgtcgccggtagtcgaggcgggcgcatggttctggtcggccatgtcgggctcgagcccgtcggtgcggtcggcctcggtgaaggtctggtccgtcatgttcaaacccccacttcgcggcgctgttcgaccaggcgccagtcctcggtggcgaacacctcttcgaacatggtcttcacactcgggcgcgactggcccagggtgccgatggcttcggattccttggcggcggcgcggacctgttcgaccgcgtctttcagcgcctcggcgtgccggtcgtcgtcccattcaccgatcacagtcaggtgctggcgcagccgctccagcggatcacccaaaggccaattctcgtgctcgtctcccgggcgatagcggctgggatcgtcagacgtcgaatgcggggcgccgcgataggtgaacagctcgatcaccgtcgcgccctggttggtgcgtgcgcgctcttccgcccaggcggtggccgcccagacagccaggaagtcgttgccgtcgacccgcagagccggcaggccatagccgatcgccttggacgcaaaggtggtctcaagtccccccgcaatgccctggaaggacgaaatggcccactggttgttgacgatattcaggatcgccggcgcccgatagacggaggcgaacgtcagggccgagtggaagtcgctttccgccgtggagccgtcgccgatccaggtgatggcgatcttgtcgtcgccgcgaatggcgctagccatcgcccaacccaccgcctgcgggtactgggtgcccaggttgcccgagatggtgaagaagccgaaatccttggccgaatacatgatcggcagctggcggcctttgatcgggtcggcggcgttggagtagatctggttcatcatggtcgccagcggatagtcgcgcgcgatcagaaggccctgctggcgataggtgggaaagcccatgtcctcgcggctcagcagcatgccctgcgccaccgcgatcgcctcctcgccggtgcacttcatgtagaagctggtcttgccctggcggtgggcgcggtgcatccggtcgtcgaacgcccgcgtcaggatcatggccttcagcccccggcgcagggtttcgggatccagcttgggatcccaggggccgacggcccgcccctcgtcgtccagcacccgcaccagccgaaaggcgtgatcgcgcatgtcatagggggcgctggacacctctgggcgttcgaccgcgccggcggggtcaagctgcagatggctgaagtccggcgcatcgccgggacgtcccgacggctccggcacgcgcaacgacagcggttgggtgttctttatggtcatcaagcccgtccggttgatccgtacgcgtttcctcaaaggtccagatagcatgtcacgcaaaagggcgcttgctcaatccaacctttgagaatacggatttggggtattttatttcgccataacaataaaaagtggaggaagcattggcggacgaactcgaccctatcgacgcccggatcctggacatcctgcaacaggacgcggggctgtccgtggcggaagtcgccgaccgcgtcggcctgtcggcctcgccctgctggcggcggatcaagcggctggaggactccggcatgatcaccaagcgggtgaccctgctgaacgcagccaagctgggtctcgacttcgaggtctacgccatcgtcaagctgatgctgccgtcatcggagaacctggacgtgttcgaggccgccgtgtcgggctggcccgaggtggttcaatgcgcgaccgtgacggggcgcgacgactatgtgctgcgggtcatcacctccgacatgcacgcctttgacctcttcctgcgcgaaaagctgctggcgctgggcatcgtttcggattgcgaaagccacatcgtcacccgtggggtgaagaacgtgaccgccctgcctcttggcatcgtgaccccgcacgtcggataatcgcgccctctttccgggagggaccaccatgatcgagatgatgatcgacgcgcgccgcaaggacctcggcggcttcgaggtcgggcgcgtgctgccgtttcacctgcgccgcatggtcgggccgttcatcttcctggaccagatgggaccggccgagttcgcgccgggcgccgacaacatcaatgtgcggccgcatccgcacatcggcctttcgaccctgacctatctgttcgagggcgaaatcctgcaccacgacaacaccggggccaaccaggcgatccggccgggcgaggtcaattggatgacggcgggcagcggcatcgtccattccgaacgcaccgacccgctgaagaaggccaggggcgggccgatgcatggcatgcaggcctggatcgccctgccggacgaggccgaggaggcggacccgtcctttcaccacttcggcgaggacgcccagccggcctatgacaacaagggcctgttcgcccggctggtcgcgggcgaggcctacggcgccaaggccgcggcgccgacccactcgcccctgttctacctgcattgggagctggcggagggggtgcgcaccgcgccgcctcccggccggagcttccgcaagtcgggcgacggctactccgagcgcgcgctttatgtcgccaagggccgcatcgaggtcggcgaccgggtcgtcgaggcgggtcagatggcggtgctggagccgaccgccgaacccaccgtcaaggcgctggagccctcgaccgtcatggccctgggcggagagccggtcggcgagcggctgatctggtggaacttcgtggcctcgtctcaagcgcgcatcgacgcggccaaggccgactggcgcgccggccgcatgcgcctgcccgacgccgaccatctcgagttcattccgctgccggaagagccggtccgcgcccagactccgccggagcccgccaagcctgagccgacccacccggtctgaccacgccgcgtttgcagccccgcgcccaaagcgataacgcctgcgatcatgaacttcgacttcgacgcccaggtcaccgccgccctgttcgaccgcacaggggccgtcttcgccctgggcgacgggtcggtgcgcttcgacgaccgtacggtggtccaggcgcatgacggcgcggcgctgtgcgcggccgttcatccctccggcgaaggcgtggtgaccggcggcgacgacggccaggtggtctggagccgacgcgatgcggacgcggtggtgctggcctcggcccggaaccagtggatcgacagcatcgacgcggcggccgcgtccggcctgatcgccttctccttcggccgcacgctggcggtgattgacgccaaggatcccgccttccgccgcgactttgttcatgagcgcaccgtctcgggcgtcgccttcgagcccaaggggcggcggatcgcgacctccacatacggcggggcagccctgtggtacgcgcggatcgaaaagcagcagccggtcctgatgaaatgggcgggctcgcacaccgccgtggccttttcgcccgacggcgcattcgtcgttaccaccatgcaggacaaccagctgcacggctggcggctgaaggacgccaagaacctgcgcatgggcggctatcccggcaaggtccgctcggtggcctttctgtcaaacggccagctgatggcgacctcgggcgcgcaaggggtggtgatgtggccgttcatcggctccaacggtccgatggggcgcgaggcgaccgagatcggctttgacgacaccactgtggtcaacctggtcgccggccgggccgatcacgggcgggtggcggcgggactgggcgacggccgtgtctgggtggccgctccggccgatcaggggctgcagttcgtcaaggccgacaagggcgcgccgatcacggccctggctctgagccccgccgccgcccgcgtcgcctgggccgatgaggacggccgcgccggcgtcgcggacgtcggctgacgtgaacgcgccggccgtccagtccaggcctcggcgctcctggcgacgagccgtcctgatcgccttcgccgtcctgtgtctgctgccgctaatcggcgtcctgctgcatgccgtggtcccgccgccgccgaccatcctgatgtggcagcgtgtcgtggcgggcgatgggctggactatcgctggcgaggcctgaacgacatctcgcccaatctggtcaacgccgccatcgccagcgaggacgcccgcttctgcagccacgcaggtttcgacatggaggcgatcgaacaggcgctggacaacaacgccgacggcggacgcatccggggcggatcgaccatcagccagcagaccgccaagaacgtcttcctgtggccccagcgcggctggatccgcaagggcctcgaggccggctacaccgtgctgatcgaaacagtgtggtccaagcggcggatcatggaggtctatctgaacgtcgccgagttcgcgccgggcgtgtacggcgccgaggccgcctctcgccgtctgttcggcaagagcgcgcgcgacctgaccccgcgcgaggcggcgcgcctggccgccgtcctgccggcgccgcgtcgctacaaggcggcgacgccgggtccttacgtgcgcagacgcaccgcccgcatccaggcggccgcgaacacggtgcgcaatcaagggctcagcgcctgcgtcctgcgcccacgcggatcggcttgacgcgaagcgccgcctcccgtctcctgcgaccgctcaaggagaaaaacaccatgaagcgtcagctgatggccgccgtcgcggtctgcgccctgtctttcaccgccggctgcgcctccacgacgccgcaaccgactgagcgttacgccgacggcggcgggccggccacgacacccctgctgcaggtcgcggccgccggcgcgacctatccggcgaccgccgaaggcgcggccgcctttgtcgccgacaccgaggcgaaatacgccgagcttagcgaatacgcctcgcgcgtcgcctggacgcgggccaccaacatcaccttcgacaccatgtggctggaggccaaggtcaacgccgagatgaccgagttcggcgtccaggccgccaacggcgccgcccgcttcaacgatgtggaagtggcccctgacgtccggcgcaagctgaacctgctgcgtcaggcgctggtgctgccggcgccgaaccggccgggcgccgccgacgagctggcccacatcaccacccggctggactcgacctactcgaccggcaagttcgactacaagggcgagccgatcaccctggacgaggcctcgctgatcctggccgacagccgcgatccggcggagacaaaggcgctgtacgagggctggcgcaccatctcgccggtgatgcaggccgactacgcccgcatggtcgccatcgccaacgagggcgcgcgcgagctgggctacgccgacaccggcgccctgtggcgctcgggctacgacatggcgccggacgccttcgccgccgaaaccgaccggctgtgggcgcaggtgaagccgttctacgagaacctgcactgctatgtgcgcggtcgattgaacgccaagtacggcgatgcggtccagccggaccagggtccaatccgcgccgacctgctcggcaacatgtggtcgcagcagtggggcaacatctatgacgtggtggccccggtgcagggcggccgctcgtcctatgacctgactgaactgctcaagaccgccgactacgacccgctgaagatggtcaagacgggcgagaacttctacgtctccatgggtatcgcgcccctgccgcagaccttctgggagcgcagccagatcacccggccgcgcgaccgcgaggtggtctgccacgcctcggcctgggatctcgacaacgccgacgacatccgcatcaagatgtgcaccaacgtcaatggcgacgacttctacaccgtgcatcacgaactggggcacaacgtctatcagcgcgcctacaagaaccagccgatgctgttccggaacggcgccaacgacggcttccacgaggccatcggcgacttcgtcggcctgtcggcgctgacccccacctatctgaaccagatcgggctgctgcagaccacgcccggcgcggaggaggacatccccttcctgctgaagatggccctggacaagatcgcctttctgccgttcggcctgatggtcgaccgctggcgctggggcgtgttctcgggcgagacgacgccggagcggtacaacgccgcctggaacgccgacatgctgcgctaccagggtctggtcccgcccggaccgcgccccgccgacgccttcgatcccggcgccaaataccacgtgccgggcaacacgccctacacccgctacttcctggcccacatctaccagttccagttccaccgcgcggcctgcaagcaggcgggatggaccggcccgctgcaccgctgctcgatctatgggaacaccgaggtcggccagcgcttcaacgccatgatggagatgggccagtcgcgcccgtggcccgaggcgatgcaggccttcaccggcgagacaacgaatgatgcatcggccatcgccgactatttcgcgccgctgaacacctggctgatccagcagaaccgcgggcgggactgcggctggtccgccgcctgacgcggaacatcgttcgttaaccttcgccggtagcggtttcttgaccgcgccggcgcatcctttcccagacgggcaagttgcgcccgatggggaagacgaccttggtcaacggccttttcacccgcctttgtcgcttcacccgccgcctaggcggaaacgagcgcggcaatgtggcgatgatcttcgccttcagcctgccggtgttggccatgatatcgctgggcggcatcgactatcagcgcgcctccaccgcccggtccaatctgcaggacgccctggatgcggcgaccctggcggcggcgcgcgcgcccaccaatgacgcaggcgcgctgaaccagatcggccgggcggcgctgagagccaacctggccgcttctcagaccggagccttcaacgacagcgacgccaccttcacgctggacgccaaccaggtcgtgatcgccgaggcgaccatgcaggtgaacaccctgatcgccaatgtggtgttgccgccttacggccggttctttgacgaccagttgccggtcaccgtgcactccgaggtcaaccgggcgtccaagaacatcgaggtggcgctggtcctcgacgtcacgggctccatgcgcggcagacggatcgccgatctgaaggatgcggccaggcagttggtcgaaatcgtcgttcaggacgagcaggaaccgttctactcccggatggccatcatcccctactcctccggcgtcaacctgaactcatcccggattggggctggcgactaccgcgccttggcgcgaggcgccccgcctgcgcccgtacgcatcaccaacgccgcctggatgacgggctcgtccatgcctgtcagcagcattaaccgttccagcggcacagtgaccgccaccagacatgggttcagcaagggcgactatgtctggctgcgcgacgtccgcgacatgaacggcttgaacaatcgggcgtaccgcgtcggagacgtcacccgagacaccttggagctgcagactttcaacggctcaaactggtttgacatcgacacgcgcagctactcccgaaacggctccagcggctcgctgagcaaatgcctgcttcgcgactgctttgtcgtcatcacggcgaacaaccaccgcatgcgagcgaccgatccggatacgggggacgccggctcagtttacatcgagggtgtgaatgggatggacatccagggcggctacgagatcgccaacgtcaccgcgaacacgttctccatcaataagagcggaccctttggctcgttcaggacaggcgccgaggccttctgcggcaacgacggctgcaagtaccgcgtcttccgcagcgtgaacgggagcctgcttgatcgcgagctgagcgactgcgtcaccgagcggacgggaggcgagcggtataccgagaccaccgcctccacggctcatgtcggtcgcctttatcccagcggctcgggagataacatgtgcacgcaatccagcgtcctgccgctcggccacaaccgcgacgacatgaacagcctgatcggcgtgtcgtccaatgtgtccagcgggttgcaggcgggcggcttcacggcaggtcacatcggcctggcctggggatggtacgcagtgtctcctgagttcgggtccttctggccgacggccccggcggcctatgacaccaatcgcacgctcaaggcggtcatcctgatgaccgacggcgagttcaacatgaaccattgctcgggcgtcatggcgcgcaactccgggggcggcggcgaccgcatcgactgcgacgcgccgaacgggtcatcgttcactcaagcgagagaactgtgcgcggccatgaaacggaagggcgtggttctttacacggtgggattccaggtttcctcgacgagctcagccggcaggttcctcagcgagtgcgccaccagcaacagccatgcctttattgcagcttccggggctgatctgtccgagtcgttcagggctatcggccgcgacatcacccgcctgcgcatctccaagtagggccggcggacacgccgtcagatcagccggatctcgcgcagccgctcggtcaggtaatcctcggccgtgatcgccttgccggcgtagcggtcgggattgtccggcgtcaccgcggacggcaggctctcgatccggaagtccggattgaaatgcaggaagaagggcgtggagtagcgcgcaaagccgcgcctctccggcgccgggttgaccacgcggtgggtcgtcgacggcaggatgtggttggtcagacgctgcagcatgtcgccgatgttgaccaccaaggcgccgggcggcggcgcgatgtctagccagctgccgtccttttccttcagctgaagcccggcctcctcggcgcccagcagcagggtgatgacgttgatgtcctcgtgcgcgccggcgcgcacgcccggcgcatccgccgggaccgggggatagtgcagcatgcgcaggacgctgttgcccatctcgaccttgtcgtcgaagaagtcgtcagccagcttcagatagcgggcgatggcgcgcaggatcttgcgccccagatcatccatggccgtaaacatgccgtacaggtgctcgcggaagccctccacctccgtgggccaaaggttgtcgcgcatgtagcgacgataggggtgcccctccggcagttcgcggccgacgtgccagaactccttcaggtccaccgccgccgcgcccttggccgcctcgacgccgaacggcgtcagccctcgggcgccgccggtcccgggcacgtgataccggcgcttgacctcttcgggcagggcgaaaaaggctttcgcatcgtcgatcgccgcctcgatcacctgctcgtccaggccgtgatcggctacgaccgcgaacccgtatcgctgaaacgaaacgccgaggtcgtcggaaaaacgctggaagtcgcgatcgtacagcgtcatcgatacgggctggatgcccgcagcggcggaagattgggtcacggcgtcggtccctgttcggagtctgccggctgcatacgcccaaagccgcggcttgtcaggtcgggggcgaccctgttcatcgacggtacaggtcggaaccttcacggtaagggcggcgtttttcccgccactgaaccaacaaggagccgcagccatgcgcaccccgttcgtctctcgcacggccataatcggcgtcagcatcgccgccctgatgggcgccgccgcctgcaccaccacagatccctacagctccgcgccgcagcgcaacaacaccggcacgggcgcgatcgccggcgccttgggcggcgccttgctcggctatctcacgaacaccaacaacagcgaggaaggccgcaagaacgccctgatcggcgcaggcatcggcgcgctgggtggcgcggccgtcggccagtacatggatcgccagcagcgcgcgctcgagaccgaactgtccggcaccggggtcggcgtggcgcgtcagggcgacaacctggtgctgcgcatgccctcggacgtgaccttcgccaccaatcagtcctcgatcgatcccggcttcaccccggtgctggacgatgtggcgcgcgtgctgcagcagtatgaccaatccaccgtggatatcatcgggcacaccgactcctccggcggagacgcgatcaaccagcccctgtccgagcgtcgcgcctccagcgtcgcgggcgagctggtgcggcgcggcgtcctggcggagcggctgttcgtcgccggcaatagctcccggaacccggtggcgtccaacgacacagcgcagggaaaggctcagaaccgtcgggtcgaaatcctgatccgcccgttccgcggctaagctccgcgattccgaagatggaggggggctgcgccaggcggagcccctttttcgtctcacaccgatccgtgacttgcgcctaggcgtccgccatgattccgctggctggaatggcgcatgagggcgggccgtgacgacgcgggcggatgatctccggcaggggctgaggctggcggcggttgcggtggcgtcggcggtgatcgcggccgcagcggtgatcggcgcgggcctgcggctggcgcccgccgaggcggaagcttcgcggctttcaacgacccggaagacagccagccccgcaccaccgcctcacgacgccccatactaagagccgcggcctgacgatcctgcgccgatcggctagatggggctcgcctgcctccggtggactgacgctctgttcgacgtgtcgacctcgaccgccgatcgacatccattcacgccaggctacgcaaaaggccgccgctcttttggagcgacggcctgatgttcgtcatcggttttcttgatccggttcgggagcgagagggccggcgggccggctctctcgtccctggctcgggtcttagaagttgatgtcgacggtggcgcgacggttcagcggttcgcgcacgccgtcggcggtggcgcgggccagctggggttcgccgcggccgtccagcgacaccacgccgcccgaca

(The sequence listing continues in the following parts.)